European Patent Application EP 4 700 135 A2, published February 25, 2026. Title: 24종 발진열증후군 기반 바이러스 및 세균 동시 검출용 포획 프로브 세트 및 이의 용도. Applicant: 질병관리청. The sequence listing filed with the application follows.

SEQUENCE LISTING (3828 sequences)

SEQ ID NO: 1 - DNA, 120 bp, synthetic construct
  source 1..120: mol_type = other DNA
accgagcgtatatccgtaatgaaagatactgaaacggcagaaagaataaaattcttctctttacactaacagcatagtacttgagatctggatactacacatgccgtgttatcagctttc

SEQ ID NO: 2 - DNA, 120 bp, synthetic construct
  source 1..120: mol_type = other DNA
ttacactaacagcatagtacttgagatctggatactacacatgccgtgttatcagctttctttgcagaattcttgagccaaccataagaataatttatcagcttataaagcttcacggcc

SEQ ID NO: 3 - DNA, 120 bp, synthetic construct
  source 1..120: mol_type = other DNA
tttgcagaattcttgagccaaccataagaataatttatcagcttataaagcttcacggccacacaacgggagatataactttgaggtcaaagaatcaagcatgcaattgccttaaacaac

SEQ ID NO: 4 - DNA, 120 bp, synthetic construct
  source 1..120: mol_type = other DNA
acacaacgggagatataactttgaggtcaaagaatcaagcatgcaattgccttaaacaactcgaataatcttcagttcatggcccaaagcattgcaaaatgcactacgctatctagcata

SEQ ID NO: 5 - DNA, 120 bp, synthetic construct
  source 1..120: mol_type = other DNA
tcgaataatcttcagttcatggcccaaagcattgcaaaatgcactacgctatctagcatattggatatacggagctaataaggccgttgacgaaaatgcatgtgtgcgtaacacacatgc

SEQ ID NO: 6 - DNA, 120 bp, synthetic construct
  source 1..120: mol_type = other DNA
ttggatatacggagctaataaggccgttgacgaaaatgcatgtgtgcgtaacacacatgcaagaaacttgccaatcccctccccagaattttgacgattgctgacagaacccgtatagaa

SEQ ID NO: 7 - DNA, 120 bp, synthetic construct
  source 1..120: mol_type = other DNA
aagaaacttgccaatcccctccccagaattttgacgattgctgacagaacccgtatagaaagaagcatacaagaaaccaatgatatcaccagctatgacccttacccaacaaatatcgct

SEQ ID NO: 8 - DNA, 120 bp, synthetic construct
  source 1..120: mol_type = other DNA
agaagcatacaagaaaccaatgatatcaccagctatgacccttacccaacaaatatcgctcatagtaacctgtgaaagcgatataaaagaaaataagtcacctatacccggaaggattgt

SEQ ID NO: 9 - DNA, 120 bp, synthetic construct
  source 1..120: mol_type = other DNA
catagtaacctgtgaaagcgatataaaagaaaataagtcacctatacccggaaggattgtcatatctcaaaaaacagtcctctttgatgtgatgtaaggttagcttatagcttagcggga

SEQ ID NO: 10 - DNA, 120 bp, synthetic construct
  source 1..120: mol_type = other DNA
catatctcaaaaaacagtcctctttgatgtgatgtaaggttagcttatagcttagcgggattggcaattttctctaaattgtcgttatttacgcactccagcttctttttccagcctacc

SEQ ID NO: 11 - DNA, 120 bp, synthetic construct
  source 1..120: mol_type = other DNA
ttggcaattttctctaaattgtcgttatttacgcactccagcttctttttccagcctaccgccattcatgaaattaaatagcacactatcagcaggtccatatcccacaaccacacctaa

SEQ ID NO: 12 - DNA, 120 bp, synthetic construct
  source 1..120: mol_type = other DNA
gccattcatgaaattaaatagcacactatcagcaggtccatatcccacaaccacacctaattcagtaagatctttccctacagctcgtatctttttcaaatcatcttctcccatagcagc

SEQ ID NO: 13 - DNA, 120 bp, synthetic construct
  source 1..120: mol_type = other DNA
ttcagtaagatctttccctacagctcgtatctttttcaaatcatcttctcccatagcagcagatacagaatctctcttattatccaagttctgaggaccacgctgcacttcccgactctt

SEQ ID NO: 14 - DNA, 120 bp, synthetic construct
  source 1..120: mol_type = other DNA
agatacagaatctctcttattatccaagttctgaggaccacgctgcacttcccgactcttggcattagcatggatatcctccttgtctgcccctgtatcaacagtgtgttctgcatgaga

SEQ ID NO: 15 - DNA, 120 bp, synthetic construct
  source 1..120: mol_type = other DNA
ggcattagcatggatatcctccttgtctgcccctgtatcaacagtgtgttctgcatgagattctgatatatctgaagctttccccttgattaagcttccataaagcctcgctgatgccgc

SEQ ID NO: 16 - DNA, 120 bp, synthetic construct
  source 1..120: mol_type = other DNA
ttctgatatatctgaagctttccccttgattaagcttccataaagcctcgctgatgccgcagtttctgcacgaaacttcgaagccttctctgaacactcggaaaaagcgctcattacgta

SEQ ID NO: 17 - DNA, 120 bp, synthetic construct
  source 1..120: mol_type = other DNA
agtttctgcacgaaacttcgaagccttctctgaacactcggaaaaagcgctcattacgtagtgctttaaaatcgtactttgaccgctacttgggtttaacattgcgtttaccgccagcgg

SEQ ID NO: 18 - DNA, 120 bp, synthetic construct
  source 1..120: mol_type = other DNA
gtgctttaaaatcgtactttgaccgctacttgggtttaacattgcgtttaccgccagcggcacggccttcaacgatgttcttacaaccgttcttacacaacctaagaaacacgataatgc

SEQ ID NO: 19 - DNA, 120 bp, synthetic construct
  source 1..120: mol_type = other DNA
cacggccttcaacgatgttcttacaaccgttcttacacaacctaagaaacacgataatgctgatgctaatctctcaaatccccgtaacacacttcctaaaaatacacaaaatagcgcaga

SEQ ID NO: 20 - DNA, 120 bp, synthetic construct
  source 1..120: mol_type = other DNA
tgatgctaatctctcaaatccccgtaacacacttcctaaaaatacacaaaatagcgcagatactcttgaagcacccgttacagtccccctatcccttgcaatagataaatgcctagcctt

SEQ ID NO: 21 - DNA, 120 bp, synthetic construct
  source 1..120: mol_type = other DNA
tactcttgaagcacccgttacagtccccctatcccttgcaatagataaatgcctagccttctcttcaaaatacgacgctcccttatttaaacccttcacaacaacatttagcgagctgtg

SEQ ID NO: 22 - DNA, 120 bp, synthetic construct
  source 1..120: mol_type = other DNA
ctcttcaaaatacgacgctcccttatttaaacccttcacaacaacatttagcgagctgtgaacaatcatagcagccacttctaacagcccagcacagaggttaaaaggaagcgcaataag

SEQ ID NO: 23 - DNA, 120 bp, synthetic construct
  source 1..120: mol_type = other DNA
aacaatcatagcagccacttctaacagcccagcacagaggttaaaaggaagcgcaataagcaatgtaggtaaccacatggtatcaccagtgacctcattcttaatacgccttgtctctgg

SEQ ID NO: 24 - DNA, 120 bp, synthetic construct
  source 1..120: mol_type = other DNA
caatgtaggtaaccacatggtatcaccagtgacctcattcttaatacgccttgtctctggatttacttcaggattacataccacgcgcatcaatctagggtccttatcactgctgcctat

SEQ ID NO: 25 - DNA, 120 bp, synthetic construct
  source 1..120: mol_type = other DNA
atttacttcaggattacataccacgcgcatcaatctagggtccttatcactgctgcctataggaacaactctataaccctcgcatgcgattactaatcttttgttcttataacgactagg

SEQ ID NO: 26 - DNA, 120 bp, synthetic construct
  source 1..120: mol_type = other DNA
aggaacaactctataaccctcgcatgcgattactaatcttttgttcttataacgactaggatttaaacccaagatcttgaatgcgtcttctgtttgattcgtattgatcgcatagagctg

SEQ ID NO: 27 - DNA, 120 bp, synthetic construct
  source 1..120: mol_type = other DNA
atttaaacccaagatcttgaatgcgtcttctgtttgattcgtattgatcgcatagagctgcttgttatcatgagtagtgacacgctccacgcccgtgtcagcaattggcattatcggaaa

SEQ ID NO: 28 - DNA, 120 bp, synthetic construct
  source 1..120: mol_type = other DNA
cttgttatcatgagtagtgacacgctccacgcccgtgtcagcaattggcattatcggaaaagtatgcccgtctacaacaagcaaacccttgttaacccacataccttcctgcttgataga

SEQ ID NO: 29 - DNA, 120 bp, synthetic construct
  source 1..120: mol_type = other DNA
agtatgcccgtctacaacaagcaaacccttgttaacccacataccttcctgcttgatagagctagtaggcaaaaacacacaaggctgttgcctgtcaacaacctgcgaaacaaccatcgg

SEQ ID NO: 30 - DNA, 120 bp, synthetic construct
  source 1..120: mol_type = other DNA
gctagtaggcaaaaacacacaaggctgttgcctgtcaacaacctgcgaaacaaccatcggtacctttattaacctagggcgcccaaagccttcaggatccaattgcgcaaacttcttcaa

SEQ ID NO: 31 - DNA, 120 bp, synthetic construct
  source 1..120: mol_type = other DNA
tacctttattaacctagggcgcccaaagccttcaggatccaattgcgcaaacttcttcaacggattcgctataaaaccaaacgtgctcttagcaccatccaccaacctactataattcct

SEQ ID NO: 32 - DNA, 120 bp, synthetic construct
  source 1..120: mol_type = other DNA
cggattcgctataaaaccaaacgtgctcttagcaccatccaccaacctactataattcctgccccttatgcgatctccgatcccagaaaaaaaaccagctaatctacctcttttactctc

SEQ ID NO: 33 - DNA, 120 bp, synthetic construct
  source 1..120: mol_type = other DNA
gccccttatgcgatctccgatcccagaaaaaaaaccagctaatctacctcttttactctcatccccgtacattgattctcaccatttataattttgatatgctataggaaaaatattaat

SEQ ID NO: 34 - DNA, 120 bp, synthetic construct
  source 1..120: mol_type = other DNA
atccccgtacattgattctcaccatttataattttgatatgctataggaaaaatattaattccttgctagagagaaaataatacatgcagctatagcgcaacacaagctcataacacccc

SEQ ID NO: 35 - DNA, 120 bp, synthetic construct
  source 1..120: mol_type = other DNA
tccttgctagagagaaaataatacatgcagctatagcgcaacacaagctcataacaccccaagagccactatggcgaaggaaagatccaactatcttttttgatataacataccaaaggc

SEQ ID NO: 36 - DNA, 120 bp, synthetic construct
  source 1..120: mol_type = other DNA
aagagccactatggcgaaggaaagatccaactatcttttttgatataacataccaaaggcgccttacgccataataaaggcagcttgacctacatacctagcgtatgcagcaacaccacc

SEQ ID NO: 37 - DNA, 120 bp, synthetic construct
  source 1..120: mol_type = other DNA
gccttacgccataataaaggcagcttgacctacatacctagcgtatgcagcaacaccaccaaagaaaatacacaaactgttagtacagcaaataattttatgaaagtaatcagaaaagct

SEQ ID NO: 38 - DNA, 120 bp, synthetic construct
  source 1..120: mol_type = other DNA
aaagaaaatacacaaactgttagtacagcaaataattttatgaaagtaatcagaaaagctcgtagcgcatcagagcgcacataatcctccaagacaacctgcacacccaaaacaccatga

SEQ ID NO: 39 - DNA, 120 bp, synthetic construct
  source 1..120: mol_type = other DNA
cgtagcgcatcagagcgcacataatcctccaagacaacctgcacacccaaaacaccatgataaaaagccggcatcaaaaataaagcagtcaatgcccccttgtacccatgcgttaaatct

SEQ ID NO: 40 - DNA, 120 bp, synthetic construct
  source 1..120: mol_type = other DNA
taaaaagccggcatcaaaaataaagcagtcaatgcccccttgtacccatgcgttaaatctagaagccccgtagcaaaatcagaaactaataacgccttcacaaggaatattggaaccggc

SEQ ID NO: 41 - DNA, 120 bp, synthetic construct
  source 1..120: mol_type = other DNA
agaagccccgtagcaaaatcagaaactaataacgccttcacaaggaatattggaaccggcagcattaccaccgcagtcatccgctgcatccaccagtgtaaaatactctttcctgacata

SEQ ID NO: 42 - DNA, 120 bp, synthetic construct
  source 1..120: mol_type = other DNA
agcattaccaccgcagtcatccgctgcatccaccagtgtaaaatactctttcctgacatatattaactgaagaaacctataaaacccagcccgatcaacgaggtcaccgcaaaacctaac

SEQ ID NO: 43 - DNA, 120 bp, synthetic construct
  source 1..120: mol_type = other DNA
tattaactgaagaaacctataaaacccagcccgatcaacgaggtcaccgcaaaacctaacatcaaccaaccactgaaagtagcctcagatttaccaaagccaattccgcaatcccagaat

SEQ ID NO: 44 - DNA, 120 bp, synthetic construct
  source 1..120: mol_type = other DNA
atcaaccaaccactgaaagtagcctcagatttaccaaagccaattccgcaatcccagaataaatgccgaatcccgttataatagtggtaacacagcgcagcaatacagccccctattatc

SEQ ID NO: 45 - DNA, 120 bp, synthetic construct
  source 1..120: mol_type = other DNA
aaatgccgaatcccgttataatagtggtaacacagcgcagcaatacagccccctattatcacctttaccaacagtacacctatccaggagtctaacaaaccccacagctgaccagatgtc

SEQ ID NO: 46 - DNA, 120 bp, synthetic construct
  source 1..120: mol_type = other DNA
acctttaccaacagtacacctatccaggagtctaacaaaccccacagctgaccagatgtccaatgtaaagaaatcaataaccatgtaaagagagtcagccccatcaatagcaggacacca

SEQ ID NO: 47 - DNA, 120 bp, synthetic construct
  source 1..120: mol_type = other DNA
caatgtaaagaaatcaataaccatgtaaagagagtcagccccatcaatagcaggacaccagtgattctgtgcgtaatcgatagccacgccgttatcggcagcttatagacactaagatgc

SEQ ID NO: 48 - DNA, 120 bp, synthetic construct
  source 1..120: mol_type = other DNA
gtgattctgtgcgtaatcgatagccacgccgttatcggcagcttatagacactaagatgcggagacagaggcctagacctcgacactatagtagcctccggttaattcacaatagaaata

SEQ ID NO: 49 - DNA, 120 bp, synthetic construct
  source 1..120: mol_type = other DNA
ggagacagaggcctagacctcgacactatagtagcctccggttaattcacaatagaaataaagacggcggcacatttaccgacaaactaccataagatagaatactcagtaaaaagccta

SEQ ID NO: 50 - DNA, 120 bp, synthetic construct
  source 1..120: mol_type = other DNA
aagacggcggcacatttaccgacaaactaccataagatagaatactcagtaaaaagcctaaaggaggtaatccagccgcaggttcacctacagctaccttgttacgacttcaccctagtc

SEQ ID NO: 51 - DNA, 120 bp, synthetic construct
  source 1..120: mol_type = other DNA
aaggaggtaatccagccgcaggttcacctacagctaccttgttacgacttcaccctagtcactgacccaaccttaaatggctgcctcctttcggttggcgcaccagcttcgagttaagcc

SEQ ID NO: 52 - DNA, 120 bp, synthetic construct
  source 1..120: mol_type = other DNA
actgacccaaccttaaatggctgcctcctttcggttggcgcaccagcttcgagttaagccaattcccatggcgtgacgggcagtgtgtacaagacccgagaacgtattcaccgtggcatg

SEQ ID NO: 53 - DNA, 120 bp, synthetic construct
  source 1..120: mol_type = other DNA
aattcccatggcgtgacgggcagtgtgtacaagacccgagaacgtattcaccgtggcatgctgatccacgattactagcgattccgacttcatgccctcgagttgcagaggacaatccga

SEQ ID NO: 54 - DNA, 120 bp, synthetic construct
  source 1..120: mol_type = other DNA
ctgatccacgattactagcgattccgacttcatgccctcgagttgcagaggacaatccgaactgagatgacttttacggattagctcagccttgcgacattgcaacctattgtagtcacc

SEQ ID NO: 55 - DNA, 120 bp, synthetic construct
  source 1..120: mol_type = other DNA
actgagatgacttttacggattagctcagccttgcgacattgcaacctattgtagtcaccattgtagcacgtgtgtagcccaccccataagggccgtgctgacttgacatcatccccacc

SEQ ID NO: 56 - DNA, 120 bp, synthetic construct
  source 1..120: mol_type = other DNA
attgtagcacgtgtgtagcccaccccataagggccgtgctgacttgacatcatccccaccttcctccagtttaccactggcagtttccttaaagtgcccggcttaacccgctggcaacta

SEQ ID NO: 57 - DNA, 120 bp, synthetic construct
  source 1..120: mol_type = other DNA
ttcctccagtttaccactggcagtttccttaaagtgcccggcttaacccgctggcaactaaggatgagggttacgctcgttgcgggacttaacccaacatctcacgacacgagctgacga

SEQ ID NO: 58 - DNA, 120 bp, synthetic construct
  source 1..120: mol_type = other DNA
aggatgagggttacgctcgttgcgggacttaacccaacatctcacgacacgagctgacgacagccatgcagcacctgtgcgagatccagccgaactgcgcccttccgttaagaaggatct

SEQ ID NO: 59 - DNA, 120 bp, synthetic construct
  source 1..120: mol_type = other DNA
cagccatgcagcacctgtgcgagatccagccgaactgcgcccttccgttaagaaggatctaatctccatgtcaaggagtggtaaggtttttcgcgttgcatcgaattaaaccacatgctc

SEQ ID NO: 60 - DNA, 120 bp, synthetic construct
  source 1..120: mol_type = other DNA
aatctccatgtcaaggagtggtaaggtttttcgcgttgcatcgaattaaaccacatgctccaccgcttgtgcgggtccccgtcaattcctttgagttttagtcttgcgaccgtagtcccc

SEQ ID NO: 61 - DNA, 120 bp, synthetic construct
  source 1..120: mol_type = other DNA
caccgcttgtgcgggtccccgtcaattcctttgagttttagtcttgcgaccgtagtccccaggcggagtgcttaacgcgttagctacaacacagagataaaaaatccccacattcagcac

SEQ ID NO: 62 - DNA, 120 bp, synthetic construct
  source 1..120: mol_type = other DNA
aggcggagtgcttaacgcgttagctacaacacagagataaaaaatccccacattcagcactcatcgtttacagcgtggactaccagggtatctaatcctgtttgctccccacgctttcgc

SEQ ID NO: 63 - DNA, 120 bp, synthetic construct
  source 1..120: mol_type = other DNA
tcatcgtttacagcgtggactaccagggtatctaatcctgtttgctccccacgctttcgcacctcagcgtcagtaccggaccagatagccgccttcgccactggtgttcctcctaatatc

SEQ ID NO: 64 - DNA, 120 bp, synthetic construct
  source 1..120: mol_type = other DNA
acctcagcgtcagtaccggaccagatagccgccttcgccactggtgttcctcctaatatctacgaatttcacctctacactaggaattccgctatcctctcccggactctagtctggcag

SEQ ID NO: 65 - DNA, 120 bp, synthetic construct
  source 1..120: mol_type = other DNA
tacgaatttcacctctacactaggaattccgctatcctctcccggactctagtctggcagtattaaaagcagctccagggttaagccctggcatttcacctttaacttaccgaaccgcct

SEQ ID NO: 66 - DNA, 120 bp, synthetic construct
  source 1..120: mol_type = other DNA
tattaaaagcagctccagggttaagccctggcatttcacctttaacttaccgaaccgcctacatgccctttacgcccaataattccgaacaacgcttgccccctccgtattaccgcggct

SEQ ID NO: 67 - DNA, 120 bp, synthetic construct
  source 1..120: mol_type = other DNA
acatgccctttacgcccaataattccgaacaacgcttgccccctccgtattaccgcggctgctggcacggagtttgccgggacttcttctgtaggtaccgtcattatcttccctactgaa

SEQ ID NO: 68 - DNA, 120 bp, synthetic construct
  source 1..120: mol_type = other DNA
gctggcacggagtttgccgggacttcttctgtaggtaccgtcattatcttccctactgaaagagttttacaaccctaaggccttcctcactcacgcggcatagctggatcaggcttgcgc

SEQ ID NO: 69 - DNA, 120 bp, synthetic construct
  source 1..120: mol_type = other DNA
agagttttacaaccctaaggccttcctcactcacgcggcatagctggatcaggcttgcgcccattgtccaatattccccactgctgcctcccgtaggagtctggaccgtatctcagttcc

SEQ ID NO: 70 - DNA, 120 bp, synthetic construct
  source 1..120: mol_type = other DNA
ccattgtccaatattccccactgctgcctcccgtaggagtctggaccgtatctcagttccagtgtggctgatcatcctctcagaccagctatagatcatcgccttggtaggcctttaccc

SEQ ID NO: 71 - DNA, 120 bp, synthetic construct
  source 1..120: mol_type = other DNA
agtgtggctgatcatcctctcagaccagctatagatcatcgccttggtaggcctttaccctaccaactagctaatctaacataggctcatctaatagcgataaatctttcccccgcaggg

SEQ ID NO: 72 - DNA, 120 bp, synthetic construct
  source 1..120: mol_type = other DNA
taccaactagctaatctaacataggctcatctaatagcgataaatctttcccccgcagggattatacagtattacccaccatttctagtggctatcccatactactaggtagattcctat

SEQ ID NO: 73 - DNA, 120 bp, synthetic construct
  source 1..120: mol_type = other DNA
attatacagtattacccaccatttctagtggctatcccatactactaggtagattcctatgcattactcacccgtctgccactaactattctttatagcaagctataaagaataatccgt

SEQ ID NO: 74 - DNA, 120 bp, synthetic construct
  source 1..120: mol_type = other DNA
gcattactcacccgtctgccactaactattctttatagcaagctataaagaataatccgttcgacttgcatgtgttaagcttgccgccagcgttcgttctgagccaggatcaaactctca

SEQ ID NO: 75 - DNA, 120 bp, synthetic construct
  source 1..120: mol_type = other DNA
tcgacttgcatgtgttaagcttgccgccagcgttcgttctgagccaggatcaaactctcaagtttgatttacaatcacaaaagcaaattatgatctggactcatgcaaaaaccaaaacaa

SEQ ID NO: 76 - DNA, 120 bp, synthetic construct
  source 1..120: mol_type = other DNA
agtttgatttacaatcacaaaagcaaattatgatctggactcatgcaaaaaccaaaacaaaatttaagcttaagtgcattaagaaaaaaatatattagctatatgcaccgccgcctttat

SEQ ID NO: 77 - DNA, 120 bp, synthetic construct
  source 1..120: mol_type = other DNA
aatttaagcttaagtgcattaagaaaaaaatatattagctatatgcaccgccgcctttatttctactctaaattctcatcaccaaactaatcaagcaccagagccatcaagctctgggca

SEQ ID NO: 78 - DNA, 120 bp, synthetic construct
  source 1..120: mol_type = other DNA
ttctactctaaattctcatcaccaaactaatcaagcaccagagccatcaagctctgggcaggagtatcagctatagcgcctgttatgtcaatagtttttcatatattttttttaaactcc

SEQ ID NO: 79 - DNA, 120 bp, synthetic construct
  source 1..120: mol_type = other DNA
ggagtatcagctatagcgcctgttatgtcaatagtttttcatatattttttttaaactccatcacactacatcaatacaaacattgtcttttgccgctaacttactgataatctccaaga

SEQ ID NO: 80 - DNA, 120 bp, synthetic construct
  source 1..120: mol_type = other DNA
atcacactacatcaatacaaacattgtcttttgccgctaacttactgataatctccaagaaatttctcgcttgttcatctatcattcccttgataaatacttcttctctagaagcaatgc

SEQ ID NO: 81 - DNA, 120 bp, synthetic construct
  source 1..120: mol_type = other DNA
aatttctcgcttgttcatctatcattcccttgataaatacttcttctctagaagcaatgcccaatattaaaaaaggaataactgatttatgctcctcgcgaacttctataatgcaaccct

SEQ ID NO: 82 - DNA, 120 bp, synthetic construct
  source 1..120: mol_type = other DNA
ccaatattaaaaaaggaataactgatttatgctcctcgcgaacttctataatgcaaccctcagaaagcgtatctctcctaccatgaatttctaaatgatctgcggtaacttttgaaatga

SEQ ID NO: 83 - DNA, 120 bp, synthetic construct
  source 1..120: mol_type = other DNA
cagaaagcgtatctctcctaccatgaatttctaaatgatctgcggtaacttttgaaatgatcccaaacttatcaagtgcaattaacaatgcattgagtatttttctcttagattcacaca

SEQ ID NO: 84 - DNA, 120 bp, synthetic construct
  source 1..120: mol_type = other DNA
tcccaaacttatcaagtgcaattaacaatgcattgagtatttttctcttagattcacacaattttgacaggccaaagaattttgtgactcctgcagcaaatacactcacaacacatataa

SEQ ID NO: 85 - DNA, 120 bp, synthetic construct
  source 1..120: mol_type = other DNA
attttgacaggccaaagaattttgtgactcctgcagcaaatacactcacaacacatataagtggaaggtacgaaaaaatacgctgtatctcctggctttgaatttcaatacccagcatat

SEQ ID NO: 86 - DNA, 120 bp, synthetic construct
  source 1..120: mol_type = other DNA
gtggaaggtacgaaaaaatacgctgtatctcctggctttgaatttcaatacccagcatattgctaaatcccacatcgattttgtataaatggctagattgtgctgatagacggattctcc

SEQ ID NO: 87 - DNA, 120 bp, synthetic construct
  source 1..120: mol_type = other DNA
tgctaaatcccacatcgattttgtataaatggctagattgtgctgatagacggattctccctcccattctgataagaatatccagaaagctcttagtggttttatcgagcaaaacccccg

SEQ ID NO: 88 - DNA, 120 bp, synthetic construct
  source 1..120: mol_type = other DNA
ctcccattctgataagaatatccagaaagctcttagtggttttatcgagcaaaacccccgtaatagttatggctgaaccccgtaaaaccaatgccattgctacaagatgtagcactccta

SEQ ID NO: 89 - DNA, 120 bp, synthetic construct
  source 1..120: mol_type = other DNA
taatagttatggctgaaccccgtaaaaccaatgccattgctacaagatgtagcactcctactgacgaggcgggtattaccacagtttttgcataaagctctttctgtcccattattgtta

SEQ ID NO: 90 - DNA, 120 bp, synthetic construct
  source 1..120: mol_type = other DNA
ctgacgaggcgggtattaccacagtttttgcataaagctctttctgtcccattattgttatttcatcaatatttggcctcgtaaccactgatatatctgcaccaaagtgctttaatagtg

SEQ ID NO: 91 - DNA, 120 bp, synthetic construct
  source 1..120: mol_type = other DNA
tttcatcaatatttggcctcgtaaccactgatatatctgcaccaaagtgctttaatagtgtttctccagtgggggataaagaactgtcagaatatatacaatttttgcctgctatattca

SEQ ID NO: 92 - DNA, 120 bp, synthetic construct
  source 1..120: mol_type = other DNA
tttctccagtgggggataaagaactgtcagaatatatacaatttttgcctgctatattcatgctactcagcatcaaagccgttttgataacattggaggaaattacttctttctcttcta

SEQ ID NO: 93 - DNA, 120 bp, synthetic construct
  source 1..120: mol_type = other DNA
tgctactcagcatcaaagccgttttgataacattggaggaaattacttctttctcttctataggtaatgcgcaatcactaccctcaaccatcactggaaaggcttcactacgtatgaaac

SEQ ID NO: 94 - DNA, 120 bp, synthetic construct
  source 1..120: mol_type = other DNA
taggtaatgcgcaatcactaccctcaaccatcactggaaaggcttcactacgtatgaaactgcatcctgaagccttcaatatcctaatcgcttcgtatatctcagcaaaatctaagcctg

SEQ ID NO: 95 - DNA, 120 bp, synthetic construct
  source 1..120: mol_type = other DNA
tgcatcctgaagccttcaatatcctaatcgcttcgtatatctcagcaaaatctaagcctgatacctccacgcttgcatcatgggcattactattaaaaaaaagcgaagaaaatgcatgag

SEQ ID NO: 96 - DNA, 120 bp, synthetic construct
  source 1..120: mol_type = other DNA
atacctccacgcttgcatcatgggcattactattaaaaaaaagcgaagaaaatgcatgagttgataaaatgcccagcatagtaacggctatgatcgtatagtgtccaacgtctatacctc

SEQ ID NO: 97 - DNA, 120 bp, synthetic construct
  source 1..120: mol_type = other DNA
ttgataaaatgcccagcatagtaacggctatgatcgtatagtgtccaacgtctatacctccctcgggattcgaaaaaccaccaatacctactccttcaaccgaaacacagccttcctcta

SEQ ID NO: 98 - DNA, 120 bp, synthetic construct
  source 1..120: mol_type = other DNA
cctcgggattcgaaaaaccaccaatacctactccttcaaccgaaacacagccttcctctacgaaaacccgaacacccaaagatctcaaaatatcaatgacacgtgaaatcatcctatttt

SEQ ID NO: 99 - DNA, 120 bp, synthetic construct
  source 1..120: mol_type = other DNA
cgaaaacccgaacacccaaagatctcaaaatatcaatgacacgtgaaatcatcctatttttgctcacaccgtaaatttttgatgtacctacggcttgagctgcaataattaatgctgtac

SEQ ID NO: 100 - DNA, 120 bp, synthetic construct
  source 1..120: mol_type = other DNA
tgctcacaccgtaaatttttgatgtacctacggcttgagctgcaataattaatgctgtacaagatgcagtttcacacctagcaacatttgctataccccttaacacaaagccattatcga

SEQ ID NO: 101 - DNA, 120 bp, synthetic construct
  source 1..120: mol_type = other DNA
aagatgcagtttcacacctagcaacatttgctataccccttaacacaaagccattatcgagcatactatgagtagagggactcagcttatacgtgcaatatttcacctctgtacacccca

SEQ ID NO: 102 - DNA, 120 bp, synthetic construct
  source 1..120: mol_type = other DNA
gcatactatgagtagagggactcagcttatacgtgcaatatttcacctctgtacaccccatttttcatcacaccccacagttccttaacgtcgtatctattcgattcatgtacaccttct

SEQ ID NO: 103 - DNA, 120 bp, synthetic construct
  source 1..120: mol_type = other DNA
tttttcatcacaccccacagttccttaacgtcgtatctattcgattcatgtacaccttctcgtgccatagcatacgtatagacacctcagtgatgtaaattaactactattatctaagta

SEQ ID NO: 104 - DNA, 120 bp, synthetic construct
  source 1..120: mol_type = other DNA
cgtgccatagcatacgtatagacacctcagtgatgtaaattaactactattatctaagtatacccactaaccattacaaccgtaactcagatcttgttcaggattcgcaaatgctgaaca

SEQ ID NO: 105 - DNA, 120 bp, synthetic construct
  source 1..120: mol_type = other DNA
tacccactaaccattacaaccgtaactcagatcttgttcaggattcgcaaatgctgaacactctagggtttcgtactatagatatccacggtgattgatggtaatgtcatcgacccagct

SEQ ID NO: 106 - DNA, 120 bp, synthetic construct
  source 1..120: mol_type = other DNA
ctctagggtttcgtactatagatatccacggtgattgatggtaatgtcatcgacccagctgatattgaaaatctgggccaatatttccggtgtcaccaaaaaagcccccggaagttttat

SEQ ID NO: 107 - DNA, 120 bp, synthetic construct
  source 1..120: mol_type = other DNA
gatattgaaaatctgggccaatatttccggtgtcaccaaaaaagcccccggaagttttatcagaacaagatgccccttggacaaaagctctatatacacttccgctcccattgcatcccg

SEQ ID NO: 108 - DNA, 120 bp, synthetic construct
  source 1..120: mol_type = other DNA
cagaacaagatgccccttggacaaaagctctatatacacttccgctcccattgcatcccgttttaacacttcctgtaacatatgtgctatcagagtgttttgccctgtatgtatcgcaat

SEQ ID NO: 109 - DNA, 120 bp, synthetic construct
  source 1..120: mol_type = other DNA
ttttaacacttcctgtaacatatgtgctatcagagtgttttgccctgtatgtatcgcaatgcttcttaccctgcgcatcatcaaggagatgctctcatggaaattacatatgtttctgcc

SEQ ID NO: 110 - DNA, 120 bp, synthetic construct
  source 1..120: mol_type = other DNA
gcttcttaccctgcgcatcatcaaggagatgctctcatggaaattacatatgtttctgcccactaacctacccttagacgcattgtaatccatgtctatcatgacagggacaccactgtt

SEQ ID NO: 111 - DNA, 120 bp, synthetic construct
  source 1..120: mol_type = other DNA
cactaacctacccttagacgcattgtaatccatgtctatcatgacagggacaccactgttaaataaatctctgttttcttcgatagtcttactattataaaatgctacgtcattaacccc

SEQ ID NO: 112 - DNA, 120 bp, synthetic construct
  source 1..120: mol_type = other DNA
aaataaatctctgttttcttcgatagtcttactattataaaatgctacgtcattaaccccgtgtggatccgatacccttacaattgcaaatctctccttatttgcagagcgcattttaac

SEQ ID NO: 113 - DNA, 120 bp, synthetic construct
  source 1..120: mol_type = other DNA
gtgtggatccgatacccttacaattgcaaatctctccttatttgcagagcgcattttaacactcgacactaccccagctcgttttgtcacaccagattctttctcttcttgcgtgctact

SEQ ID NO: 114 - DNA, 120 bp, synthetic construct
  source 1..120: mol_type = other DNA
actcgacactaccccagctcgttttgtcacaccagattctttctcttcttgcgtgctactcacaaaccttactccgaatttgcctaacacctgctcgtacttactcaaaggatggtacct

SEQ ID NO: 115 - DNA, 120 bp, synthetic construct
  source 1..120: mol_type = other DNA
cacaaaccttactccgaatttgcctaacacctgctcgtacttactcaaaggatggtaccttaggtaaaagcctatggtcgcaaattcatgctctattttctcatcttccgtccagtcatc

SEQ ID NO: 116 - DNA, 120 bp, synthetic construct
  source 1..120: mol_type = other DNA
taggtaaaagcctatggtcgcaaattcatgctctattttctcatcttccgtccagtcatctacttcttccagttgcccttcttctttttcactaaaaagactgaactggtgcgcatccat

SEQ ID NO: 117 - DNA, 120 bp, synthetic construct
  source 1..120: mol_type = other DNA
tacttcttccagttgcccttcttctttttcactaaaaagactgaactggtgcgcatccatgctcacctttttgttttcaataatgttcagtattatgcccaatgacgcaaaaagctgcct

SEQ ID NO: 118 - DNA, 120 bp, synthetic construct
  source 1..120: mol_type = other DNA
gctcacctttttgttttcaataatgttcagtattatgcccaatgacgcaaaaagctgcctacgattaggatgtatgccgtctagcgatccggatttaattaaactttctagagtcctctt

SEQ ID NO: 119 - DNA, 120 bp, synthetic construct
  source 1..120: mol_type = other DNA
acgattaggatgtatgccgtctagcgatccggatttaattaaactttctagagtcctctttaaaggagatcgtatcctgacgttacccgcgaaatcccagatatcactatatcgaccacc

SEQ ID NO: 120 - DNA, 120 bp, synthetic construct
  source 1..120: mol_type = other DNA
taaaggagatcgtatcctgacgttacccgcgaaatcccagatatcactatatcgaccaccttcaacaggtagtatctcatgcgccgttaattgacctacattttttaaggctcccaatcc

SEQ ID NO: 121 - DNA, 120 bp, synthetic construct
  source 1..120: mol_type = other DNA
ttcaacaggtagtatctcatgcgccgttaattgacctacattttttaaggctcccaatccatatctaatcgaattccctgatacggtaaattctgcactagataaattaatatcaggcgg

SEQ ID NO: 122 - DNA, 120 bp, synthetic construct
  source 1..120: mol_type = other DNA
atatctaatcgaattccctgatacggtaaattctgcactagataaattaatatcaggcggcattacatctatgccacacatttttgcttgttggcaaagcaaacccagtttgtctttatc

SEQ ID NO: 123 - DNA, 120 bp, synthetic construct
  source 1..120: mol_type = other DNA
cattacatctatgccacacatttttgcttgttggcaaagcaaacccagtttgtctttatcatcgatatctaagttcatggaggcagtaaagaactcctttgtgtaatttgcgcgcaagta

SEQ ID NO: 124 - DNA, 120 bp, synthetic construct
  source 1..120: mol_type = other DNA
atcgatatctaagttcatggaggcagtaaagaactcctttgtgtaatttgcgcgcaagtacgctgtctgaaagcttattaacgcgtacgcagcagcatgcgatttattaaaaccataccc

SEQ ID NO: 125 - DNA, 120 bp, synthetic construct
  source 1..120: mol_type = other DNA
taagttcatggaggcagtaaagaactcctttgtgtaatttgcgcgcaagtacgctgtctgaaagcttattaacgcgtacgcagcagcatgcgatttattaaaaccataccctgcaaattt

SEQ ID NO: 126 - DNA, 120 bp, synthetic construct
  source 1..120: mol_type = other DNA
tggtaaaaggaagaattcattctgtagagtcttgtggtactgttgatggcccaggaattcgttatgtcatatttacacaagggtgtttattacgttgtcaatattgtcataatgctgata

SEQ ID NO: 127 - DNA, 120 bp, synthetic construct
  source 1..120: mol_type = other DNA
gttatgtcatatttacacaagggtgtttattacgttgtcaatattgtcataatgctgatacgtgggagatcggtaaaggaaaagaaataacagtcgaagaagtaatgcaggatgtgacat

SEQ ID NO: 128 - DNA, 120 bp, synthetic construct
  source 1..120: mol_type = other DNA
cgtgggagatcggtaaaggaaaagaaataacagtcgaagaagtaatgcaggatgtgacatgttaccttccttttattgaagcttccggaggcggtataacagttagtggtggggagccat

SEQ ID NO: 129 - DNA, 120 bp, synthetic construct
  source 1..120: mol_type = other DNA
gttaccttccttttattgaagcttccggaggcggtataacagttagtggtggggagccattattacagctagatttcttaattgaattatttaagaaatgtaaggaaattggaattcata

SEQ ID NO: 130 - DNA, 120 bp, synthetic construct
  source 1..120: mol_type = other DNA
tattacagctagatttcttaattgaattatttaagaaatgtaaggaaattggaattcatacaacaattgattcttcgggtgggtgttattctgaagaaacagaattccaaaataagctag

SEQ ID NO: 131 - DNA, 120 bp, synthetic construct
  source 1..120: mol_type = other DNA
caacaattgattcttcgggtgggtgttattctgaagaaacagaattccaaaataagctagacattttaatggagtacacagatttagttttattggatttgaaacatattgattcaaaga

SEQ ID NO: 132 - DNA, 120 bp, synthetic construct
  source 1..120: mol_type = other DNA
acattttaatggagtacacagatttagttttattggatttgaaacatattgattcaaagaaacatcgtaaattaacaggaaaaccaaatgaacatattttacaatttgctcgttatttat

SEQ ID NO: 133 - DNA, 120 bp, synthetic construct
  source 1..120: mol_type = other DNA
aacatcgtaaattaacaggaaaaccaaatgaacatattttacaatttgctcgttatttatcggataaaaataaaccgatttgggtacgacatgtattagttcctggtgttactgataatg

SEQ ID NO: 134 - DNA, 120 bp, synthetic construct
  source 1..120: mol_type = other DNA
cggataaaaataaaccgatttgggtacgacatgtattagttcctggtgttactgataatgaagaggatctacaaaagttatctagctttattcaaagtctgtctaatgttcaaaaaattg

SEQ ID NO: 135 - DNA, 120 bp, synthetic construct
  source 1..120: mol_type = other DNA
aagaggatctacaaaagttatctagctttattcaaagtctgtctaatgttcaaaaaattgaagtgttaccatatcataagcttggtgtatataaatgggaggcacttggacataagtatc

SEQ ID NO: 136 - DNA, 120 bp, synthetic construct
  source 1..120: mol_type = other DNA
aagtgttaccatatcataagcttggtgtatataaatgggaggcacttggacataagtatccacttgcgaatgtagaaccacctactgaaaaaaatgtagaacaagcaagacatattttac

SEQ ID NO: 137 - DNA, 120 bp, synthetic construct
  source 1..120: mol_type = other DNA
cacttgcgaatgtagaaccacctactgaaaaaaatgtagaacaagcaagacatattttacaagcagtctaatccaaatattggattagactttttgctttctttacaataaaacctagag

SEQ ID NO: 138 - DNA, 120 bp, synthetic construct
  source 1..120: mol_type = other DNA
aagcagtctaatccaaatattggattagactttttgctttctttacaataaaacctagagtatatatagagaaaagagtatactaaaaatagaatatccatatttttgtaaggaataagt

SEQ ID NO: 139 - DNA, 120 bp, synthetic construct
  source 1..120: mol_type = other DNA
tatatatagagaaaagagtatactaaaaatagaatatccatatttttgtaaggaataagtggagaaatttacataattgtaaagggaaatcaaaatagtaaaaagaattaagaagtaaaa

SEQ ID NO: 140 - DNA, 120 bp, synthetic construct
  source 1..120: mol_type = other DNA
ggagaaatttacataattgtaaagggaaatcaaaatagtaaaaagaattaagaagtaaaagagtgagtatcatggaatagagaacatttgtaagttattgcgaaagctcttataggaaag

SEQ ID NO: 141 - DNA, 120 bp, synthetic construct
  source 1..120: mol_type = other DNA
gagtgagtatcatggaatagagaacatttgtaagttattgcgaaagctcttataggaaagtataatgtaaagatatgagcacagataggattaaggggtcaatcttatatgctttgcata

SEQ ID NO: 142 - DNA, 120 bp, synthetic construct
  source 1..120: mol_type = other DNA
tataatgtaaagatatgagcacagataggattaaggggtcaatcttatatgctttgcatatccacgacaggtacatagctgaaagagaaatattagagtctgtttatgtaatttttaagg

SEQ ID NO: 143 - DNA, 120 bp, synthetic construct
  source 1..120: mol_type = other DNA
tccacgacaggtacatagctgaaagagaaatattagagtctgtttatgtaatttttaaggaaaatgtttttcctattgtcgtatatgcaatatggagaaacaataagctaggagtggatt

SEQ ID NO: 144 - DNA, 120 bp, synthetic construct
  source 1..120: mol_type = other DNA
aaaatgtttttcctattgtcgtatatgcaatatggagaaacaataagctaggagtggatttgtttgataaaaaaccccaaggttttaatattaactgcacattacggtaacggtcatgtg

SEQ ID NO: 145 - DNA, 120 bp, synthetic construct
  source 1..120: mol_type = other DNA
tgtttgataaaaaaccccaaggttttaatattaactgcacattacggtaacggtcatgtgcaagtagcgaaaacattagaacaaacatttcgccaaaaaggaattaaagatgtaattgta

SEQ ID NO: 146 - DNA, 120 bp, synthetic construct
  source 1..120: mol_type = other DNA
caagtagcgaaaacattagaacaaacatttcgccaaaaaggaattaaagatgtaattgtatgcgatttgttcggagaatcacatccggttataaccgatattacaaaatatttatattta

SEQ ID NO: 147 - DNA, 120 bp, synthetic construct
  source 1..120: mol_type = other DNA
tgcgatttgttcggagaatcacatccggttataaccgatattacaaaatatttatatttaaaaagttatacaataggaaaagaattatatcgcttgttttattatggcgtagaaaaaatt

SEQ ID NO: 148 - DNA, 120 bp, synthetic construct
  source 1..120: mol_type = other DNA
aaaagttatacaataggaaaagaattatatcgcttgttttattatggcgtagaaaaaatttatgataaaaaaatagcatcttggtatgcgaattttggaagaaaacgcttgaaattactt

SEQ ID NO: 149 - DNA, 120 bp, synthetic construct
  source 1..120: mol_type = other DNA
tatgataaaaaaatagcatcttggtatgcgaattttggaagaaaacgcttgaaattacttttacaagcagagaaaccggatattgttattaatacctttccgattatagctgtaccagaa

SEQ ID NO: 150 - DNA, 120 bp, synthetic construct
  source 1..120: mol_type = other DNA
ttacaagcagagaaaccggatattgttattaatacctttccgattatagctgtaccagaattaaaaaagcaaacaggtatttcaattcctgtgtataacgtattaacggatttttgtgtg

SEQ ID NO: 151 - DNA, 120 bp, synthetic construct
  source 1..120: mol_type = other DNA
ttaaaaaagcaaacaggtatttcaattcctgtgtataacgtattaacggatttttgtgtgcacaaaatatggattcatcgggaagtagatcgttattttgtagcaactgatcacgtaaaa

SEQ ID NO: 152 - DNA, 120 bp, synthetic construct
  source 1..120: mol_type = other DNA
cacaaaatatggattcatcgggaagtagatcgttattttgtagcaactgatcacgtaaaaaaagttatggttgatatcggtgtgcctgcggagcaaattgttgaaaccggaattccgatt

SEQ ID NO: 153 - DNA, 120 bp, synthetic construct
  source 1..120: mol_type = other DNA
aaagttatggttgatatcggtgtgcctgcggagcaaattgttgaaaccggaattccgattcgtagtagttttgagttaaagatcaatccagacattatatataataaatatcagttatgt

SEQ ID NO: 154 - DNA, 120 bp, synthetic construct
  source 1..120: mol_type = other DNA
cgtagtagttttgagttaaagatcaatccagacattatatataataaatatcagttatgtaagaataaaaagattttactaattgtagcaggtgctcatggggtattaggaagtgtaaaa

SEQ ID NO: 155 - DNA, 120 bp, synthetic construct
  source 1..120: mol_type = other DNA
aagaataaaaagattttactaattgtagcaggtgctcatggggtattaggaagtgtaaaagaactatgccaatcatttatgtcagtacctgatttacaagtagttgtcgtttgtgggaaa

SEQ ID NO: 156 - DNA, 120 bp, synthetic construct
  source 1..120: mol_type = other DNA
gaactatgccaatcatttatgtcagtacctgatttacaagtagttgtcgtttgtgggaaaaatgaagcattaaaacaggatttggtaggggtacaggaaacaaatcctgatgcattaaaa

SEQ ID NO: 157 - DNA, 120 bp, synthetic construct
  source 1..120: mol_type = other DNA
aatgaagcattaaaacaggatttggtaggggtacaggaaacaaatcctgatgcattaaaagtatttggttatgttgaaaatattgatgaactattccgcgttacttcttgtatgattaca

SEQ ID NO: 158 - DNA, 120 bp, synthetic construct
  source 1..120: mol_type = other DNA
gtatttggttatgttgaaaatattgatgaactattccgcgttacttcttgtatgattacaaagccaggcggtattacgttaagtgaggcggcagcattgcaagtacctgtcattttatat

SEQ ID NO: 159 - DNA, 120 bp, synthetic construct
  source 1..120: mol_type = other DNA
aagccaggcggtattacgttaagtgaggcggcagcattgcaagtacctgtcattttatataagcctgttccaggacaagaaaatgaaaatgcgatgtactttgaaagaaaaggagctgca

SEQ ID NO: 160 - DNA, 120 bp, synthetic construct
  source 1..120: mol_type = other DNA
aagcctgttccaggacaagaaaatgaaaatgcgatgtactttgaaagaaaaggagctgcagttgtcattcgtgatgatagtgaggtttttgcaaaaacagaggcgttattacaagacgat

SEQ ID NO: 161 - DNA, 120 bp, synthetic construct
  source 1..120: mol_type = other DNA
gttgtcattcgtgatgatagtgaggtttttgcaaaaacagaggcgttattacaagacgatatgaagcttcttcaaatgaaagaagcgatgaaaagcatttatcgtccggagccagctgat

SEQ ID NO: 162 - DNA, 120 bp, synthetic construct
  source 1..120: mol_type = other DNA
atgaagcttcttcaaatgaaagaagcgatgaaaagcatttatcgtccggagccagctgatcatattgtggatacaattttggcagaaaatcatgtagaaccgaatcatatacctattaaa

SEQ ID NO: 163 - DNA, 120 bp, synthetic construct
  source 1..120: mol_type = other DNA
catattgtggatacaattttggcagaaaatcatgtagaaccgaatcatatacctattaaatcacctgcacttgcacaatcatttacttaatatgaaaccctcttttgtatgtttaaagag

SEQ ID NO: 164 - DNA, 120 bp, synthetic construct
  source 1..120: mol_type = other DNA
tcacctgcacttgcacaatcatttacttaatatgaaaccctcttttgtatgtttaaagagggttctttattgttctctaagataaagacttatccacatgaagattgcgttttcattaaa

SEQ ID NO: 165 - DNA, 120 bp, synthetic construct
  source 1..120: mol_type = other DNA
ggttctttattgttctctaagataaagacttatccacatgaagattgcgttttcattaaacagtaaagtcggaatattaacaactatatccacattatccacaatttttagaaaaatatc

SEQ ID NO: 166 - DNA, 120 bp, synthetic construct
  source 1..120: mol_type = other DNA
cagtaaagtcggaatattaacaactatatccacattatccacaatttttagaaaaatatccacaattctaacatttaatgtacgttgcaatatataaacttgtgaaaggtttggtgaatt

SEQ ID NO: 167 - DNA, 120 bp, synthetic construct
  source 1..120: mol_type = other DNA
cacaattctaacatttaatgtacgttgcaatatataaacttgtgaaaggtttggtgaatttatgcacaattccataaattatgtggataacgttatccacataaaaaaaggttccttatt

SEQ ID NO: 168 - DNA, 120 bp, synthetic construct
  source 1..120: mol_type = other DNA
tatgcacaattccataaattatgtggataacgttatccacataaaaaaaggttccttatttataaggaaccttttttctactctatcacgtagaaaaaatatgtaatgagaatgaataat

SEQ ID NO: 169 - DNA, 120 bp, synthetic construct
  source 1..120: mol_type = other DNA
tataaggaaccttttttctactctatcacgtagaaaaaatatgtaatgagaatgaataattaggggggagaacttctaattattcattctcactttaaatacttttcgagcgataacccg

SEQ ID NO: 170 - DNA, 120 bp, synthetic construct
  source 1..120: mol_type = other DNA
taggggggagaacttctaattattcattctcactttaaatacttttcgagcgataacccgctgcgcgatctgctttacgaaattctcgttggtagagaacttcttgtgtactagataacg

SEQ ID NO: 171 - DNA, 120 bp, synthetic construct
  source 1..120: mol_type = other DNA
ctgcgcgatctgctttacgaaattctcgttggtagagaacttcttgtgtactagataacgcgttttttgttttgtcacgtttctttttatccattacaaatcacctcgtgtccgaaagtt

SEQ ID NO: 172 - DNA, 120 bp, synthetic construct
  source 1..120: mol_type = other DNA
cgttttttgttttgtcacgtttctttttatccattacaaatcacctcgtgtccgaaagttactatctatcgtttccaaagacatggggtgatatacgtatatatcaaaatgttaatggtt

SEQ ID NO: 173 - DNA, 120 bp, synthetic construct
  source 1..120: mol_type = other DNA
actatctatcgtttccaaagacatggggtgatatacgtatatatcaaaatgttaatggttaattattatttctgaaaatttagattatgcttcttttaagtgatgtgcatcttggaacgt

SEQ ID NO: 174 - DNA, 120 bp, synthetic construct
  source 1..120: mol_type = other DNA
aattattatttctgaaaatttagattatgcttcttttaagtgatgtgcatcttggaacgttgtatcgcgcattgtagcaagtgtatattgatcttttggaatttcatataagttatatac

SEQ ID NO: 175 - DNA, 120 bp, synthetic construct
  source 1..120: mol_type = other DNA
tgtatcgcgcattgtagcaagtgtatattgatcttttggaatttcatataagttatatacttcttcattcgcattaatttcatcataaacagcttttcttgtttcatttgctagatttac

SEQ ID NO: 176 - DNA, 120 bp, synthetic construct
  source 1..120: mol_type = other DNA
ttcttcattcgcattaatttcatcataaacagcttttcttgtttcatttgctagatttacatattgtaatttctctgcagctttaatagaacgaatatttattttgcgaatacgcataaa

SEQ ID NO: 177 - DNA, 120 bp, synthetic construct
  source 1..120: mol_type = other DNA
atattgtaatttctctgcagctttaatagaacgaatatttattttgcgaatacgcataaagattgtttcaatatctagctcgtagaaaagttcgctaaaaaatgaatcttttgccaattt

SEQ ID NO: 178 - DNA, 120 bp, synthetic construct
  source 1..120: mol_type = other DNA
gattgtttcaatatctagctcgtagaaaagttcgctaaaaaatgaatcttttgccaatttattgtagccttttccatgataaggtttgccaagccatgttccaaggaatccagctttttc

SEQ ID NO: 179 - DNA, 120 bp, synthetic construct
  source 1..120: mol_type = other DNA
attgtagccttttccatgataaggtttgccaagccatgttccaaggaatccagctttttcttgcacatcaaataaagtaattgttccgatagggttaccccattcatctaaaattgtgcg

SEQ ID NO: 180 - DNA, 120 bp, synthetic construct
  source 1..120: mol_type = other DNA
ttgcacatcaaataaagtaattgttccgatagggttaccccattcatctaaaattgtgcgtgaaattaattccccacgctcttcagcttcaatcgtttgtttcgttaaaaataaatattc

SEQ ID NO: 181 - DNA, 120 bp, synthetic construct
  source 1..120: mol_type = other DNA
tgaaattaattccccacgctcttcagcttcaatcgtttgtttcgttaaaaataaatattcctcataagaataagccttttgacgcacaaaagggaagacagctggatccaccattaactc

SEQ ID NO: 182 - DNA, 120 bp, synthetic construct
  source 1..120: mol_type = other DNA
ctcataagaataagccttttgacgcacaaaagggaagacagctggatccaccattaactcgtatagaacgtggctgtcgtgtaagtcgcgtttttttaacatactaactcctcctcacac

SEQ ID NO: 183 - DNA, 120 bp, synthetic construct
  source 1..120: mol_type = other DNA
gtatagaacgtggctgtcgtgtaagtcgcgtttttttaacatactaactcctcctcacacgagggtagcatgacgaaaaaacaccccaccctcgaaatttttatatcaatctttaaaaaa

SEQ ID NO: 184 - DNA, 120 bp, synthetic construct
  source 1..120: mol_type = other DNA
gagggtagcatgacgaaaaaacaccccaccctcgaaatttttatatcaatctttaaaaaatttcggggtgggaatcgaacccactagaaccagtttctaacgctggtggcgcaccatttg

SEQ ID NO: 185 - DNA, 120 bp, synthetic construct
  source 1..120: mol_type = other DNA
tttcggggtgggaatcgaacccactagaaccagtttctaacgctggtggcgcaccatttgccttccccattcatcaatttgaaaatgataatcacgacacaaattgattatggtttcatt

SEQ ID NO: 186 - DNA, 120 bp, synthetic construct
  source 1..120: mol_type = other DNA
ccttccccattcatcaatttgaaaatgataatcacgacacaaattgattatggtttcattcagtttataatcgtataatactttatctagtcaaaaaaataaactagttttttttatttt

SEQ ID NO: 187 - DNA, 120 bp, synthetic construct
  source 1..120: mol_type = other DNA
cagtttataatcgtataatactttatctagtcaaaaaaataaactagttttttttattttttttgtaaattatttttccatcaatcatagttagtacaggcttggctaaataatggaaag

SEQ ID NO: 188 - DNA, 120 bp, synthetic construct
  source 1..120: mol_type = other DNA
ttttgtaaattatttttccatcaatcatagttagtacaggcttggctaaataatggaaaggatgatgggtccacagcacaagatcagcgtcttttccgacctcaatgcttccaattctat

SEQ ID NO: 189 - DNA, 120 bp, synthetic construct
  source 1..120: mol_type = other DNA
gatgatgggtccacagcacaagatcagcgtcttttccgacctcaatgcttccaattctatcctctaaacgtaaatttcgtgctggaaatatagtgattccttctagtgcagttttttcgt

SEQ ID NO: 190 - DNA, 120 bp, synthetic construct
  source 1..120: mol_type = other DNA
cctctaaacgtaaatttcgtgctggaaatatagtgattccttctagtgcagttttttcgtctaatccttcccttacagcaacagcagcacaaagatttaaatattgaatgggtgtatagg

SEQ ID NO: 191 - DNA, 120 bp, synthetic construct
  source 1..120: mol_type = other DNA
ctaatccttcccttacagcaacagcagcacaaagatttaaatattgaatgggtgtataggggtgatctgttgtgatggaaacttccactccatttttcgataatatatggtaagtatccc

SEQ ID NO: 192 - DNA, 120 bp, synthetic construct
  source 1..120: mol_type = other DNA
ggtgatctgttgtgatggaaacttccactccatttttcgataatatatggtaagtatcccatgttttgtttttaagttcaattttagaacggcgtgtaagcgtggggccaactgaaactt

SEQ ID NO: 193 - DNA, 120 bp, synthetic construct
  source 1..120: mol_type = other DNA
atgttttgtttttaagttcaattttagaacggcgtgtaagcgtggggccaactgaaactttcaaattgtgcttcgaaagttcctcaataataaagtgtccttctgtacaatgttcaatac

SEQ ID NO: 194 - DNA, 120 bp, synthetic construct
  source 1..120: mol_type = other DNA
tcaaattgtgcttcgaaagttcctcaataataaagtgtccttctgtacaatgttcaatacgtaaatcgagattgaactctgttgcaaaacgtagagcagaactaatatcatctgctcggt

SEQ ID NO: 195 - DNA, 120 bp, synthetic construct
  source 1..120: mol_type = other DNA
gtaaatcgagattgaactctgttgcaaaacgtagagcagaactaatatcatctgctcggtgagcgtggatacgtacgggtatttcgcggcgtaatgcttttaaaataggaagcattcgaa

SEQ ID NO: 196 - DNA, 120 bp, synthetic construct
  source 1..120: mol_type = other DNA
gagcgtggatacgtacgggtatttcgcggcgtaatgcttttaaaataggaagcattcgaaaatcagcttcatgcccgtagtgttgtgcttcataaaatgattcccgaagtaatcccataa

SEQ ID NO: 197 - DNA, 120 bp, synthetic construct
  source 1..120: mol_type = other DNA
aatcagcttcatgcccgtagtgttgtgcttcataaaatgattcccgaagtaatcccataattcccatacgcgtaatggactcttttgttccattactatggacttttttaggattttcgc

SEQ ID NO: 198 - DNA, 120 bp, synthetic construct
  source 1..120: mol_type = other DNA
ttcccatacgcgtaatggactcttttgttccattactatggacttttttaggattttcgccaaaggcaatctttaagccagcaggttcttgaataatcatatgatcaatacaagttccgg

SEQ ID NO: 199 - DNA, 120 bp, synthetic construct
  source 1..120: mol_type = other DNA
caaaggcaatctttaagccagcaggttcttgaataatcatatgatcaatacaagttccggctgtttttattacacaagtcgtaccaccaataatgttttgacttcctggcataacgtgaa

SEQ ID NO: 200 - DNA, 120 bp, synthetic construct
  source 1..120: mol_type = other DNA
ctgtttttattacacaagtcgtaccaccaataatgttttgacttcctggcataacgtgaacagttgtaattccattttgtacagcatcttgaaatgcaatatccaaagggtggattccgt

SEQ ID NO: 201 - DNA, 120 bp, synthetic construct
  source 1..120: mol_type = other DNA
cagttgtaattccattttgtacagcatcttgaaatgcaatatccaaagggtggattccgtctaaagaacggatatgtggtgttgaaacttcagatgtttcatttgcatcattgccagccc

SEQ ID NO: 202 - DNA, 120 bp, synthetic construct
  source 1..120: mol_type = other DNA
ctaaagaacggatatgtggtgttgaaacttcagatgtttcatttgcatcattgccagcccaaccagtaccttcatcgtagagaccaagatgagtatggacatcaataaatccaggtaaaa

SEQ ID NO: 203 - DNA, 120 bp, synthetic construct
  source 1..120: mol_type = other DNA
aaccagtaccttcatcgtagagaccaagatgagtatggacatcaataaatccaggtaaaagatgaagagcacgtgcatctataactgtcatatcttgagtaggttgaatgaaaggcttga

SEQ ID NO: 204 - DNA, 120 bp, synthetic construct
  source 1..120: mol_type = other DNA
gatgaagagcacgtgcatctataactgtcatatcttgagtaggttgaatgaaaggcttgacctcagcaattttttctcctataacgagtacatccccttgaaatttttgggatgtaatag

SEQ ID NO: 205 - DNA, 120 bp, synthetic construct
  source 1..120: mol_type = other DNA
cctcagcaattttttctcctataacgagtacatccccttgaaatttttgggatgtaataggatagaccatggcttgtttgagcaatattttcataggtacctcatttctgttactttata

SEQ ID NO: 206 - DNA, 120 bp, synthetic construct
  source 1..120: mol_type = other DNA
gatagaccatggcttgtttgagcaatattttcataggtacctcatttctgttactttataatgttaatggaatgtaaggaaaagtaactgaacgattatttgtgtaataatgctccggat

SEQ ID NO: 207 - DNA, 120 bp, synthetic construct
  source 1..120: mol_type = other DNA
atgttaatggaatgtaaggaaaagtaactgaacgattatttgtgtaataatgctccggattctaggaaatgaaaattttggaagtaacccctgtaaaactatgttttagaagtactacat

SEQ ID NO: 208 - DNA, 120 bp, synthetic construct
  source 1..120: mol_type = other DNA
tctaggaaatgaaaattttggaagtaacccctgtaaaactatgttttagaagtactacattgtatgcgaaagtatattttgtaatgcatggtctattgttggaaatgtgtattgataccc

SEQ ID NO: 209 - DNA, 120 bp, synthetic construct
  source 1..120: mol_type = other DNA
tgtatgcgaaagtatattttgtaatgcatggtctattgttggaaatgtgtattgatacccatgctcaattgctttactaggtaatacatgttgtccttctagtacaagtatgctcatctc

SEQ ID NO: 210 - DNA, 120 bp, synthetic construct
  source 1..120: mol_type = other DNA
atgctcaattgctttactaggtaatacatgttgtccttctagtacaagtatgctcatctcacctaataaagcatgaagcataaatgaagggacaggtaaccaatgaggttttttcattat

SEQ ID NO: 211 - DNA, 120 bp, synthetic construct
  source 1..120: mol_type = other DNA
acctaataaagcatgaagcataaatgaagggacaggtaaccaatgaggttttttcattatagttgcaatggtttctccaaatcccttcattcttataggctctggagctgtaatgttgag

SEQ ID NO: 212 - DNA, 120 bp, synthetic construct
  source 1..120: mol_type = other DNA
agttgcaatggtttctccaaatcccttcattcttataggctctggagctgtaatgttgagcgggccatcaatttcttttttgtgtatgatgaaatcaatcatggaagcgacatcgtctat

SEQ ID NO: 213 - DNA, 120 bp, synthetic construct
  source 1..120: mol_type = other DNA
cgggccatcaatttcttttttgtgtatgatgaaatcaatcatggaagcgacatcgtctatatgaatccatgataaccattgctttccagatccaactgtacctccgatatagaattgata

SEQ ID NO: 214 - DNA, 120 bp, synthetic construct
  source 1..120: mol_type = other DNA
atgaatccatgataaccattgctttccagatccaactgtacctccgatatagaattgatagggaagtagcattttgggaagggctcctccgtctggacctaatatgactccgaatcgtgc

SEQ ID NO: 215 - DNA, 120 bp, synthetic construct
  source 1..120: mol_type = other DNA
gggaagtagcattttgggaagggctcctccgtctggacctaatatgactccgaatcgtgcatagattgttcgtattccgagagagcgtgctttagatgcttcttgttcccatgaatatac

SEQ ID NO: 216 - DNA, 120 bp, synthetic construct
  source 1..120: mol_type = other DNA
atagattgttcgtattccgagagagcgtgctttagatgcttcttgttcccatgaatatactgtatttgctaaaaagtcatttccgggagtcacatgctgttctgtaaaagactcggtttc

SEQ ID NO: 217 - DNA, 120 bp, synthetic construct
  source 1..120: mol_type = other DNA
tgtatttgctaaaaagtcatttccgggagtcacatgctgttctgtaaaagactcggtttcagacgttccatagtatccaattgcactcgcgttaataaatgtatgtggttttgcagggag

SEQ ID NO: 218 - DNA, 120 bp, synthetic construct
  source 1..120: mol_type = other DNA
agacgttccatagtatccaattgcactcgcgttaataaatgtatgtggttttgcagggagtgcctgcaattgtttaatgagtccttttgttgtttgaattctactgtttaaaatgatttt

SEQ ID NO: 219 - DNA, 120 bp, synthetic construct
  source 1..120: mol_type = other DNA
tgcctgcaattgtttaatgagtccttttgttgtttgaattctactgtttaaaatgattttcttttgtttctttgtccatctactattaatagactctccagctagattaataactacatc

SEQ ID NO: 220 - DNA, 120 bp, synthetic construct
  source 1..120: mol_type = other DNA
cttttgtttctttgtccatctactattaatagactctccagctagattaataactacatcaatagaagagagagggaaggtttgtaaatctggtgtccattgcacatactgaaggttagg

SEQ ID NO: 221 - DNA, 120 bp, synthetic construct
  source 1..120: mol_type = other DNA
aatagaagagagagggaaggtttgtaaatctggtgtccattgcacatactgaaggttagggtgagaagtttcagtagttttttttcttgtgagaatgtaaaccgtatatcctttttgaat

SEQ ID NO: 222 - DNA, 120 bp, synthetic construct
  source 1..120: mol_type = other DNA
gtgagaagtttcagtagttttttttcttgtgagaatgtaaaccgtatatcctttttgaataaaaaaagtagaaaggtatgtgccgataaagccggtaccaccagaaattgcgattttcac

SEQ ID NO: 223 - DNA, 120 bp, synthetic construct
  source 1..120: mol_type = other DNA
aaaaaaagtagaaaggtatgtgccgataaagccggtaccaccagaaattgcgattttcacaattatttcctcctcattatatatattcttgaaaagcaaaaacgttcctcgactatgtta

SEQ ID NO: 224 - DNA, 120 bp, synthetic construct
  source 1..120: mol_type = other DNA
aattatttcctcctcattatatatattcttgaaaagcaaaaacgttcctcgactatgttaaaataatagagaggtgagagtatggctgtcattacaaaaatagaagtgcaaaaacgatcg

SEQ ID NO: 225 - DNA, 120 bp, synthetic construct
  source 1..120: mol_type = other DNA
aaataatagagaggtgagagtatggctgtcattacaaaaatagaagtgcaaaaacgatcgaaagaacggtttaatatttatatcgataaaggtcaaggtgaagaatacggatttagtgtg

SEQ ID NO: 226 - DNA, 120 bp, synthetic construct
  source 1..120: mol_type = other DNA
aaagaacggtttaatatttatatcgataaaggtcaaggtgaagaatacggatttagtgtgaacgaagtaatcttaataaagcacggattacaaaagggcttagaaattgatgaaatagcg

SEQ ID NO: 227 - DNA, 120 bp, synthetic construct
  source 1..120: mol_type = other DNA
aacgaagtaatcttaataaagcacggattacaaaagggcttagaaattgatgaaatagcgttaggaaatattttgtacaatgaagaggtacaaaaagcatatttacaagcaatctcctat

SEQ ID NO: 228 - DNA, 120 bp, synthetic construct
  source 1..120: mol_type = other DNA
ttaggaaatattttgtacaatgaagaggtacaaaaagcatatttacaagcaatctcctatttatcctatcaaatgagaacgaaactagaaatagaagatttcttacgaaaaaaagaagtg

SEQ ID NO: 229 - DNA, 120 bp, synthetic construct
  source 1..120: mol_type = other DNA
ttatcctatcaaatgagaacgaaactagaaatagaagatttcttacgaaaaaaagaagtgggacaagccatcatctctgaagtcgtttcgaaattattacatgaccgatatattaatgat

SEQ ID NO: 230 - DNA, 120 bp, synthetic construct
  source 1..120: mol_type = other DNA
ggacaagccatcatctctgaagtcgtttcgaaattattacatgaccgatatattaatgataaagagtatgctattttatatacgagaacgcaaagtaatgtgaatcgaaaaggtccaacg

SEQ ID NO: 231 - DNA, 120 bp, synthetic construct
  source 1..120: mol_type = other DNA
aaagagtatgctattttatatacgagaacgcaaagtaatgtgaatcgaaaaggtccaacggttattaaaagagagttgttaaataaaggtgttcaggatctaattattatgcatagttta

SEQ ID NO: 232 - DNA, 120 bp, synthetic construct
  source 1..120: mol_type = other DNA
gttattaaaagagagttgttaaataaaggtgttcaggatctaattattatgcatagtttacaagaatatacgaaggaaaagcaaattgagaatgctttaattcttatagaaaagaagaaa

SEQ ID NO: 233 - DNA, 120 bp, synthetic construct
  source 1..120: mol_type = other DNA
caagaatatacgaaggaaaagcaaattgagaatgctttaattcttatagaaaagaagaaaaagtcttatcaaaagcattcctttttacaaatgaaactaaagttagatgaaatgcttgtt

SEQ ID NO: 234 - DNA, 120 bp, synthetic construct
  source 1..120: mol_type = other DNA
aagtcttatcaaaagcattcctttttacaaatgaaactaaagttagatgaaatgcttgttcgtaaaggatattctagagatgtgattcaaatttgtttggaagaattgaaagacgaaaaa

SEQ ID NO: 235 - DNA, 120 bp, synthetic construct
  source 1..120: mol_type = other DNA
cgtaaaggatattctagagatgtgattcaaatttgtttggaagaattgaaagacgaaaaagatgacgaaaagcaacaagaagcgttacactatcatgggaacaaatactatgagaaatat

SEQ ID NO: 236 - DNA, 120 bp, synthetic construct
  source 1..120: mol_type = other DNA
gatgacgaaaagcaacaagaagcgttacactatcatgggaacaaatactatgagaaatataagaagtatgatggatggacgtttgaaaataagatgaaacaagcgttatatcgtaaagga

SEQ ID NO: 237 - DNA, 120 bp, synthetic construct
  source 1..120: mol_type = other DNA
aagaagtatgatggatggacgtttgaaaataagatgaaacaagcgttatatcgtaaaggattctctattgatgagatagagatatttttgcaaatgaaacgtgaagagggatgagggaat

SEQ ID NO: 238 - DNA, 120 bp, synthetic construct
  source 1..120: mol_type = other DNA
ttctctattgatgagatagagatatttttgcaaatgaaacgtgaagagggatgagggaataaaatgaatatgccaaaacgctacagtgaaatgacaccatatgagctaagggaagaaatt

SEQ ID NO: 239 - DNA, 120 bp, synthetic construct
  source 1..120: mol_type = other DNA
aaaatgaatatgccaaaacgctacagtgaaatgacaccatatgagctaagggaagaaattggggttttgaaagagcaagcaataaaagctgagcaacttggaattgtaaatgagttcgat

SEQ ID NO: 240 - DNA, 120 bp, synthetic construct
  source 1..120: mol_type = other DNA
ggggttttgaaagagcaagcaataaaagctgagcaacttggaattgtaaatgagttcgatgtattaatgcgaaagatagcaatggctcgtgcttatatgactgacataaataaattccat

SEQ ID NO: 241 - DNA, 120 bp, synthetic construct
  source 1..120: mol_type = other DNA
gtattaatgcgaaagatagcaatggctcgtgcttatatgactgacataaataaattccatattggtgagacgtatgaattagtagaagaacctggtatattatttgaaattacgtatttc

SEQ ID NO: 242 - DNA, 120 bp, synthetic construct
  source 1..120: mol_type = other DNA
attggtgagacgtatgaattagtagaagaacctggtatattatttgaaattacgtatttcaatggggtatttgcttggggacataagcaaaatgataatgaagagattggaataccgatt

SEQ ID NO: 243 - DNA, 120 bp, synthetic construct
  source 1..120: mol_type = other DNA
aatggggtatttgcttggggacataagcaaaatgataatgaagagattggaataccgatttctttattacaagaaaaataaaaaccagagagcgaatatctctctggttttcatctttgg

SEQ ID NO: 244 - DNA, 120 bp, synthetic construct
  source 1..120: mol_type = other DNA
tctttattacaagaaaaataaaaaccagagagcgaatatctctctggttttcatctttggtaggcgttacaggagataggagattctaaaattggcgttttttacattcattcgccaata

SEQ ID NO: 245 - DNA, 120 bp, synthetic construct
  source 1..120: mol_type = other DNA
taggcgttacaggagataggagattctaaaattggcgttttttacattcattcgccaatataatgagagactgggtttgttgcgtctgtccgttaacttgcgcttttgcatgtttcggac

SEQ ID NO: 246 - DNA, 120 bp, synthetic construct
  source 1..120: mol_type = other DNA
taatgagagactgggtttgttgcgtctgtccgttaacttgcgcttttgcatgtttcggacgagtccacgtatggttaaataattcagaacgactatctaagcgatcacggtagctcatct

SEQ ID NO: 247 - DNA, 120 bp, synthetic construct
  source 1..120: mol_type = other DNA
gagtccacgtatggttaaataattcagaacgactatctaagcgatcacggtagctcatctttatcacctcgtgtaggaagttgaagttaaattactttgtactactcttcctgctgattt

SEQ ID NO: 248 - DNA, 120 bp, synthetic construct
  source 1..120: mol_type = other DNA
ttatcacctcgtgtaggaagttgaagttaaattactttgtactactcttcctgctgatttgcagcacgcatacgttcttgtgggtgcgtgttaattgtgccgttaggtcgcttcgaagcg

SEQ ID NO: 249 - DNA, 120 bp, synthetic construct
  source 1..120: mol_type = other DNA
gcagcacgcatacgttcttgtgggtgcgtgttaattgtgccgttaggtcgcttcgaagcgaagcgtgatttcgctttcggttgaccgtcgattttgctgttgttttttgactcagaccaa

SEQ ID NO: 250 - DNA, 120 bp, synthetic construct
  source 1..120: mol_type = other DNA
aagcgtgatttcgctttcggttgaccgtcgattttgctgttgttttttgactcagaccaaaattcggcttgtttacccattgcgaacgccctcctcatcatcagttgatacctcttgaag

SEQ ID NO: 251 - DNA, 120 bp, synthetic construct
  source 1..120: mol_type = other DNA
aattcggcttgtttacccattgcgaacgccctcctcatcatcagttgatacctcttgaagaagtatcaattatagaatgtgcaaaatagaagaaactatcctttagaaatgaagggataa

SEQ ID NO: 252 - DNA, 120 bp, synthetic construct
  source 1..120: mol_type = other DNA
aagtatcaattatagaatgtgcaaaatagaagaaactatcctttagaaatgaagggataattaggtaaaggagattagaacatgaatgatatttatgaagcattaacgaaagaactatta

SEQ ID NO: 253 - DNA, 120 bp, synthetic construct
  source 1..120: mol_type = other DNA
ttaggtaaaggagattagaacatgaatgatatttatgaagcattaacgaaagaactattagagaaaaatgacaaactttcttatgcacaagctcgtgcgtgggttgaattactgtgggaa

SEQ ID NO: 254 - DNA, 120 bp, synthetic construct
  source 1..120: mol_type = other DNA
gagaaaaatgacaaactttcttatgcacaagctcgtgcgtgggttgaattactgtgggaagattttcaaacaacttatgcgaaatcaggtcgttatcaaggagaagaaatgactgaacaa

SEQ ID NO: 255 - DNA, 120 bp, synthetic construct
  source 1..120: mol_type = other DNA
gattttcaaacaacttatgcgaaatcaggtcgttatcaaggagaagaaatgactgaacaagtggtgcgatcatggattaataatcatggaggacgccttcatgaaatgcgtacaaataat

SEQ ID NO: 256 - DNA, 120 bp, synthetic construct
  source 1..120: mol_type = other DNA
gtggtgcgatcatggattaataatcatggaggacgccttcatgaaatgcgtacaaataatccgaaatatagccatctaatcaatcaagaagatcatttgaaacattaaaaaaagcgactt

SEQ ID NO: 257 - DNA, 120 bp, synthetic construct
  source 1..120: mol_type = other DNA
ccgaaatatagccatctaatcaatcaagaagatcatttgaaacattaaaaaaagcgacttaagtcgctttttttaatgtggaagtaactccagtttttttcgaagtttttcttcactaaa

SEQ ID NO: 258 - DNA, 120 bp, synthetic construct
  source 1..120: mol_type = other DNA
aagtcgctttttttaatgtggaagtaactccagtttttttcgaagtttttcttcactaaaaatccatcctgtataggaactaataatatttaaattatgatcgagttgaacgattgcaac

SEQ ID NO: 259 - DNA, 120 bp, synthetic construct
  source 1..120: mol_type = other DNA
aatccatcctgtataggaactaataatatttaaattatgatcgagttgaacgattgcaacgaatggataataatctttactgcgatatcgcaaatcaatgaatcgaacttcataataatg

SEQ ID NO: 260 - DNA, 120 bp, synthetic construct
  source 1..120: mol_type = other DNA
gaatggataataatctttactgcgatatcgcaaatcaatgaatcgaacttcataataatgatcataatcgaaaatatcccagcgatacacaggagagaaagataaaaacgctgagatgtt

SEQ ID NO: 261 - DNA, 120 bp, synthetic construct
  source 1..120: mol_type = other DNA
atcataatcgaaaatatcccagcgatacacaggagagaaagataaaaacgctgagatgttttcatcttgtttagctgcgcgcataatagcattatctgggaacggtacccgatcgaactt

SEQ ID NO: 262 - DNA, 120 bp, synthetic construct
  source 1..120: mol_type = other DNA
ttcatcttgtttagctgcgcgcataatagcattatctgggaacggtacccgatcgaacttgtcatatatcatgatattaccacggtgccatctcgcaacgtagtaataatcagccgtaac

SEQ ID NO: 263 - DNA, 120 bp, synthetic construct
  source 1..120: mol_type = other DNA
gtcatatatcatgatattaccacggtgccatctcgcaacgtagtaataatcagccgtaacgactgctaaatggtaatgataaaatcggtaagaaggagaaatgataatcttttcgacatt

SEQ ID NO: 264 - DNA, 120 bp, synthetic construct
  source 1..120: mol_type = other DNA
gactgctaaatggtaatgataaaatcggtaagaaggagaaatgataatcttttcgacatttttgaaacgtttgtgtacaacgcttcttatatttctgtgcataataatccgtccgatgta

SEQ ID NO: 265 - DNA, 120 bp, synthetic construct
  source 1..120: mol_type = other DNA
tttgaaacgtttgtgtacaacgcttcttatatttctgtgcataataatccgtccgatgtagtaaataatcattaatatatacgctgctaaggcagtataccctttatgggaacctacgag

SEQ ID NO: 266 - DNA, 120 bp, synthetic construct
  source 1..120: mol_type = other DNA
gtaaataatcattaatatatacgctgctaaggcagtataccctttatgggaacctacgagcatacaagcaattgcgagtatatggataaagaaaatgacggtatcaaatgtattaatgat

SEQ ID NO: 267 - DNA, 120 bp, synthetic construct
  source 1..120: mol_type = other DNA
catacaagcaattgcgagtatatggataaagaaaatgacggtatcaaatgtattaatgatgccgagtgctacccatttttttgtgaagggccgtaatgcttgtgtaccgtaggcattgaa

SEQ ID NO: 268 - DNA, 120 bp, synthetic construct
  source 1..120: mol_type = other DNA
gccgagtgctacccatttttttgtgaagggccgtaatgcttgtgtaccgtaggcattgaaaatatctacaaagacgtgaagaaagaccgcaataaatgaccaaagtagtagatgaagata

SEQ ID NO: 269 - DNA, 120 bp, synthetic construct
  source 1..120: mol_type = other DNA
aatatctacaaagacgtgaagaaagaccgcaataaatgaccaaagtagtagatgaagatatggagcgtctgaaaagaaggcgaaagagatgccacttataaggaacgaccaaagaattac

SEQ ID NO: 270 - DNA, 120 bp, synthetic construct
  source 1..120: mol_type = other DNA
tggagcgtctgaaaagaaggcgaaagagatgccacttataaggaacgaccaaagaattactgcaggaatggaatgagtaatcccgcgatgatttcttatatatttagcgttattacgcaa

SEQ ID NO: 271 - DNA, 120 bp, synthetic construct
  source 1..120: mol_type = other DNA
tgcaggaatggaatgagtaatcccgcgatgatttcttatatatttagcgttattacgcaattttaaaactgtatcgatgtcaggaatattggaaccagcaattgtagcaagcataacagc

SEQ ID NO: 272 - DNA, 120 bp, synthetic construct
  source 1..120: mol_type = other DNA
ttttaaaactgtatcgatgtcaggaatattggaaccagcaattgtagcaagcataacagcttgaggaccaatatcactttgtgctatggctggatctaacgtggccaaactgcctagagt

SEQ ID NO: 273 - DNA, 120 bp, synthetic construct
  source 1..120: mol_type = other DNA
ttgaggaccaatatcactttgtgctatggctggatctaacgtggccaaactgcctagagtaacgcccataacaaggtgagtggctgtgtccatagaaatccacctccgttttttattaat

SEQ ID NO: 274 - DNA, 120 bp, synthetic construct
  source 1..120: mol_type = other DNA
aacgcccataacaaggtgagtggctgtgtccatagaaatccacctccgttttttattaatgtaactctttttattcgatacctcaagtcctttgccttctatttcctatgtcatcttact

SEQ ID NO: 275 - DNA, 120 bp, synthetic construct
  source 1..120: mol_type = other DNA
gtaactctttttattcgatacctcaagtcctttgccttctatttcctatgtcatcttacttaaattttttcctaaaatctttataatagtacttatatgcaaaaaaatgagggggatcaa

SEQ ID NO: 276 - DNA, 120 bp, synthetic construct
  source 1..120: mol_type = other DNA
taaattttttcctaaaatctttataatagtacttatatgcaaaaaaatgagggggatcaagtttgacacttgaaatattaaataactttaacatagagcagtttcaaaatgatttaattg

SEQ ID NO: 277 - DNA, 120 bp, synthetic construct
  source 1..120: mol_type = other DNA
gtttgacacttgaaatattaaataactttaacatagagcagtttcaaaatgatttaattggttggtttgaaaaagagcaacgtgacttaccgtggcgtaaaaataaagatccataccgcg

SEQ ID NO: 278 - DNA, 120 bp, synthetic construct
  source 1..120: mol_type = other DNA
gttggtttgaaaaagagcaacgtgacttaccgtggcgtaaaaataaagatccataccgcgtttgggtttcggaaattatgttgcagcaaacgagggtagaagctgtaaaaccatattacg

SEQ ID NO: 279 - DNA, 120 bp, synthetic construct
  source 1..120: mol_type = other DNA
tttgggtttcggaaattatgttgcagcaaacgagggtagaagctgtaaaaccatattacgcgaattttatggggaagtttcctactctagaagctttggccaatgctgatgatgaagaag

SEQ ID NO: 280 - DNA, 120 bp, synthetic construct
  source 1..120: mol_type = other DNA
cgaattttatggggaagtttcctactctagaagctttggccaatgctgatgatgaagaagtgttaaaagcatgggaaggtttagggtattattctagagcgcgaaatttacatgcggctg

SEQ ID NO: 281 - DNA, 120 bp, synthetic construct
  source 1..120: mol_type = other DNA
tgttaaaagcatgggaaggtttagggtattattctagagcgcgaaatttacatgcggctgtaaaagaagtaaaagaagtatatggcgggattgtgccaagtgatgtaaagaagattgaga

SEQ ID NO: 282 - DNA, 120 bp, synthetic construct
  source 1..120: mol_type = other DNA
taaaagaagtaaaagaagtatatggcgggattgtgccaagtgatgtaaagaagattgagaaattaaaaggagtcggcccctatacaaaaggtgctattttaagtatcgcatatggcatac

SEQ ID NO: 283 - DNA, 120 bp, synthetic construct
  source 1..120: mol_type = other DNA
aattaaaaggagtcggcccctatacaaaaggtgctattttaagtatcgcatatggcataccagagccggcagttgacggaaatgttgtgcgtgtattgtctcgtattttatcagtatggg

SEQ ID NO: 284 - DNA, 120 bp, synthetic construct
  source 1..120: mol_type = other DNA
cagagccggcagttgacggaaatgttgtgcgtgtattgtctcgtattttatcagtatgggatgacattgcaaaaccgaaaactagaaaagtgtttgaagagattgtgcgtgaaattattt

SEQ ID NO: 285 - DNA, 120 bp, synthetic construct
  source 1..120: mol_type = other DNA
atgacattgcaaaaccgaaaactagaaaagtgtttgaagagattgtgcgtgaaattatttcggctgaaaatccatcttattttaatcaaggtttgatggaattaggagcactgatttgta

SEQ ID NO: 286 - DNA, 120 bp, synthetic construct
  source 1..120: mol_type = other DNA
cggctgaaaatccatcttattttaatcaaggtttgatggaattaggagcactgatttgtattcctaaaaatccagcatgcttactttgtcctgttcgtgagcattgcaggggatatgctg

SEQ ID NO: 287 - DNA, 120 bp, synthetic construct
  source 1..120: mol_type = other DNA
ttcctaaaaatccagcatgcttactttgtcctgttcgtgagcattgcaggggatatgctgaaggtgttcaaaaggaattaccagtaaaaagtaaagcgaaagctcctacgatggtaccga

SEQ ID NO: 288 - DNA, 120 bp, synthetic construct
  source 1..120: mol_type = other DNA
aaggtgttcaaaaggaattaccagtaaaaagtaaagcgaaagctcctacgatggtaccgattgttgcaggagtacttcaaacggaagatggtcgttacgtcattaataaacgtccaagta

SEQ ID NO: 289 - DNA, 120 bp, synthetic construct
  source 1..120: mol_type = other DNA
ttgttgcaggagtacttcaaacggaagatggtcgttacgtcattaataaacgtccaagtaccggtttattagctaatatgtgggagtttccgaatgttgaacttggcgaagggattcgta

SEQ ID NO: 290 - DNA, 120 bp, synthetic construct
  source 1..120: mol_type = other DNA
ccggtttattagctaatatgtgggagtttccgaatgttgaacttggcgaagggattcgtaatcagaaggaacagcttatagattatatgaaggaaaaatttgagctttcgatttctattg

SEQ ID NO: 291 - DNA, 120 bp, synthetic construct
  source 1..120: mol_type = other DNA
atcagaaggaacagcttatagattatatgaaggaaaaatttgagctttcgatttctattgaagaatacgcaatgaatgtacaacatacgtttacacatcgtacttgggatatattcgtat

SEQ ID NO: 292 - DNA, 120 bp, synthetic construct
  source 1..120: mol_type = other DNA
aagaatacgcaatgaatgtacaacatacgtttacacatcgtacttgggatatattcgtattttatggaaaagtaactggtgatattgttgaaacagatacattgaaatttgtatcgaaag

SEQ ID NO: 293 - DNA, 120 bp, synthetic construct
  source 1..120: mol_type = other DNA
tttatggaaaagtaactggtgatattgttgaaacagatacattgaaatttgtatcgaaagaagcatttgagcagttacctttctctaaatcgcatcgtacgatttatgagaattgtgttg

SEQ ID NO: 294 - DNA, 120 bp, synthetic construct
  source 1..120: mol_type = other DNA
aagcatttgagcagttacctttctctaaatcgcatcgtacgatttatgagaattgtgttgagaaaattacaatgcaataaacaaaaaaagtgttcccaggttgggaacacttttttaatc

SEQ ID NO: 295 - DNA, 120 bp, synthetic construct
  source 1..120: mol_type = other DNA
agaaaattacaatgcaataaacaaaaaaagtgttcccaggttgggaacacttttttaatcgtaagaaatttttgtcccatgagtccaactagcttcaccttcttgtaagccacctcttga

SEQ ID NO: 296 - DNA, 120 bp, synthetic construct
  source 1..120: mol_type = other DNA
gtaagaaatttttgtcccatgagtccaactagcttcaccttcttgtaagccacctcttgattcaatttctattacaatttctttgtaaatactttgaccttccgcgtttaaataaggcaa

SEQ ID NO: 297 - DNA, 120 bp, synthetic construct
  source 1..120: mol_type = other DNA
ttcaatttctattacaatttctttgtaaatactttgaccttccgcgtttaaataaggcaaaatctgttgtaatgaatgatgaaaataagctaattcatcttctttccattcgttttttga

SEQ ID NO: 298 - DNA, 120 bp, synthetic construct
  source 1..120: mol_type = other DNA
aatctgttgtaatgaatgatgaaaataagctaattcatcttctttccattcgttttttgaaaccattgttagttcagtcatatcgcgtcctatatacatattcccacctccattttctat

SEQ ID NO: 299 - DNA, 120 bp, synthetic construct
  source 1..120: mol_type = other DNA
aaccattgttagttcagtcatatcgcgtcctatatacatattcccacctccattttctatagtttgaatgagtaacaagagatatatgcggaattttttcaaaagaaaattacggatagc

SEQ ID NO: 300 - DNA, 120 bp, synthetic construct
  source 1..120: mol_type = other DNA
agtttgaatgagtaacaagagatatatgcggaattttttcaaaagaaaattacggatagcttctagttgaattggttacattattgattgtggaggtgagaaagatgagtaaaaaacaac

SEQ ID NO: 301 - DNA, 120 bp, synthetic construct
  source 1..120: mol_type = other DNA
ttctagttgaattggttacattattgattgtggaggtgagaaagatgagtaaaaaacaacaaggttataacaaggcaacttctggtgctagcattcaaagcacaaatgctagttatggta

SEQ ID NO: 302 - DNA, 120 bp, synthetic construct
  source 1..120: mol_type = other DNA
aaggttataacaaggcaacttctggtgctagcattcaaagcacaaatgctagttatggtacagagtttgcgactgaaacaaatgtacaagcagtaaaacaagcaaacgcacaatcagaag

SEQ ID NO: 303 - DNA, 120 bp, synthetic construct
  source 1..120: mol_type = other DNA
cagagtttgcgactgaaacaaatgtacaagcagtaaaacaagcaaacgcacaatcagaagctaagaaagcgcaagcttctggtgctagcattcaaagcacaaatgctagttatggtacag

SEQ ID NO: 304 - DNA, 120 bp, synthetic construct
  source 1..120: mol_type = other DNA
ctaagaaagcgcaagcttctggtgctagcattcaaagcacaaatgctagttatggtacagaatttgcaactgaaacagacgtgcatgctgtgaaaaaacaaaatgcacaatcagctgcaa

SEQ ID NO: 305 - DNA, 120 bp, synthetic construct
  source 1..120: mol_type = other DNA
aatttgcaactgaaacagacgtgcatgctgtgaaaaaacaaaatgcacaatcagctgcaaaacaatcacaatcttctagttcaaatcagtaatgaaagaaaaacacttctctaactcgtg

SEQ ID NO: 306 - DNA, 120 bp, synthetic construct
  source 1..120: mol_type = other DNA
aacaatcacaatcttctagttcaaatcagtaatgaaagaaaaacacttctctaactcgtgagaagtgttttctttgtgctttggccatggtaatgaaaataaatcgaacgacataacttc

SEQ ID NO: 307 - DNA, 120 bp, synthetic construct
  source 1..120: mol_type = other DNA
agaagtgttttctttgtgctttggccatggtaatgaaaataaatcgaacgacataacttctaataagtcaacaaatgtagtcaaaggagaaggaagttacaggttagaaatatgtaatga

SEQ ID NO: 308 - DNA, 120 bp, synthetic construct
  source 1..120: mol_type = other DNA
taataagtcaacaaatgtagtcaaaggagaaggaagttacaggttagaaatatgtaatgaggaataataactgataaataagttcaaaagggggtaagtaatgaacgattttgataagtt

SEQ ID NO: 309 - DNA, 120 bp, synthetic construct
  source 1..120: mol_type = other DNA
ggaataataactgataaataagttcaaaagggggtaagtaatgaacgattttgataagttggtaggagagcaattggaaacgatggatgagttgttgaaattacaagctcatctagaaaa

SEQ ID NO: 310 - DNA, 120 bp, synthetic construct
  source 1..120: mol_type = other DNA
ggtaggagagcaattggaaacgatggatgagttgttgaaattacaagctcatctagaaaagtatcagcaaattgaaatgagcgaaaaggatacgtgcgataaaaaggaattacattttat

SEQ ID NO: 311 - DNA, 120 bp, synthetic construct
  source 1..120: mol_type = other DNA
gtatcagcaaattgaaatgagcgaaaaggatacgtgcgataaaaaggaattacattttatccgccaggaaatatatagaacagaattagcactcaagctattgcatgagaaatttgaaga

SEQ ID NO: 312 - DNA, 120 bp, synthetic construct
  source 1..120: mol_type = other DNA
ccgccaggaaatatatagaacagaattagcactcaagctattgcatgagaaatttgaagagcaaacaaatagtgtgattcaatcttttgaaactgaaaaaatgatttcaaatttaggata

SEQ ID NO: 313 - DNA, 120 bp, synthetic construct
  source 1..120: mol_type = other DNA
gcaaacaaatagtgtgattcaatcttttgaaactgaaaaaatgatttcaaatttaggataagatataccgctatcttcagataaaaggtccttctttacatggaaataaagaagggcttt

SEQ ID NO: 314 - DNA, 120 bp, synthetic construct
  source 1..120: mol_type = other DNA
agatataccgctatcttcagataaaaggtccttctttacatggaaataaagaagggctttttttattctcatttcctcgttttgcccgtaacctaagaagattaggagtatggtattcag

SEQ ID NO: 315 - DNA, 120 bp, synthetic construct
  source 1..120: mol_type = other DNA
ttttattctcatttcctcgttttgcccgtaacctaagaagattaggagtatggtattcagtgtgaaaaatggagccttagcgctttagttttaaaatttcgacaaaaaagttataataga

SEQ ID NO: 316 - DNA, 120 bp, synthetic construct
  source 1..120: mol_type = other DNA
tgtgaaaaatggagccttagcgctttagttttaaaatttcgacaaaaaagttataatagaaaaaaagtgaatgcagctcaaagggcatttgcagttgaaagaagggagcatatatgggat

SEQ ID NO: 317 - DNA, 120 bp, synthetic construct
  source 1..120: mol_type = other DNA
aaaaaagtgaatgcagctcaaagggcatttgcagttgaaagaagggagcatatatgggatttcccaaagaaggagaaaaagtacaaatacatagttataaacataatggctccattcata

SEQ ID NO: 318 - DNA, 120 bp, synthetic construct
  source 1..120: mol_type = other DNA
ttcccaaagaaggagaaaaagtacaaatacatagttataaacataatggctccattcatagaatgtggaaagagacaacaattttaaaagggacacagagtcttgtaatcggagcgaatg

SEQ ID NO: 319 - DNA, 120 bp, synthetic construct
  source 1..120: mol_type = other DNA
gaatgtggaaagagacaacaattttaaaagggacacagagtcttgtaatcggagcgaatgatcgtacagtagtgacggaatcagatggccgaacatggattactcgtgaaccagcaattt

SEQ ID NO: 320 - DNA, 120 bp, synthetic construct
  source 1..120: mol_type = other DNA
atcgtacagtagtgacggaatcagatggccgaacatggattactcgtgaaccagcaatttgttattttcatgaaaactattggtttaatgtaattggaatgttaagggaagagggagtat

SEQ ID NO: 321 - DNA, 120 bp, synthetic construct
  source 1..120: mol_type = other DNA
gttattttcatgaaaactattggtttaatgtaattggaatgttaagggaagagggagtatactattattgtaatttaagctcaccttttgcatatgattctgaagcgttaaagtatattg

SEQ ID NO: 322 - DNA, 120 bp, synthetic construct
  source 1..120: mol_type = other DNA
actattattgtaatttaagctcaccttttgcatatgattctgaagcgttaaagtatattgattatgatttagatattaaagtgtatccagacatgacatatacgcttttagatgaagatg

SEQ ID NO: 323 - DNA, 120 bp, synthetic construct
  source 1..120: mol_type = other DNA
attatgatttagatattaaagtgtatccagacatgacatatacgcttttagatgaagatgagtatgaaaaacatagtcaaattatgcaatatccacctgttattgatacgattttaaaac

SEQ ID NO: 324 - DNA, 120 bp, synthetic construct
  source 1..120: mol_type = other DNA
agtatgaaaaacatagtcaaattatgcaatatccacctgttattgatacgattttaaaacgaaatgtagcacaattaacgcaatggattcatcaaagaaaaggaccattcgcgccagatt

SEQ ID NO: 325 - DNA, 120 bp, synthetic construct
  source 1..120: mol_type = other DNA
gaaatgtagcacaattaacgcaatggattcatcaaagaaaaggaccattcgcgccagattttgtagatatgtggtatgagagatatttaatgtacagaaattaacacaaacctgcagggg

SEQ ID NO: 326 - DNA, 120 bp, synthetic construct
  source 1..120: mol_type = other DNA
ttgtagatatgtggtatgagagatatttaatgtacagaaattaacacaaacctgcaggggatttcccggcaggtttgtcctattagaggggggattatgtgcaaggtataaaaagatatt

SEQ ID NO: 327 - DNA, 120 bp, synthetic construct
  source 1..120: mol_type = other DNA
atttcccggcaggtttgtcctattagaggggggattatgtgcaaggtataaaaagatatttgcaatttgttaaaccatatcgatggcttattgctattacgattatgattggtctagtta

SEQ ID NO: 328 - DNA, 120 bp, synthetic construct
  source 1..120: mol_type = other DNA
tgcaatttgttaaaccatatcgatggcttattgctattacgattatgattggtctagttaaattcggcatcccgcttattatgccgtggttattaaaatatattattgatgatgtaattc

SEQ ID NO: 329 - DNA, 120 bp, synthetic construct
  source 1..120: mol_type = other DNA
aattcggcatcccgcttattatgccgtggttattaaaatatattattgatgatgtaattcagggcgcagggtcacttcaagataaaacgtcccaactagtaacagcgattgggattgctt

SEQ ID NO: 330 - DNA, 120 bp, synthetic construct
  source 1..120: mol_type = other DNA
agggcgcagggtcacttcaagataaaacgtcccaactagtaacagcgattgggattgctttttttatttttgcagtattaagaccgccaattgaatattatcgtcaatatttcgcgcaac

SEQ ID NO: 331 - DNA, 120 bp, synthetic construct
  source 1..120: mol_type = other DNA
tttttatttttgcagtattaagaccgccaattgaatattatcgtcaatatttcgcgcaacgtattgcaaatacaatactatatgatttgcgaaagcatatttttggtcatttacaaaagt

SEQ ID NO: 332 - DNA, 120 bp, synthetic construct
  source 1..120: mol_type = other DNA
gtattgcaaatacaatactatatgatttgcgaaagcatatttttggtcatttacaaaagttgagtttacgctattattcgaatacaaaaacaggggagattatttcacgtgtcattcatg

SEQ ID NO: 333 - DNA, 120 bp, synthetic construct
  source 1..120: mol_type = other DNA
tgagtttacgctattattcgaatacaaaaacaggggagattatttcacgtgtcattcatgatgtagaacaaacgaaggactttgtaattactggtttgatgaatgtttggttagatacgg

SEQ ID NO: 334 - DNA, 120 bp, synthetic construct
  source 1..120: mol_type = other DNA
atgtagaacaaacgaaggactttgtaattactggtttgatgaatgtttggttagatacggcaacaattgctatcgctattattgttatgttttctatgaatataaaattgacatttgttg

SEQ ID NO: 335 - DNA, 120 bp, synthetic construct
  source 1..120: mol_type = other DNA
caacaattgctatcgctattattgttatgttttctatgaatataaaattgacatttgttgcgctattaattttacctatttatgtagtagcagtgaaatattttttcgggcgtcttcgta

SEQ ID NO: 336 - DNA, 120 bp, synthetic construct
  source 1..120: mol_type = other DNA
cgctattaattttacctatttatgtagtagcagtgaaatattttttcgggcgtcttcgtaaattgacgaaggagcgttcacaagcgttagcaacgatgcaaggatatttacatgaacgta

SEQ ID NO: 337 - DNA, 120 bp, synthetic construct
  source 1..120: mol_type = other DNA
aattgacgaaggagcgttcacaagcgttagcaacgatgcaaggatatttacatgaacgtattcaagggatgcaagtgacacgtagctttgcattagaagagtatgaggggaagcagtttg

SEQ ID NO: 338 - DNA, 120 bp, synthetic construct
  source 1..120: mol_type = other DNA
ttcaagggatgcaagtgacacgtagctttgcattagaagagtatgaggggaagcagtttgaaaaaagaaataatgaatttttgacgaaagcgttaacgcatacgagttggacggcgagaa

SEQ ID NO: 339 - DNA, 120 bp, synthetic construct
  source 1..120: mol_type = other DNA
aaaaaagaaataatgaatttttgacgaaagcgttaacgcatacgagttggacggcgagaacattttcggcagtaaatacgttaacagatttagggccgttacttgtaattggttttgcag

SEQ ID NO: 340 - DNA, 120 bp, synthetic construct
  source 1..120: mol_type = other DNA
cattttcggcagtaaatacgttaacagatttagggccgttacttgtaattggttttgcagcatatgaagtgattcaggggcagttaacattagggactatggttgcctttgtcggatata

SEQ ID NO: 341 - DNA, 120 bp, synthetic construct
  source 1..120: mol_type = other DNA
catatgaagtgattcaggggcagttaacattagggactatggttgcctttgtcggatatatggatagtttgtatagtccgcttcgccgccttgttaattcatctacgacattaacgcagt

SEQ ID NO: 342 - DNA, 120 bp, synthetic construct
  source 1..120: mol_type = other DNA
tggatagtttgtatagtccgcttcgccgccttgttaattcatctacgacattaacgcagtctttcgcatcgatggaccgagtgtttgaactgttagatgaaaaatacgatattgtcaatg

SEQ ID NO: 343 - DNA, 120 bp, synthetic construct
  source 1..120: mol_type = other DNA
ctttcgcatcgatggaccgagtgtttgaactgttagatgaaaaatacgatattgtcaatgtgccaagtgcagtacaaacgaaaaaattaaatggtgaagtgatatttgataatgtatctt

SEQ ID NO: 344 - DNA, 120 bp, synthetic construct
  source 1..120: mol_type = other DNA
tgccaagtgcagtacaaacgaaaaaattaaatggtgaagtgatatttgataatgtatcttttcgttataatgcggatgaaaaagagatattacataacctttcgttaactatgttgccag

SEQ ID NO: 345 - DNA, 120 bp, synthetic construct
  source 1..120: mol_type = other DNA
ttcgttataatgcggatgaaaaagagatattacataacctttcgttaactatgttgccaggagagaaggtagcacttgtaggagcgagtgggggagggaagtcatctcttgctagtttaa

SEQ ID NO: 346 - DNA, 120 bp, synthetic construct
  source 1..120: mol_type = other DNA
gagagaaggtagcacttgtaggagcgagtgggggagggaagtcatctcttgctagtttaattcctcgtttctatgatgtttcctcaggggcagtttatgtagatggaatagatgtcagaa

SEQ ID NO: 347 - DNA, 120 bp, synthetic construct
  source 1..120: mol_type = other DNA
ttcctcgtttctatgatgtttcctcaggggcagtttatgtagatggaatagatgtcagaaagtatgatatgagaaatttacgtagccatattggaattgtactgcaagataatttgttat

SEQ ID NO: 348 - DNA, 120 bp, synthetic construct
  source 1..120: mol_type = other DNA
agtatgatatgagaaatttacgtagccatattggaattgtactgcaagataatttgttatttagcgatacaatcggggcaaacattttatatggaaatccgaaagctacagaggaagaag

SEQ ID NO: 349 - DNA, 120 bp, synthetic construct
  source 1..120: mol_type = other DNA
ttagcgatacaatcggggcaaacattttatatggaaatccgaaagctacagaggaagaagtaattgcagctgctaaagctgcgcaaattcatgattttattatagagttacctgatggtt

SEQ ID NO: 350 - DNA, 120 bp, synthetic construct
  source 1..120: mol_type = other DNA
taattgcagctgctaaagctgcgcaaattcatgattttattatagagttacctgatggttatgatactgtcgttggggaacgtggtgtgaagttatctggtggtcaaaggcaacgtgtag

SEQ ID NO: 351 - DNA, 120 bp, synthetic construct
  source 1..120: mol_type = other DNA
atgatactgtcgttggggaacgtggtgtgaagttatctggtggtcaaaggcaacgtgtagcgattgcacgagtgtttttaaagaatccatcattacttatattagatgaagcgactcccg

SEQ ID NO: 352 - DNA, 120 bp, synthetic construct
  source 1..120: mol_type = other DNA
cgattgcacgagtgtttttaaagaatccatcattacttatattagatgaagcgactcccgctttagatttagaaaatgaacgatatattcaagaggcgcttcagacgttagctgctgatc

SEQ ID NO: 353 - DNA, 120 bp, synthetic construct
  source 1..120: mol_type = other DNA
ctttagatttagaaaatgaacgatatattcaagaggcgcttcagacgttagctgctgatcgaacgacaatcataattgcacatcgattggcgacgattacgcatgtggatacgattattt

SEQ ID NO: 354 - DNA, 120 bp, synthetic construct
  source 1..120: mol_type = other DNA
gaacgacaatcataattgcacatcgattggcgacgattacgcatgtggatacgattatttacattgaagatggtgaaattaaagaaacaggttctcatgaagaattaatgaaaaaaagag

SEQ ID NO: 355 - DNA, 120 bp, synthetic construct
  source 1..120: mol_type = other DNA
acattgaagatggtgaaattaaagaaacaggttctcatgaagaattaatgaaaaaaagaggatattattacaacttatatcaacttcaacatataacagaaacagctcctttagcgtaaa

SEQ ID NO: 356 - DNA, 120 bp, synthetic construct
  source 1..120: mol_type = other DNA
gatattattacaacttatatcaacttcaacatataacagaaacagctcctttagcgtaaaaggagctgttttttattcgtcttcttttttatcatcgattttaagttctgcttctggttt

SEQ ID NO: 357 - DNA, 120 bp, synthetic construct
  source 1..120: mol_type = other DNA
aggagctgttttttattcgtcttcttttttatcatcgattttaagttctgcttctggtttatggtatgtgtagaagctatccacaagtaaatctaaatgctctacttcttcactatagtt

SEQ ID NO: 358 - DNA, 120 bp, synthetic construct
  source 1..120: mol_type = other DNA
atggtatgtgtagaagctatccacaagtaaatctaaatgctctacttcttcactatagttaataatggcagaaataagagggaagagatgtagccatgttttatatgcttcttcatcgtc

SEQ ID NO: 359 - DNA, 120 bp, synthetic construct
  source 1..120: mol_type = other DNA
aataatggcagaaataagagggaagagatgtagccatgttttatatgcttcttcatcgtccttgttttgatattccataaagatatcaattaattcttgtttacctgtttcaacttcatc

SEQ ID NO: 360 - DNA, 120 bp, synthetic construct
  source 1..120: mol_type = other DNA
cttgttttgatattccataaagatatcaattaattcttgtttacctgtttcaacttcatcaagcatttcaacggattgttgtttttttgctttaccaataaattttaataaaacttgttc

SEQ ID NO: 361 - DNA, 120 bp, synthetic construct
  source 1..120: mol_type = other DNA
aagcatttcaacggattgttgtttttttgctttaccaataaattttaataaaacttgttcatggtaatgcgttaatgaatcaagttcgttttggatagattcttgaaattcttctggcat

SEQ ID NO: 362 - DNA, 120 bp, synthetic construct
  source 1..120: mol_type = other DNA
atggtaatgcgttaatgaatcaagttcgttttggatagattcttgaaattcttctggcatatagcgcaattcattttcagtacgatgtaatgattttaacgtacttaaagcacggcttgt

SEQ ID NO: 363 - DNA, 120 bp, synthetic construct
  source 1..120: mol_type = other DNA
atagcgcaattcattttcagtacgatgtaatgattttaacgtacttaaagcacggcttgtcgtcgctaacatttgtctgaataaaacgagcttacgaatttttgcgaactgtactttttt

SEQ ID NO: 364 - DNA, 120 bp, synthetic construct
  source 1..120: mol_type = other DNA
cgtcgctaacatttgtctgaataaaacgagcttacgaatttttgcgaactgtacttttttcgtgtaacttctttcttctttatacagcaaatagtaatggtttaatttgatcattttttc

SEQ ID NO: 365 - DNA, 120 bp, synthetic construct
  source 1..120: mol_type = other DNA
cgtgtaacttctttcttctttatacagcaaatagtaatggtttaatttgatcattttttctttcatacgatcaatatcagtttttaacgttgtaaaatcagaagcttgcctgctattcat

SEQ ID NO: 366 - DNA, 120 bp, synthetic construct
  source 1..120: mol_type = other DNA
tttcatacgatcaatatcagtttttaacgttgtaaaatcagaagcttgcctgctattcattcgaatccattttacaatttcttctgtgttatcaacgatgcgatgatatagctttgtttc

SEQ ID NO: 367 - DNA, 120 bp, synthetic construct
  source 1..120: mol_type = other DNA
tcgaatccattttacaatttcttctgtgttatcaacgatgcgatgatatagctttgtttcgtattttggcggcataaatactaaatttacaagtgaagcggcaataataccaaccataat

SEQ ID NO: 368 - DNA, 120 bp, synthetic construct
  source 1..120: mol_type = other DNA
gtattttggcggcataaatactaaatttacaagtgaagcggcaataataccaaccataatcgtcgcaaatcgaagtaaggcaaaactaaagaaatcttcgccctgatattccataatagc

SEQ ID NO: 369 - DNA, 120 bp, synthetic construct
  source 1..120: mol_type = other DNA
cgtcgcaaatcgaagtaaggcaaaactaaagaaatcttcgccctgatattccataatagcgataacagttactaaagcgattgatattgtgttttctaatcgtaattgcaatgtaagagc

SEQ ID NO: 370 - DNA, 120 bp, synthetic construct
  source 1..120: mol_type = other DNA
gataacagttactaaagcgattgatattgtgttttctaatcgtaattgcaatgtaagagcaattactaatatacatgttaatccaataataaaaggattatgtccaaaagcagtagcgaa

SEQ ID NO: 371 - DNA, 120 bp, synthetic construct
  source 1..120: mol_type = other DNA
aattactaatatacatgttaatccaataataaaaggattatgtccaaaagcagtagcgaatgcgatagcgaataccgcaccaatgacgtttgcttgaatttgttcaagtgcagttaaata

SEQ ID NO: 372 - DNA, 120 bp, synthetic construct
  source 1..120: mol_type = other DNA
tgcgatagcgaataccgcaccaatgacgtttgcttgaatttgttcaagtgcagttaaatacgaacggtatacagacggttgaacagcgaagatagctgagattcccgcaaataccggact

SEQ ID NO: 373 - DNA, 120 bp, synthetic construct
  source 1..120: mol_type = other DNA
cgaacggtatacagacggttgaacagcgaagatagctgagattcccgcaaataccggactcggtaagttaagtaaaatacaagcaaataaagctaaagtgatggcaatacccgtttttaa

SEQ ID NO: 374 - DNA, 120 bp, synthetic construct
  source 1..120: mol_type = other DNA
cggtaagttaagtaaaatacaagcaaataaagctaaagtgatggcaatacccgtttttaaaatgcgagcaccaagtttcataccctaaataagatcctttctcttgtcataatgaatgta

SEQ ID NO: 375 - DNA, 120 bp, synthetic construct
  source 1..120: mol_type = other DNA
aatgcgagcaccaagtttcataccctaaataagatcctttctcttgtcataatgaatgtacaacatgatactatacattcattacaatatgttagcaagtgatattttagtgacgttaat

SEQ ID NO: 376 - DNA, 120 bp, synthetic construct
  source 1..120: mol_type = other DNA
caacatgatactatacattcattacaatatgttagcaagtgatattttagtgacgttaataagaaattaagattcattttatactttttcctaattcttttgaaacatcaatttttagta

SEQ ID NO: 377 - DNA, 120 bp, synthetic construct
  source 1..120: mol_type = other DNA
aagaaattaagattcattttatactttttcctaattcttttgaaacatcaatttttagtaaaaaaacctgctgaattccagcaggtttcaaattgttactatagattactatgagaagtg

SEQ ID NO: 378 - DNA, 120 bp, synthetic construct
  source 1..120: mol_type = other DNA
aaaaaacctgctgaattccagcaggtttcaaattgttactatagattactatgagaagtgtacttcgtcaatttttttcttgaaggtgaaaaataggtatatcactctgttgagatagat

SEQ ID NO: 379 - DNA, 120 bp, synthetic construct
  source 1..120: mol_type = other DNA
tacttcgtcaatttttttcttgaaggtgaaaaataggtatatcactctgttgagatagatggatcagcctgctctttcttcgggatgatttcaaaaaactgttgctgcatatcatcgagt

SEQ ID NO: 380 - DNA, 120 bp, synthetic construct
  source 1..120: mol_type = other DNA
ggatcagcctgctctttcttcgggatgatttcaaaaaactgttgctgcatatcatcgagtaacggtgttaacaaagcaacttcttcatattgttcatgttcatttaatacacggatataa

SEQ ID NO: 381 - DNA, 120 bp, synthetic construct
  source 1..120: mol_type = other DNA
aacggtgttaacaaagcaacttcttcatattgttcatgttcatttaatacacggatataatctagtaataactcgtttacatctcgcacaccatttttactaattggttgcaatgtaaca

SEQ ID NO: 382 - DNA, 120 bp, synthetic construct
  source 1..120: mol_type = other DNA
tctagtaataactcgtttacatctcgcacaccatttttactaattggttgcaatgtaacatttgctccttttgcgattcttctttttaaggcctgttctgttaaacctaagcttgaatca

SEQ ID NO: 383 - DNA, 120 bp, synthetic construct
  source 1..120: mol_type = other DNA
tttgctccttttgcgattcttctttttaaggcctgttctgttaaacctaagcttgaatcatgacgtaaataaacaacgccgccagtcataccagcacagatccatggaccaggatcccct

SEQ ID NO: 384 - DNA, 120 bp, synthetic construct
  source 1..120: mol_type = other DNA
tgacgtaaataaacaacgccgccagtcataccagcacagatccatggaccaggatcccctaaaacaagcgctcgcccatttgtcatatattcaaaagcaaaacctttaatattagagtat

SEQ ID NO: 385 - DNA, 120 bp, synthetic construct
  source 1..120: mol_type = other DNA
aaaacaagcgctcgcccatttgtcatatattcaaaagcaaaacctttaatattagagtatgctcctatattcccttgctctttttcacggagtggctttgtcatgcgccctccaattatc

SEQ ID NO: 386 - DNA, 120 bp, synthetic construct
  source 1..120: mol_type = other DNA
gctcctatattcccttgctctttttcacggagtggctttgtcatgcgccctccaattatcatgtctgctccagagagacgaatgccagcgcgagcatcagcgttaccttgaacgtataac

SEQ ID NO: 387 - DNA, 120 bp, synthetic construct
  source 1..120: mol_type = other DNA
atgtctgctccagagagacgaatgccagcgcgagcatcagcgttaccttgaacgtataacgctcctttttgtgcaccgtatccaaaaccttttccgacagaaccgttataatataggcca

SEQ ID NO: 388 - DNA, 120 bp, synthetic construct
  source 1..120: mol_type = other DNA
gctcctttttgtgcaccgtatccaaaaccttttccgacagaaccgttataatataggccatcttttccttttgcttttgttatataaataccaccaccaaaggaggttttaccaatacca

SEQ ID NO: 389 - DNA, 120 bp, synthetic construct
  source 1..120: mol_type = other DNA
tcttttccttttgcttttgttatataaataccaccaccaaaggaggttttaccaataccatcttgtgcaccgccatttacatgtataaataaattttcactattgtaagcacctaatcca

SEQ ID NO: 390 - DNA, 120 bp, synthetic construct
  source 1..120: mol_type = other DNA
tcttgtgcaccgccatttacatgtataaataaattttcactattgtaagcacctaatccatttccaggaatcgagccattcgtatactttaatgtcagtggttcaagttttgtatcttca

SEQ ID NO: 391 - DNA, 120 bp, synthetic construct
  source 1..120: mol_type = other DNA
tttccaggaatcgagccattcgtatactttaatgtcagtggttcaagttttgtatcttcatataatttactacgcacgcgatagcaagattctagaccgcccataacgcgttgctctaca

SEQ ID NO: 392 - DNA, 120 bp, synthetic construct
  source 1..120: mol_type = other DNA
tataatttactacgcacgcgatagcaagattctagaccgcccataacgcgttgctctacaccaacgcctactaattcttttgaatgaggggaatgaatgggttcaaattgtttttctagt

SEQ ID NO: 393 - DNA, 120 bp, synthetic construct
  source 1..120: mol_type = other DNA
ccaacgcctactaattcttttgaatgaggggaatgaatgggttcaaattgtttttctagtacgtgttctgtttttataacagatggatgttctatcgtttgtagtaaattacataagttt

SEQ ID NO: 394 - DNA, 120 bp, synthetic construct
  source 1..120: mol_type = other DNA
acgtgttctgtttttataacagatggatgttctatcgtttgtagtaaattacataagtttaataaatttttgcctcgaacttgttctaataaatcagaccgcccgacaatttcttgtaag

SEQ ID NO: 395 - DNA, 120 bp, synthetic construct
  source 1..120: mol_type = other DNA
aataaatttttgcctcgaacttgttctaataaatcagaccgcccgacaatttcttgtaagtttgtatagccaagatttcctgttaatcgttttagttcttcaccaaaagtagtgaataaa

SEQ ID NO: 396 - DNA, 120 bp, synthetic construct
  source 1..120: mol_type = other DNA
tttgtatagccaagatttcctgttaatcgttttagttcttcaccaaaagtagtgaataaatgtaataatccagccacggcactttctagttcgcgtgggacgaagcggcgtaatccgtgt

SEQ ID NO: 397 - DNA, 120 bp, synthetic construct
  source 1..120: mol_type = other DNA
tgtaataatccagccacggcactttctagttcgcgtgggacgaagcggcgtaatccgtgttcttttgcctgagcttcagattcaatttgtgttgcaattccaacgtgacaagtatctaga

SEQ ID NO: 398 - DNA, 120 bp, synthetic construct
  source 1..120: mol_type = other DNA
tcttttgcctgagcttcagattcaatttgtgttgcaattccaacgtgacaagtatctagatgacatccgcggcaagttgtacagccgattgcaatcatggataatgtaccaaatccaatg

SEQ ID NO: 399 - DNA, 120 bp, synthetic construct
  source 1..120: mol_type = other DNA
tgacatccgcggcaagttgtacagccgattgcaatcatggataatgtaccaaatccaatgcgatttgctccgaggagcatgattttcaaggcatcattaacacttcgaataccaccatca

SEQ ID NO: 400 - DNA, 120 bp, synthetic construct
  source 1..120: mol_type = other DNA
cgatttgctccgaggagcatgattttcaaggcatcattaacacttcgaataccaccatcagcccaaatttctacgttatgtctcatatttgcttctaataaagcattgtgagcggctttc

SEQ ID NO: 401 - DNA, 120 bp, synthetic construct
  source 1..120: mol_type = other DNA
gcccaaatttctacgttatgtctcatatttgcttctaataaagcattgtgagcggctttcacaccaatttctacaggaaggcctacatgttgcaatgcgtgaatacgtgcagcccctgta

SEQ ID NO: 402 - DNA, 120 bp, synthetic construct
  source 1..120: mol_type = other DNA
acaccaatttctacaggaaggcctacatgttgcaatgcgtgaatacgtgcagcccctgtaccaccatcaaatccgctaatattaataaaatcagcaccagcttttgcgatgccaacagca

SEQ ID NO: 403 - DNA, 120 bp, synthetic construct
  source 1..120: mol_type = other DNA
ccaccatcaaatccgctaatattaataaaatcagcaccagcttttgcgatgccaacagcaattgttccaatattagggacaacaggaacctttacagctactttcgcaagttgattagcc

SEQ ID NO: 404 - DNA, 120 bp, synthetic construct
  source 1..120: mol_type = other DNA
attgttccaatattagggacaacaggaacctttacagctactttcgcaagttgattagccgttttaatttctgtaatcatttgagctaaatcttcaatggaataaatatcatggttgtta

SEQ ID NO: 405 - DNA, 120 bp, synthetic construct
  source 1..120: mol_type = other DNA
gttttaatttctgtaatcatttgagctaaatcttcaatggaataaatatcatggttgttagaaggtgaaattaaatctgagccaattgttgcattgcgtgcttcagcgattttggctgtt

SEQ ID NO: 406 - DNA, 120 bp, synthetic construct
  source 1..120: mol_type = other DNA
gaaggtgaaattaaatctgagccaattgttgcattgcgtgcttcagcgattttggctgttacttttgaacctggcaaatgtccaccttcaccaggctttgcgccttgcccaatttttatt

SEQ ID NO: 407 - DNA, 120 bp, synthetic construct
  source 1..120: mol_type = other DNA
acttttgaacctggcaaatgtccaccttcaccaggctttgcgccttgcccaatttttatttcaattaagtttgatgaatttagtagttcggcgtttacgccaaatcgcccagatgcaact

SEQ ID NO: 408 - DNA, 120 bp, synthetic construct
  source 1..120: mol_type = other DNA
tcaattaagtttgatgaatttagtagttcggcgtttacgccaaatcgcccagatgcaacttgttgtccacgtgtatgtggatattttccaatcatatctttaatttcgccgccttcaccg

SEQ ID NO: 409 - DNA, 120 bp, synthetic construct
  source 1..120: mol_type = other DNA
tgttgtccacgtgtatgtggatattttccaatcatatctttaatttcgccgccttcaccgttcaagctaatcatatttagctggtcggccgcttctgcatatgcacgaaaggcaatttca

SEQ ID NO: 410 - DNA, 120 bp, synthetic construct
  source 1..120: mol_type = other DNA
ttcaagctaatcatatttagctggtcggccgcttctgcatatgcacgaaaggcaatttcattttgagagccaaatgacatggaactaataataaatggtaaatcatgattttgaatactg

SEQ ID NO: 411 - DNA, 120 bp, synthetic construct
  source 1..120: mol_type = other DNA
ttttgagagccaaatgacatggaactaataataaatggtaaatcatgattttgaatactgatagatacctcttcagttggaatgacatgttttgtttctttcgtttgaataaggtgtcta

SEQ ID NO: 412 - DNA, 120 bp, synthetic construct
  source 1..120: mol_type = other DNA
atagatacctcttcagttggaatgacatgttttgtttctttcgtttgaataaggtgtctaatcgcaattggattattttcttctaattcacttaacttgtcacggtaatcatcataagag

SEQ ID NO: 413 - DNA, 120 bp, synthetic construct
  source 1..120: mol_type = other DNA
atcgcaattggattattttcttctaattcacttaacttgtcacggtaatcatcataagagtttccttttgcgacatcaccgattgctttccaaattcgcgggaatatatgaaaagatttt

SEQ ID NO: 414 - DNA, 120 bp, synthetic construct
  source 1..120: mol_type = other DNA
tttccttttgcgacatcaccgattgctttccaaattcgcgggaatatatgaaaagattttcgtattctaactttcggatcgttataatcatccgctcgcatttgtgcatcttcagcaagt

SEQ ID NO: 415 - DNA, 120 bp, synthetic construct
  source 1..120: mol_type = other DNA
cgtattctaactttcggatcgttataatcatccgctcgcatttgtgcatcttcagcaagtgattcaagagaaaaggctaaatcatttgaacctaagaaatttgtaatttgcaatatattt

SEQ ID NO: 416 - DNA, 120 bp, synthetic construct
  source 1..120: mol_type = other DNA
gattcaagagaaaaggctaaatcatttgaacctaagaaatttgtaatttgcaatatatttgcgatttcctcatgtaatccaatagaagaatagaggcgaccgtaaccacgcaattcatga

SEQ ID NO: 417 - DNA, 120 bp, synthetic construct
  source 1..120: mol_type = other DNA
gcgatttcctcatgtaatccaatagaagaatagaggcgaccgtaaccacgcaattcatgaattccaattgttgaaatgactttctccagtcctttattaagtgcattgtataaattcgta

SEQ ID NO: 418 - DNA, 120 bp, synthetic construct
  source 1..120: mol_type = other DNA
attccaattgttgaaatgactttctccagtcctttattaagtgcattgtataaattcgtaattggtgtttttgtcccatcatttacggttgcaaataataaatagggattaatactatct

SEQ ID NO: 419 - DNA, 120 bp, synthetic construct
  source 1..120: mol_type = other DNA
attggtgtttttgtcccatcatttacggttgcaaataataaatagggattaatactatctgctcctaatccatgcagtgtgacgatatcgtgtaaggagcgaagggcacccgagcgtata

SEQ ID NO: 420 - DNA, 120 bp, synthetic construct
  source 1..120: mol_type = other DNA
gctcctaatccatgcagtgtgacgatatcgtgtaaggagcgaagggcacccgagcgtataacgagagagcagtttcgacgtaatttattttcgcttaatacttgatgtactttagcagta

SEQ ID NO: 421 - DNA, 120 bp, synthetic construct
  source 1..120: mol_type = other DNA
acgagagagcagtttcgacgtaatttattttcgcttaatacttgatgtactttagcagtaactaaatgtggatcaatccataaccgttcatttagatgagcatcggcatcgtctattaat

SEQ ID NO: 422 - DNA, 120 bp, synthetic construct
  source 1..120: mol_type = other DNA
actaaatgtggatcaatccataaccgttcatttagatgagcatcggcatcgtctattaatagtagggaagctccatcgttcacggctgttatcgcttcagaactaattcgacttaaggcg

SEQ ID NO: 423 - DNA, 120 bp, synthetic construct
  source 1..120: mol_type = other DNA
agtagggaagctccatcgttcacggctgttatcgcttcagaactaattcgacttaaggcgcattgtaaagtttctgcctgactgaatgtagcagaaatggtagcgatagagctatgagtg

SEQ ID NO: 424 - DNA, 120 bp, synthetic construct
  source 1..120: mol_type = other DNA
cattgtaaagtttctgcctgactgaatgtagcagaaatggtagcgatagagctatgagtgttgaatagttctataagttgttcatacgtaattgtgtgtaattcctgtgcaatagattgt

SEQ ID NO: 425 - DNA, 120 bp, synthetic construct
  source 1..120: mol_type = other DNA
ttgaatagttctataagttgttcatacgtaattgtgtgtaattcctgtgcaatagattgtgccacgcttccttctaaaataatgggggaaagcatctcaactacaaatggttttttcgca

SEQ ID NO: 426 - DNA, 120 bp, synthetic construct
  source 1..120: mol_type = other DNA
gccacgcttccttctaaaataatgggggaaagcatctcaactacaaatggttttttcgcatcgcttaataaacttggtcgctctccaagtatcgttcgtgtggagaagtgttcgacctct

SEQ ID NO: 427 - DNA, 120 bp, synthetic construct
  source 1..120: mol_type = other DNA
tcgcttaataaacttggtcgctctccaagtatcgttcgtgtggagaagtgttcgacctctcgatcgcgatcgattgctgggtttgtaacaacagctacactttccttaatgaagtcagcg

SEQ ID NO: 428 - DNA, 120 bp, synthetic construct
  source 1..120: mol_type = other DNA
cgatcgcgatcgattgctgggtttgtaacaacagctacactttccttaatgaagtcagcgatatttcgtctatcagtatcgagtgcggcaagtggtgagtcatgcccaagtgagcggatt

SEQ ID NO: 429 - DNA, 120 bp, synthetic construct
  source 1..120: mol_type = other DNA
atatttcgtctatcagtatcgagtgcggcaagtggtgagtcatgcccaagtgagcggattggctcaacgccttttgttgccatctgttcaagaagctgaatatgttctcggtcccatccg

SEQ ID NO: 430 - DNA, 120 bp, synthetic construct
  source 1..120: mol_type = other DNA
ggctcaacgccttttgttgccatctgttcaagaagctgaatatgttctcggtcccatccgaaagcaacatattgtttcgtttcaacttgcatagaatcacatgcatctggaatttctttc

SEQ ID NO: 431 - DNA, 120 bp, synthetic construct
  source 1..120: mol_type = other DNA
aaagcaacatattgtttcgtttcaacttgcatagaatcacatgcatctggaatttctttcgttttagggatagataaatgtaaatgataattggtaacatccactttctttttaaaacgg

SEQ ID NO: 432 - DNA, 120 bp, synthetic construct
  source 1..120: mol_type = other DNA
gttttagggatagataaatgtaaatgataattggtaacatccactttctttttaaaacggttatatacttgagtttggtagtcgtcatgttcgtagagtacaagttcatcttgttcattc

SEQ ID NO: 433 - DNA, 120 bp, synthetic construct
  source 1..120: mol_type = other DNA
ttatatacttgagtttggtagtcgtcatgttcgtagagtacaagttcatcttgttcattccactttaggccgactttttctcctggagcgagtggttttggttctgctacatattcagtt

SEQ ID NO: 434 - DNA, 120 bp, synthetic construct
  source 1..120: mol_type = other DNA
cactttaggccgactttttctcctggagcgagtggttttggttctgctacatattcagttggtgatacaactccaggttcagaagagaaaatataagagctttctatttcaaccttccat

SEQ ID NO: 435 - DNA, 120 bp, synthetic construct
  source 1..120: mol_type = other DNA
ggtgatacaactccaggttcagaagagaaaatataagagctttctatttcaaccttccatactggtcgaagtccaagggaatccacgctgaaaacagcttcatctttataacgtgaaata

SEQ ID NO: 436 - DNA, 120 bp, synthetic construct
  source 1..120: mol_type = other DNA
actggtcgaagtccaagggaatccacgctgaaaacagcttcatctttataacgtgaaataatgccagctggaccttgcgcaaaatggccccatgcttcacgtatatacgtatataaatct

SEQ ID NO: 437 - DNA, 120 bp, synthetic construct
  source 1..120: mol_type = other DNA
atgccagctggaccttgcgcaaaatggccccatgcttcacgtatatacgtatataaatcttgtaaatgtgtttcataaagtttaatttcattaataattggtgggaatagtatatccatt

SEQ ID NO: 438 - DNA, 120 bp, synthetic construct
  source 1..120: mol_type = other DNA
tgtaaatgtgtttcataaagtttaatttcattaataattggtgggaatagtatatccattgcttcaaataaactgtagccgtattgaacaagtagagtttctaaggtgcggtttaaatct

SEQ ID NO: 439 - DNA, 120 bp, synthetic construct
  source 1..120: mol_type = other DNA
gcttcaaataaactgtagccgtattgaacaagtagagtttctaaggtgcggtttaaatcttgggagtcactgcccccagcagtaaggggaacgtgaatcatttcagcttgatcgcgtaat

SEQ ID NO: 440 - DNA, 120 bp, synthetic construct
  source 1..120: mol_type = other DNA
tgggagtcactgcccccagcagtaaggggaacgtgaatcatttcagcttgatcgcgtaattttgcaattgtgttaatttcaccattatgtccgagaatactaaatggttgtacacgaaaa

SEQ ID NO: 441 - DNA, 120 bp, synthetic construct
  source 1..120: mol_type = other DNA
tttgcaattgtgttaatttcaccattatgtccgagaatactaaatggttgtacacgaaaaaaattagataatgtattagtagaatagcgattgtgtcctagtgtcatagttgaagcgata

SEQ ID NO: 442 - DNA, 120 bp, synthetic construct
  source 1..120: mol_type = other DNA
aaattagataatgtattagtagaatagcgattgtgtcctagtgtcatagttgaagcgataagtgggtgttgtaaatcattgtaataggcaacaagtgtatccccagcaccgagaacttta

SEQ ID NO: 443 - DNA, 120 bp, synthetic construct
  source 1..120: mol_type = other DNA
agtgggtgttgtaaatcattgtaataggcaacaagtgtatccccagcaccgagaactttatatacaacgtgatcacgacttaaggaagcaacatgaatcgcttcgttttcctctattttt

SEQ ID NO: 444 - DNA, 120 bp, synthetic construct
  source 1..120: mol_type = other DNA
tatacaacgtgatcacgacttaaggaagcaacatgaatcgcttcgttttcctctatttttatcgttactgaaaataaggtttgctcaatatttacaacttcattttctgcgataagggca

SEQ ID NO: 445 - DNA, 120 bp, synthetic construct
  source 1..120: mol_type = other DNA
atcgttactgaaaataaggtttgctcaatatttacaacttcattttctgcgataagggcaacttgccaaaataaaggttcttcttgtttaccaagtggaccgagtgcatcggagtttatt

SEQ ID NO: 446 - DNA, 120 bp, synthetic construct
  source 1..120: mol_type = other DNA
acttgccaaaataaaggttcttcttgtttaccaagtggaccgagtgcatcggagtttattacattgtcactttcgaaaagaattgcaaagttttcgttgtttagttgtgtacgaatatga

SEQ ID NO: 447 - DNA, 120 bp, synthetic construct
  source 1..120: mol_type = other DNA
acattgtcactttcgaaaagaattgcaaagttttcgttgtttagttgtgtacgaatatgattttttaaatcaactatattctcgtttttgtttagaaaaaaatgtccaacgataaagtgg

SEQ ID NO: 448 - DNA, 120 bp, synthetic construct
  source 1..120: mol_type = other DNA
ttttttaaatcaactatattctcgtttttgtttagaaaaaaatgtccaacgataaagtggggatgatccacgatcgttggattatatccgctactttttaatttttcattccaaagagct

SEQ ID NO: 449 - DNA, 120 bp, synthetic construct
  source 1..120: mol_type = other DNA
ggatgatccacgatcgttggattatatccgctactttttaatttttcattccaaagagcttttggtacatcaatgtgaatgccgattccatcaccttcgccattaatgaagccagctcta

SEQ ID NO: 450 - DNA, 120 bp, synthetic construct
  source 1..120: mol_type = other DNA
tttggtacatcaatgtgaatgccgattccatcaccttcgccattaatgaagccagctctatgattcattttgacgagcgattgtatgcagaggtcaatgttttcttttgtaggaattttt

SEQ ID NO: 451 - DNA, 120 bp, synthetic construct
  source 1..120: mol_type = other DNA
tgattcattttgacgagcgattgtatgcagaggtcaatgttttcttttgtaggaatttttcgtttctccataacggaaacgattccacacgcatcatgttctgcatttttataatctcga

SEQ ID NO: 452 - DNA, 120 bp, synthetic construct
  source 1..120: mol_type = other DNA
cgtttctccataacggaaacgattccacacgcatcatgttctgcatttttataatctcgaaataaagacggtgtccatgtatttgttttattgagcatccgtcaatcccccctcttgtaa

SEQ ID NO: 453 - DNA, 120 bp, synthetic construct
  source 1..120: mol_type = other DNA
aataaagacggtgtccatgtatttgttttattgagcatccgtcaatcccccctcttgtaaaagttagaataatcttactatttaaggtgtagatcaccttgtacacagagatagtagtga

SEQ ID NO: 454 - DNA, 120 bp, synthetic construct
  source 1..120: mol_type = other DNA
aagttagaataatcttactatttaaggtgtagatcaccttgtacacagagatagtagtgatgtaaaagaatataaaacagataattatgaataattatactattaatacgggatttatga

SEQ ID NO: 455 - DNA, 120 bp, synthetic construct
  source 1..120: mol_type = other DNA
tgtaaaagaatataaaacagataattatgaataattatactattaatacgggatttatgaaatagaaaaaaggaaaaaagaaagatgtgctttctttttttccttttaatgatgagatta

SEQ ID NO: 456 - DNA, 120 bp, synthetic construct
  source 1..120: mol_type = other DNA
aatagaaaaaaggaaaaaagaaagatgtgctttctttttttccttttaatgatgagattatttattgtctgctaaagcagcaaatgctctgcctacagcttcaattgtatattcaatatc

SEQ ID NO: 457 - DNA, 120 bp, synthetic construct
  source 1..120: mol_type = other DNA
tttattgtctgctaaagcagcaaatgctctgcctacagcttcaattgtatattcaatatcttcttttgtatgctctgttgttaagaaccatgcctcgtatttagaaggtgctaagttaac

SEQ ID NO: 458 - DNA, 120 bp, synthetic construct
  source 1..120: mol_type = other DNA
ttcttttgtatgctctgttgttaagaaccatgcctcgtatttagaaggtgctaagttaacgccttcttgaagcattagcttgaagaatttgccgaacatttccccatctgtatcttgtgc

SEQ ID NO: 459 - DNA, 120 bp, synthetic construct
  source 1..120: mol_type = other DNA
gccttcttgaagcattagcttgaagaatttgccgaacatttccccatctgtatcttgtgctgcatcgtaatcttcaattgtatttgttgtgaagtatacagttaaagcaccttttagacg

SEQ ID NO: 460 - DNA, 120 bp, synthetic construct
  source 1..120: mol_type = other DNA
tgcatcgtaatcttcaattgtatttgttgtgaagtatacagttaaagcaccttttagacggtttaatgtaatatcgatattatgttttgcagcttgctctaaaattcctttttcaagcat

SEQ ID NO: 461 - DNA, 120 bp, synthetic construct
  source 1..120: mol_type = other DNA
gtttaatgtaatatcgatattatgttttgcagcttgctctaaaattcctttttcaagcattgcaccaagctcatctaatttctcataaagcccttcttgttgaagaacttctagacaagc

SEQ ID NO: 462 - DNA, 120 bp, synthetic construct
  source 1..120: mol_type = other DNA
tgcaccaagctcatctaatttctcataaagcccttcttgttgaagaacttctagacaagcaataccagatgccatagaagcaggatttcctgccattgtaccagcttgatatgcaggtcc

SEQ ID NO: 463 - DNA, 120 bp, synthetic construct
  source 1..120: mol_type = other DNA
aataccagatgccatagaagcaggatttcctgccattgtaccagcttgatatgcaggtccgagcggggcaacttgttccataatttctttcttaccaccgtaagcaccgattggtagtcc

SEQ ID NO: 464 - DNA, 120 bp, synthetic construct
  source 1..120: mol_type = other DNA
gagcggggcaacttgttccataatttctttcttaccaccgtaagcaccgattggtagtccgccgccgataactttaccaagcgctgttaagtctggtgttacgccaagtaagtcttgagc

SEQ ID NO: 465 - DNA, 120 bp, synthetic construct
  source 1..120: mol_type = other DNA
gccgccgataactttaccaagcgctgttaagtctggtgttacgccaagtaagtcttgagcgccaccgtacatgaagcggaaagcggtaataacttcatcataaattactaatgcaccagc

SEQ ID NO: 466 - DNA, 120 bp, synthetic construct
  source 1..120: mol_type = other DNA
gccaccgtacatgaagcggaaagcggtaataacttcatcataaattactaatgcaccagcttcatgaacaagttcattcactttctcaaggaagccaggttttggctctacaataccgaa

SEQ ID NO: 467 - DNA, 120 bp, synthetic construct
  source 1..120: mol_type = other DNA
ttcatgaacaagttcattcactttctcaaggaagccaggttttggctctacaataccgaagtttccaacaatcggttctacaagaatagctgctacctcatgtccccatttatctaatgc

SEQ ID NO: 468 - DNA, 120 bp, synthetic construct
  source 1..120: mol_type = other DNA
gtttccaacaatcggttctacaagaatagctgctacctcatgtccccatttatctaatgcttcttttaaagtttctacattattaaatggaacagtaataacttcttgagcgatactttg

SEQ ID NO: 469 - DNA, 120 bp, synthetic construct
  source 1..120: mol_type = other DNA
ttcttttaaagtttctacattattaaatggaacagtaataacttcttgagcgatactttgtggtacaccggctgagtcaggggttcctagtgtagaagggccagatccagctgctacaag

SEQ ID NO: 470 - DNA, 120 bp, synthetic construct
  source 1..120: mol_type = other DNA
tggtacaccggctgagtcaggggttcctagtgtagaagggccagatccagctgctacaagtactaaatcagaatgaccatggtaacaaccagcaaatttcataatttttgtgcggcctgt

SEQ ID NO: 471 - DNA, 120 bp, synthetic construct
  source 1..120: mol_type = other DNA
tactaaatcagaatgaccatggtaacaaccagcaaatttcataatttttgtgcggcctgtgtaagcacgagcgacacgaattgttgtcattactgcttcagtaccagagtttacgaagcg

SEQ ID NO: 472 - DNA, 120 bp, synthetic construct
  source 1..120: mol_type = other DNA
gtaagcacgagcgacacgaattgttgtcattactgcttcagtaccagagtttacgaagcggactttatctaatgcaggcattgcttcttttaacatttttgcaaattttacttctagtgc

SEQ ID NO: 473 - DNA, 120 bp, synthetic construct
  source 1..120: mol_type = other DNA
gactttatctaatgcaggcattgcttcttttaacatttttgcaaattttacttctagtgctgttggtgttccgtaaagtacaccattttcagcagcagttgtaattgcttttgtgatgtg

SEQ ID NO: 474 - DNA, 120 bp, synthetic construct
  source 1..120: mol_type = other DNA
tgttggtgttccgtaaagtacaccattttcagcagcagttgtaattgcttttgtgatgtgtgggtgagcgtgtccagtaataataggaccgtatgctgctaaataatcgatatatttatt

SEQ ID NO: 475 - DNA, 120 bp, synthetic construct
  source 1..120: mol_type = other DNA
tgggtgagcgtgtccagtaataataggaccgtatgctgctaaataatcgatatatttatttccgtctacatcccagaaataagcaccttttccgcgttccatagcaataggagcgccgcc

SEQ ID NO: 476 - DNA, 120 bp, synthetic construct
  source 1..120: mol_type = other DNA
tccgtctacatcccagaaataagcaccttttccgcgttccatagcaataggagcgccgccgccaactgctttaaaagaacgagaaggactattaacgccgccaacgatatgttctaaagc

SEQ ID NO: 477 - DNA, 120 bp, synthetic construct
  source 1..120: mol_type = other DNA
agcaataggagcgccgccgccaactgctttaaaagaacgagaaggactattaacgccgccaacgatatgttctaaagcttctttatgtaatgcttctgattttgtgaatttcactaccat

SEQ ID NO: 478 - DNA, 120 bp, synthetic construct
  source 1..120: mol_type = other DNA
tgaaaaaacgaaaagtgttaataccattaatggcattgtctacgatattagtttcaagcacaggtaatttagaggtgattcaggcagaagttaaacaggagaaccggttattaaatgaat

SEQ ID NO: 479 - DNA, 120 bp, synthetic construct
  source 1..120: mol_type = other DNA
caggtaatttagaggtgattcaggcagaagttaaacaggagaaccggttattaaatgaatcagaatcaagttcccaggggttactaggatactattttagtgatttgaattttcaagcac

SEQ ID NO: 480 - DNA, 120 bp, synthetic construct
  source 1..120: mol_type = other DNA
cagaatcaagttcccaggggttactaggatactattttagtgatttgaattttcaagcacccatggtggttacctcttctactacaggggatttatctattcctagttctgagttagaaa

SEQ ID NO: 481 - DNA, 120 bp, synthetic construct
  source 1..120: mol_type = other DNA
ccatggtggttacctcttctactacaggggatttatctattcctagttctgagttagaaaatattccatcggaaaaccaatattttcaatctgctatttggtcaggatttatcaaagtta

SEQ ID NO: 482 - DNA, 120 bp, synthetic construct
  source 1..120: mol_type = other DNA
atattccatcggaaaaccaatattttcaatctgctatttggtcaggatttatcaaagttaagaagagtgatgaatatacatttgctacttccgctgataatcatgtaacaatgtgggtag

SEQ ID NO: 483 - DNA, 120 bp, synthetic construct
  source 1..120: mol_type = other DNA
agaagagtgatgaatatacatttgctacttccgctgataatcatgtaacaatgtgggtagatgaccaagaagtgattaataaagcttctaattctaacaaaatcagattagaaaaaggaa

SEQ ID NO: 484 - DNA, 120 bp, synthetic construct
  source 1..120: mol_type = other DNA
atgaccaagaagtgattaataaagcttctaattctaacaaaatcagattagaaaaaggaagattatatcaaataaaaattcaatatcaacgagaaaatcctactgaaaaaggattggatt

SEQ ID NO: 485 - DNA, 120 bp, synthetic construct
  source 1..120: mol_type = other DNA
gattatatcaaataaaaattcaatatcaacgagaaaatcctactgaaaaaggattggatttcaagttgtactggaccgattctcaaaataaaaaagaagtgatttctagtgataacttac

SEQ ID NO: 486 - DNA, 120 bp, synthetic construct
  source 1..120: mol_type = other DNA
tcaagttgtactggaccgattctcaaaataaaaaagaagtgatttctagtgataacttacaattgccagaattaaaacaaaaatcttcgaactcaagaaaaaagcgaagtacaagtgctg

SEQ ID NO: 487 - DNA, 120 bp, synthetic construct
  source 1..120: mol_type = other DNA
aattgccagaattaaaacaaaaatcttcgaactcaagaaaaaagcgaagtacaagtgctggacctacggttccagaccgtgacaatgatggaatccctgattcattagaggtagaaggat

SEQ ID NO: 488 - DNA, 120 bp, synthetic construct
  source 1..120: mol_type = other DNA
gacctacggttccagaccgtgacaatgatggaatccctgattcattagaggtagaaggatatacggttgatgtcaaaaataaaagaacttttctttcaccatggatttctaatattcatg

SEQ ID NO: 489 - DNA, 120 bp, synthetic construct
  source 1..120: mol_type = other DNA
atacggttgatgtcaaaaataaaagaacttttctttcaccatggatttctaatattcatgaaaagaaaggattaaccaaatataaatcatctcctgaaaaatggagcacggcttctgatc

SEQ ID NO: 490 - DNA, 120 bp, synthetic construct
  source 1..120: mol_type = other DNA
aaaagaaaggattaaccaaatataaatcatctcctgaaaaatggagcacggcttctgatccgtacagtgatttcgaaaaggttacaggacggattgataagaatgtatcaccagaggcaa

SEQ ID NO: 491 - DNA, 120 bp, synthetic construct
  source 1..120: mol_type = other DNA
cgtacagtgatttcgaaaaggttacaggacggattgataagaatgtatcaccagaggcaagacacccccttgtggcagcttatccgattgtacatgtagatatggagaatattattctct

SEQ ID NO: 492 - DNA, 120 bp, synthetic construct
  source 1..120: mol_type = other DNA
gacacccccttgtggcagcttatccgattgtacatgtagatatggagaatattattctctcaaaaaatgaggatcaatccacacagaatactgatagtcaaacgagaacaataagtaaaa

SEQ ID NO: 493 - DNA, 120 bp, synthetic construct
  source 1..120: mol_type = other DNA
caaaaaatgaggatcaatccacacagaatactgatagtcaaacgagaacaataagtaaaaatacttctacaagtaggacacatactagtgaagtacatggaaatgcagaagtgcatgcgt

SEQ ID NO: 494 - DNA, 120 bp, synthetic construct
  source 1..120: mol_type = other DNA
atacttctacaagtaggacacatactagtgaagtacatggaaatgcagaagtgcatgcgtcgttctttgatattggtgggagtgtatctgcaggatttagtaattcgaattcaagtacgg

SEQ ID NO: 495 - DNA, 120 bp, synthetic construct
  source 1..120: mol_type = other DNA
cgttctttgatattggtgggagtgtatctgcaggatttagtaattcgaattcaagtacggtcgcaattgatcattcactatctctagcaggggaaagaacttgggctgaaacaatgggtt

SEQ ID NO: 496 - DNA, 120 bp, synthetic construct
  source 1..120: mol_type = other DNA
tcgcaattgatcattcactatctctagcaggggaaagaacttgggctgaaacaatgggtttaaataccgctgatacagcaagattaaatgccaatattagatatgtaaatactgggacgg

SEQ ID NO: 497 - DNA, 120 bp, synthetic construct
  source 1..120: mol_type = other DNA
taaataccgctgatacagcaagattaaatgccaatattagatatgtaaatactgggacggctccaatctacaacgtgttaccaacgacttcgttagtgttaggaaaaaatcaaacactcg

SEQ ID NO: 498 - DNA, 120 bp, synthetic construct
  source 1..120: mol_type = other DNA
ctccaatctacaacgtgttaccaacgacttcgttagtgttaggaaaaaatcaaacactcgcgacaattaaagctaaggaaaaccaattaagtcaaatacttgcacctaataattattatc

SEQ ID NO: 499 - DNA, 120 bp, synthetic construct
  source 1..120: mol_type = other DNA
cgacaattaaagctaaggaaaaccaattaagtcaaatacttgcacctaataattattatccttctaaaaacttggcgccaatcgcattaaatgcacaagacgatttcagttctactccaa

SEQ ID NO: 500 - DNA, 120 bp, synthetic construct
  source 1..120: mol_type = other DNA
cttctaaaaacttggcgccaatcgcattaaatgcacaagacgatttcagttctactccaattacaatgaattacaatcaatttcttgagttagaaaaaacgaaacaattaagattagata

SEQ ID NO: 501 - DNA, 120 bp, synthetic construct
  source 1..120: mol_type = other DNA
ttacaatgaattacaatcaatttcttgagttagaaaaaacgaaacaattaagattagatacggatcaagtatatgggaatatagcaacatacaattttgaaaatggaagagtgagggtgg

SEQ ID NO: 502 - DNA, 120 bp, synthetic construct
  source 1..120: mol_type = other DNA
cggatcaagtatatgggaatatagcaacatacaattttgaaaatggaagagtgagggtggatacaggctcgaactggagtgaagtgttaccgcaaattcaagaaacaactgcacgtatca

SEQ ID NO: 503 - DNA, 120 bp, synthetic construct
  source 1..120: mol_type = other DNA
atacaggctcgaactggagtgaagtgttaccgcaaattcaagaaacaactgcacgtatcatttttaatggaaaagatttaaatctggtagaaaggcggatagcggcggttaatcctagtg

SEQ ID NO: 504 - DNA, 120 bp, synthetic construct
  source 1..120: mol_type = other DNA
tttttaatggaaaagatttaaatctggtagaaaggcggatagcggcggttaatcctagtgatccattagaaacgactaaaccggatatgacattaaaagaagcccttaaaatagcatttg

SEQ ID NO: 505 - DNA, 120 bp, synthetic construct
  source 1..120: mol_type = other DNA
atccattagaaacgactaaaccggatatgacattaaaagaagcccttaaaatagcatttggatttaacgaaccgaatggaaacttacaatatcaagggaaagacataaccgaatttgatt

SEQ ID NO: 506 - DNA, 120 bp, synthetic construct
  source 1..120: mol_type = other DNA
gatttaacgaaccgaatggaaacttacaatatcaagggaaagacataaccgaatttgattttaatttcgatcaacaaacatctcaaaatatcaagaatcagttagcggaattaaacgcaa

SEQ ID NO: 507 - DNA, 120 bp, synthetic construct
  source 1..120: mol_type = other DNA
ttaatttcgatcaacaaacatctcaaaatatcaagaatcagttagcggaattaaacgcaactaacatatatactgtattagataaaatcaaattaaatgcaaaaatgaatattttaataa

SEQ ID NO: 508 - DNA, 120 bp, synthetic construct
  source 1..120: mol_type = other DNA
ctaacatatatactgtattagataaaatcaaattaaatgcaaaaatgaatattttaataagagataaacgttttcattatgatagaaataacatagcagttggggcggatgagtcagtag

SEQ ID NO: 509 - DNA, 120 bp, synthetic construct
  source 1..120: mol_type = other DNA
gagataaacgttttcattatgatagaaataacatagcagttggggcggatgagtcagtagttaaggaggctcatagagaagtaattaattcgtcaacagagggattattgttaaatattg

SEQ ID NO: 510 - DNA, 120 bp, synthetic construct
  source 1..120: mol_type = other DNA
ttaaggaggctcatagagaagtaattaattcgtcaacagagggattattgttaaatattgataaggatataagaaaaatattatcaggttatattgtagaaattgaagatactgaagggc

SEQ ID NO: 511 - DNA, 120 bp, synthetic construct
  source 1..120: mol_type = other DNA
ataaggatataagaaaaatattatcaggttatattgtagaaattgaagatactgaagggcttaaagaagttataaatgacagatatgatatgttgaatatttctagtttacggcaagatg

SEQ ID NO: 512 - DNA, 120 bp, synthetic construct
  source 1..120: mol_type = other DNA
ttaaagaagttataaatgacagatatgatatgttgaatatttctagtttacggcaagatggaaaaacatttatagattttaaaaaatataatgataaattaccgttatatataagtaatc

SEQ ID NO: 513 - DNA, 120 bp, synthetic construct
  source 1..120: mol_type = other DNA
gaaaaacatttatagattttaaaaaatataatgataaattaccgttatatataagtaatcccaattataaggtaaatgtatatgctgttactaaagaaaacactattattaatcctagtg

SEQ ID NO: 514 - DNA, 120 bp, synthetic construct
  source 1..120: mol_type = other DNA
ccaattataaggtaaatgtatatgctgttactaaagaaaacactattattaatcctagtgagaatggggatactagtaccaacgggatcaagaaaattttaatcttttctaaaaaaggct

SEQ ID NO: 515 - DNA, 120 bp, synthetic construct
  source 1..120: mol_type = other DNA
agaatggggatactagtaccaacgggatcaagaaaattttaatcttttctaaaaaaggctatgagataggataaggtaattctaggtgatttttaaattatctaaaaaacagtaaaatta

SEQ ID NO: 516 - DNA, 120 bp, synthetic construct
  source 1..120: mol_type = other DNA
atgagataggataaggtaattctaggtgatttttaaattatctaaaaaacagtaaaattaaaacatactctttttgtaagaaatacaaggagagtatgttttaaacagtaatctaaatca

SEQ ID NO: 517 - DNA, 120 bp, synthetic construct
  source 1..120: mol_type = other DNA
aaacatactctttttgtaagaaatacaaggagagtatgttttaaacagtaatctaaatcatcataatcctttgagattgtttgtaggatccataaaaacttagagaaaatgaaacatcca

SEQ ID NO: 518 - DNA, 120 bp, synthetic construct
  source 1..120: mol_type = other DNA
tcataatcctttgagattgtttgtaggatccataaaaacttagagaaaatgaaacatccaatgattctatatacaattgtgcgaagtatctggagtttagaaagcacagaaaaatttaat

SEQ ID NO: 519 - DNA, 120 bp, synthetic construct
  source 1..120: mol_type = other DNA
atgattctatatacaattgtgcgaagtatctggagtttagaaagcacagaaaaatttaattagaggacaattgcacattcaataagatatctataatatattgatgctcaaaataaaggt

SEQ ID NO: 520 - DNA, 120 bp, synthetic construct
  source 1..120: mol_type = other DNA
tagaggacaattgcacattcaataagatatctataatatattgatgctcaaaataaaggttcatgccttaaggaatgtagtaaaggtgtgctgttcaggtgcagaaacggttctatgtat

SEQ ID NO: 521 - DNA, 120 bp, synthetic construct
  source 1..120: mol_type = other DNA
tcatgccttaaggaatgtagtaaaggtgtgctgttcaggtgcagaaacggttctatgtattaaggtaagggtgtcttactaacagcatagcagaaatctatattgcgaaaagactttaat

SEQ ID NO: 522 - DNA, 120 bp, synthetic construct
  source 1..120: mol_type = other DNA
taaggtaagggtgtcttactaacagcatagcagaaatctatattgcgaaaagactttaattattataggtagttagtagattagacgaaacgagcgccaatgaactaattacactacatt

SEQ ID NO: 523 - DNA, 120 bp, synthetic construct
  source 1..120: mol_type = other DNA
tattataggtagttagtagattagacgaaacgagcgccaatgaactaattacactacattaatgagcaaaagttaatacggtaaatagatagtatgattgaaattgataaggaccacaag

SEQ ID NO: 524 - DNA, 120 bp, synthetic construct
  source 1..120: mol_type = other DNA
aatgagcaaaagttaatacggtaaatagatagtatgattgaaattgataaggaccacaagagcgtggcaaatatattgaaagagaaagcaactgccaaaaatattcttctgttggaaaag

SEQ ID NO: 525 - DNA, 120 bp, synthetic construct
  source 1..120: mol_type = other DNA
agcgtggcaaatatattgaaagagaaagcaactgccaaaaatattcttctgttggaaaagataaaagtggtaatttaggaatatagtttatataatttatcacgatatagggactatact

SEQ ID NO: 526 - DNA, 120 bp, synthetic construct
  source 1..120: mol_type = other DNA
ataaaagtggtaatttaggaatatagtttatataatttatcacgatatagggactatactctaaatcaattaatagaaaatatgaggttaaagaatctatacatttcttgttttatttct

SEQ ID NO: 527 - DNA, 120 bp, synthetic construct
  source 1..120: mol_type = other DNA
ctaaatcaattaatagaaaatatgaggttaaagaatctatacatttcttgttttatttctttataatttaatttaaaaatactataaaaatcctaaattagatattaaaaatagtgtgcg

SEQ ID NO: 528 - DNA, 120 bp, synthetic construct
  source 1..120: mol_type = other DNA
ttataatttaatttaaaaatactataaaaatcctaaattagatattaaaaatagtgtgcgaaagttcttaaaaacttaatattaaaatcatattaatattatacattagaattatataat

SEQ ID NO: 529 - DNA, 120 bp, synthetic construct
  source 1..120: mol_type = other DNA
aaagttcttaaaaacttaatattaaaatcatattaatattatacattagaattatataatcagtttattatacaaaacatcacaatgtacgaacataataatgtcatattattaaaaggt

SEQ ID NO: 530 - DNA, 120 bp, synthetic construct
  source 1..120: mol_type = other DNA
cagtttattatacaaaacatcacaatgtacgaacataataatgtcatattattaaaaggttaaactacattaaaacataaagagagaggaattgctatgacagtatttgtagatcataaa

SEQ ID NO: 531 - DNA, 120 bp, synthetic construct
  source 1..120: mol_type = other DNA
taaactacattaaaacataaagagagaggaattgctatgacagtatttgtagatcataaaattgaatacatgagtttagaagatgatgctgaacttttaaaaacaatggcacatcctatg

SEQ ID NO: 532 - DNA, 120 bp, synthetic construct
  source 1..120: mol_type = other DNA
attgaatacatgagtttagaagatgatgctgaacttttaaaaacaatggcacatcctatgcgtttaaaaatagtcaatgaactttacaaacataaagcattaaatgtaacgcaaatcatt

SEQ ID NO: 533 - DNA, 120 bp, synthetic construct
  source 1..120: mol_type = other DNA
cgtttaaaaatagtcaatgaactttacaaacataaagcattaaatgtaacgcaaatcattcaaatcttaaaactaccacaatcaactgtatcccagcatttatgtaaaatgagaggaaaa

SEQ ID NO: 534 - DNA, 120 bp, synthetic construct
  source 1..120: mol_type = other DNA
caaatcttaaaactaccacaatcaactgtatcccagcatttatgtaaaatgagaggaaaagttttaaaaagaaatcgacaaggtttagagatatactatagcattaataatccaaaagtt

SEQ ID NO: 535 - DNA, 120 bp, synthetic construct
  source 1..120: mol_type = other DNA
catttatgtaaaatgagaggaaaagttttaaaaagaaatcgacaaggtttagagatatactatagcattaataatccaaaagttgaagggattattaagttgttaaaccctatccaatag

SEQ ID NO: 536 - DNA, 120 bp, synthetic construct
  source 1..120: mol_type = other DNA
taaatcacttttgcttgctttttgccaatttgttcttccataatcatatcgattaatggctcagctgcaccatgaatattacccactccatatacaatccgattttttaaatatggacgc

SEQ ID NO: 537 - DNA, 120 bp, synthetic construct
  source 1..120: mol_type = other DNA
tcagctgcaccatgaatattacccactccatatacaatccgattttttaaatatggacgcatacgagacataatttcacttgttgaccagccttctaagttccaatactcttgcgttgga

SEQ ID NO: 538 - DNA, 120 bp, synthetic construct
  source 1..120: mol_type = other DNA
atacgagacataatttcacttgttgaccagccttctaagttccaatactcttgcgttggaatatctcctttttcaaaagcacttgtaataggtgcagtcgtttctccaatcgcaataact

SEQ ID NO: 539 - DNA, 120 bp, synthetic construct
  source 1..120: mol_type = other DNA
atatctcctttttcaaaagcacttgtaataggtgcagtcgtttctccaatcgcaataactatttccgctttaatatatggcaaaacatccctagcaaactgctcagtacgatcaacgcgg

SEQ ID NO: 540 - DNA, 120 bp, synthetic construct
  source 1..120: mol_type = other DNA
atttccgctttaatatatggcaaaacatccctagcaaactgctcagtacgatcaacgcggtcagggcggcaattcataattacaattggagctagattactatatccaaaatcatccaca

SEQ ID NO: 541 - DNA, 120 bp, synthetic construct
  source 1..120: mol_type = other DNA
tcagggcggcaattcataattacaattggagctagattactatatccaaaatcatccacacgttcccaaatacgtaatgttgatgagggatcattcgctgcaaaaccatttacgaagaac

SEQ ID NO: 542 - DNA, 120 bp, synthetic construct
  source 1..120: mol_type = other DNA
cgttcccaaatacgtaatgttgatgagggatcattcgctgcaaaaccatttacgaagaacgcaggcttagattggtcagcaaaacgtgtaattctcattgctcctggatccggatgagca

SEQ ID NO: 543 - DNA, 120 bp, synthetic construct
  source 1..120: mol_type = other DNA
gcaggcttagattggtcagcaaaacgtgtaattctcattgctcctggatccggatgagcattcaacataccacggaatgctgtttcctcatcaatcccaagagcctctgctaccgctaaa

SEQ ID NO: 544 - DNA, 120 bp, synthetic construct
  source 1..120: mol_type = other DNA
ttcaacataccacggaatgctgtttcctcatcaatcccaagagcctctgctaccgctaaagcaagcgatgcattatctgggaagaccatgtaatcaaattttcgtaagaattcttctgaa

SEQ ID NO: 545 - DNA, 120 bp, synthetic construct
  source 1..120: mol_type = other DNA
gcaagcgatgcattatctgggaagaccatgtaatcaaattttcgtaagaattcttctgaaattctagaattatccgcaacaatcacttttgtatttctctcttctgcaacctctttaaag

SEQ ID NO: 546 - DNA, 120 bp, synthetic construct
  source 1..120: mol_type = other DNA
attctagaattatccgcaacaatcacttttgtatttctctcttctgcaacctctttaaagtaatccaagtattcactttcaatagtgactaaatgtccattatatggaatggtagcagtg

SEQ ID NO: 547 - DNA, 120 bp, synthetic construct
  source 1..120: mol_type = other DNA
taatccaagtattcactttcaatagtgactaaatgtccattatatggaatggtagcagtgaaagcttcagctacttcgtcaagtgtaggtcccataacatccatatgatcttctaaaaca

SEQ ID NO: 548 - DNA, 120 bp, synthetic construct
  source 1..120: mol_type = other DNA
aaagcttcagctacttcgtcaagtgtaggtcccataacatccatatgatcttctaaaacatttacaatcactccaacatttgcttgaatcattttattttggaagataatttgataatcg

SEQ ID NO: 549 - DNA, 120 bp, synthetic construct
  source 1..120: mol_type = other DNA
tttacaatcactccaacatttgcttgaatcattttattttggaagataatttgataatcgggttgaactgccatacattcacaaataagtgcttctgcttctaaatcagcagcctcttta

SEQ ID NO: 550 - DNA, 120 bp, synthetic construct
  source 1..120: mol_type = other DNA
ggttgaactgccatacattcacaaataagtgcttctgcttctaaatcagcagcctctttaactaccctgcgttgctcaccgatattaggaccttctttacggcgcttaatcggttgctcc

SEQ ID NO: 551 - DNA, 120 bp, synthetic construct
  source 1..120: mol_type = other DNA
actaccctgcgttgctcaccgatattaggaccttctttacggcgcttaatcggttgctcctcgtcagtaaaccaatatatcattcgcgcagatgtaccagttgttttccctacagtctta

SEQ ID NO: 552 - DNA, 120 bp, synthetic construct
  source 1..120: mol_type = other DNA
tcgtcagtaaaccaatatatcattcgcgcagatgtaccagttgttttccctacagtcttatatttcgcttcttgtacaacacctgtaattagtcttgtaacggtagatttacctcgaatt

SEQ ID NO: 553 - DNA, 120 bp, synthetic construct
  source 1..120: mol_type = other DNA
tatttcgcttcttgtacaacacctgtaattagtcttgtaacggtagatttacctcgaattccatttatgtttactcgaattgggatagaattgagccttttctgatggcaacgttgttcc

SEQ ID NO: 554 - DNA, 120 bp, synthetic construct
  source 1..120: mol_type = other DNA
ccatttatgtttactcgaattgggatagaattgagccttttctgatggcaacgttgttcccatataccataaataatcaaaaacactgtacatatacctattatgaagatcatctgtatt

SEQ ID NO: 555 - DNA, 120 bp, synthetic construct
  source 1..120: mol_type = other DNA
catataccataaataatcaaaaacactgtacatatacctattatgaagatcatctgtattaatcccttcctgcttttcgatttcttgcttattaagatatttcgacttaagtagagtcgt

SEQ ID NO: 556 - DNA, 120 bp, synthetic construct
  source 1..120: mol_type = other DNA
aatcccttcctgcttttcgatttcttgcttattaagatatttcgacttaagtagagtcgttgataccaattaaaaattaggtggttccctgcatatacaacaccgaattcatctgagtat

SEQ ID NO: 557 - DNA, 120 bp, synthetic construct
  source 1..120: mol_type = other DNA
tgataccaattaaaaattaggtggttccctgcatatacaacaccgaattcatctgagtataattctgaaatcctatgttcaatgcgtattgcctcatcatgtttcaatattcttacaatt

SEQ ID NO: 558 - DNA, 120 bp, synthetic construct
  source 1..120: mol_type = other DNA
aattaggtggttccctgcatatacaacaccgaattcatctgagtataattctgaaatcctatgttcaatgcgtattgcctcatcatgtttcaatattcttacaatttttatgtttttcat

SEQ ID NO: 559 - DNA, 120 bp, synthetic construct
  source 1..120: mol_type = other DNA
tgtgcgatttgttatcttgccgccataagaatgacaagcgctatctgttatccccatataagcttccgtttcaacaattctggtaactatttcctctttgtcgatctttctgatcaacaa

SEQ ID NO: 560 - DNA, 120 bp, synthetic construct
  source 1..120: mol_type = other DNA
agcttccgtttcaacaattctggtaactatttcctctttgtcgatctttctgatcaacaaattaccaagcaataactttgcaacggtagtagcatcttgcaaaaaaaaatatcgatccat

SEQ ID NO: 561 - DNA, 120 bp, synthetic construct
  source 1..120: mol_type = other DNA
attaccaagcaataactttgcaacggtagtagcatcttgcaaaaaaaaatatcgatccataagctcaattttaaaacaaaataataataaaaattattaccaaaacacacatgtaaaata

SEQ ID NO: 562 - DNA, 120 bp, synthetic construct
  source 1..120: mol_type = other DNA
aagctcaattttaaaacaaaataataataaaaattattaccaaaacacacatgtaaaatatgaaaacatattgcctagaataaaaataaaaactaaaatcatttaatcacccagtaaata

SEQ ID NO: 563 - DNA, 120 bp, synthetic construct
  source 1..120: mol_type = other DNA
tgaaaacatattgcctagaataaaaataaaaactaaaatcatttaatcacccagtaaatacatattttaaataaattcttggttgattaataaatttttttgattaaaaatcaaaaaaat

SEQ ID NO: 564 - DNA, 120 bp, synthetic construct
  source 1..120: mol_type = other DNA
catattttaaataaattcttggttgattaataaatttttttgattaaaaatcaaaaaaatttaaaaagttgaactagttcaacttaaatcagcttatatgaaaatgctaatctaaaatac

SEQ ID NO: 565 - DNA, 120 bp, synthetic construct
  source 1..120: mol_type = other DNA
ttaaaaagttgaactagttcaacttaaatcagcttatatgaaaatgctaatctaaaatacaaaatatcgaatattgacaaatatataaaaattataaactatatgcaatatctcttacat

SEQ ID NO: 566 - DNA, 120 bp, synthetic construct
  source 1..120: mol_type = other DNA
aaaatatcgaatattgacaaatatataaaaattataaactatatgcaatatctcttacatcttgaaaagatataagagatattgacaaaatcataagatttaaataaaatttgtaaagaa

SEQ ID NO: 567 - DNA, 120 bp, synthetic construct
  source 1..120: mol_type = other DNA
cttgaaaagatataagagatattgacaaaatcataagatttaaataaaatttgtaaagaattgatatgcttaagggatcatagctcaggtggttagagcgcaggtctgataaacctgagg

SEQ ID NO: 568 - DNA, 120 bp, synthetic construct
  source 1..120: mol_type = other DNA
ttgatatgcttaagggatcatagctcaggtggttagagcgcaggtctgataaacctgaggtcggatgttcaactcatcctggtcccaatgtattccattgttttaattacgacaatactg

SEQ ID NO: 569 - DNA, 120 bp, synthetic construct
  source 1..120: mol_type = other DNA
tcggatgttcaactcatcctggtcccaatgtattccattgttttaattacgacaatactgttttaagctataattaataagaaaaacaaaaatttattcaatttctatattaaggtatac

SEQ ID NO: 570 - DNA, 120 bp, synthetic construct
  source 1..120: mol_type = other DNA
ttttaagctataattaataagaaaaacaaaaatttattcaatttctatattaaggtatacacgattactaacaattacaacttcatgccattgagtgtcgggcaaatccaaactgaaatc

SEQ ID NO: 571 - DNA, 120 bp, synthetic construct
  source 1..120: mol_type = other DNA
acgattactaacaattacaacttcatgccattgagtgtcgggcaaatccaaactgaaatctgctttatagtattttgcttagcttttttgagttattgttgcaaacttgtaacctaaaac

SEQ ID NO: 572 - DNA, 120 bp, synthetic construct
  source 1..120: mol_type = other DNA
tgctttatagtattttgcttagcttttttgagttattgttgcaaacttgtaacctaaaacataagagcgataacgatttaatgcaatctttgccttcctccaacttataactggcaatct

SEQ ID NO: 573 - DNA, 120 bp, synthetic construct
  source 1..120: mol_type = other DNA
ataagagcgataacgatttaatgcaatctttgccttcctccaacttataactggcaatcttatccgaatccctaccactaaatactggcaacgataataaggatttaagctcgctacaat

SEQ ID NO: 574 - DNA, 120 bp, synthetic construct
  source 1..120: mol_type = other DNA
tatccgaatccctaccactaaatactggcaacgataataaggatttaagctcgctacaatacttgtccctctctcagacatcacacttagtaatctacattatttcctaactaaaaacta

SEQ ID NO: 575 - DNA, 120 bp, synthetic construct
  source 1..120: mol_type = other DNA
acttgtccctctctcagacatcacacttagtaatctacattatttcctaactaaaaactatttactaaatgcagatcgtttataaaataggctgctgaaaaatacaatcctgtttaatcc

SEQ ID NO: 576 - DNA, 120 bp, synthetic construct
  source 1..120: mol_type = other DNA
tttactaaatgcagatcgtttataaaataggctgctgaaaaatacaatcctgtttaatccttgcactttagcgaaacaacttcgggttttatcgaaagcttgcttttgcttctagacatt

SEQ ID NO: 577 - DNA, 120 bp, synthetic construct
  source 1..120: mol_type = other DNA
ttgcactttagcgaaacaacttcgggttttatcgaaagcttgcttttgcttctagacatttttcttaatatcaacagatctcaacttaacccagaaattttaacttcttgtgtttcacat

SEQ ID NO: 578 - DNA, 120 bp, synthetic construct
  source 1..120: mol_type = other DNA
tttcttaatatcaacagatctcaacttaacccagaaattttaacttcttgtgtttcacattccaacaattactttaacaaagttacttaaaaacatacttaattacaatttagggcataa

SEQ ID NO: 579 - DNA, 120 bp, synthetic construct
  source 1..120: mol_type = other DNA
tccaacaattactttaacaaagttacttaaaaacatacttaattacaatttagggcataagcccaatggaggttaagggactcgaacccttgaccctcggcttgcaaagccgatgctcta

SEQ ID NO: 580 - DNA, 120 bp, synthetic construct
  source 1..120: mol_type = other DNA
gcccaatggaggttaagggactcgaacccttgaccctcggcttgcaaagccgatgctctagccaactgagctaaacccccaaaatgacctaaaattaagtctaagcctaataaaactatt

SEQ ID NO: 581 - DNA, 120 bp, synthetic construct
  source 1..120: mol_type = other DNA
gccaactgagctaaacccccaaaatgacctaaaattaagtctaagcctaataaaactatttaatatcaataatttaatacataaacttctcttaaacttacataaataacactggtttta

SEQ ID NO: 582 - DNA, 120 bp, synthetic construct
  source 1..120: mol_type = other DNA
taatatcaataatttaatacataaacttctcttaaacttacataaataacactggttttaaaaactctcttatcaaaagaaaagagtagggaagagttaatggaattagccttagtttat

SEQ ID NO: 583 - DNA, 120 bp, synthetic construct
  source 1..120: mol_type = other DNA
aaaactctcttatcaaaagaaaagagtagggaagagttaatggaattagccttagtttatctttctcttagaaaggaggtgatccagccgcactttccagtacggctaccttgttacgac

SEQ ID NO: 584 - DNA, 120 bp, synthetic construct
  source 1..120: mol_type = other DNA
ctttctcttagaaaggaggtgatccagccgcactttccagtacggctaccttgttacgacttcacccccctcactaaacataccttaaataccttcctcccttacgggttagaataatag

SEQ ID NO: 585 - DNA, 120 bp, synthetic construct
  source 1..120: mol_type = other DNA
ttcacccccctcactaaacataccttaaataccttcctcccttacgggttagaataatagcttcgggtatcctcaactcgggtggtgtgacgggcggtgtgtacaaggcccgagaacgta

SEQ ID NO: 586 - DNA, 120 bp, synthetic construct
  source 1..120: mol_type = other DNA
cttcgggtatcctcaactcgggtggtgtgacgggcggtgtgtacaaggcccgagaacgtattcaccgtatcattctgatatacgattactagcgattccaacttcatgaagtcgagtttc

SEQ ID NO: 587 - DNA, 120 bp, synthetic construct
  source 1..120: mol_type = other DNA
ttcaccgtatcattctgatatacgattactagcgattccaacttcatgaagtcgagtttcagacttcaatccggactgagacctgctttatgcgttttgcttcacatcactgtttcgctt

SEQ ID NO: 588 - DNA, 120 bp, synthetic construct
  source 1..120: mol_type = other DNA
agacttcaatccggactgagacctgctttatgcgttttgcttcacatcactgtttcgcttcgctttgtacaggccattgtagcacgtgtgtagcccaggacataagggccatgatgattt

SEQ ID NO: 589 - DNA, 120 bp, synthetic construct
  source 1..120: mol_type = other DNA
cgctttgtacaggccattgtagcacgtgtgtagcccaggacataagggccatgatgatttgacgtcatcctcaccttcctccgacttatcaccggcagtcttatctgagtccccaccatt

SEQ ID NO: 590 - DNA, 120 bp, synthetic construct
  source 1..120: mol_type = other DNA
gacgtcatcctcaccttcctccgacttatcaccggcagtcttatctgagtccccaccattacatgctggtaacagataacaagggttgcgctcgttgcgggacttaacccaacacctcac

SEQ ID NO: 591 - DNA, 120 bp, synthetic construct
  source 1..120: mol_type = other DNA
acatgctggtaacagataacaagggttgcgctcgttgcgggacttaacccaacacctcacagcacgagctgacgacaaccatgcagcacctgtatatagaccccaaacggggaataatta

SEQ ID NO: 592 - DNA, 120 bp, synthetic construct
  source 1..120: mol_type = other DNA
agcacgagctgacgacaaccatgcagcacctgtatatagaccccaaacggggaataattatctctaactatatcctatatatgtcaagccctggtaaggttcctcgcgtatcatcgaatt

SEQ ID NO: 593 - DNA, 120 bp, synthetic construct
  source 1..120: mol_type = other DNA
tctctaactatatcctatatatgtcaagccctggtaaggttcctcgcgtatcatcgaattaaaccacatgctccaccgcttgtgcgggcccccgtcaattcctttgagtttcactcttgc

SEQ ID NO: 594 - DNA, 120 bp, synthetic construct
  source 1..120: mol_type = other DNA
aaaccacatgctccaccgcttgtgcgggcccccgtcaattcctttgagtttcactcttgcgagcatactccccaggcggcacacttaacacgttagcttcggtactaacttttagttaac

SEQ ID NO: 595 - DNA, 120 bp, synthetic construct
  source 1..120: mol_type = other DNA
gagcatactccccaggcggcacacttaacacgttagcttcggtactaacttttagttaacaccaagtgtgcatcgtttacagcgtagactaccagggtatctaatcctgtttgctcccta

SEQ ID NO: 596 - DNA, 120 bp, synthetic construct
  source 1..120: mol_type = other DNA
accaagtgtgcatcgtttacagcgtagactaccagggtatctaatcctgtttgctccctacgctttcgtgactcagcgtcagtcttgacccagaagttcgccttcgcctccggtattctt

SEQ ID NO: 597 - DNA, 120 bp, synthetic construct
  source 1..120: mol_type = other DNA
cgctttcgtgactcagcgtcagtcttgacccagaagttcgccttcgcctccggtattctttctgatatcaacagattccacccttacaccagaaattctaacttcctctatcagactcta

SEQ ID NO: 598 - DNA, 120 bp, synthetic construct
  source 1..120: mol_type = other DNA
tctgatatcaacagattccacccttacaccagaaattctaacttcctctatcagactctagacatatagtttccaacataggtccacagttgagctgtggtattttatgcatagacttat

SEQ ID NO: 599 - DNA, 120 bp, synthetic construct
  source 1..120: mol_type = other DNA
gacatatagtttccaacataggtccacagttgagctgtggtattttatgcatagacttatatatccgcctactcaccctttacgcccaataatcccgaacaacgctcgccccttacgtat

SEQ ID NO: 600 - DNA, 120 bp, synthetic construct
  source 1..120: mol_type = other DNA
atatccgcctactcaccctttacgcccaataatcccgaacaacgctcgccccttacgtattaccgcggctgctggcacgtaattagccggggcttattcataaattaacgtcatcacttt

SEQ ID NO: 601 - DNA, 120 bp, synthetic construct
  source 1..120: mol_type = other DNA
taccgcggctgctggcacgtaattagccggggcttattcataaattaacgtcatcactttgtcatttcctacaaagcttattcctcatttataaaagaattttacaatctttcgaccttc

SEQ ID NO: 602 - DNA, 120 bp, synthetic construct
  source 1..120: mol_type = other DNA
gtcatttcctacaaagcttattcctcatttataaaagaattttacaatctttcgaccttcttcattcacgcagtgtcgctccgtcaggctttcgcccattgcggaagattcttagctgct

SEQ ID NO: 603 - DNA, 120 bp, synthetic construct
  source 1..120: mol_type = other DNA
ttcattcacgcagtgtcgctccgtcaggctttcgcccattgcggaagattcttagctgctgcctcccgtaggagtctggaccgtatctcagttccagtgtgaccgttcaccctctcaggc

SEQ ID NO: 604 - DNA, 120 bp, synthetic construct
  source 1..120: mol_type = other DNA
gcctcccgtaggagtctggaccgtatctcagttccagtgtgaccgttcaccctctcaggccggttacttatcattgccttggtaggcatttaccctaccaactagctaataagacgcaga

SEQ ID NO: 605 - DNA, 120 bp, synthetic construct
  source 1..120: mol_type = other DNA
cggttacttatcattgccttggtaggcatttaccctaccaactagctaataagacgcagactcatctacaagcgaagctttaaaggcttcctttcatcaattaacaaattaattgacctt

SEQ ID NO: 606 - DNA, 120 bp, synthetic construct
  source 1..120: mol_type = other DNA
ctcatctacaagcgaagctttaaaggcttcctttcatcaattaacaaattaattgaccttattcggtattagctactatttctaatagttatccccatctcataggtagatcatccacgc

SEQ ID NO: 607 - DNA, 120 bp, synthetic construct
  source 1..120: mol_type = other DNA
attcggtattagctactatttctaatagttatccccatctcataggtagatcatccacgcgttactcacccgttcgccactgaatgtattgctacatcccgtttgacttgcatgcttaag

SEQ ID NO: 608 - DNA, 120 bp, synthetic construct
  source 1..120: mol_type = other DNA
gttactcacccgttcgccactgaatgtattgctacatcccgtttgacttgcatgcttaagacgcactgccagcgttagttctaagccaggatcaaactcttcgttattttatttttttat

SEQ ID NO: 609 - DNA, 120 bp, synthetic construct
  source 1..120: mol_type = other DNA
acgcactgccagcgttagttctaagccaggatcaaactcttcgttattttatttttttatttaaaaaaattaacaggttttgtttattcttttggcttttaaccttacttaactcttccc

SEQ ID NO: 610 - DNA, 120 bp, synthetic construct
  source 1..120: mol_type = other DNA
ttaaaaaaattaacaggttttgtttattcttttggcttttaaccttacttaactcttcccttctctcatcttccaataatcatttcaacctttaatactttaacaaaagaagaatcatat

SEQ ID NO: 611 - DNA, 120 bp, synthetic construct
  source 1..120: mol_type = other DNA
ttctctcatcttccaataatcatttcaacctttaatactttaacaaaagaagaatcatattgtcaatacctttgcattatttttattaatataaaatgtaaaaaaataaattttattaat

SEQ ID NO: 612 - DNA, 120 bp, synthetic construct
  source 1..120: mol_type = other DNA
tgtcaatacctttgcattatttttattaatataaaatgtaaaaaaataaattttattaataaacagtgataaaagcattaacagccacacttttcattaacaggcaaagttgtaaaaatt

SEQ ID NO: 613 - DNA, 120 bp, synthetic construct
  source 1..120: mol_type = other DNA
aaacagtgataaaagcattaacagccacacttttcattaacaggcaaagttgtaaaaattttttttaatttatttcccaatttagcttttaaataatcaaaaaaggttctgaaattttca

SEQ ID NO: 614 - DNA, 120 bp, synthetic construct
  source 1..120: mol_type = other DNA
ttttttaatttatttcccaatttagcttttaaataatcaaaaaaggttctgaaattttcattatctcctttaaacttaatccacagttctttaaaggttaaaattccttccctaagatcc

SEQ ID NO: 615 - DNA, 120 bp, synthetic construct
  source 1..120: mol_type = other DNA
ttatctcctttaaacttaatccacagttctttaaaggttaaaattccttccctaagatccttgtaattggaaaaagcagcagcacagtcgctatacattaaattataaaaatcagaatct

SEQ ID NO: 616 - DNA, 120 bp, synthetic construct
  source 1..120: mol_type = other DNA
ttgtaattggaaaaagcagcagcacagtcgctatacattaaattataaaaatcagaatcttgtttatctttaaaaaaatctatacttggtattttcttggcaaaggcgaatcctctctca

SEQ ID NO: 617 - DNA, 120 bp, synthetic construct
  source 1..120: mol_type = other DNA
tgtttatctttaaaaaaatctatacttggtattttcttggcaaaggcgaatcctctctcataagccgtgccagaatcaacataattaaccaaggctaaaacaatatcgctactaactagc

SEQ ID NO: 618 - DNA, 120 bp, synthetic construct
  source 1..120: mol_type = other DNA
taagccgtgccagaatcaacataattaaccaaggctaaaacaatatcgctactaactagctcttttaaatctatttctcttatcttctcccttatatctctatttacaaacttataatca

SEQ ID NO: 619 - DNA, 120 bp, synthetic construct
  source 1..120: mol_type = other DNA
tcttttaaatctatttctcttatcttctcccttatatctctatttacaaacttataatcaaccttttcaagcaatcccatctttttgacagcatgatgctctggagaaaatacttctaaa

SEQ ID NO: 620 - DNA, 120 bp, synthetic construct
  source 1..120: mol_type = other DNA
accttttcaagcaatcccatctttttgacagcatgatgctctggagaaaatacttctaaattaaactcttcaagaaatttcaaaacctcatcccttagtttaatttcctcttccttaaaa

SEQ ID NO: 621 - DNA, 120 bp, synthetic construct
  source 1..120: mol_type = other DNA
ttaaactcttcaagaaatttcaaaacctcatcccttagtttaatttcctcttccttaaaaaatggagaggctaaataaatcttcataaaaacccctatcaaaattcaagtataacacaat

SEQ ID NO: 622 - DNA, 120 bp, synthetic construct
  source 1..120: mol_type = other DNA
aatggagaggctaaataaatcttcataaaaacccctatcaaaattcaagtataacacaataaatcaatcgagtaaaatcaagaataaataaatttttaaaatccaagtagaaaacattta

SEQ ID NO: 623 - DNA, 120 bp, synthetic construct
  source 1..120: mol_type = other DNA
aaatcaatcgagtaaaatcaagaataaataaatttttaaaatccaagtagaaaacatttattatgaacgacttctgctgactagaatagtaaactctcctttaaccttatccttactcga

SEQ ID NO: 624 - DNA, 120 bp, synthetic construct
  source 1..120: mol_type = other DNA
ttatgaacgacttctgctgactagaatagtaaactctcctttaaccttatccttactcgattcaaaatatttttttaattctaaaggtttgccaatttgatattcttcataaatttttgt

SEQ ID NO: 625 - DNA, 120 bp, synthetic construct
  source 1..120: mol_type = other DNA
ttcaaaatatttttttaattctaaaggtttgccaatttgatattcttcataaatttttgtcatctcgcgaccaataagaaccttcgcatctaaactaacagaagaaatttcaacaagcaa

SEQ ID NO: 626 - DNA, 120 bp, synthetic construct
  source 1..120: mol_type = other DNA
catctcgcgaccaataagaaccttcgcatctaaactaacagaagaaatttcaacaagcaatttcaaaattctatgaccagattcaagcagaacaaaagcatctccccttttatatagctc

SEQ ID NO: 627 - DNA, 120 bp, synthetic construct
  source 1..120: mol_type = other DNA
tttcaaaattctatgaccagattcaagcagaacaaaagcatctccccttttatatagctcagcaattcttttaaatcttttaaggcctttgttaggcaaaaatccctcaaaaaacactga

SEQ ID NO: 628 - DNA, 120 bp, synthetic construct
  source 1..120: mol_type = other DNA
agcaattcttttaaatcttttaaggcctttgttaggcaaaaatccctcaaaaaacactgatttatctctaaaaggattaacacttacaattgtattaaaagaacttactccaggaattgg

SEQ ID NO: 629 - DNA, 120 bp, synthetic construct
  source 1..120: mol_type = other DNA
tttatctctaaaaggattaacacttacaattgtattaaaagaacttactccaggaattggacaaactttgtatccctctctaaaagcagcagcaactaataagctgcccggatcactaag

SEQ ID NO: 630 - DNA, 120 bp, synthetic construct
  source 1..120: mol_type = other DNA
acaaactttgtatccctctctaaaagcagcagcaactaataagctgcccggatcactaagccctggagtaccagcatcgctaacaaaagcaacagaatttccttttgccaaataatccaa

SEQ ID NO: 631 - DNA, 120 bp, synthetic construct
  source 1..120: mol_type = other DNA
ccctggagtaccagcatcgctaacaaaagcaacagaatttccttttgccaaataatccaatagcaagcttatcttcttgttttctgttacggcattacaagaaatcatttttttattaat

SEQ ID NO: 632 - DNA, 120 bp, synthetic construct
  source 1..120: mol_type = other DNA
tagcaagcttatcttcttgttttctgttacggcattacaagaaatcatttttttattaattttatatcgagacaaaagtttgctagttactctcgtatcttccgcaaagataacatttac

SEQ ID NO: 633 - DNA, 120 bp, synthetic construct
  source 1..120: mol_type = other DNA
tttatatcgagacaaaagtttgctagttactctcgtatcttccgcaaagataacatttaccgattttaaaacatcaattgctctataagtaatatcttctaaattgcctattggcgtacc

SEQ ID NO: 634 - DNA, 120 bp, synthetic construct
  source 1..120: mol_type = other DNA
tccgcaaagataacatttaccgattttaaaacatcaattgctctataagtaatatcttctaaattgcctattggcgtaccaacaatatataacacggccccttttaattcctccaaaact

SEQ ID NO: 635 - DNA, 120 bp, synthetic construct
  source 1..120: mol_type = other DNA
aatcttaaatccaaatgaaaatataggttttgcctcataccaagttgaagatttcattaaagaaataattgatcctattcttgaaaataaataaggaatactaatatttagaaacaaatc

SEQ ID NO: 636 - DNA, 120 bp, synthetic construct
  source 1..120: mol_type = other DNA
agaaataattgatcctattcttgaaaataaataaggaatactaatatttagaaacaaatctattatcccttatgtaaaatcgccaaagcttattcgcatactcctcacctgcataatcaa

SEQ ID NO: 637 - DNA, 120 bp, synthetic construct
  source 1..120: mol_type = other DNA
tattatcccttatgtaaaatcgccaaagcttattcgcatactcctcacctgcataatcaacatttattctctttgagcatgccacttcaaaatcaaaagataaatcttttcttaagaaaa

SEQ ID NO: 638 - DNA, 120 bp, synthetic construct
  source 1..120: mol_type = other DNA
catttattctctttgagcatgccacttcaaaatcaaaagataaatcttttcttaagaaaagttcacaattattaagaagatctctattattaaactttaaatctatatttaaaaacttag

SEQ ID NO: 639 - DNA, 120 bp, synthetic construct
  source 1..120: mol_type = other DNA
gttcacaattattaagaagatctctattattaaactttaaatctatatttaaaaacttagtaagcttaccaggcccattagttaacaatccatcaacttttggagaaataggctcaatag

SEQ ID NO: 640 - DNA, 120 bp, synthetic construct
  source 1..120: mol_type = other DNA
taagcttaccaggcccattagttaacaatccatcaacttttggagaaataggctcaatagctcttattaaaacagcatggggattatgttcattagatgccacaacgtttaacatgtaat

SEQ ID NO: 641 - DNA, 120 bp, synthetic construct
  source 1..120: mol_type = other DNA
ctcttattaaaacagcatggggattatgttcattagatgccacaacgtttaacatgtaatacataccataaatcatataaacataaacatatcccccaatattatacatggcaatggtac

SEQ ID NO: 642 - DNA, 120 bp, synthetic construct
  source 1..120: mol_type = other DNA
acataccataaatcatataaacataaacatatcccccaatattatacatggcaatggtacgatttgttcttcttcccccataagcatggcaggctttatctactacacccatataagctt

SEQ ID NO: 643 - DNA, 120 bp, synthetic construct
  source 1..120: mol_type = other DNA
gatttgttcttcttcccccataagcatggcaggctttatctactacacccatataagcttccgtctcgacaattcttgaaataatttctttgccatctatttttctaatcagcaagtgcc

SEQ ID NO: 644 - DNA, 120 bp, synthetic construct
  source 1..120: mol_type = other DNA
ccgtctcgacaattcttgaaataatttctttgccatctatttttctaatcagcaagtgcccaagcaaagactcagccacaacaatagcatcctgcataaaaaactctctattcattagta

SEQ ID NO: 645 - DNA, 120 bp, synthetic construct
  source 1..120: mol_type = other DNA
caagcaaagactcagccacaacaatagcatcctgcataaaaaactctctattcattagtacaattctaaactaaaacaaaaatcaaattcaaaacttattgtttcaaaacttattgcaat

SEQ ID NO: 646 - DNA, 120 bp, synthetic construct
  source 1..120: mol_type = other DNA
caattctaaactaaaacaaaaatcaaattcaaaacttattgtttcaaaacttattgcaattggcacaagtgttaaataacaattaaaaataacagacaattatcatggaaaaataaagcg

SEQ ID NO: 647 - DNA, 120 bp, synthetic construct
  source 1..120: mol_type = other DNA
tggcacaagtgttaaataacaattaaaaataacagacaattatcatggaaaaataaagcgtatattgacaaacgcaataaagttaaatagaatcttaaagggtaagaatattttagggat

SEQ ID NO: 648 - DNA, 120 bp, synthetic construct
  source 1..120: mol_type = other DNA
tatattgacaaacgcaataaagttaaatagaatcttaaagggtaagaatattttagggatcatagctcaggtggttagagcgcaggtctgataaacctgaggtcggaggttcaactcctc

SEQ ID NO: 649 - DNA, 120 bp, synthetic construct
  source 1..120: mol_type = other DNA
catagctcaggtggttagagcgcaggtctgataaacctgaggtcggaggttcaactcctcctggtcccaattttacactcaaatccttttaaagatctaatgagctaggtaaaatagttc

SEQ ID NO: 650 - DNA, 120 bp, synthetic construct
  source 1..120: mol_type = other DNA
ctggtcccaattttacactcaaatccttttaaagatctaatgagctaggtaaaatagttcaaaacgtatttttgaaagtttgttcttaagttttagtcaagcttcacatctgcaataaaa

SEQ ID NO: 651 - DNA, 120 bp, synthetic construct
  source 1..120: mol_type = other DNA
aaaacgtatttttgaaagtttgttcttaagttttagtcaagcttcacatctgcaataaaaatttatcactaaaccacaaagaatgggtaatataataattaaaaccacaagcttaaatat

SEQ ID NO: 652 - DNA, 120 bp, synthetic construct
  source 1..120: mol_type = other DNA
atttatcactaaaccacaaagaatgggtaatataataattaaaaccacaagcttaaatattaaaccatgtattatattcatatattatattgattcactcaagataaacacaaacatcaa

SEQ ID NO: 653 - DNA, 120 bp, synthetic construct
  source 1..120: mol_type = other DNA
taaaccatgtattatattcatatattatattgattcactcaagataaacacaaacatcaaccatattaaactttacatgaagtaatattatttcctacaaactacaaaaacttaaattaa

SEQ ID NO: 654 - DNA, 120 bp, synthetic construct
  source 1..120: mol_type = other DNA
ccatattaaactttacatgaagtaatattatttcctacaaactacaaaaacttaaattaatctaaataagataacttaaaaataacatgaataacatatcgttattttttattatctatc

SEQ ID NO: 655 - DNA, 120 bp, synthetic construct
  source 1..120: mol_type = other DNA
tctaaataagataacttaaaaataacatgaataacatatcgttattttttattatctatcctatagatgcaatctattgacctaataaattcttaaacttaagcaaaaattttaaaaaag

SEQ ID NO: 656 - DNA, 120 bp, synthetic construct
  source 1..120: mol_type = other DNA
ctatagatgcaatctattgacctaataaattcttaaacttaagcaaaaattttaaaaaagaaatgttttatttggacatctaaattttaattagattatttttaatcattaaagacaatt

SEQ ID NO: 657 - DNA, 120 bp, synthetic construct
  source 1..120: mol_type = other DNA
aaatgttttatttggacatctaaattttaattagattatttttaatcattaaagacaattttaattgataaatcacaggctgatatttaaaagatacaacctccattcatttttgcaata

SEQ ID NO: 658 - DNA, 120 bp, synthetic construct
  source 1..120: mol_type = other DNA
ttaattgataaatcacaggctgatatttaaaagatacaacctccattcatttttgcaataaacaaatggaggttaagggactcgaacccttgacccccggcttgcaaagccgatgctcta

SEQ ID NO: 659 - DNA, 120 bp, synthetic construct
  source 1..120: mol_type = other DNA
aacaaatggaggttaagggactcgaacccttgacccccggcttgcaaagccgatgctctaaaccaactgagctaaacccccaaaaaaatctttgaaaagacaaaggaagagttaaaataa

SEQ ID NO: 660 - DNA, 120 bp, synthetic construct
  source 1..120: mol_type = other DNA
aaccaactgagctaaacccccaaaaaaatctttgaaaagacaaaggaagagttaaaataatgctttaccttaaataattaaatcatttctttctcttagaaaggaggtgatccagccaca

SEQ ID NO: 661 - DNA, 120 bp, synthetic construct
  source 1..120: mol_type = other DNA
tgctttaccttaaataattaaatcatttctttctcttagaaaggaggtgatccagccacactttccagtacggctaccttgttacgacttcacccccctcactaaacataccttagatac

SEQ ID NO: 662 - DNA, 120 bp, synthetic construct
  source 1..120: mol_type = other DNA
ctttccagtacggctaccttgttacgacttcacccccctcactaaacataccttagataccttcctcccttgcgggttagaataatagcttcgggtatcctcaactcgggtggtgtgacg

SEQ ID NO: 663 - DNA, 120 bp, synthetic construct
  source 1..120: mol_type = other DNA
cttcctcccttgcgggttagaataatagcttcgggtatcctcaactcgggtggtgtgacgggcggtgtgtacaaggcccgagaacgtattcaccgtatcattctgatatacgattactag

SEQ ID NO: 664 - DNA, 120 bp, synthetic construct
  source 1..120: mol_type = other DNA
ggcggtgtgtacaaggcccgagaacgtattcaccgtatcattctgatatacgattactagcgattccaacttcatgaagtcgagtttcagacttcaatctggactgagacctgctttatg

SEQ ID NO: 665 - DNA, 120 bp, synthetic construct
  source 1..120: mol_type = other DNA
cgattccaacttcatgaagtcgagtttcagacttcaatctggactgagacctgctttatgcgttttgcttcacatcactgtttcgcgtcgctttgtacaggccattgtagcacgtgtgta

SEQ ID NO: 666 - DNA, 120 bp, synthetic construct
  source 1..120: mol_type = other DNA
cgttttgcttcacatcactgtttcgcgtcgctttgtacaggccattgtagcacgtgtgtagcccaggacataagggccatgatgatttgacgtcatcctcaccttcctccggcttatcac

SEQ ID NO: 667 - DNA, 120 bp, synthetic construct
  source 1..120: mol_type = other DNA
gcccaggacataagggccatgatgatttgacgtcatcctcaccttcctccggcttatcaccggcagtctcgtctgagtccccatctttacatgctggtaacagacaataagggttgcgct

SEQ ID NO: 668 - DNA, 120 bp, synthetic construct
  source 1..120: mol_type = other DNA
cggcagtctcgtctgagtccccatctttacatgctggtaacagacaataagggttgcgctcgttgcgggacttaacccaacacctcacagcacgagctgacgacaaccatgcagcacctg

SEQ ID NO: 669 - DNA, 120 bp, synthetic construct
  source 1..120: mol_type = other DNA
cgttgcgggacttaacccaacacctcacagcacgagctgacgacaaccatgcagcacctgtatacagaccccaaacggggaatagttatctctaactacatcctgtatatgtcaagccct

SEQ ID NO: 670 - DNA, 120 bp, synthetic construct
  source 1..120: mol_type = other DNA
tatacagaccccaaacggggaatagttatctctaactacatcctgtatatgtcaagccctggtaaggttcctcgcgtatcatcgaattaaaccacatgctccaccgcttgtgcgggcccc

SEQ ID NO: 671 - DNA, 120 bp, synthetic construct
  source 1..120: mol_type = other DNA
ggtaaggttcctcgcgtatcatcgaattaaaccacatgctccaccgcttgtgcgggcccccgtcaattcctttgagtttcactcttgcgagcatactccccaggcggcacacttaacacg

SEQ ID NO: 672 - DNA, 120 bp, synthetic construct
  source 1..120: mol_type = other DNA
cgtcaattcctttgagtttcactcttgcgagcatactccccaggcggcacacttaacacgttagcttcggtactaacctttcgattaacaccaagtgtgcatcgtttacagcgtagacta

SEQ ID NO: 673 - DNA, 120 bp, synthetic construct
  source 1..120: mol_type = other DNA
ttagcttcggtactaacctttcgattaacaccaagtgtgcatcgtttacagcgtagactaccagggtatctaatcctgtttgctccctacgctttcgtgactcagcgtcagtcttgaccc

SEQ ID NO: 674 - DNA, 120 bp, synthetic construct
  source 1..120: mol_type = other DNA
ccagggtatctaatcctgtttgctccctacgctttcgtgactcagcgtcagtcttgacccagaagttcgccttcgcctctggtattcttcctgatatcaacagattccacccttacacca

SEQ ID NO: 675 - DNA, 120 bp, synthetic construct
  source 1..120: mol_type = other DNA
agaagttcgccttcgcctctggtattcttcctgatatcaacagattccacccttacaccaggaattctaacttcccctatcagactctagtcatgcagtttccagcatattcccacagtt

SEQ ID NO: 676 - DNA, 120 bp, synthetic construct
  source 1..120: mol_type = other DNA
ggaattctaacttcccctatcagactctagtcatgcagtttccagcatattcccacagttgagctgtggtattttacgcatagacttgcatatccgcctactcaccctttacgcccaata

SEQ ID NO: 677 - DNA, 120 bp, synthetic construct
  source 1..120: mol_type = other DNA
gagctgtggtattttacgcatagacttgcatatccgcctactcaccctttacgcccaataatcccgaacaacgctcgccccttacgtattaccgcggctgctggcacgtaattagccggg

SEQ ID NO: 678 - DNA, 120 bp, synthetic construct
  source 1..120: mol_type = other DNA
atcccgaacaacgctcgccccttacgtattaccgcggctgctggcacgtaattagccggggcttattcataaattaacgtcatcactttgtcatttcctacaaagcttattcctcattta

SEQ ID NO: 679 - DNA, 120 bp, synthetic construct
  source 1..120: mol_type = other DNA
gcttattcataaattaacgtcatcactttgtcatttcctacaaagcttattcctcatttataaaagaactttacaatctttcgaccttcttcgttcacgcagtgtcgctccgtcaggctt

SEQ ID NO: 680 - DNA, 120 bp, synthetic construct
  source 1..120: mol_type = other DNA
taaaagaactttacaatctttcgaccttcttcgttcacgcagtgtcgctccgtcaggctttcgcccattgcggaagattcttagctgctgcctcccgtaggagtctggaccgtatctcag

SEQ ID NO: 681 - DNA, 120 bp, synthetic construct
  source 1..120: mol_type = other DNA
tcgcccattgcggaagattcttagctgctgcctcccgtaggagtctggaccgtatctcagttccagtgtgaccgttcaccctctcaggccggttacttatcacagccttggtaggccttt

SEQ ID NO: 682 - DNA, 120 bp, synthetic construct
  source 1..120: mol_type = other DNA
ttccagtgtgaccgttcaccctctcaggccggttacttatcacagccttggtaggcctttaccccaccaactagctaataagacgcagactcatctacaagcgaagctttaaaggcttcc

SEQ ID NO: 683 - DNA, 120 bp, synthetic construct
  source 1..120: mol_type = other DNA
accccaccaactagctaataagacgcagactcatctacaagcgaagctttaaaggcttcctttcatcaattaacatcttaattgaccttattcggtattagctactatttctaatagtta

SEQ ID NO: 684 - DNA, 120 bp, synthetic construct
  source 1..120: mol_type = other DNA
tttcatcaattaacatcttaattgaccttattcggtattagctactatttctaatagttatccccatctcataggtagattatccacgcgttactcacccgttcgccactgaatgtattg

SEQ ID NO: 685 - DNA, 120 bp, synthetic construct
  source 1..120: mol_type = other DNA
tccccatctcataggtagattatccacgcgttactcacccgttcgccactgaatgtattgctacattccgtctgacttgcatgcttaagacgcactgccagcgttagttctaagccagga

SEQ ID NO: 686 - DNA, 120 bp, synthetic construct
  source 1..120: mol_type = other DNA
ctacattccgtctgacttgcatgcttaagacgcactgccagcgttagttctaagccaggatcaaactcttcgttatttttattttcttcttttaaaattaacaggttattcattttattt

SEQ ID NO: 687 - DNA, 120 bp, synthetic construct
  source 1..120: mol_type = other DNA
tcaaactcttcgttatttttattttcttcttttaaaattaacaggttattcattttatttggcttattaaaccttacttaactcttcccttctcttctcttccaattctcaatatcaact

SEQ ID NO: 688 - DNA, 120 bp, synthetic construct
  source 1..120: mol_type = other DNA
ggcttattaaaccttacttaactcttcccttctcttctcttccaattctcaatatcaactcttactactttataacatacgttaagctttgtcaatacttaaacatttatttttttatat

SEQ ID NO: 689 - DNA, 120 bp, synthetic construct
  source 1..120: mol_type = other DNA
cttactactttataacatacgttaagctttgtcaatacttaaacatttatttttttatattactattttttaacagattgttttcatgatcttttattctgctatcttgcactaatcgcc

SEQ ID NO: 690 - DNA, 120 bp, synthetic construct
  source 1..120: mol_type = other DNA
tactattttttaacagattgttttcatgatcttttattctgctatcttgcactaatcgcctaacaacacctaaaacactgcctataccctcatatccattataatgattgcctcttaaat

SEQ ID NO: 691 - DNA, 120 bp, synthetic construct
  source 1..120: mol_type = other DNA
taacaacacctaaaacactgcctataccctcatatccattataatgattgcctcttaaattagcaccaaagacacttttaaatccagctttcaaagctgcaataaccttactctcaatat

SEQ ID NO: 692 - DNA, 120 bp, synthetic construct
  source 1..120: mol_type = other DNA
tagcaccaaagacacttttaaatccagctttcaaagctgcaataaccttactctcaatattagaggatactttaatttctcctgagagagaaatctcacctgtaaagattaactcttgac

SEQ ID NO: 693 - DNA, 120 bp, synthetic construct
  source 1..120: mol_type = other DNA
tagaggatactttaatttctcctgagagagaaatctcacctgtaaagattaactcttgactgataataacattagtcttagcagaaaataatgcaactaaaacggcaagttcaatctcta

SEQ ID NO: 694 - DNA, 120 bp, synthetic construct
  source 1..120: mol_type = other DNA
tgataataacattagtcttagcagaaaataatgcaactaaaacggcaagttcaatctctacatcatcaatcctaagccccccagaaacattaacatagatatcatcattattaaaattaa

SEQ ID NO: 695 - DNA, 120 bp, synthetic construct
  source 1..120: mol_type = other DNA
catcatcaatcctaagccccccagaaacattaacatagatatcatcattattaaaattaagatttaaatacttactaataacagctaaaattcttgatatttttttagaatctattttct

SEQ ID NO: 696 - DNA, 120 bp, synthetic construct
  source 1..120: mol_type = other DNA
gatttaaatacttactaataacagctaaaattcttgatatttttttagaatctattttctctgaaaaaattctagaaatattcatgcctgtccttgtaattaaagcctgtatctcaacaa

SEQ ID NO: 697 - DNA, 120 bp, synthetic construct
  source 1..120: mol_type = other DNA
ctgaaaaaattctagaaatattcatgcctgtccttgtaattaaagcctgtatctcaacaaataagactctactcccctcattaataattccaatagcaatacctgaggatatctcttctt

SEQ ID NO: 698 - DNA, 120 bp, synthetic construct
  source 1..120: mol_type = other DNA
ataagactctactcccctcattaataattccaatagcaatacctgaggatatctcttctttcctctccaaaaagatagaagatggatctttaatctcaacaagtcccaaactcgtcattt

SEQ ID NO: 699 - DNA, 120 bp, synthetic construct
  source 1..120: mol_type = other DNA
tcctctccaaaaagatagaagatggatctttaatctcaacaagtcccaaactcgtcatttcaaaaatacctatctcattaacagtaccaaacctattcttagtagctctaagcatacgca

SEQ ID NO: 700 - DNA, 120 bp, synthetic construct
  source 1..120: mol_type = other DNA
caaaaatacctatctcattaacagtaccaaacctattcttagtagctctaagcatacgcaaagatttttttgcctcttcaaaataaaaaacagaatctaccatatgctctattatttttg

SEQ ID NO: 701 - DNA, 120 bp, synthetic construct
  source 1..120: mol_type = other DNA
aagatttttttgcctcttcaaaataaaaaacagaatctaccatatgctctattatttttggtcccgctaaaataccatcctttgtaacatgtcccactaaacataaagttatattctttc

SEQ ID NO: 702 - DNA, 120 bp, synthetic construct
  source 1..120: mol_type = other DNA
gtcccgctaaaataccatcctttgtaacatgtcccactaaacataaagttatattctttccctttgcccactctacaagcttgtaaacacaatgttttaactgagcaaccccgccaagac

SEQ ID NO: 703 - DNA, 120 bp, synthetic construct
  source 1..120: mol_type = other DNA
cctttgcccactctacaagcttgtaaacacaatgttttaactgagcaaccccgccaagactaccttgcacttctcttgaattcaaagtttgaatagaatcaacaactataaagtcaagct

SEQ ID NO: 704 - DNA, 120 bp, synthetic construct
  source 1..120: mol_type = other DNA
taccttgcacttctcttgaattcaaagtttgaatagaatcaacaactataaagtcaagctcaatatttgcaagcatttctattaaagcatcaacatctacctcattagttatcaatatat

SEQ ID NO: 705 - DNA, 120 bp, synthetic construct
  source 1..120: mol_type = other DNA
caatatttgcaagcatttctattaaagcatcaacatctacctcattagttatcaatatatcagaagaaattttaagcctatttgctctcaacttaatttgtggaattgattcctcacccg

SEQ ID NO: 706 - DNA, 120 bp, synthetic construct
  source 1..120: mol_type = other DNA
cagaagaaattttaagcctatttgctctcaacttaatttgtggaattgattcctcacccgcaagataaagcacattcttgccatcaagtgagagaatactagaaatctgaagtaaaaaag

SEQ ID NO: 707 - DNA, 120 bp, synthetic construct
  source 1..120: mol_type = other DNA
caagataaagcacattcttgccatcaagtgagagaatactagaaatctgaagtaaaaaagttgattttccaatgccaggctctcctgatatcaaaattgcactaccaattacaatcccag

SEQ ID NO: 708 - DNA, 120 bp, synthetic construct
  source 1..120: mol_type = other DNA
ttgattttccaatgccaggctctcctgatatcaaaattgcactaccaattacaatcccagcaccaagaactctatcaaactcttcaatgcctgttaaatacctaacattatcaacttgct

SEQ ID NO: 709 - DNA, 120 bp, synthetic construct
  source 1..120: mol_type = other DNA
caccaagaactctatcaaactcttcaatgcctgttaaatacctaacattatcaacttgcttaaaatcttttaaagaaaaaatctcactttttgacttacttaagtttgtcccataaccag

SEQ ID NO: 710 - DNA, 120 bp, synthetic construct
  source 1..120: mol_type = other DNA
taaaatcttttaaagaaaaaatctcactttttgacttacttaagtttgtcccataaccagatttaggttcaacataatgctctaaactttcccaactaaaacactcaggacacttcccta

SEQ ID NO: 711 - DNA, 120 bp, synthetic construct
  source 1..120: mol_type = other DNA
atttaggttcaacataatgctctaaactttcccaactaaaacactcaggacacttccctagccattttaaagatttatatccacaatttaaacatttataaatttccttatctttctttt

SEQ ID NO: 712 - DNA, 120 bp, synthetic construct
  source 1..120: mol_type = other DNA
cctagccattttaaagatttatatccacaatttaaacatttataaatttccttatctttcttttttgccataaaacctcaataggtaaactttttttcatttggacaagtgataaaacta

SEQ ID NO: 713 - DNA, 120 bp, synthetic construct
  source 1..120: mol_type = other DNA
tgagacacacgtagcctaccagtttcttactgctctactctgcaaagcaagagattaagaacccatcatggatcctgtgtacgtggacatagacgctgacagcgcctttttgaaggccct

SEQ ID NO: 714 - DNA, 120 bp, synthetic construct
  source 1..120: mol_type = other DNA
acccatcatggatcctgtgtacgtggacatagacgctgacagcgcctttttgaaggccctgcaacgtgcgtaccccatgtttgaggtggaacctaggcaggtcacaccgaatgaccatgc

SEQ ID NO: 715 - DNA, 120 bp, synthetic construct
  source 1..120: mol_type = other DNA
gcaacgtgcgtaccccatgtttgaggtggaacctaggcaggtcacaccgaatgaccatgctaatgctagagcgttctcgcatctagctataaaactaatagagcaggaaattgatcccga

SEQ ID NO: 716 - DNA, 120 bp, synthetic construct
  source 1..120: mol_type = other DNA
taatgctagagcgttctcgcatctagctataaaactaatagagcaggaaattgatcccgactcaaccatcctggatattggtagtgcgccagcaaggaggatgatgtcggacaggaagta

SEQ ID NO: 717 - DNA, 120 bp, synthetic construct
  source 1..120: mol_type = other DNA
ctcaaccatcctggatattggtagtgcgccagcaaggaggatgatgtcggacaggaagtaccactgcgtttgcccgatgcgcagtgcagaagatcccgagagactcgccaattatgcgag

SEQ ID NO: 718 - DNA, 120 bp, synthetic construct
  source 1..120: mol_type = other DNA
ccactgcgtttgcccgatgcgcagtgcagaagatcccgagagactcgccaattatgcgagaaagctagcatctgccgcaggaaaagtcctggacagaaacatctctggaaagatcgggga

SEQ ID NO: 719 - DNA, 120 bp, synthetic construct
  source 1..120: mol_type = other DNA
aaagctagcatctgccgcaggaaaagtcctggacagaaacatctctggaaagatcggggacttacaagcagtaatggccgtgccagacacggagacgccaacattctgcttacacacaga

SEQ ID NO: 720 - DNA, 120 bp, synthetic construct
  source 1..120: mol_type = other DNA
cttacaagcagtaatggccgtgccagacacggagacgccaacattctgcttacacacagatgtatcatgtagacagagagcagacgtcgcgatataccaagacgtctatgctgtacacgc

SEQ ID NO: 721 - DNA, 120 bp, synthetic construct
  source 1..120: mol_type = other DNA
tgtatcatgtagacagagagcagacgtcgcgatataccaagacgtctatgctgtacacgcacccacgtcgctataccaccaggcgattaaaggggtccgattggcgtactgggtagggtt

SEQ ID NO: 722 - DNA, 120 bp, synthetic construct
  source 1..120: mol_type = other DNA
acccacgtcgctataccaccaggcgattaaaggggtccgattggcgtactgggtagggtttgacacaaccccgttcatgtacaatgccatggcgggtgcctacccctcatactcgacaaa

SEQ ID NO: 723 - DNA, 120 bp, synthetic construct
  source 1..120: mol_type = other DNA
tgacacaaccccgttcatgtacaatgccatggcgggtgcctacccctcatactcgacaaattgggcagatgagcaggtactgaaggctaagaacataggattatgttcaacagacctgac

SEQ ID NO: 724 - DNA, 120 bp, synthetic construct
  source 1..120: mol_type = other DNA
ttgggcagatgagcaggtactgaaggctaagaacataggattatgttcaacagacctgacggaaggtagacgaggcaaattgtctattatgagaggaaaaaagctagaaccgtgcgaccg

SEQ ID NO: 725 - DNA, 120 bp, synthetic construct
  source 1..120: mol_type = other DNA
ggaaggtagacgaggcaaattgtctattatgagaggaaaaaagctagaaccgtgcgaccgtgtgctgttctcagtagggtcaacgctctacccggaaagccgtaagctacttaagagctg

SEQ ID NO: 726 - DNA, 120 bp, synthetic construct
  source 1..120: mol_type = other DNA
tgtgctgttctcagtagggtcaacgctctacccggaaagccgtaagctacttaagagctggcacctaccatcggtgttccatttaaagggcaagctcagcttcacatgccgctgtgatac

SEQ ID NO: 727 - DNA, 120 bp, synthetic construct
  source 1..120: mol_type = other DNA
gcacctaccatcggtgttccatttaaagggcaagctcagcttcacatgccgctgtgatacagtggtttcgtgcgaaggctacgtcgttaagagaataacgatgagcccaggcctttacgg

SEQ ID NO: 728 - DNA, 120 bp, synthetic construct
  source 1..120: mol_type = other DNA
agtggtttcgtgcgaaggctacgtcgttaagagaataacgatgagcccaggcctttacggaaaaaccacagggtatgcggtaacccaccacgcagacggattcctgatgtgcaagaccac

SEQ ID NO: 729 - DNA, 120 bp, synthetic construct
  source 1..120: mol_type = other DNA
aaaaaccacagggtatgcggtaacccaccacgcagacggattcctgatgtgcaagaccaccgacacggttgacggcgaaagagtgtcattctcggtgtgcacgtacgtgccggcgaccat

SEQ ID NO: 730 - DNA, 120 bp, synthetic construct
  source 1..120: mol_type = other DNA
cgacacggttgacggcgaaagagtgtcattctcggtgtgcacgtacgtgccggcgaccatttgtgatcaaatgaccggcatccttgctacagaagtcacgccggaggatgcacagaagct

SEQ ID NO: 731 - DNA, 120 bp, synthetic construct
  source 1..120: mol_type = other DNA
ttgtgatcaaatgaccggcatccttgctacagaagtcacgccggaggatgcacagaagctgttggtggggctgaaccagagaatagtggttaacggcagaacgcaacggaatacgaacac

SEQ ID NO: 732 - DNA, 120 bp, synthetic construct
  source 1..120: mol_type = other DNA
gttggtggggctgaaccagagaatagtggttaacggcagaacgcaacggaatacgaacaccatgaaaaactatatgattcccgtggtcgcccaagccttcagtaagtgggcaaaggagtg

SEQ ID NO: 733 - DNA, 120 bp, synthetic construct
  source 1..120: mol_type = other DNA
catgaaaaactatatgattcccgtggtcgcccaagccttcagtaagtgggcaaaggagtgccggaaagacatggaagatgaaaaactcctgggggtcagagaaagaacactgacctgctg

SEQ ID NO: 734 - DNA, 120 bp, synthetic construct
  source 1..120: mol_type = other DNA
ccggaaagacatggaagatgaaaaactcctgggggtcagagaaagaacactgacctgctgctgtctatgggcatttaagaagcagaaaacacacacggtctacaagaggcctgataccca

SEQ ID NO: 735 - DNA, 120 bp, synthetic construct
  source 1..120: mol_type = other DNA
ctgtctatgggcatttaagaagcagaaaacacacacggtctacaagaggcctgatacccagtcaattcagaaggttcaggccgagtttgacagctttgtggtaccgagcctgtggtcgtc

SEQ ID NO: 736 - DNA, 120 bp, synthetic construct
  source 1..120: mol_type = other DNA
gtcaattcagaaggttcaggccgagtttgacagctttgtggtaccgagcctgtggtcgtccgggttgtcaatcccgttgaggactagaatcaaatggttgttaagcaaggtgccaaaaac

SEQ ID NO: 737 - DNA, 120 bp, synthetic construct
  source 1..120: mol_type = other DNA
cgggttgtcaatcccgttgaggactagaatcaaatggttgttaagcaaggtgccaaaaaccgacctgaccccatacagcggggacgcccaagaagcccgggacgcagaaaaagaagcaga

SEQ ID NO: 738 - DNA, 120 bp, synthetic construct
  source 1..120: mol_type = other DNA
cgacctgaccccatacagcggggacgcccaagaagcccgggacgcagaaaaagaagcagaggaagaacgagaagcagaactgactcttgaagccctaccaccccttcaggcagcacagga

SEQ ID NO: 739 - DNA, 120 bp, synthetic construct
  source 1..120: mol_type = other DNA
ggaagaacgagaagcagaactgactcttgaagccctaccaccccttcaggcagcacaggaagatgttcaggtcgaaatcgacgtggaacagcttgaggacagagcgggtgcaggaataat

SEQ ID NO: 740 - DNA, 120 bp, synthetic construct
  source 1..120: mol_type = other DNA
agatgttcaggtcgaaatcgacgtggaacagcttgaggacagagcgggtgcaggaataatagagactccgagaggagctatcaaagttactgcccaaccaacagaccacgtcgtgggaga

SEQ ID NO: 741 - DNA, 120 bp, synthetic construct
  source 1..120: mol_type = other DNA
agagactccgagaggagctatcaaagttactgcccaaccaacagaccacgtcgtgggagagtacttggttctttccccgcagaccgtactacgtagccaaaagcttagcctgattcacgc

SEQ ID NO: 742 - DNA, 120 bp, synthetic construct
  source 1..120: mol_type = other DNA
gtacttggttctttccccgcagaccgtactacgtagccaaaagcttagcctgattcacgctttggcggagcaagtgaagacgtgcacgcacagcggacgagcagggaggtatgcggtcga

SEQ ID NO: 743 - DNA, 120 bp, synthetic construct
  source 1..120: mol_type = other DNA
tttggcggagcaagtgaagacgtgcacgcacagcggacgagcagggaggtatgcggtcgaagcgtacgacggcagagtcctagtgccctcaggctacgcaatctcgcctgaagacttcca

SEQ ID NO: 744 - DNA, 120 bp, synthetic construct
  source 1..120: mol_type = other DNA
agcgtacgacggcagagtcctagtgccctcaggctacgcaatctcgcctgaagacttccagagcctaagcgaaagcgcaacgatggtgtacaacgaaagagagttcgtaaacagaaagct

SEQ ID NO: 745 - DNA, 120 bp, synthetic construct
  source 1..120: mol_type = other DNA
gagcctaagcgaaagcgcaacgatggtgtacaacgaaagagagttcgtaaacagaaagctacaccatattgcgatgcatggaccagccctgaacaccgacgaagagtcgtatgagctggt

SEQ ID NO: 746 - DNA, 120 bp, synthetic construct
  source 1..120: mol_type = other DNA
acaccatattgcgatgcatggaccagccctgaacaccgacgaagagtcgtatgagctggtgagggcagagaggacagaacacgagtacgtctacgacgtggaccagagaagatgctgtaa

SEQ ID NO: 747 - DNA, 120 bp, synthetic construct
  source 1..120: mol_type = other DNA
gagggcagagaggacagaacacgagtacgtctacgacgtggaccagagaagatgctgtaagaaggaagaagctgcaggactggtactggtgggcgacttgactaatccgccctaccacga

SEQ ID NO: 748 - DNA, 120 bp, synthetic construct
  source 1..120: mol_type = other DNA
gaaggaagaagctgcaggactggtactggtgggcgacttgactaatccgccctaccacgaattcgcatatgaagggctaaaaatccgccctgcctgcccatacaaaattgcagtcatagg

SEQ ID NO: 749 - DNA, 120 bp, synthetic construct
  source 1..120: mol_type = other DNA
attcgcatatgaagggctaaaaatccgccctgcctgcccatacaaaattgcagtcataggagtcttcggagtaccaggatctggcaagtcagctattatcaagaacctagttaccaggca

SEQ ID NO: 750 - DNA, 120 bp, synthetic construct
  source 1..120: mol_type = other DNA
agtcttcggagtaccaggatctggcaagtcagctattatcaagaacctagttaccaggcaagacctggtgactagcggaaagaaagaaaactgccaagaaatcaccaccgacgtgatgag

SEQ ID NO: 751 - DNA, 120 bp, synthetic construct
  source 1..120: mol_type = other DNA
agacctggtgactagcggaaagaaagaaaactgccaagaaatcaccaccgacgtgatgagacagagaggtctagagatatctgcacgtacggttgactcgctgctcttgaatggatgtaa

SEQ ID NO: 752 - DNA, 120 bp, synthetic construct
  source 1..120: mol_type = other DNA
acagagaggtctagagatatctgcacgtacggttgactcgctgctcttgaatggatgtaacagaccagtcgacgtgttgtacgtagacgaggcgtttgcgtgccactctggaacgttact

SEQ ID NO: 753 - DNA, 120 bp, synthetic construct
  source 1..120: mol_type = other DNA
cagaccagtcgacgtgttgtacgtagacgaggcgtttgcgtgccactctggaacgttacttgcattgatcgccttggtgagaccaagacagaaagttgtactttgtggtgacccgaagca

SEQ ID NO: 754 - DNA, 120 bp, synthetic construct
  source 1..120: mol_type = other DNA
tgcattgatcgccttggtgagaccaagacagaaagttgtactttgtggtgacccgaagcagtgcggcttcttcaatatgatgcagatgaaagtcaactataatcacaacatctgcaccca

SEQ ID NO: 755 - DNA, 120 bp, synthetic construct
  source 1..120: mol_type = other DNA
gtgcggcttcttcaatatgatgcagatgaaagtcaactataatcacaacatctgcacccaagtgtaccacaaaagtatctccaggcggtgtacactgcctgtgactgccattgtgtcatc

SEQ ID NO: 756 - DNA, 120 bp, synthetic construct
  source 1..120: mol_type = other DNA
agtgtaccacaaaagtatctccaggcggtgtacactgcctgtgactgccattgtgtcatcgttgcattacgaaggcaaaatgcgcactacgaatgagtacaacaagccgattgtagtgga

SEQ ID NO: 757 - DNA, 120 bp, synthetic construct
  source 1..120: mol_type = other DNA
gttgcattacgaaggcaaaatgcgcactacgaatgagtacaacaagccgattgtagtggacactacaggctcaacaaaacctgaccctggagatctcgtgttaacgtgcttcagaggatg

SEQ ID NO: 758 - DNA, 120 bp, synthetic construct
  source 1..120: mol_type = other DNA
cactacaggctcaacaaaacctgaccctggagatctcgtgttaacgtgcttcagaggatgggttaaacaactgcaaattgactatcgtggacacgaggtcatgacagcagccgcatccca

SEQ ID NO: 759 - DNA, 120 bp, synthetic construct
  source 1..120: mol_type = other DNA
ggttaaacaactgcaaattgactatcgtggacacgaggtcatgacagcagccgcatcccaagggttaaccagaaaaggagtttacgcagttaggcaaaaagttaacgaaaacccgcttta

SEQ ID NO: 760 - DNA, 120 bp, synthetic construct
  source 1..120: mol_type = other DNA
agggttaaccagaaaaggagtttacgcagttaggcaaaaagttaacgaaaacccgctttatgcatcaacgtcagagcacgtcaacgtactcctaacgcgtacggaaggtaaactggtatg

SEQ ID NO: 761 - DNA, 120 bp, synthetic construct
  source 1..120: mol_type = other DNA
tgcatcaacgtcagagcacgtcaacgtactcctaacgcgtacggaaggtaaactggtatggaagacactctccggtgacccgtggataaagacgctgcagaacccaccgaaaggaaactt

SEQ ID NO: 762 - DNA, 120 bp, synthetic construct
  source 1..120: mol_type = other DNA
gaagacactctccggtgacccgtggataaagacgctgcagaacccaccgaaaggaaacttcaaagcaactattaaggagtgggaggtggagcatgcatcaataatggcgggcatctgcag

SEQ ID NO: 763 - DNA, 120 bp, synthetic construct
  source 1..120: mol_type = other DNA
caaagcaactattaaggagtgggaggtggagcatgcatcaataatggcgggcatctgcagtcaccaaatgacctttgatacattccaaaacaaagccaacgtttgttgggctaagagttt

SEQ ID NO: 764 - DNA, 120 bp, synthetic construct
  source 1..120: mol_type = other DNA
tcaccaaatgacctttgatacattccaaaacaaagccaacgtttgttgggctaagagtttggtccctatcctcgaaacagcggggataaaactaaacgacaggcagtggtcccagataat

SEQ ID NO: 765 - DNA, 120 bp, synthetic construct
  source 1..120: mol_type = other DNA
ggtccctatcctcgaaacagcggggataaaactaaacgacaggcagtggtcccagataattcaagccttcaaagaagacaaagcatattcacccgaagtagccctgaatgaaatatgcac

SEQ ID NO: 766 - DNA, 120 bp, synthetic construct
  source 1..120: mol_type = other DNA
tcaagccttcaaagaagacaaagcatattcacccgaagtagccctgaatgaaatatgcacgcgcatgtatggggtggatctagacagcgggctattttctaaaccgttggtgtctgtgta

SEQ ID NO: 767 - DNA, 120 bp, synthetic construct
  source 1..120: mol_type = other DNA
gcgcatgtatggggtggatctagacagcgggctattttctaaaccgttggtgtctgtgtattacgcggataaccactgggataataggcctggagggaagatgttcggattcaaccccga

SEQ ID NO: 768 - DNA, 120 bp, synthetic construct
  source 1..120: mol_type = other DNA
ttacgcggataaccactgggataataggcctggagggaagatgttcggattcaaccccgaggcagcatccattctagaaagaaagtatccatttacaaaagggaagtggaacatcaacaa

SEQ ID NO: 769 - DNA, 120 bp, synthetic construct
  source 1..120: mol_type = other DNA
ggcagcatccattctagaaagaaagtatccatttacaaaagggaagtggaacatcaacaagcagatctgcgtgactaccaggaggatagaagacttcaaccctaccaccaacattatacc

SEQ ID NO: 770 - DNA, 120 bp, synthetic construct
  source 1..120: mol_type = other DNA
gcagatctgcgtgactaccaggaggatagaagacttcaaccctaccaccaacattataccggccaacaggagactaccacactcattagtggccgaacaccgcccagtaaaaggggaaag

SEQ ID NO: 771 - DNA, 120 bp, synthetic construct
  source 1..120: mol_type = other DNA
ggccaacaggagactaccacactcattagtggccgaacaccgcccagtaaaaggggaaagaatggaatggctggttaacaagataaacggccaccacgtgctcctggtcagtggctgtag

SEQ ID NO: 772 - DNA, 120 bp, synthetic construct
  source 1..120: mol_type = other DNA
aatggaatggctggttaacaagataaacggccaccacgtgctcctggtcagtggctgtagccttgcactgcctactaagagagtcacttgggtagcgccactaggtgtccgcggagcgga

SEQ ID NO: 773 - DNA, 120 bp, synthetic construct
  source 1..120: mol_type = other DNA
ccttgcactgcctactaagagagtcacttgggtagcgccactaggtgtccgcggagcggactatacatacaacctagagttgggtctgccagcaacgcttggtaggtatgacctagtggt

SEQ ID NO: 774 - DNA, 120 bp, synthetic construct
  source 1..120: mol_type = other DNA
ctatacatacaacctagagttgggtctgccagcaacgcttggtaggtatgacctagtggtcataaacatccacacaccttttcgcatacaccattatcaacagtgcgtagaccacgcaat

SEQ ID NO: 775 - DNA, 120 bp, synthetic construct
  source 1..120: mol_type = other DNA
cataaacatccacacaccttttcgcatacaccattatcaacagtgcgtagaccacgcaatgaaactgcaaatgctcgggggtgactcattgagactgctcaaaccgggtggctctctatt

SEQ ID NO: 776 - DNA, 120 bp, synthetic construct
  source 1..120: mol_type = other DNA
gaaactgcaaatgctcgggggtgactcattgagactgctcaaaccgggtggctctctattgatcagagcatatggttacgcagatagaaccagtgaacgagtcatctgcgtattgggacg

SEQ ID NO: 777 - DNA, 120 bp, synthetic construct
  source 1..120: mol_type = other DNA
gatcagagcatatggttacgcagatagaaccagtgaacgagtcatctgcgtattgggacgcaagtttagatcatctagagcgttgaaaccaccatgtgtcaccagcaacactgagatgtt

SEQ ID NO: 778 - DNA, 120 bp, synthetic construct
  source 1..120: mol_type = other DNA
caagtttagatcatctagagcgttgaaaccaccatgtgtcaccagcaacactgagatgttttttctattcagcaactttgacaatggcagaaggaatttcacaactcatgtcatgaacaa

SEQ ID NO: 779 - DNA, 120 bp, synthetic construct
  source 1..120: mol_type = other DNA
ttttctattcagcaactttgacaatggcagaaggaatttcacaactcatgtcatgaacaatcaactgaatgcagcctttgtaggacaggccacccgagcaggatgtgcaccgtcgtaccg

SEQ ID NO: 780 - DNA, 120 bp, synthetic construct
  source 1..120: mol_type = other DNA
tcaactgaatgcagcctttgtaggacaggccacccgagcaggatgtgcaccgtcgtaccgggtaaaacgcatggatatcgcgaagaacgatgaagagtgcgtagtcaacgccgccaaccc

SEQ ID NO: 781 - DNA, 120 bp, synthetic construct
  source 1..120: mol_type = other DNA
ggtaaaacgcatggatatcgcgaagaacgatgaagagtgcgtagtcaacgccgccaaccctcgcgggttaccaggtgacggtgtttgcaaggcagtatacaaaaaatggccggagtcctt

SEQ ID NO: 782 - DNA, 120 bp, synthetic construct
  source 1..120: mol_type = other DNA
tcgcgggttaccaggtgacggtgtttgcaaggcagtatacaaaaaatggccggagtcctttaagaacagtgcaacaccagtgggaaccgcaaaaacagtcatgtgcggtacgtatccagt

SEQ ID NO: 783 - DNA, 120 bp, synthetic construct
  source 1..120: mol_type = other DNA
taagaacagtgcaacaccagtgggaaccgcaaaaacagtcatgtgcggtacgtatccagtaatccacgccgttggaccaaacttctctaattattcggagtctgaaggggaccgagaatt

SEQ ID NO: 784 - DNA, 120 bp, synthetic construct
  source 1..120: mol_type = other DNA
aatccacgccgttggaccaaacttctctaattattcggagtctgaaggggaccgagaattggcggctgcctatcgagaagtcgcaaaggaggtaactagactgggagtaaatagtgtagc

SEQ ID NO: 785 - DNA, 120 bp, synthetic construct
  source 1..120: mol_type = other DNA
ggcggctgcctatcgagaagtcgcaaaggaggtaactagactgggagtaaatagtgtagctatacctctcctctccacaggtgtatactcaggagggaaagacaggctgacccagtcact

SEQ ID NO: 786 - DNA, 120 bp, synthetic construct
  source 1..120: mol_type = other DNA
tatacctctcctctccacaggtgtatactcaggagggaaagacaggctgacccagtcactgaaccacctctttacagccatggactcgacggatgcagacgtggtcatctactgccgcga

SEQ ID NO: 787 - DNA, 120 bp, synthetic construct
  source 1..120: mol_type = other DNA
gaaccacctctttacagccatggactcgacggatgcagacgtggtcatctactgccgcgacaaagaatgggagaagaaaatatctgaggccatacagatgcggacccaagtggagctgct

SEQ ID NO: 788 - DNA, 120 bp, synthetic construct
  source 1..120: mol_type = other DNA
caaagaatgggagaagaaaatatctgaggccatacagatgcggacccaagtggagctgctggatgagcacatctccatagactgcgatgttgttcgcgtgcaccctgacagcagcttggc

SEQ ID NO: 789 - DNA, 120 bp, synthetic construct
  source 1..120: mol_type = other DNA
ggatgagcacatctccatagactgcgatgttgttcgcgtgcaccctgacagcagcttggcaggcagaaaaggatacagcaccacggaaggcgcactgtactcatatctagaagggacccg

SEQ ID NO: 790 - DNA, 120 bp, synthetic construct
  source 1..120: mol_type = other DNA
aggcagaaaaggatacagcaccacggaaggcgcactgtactcatatctagaagggacccgttttcaccaaacggcagtggatatggcagagatatatactatgtggccaaagcaaacaga

SEQ ID NO: 791 - DNA, 120 bp, synthetic construct
  source 1..120: mol_type = other DNA
ttttcaccaaacggcagtggatatggcagagatatatactatgtggccaaagcaaacagaggccaacgagcaagtttgcctatatgccctgggggaaagtattgaatcgatcaggcagaa

SEQ ID NO: 792 - DNA, 120 bp, synthetic construct
  source 1..120: mol_type = other DNA
ggccaacgagcaagtttgcctatatgccctgggggaaagtattgaatcgatcaggcagaaatgcccggtggatgatgcagatgcatcatctcccccgaaaactgtcccgtgcctctgccg

SEQ ID NO: 793 - DNA, 120 bp, synthetic construct
  source 1..120: mol_type = other DNA
atgcccggtggatgatgcagatgcatcatctcccccgaaaactgtcccgtgcctctgccgttacgccatgacaccagaacgcgttacccgacttcgcatgaaccatgtcacaagcataat

SEQ ID NO: 794 - DNA, 120 bp, synthetic construct
  source 1..120: mol_type = other DNA
ttacgccatgacaccagaacgcgttacccgacttcgcatgaaccatgtcacaagcataattgtgtgttcttcgtttccccttccaaagtacaaaatagaaggagtgcaaaaagtcaaatg

SEQ ID NO: 795 - DNA, 120 bp, synthetic construct
  source 1..120: mol_type = other DNA
tgtgtgttcttcgtttccccttccaaagtacaaaatagaaggagtgcaaaaagtcaaatgctccaaggtaatgctatttgaccacaacgtgccatcgcgcgtaagtccaagggaatacag

SEQ ID NO: 796 - DNA, 120 bp, synthetic construct
  source 1..120: mol_type = other DNA
ctccaaggtaatgctatttgaccacaacgtgccatcgcgcgtaagtccaagggaatacagaccttcccaggagtctgtacaggaagcgagtacgaccacgtcactgacgcatagccaatt

SEQ ID NO: 797 - DNA, 120 bp, synthetic construct
  source 1..120: mol_type = other DNA
accttcccaggagtctgtacaggaagcgagtacgaccacgtcactgacgcatagccaattcgatctaagcgttgacggcaagatactgcccgtcccgtcagacctggatgctgacgcccc

SEQ ID NO: 798 - DNA, 120 bp, synthetic construct
  source 1..120: mol_type = other DNA
cgatctaagcgttgacggcaagatactgcccgtcccgtcagacctggatgctgacgccccagccctagaaccagcccttgacgacggggcgatacacacgttgccatctgcaaccggaaa

SEQ ID NO: 799 - DNA, 120 bp, synthetic construct
  source 1..120: mol_type = other DNA
agccctagaaccagcccttgacgacggggcgatacacacgttgccatctgcaaccggaaaccttgcggccgtgtctgactgggtaatgagcaccgtacctgtcgcgccgcccagaagaag

SEQ ID NO: 800 - DNA, 120 bp, synthetic construct
  source 1..120: mol_type = other DNA
ccttgcggccgtgtctgactgggtaatgagcaccgtacctgtcgcgccgcccagaagaaggcgagggagaaacctgactgtgacatgcgacgagagagaagggaatataacacccatggc

SEQ ID NO: 801 - DNA, 120 bp, synthetic construct
  source 1..120: mol_type = other DNA
gcgagggagaaacctgactgtgacatgcgacgagagagaagggaatataacacccatggctagcgtccgattctttagggcagagctgtgtccagtcgtacaagaaacagcggagacgcg

SEQ ID NO: 802 - DNA, 120 bp, synthetic construct
  source 1..120: mol_type = other DNA
tagcgtccgattctttagggcagagctgtgtccagtcgtacaagaaacagcggagacgcgtgacacagctatgtctcttcaggcaccgccgagtaccgccacggaactgagtcacccgcc

SEQ ID NO: 803 - DNA, 120 bp, synthetic construct
  source 1..120: mol_type = other DNA
tgacacagctatgtctcttcaggcaccgccgagtaccgccacggaactgagtcacccgccgatctccttcggtgcaccaagcgagacgttccccatcacatttggggacttcaacgaagg

SEQ ID NO: 804 - DNA, 120 bp, synthetic construct
  source 1..120: mol_type = other DNA
gatctccttcggtgcaccaagcgagacgttccccatcacatttggggacttcaacgaaggagaaatcgaaagcttgtcttctgagctactaactttcggagacttcctacccggagaagt

SEQ ID NO: 805 - DNA, 120 bp, synthetic construct
  source 1..120: mol_type = other DNA
agaaatcgaaagcttgtcttctgagctactaactttcggagacttcctacccggagaagtggatgatttgacagatagcgactggtccacgtgctcagacacggacgacgagttacgact

SEQ ID NO: 806 - DNA, 120 bp, synthetic construct
  source 1..120: mol_type = other DNA
ggatgatttgacagatagcgactggtccacgtgctcagacacggacgacgagttacgactagacagggcaggtgggtatatattctcgtcggacactggtccaggtcatttacaacagaa

SEQ ID NO: 807 - DNA, 120 bp, synthetic construct
  source 1..120: mol_type = other DNA
agacagggcaggtgggtatatattctcgtcggacactggtccaggtcatttacaacagaagtcagtacgccagtcagtgctgccggtgaacaccctggaggaagtccacgaggagaagtg

SEQ ID NO: 808 - DNA, 120 bp, synthetic construct
  source 1..120: mol_type = other DNA
gtcagtacgccagtcagtgctgccggtgaacaccctggaggaagtccacgaggagaagtgttacccacctaagctggatgaagcaaaggagcaactactacttaagaaactccaggagag

SEQ ID NO: 809 - DNA, 120 bp, synthetic construct
  source 1..120: mol_type = other DNA
ttacccacctaagctggatgaagcaaaggagcaactactacttaagaaactccaggagagtgcatccatggccaacagaagcaggtatcagtcgcgcaaagtagaaaacatgaaagcaac

SEQ ID NO: 810 - DNA, 120 bp, synthetic construct
  source 1..120: mol_type = other DNA
tgcatccatggccaacagaagcaggtatcagtcgcgcaaagtagaaaacatgaaagcaacaatcatccagagactaaagagaggctgtagattatacttaatgtcagagaccccaaaagt

SEQ ID NO: 811 - DNA, 120 bp, synthetic construct
  source 1..120: mol_type = other DNA
aatcatccagagactaaagagaggctgtagattatacttaatgtcagagaccccaaaagtccctacctaccggaccacatatccggcgcctgtgtactcgcctccgattaacgtccgact

SEQ ID NO: 812 - DNA, 120 bp, synthetic construct
  source 1..120: mol_type = other DNA
ccctacctaccggaccacatatccggcgcctgtgtactcgcctccgattaacgtccgactgtccaaccccgagtccgcagtggcagcatgcaatgagttcttggctagaaactatccaac

SEQ ID NO: 813 - DNA, 120 bp, synthetic construct
  source 1..120: mol_type = other DNA
gtccaaccccgagtccgcagtggcagcatgcaatgagttcttggctagaaactatccaactgtttcatcataccaaatcaccgacgagtatgatgcatatctagacatggtggacgggtc

SEQ ID NO: 814 - DNA, 120 bp, synthetic construct
  source 1..120: mol_type = other DNA
tgtttcatcataccaaatcaccgacgagtatgatgcatatctagacatggtggacgggtcggagagttgtctggaccgagcgacattcaatccgtcaaaacttaggagctacccaaaaca

SEQ ID NO: 815 - DNA, 120 bp, synthetic construct
  source 1..120: mol_type = other DNA
ggagagttgtctggaccgagcgacattcaatccgtcaaaacttaggagctacccaaaacagcacgcttaccacgcgccctccatcagaagcgctgtaccgtccccattccagaacacact

SEQ ID NO: 816 - DNA, 120 bp, synthetic construct
  source 1..120: mol_type = other DNA
gcacgcttaccacgcgccctccatcagaagcgctgtaccgtccccattccagaacacactacagaatgtactggcagcagccacgaaaagaaactgcaacgtcacacagatgagggaatt

SEQ ID NO: 817 - DNA, 120 bp, synthetic construct
  source 1..120: mol_type = other DNA
acagaatgtactggcagcagccacgaaaagaaactgcaacgtcacacagatgagggaattacccactttggactcagcagtattcaacgtggagtgtttcaaaaaattcgcatgcaacca

SEQ ID NO: 818 - DNA, 120 bp, synthetic construct
  source 1..120: mol_type = other DNA
acccactttggactcagcagtattcaacgtggagtgtttcaaaaaattcgcatgcaaccaagaatactgggaagaatttgctgccagccctatcaggataacaactgagaatttaacaac

SEQ ID NO: 819 - DNA, 120 bp, synthetic construct
  source 1..120: mol_type = other DNA
agaatactgggaagaatttgctgccagccctatcaggataacaactgagaatttaacaacctatgttactaaactaaaggggccaaaagcagcagcgctatttgcaagaacccataatct

SEQ ID NO: 820 - DNA, 120 bp, synthetic construct
  source 1..120: mol_type = other DNA
ctatgttactaaactaaaggggccaaaagcagcagcgctatttgcaagaacccataatctgctgccactgcaggaagtgccaatggataggttcacagtagacatgaaaagggatgtgaa

SEQ ID NO: 821 - DNA, 120 bp, synthetic construct
  source 1..120: mol_type = other DNA
gctgccactgcaggaagtgccaatggataggttcacagtagacatgaaaagggatgtgaaggtgactcctggtacaaagcacacagaggaaagacctaaggtacaggttatacaggcggc

SEQ ID NO: 822 - DNA, 120 bp, synthetic construct
  source 1..120: mol_type = other DNA
ggtgactcctggtacaaagcacacagaggaaagacctaaggtacaggttatacaggcggctgaacccttggcaacagcatacctatgtgggattcacagagagctggttaggaggctgaa

SEQ ID NO: 823 - DNA, 120 bp, synthetic construct
  source 1..120: mol_type = other DNA
tgaacccttggcaacagcatacctatgtgggattcacagagagctggttaggaggctgaacgccgtcctcctacccaatgtacatacactatttgacatgtctgccgaggatttcgatgc

SEQ ID NO: 824 - DNA, 120 bp, synthetic construct
  source 1..120: mol_type = other DNA
cgccgtcctcctacccaatgtacatacactatttgacatgtctgccgaggatttcgatgccatcatagccgcacactttaagccaggagacactgttttagaaacggacatagcctcctt

SEQ ID NO: 825 - DNA, 120 bp, synthetic construct
  source 1..120: mol_type = other DNA
catcatagccgcacactttaagccaggagacactgttttagaaacggacatagcctcctttgataagagccaagatgattcacttgcgcttactgctttaatgctgttagaggatttagg

SEQ ID NO: 826 - DNA, 120 bp, synthetic construct
  source 1..120: mol_type = other DNA
tgataagagccaagatgattcacttgcgcttactgctttaatgctgttagaggatttaggggtggatcactccctgttggacttgatagaggctgctttcggagagatttccagctgtca

SEQ ID NO: 827 - DNA, 120 bp, synthetic construct
  source 1..120: mol_type = other DNA
ggtggatcactccctgttggacttgatagaggctgctttcggagagatttccagctgtcatctaccgacaggtacgcgcttcaagttcggcgccatgatgaaatctggtatgttcctaac

SEQ ID NO: 828 - DNA, 120 bp, synthetic construct
  source 1..120: mol_type = other DNA
tctaccgacaggtacgcgcttcaagttcggcgccatgatgaaatctggtatgttcctaactctgttcgtcaacacactgctaaatatcaccatcgccagccgagtgctggaagatcgtct

SEQ ID NO: 829 - DNA, 120 bp, synthetic construct
  source 1..120: mol_type = other DNA
tctgttcgtcaacacactgctaaatatcaccatcgccagccgagtgctggaagatcgtctgacaaaatccgcgtgcgcagccttcatcggcgacgacaacataatacatggagtcgtctc

SEQ ID NO: 830 - DNA, 120 bp, synthetic construct
  source 1..120: mol_type = other DNA
gacaaaatccgcgtgcgcagccttcatcggcgacgacaacataatacatggagtcgtctccgatgaattgatggcagccagatgcgccacttggatgaacatggaagtgaagatcataga

SEQ ID NO: 831 - DNA, 120 bp, synthetic construct
  source 1..120: mol_type = other DNA
cgatgaattgatggcagccagatgcgccacttggatgaacatggaagtgaagatcatagatgcagttgtatcccagaaagccccttacttttgtggagggtttatactgcacgatatcgt

SEQ ID NO: 832 - DNA, 120 bp, synthetic construct
  source 1..120: mol_type = other DNA
tgcagttgtatcccagaaagccccttacttttgtggagggtttatactgcacgatatcgtgacaggaacagcttgcagagtggcagacccgctaaaaaggctatttaaactgggcaaacc

SEQ ID NO: 833 - DNA, 120 bp, synthetic construct
  source 1..120: mol_type = other DNA
gacaggaacagcttgcagagtggcagacccgctaaaaaggctatttaaactgggcaaaccgctagcggcaggtgacgaacaagatgaggatagaagacgagcgctggctgacgaagtggt

SEQ ID NO: 834 - DNA, 120 bp, synthetic construct
  source 1..120: mol_type = other DNA
gctagcggcaggtgacgaacaagatgaggatagaagacgagcgctggctgacgaagtggtcagatggcaacgaacagggctaattgatgagttggagaaagcggtatactctaggtatga

SEQ ID NO: 835 - DNA, 120 bp, synthetic construct
  source 1..120: mol_type = other DNA
cagatggcaacgaacagggctaattgatgagttggagaaagcggtatactctaggtatgaagtgcagggtatatcagttgtggtaatgtccatggccacctttgcaagctccagatccaa

SEQ ID NO: 836 - DNA, 120 bp, synthetic construct
  source 1..120: mol_type = other DNA
agtgcagggtatatcagttgtggtaatgtccatggccacctttgcaagctccagatccaacttcgagaagctcagaggacccgtcgtaactttgtacggcggtcctaaataggtacgcac

SEQ ID NO: 837 - DNA, 120 bp, synthetic construct
  source 1..120: mol_type = other DNA
cttcgagaagctcagaggacccgtcgtaactttgtacggcggtcctaaataggtacgcactacagctacctattttgcagaagccgacagtaagtacctaaacactaatcagctacaatg

SEQ ID NO: 838 - DNA, 120 bp, synthetic construct
  source 1..120: mol_type = other DNA
tacagctacctattttgcagaagccgacagtaagtacctaaacactaatcagctacaatggagttcatcccaacccaaactttttacaacaggaggtaccagcctcgaccctggactccg

SEQ ID NO: 839 - DNA, 120 bp, synthetic construct
  source 1..120: mol_type = other DNA
gagttcatcccaacccaaactttttacaacaggaggtaccagcctcgaccctggactccgcgccctactatccaagtcatcaggcccagaccgcgcccgcagaggcaagctgggcaactt

SEQ ID NO: 840 - DNA, 120 bp, synthetic construct
  source 1..120: mol_type = other DNA
cgccctactatccaagtcatcaggcccagaccgcgcccgcagaggcaagctgggcaacttgcccagctgatctcagcagttaataaactgacaatgcgcgcggtaccccaacagaagcca

SEQ ID NO: 841 - DNA, 120 bp, synthetic construct
  source 1..120: mol_type = other DNA
gcccagctgatctcagcagttaataaactgacaatgcgcgcggtaccccaacagaagccacgcaggaatcggaagaataagaagcaaaagcaaaagcaacaggcgccacaaaacaacaca

SEQ ID NO: 842 - DNA, 120 bp, synthetic construct
  source 1..120: mol_type = other DNA
cgcaggaatcggaagaataagaagcaaaagcaaaagcaacaggcgccacaaaacaacacaaaccaaaagaagcagccacctaaaaagaaaccagctcaaaagaaaaagaagccgggccgc

SEQ ID NO: 843 - DNA, 120 bp, synthetic construct
  source 1..120: mol_type = other DNA
aaccaaaagaagcagccacctaaaaagaaaccagctcaaaagaaaaagaagccgggccgcagagagaggatgtgcatgaaaatcgaaaatgactgtattttcgaagtcaagcacgaaggt

SEQ ID NO: 844 - DNA, 120 bp, synthetic construct
  source 1..120: mol_type = other DNA
agagagaggatgtgcatgaaaatcgaaaatgactgtattttcgaagtcaagcacgaaggtaaggtaacaggttacgcgtgcttggtgggggacaaagtaatgaaaccagcacacgtaaag

SEQ ID NO: 845 - DNA, 120 bp, synthetic construct
  source 1..120: mol_type = other DNA
aaggtaacaggttacgcgtgcttggtgggggacaaagtaatgaaaccagcacacgtaaaggggaccatcgataacgcggacctggccaaattggcctttaagcggtcatctaagtacgac

SEQ ID NO: 846 - DNA, 120 bp, synthetic construct
  source 1..120: mol_type = other DNA
gggaccatcgataacgcggacctggccaaattggcctttaagcggtcatctaagtacgaccttgaatgcgcgcagatacccgtgcacatgaagtccgacgcttcgaagttcacccatgag

SEQ ID NO: 847 - DNA, 120 bp, synthetic construct
  source 1..120: mol_type = other DNA
cttgaatgcgcgcagatacccgtgcacatgaagtccgacgcttcgaagttcacccatgagaaaccggaggggtactacaactggcaccacggagcagtacagtactcaggaggccggttc

SEQ ID NO: 848 - DNA, 120 bp, synthetic construct
  source 1..120: mol_type = other DNA
aaaccggaggggtactacaactggcaccacggagcagtacagtactcaggaggccggttcaccatccctacaggtgcgggcaaaccaggggacagcggtagaccgatcttcgacaacaag

SEQ ID NO: 849 - DNA, 120 bp, synthetic construct
  source 1..120: mol_type = other DNA
accatccctacaggtgcgggcaaaccaggggacagcggtagaccgatcttcgacaacaagggacgcgtggtggccatagtcttaggaggagctaatgaaggagcccgtacagccctctca

SEQ ID NO: 850 - DNA, 120 bp, synthetic construct
  source 1..120: mol_type = other DNA
ggacgcgtggtggccatagtcttaggaggagctaatgaaggagcccgtacagccctctcagtggtgacctggaataaagacattgtcactaaaatcacccctgagggagccgaagagtgg

SEQ ID NO: 851 - DNA, 120 bp, synthetic construct
  source 1..120: mol_type = other DNA
gtggtgacctggaataaagacattgtcactaaaatcacccctgagggagccgaagagtggagtcttgccatcccagttatgtgcctgttggcaaataccacgttcccctgctcccagccc

SEQ ID NO: 852 - DNA, 120 bp, synthetic construct
  source 1..120: mol_type = other DNA
agtcttgccatcccagttatgtgcctgttggcaaataccacgttcccctgctcccagcccccttgcataccctgctgctacgaaaaggaaccggaggaaaccctacgcatgcttgaggac

SEQ ID NO: 853 - DNA, 120 bp, synthetic construct
  source 1..120: mol_type = other DNA
ccttgcataccctgctgctacgaaaaggaaccggaggaaaccctacgcatgcttgaggacaacgtcatgagacctgggtactatcagctgctacaagcatcattaacatgttctccccac

SEQ ID NO: 854 - DNA, 120 bp, synthetic construct
  source 1..120: mol_type = other DNA
aacgtcatgagacctgggtactatcagctgctacaagcatcattaacatgttctccccaccgccagcgacgcagcaccaaggacaacttcaatgtctataaagccacaagaccatactta

SEQ ID NO: 855 - DNA, 120 bp, synthetic construct
  source 1..120: mol_type = other DNA
cgccagcgacgcagcaccaaggacaacttcaatgtctataaagccacaagaccatacttagctcactgtcccgactgtggagaagggcactcgtgccatagtcccgtagcactagaacgc

SEQ ID NO: 856 - DNA, 120 bp, synthetic construct
  source 1..120: mol_type = other DNA
gctcactgtcccgactgtggagaagggcactcgtgccatagtcccgtagcactagaacgcatcagaaatgaagcgacagacgggacgctgaaaatccaggtctccttgcaaattggaata

SEQ ID NO: 857 - DNA, 120 bp, synthetic construct
  source 1..120: mol_type = other DNA
atcagaaatgaagcgacagacgggacgctgaaaatccaggtctccttgcaaattggaatagggacggatgatagccatgattggaccaagctgcgttacatggacaatcacataccagca

SEQ ID NO: 858 - DNA, 120 bp, synthetic construct
  source 1..120: mol_type = other DNA
gggacggatgatagccatgattggaccaagctgcgttacatggacaatcacataccagcagacgcagggagggccgggctatttgtaagaacatcagcaccatgcacgattactggaaca

SEQ ID NO: 859 - DNA, 120 bp, synthetic construct
  source 1..120: mol_type = other DNA
gacgcagggagggccgggctatttgtaagaacatcagcaccatgcacgattactggaacaatgggacacttcatcctggcccgatgtccgaaaggagaaactctgacggtgggattcact

SEQ ID NO: 860 - DNA, 120 bp, synthetic construct
  source 1..120: mol_type = other DNA
atgggacacttcatcctggcccgatgtccgaaaggagaaactctgacggtgggattcactgacagtaggaagattagtcactcatgtacgcacccatttcaccacgaccctcctgtgata

SEQ ID NO: 861 - DNA, 120 bp, synthetic construct
  source 1..120: mol_type = other DNA
gacagtaggaagattagtcactcatgtacgcacccatttcaccacgaccctcctgtgataggccgggaaaaattccattcccgaccgcagcacggtaaagagctaccttgcagcacgtac

SEQ ID NO: 862 - DNA, 120 bp, synthetic construct
  source 1..120: mol_type = other DNA
ggccgggaaaaattccattcccgaccgcagcacggtaaagagctaccttgcagcacgtacgtgcagagcaacgccgcaactgccgaggagatagaggtacacatgcccccagacacccct

SEQ ID NO: 863 - DNA, 120 bp, synthetic construct
  source 1..120: mol_type = other DNA
gtgcagagcaacgccgcaactgccgaggagatagaggtacacatgcccccagacacccctgatcgcacattgctgtcacaacagtccggcaacgtaaagatcacagtcaacggccggacg

SEQ ID NO: 864 - DNA, 120 bp, synthetic construct
  source 1..120: mol_type = other DNA
gatcgcacattgctgtcacaacagtccggcaacgtaaagatcacagtcaacggccggacggtgcggtataagtgtaattgcggtggctcaaatgaaggactaataactacagataaagtg

SEQ ID NO: 865 - DNA, 120 bp, synthetic construct
  source 1..120: mol_type = other DNA
gtgcggtataagtgtaattgcggtggctcaaatgaaggactaataactacagataaagtgattaataactgcaaggttgatcaatgtcatgccgcggtcaccaatcacaaaaagtggcag

SEQ ID NO: 866 - DNA, 120 bp, synthetic construct
  source 1..120: mol_type = other DNA
attaataactgcaaggttgatcaatgtcatgccgcggtcaccaatcacaaaaagtggcagtataactcccctctggtcccgcgtaacgctgaactcggggaccgaaaaggaaaaattcac

SEQ ID NO: 867 - DNA, 120 bp, synthetic construct
  source 1..120: mol_type = other DNA
tataactcccctctggtcccgcgtaacgctgaactcggggaccgaaaaggaaaaattcacatcccgtttccgctggcaaatgtaacatgcatggtgcctaaagcaaggaaccccaccgtg

SEQ ID NO: 868 - DNA, 120 bp, synthetic construct
  source 1..120: mol_type = other DNA
atcccgtttccgctggcaaatgtaacatgcatggtgcctaaagcaaggaaccccaccgtgacgtacgggaaaaaccaagtcatcatgctactgtatcctgaccacccaacactcctgtcc

SEQ ID NO: 869 - DNA, 120 bp, synthetic construct
  source 1..120: mol_type = other DNA
acgtacgggaaaaaccaagtcatcatgctactgtatcctgaccacccaacactcctgtcctaccggagtatgggagaagaaccaaactatcaagaagagtgggtgacgcacaagaaggag

SEQ ID NO: 870 - DNA, 120 bp, synthetic construct
  source 1..120: mol_type = other DNA
taccggagtatgggagaagaaccaaactatcaagaagagtgggtgacgcacaagaaggaggtcgtgctaaccgtgccgactgaagggctcgaggttacgtggggcaacaacgagccgtat

SEQ ID NO: 871 - DNA, 120 bp, synthetic construct
  source 1..120: mol_type = other DNA
gtcgtgctaaccgtgccgactgaagggctcgaggttacgtggggcaacaacgagccgtataagtattggccgcagttatctgcaaacggtacagcccacggccacccgcatgagataatc

SEQ ID NO: 872 - DNA, 120 bp, synthetic construct
  source 1..120: mol_type = other DNA
aagtattggccgcagttatctgcaaacggtacagcccacggccacccgcatgagataatcttgtactattatgagctgtaccctactatgactgtagtagttgtgtcagtggcctcgttc

SEQ ID NO: 873 - DNA, 120 bp, synthetic construct
  source 1..120: mol_type = other DNA
ttgtactattatgagctgtaccctactatgactgtagtagttgtgtcagtggcctcgttcatactcctgtcgatggtgggtatggcagtggggatgtgcatgtgtgcacgacgcagatgc

SEQ ID NO: 874 - DNA, 120 bp, synthetic construct
  source 1..120: mol_type = other DNA
atactcctgtcgatggtgggtatggcagtggggatgtgcatgtgtgcacgacgcagatgcatcacaccatacgaactgacaccaggagctaccgtccctttcctgcttagcctaatatgc

SEQ ID NO: 875 - DNA, 120 bp, synthetic construct
  source 1..120: mol_type = other DNA
atcacaccatacgaactgacaccaggagctaccgtccctttcctgcttagcctaatatgctgcatcagaacagctaaagcggccacataccaagaggctgcggtatacctgtggaacgag

SEQ ID NO: 876 - DNA, 120 bp, synthetic construct
  source 1..120: mol_type = other DNA
tgcatcagaacagctaaagcggccacataccaagaggctgcggtatacctgtggaacgagcagcaacctttgttttggctacaagcccttattccgctggcagccctgattgtcctatgc

SEQ ID NO: 877 - DNA, 120 bp, synthetic construct
  source 1..120: mol_type = other DNA
cagcaacctttgttttggctacaagcccttattccgctggcagccctgattgtcctatgcaactgtctgagactcttaccatgctgttgtaaaacgttggcttttttagccgtaatgagc

SEQ ID NO: 878 - DNA, 120 bp, synthetic construct
  source 1..120: mol_type = other DNA
aactgtctgagactcttaccatgctgttgtaaaacgttggcttttttagccgtaatgagcatcggtgcccacactgtgagcgcgtacgaacacgtaacagtgatcccgaacacggtggga

SEQ ID NO: 879 - DNA, 120 bp, synthetic construct
  source 1..120: mol_type = other DNA
atcggtgcccacactgtgagcgcgtacgaacacgtaacagtgatcccgaacacggtgggagtaccgtataagactctagtcaacagaccgggctacagccccatggtactggagatggag

SEQ ID NO: 880 - DNA, 120 bp, synthetic construct
  source 1..120: mol_type = other DNA
gtaccgtataagactctagtcaacagaccgggctacagccccatggtactggagatggagctactgtcagtcactttggagccaacgctatcgcttgattacatcacgtgcgaatacaaa

SEQ ID NO: 881 - DNA, 120 bp, synthetic construct
  source 1..120: mol_type = other DNA
ctactgtcagtcactttggagccaacgctatcgcttgattacatcacgtgcgaatacaaaaccgtcatcccgtctccgtacgtgaaatgctgcggtacagcagagtgcaaggacaaaaac

SEQ ID NO: 882 - DNA, 120 bp, synthetic construct
  source 1..120: mol_type = other DNA
accgtcatcccgtctccgtacgtgaaatgctgcggtacagcagagtgcaaggacaaaaacctacctgactacagctgtaaggtcttcaccggcgtctacccatttatgtggggcggcgcc

SEQ ID NO: 883 - DNA, 120 bp, synthetic construct
  source 1..120: mol_type = other DNA
ctacctgactacagctgtaaggtcttcaccggcgtctacccatttatgtggggcggcgcctactgcttctgcgacgctgaaaacacgcaattgagcgaagcacatgtggagaagtccgaa

SEQ ID NO: 884 - DNA, 120 bp, synthetic construct
  source 1..120: mol_type = other DNA
tactgcttctgcgacgctgaaaacacgcaattgagcgaagcacatgtggagaagtccgaatcatgcaaaacagaatttgcatcagcatacagggctcataccgcatccgcatcagctaag

SEQ ID NO: 885 - DNA, 120 bp, synthetic construct
  source 1..120: mol_type = other DNA
tcatgcaaaacagaatttgcatcagcatacagggctcataccgcatccgcatcagctaagctccgcgtcctttaccaaggaaataacatcactgtaactgcctatgcaaacggcgaccat

SEQ ID NO: 886 - DNA, 120 bp, synthetic construct
  source 1..120: mol_type = other DNA
ctccgcgtcctttaccaaggaaataacatcactgtaactgcctatgcaaacggcgaccatgccgtcacagttaaggacgccaaattcattgtggggccaatgtcttcagcctggacacct

SEQ ID NO: 887 - DNA, 120 bp, synthetic construct
  source 1..120: mol_type = other DNA
gccgtcacagttaaggacgccaaattcattgtggggccaatgtcttcagcctggacacctttcgacaacaaaatcgtggtgtacaaaggtgacgtttacaacatggactacccgcccttt

SEQ ID NO: 888 - DNA, 120 bp, synthetic construct
  source 1..120: mol_type = other DNA
ttcgacaacaaaatcgtggtgtacaaaggtgacgtttacaacatggactacccgccctttggcgcaggaagaccaggacaatttggcgatatccaaagtcgcacgcctgagagcaaagac

SEQ ID NO: 889 - DNA, 120 bp, synthetic construct
  source 1..120: mol_type = other DNA
ggcgcaggaagaccaggacaatttggcgatatccaaagtcgcacgcctgagagcaaagacgtctatgctaacacacaactggtactgcagagaccggctgcgggtacggtacacgtgcca

SEQ ID NO: 890 - DNA, 120 bp, synthetic construct
  source 1..120: mol_type = other DNA
gtctatgctaacacacaactggtactgcagagaccggctgcgggtacggtacacgtgccatactctcaggcaccatctggctttaagtattggttaaaagaacgaggggcgtcgctacag

SEQ ID NO: 891 - DNA, 120 bp, synthetic construct
  source 1..120: mol_type = other DNA
tactctcaggcaccatctggctttaagtattggttaaaagaacgaggggcgtcgctacagcacacagcaccatttggctgccaaatagcaacaaacccggtaagagcgatgaactgcgcc

SEQ ID NO: 892 - DNA, 120 bp, synthetic construct
  source 1..120: mol_type = other DNA
cacacagcaccatttggctgccaaatagcaacaaacccggtaagagcgatgaactgcgccgtagggaacatgcccatctccatcgacataccggatgcggccttcactagggtcgtcgac

SEQ ID NO: 893 - DNA, 120 bp, synthetic construct
  source 1..120: mol_type = other DNA
gtagggaacatgcccatctccatcgacataccggatgcggccttcactagggtcgtcgacgcgccctctttaacggacatgtcatgcgaggtaccagcctgcacccattcctcagacttt

SEQ ID NO: 894 - DNA, 120 bp, synthetic construct
  source 1..120: mol_type = other DNA
gcgccctctttaacggacatgtcatgcgaggtaccagcctgcacccattcctcagactttgggggcgtcgccattattaaatatgcagtcagcaagaaaggcaagtgtgcggtgcattcg

SEQ ID NO: 895 - DNA, 120 bp, synthetic construct
  source 1..120: mol_type = other DNA
gggggcgtcgccattattaaatatgcagtcagcaagaaaggcaagtgtgcggtgcattcgatgaccaacgccgtcactatccgggaagctgagatagaagttgaagggaattctcagctg

SEQ ID NO: 896 - DNA, 120 bp, synthetic construct
  source 1..120: mol_type = other DNA
atgaccaacgccgtcactatccgggaagctgagatagaagttgaagggaattctcagctgcaaatctctttctcgacggccttggccagcgccgaattccgcgtacaagtctgttctaca

SEQ ID NO: 897 - DNA, 120 bp, synthetic construct
  source 1..120: mol_type = other DNA
caaatctctttctcgacggccttggccagcgccgaattccgcgtacaagtctgttctacacaagtacactgtgcagccgagtgccaccctccgaaggaccacatagtcaactacccggcg

SEQ ID NO: 898 - DNA, 120 bp, synthetic construct
  source 1..120: mol_type = other DNA
caagtacactgtgcagccgagtgccaccctccgaaggaccacatagtcaactacccggcgtcacataccaccctcggggtccaggacatttccgctacggcgatgtcatgggtgcagaag

SEQ ID NO: 899 - DNA, 120 bp, synthetic construct
  source 1..120: mol_type = other DNA
tcacataccaccctcggggtccaggacatttccgctacggcgatgtcatgggtgcagaagatcacgggaggtgtgggactggttgtcgctgttgcagcactgattctaatcgtggtgcta

SEQ ID NO: 900 - DNA, 120 bp, synthetic construct
  source 1..120: mol_type = other DNA
atcacgggaggtgtgggactggttgtcgctgttgcagcactgattctaatcgtggtgctatgcgtgtcgttcagcaggcactaacttgacgactaagcatgaaggtatatgtgtccccta

SEQ ID NO: 901 - DNA, 120 bp, synthetic construct
  source 1..120: mol_type = other DNA
tgcgtgtcgttcagcaggcactaacttgacgactaagcatgaaggtatatgtgtcccctaagagacacaccgtatatagctaataatctgtagatcaaagggctatataacccctgaata

SEQ ID NO: 902 - DNA, 120 bp, synthetic construct
  source 1..120: mol_type = other DNA
agagacacaccgtatatagctaataatctgtagatcaaagggctatataacccctgaatagtaacaaaatacaaaatcactaaaaattataaaaaacagaaaaatatataaataggtata

SEQ ID NO: 903 - DNA, 120 bp, synthetic construct
  source 1..120: mol_type = other DNA
gtaacaaaatacaaaatcactaaaaattataaaaaacagaaaaatatataaataggtatacgtgtcccctaagagacacattgtatgtaggtgataagtatagatcaaagggccgaacaa

SEQ ID NO: 904 - DNA, 120 bp, synthetic construct
  source 1..120: mol_type = other DNA
cgtgtcccctaagagacacattgtatgtaggtgataagtatagatcaaagggccgaacaacccctgaatagtaacaaaatataaaaattaataaaaatcataaaatagaaaaaccataaa

SEQ ID NO: 905 - DNA, 120 bp, synthetic construct
  source 1..120: mol_type = other DNA
cccctgaatagtaacaaaatataaaaattaataaaaatcataaaatagaaaaaccataaacagaagtagttcaaagggctataaaaacccctgaatagtaacaaaacataaaactaataa

SEQ ID NO: 906 - DNA, 120 bp, synthetic construct
  source 1..120: mol_type = other DNA
cagaagtagttcaaagggctataaaaacccctgaatagtaacaaaacataaaactaataaaaatcaaatgaataccataattggcaaacggaagagatgtaggtacttaagcttcctaaa

SEQ ID NO: 907 - DNA, 120 bp, synthetic construct
  source 1..120: mol_type = other DNA
aaatcaaatgaataccataattggcaaacggaagagatgtaggtacttaagcttcctaaaagcagccgaactcactttgagatgtaggcatagcataccgaactcttccacgattctccg

SEQ ID NO: 908 - DNA, 120 bp, synthetic construct
  source 1..120: mol_type = other DNA
tgaataccataattggcaaacggaagagatgtaggtacttaagcttcctaaaagcagccgaactcactttgagatgtaggcatagcataccgaactcttccacgattctccgaacccaca

SEQ ID NO: 909 - DNA, 120 bp, synthetic construct
  source 1..120: mol_type = other DNA
ttagcgaataaaaatgcgcggatcatttgggcgcttttaacacgccaagaaacgtatcgctgtggcgcctaaacaccgccgtgggtaaaaaaaagaattaacaaaaggagacacaccaac

SEQ ID NO: 910 - DNA, 120 bp, synthetic construct
  source 1..120: mol_type = other DNA
tgtggcgcctaaacaccgccgtgggtaaaaaaaagaattaacaaaaggagacacaccaaccgagttcgaaacaatgagggctgatgaaagtaaggtaaaacctgaggttgattaagctga

SEQ ID NO: 911 - DNA, 120 bp, synthetic construct
  source 1..120: mol_type = other DNA
cgagttcgaaacaatgagggctgatgaaagtaaggtaaaacctgaggttgattaagctgattcatacggtggctctgtgaagtcgatagcccgataagcatcaacctttcataattcatc

SEQ ID NO: 912 - DNA, 120 bp, synthetic construct
  source 1..120: mol_type = other DNA
ttcatacggtggctctgtgaagtcgatagcccgataagcatcaacctttcataattcatcaaggcaccaatggtggccaatttaaattgtgatgccggatatacgaatgcaaccgctttc

SEQ ID NO: 913 - DNA, 120 bp, synthetic construct
  source 1..120: mol_type = other DNA
aaggcaccaatggtggccaatttaaattgtgatgccggatatacgaatgcaaccgctttcttttcatcaaaactgattgttgacaacaagggtgggtctatatacgtatgaagcgaaata

SEQ ID NO: 914 - DNA, 120 bp, synthetic construct
  source 1..120: mol_type = other DNA
ttttcatcaaaactgattgttgacaacaagggtgggtctatatacgtatgaagcgaaatacgggaaaaggcatggcgcatatcattacccacaagtcacagccatttcgtcattcccgcg

SEQ ID NO: 915 - DNA, 120 bp, synthetic construct
  source 1..120: mol_type = other DNA
cgggaaaaggcatggcgcatatcattacccacaagtcacagccatttcgtcattcccgcgcaggcgggaactaggtgcaccttcggtgcgctgcgcacaggtgcgctggatccccgcctg

SEQ ID NO: 916 - DNA, 120 bp, synthetic construct
  source 1..120: mol_type = other DNA
caggcgggaactaggtgcaccttcggtgcgctgcgcacaggtgcgctggatccccgcctgcgcggggatgacgaggggggcgggatggcgaggggtggggaatgacgggttttaagtttt

SEQ ID NO: 917 - DNA, 120 bp, synthetic construct
  source 1..120: mol_type = other DNA
cgcggggatgacgaggggggcgggatggcgaggggtggggaatgacgggttttaagtttttgtcttttaccactgggggagtgatatgggtatgatgtcgtttcccttacaaaaccggtg

SEQ ID NO: 918 - DNA, 120 bp, synthetic construct
  source 1..120: mol_type = other DNA
tgtcttttaccactgggggagtgatatgggtatgatgtcgtttcccttacaaaaccggtggggcttgaaggggaaagaaatttaggatattaatggaagtctgccaataatgcctggagg

SEQ ID NO: 919 - DNA, 120 bp, synthetic construct
  source 1..120: mol_type = other DNA
gggcttgaaggggaaagaaatttaggatattaatggaagtctgccaataatgcctggaggttgcattatgtacaggtatggaaacctcttccaaacaccgatccttcgctcaccactcga

SEQ ID NO: 920 - DNA, 120 bp, synthetic construct
  source 1..120: mol_type = other DNA
ttgcattatgtacaggtatggaaacctcttccaaacaccgatccttcgctcaccactcgaagatcaattctctgactatgtattatggcggttggattgtgagccattcgtagaggtctt

SEQ ID NO: 921 - DNA, 120 bp, synthetic construct
  source 1..120: mol_type = other DNA
agatcaattctctgactatgtattatggcggttggattgtgagccattcgtagaggtcttagaaagaacctgccgtatgaatgatgaaaagctgcgaacccaaaacgtggaagcgaccct

SEQ ID NO: 922 - DNA, 120 bp, synthetic construct
  source 1..120: mol_type = other DNA
agaaagaacctgccgtatgaatgatgaaaagctgcgaacccaaaacgtggaagcgaccctatttgattcggccaagaaaccggaaatttcgtttgcggattatatttggcgaatagtcgc

SEQ ID NO: 923 - DNA, 120 bp, synthetic construct
  source 1..120: mol_type = other DNA
atttgattcggccaagaaaccggaaatttcgtttgcggattatatttggcgaatagtcgcctatgcgagactgacccattcccaaatgatccatacgttaatttacctcgataggtgtca

SEQ ID NO: 924 - DNA, 120 bp, synthetic construct
  source 1..120: mol_type = other DNA
ctatgcgagactgacccattcccaaatgatccatacgttaatttacctcgataggtgtcaagaaaatttttttttaacttctttaaatttttatcgcttattcctagtcgctgctttagt

SEQ ID NO: 925 - DNA, 120 bp, synthetic construct
  source 1..120: mol_type = other DNA
agaaaatttttttttaacttctttaaatttttatcgcttattcctagtcgctgctttagtggcacaaaaatttcatcaagatgattctttttccaacaaaagttttgctgatttagtagg

SEQ ID NO: 926 - DNA, 120 bp, synthetic construct
  source 1..120: mol_type = other DNA
ggcacaaaaatttcatcaagatgattctttttccaacaaaagttttgctgatttagtaggaattacggtcaaagagttaaatatacttgaagcaaaattcttatttgctattagttttag

SEQ ID NO: 927 - DNA, 120 bp, synthetic construct
  source 1..120: mol_type = other DNA
aattacggtcaaagagttaaatatacttgaagcaaaattcttatttgctattagttttagtctttatgttttaccaaaaacctataaagaatataatcgaattgtgggtggacaaagaat

SEQ ID NO: 928 - DNA, 120 bp, synthetic construct
  source 1..120: mol_type = other DNA
tctttatgttttaccaaaaacctataaagaatataatcgaattgtgggtggacaaagaattaaccgccaattagtggaggcaaggcgatcgaatctatcgtttttttctcttttccctca

SEQ ID NO: 929 - DNA, 120 bp, synthetic construct
  source 1..120: mol_type = other DNA
taaccgccaattagtggaggcaaggcgatcgaatctatcgtttttttctcttttccctcatacagttaatacctttcctcacaggaagagaaattcttatcactttttacatcgccctcg

SEQ ID NO: 930 - DNA, 120 bp, synthetic construct
  source 1..120: mol_type = other DNA
tacagttaatacctttcctcacaggaagagaaattcttatcactttttacatcgccctcgattctaatattgctttttacaaaaagtctctttaataccgaattttccgataaataaggc

SEQ ID NO: 931 - DNA, 120 bp, synthetic construct
  source 1..120: mol_type = other DNA
attctaatattgctttttacaaaaagtctctttaataccgaattttccgataaataaggctaataaaaatagcaagggaatcatcgtaagcgcaacttgataagcataggtactatagat

SEQ ID NO: 932 - DNA, 120 bp, synthetic construct
  source 1..120: mol_type = other DNA
taataaaaatagcaagggaatcatcgtaagcgcaacttgataagcataggtactatagataggagcatttcccaacattcgaccgtcccagaatttatccaacaataaacctacaatcgg

SEQ ID NO: 933 - DNA, 120 bp, synthetic construct
  source 1..120: mol_type = other DNA
aggagcatttcccaacattcgaccgtcccagaatttatccaacaataaacctacaatcggttgtaaaataacaccggcgaaaataatacccatattggttaagcctgacgcagtccccac

SEQ ID NO: 934 - DNA, 120 bp, synthetic construct
  source 1..120: mol_type = other DNA
ttgtaaaataacaccggcgaaaataatacccatattggttaagcctgacgcagtccccacggcttgagcatgattattatcgatgaccaggccgaaagagatgaccatggcagaacaggc

SEQ ID NO: 935 - DNA, 120 bp, synthetic construct
  source 1..120: mol_type = other DNA
ggcttgagcatgattattatcgatgaccaggccgaaagagatgaccatggcagaacaggccgcgccgaagaggaagagacaaacggctaacagcatttgaggcaaagcgggaacatacaa

SEQ ID NO: 936 - DNA, 120 bp, synthetic construct
  source 1..120: mol_type = other DNA
cgcgccgaagaggaagagacaaacggctaacagcatttgaggcaaagcgggaacatacaaaattaaagaggcgacaacaaatcctaaaagagcagccgtaaccatgggtagccggcgtcg

SEQ ID NO: 937 - DNA, 120 bp, synthetic construct
  source 1..120: mol_type = other DNA
aattaaagaggcgacaacaaatcctaaaagagcagccgtaaccatgggtagccggcgtcgttgaatagcattcgtccaccaaccgaaaaaaggcccgccgacggcgatgccaagccagat

SEQ ID NO: 938 - DNA, 120 bp, synthetic construct
  source 1..120: mol_type = other DNA
ttgaatagcattcgtccaccaaccgaaaaaaggcccgccgacggcgatgccaagccagattagagagagcaaagccgtggtgtgaacattcgtaaattgatgggaacttacgagaaataa

SEQ ID NO: 939 - DNA, 120 bp, synthetic construct
  source 1..120: mol_type = other DNA
tagagagagcaaagccgtggtgtgaacattcgtaaattgatgggaacttacgagaaataaagcgccccatgaagtagcgaacaatgccgtcggcccccaaatggcaaaaccgaacaatgc

SEQ ID NO: 940 - DNA, 120 bp, synthetic construct
  source 1..120: mol_type = other DNA
agcgccccatgaagtagcgaacaatgccgtcggcccccaaatggcaaaaccgaacaatgcaatccaccatgattgcgtccgtttaaagacatcgcgtaaataaagacggttttcttgtgc

SEQ ID NO: 941 - DNA, 120 bp, synthetic construct
  source 1..120: mol_type = other DNA
aatccaccatgattgcgtccgtttaaagacatcgcgtaaataaagacggttttcttgtgccagcaatttagcggcggctttggttaggtgggattccttaggtttatcccgaataactat

SEQ ID NO: 942 - DNA, 120 bp, synthetic construct
  source 1..120: mol_type = other DNA
cagcaatttagcggcggctttggttaggtgggattccttaggtttatcccgaataactatccagttaaggatggtaagtaaaaatcccaatgccgcaataaagtaagtcgttcgttgcca

SEQ ID NO: 943 - DNA, 120 bp, synthetic construct
  source 1..120: mol_type = other DNA
ccagttaaggatggtaagtaaaaatcccaatgccgcaataaagtaagtcgttcgttgccaaccatacaggtttgcaaaatgcgccacgggcgctgagccgataacagcgccagcgcaccc

SEQ ID NO: 944 - DNA, 120 bp, synthetic construct
  source 1..120: mol_type = other DNA
accatacaggtttgcaaaatgcgccacgggcgctgagccgataacagcgccagcgcacccaagcacttgcaccagtcccgcatacatggcaaaccgcttagcacccaaccaataagcgcc

SEQ ID NO: 945 - DNA, 120 bp, synthetic construct
  source 1..120: mol_type = other DNA
aagcacttgcaccagtcccgcatacatggcaaaccgcttagcacccaaccaataagcgccgacccataaagcgccgagataagcgatggaagcggtaaatcccataataaaacgagcaat

SEQ ID NO: 946 - DNA, 120 bp, synthetic construct
  source 1..120: mol_type = other DNA
gacccataaagcgccgagataagcgatggaagcggtaaatcccataataaaacgagcaatgacagcgagaggaaaataagtagtggacgcaaagataagcgttgctatcgagcaaactag

SEQ ID NO: 947 - DNA, 120 bp, synthetic construct
  source 1..120: mol_type = other DNA
gacagcgagaggaaaataagtagtggacgcaaagataagcgttgctatcgagcaaactagaagccctaaagaaagcaaacgacgcgcgccgaatttatcgcacaacatgcccgatggaat

SEQ ID NO: 948 - DNA, 120 bp, synthetic construct
  source 1..120: mol_type = other DNA
aagccctaaagaaagcaaacgacgcgcgccgaatttatcgcacaacatgcccgatggaatttgcatcaaggcgtagccgtaaaaaaaaccgctaaataaaatactgagttcacccgcttg

SEQ ID NO: 949 - DNA, 120 bp, synthetic construct
  source 1..120: mol_type = other DNA
ttgcatcaaggcgtagccgtaaaaaaaaccgctaaataaaatactgagttcacccgcttgaattttgaacgcgtctaataactcatgcgcaatagccatcggcatgacgcggactaaaaa

SEQ ID NO: 950 - DNA, 120 bp, synthetic construct
  source 1..120: mol_type = other DNA
aattttgaacgcgtctaataactcatgcgcaatagccatcggcatgacgcggactaaaaaatcgtacgcgtaaaaggaagaagcgacgatgcctacaattaatggtgtcagccaaagatg

SEQ ID NO: 951 - DNA, 120 bp, synthetic construct
  source 1..120: mol_type = other DNA
atcgtacgcgtaaaaggaagaagcgacgatgcctacaattaatggtgtcagccaaagatgaagtttggtatttttcttactgatcagcataattatcctctgtgcgaaatttatggccct

SEQ ID NO: 952 - DNA, 120 bp, synthetic construct
  source 1..120: mol_type = other DNA
aagtttggtatttttcttactgatcagcataattatcctctgtgcgaaatttatggccctttgtactccctctccaatgatgccataataaatcagattatgaggggaaggagtccctaa

SEQ ID NO: 953 - DNA, 120 bp, synthetic construct
  source 1..120: mol_type = other DNA
ttgtactccctctccaatgatgccataataaatcagattatgaggggaaggagtccctaatgtattgtcgtaagcgaatattcatccgctgtttttacattttaatgcttacctttggtc

SEQ ID NO: 954 - DNA, 120 bp, synthetic construct
  source 1..120: mol_type = other DNA
tgtattgtcgtaagcgaatattcatccgctgtttttacattttaatgcttacctttggtctgcttggaatagcatcccacattattgctcaaaataatacccgtagattagccattttaa

SEQ ID NO: 955 - DNA, 120 bp, synthetic construct
  source 1..120: mol_type = other DNA
tgcttggaatagcatcccacattattgctcaaaataatacccgtagattagccattttaatcgacataaaaggcggtattggtccagccaccgccgatttttttcatcgcagtctaaagc

SEQ ID NO: 956 - DNA, 120 bp, synthetic construct
  source 1..120: mol_type = other DNA
tcgacataaaaggcggtattggtccagccaccgccgatttttttcatcgcagtctaaagcaagccactgaaaaaaaagcacaagttattattttacaacttgacacgcctggcggtttag

SEQ ID NO: 957 - DNA, 120 bp, synthetic construct
  source 1..120: mol_type = other DNA
aagccactgaaaaaaaagcacaagttattattttacaacttgacacgcctggcggtttagtgactgccatgcgcgatattattaaagatatcctcgcctcgcccatcccagtcatcggct

SEQ ID NO: 958 - DNA, 120 bp, synthetic construct
  source 1..120: mol_type = other DNA
tgactgccatgcgcgatattattaaagatatcctcgcctcgcccatcccagtcatcggctacgtagcgccgagcggtgcccatgcggcgagtgcgggcacttatattttatacgccactc

SEQ ID NO: 959 - DNA, 120 bp, synthetic construct
  source 1..120: mol_type = other DNA
acgtagcgccgagcggtgcccatgcggcgagtgcgggcacttatattttatacgccactcatatcgccgccatggcccctggaaccaatttaggggctgcgacgccgatcgctattggca

SEQ ID NO: 960 - DNA, 120 bp, synthetic construct
  source 1..120: mol_type = other DNA
atatcgccgccatggcccctggaaccaatttaggggctgcgacgccgatcgctattggcacacccggcggcagttctcctgaaaagggtaacgaaaaaaaagaaggagctaaaaaagcac

SEQ ID NO: 961 - DNA, 120 bp, synthetic construct
  source 1..120: mol_type = other DNA
cacccggcggcagttctcctgaaaagggtaacgaaaaaaaagaaggagctaaaaaagcaccggcgcaaaaaaccgcggctgaaaaaaaagccattagcgatgcgagagcctatattcgca

SEQ ID NO: 962 - DNA, 120 bp, synthetic construct
  source 1..120: mol_type = other DNA
cggcgcaaaaaaccgcggctgaaaaaaaagccattagcgatgcgagagcctatattcgcagtttagcgcaactgcgcggtcgaaacgtggaatgggcagaaagtgcggtcgttgaagcag

SEQ ID NO: 963 - DNA, 120 bp, synthetic construct
  source 1..120: mol_type = other DNA
gtttagcgcaactgcgcggtcgaaacgtggaatgggcagaaagtgcggtcgttgaagcagaaagcctttccgccgaagaagcatataaaattaaagtaattaatatcattgcgtcgaata

SEQ ID NO: 964 - DNA, 120 bp, synthetic construct
  source 1..120: mol_type = other DNA
aaagcctttccgccgaagaagcatataaaattaaagtaattaatatcattgcgtcgaatatccctaatttactagaacaagcgaatggcataaaaattagcgtgcgcggcgaaacgcaaa

SEQ ID NO: 965 - DNA, 120 bp, synthetic construct
  source 1..120: mol_type = other DNA
tccctaatttactagaacaagcgaatggcataaaaattagcgtgcgcggcgaaacgcaaaccgtaaacaccgccaatctggaaatagaaaaagtagaacccgattggcgaacgcgctttt

SEQ ID NO: 966 - DNA, 120 bp, synthetic construct
  source 1..120: mol_type = other DNA
ccgtaaacaccgccaatctggaaatagaaaaagtagaacccgattggcgaacgcgctttttaagcgtgattacggactccagcgttgcctatattttattgatgatcggtttttatggga

SEQ ID NO: 967 - DNA, 120 bp, synthetic construct
  source 1..120: mol_type = other DNA
taagcgtgattacggactccagcgttgcctatattttattgatgatcggtttttatgggatattttttgaatttattaatcccggttttattgttccgggggtggtgggcgctatttcct

SEQ ID NO: 968 - DNA, 120 bp, synthetic construct
  source 1..120: mol_type = other DNA
tattttttgaatttattaatcccggttttattgttccgggggtggtgggcgctatttccttattgttagcgctttacgcgtttcaattgctgccaatcaattacgcgggtttagcgttga

SEQ ID NO: 969 - DNA, 120 bp, synthetic construct
  source 1..120: mol_type = other DNA
tattgttagcgctttacgcgtttcaattgctgccaatcaattacgcgggtttagcgttgattttattgggattggctttcattgttgcggaagctttcatgccgagttttggcatgttgg

SEQ ID NO: 970 - DNA, 120 bp, synthetic construct
  source 1..120: mol_type = other DNA
ttttattgggattggctttcattgttgcggaagctttcatgccgagttttggcatgttgggtattggcggcggtgttgcatttgttatcggttctattatgctaatgagaacagatgcaa

SEQ ID NO: 971 - DNA, 120 bp, synthetic construct
  source 1..120: mol_type = other DNA
gtattggcggcggtgttgcatttgttatcggttctattatgctaatgagaacagatgcaattggctttggaattcccatgtatttaatcatcgctatcgctattgtcaccatagccttct

SEQ ID NO: 972 - DNA, 120 bp, synthetic construct
  source 1..120: mol_type = other DNA
ttggctttggaattcccatgtatttaatcatcgctatcgctattgtcaccatagccttctttttactcgttttaagtatcgcgtttcgttcgcgggggcgcccgattgtgagtggtcgag

SEQ ID NO: 973 - DNA, 120 bp, synthetic construct
  source 1..120: mol_type = other DNA
ttttactcgttttaagtatcgcgtttcgttcgcgggggcgcccgattgtgagtggtcgagaagcggtgattggaaagcgcggcgttgtcaatgtcagcgataaacgcatgtgggtgcgta

SEQ ID NO: 974 - DNA, 120 bp, synthetic construct
  source 1..120: mol_type = other DNA
aagcggtgattggaaagcgcggcgttgtcaatgtcagcgataaacgcatgtgggtgcgtatcgaaggcgagcgttggcaatgtaaaagtgatgttccccttcaagatggcgatgaagtcg

SEQ ID NO: 975 - DNA, 120 bp, synthetic construct
  source 1..120: mol_type = other DNA
tcgaaggcgagcgttggcaatgtaaaagtgatgttccccttcaagatggcgatgaagtcgtcgttgaacgactcgaaggattattttgtgtggtcaaaccagtggagaaaaaataatgat

SEQ ID NO: 976 - DNA, 120 bp, synthetic construct
  source 1..120: mol_type = other DNA
tcgttgaacgactcgaaggattattttgtgtggtcaaaccagtggagaaaaaataatgatgattgttctgattgtaatagcggtattggttttactgttattgttttccgctatccatat

SEQ ID NO: 977 - DNA, 120 bp, synthetic construct
  source 1..120: mol_type = other DNA
gattgttctgattgtaatagcggtattggttttactgttattgttttccgctatccatattctgaaagagtacgagcgcggcgttattttcactttaggtcgtttttggaaagtgaaggg

SEQ ID NO: 978 - DNA, 120 bp, synthetic construct
  source 1..120: mol_type = other DNA
tctgaaagagtacgagcgcggcgttattttcactttaggtcgtttttggaaagtgaagggtccaggcttaatcatcgtcgtgccgattattcaacaaattgttcgcacgcatttgcgaac

SEQ ID NO: 979 - DNA, 120 bp, synthetic construct
  source 1..120: mol_type = other DNA
tccaggcttaatcatcgtcgtgccgattattcaacaaattgttcgcacgcatttgcgaacagttgtgatggatgtgcctagccaggatgttatttcccgcgataatgtttccgtgcgagt

SEQ ID NO: 980 - DNA, 120 bp, synthetic construct
  source 1..120: mol_type = other DNA
agttgtgatggatgtgcctagccaggatgttatttcccgcgataatgtttccgtgcgagtgaacgcggttgtttattttcgggtgattgatcccgagcgcgcgattattcaggttgagga

SEQ ID NO: 981 - DNA, 120 bp, synthetic construct
  source 1..120: mol_type = other DNA
gaacgcggttgtttattttcgggtgattgatcccgagcgcgcgattattcaggttgaggattattacgaagcgacgagtcaattggcgcaaaccacactgcgttccgtattgggccaaca

SEQ ID NO: 982 - DNA, 120 bp, synthetic construct
  source 1..120: mol_type = other DNA
ttattacgaagcgacgagtcaattggcgcaaaccacactgcgttccgtattgggccaacacgaactcgatgaaatgctggccgaacgagagaagttaaacaaagatattcaagaaatttt

SEQ ID NO: 983 - DNA, 120 bp, synthetic construct
  source 1..120: mol_type = other DNA
cgaactcgatgaaatgctggccgaacgagagaagttaaacaaagatattcaagaaattttagatgcggaaacagacgcgtggggtattaaagtcgccaacgtcgaaattaaacatgtcga

SEQ ID NO: 984 - DNA, 120 bp, synthetic construct
  source 1..120: mol_type = other DNA
agatgcggaaacagacgcgtggggtattaaagtcgccaacgtcgaaattaaacatgtcgatttggaagaaagcatggttcgcgccatcgcccgccaagccgaggctgaacgggaacgacg

SEQ ID NO: 985 - DNA, 120 bp, synthetic construct
  source 1..120: mol_type = other DNA
tttggaagaaagcatggttcgcgccatcgcccgccaagccgaggctgaacgggaacgacgggcaaaagtgattaacgcagaaggcgaatttcaagccgcccaacgcttaaaagaagccgc

SEQ ID NO: 986 - DNA, 120 bp, synthetic construct
  source 1..120: mol_type = other DNA
ggcaaaagtgattaacgcagaaggcgaatttcaagccgcccaacgcttaaaagaagccgctgaaattctggcaaaacagccgcaatcgttacaattgcgttatatgcaaacgttaatgga

SEQ ID NO: 987 - DNA, 120 bp, synthetic construct
  source 1..120: mol_type = other DNA
tgaaattctggcaaaacagccgcaatcgttacaattgcgttatatgcaaacgttaatggatttagccagcgataaaacttcaaccattgtcttccccatgccaatcgatattttaaaaat

SEQ ID NO: 988 - DNA, 120 bp, synthetic construct
  source 1..120: mol_type = other DNA
tttagccagcgataaaacttcaaccattgtcttccccatgccaatcgatattttaaaaattttcgaaaagaaagtaagtgattaattatgtagcccaatgaaatggacccaccccttaaa

SEQ ID NO: 989 - DNA, 120 bp, synthetic construct
  source 1..120: mol_type = other DNA
tttcgaaaagaaagtaagtgattaattatgtagcccaatgaaatggacccaccccttaaagacggcgtcataatgcgccaacatagaatttctattttcaaaaaaaggagaaggtccatg

SEQ ID NO: 990 - DNA, 120 bp, synthetic construct
  source 1..120: mol_type = other DNA
gacggcgtcataatgcgccaacatagaatttctattttcaaaaaaaggagaaggtccatgaaagatattaaaatactgggtgttgatattgcaaaagatgtttttcaactgtgtggaatt

SEQ ID NO: 991 - DNA, 120 bp, synthetic construct
  source 1..120: mol_type = other DNA
aaagatattaaaatactgggtgttgatattgcaaaagatgtttttcaactgtgtggaattgatgagtggggtaaagtgatctacacgagacgggttaagcgtgctcagtatgtatccacc

SEQ ID NO: 992 - DNA, 120 bp, synthetic construct
  source 1..120: mol_type = other DNA
gatgagtggggtaaagtgatctacacgagacgggttaagcgtgctcagtatgtatccaccgtagccagtcttaaggtgggctgcgtggtgatggaagcgtgtggaggagcgaaccattgg

SEQ ID NO: 993 - DNA, 120 bp, synthetic construct
  source 1..120: mol_type = other DNA
gtagccagtcttaaggtgggctgcgtggtgatggaagcgtgtggaggagcgaaccattggtatcggacgtttatggggatgggtatcccaacgcagttgatcagtccgcagcacgtcaaa

SEQ ID NO: 994 - DNA, 120 bp, synthetic construct
  source 1..120: mol_type = other DNA
tatcggacgtttatggggatgggtatcccaacgcagttgatcagtccgcagcacgtcaaaccgtatgtcaaaagtaacaagaatgatcgtaacgatgcgcaggcgatagctgaagcggct

SEQ ID NO: 995 - DNA, 120 bp, synthetic construct
  source 1..120: mol_type = other DNA
ccgtatgtcaaaagtaacaagaatgatcgtaacgatgcgcaggcgatagctgaagcggcttcccgcgcctcgatgcggtttgtgcggggtaaaacggtggaacaacaagacgttcaagcg

SEQ ID NO: 996 - DNA, 120 bp, synthetic construct
  source 1..120: mol_type = other DNA
tcccgcgcctcgatgcggtttgtgcggggtaaaacggtggaacaacaagacgttcaagcgctgttaaagatacgcgatcgtttagtcaaaagccgcacggcgctgatcaatgagattcgg

SEQ ID NO: 997 - DNA, 120 bp, synthetic construct
  source 1..120: mol_type = other DNA
ctgttaaagatacgcgatcgtttagtcaaaagccgcacggcgctgatcaatgagattcgggggttgttgcaagaatacggactcacgatggcgcgtggtgccaagcgattttatgaagag

SEQ ID NO: 998 - DNA, 120 bp, synthetic construct
  source 1..120: mol_type = other DNA
gggttgttgcaagaatacggactcacgatggcgcgtggtgccaagcgattttatgaagagctcccgttgattttagcgagcgaagcggtgggattaacaccgcggatgaaacgggtgttg

SEQ ID NO: 999 - DNA, 120 bp, synthetic construct
  source 1..120: mol_type = other DNA
ctcccgttgattttagcgagcgaagcggtgggattaacaccgcggatgaaacgggtgttgaattgtttgtataccgaattgttgaaccgggacgaagcgattggtgattacgaggaggaa

SEQ ID NO: 1000 - DNA, 120 bp, synthetic construct
  source 1..120: mol_type = other DNA
aattgtttgtataccgaattgttgaaccgggacgaagcgattggtgattacgaggaggaattaaaagcggtggcaaaagccaatgaggattgtcaacgggtacagagcatcccgggggtg

SEQ ID NO: 1001 - DNA, 120 bp, synthetic construct
  source 1..120: mol_type = other DNA
ttaaaagcggtggcaaaagccaatgaggattgtcaacgggtacagagcatcccgggggtgggttatttaacggcgctctcggtttatgcgagcgtgggtgacattcatcaatttcatcgt

SEQ ID NO: 1002 - DNA, 120 bp, synthetic construct
  source 1..120: mol_type = other DNA
ggttatttaacggcgctctcggtttatgcgagcgtgggtgacattcatcaatttcatcgttcccggcagttgtcggcgtttattgggttggtccctcgacaacattcgagtgggaataag

SEQ ID NO: 1003 - DNA, 120 bp, synthetic construct
  source 1..120: mol_type = other DNA
tcccggcagttgtcggcgtttattgggttggtccctcgacaacattcgagtgggaataaggaggtgttgttggggattagtaaacgcggcaatgtgatgttaaggacgttattgattcat

SEQ ID NO: 1004 - DNA, 120 bp, synthetic construct
  source 1..120: mol_type = other DNA
gaggtgttgttggggattagtaaacgcggcaatgtgatgttaaggacgttattgattcatggcgcccgtgcgctattgcgtcatgtaaaaaataaaacggataaaaagagtctgtggtta

SEQ ID NO: 1005 - DNA, 120 bp, synthetic construct
  source 1..120: mol_type = other DNA
ggcgcccgtgcgctattgcgtcatgtaaaaaataaaacggataaaaagagtctgtggttaaaagcactcattgagcgccgcggaatgaatcgcgcttgtgtggcgttagcgaataaaaat

SEQ ID NO: 1006 - DNA, 120 bp, synthetic construct
  source 1..120: mol_type = other DNA
aaagcactcattgagcgccgcggaatgaatcgcgcttgtgtggcgttagcgaataaaaatgcgccgatcatttgggcgcttttaacacgccaagaaacgtatcgctgtggcgcctaaaca

SEQ ID NO: 1007 - DNA, 120 bp, synthetic construct
  source 1..120: mol_type = other DNA
gcgccgatcatttgggcgcttttaacacgccaagaaacgtatcgctgtggcgcctaaacaccgccgtgggtaaaaaaaagaattaacaaaaggagacacaccaaccgagttcgaaacaat

SEQ ID NO: 1008 - DNA, 120 bp, synthetic construct
  source 1..120: mol_type = other DNA
ccgccgtgggtaaaaaaaagaattaacaaaaggagacacaccaaccgagttcgaaacaatgagggctgatgaaagtaaggtaaaacctgaggttgattaagctgattcatacggtggctc

SEQ ID NO: 1009 - DNA, 120 bp, synthetic construct
  source 1..120: mol_type = other DNA
gagggctgatgaaagtaaggtaaaacctgaggttgattaagctgattcatacggtggctctgtgaagccgatagcccgataagcatcaaccttgcataattcatcaaggcaccaatggtg

SEQ ID NO: 1010 - DNA, 120 bp, synthetic construct
  source 1..120: mol_type = other DNA
tgtgaagccgatagcccgataagcatcaaccttgcataattcatcaaggcaccaatggtggccaatttaaattgtgatgccggatatacgaatgcaaccgctttcttttcatcaaaactg

SEQ ID NO: 1011 - DNA, 120 bp, synthetic construct
  source 1..120: mol_type = other DNA
gccaatttaaattgtgatgccggatatacgaatgcaaccgctttcttttcatcaaaactgattgttgacaacaagggtgggtccatatacgtatgacgcgaacggaaggcagaagacaga

SEQ ID NO: 1012 - DNA, 120 bp, synthetic construct
  source 1..120: mol_type = other DNA
attgttgacaacaagggtgggtccatatacgtatgacgcgaacggaaggcagaagacagagggcagaagacagaggacagaaggcagaagacagtggttgtgtcgctacgcaacaactaa

SEQ ID NO: 1013 - DNA, 120 bp, synthetic construct
  source 1..120: mol_type = other DNA
gggcagaagacagaggacagaaggcagaagacagtggttgtgtcgctacgcaacaactaaattttataaattaattgtggcgaagccacacgaacactgtcctctgtcctctgcctaggg

SEQ ID NO: 1014 - DNA, 120 bp, synthetic construct
  source 1..120: mol_type = other DNA
attttataaattaattgtggcgaagccacacgaacactgtcctctgtcctctgcctagggaatcacggtatttactcatttatttttcctttttactctttctcgatgagtcattcacct

SEQ ID NO: 1015 - DNA, 120 bp, synthetic construct
  source 1..120: mol_type = other DNA
aatcacggtatttactcatttatttttcctttttactctttctcgatgagtcattcaccttcttacgggtttacattgcttgaggtattaattgcctggtctattttatccggtatttta

SEQ ID NO: 1016 - DNA, 120 bp, synthetic construct
  source 1..120: mol_type = other DNA
tcttacgggtttacattgcttgaggtattaattgcctggtctattttatccggtattttattaagtgttttgtttttacaaatcgatgaggttcgccatattcgtcatgcttattattac

SEQ ID NO: 1017 - DNA, 120 bp, synthetic construct
  source 1..120: mol_type = other DNA
ttaagtgttttgtttttacaaatcgatgaggttcgccatattcgtcatgcttattattacagcgtagctacggttcaattacgatctttaatagaacgactgcgcgcgaatcaaacttcc

SEQ ID NO: 1018 - DNA, 120 bp, synthetic construct
  source 1..120: mol_type = other DNA
agcgtagctacggttcaattacgatctttaatagaacgactgcgcgcgaatcaaacttccgttgcgcgtgaacgggaatggagggattggaataatgagaataagggggtgttgccgcaa

SEQ ID NO: 1019 - DNA, 120 bp, synthetic construct
  source 1..120: mol_type = other DNA
gttgcgcgtgaacgggaatggagggattggaataatgagaataagggggtgttgccgcaaggagaagggaattatcgctgtgaacgacgtatttgccacgtgaccgttcattagcgggag

SEQ ID NO: 1020 - DNA, 120 bp, synthetic construct
  source 1..120: mol_type = other DNA
ggagaagggaattatcgctgtgaacgacgtatttgccacgtgaccgttcattagcgggagagaaaaatacaaactttatctttggttgcagcggtatgaaattgcaaacagggttcagtc

SEQ ID NO: 1021 - DNA, 120 bp, synthetic construct
  source 1..120: mol_type = other DNA
agaaaaatacaaactttatctttggttgcagcggtatgaaattgcaaacagggttcagtctaattgaattattggtgtctctgtttttaggctctttattaatgattatgcttgtgaaac

SEQ ID NO: 1022 - DNA, 120 bp, synthetic construct
  source 1..120: mol_type = other DNA
taattgaattattggtgtctctgtttttaggctctttattaatgattatgcttgtgaaactctatttcagctttcgtgaaaccgcacaatggcaggataccctagcagccattcaagaac

SEQ ID NO: 1023 - DNA, 120 bp, synthetic construct
  source 1..120: mol_type = other DNA
tctatttcagctttcgtgaaaccgcacaatggcaggataccctagcagccattcaagaacgcgaacggtttggtgcgtatttcttagcgcaacgcattcgacaagcgggcgattcgactt

SEQ ID NO: 1024 - DNA, 120 bp, synthetic construct
  source 1..120: mol_type = other DNA
gcgaacggtttggtgcgtatttcttagcgcaacgcattcgacaagcgggcgattcgacttgtgaacctggtgaaacggtggatcaatcaaatgccgttatagggtacgattcagatcatt

SEQ ID NO: 1025 - DNA, 120 bp, synthetic construct
  source 1..120: mol_type = other DNA
gtgaacctggtgaaacggtggatcaatcaaatgccgttatagggtacgattcagatcatttgccgcccgatttacgcaaagaaagcattcctaattctgacgtcatcgttattggcgaat

SEQ ID NO: 1026 - DNA, 120 bp, synthetic construct
  source 1..120: mol_type = other DNA
tgccgcccgatttacgcaaagaaagcattcctaattctgacgtcatcgttattggcgaatgcttgcgttatcacaataagttacaatttataaaaaccgcttattttatcagcgatacgc

SEQ ID NO: 1027 - DNA, 120 bp, synthetic construct
  source 1..120: mol_type = other DNA
gcttgcgttatcacaataagttacaatttataaaaaccgcttattttatcagcgatacgcatcgcaaagaaaaggggaaaccagtttttttgtatgaaaaaccaatggatggggcgcggc

SEQ ID NO: 1028 - DNA, 120 bp, synthetic construct
  source 1..120: mol_type = other DNA
atcgcaaagaaaaggggaaaccagtttttttgtatgaaaaaccaatggatggggcgcggcaggaactaattgccgacgttaataaattaaccattcactatggggtttcctcttctgacc

SEQ ID NO: 1029 - DNA, 120 bp, synthetic construct
  source 1..120: mol_type = other DNA
aggaactaattgccgacgttaataaattaaccattcactatggggtttcctcttctgaccgtcaatccattcgttattaccacactgccgccgcaattaaaaactgggaagctatcaaaa

SEQ ID NO: 1030 - DNA, 120 bp, synthetic construct
  source 1..120: mol_type = other DNA
gtcaatccattcgttattaccacactgccgccgcaattaaaaactgggaagctatcaaaagcgtcaatctaacgctttttttcattctaatttaatgcttcttaaaaaatggcatctgta

SEQ ID NO: 1031 - DNA, 120 bp, synthetic construct
  source 1..120: mol_type = other DNA
gcgtcaatctaacgctttttttcattctaatttaatgcttcttaaaaaatggcatctgtatgtgactttgcgagaaagattttgaaatcccaacaggcagagcaaggaatgatactggtc

SEQ ID NO: 1032 - DNA, 120 bp, synthetic construct
  source 1..120: mol_type = other DNA
tgtgactttgcgagaaagattttgaaatcccaacaggcagagcaaggaatgatactggtcagcgtacttttattcctatttgcgctgagtttattaatgacagcgcatcttgaacttcac

SEQ ID NO: 1033 - DNA, 120 bp, synthetic construct
  source 1..120: mol_type = other DNA
agcgtacttttattcctatttgcgctgagtttattaatgacagcgcatcttgaacttcacttgctcgaaactaaaatgagtgaaaataattatcatcgaattgtcacctttgaagcagct

SEQ ID NO: 1034 - DNA, 120 bp, synthetic construct
  source 1..120: mol_type = other DNA
ttgctcgaaactaaaatgagtgaaaataattatcatcgaattgtcacctttgaagcagctgaagcaggtttgatggcggctgaagcttcaatacaaggaaaatcattttcactaccgtct

SEQ ID NO: 1035 - DNA, 120 bp, synthetic construct
  source 1..120: mol_type = other DNA
gaagcaggtttgatggcggctgaagcttcaatacaaggaaaatcattttcactaccgtcttcgggggcgacagtgaattatcatattcagttaatgggcacggacgcttgtgataaaaaa

SEQ ID NO: 1036 - DNA, 120 bp, synthetic construct
  source 1..120: mol_type = other DNA
tcgggggcgacagtgaattatcatattcagttaatgggcacggacgcttgtgataaaaaacggtatcgcattacggctgatgccctttttcatcgaagcaaagtggctttgctcagtgag

SEQ ID NO: 1037 - DNA, 120 bp, synthetic construct
  source 1..120: mol_type = other DNA
cggtatcgcattacggctgatgccctttttcatcgaagcaaagtggctttgctcagtgagtatgaatacttattgtcaacgacaaaaccagcctgtaaaaaagaagtaattaatcgtcgc

SEQ ID NO: 1038 - DNA, 120 bp, synthetic construct
  source 1..120: mol_type = other DNA
tatgaatacttattgtcaacgacaaaaccagcctgtaaaaaagaagtaattaatcgtcgcacgtattggaaaagactttaaaaagggttgagcctgtcggctcaacctgctatgttttat

SEQ ID NO: 1039 - DNA, 120 bp, synthetic construct
  source 1..120: mol_type = other DNA
acgtattggaaaagactttaaaaagggttgagcctgtcggctcaacctgctatgttttattctcaataatcgaaacctgcgccagcccatttaatactgccgcgatacgaatgacatgtt

SEQ ID NO: 1040 - DNA, 120 bp, synthetic construct
  source 1..120: mol_type = other DNA
tctcaataatcgaaacctgcgccagcccatttaatactgccgcgatacgaatgacatgttgaatggaatgtttgctgaaaccagctttaattaatgtattagcatgggcatcaatacaca

SEQ ID NO: 1041 - DNA, 120 bp, synthetic construct
  source 1..120: mol_type = other DNA
gaatggaatgtttgctgaaaccagctttaattaatgtattagcatgggcatcaatacacaagccgcaaccattgatggcagaaacggctaaggaataaagttcaaaatcttttttatcga

SEQ ID NO: 1042 - DNA, 120 bp, synthetic construct
  source 1..120: mol_type = other DNA
agccgcaaccattgatggcagaaacggctaaggaataaagttcaaaatcttttttatcgatgccaggatttgcgattatattcatgcgcaaattagcgggtaggcgttggtattcactgt

SEQ ID NO: 1043 - DNA, 120 bp, synthetic construct
  source 1..120: mol_type = other DNA
tgccaggatttgcgattatattcatgcgcaaattagcgggtaggcgttggtattcactgtcttttaccaaatgcacgaagcgataataaatattattcatcgccataatgctggccgccg

SEQ ID NO: 1044 - DNA, 120 bp, synthetic construct
  source 1..120: mol_type = other DNA
cttttaccaaatgcacgaagcgataataaatattattcatcgccataatgctggccgccgctttaatggcctgtaaggtcgattcatcaagctcagcttcggctttttgaaaaatgagct

SEQ ID NO: 1045 - DNA, 120 bp, synthetic construct
  source 1..120: mol_type = other DNA
ctttaatggcctgtaaggtcgattcatcaagctcagcttcggctttttgaaaaatgagctcgattaactgacgatttcgtgtagcataagcaacggctaatgcaacacctgtgatttgtt

SEQ ID NO: 1046 - DNA, 120 bp, synthetic construct
  source 1..120: mol_type = other DNA
cgattaactgacgatttcgtgtagcataagcaacggctaatgcaacacctgtgatttgttgatttgatagttcgctcgaaggcgactcacttaatacttgcgttagatttaattttaaat

SEQ ID NO: 1047 - DNA, 120 bp, synthetic construct
  source 1..120: mol_type = other DNA
gatttgatagttcgctcgaaggcgactcacttaatacttgcgttagatttaattttaaatcttttgcataatcgggtaattgatctttgtaagtttgtaacatgtttattctcctcacgt

SEQ ID NO: 1048 - DNA, 120 bp, synthetic construct
  source 1..120: mol_type = other DNA
cttttgcataatcgggtaattgatctttgtaagtttgtaacatgtttattctcctcacgtagcccaatgaaatggacccaccccttaaagacggcgtcataatgcgccaacatagaattt

SEQ ID NO: 1049 - DNA, 120 bp, synthetic construct
  source 1..120: mol_type = other DNA
agcccaatgaaatggacccaccccttaaagacggcgtcataatgcgccaacatagaatttctattttcaaaaaaaggagaaggtccatgaaagatattaaaatactgggtgttgatattg

SEQ ID NO: 1050 - DNA, 120 bp, synthetic construct
  source 1..120: mol_type = other DNA
ctattttcaaaaaaaggagaaggtccatgaaagatattaaaatactgggtgttgatattgcaaaagatgtttttcaactgtgtggaattgatgagtggggtaaagtgatctacacgagac

SEQ ID NO: 1051 - DNA, 120 bp, synthetic construct
  source 1..120: mol_type = other DNA
caaaagatgtttttcaactgtgtggaattgatgagtggggtaaagtgatctacacgagacgggttaagcgtgctcagtatgtatccaccgtagccagtcttaaggtgggctgcgtggtga

SEQ ID NO: 1052 - DNA, 120 bp, synthetic construct
  source 1..120: mol_type = other DNA
gggttaagcgtgctcagtatgtatccaccgtagccagtcttaaggtgggctgcgtggtgatggaagcgtgtggaggagcgaaccattggtatcggacgtttatggggatgggtatcccaa

SEQ ID NO: 1053 - DNA, 120 bp, synthetic construct
  source 1..120: mol_type = other DNA
tggaagcgtgtggaggagcgaaccattggtatcggacgtttatggggatgggtatcccaacgcagttgatcagtccgcagcacgtcaaaccgtatgtcaaaagtaacaagaatgatcgta

SEQ ID NO: 1054 - DNA, 120 bp, synthetic construct
  source 1..120: mol_type = other DNA
cgcagttgatcagtccgcagcacgtcaaaccgtatgtcaaaagtaacaagaatgatcgtaacgatgcgcaggcgatagctgaagcggcttcccgcgcctcgatgcggtttgtgcggggta

SEQ ID NO: 1055 - DNA, 120 bp, synthetic construct
  source 1..120: mol_type = other DNA
acgatgcgcaggcgatagctgaagcggcttcccgcgcctcgatgcggtttgtgcggggtaaaacggtggaacaacaagacgttcaagcgctgttaaagatacgcgatcgtttagtcaaaa

SEQ ID NO: 1056 - DNA, 120 bp, synthetic construct
  source 1..120: mol_type = other DNA
aaacggtggaacaacaagacgttcaagcgctgttaaagatacgcgatcgtttagtcaaaagccgcacggcgctgatcaatgagattcgggggttgttgcaagaatacggactcacgatgg

SEQ ID NO: 1057 - DNA, 120 bp, synthetic construct
  source 1..120: mol_type = other DNA
gccgcacggcgctgatcaatgagattcgggggttgttgcaagaatacggactcacgatggcgcgtggtgccaagcgattttatgaagagctcccgttgattttagcgagcgaagcggtgg

SEQ ID NO: 1058 - DNA, 120 bp, synthetic construct
  source 1..120: mol_type = other DNA
cgcgtggtgccaagcgattttatgaagagctcccgttgattttagcgagcgaagcggtgggattaacaccgcggatgaaacgggtgttgaattgtttgtataccgaattgttgaaccggg

SEQ ID NO: 1059 - DNA, 120 bp, synthetic construct
  source 1..120: mol_type = other DNA
gattaacaccgcggatgaaacgggtgttgaattgtttgtataccgaattgttgaaccgggacgaagcgattggtgattacgaggaggaattaaaagcggtggcaaaagccaatgaggatt

SEQ ID NO: 1060 - DNA, 120 bp, synthetic construct
  source 1..120: mol_type = other DNA
acgaagcgattggtgattacgaggaggaattaaaagcggtggcaaaagccaatgaggattgtcaacgggtacagagcatcccgggggtgggttatttaacggcgctctcggtttatgcga

SEQ ID NO: 1061 - DNA, 120 bp, synthetic construct
  source 1..120: mol_type = other DNA
gtcaacgggtacagagcatcccgggggtgggttatttaacggcgctctcggtttatgcgagcgtggtgacattcatcaatttcatcgttcccggcagttgtcggcgtttattgggttggt

SEQ ID NO: 1062 - DNA, 120 bp, synthetic construct
  source 1..120: mol_type = other DNA
gcgtggtgacattcatcaatttcatcgttcccggcagttgtcggcgtttattgggttggtccctcgacaacattcgagtgggaataaggaggtgttgttggggattagtaaacgcggcaa

SEQ ID NO: 1063 - DNA, 120 bp, synthetic construct
  source 1..120: mol_type = other DNA
ccctcgacaacattcgagtgggaataaggaggtgttgttggggattagtaaacgcggcaatgtgatgttaaggacgttattgattcatggcgcccgtgcgctattgcgtcatgtaaaaaa

SEQ ID NO: 1064 - DNA, 120 bp, synthetic construct
  source 1..120: mol_type = other DNA
tgtgatgttaaggacgttattgattcatggcgcccgtgcgctattgcgtcatgtaaaaaataaaacggataaaaagagtctgtggttaaaagcacccattgagcgccgcggaatgaatcg

SEQ ID NO: 1065 - DNA, 120 bp, synthetic construct
  source 1..120: mol_type = other DNA
taaaacggataaaaagagtctgtggttaaaagcacccattgagcgccgcggaatgaatcgcgcttgtgtggcgttagcgaataaaaatgcgcggatcatttgggcgcttttaacacgcca

SEQ ID NO: 1066 - DNA, 120 bp, synthetic construct
  source 1..120: mol_type = other DNA
cgcttgtgtggcgttagcgaataaaaatgcgcggatcatttgggcgcttttaacacgccaagaaacgtatcgctgtggcgcctaaacaccgccgtgggtaaaaaaaagaattaacaaaag

SEQ ID NO: 1067 - DNA, 120 bp, synthetic construct
  source 1..120: mol_type = other DNA
agaaacgtatcgctgtggcgcctaaacaccgccgtgggtaaaaaaaagaattaacaaaaggagacacaccaaccgagttcgaaacaatgagggctgatgaaagtaaggtaaaacctgagg

SEQ ID NO: 1068 - DNA, 120 bp, synthetic construct
  source 1..120: mol_type = other DNA
gagacacaccaaccgagttcgaaacaatgagggctgatgaaagtaaggtaaaacctgaggttgattaagctgattcatacggtggctctgtgaagccgatagcccgataagcatcaacct

SEQ ID NO: 1069 - DNA, 120 bp, synthetic construct
  source 1..120: mol_type = other DNA
ttgattaagctgattcatacggtggctctgtgaagccgatagcccgataagcatcaaccttgcataattcatcaaggcaccaatggtggccaatttaaattgtgatgccggatatacgaa

SEQ ID NO: 1070 - DNA, 120 bp, synthetic construct
  source 1..120: mol_type = other DNA
tgcataattcatcaaggcaccaatggtggccaatttaaattgtgatgccggatatacgaatgcaaccgctttcttttcatcaaaactgattgttgacaacaagggtgggtccatatacgt

SEQ ID NO: 1071 - DNA, 120 bp, synthetic construct
  source 1..120: mol_type = other DNA
tgcaaccgctttcttttcatcaaaactgattgttgacaacaagggtgggtccatatacgtatgaagcgcagcgaaatacggggaattgcctttatttcccggcatttcgctgcgcttcat

SEQ ID NO: 1072 - DNA, 120 bp, synthetic construct
  source 1..120: mol_type = other DNA
atgaagcgcagcgaaatacggggaattgcctttatttcccggcatttcgctgcgcttcatacgggctacttagcgcggttaggcaaccacaattgtttcttcgccttgctgccagttgca

SEQ ID NO: 1073 - DNA, 120 bp, synthetic construct
  source 1..120: mol_type = other DNA
acgggctacttagcgcggttaggcaaccacaattgtttcttcgccttgctgccagttgcaagggcagagttcatcggtttgtaaagcgtcaagaacgcgcaaaacctcttgaggattgcg

SEQ ID NO: 1074 - DNA, 120 bp, synthetic construct
  source 1..120: mol_type = other DNA
agggcagagttcatcggtttgtaaagcgtcaagaacgcgcaaaacctcttgaggattgcggccaacgttgaggtcgttcaccattacaaaacgcacgatgtggttaggatcaacgataaa

SEQ ID NO: 1075 - DNA, 120 bp, synthetic construct
  source 1..120: mol_type = other DNA
gccaacgttgaggtcgttcaccattacaaaacgcacgatgtggttaggatcaacgataaaggtggcacgttccgctacgccttctttttcgttcaaaataccgaggcgttgtgacaagtc

SEQ ID NO: 1076 - DNA, 120 bp, synthetic construct
  source 1..120: mol_type = other DNA
ggtggcacgttccgctacgccttctttttcgttcaaaataccgaggcgttgtgacaagtcacgtcggatgtcggacagcatggggaacggtaattggctaagctcttctttttctcgccg

SEQ ID NO: 1077 - DNA, 120 bp, synthetic construct
  source 1..120: mol_type = other DNA
acgtcggatgtcggacagcatggggaacggtaattggctaagctcttctttttctcgccgccaagctaaatggacaaattcggagtcgacgctggcgccgagcacctgcgcatcgcggtc

SEQ ID NO: 1078 - DNA, 120 bp, synthetic construct
  source 1..120: mol_type = other DNA
ccaagctaaatggacaaattcggagtcgacgctggcgccgagcacctgcgcatcgcggtcagcaaattcgccattcagtcgcccaaattcagcaatttctgtcggacatacaaaggtaaa

SEQ ID NO: 1079 - DNA, 120 bp, synthetic construct
  source 1..120: mol_type = other DNA
agcaaattcgccattcagtcgcccaaattcagcaatttctgtcggacatacaaaggtaaagtccttaggccagaagaagaggacgagccatttgttcgcatagcttttttcgttgatttc

SEQ ID NO: 1080 - DNA, 120 bp, synthetic construct
  source 1..120: mol_type = other DNA
gtccttaggccagaagaagaggacgagccatttgttcgcatagcttttttcgttgatttcggtaaaggctttgttaacatcattgctgattacagcctttaatgaaaatgaaggaaattg

SEQ ID NO: 1081 - DNA, 120 bp, synthetic construct
  source 1..120: mol_type = other DNA
ggtaaaggctttgttaacatcattgctgattacagcctttaatgaaaatgaaggaaattgttcgccgatttttatcatggttttctcctgtagaaatggcagttgttaacagtacaaagg

SEQ ID NO: 1082 - DNA, 120 bp, synthetic construct
  source 1..120: mol_type = other DNA
ttcgccgatttttatcatggttttctcctgtagaaatggcagttgttaacagtacaaaggtattaaaacaaagaatctatgattgataaaattgattatatttattatactaatagaaat

SEQ ID NO: 1083 - DNA, 120 bp, synthetic construct
  source 1..120: mol_type = other DNA
tttctcctgtagaaatggcagttgttaacagtacaaaggtattaaaacaaagaatctatgattgataaaattgattatatttattatactaatagaaattttttatcatacttgggtcta

SEQ ID NO: 1084 - DNA, 120 bp, synthetic construct
  source 1..120: mol_type = other DNA
agttgttagtctacgtggaccgacaagaacagtttcgaatcggaagcttgcttaacgtagttctaacagttttttattagagagcagatctctgatgaacaaccaacggaagaagacggg

SEQ ID NO: 1085 - DNA, 120 bp, synthetic construct
  source 1..120: mol_type = other DNA
ttctaacagttttttattagagagcagatctctgatgaacaaccaacggaagaagacgggtcgaccgtctttcaatatgctgaaacgcgcgagaaaccgcgtgtcaactggttcacagtt

SEQ ID NO: 1086 - DNA, 120 bp, synthetic construct
  source 1..120: mol_type = other DNA
tcgaccgtctttcaatatgctgaaacgcgcgagaaaccgcgtgtcaactggttcacagttggcgaagagattctcaaaaggattgctctcaggccaaggacccatgaaaatggtgatggc

SEQ ID NO: 1087 - DNA, 120 bp, synthetic construct
  source 1..120: mol_type = other DNA
ggcgaagagattctcaaaaggattgctctcaggccaaggacccatgaaaatggtgatggctttcatagcattcctaagatttctagccatacccccaacagcaggaattttggctagatg

SEQ ID NO: 1088 - DNA, 120 bp, synthetic construct
  source 1..120: mol_type = other DNA
tttcatagcattcctaagatttctagccatacccccaacagcaggaattttggctagatggagctcattcaagaagaatggagcgatcaaagtgttacggggtttcaaaaaagagatctc

SEQ ID NO: 1089 - DNA, 120 bp, synthetic construct
  source 1..120: mol_type = other DNA
gagctcattcaagaagaatggagcgatcaaagtgttacggggtttcaaaaaagagatctcaagcatgctgaacataatgaacaggaggaaaagatccgtgaccatgctcctcatgctgct

SEQ ID NO: 1090 - DNA, 120 bp, synthetic construct
  source 1..120: mol_type = other DNA
aagcatgctgaacataatgaacaggaggaaaagatccgtgaccatgctcctcatgctgctgcccacagctctggcgttccatttgaccacacgagggggagaaccacacatgatagttag

SEQ ID NO: 1091 - DNA, 120 bp, synthetic construct
  source 1..120: mol_type = other DNA
gcccacagctctggcgttccatttgaccacacgagggggagaaccacacatgatagttagcaagcaggaaagaggaaagtcactcctgtttaagacctctgcaggtgtcaacatgtgcac

SEQ ID NO: 1092 - DNA, 120 bp, synthetic construct
  source 1..120: mol_type = other DNA
caagcaggaaagaggaaagtcactcctgtttaagacctctgcaggtgtcaacatgtgcaccctcattgcaatggatttgggagagttatgtgaggatacaatgacctacaaatgcccccg

SEQ ID NO: 1093 - DNA, 120 bp, synthetic construct
  source 1..120: mol_type = other DNA
cctcattgcaatggatttgggagagttatgtgaggatacaatgacctacaaatgcccccggatcactgaagcggaaccagatgatgttgattgctggtgcaatgccacggacacatgggt

SEQ ID NO: 1094 - DNA, 120 bp, synthetic construct
  source 1..120: mol_type = other DNA
gatcactgaagcggaaccagatgatgttgattgctggtgcaatgccacggacacatgggtgacctatgggacgtgttctcagactggcgaacaccgacgggataaacgttctgtcgcatt

SEQ ID NO: 1095 - DNA, 120 bp, synthetic construct
  source 1..120: mol_type = other DNA
gacctatgggacgtgttctcagactggcgaacaccgacgggataaacgttctgtcgcattggccccacacgtggggcttggtctcgaaacaagaaccgaaacgtggatgtcctctgaagg

SEQ ID NO: 1096 - DNA, 120 bp, synthetic construct
  source 1..120: mol_type = other DNA
ggccccacacgtggggcttggtctcgaaacaagaaccgaaacgtggatgtcctctgaaggcgcctggagacagatacaaaaagtggagacttgggccttgagacacccaggattcacggt

SEQ ID NO: 1097 - DNA, 120 bp, synthetic construct
  source 1..120: mol_type = other DNA
cgcctggagacagatacaaaaagtggagacttgggccttgagacacccaggattcacggtgatagccctttttctagcacatgccataggaacatccattacccagaaagggatcatctt

SEQ ID NO: 1098 - DNA, 120 bp, synthetic construct
  source 1..120: mol_type = other DNA
gatagccctttttctagcacatgccataggaacatccattacccagaaagggatcatcttcattttgctgatgctggtgacaccatcaatggccatgcgatgtgtgggaataggtaacag

SEQ ID NO: 1099 - DNA, 120 bp, synthetic construct
  source 1..120: mol_type = other DNA
cattttgctgatgctggtgacaccatcaatggccatgcgatgtgtgggaataggtaacagagacttcgttgaaggattgtcaggagcaacatgggtggatgtggtactggagcatggaag

SEQ ID NO: 1100 - DNA, 120 bp, synthetic construct
  source 1..120: mol_type = other DNA
agacttcgttgaaggattgtcaggagcaacatgggtggatgtggtactggagcatggaagctgcgtcaccaccatggcaaaagataaaccaacattggacattgaactcttgaagacgga

SEQ ID NO: 1101 - DNA, 120 bp, synthetic construct
  source 1..120: mol_type = other DNA
ctgcgtcaccaccatggcaaaagataaaccaacattggacattgaactcttgaagacggaggtcacgaaccctgccgtcttgcgcaaactgtgcattgaagctaaaatatcaaacaccac

SEQ ID NO: 1102 - DNA, 120 bp, synthetic construct
  source 1..120: mol_type = other DNA
ggtcacgaaccctgccgtcttgcgcaaactgtgcattgaagctaaaatatcaaacaccactaccgattcaagatgtccaacacaaggagaagctacactggtggaagaacaagacgcgaa

SEQ ID NO: 1103 - DNA, 120 bp, synthetic construct
  source 1..120: mol_type = other DNA
taccgattcaagatgtccaacacaaggagaagctacactggtggaagaacaagacgcgaactttgtgtgtcgacgaacattcgtggacagaggctggggtaatggttgtggactattcgg

SEQ ID NO: 1104 - DNA, 120 bp, synthetic construct
  source 1..120: mol_type = other DNA
ctttgtgtgtcgacgaacattcgtggacagaggctggggtaatggttgtggactattcgggaagggaagcttactaacgtgtgctaagtttaagtgtgtgacaaaacttgaaggaaagat

SEQ ID NO: 1105 - DNA, 120 bp, synthetic construct
  source 1..120: mol_type = other DNA
gaagggaagcttactaacgtgtgctaagtttaagtgtgtgacaaaacttgaaggaaagatagttcaatatgaaaacttaaaatattcggtgatagtcacagtccacactggggaccagca

SEQ ID NO: 1106 - DNA, 120 bp, synthetic construct
  source 1..120: mol_type = other DNA
agttcaatatgaaaacttaaaatattcggtgatagtcacagtccacactggggaccagcaccaggtaggaaatgagactacagaacatggaacaattgcaaccataacacctcaagctcc

SEQ ID NO: 1107 - DNA, 120 bp, synthetic construct
  source 1..120: mol_type = other DNA
ccaggtaggaaatgagactacagaacatggaacaattgcaaccataacacctcaagctcccacgtcggaaatacagctgactgactacggagcccttacattggactgctcacctagaac

SEQ ID NO: 1108 - DNA, 120 bp, synthetic construct
  source 1..120: mol_type = other DNA
cacgtcggaaatacagctgactgactacggagcccttacattggactgctcacctagaacagggctggactttaatgagatggtgctgttgacaatgaaagaaaaatcatggcttgtcca

SEQ ID NO: 1109 - DNA, 120 bp, synthetic construct
  source 1..120: mol_type = other DNA
agggctggactttaatgagatggtgctgttgacaatgaaagaaaaatcatggcttgtccacaaacaatggtttctagacttaccattgccttggacctcgggggcttcaacatctcaaga

SEQ ID NO: 1110 - DNA, 120 bp, synthetic construct
  source 1..120: mol_type = other DNA
caaacaatggtttctagacttaccattgccttggacctcgggggcttcaacatctcaagagacttggaacagacaagatctgctggtcacatttaagacagctcacgcaaagaagcagga

SEQ ID NO: 1111 - DNA, 120 bp, synthetic construct
  source 1..120: mol_type = other DNA
gacttggaacagacaagatctgctggtcacatttaagacagctcacgcaaagaagcaggaagtagtcgtactggggtcacaagaaggagcaatgcacactgcgttgactggggcgacaga

SEQ ID NO: 1112 - DNA, 120 bp, synthetic construct
  source 1..120: mol_type = other DNA
agtagtcgtactggggtcacaagaaggagcaatgcacactgcgttgactggggcgacagaaatccagacgtcaggaacgacgacaatcttcgcaggacacctgaaatgtagactaaaaat

SEQ ID NO: 1113 - DNA, 120 bp, synthetic construct
  source 1..120: mol_type = other DNA
aatccagacgtcaggaacgacgacaatcttcgcaggacacctgaaatgtagactaaaaatggataaactgactttaaaaggggtgtcatatgtgatgtgcacaggctcatttaagctaga

SEQ ID NO: 1114 - DNA, 120 bp, synthetic construct
  source 1..120: mol_type = other DNA
ggataaactgactttaaaaggggtgtcatatgtgatgtgcacaggctcatttaagctagagaaggaagtggctgagacccagcatggaactgtcctagtgcaggttaaatatgaaggaac

SEQ ID NO: 1115 - DNA, 120 bp, synthetic construct
  source 1..120: mol_type = other DNA
gaaggaagtggctgagacccagcatggaactgtcctagtgcaggttaaatatgaaggaacagatgcaccatgcaagattccaatttcaacccaagatgagaaaggagtgacccagaatgg

SEQ ID NO: 1116 - DNA, 120 bp, synthetic construct
  source 1..120: mol_type = other DNA
agatgcaccatgcaagattccaatttcaacccaagatgagaaaggagtgacccagaatgggagattgataacagccaatcccatagttactgacaaagaaaaaccagtcaacattgaaac

SEQ ID NO: 1117 - DNA, 120 bp, synthetic construct
  source 1..120: mol_type = other DNA
gagattgataacagccaatcccatagttactgacaaagaaaaaccagtcaacattgaaacagaaccaccctttggcgagagttacatcgtgataggggcgggtgaaaaagctttgaaact

SEQ ID NO: 1118 - DNA, 120 bp, synthetic construct
  source 1..120: mol_type = other DNA
agaaccaccctttggcgagagttacatcgtgataggggcgggtgaaaaagctttgaaactaagctggttcaagaaaggaagcagcatagggaaaatgttcgaagccaccgcccggggagc

SEQ ID NO: 1119 - DNA, 120 bp, synthetic construct
  source 1..120: mol_type = other DNA
aagctggttcaagaaaggaagcagcatagggaaaatgttcgaagccaccgcccggggagcacgaaggatggctatcctgggggacacagcatgggacttcggttccataggaggggtgtt

SEQ ID NO: 1120 - DNA, 120 bp, synthetic construct
  source 1..120: mol_type = other DNA
acgaaggatggctatcctgggggacacagcatgggacttcggttccataggaggggtgttcacatctttgggaaaattggtacaccaggtttttggaaccgcatatggggtcttgttcag

SEQ ID NO: 1121 - DNA, 120 bp, synthetic construct
  source 1..120: mol_type = other DNA
cacatctttgggaaaattggtacaccaggtttttggaaccgcatatggggtcttgttcagcggtgtttcctggaccatgaaaataggaataggggttctgctgacatggctaggattgaa

SEQ ID NO: 1122 - DNA, 120 bp, synthetic construct
  source 1..120: mol_type = other DNA
cggtgtttcctggaccatgaaaataggaataggggttctgctgacatggctaggattgaattcaaggagcacgtcactctcgatgacgtgcattgcagttggcatggtcacactgtacct

SEQ ID NO: 1123 - DNA, 120 bp, synthetic construct
  source 1..120: mol_type = other DNA
ttcaaggagcacgtcactctcgatgacgtgcattgcagttggcatggtcacactgtacctaggagtcatggttcaagcggactcggggtgtgtgatcaactggaagggcagagaactcaa

SEQ ID NO: 1124 - DNA, 120 bp, synthetic construct
  source 1..120: mol_type = other DNA
aggagtcatggttcaagcggactcggggtgtgtgatcaactggaagggcagagaactcaagtgtggaagtggcatctttgtcactaatgaagtccacacttggacagagcaatataaatt

SEQ ID NO: 1125 - DNA, 120 bp, synthetic construct
  source 1..120: mol_type = other DNA
gtgtggaagtggcatctttgtcactaatgaagtccacacttggacagagcaatataaattccaggctgactccccaaaaagactatcagcagccattgggaaggcatgggaggaaggcgt

SEQ ID NO: 1126 - DNA, 120 bp, synthetic construct
  source 1..120: mol_type = other DNA
ccaggctgactccccaaaaagactatcagcagccattgggaaggcatgggaggaaggcgtgtgtggaattcgatcagccacacgtcttgagaacatcatgtggaagcaaatatcaaatga

SEQ ID NO: 1127 - DNA, 120 bp, synthetic construct
  source 1..120: mol_type = other DNA
gtgtggaattcgatcagccacacgtcttgagaacatcatgtggaagcaaatatcaaatgaattgaaccacattctacttgaaaatgacatgaaattcacagtggttgtaggagacgctaa

SEQ ID NO: 1128 - DNA, 120 bp, synthetic construct
  source 1..120: mol_type = other DNA
attgaaccacattctacttgaaaatgacatgaaattcacagtggttgtaggagacgctaatggaatcttgacccaaggaaaaaagatgattaggccacaacccatggaacacaaatactc

SEQ ID NO: 1129 - DNA, 120 bp, synthetic construct
  source 1..120: mol_type = other DNA
tggaatcttgacccaaggaaaaaagatgattaggccacaacccatggaacacaaatactcatggaaaagctggggaaaagccaaaatcataggagcagacacacagaatactaccttcat

SEQ ID NO: 1130 - DNA, 120 bp, synthetic construct
  source 1..120: mol_type = other DNA
atggaaaagctggggaaaagccaaaatcataggagcagacacacagaatactaccttcatcatcgacggcccagatactccagaatgccccgatgaccagagagcatggaacatttggga

SEQ ID NO: 1131 - DNA, 120 bp, synthetic construct
  source 1..120: mol_type = other DNA
catcgacggcccagatactccagaatgccccgatgaccagagagcatggaacatttgggaagttgaggactatgggtttggagttttcacgacaaacatatggctgaaattgcgtgactc

SEQ ID NO: 1132 - DNA, 120 bp, synthetic construct
  source 1..120: mol_type = other DNA
agttgaggactatgggtttggagttttcacgacaaacatatggctgaaattgcgtgactcctacacccaaatgtgtgaccaccggctaatgtcagctgccatcaaggacagcaaggcagt

SEQ ID NO: 1133 - DNA, 120 bp, synthetic construct
  source 1..120: mol_type = other DNA
ctacacccaaatgtgtgaccaccggctaatgtcagctgccatcaaggacagcaaggcagtccatgctgacatggggtactggatagaaagtgaaaagaacgagacctggaagctagcgag

SEQ ID NO: 1134 - DNA, 120 bp, synthetic construct
  source 1..120: mol_type = other DNA
ccatgctgacatggggtactggatagaaagtgaaaagaacgagacctggaagctagcgagagcctccttcatagaagtgaagacatgcatctggccaagatcccacactctatggagcaa

SEQ ID NO: 1135 - DNA, 120 bp, synthetic construct
  source 1..120: mol_type = other DNA
agcctccttcatagaagtgaagacatgcatctggccaagatcccacactctatggagcaatggagtcttggaaagtgaaatgataatcccaaagatatatggaggaccaatatctcagca

SEQ ID NO: 1136 - DNA, 120 bp, synthetic construct
  source 1..120: mol_type = other DNA
tggagtcttggaaagtgaaatgataatcccaaagatatatggaggaccaatatctcagcacaactacagaccagggtatttcacacaaacagcagggccatggcacctaggcaagttgga

SEQ ID NO: 1137 - DNA, 120 bp, synthetic construct
  source 1..120: mol_type = other DNA
caactacagaccagggtatttcacacaaacagcagggccatggcacctaggcaagttggaattagactttaatttgtgtgaaggcaccacagtagttgtggatgaacattgtggaaatcg

SEQ ID NO: 1138 - DNA, 120 bp, synthetic construct
  source 1..120: mol_type = other DNA
attagactttaatttgtgtgaaggcaccacagtagttgtggatgaacattgtggaaatcgaggtccatctcttagaactacaacagtcacaggaaagataatccatgaatggtgttgcag

SEQ ID NO: 1139 - DNA, 120 bp, synthetic construct
  source 1..120: mol_type = other DNA
aggtccatctcttagaactacaacagtcacaggaaagataatccatgaatggtgttgcagatcctgcacgctaccccccctacgcttcagaggagaagacggatgttggtatggcatgga

SEQ ID NO: 1140 - DNA, 120 bp, synthetic construct
  source 1..120: mol_type = other DNA
atcctgcacgctaccccccctacgcttcagaggagaagacggatgttggtatggcatggaaatcagaccagttaaggagaaggaagagaatctagtcaggtcaatggtctctgcagggtc

SEQ ID NO: 1141 - DNA, 120 bp, synthetic construct
  source 1..120: mol_type = other DNA
aatcagaccagttaaggagaaggaagagaatctagtcaggtcaatggtctctgcagggtcaggagaagtggacagtttttcattgggactactatgcgtatcaataatgattgaagaagt

SEQ ID NO: 1142 - DNA, 120 bp, synthetic construct
  source 1..120: mol_type = other DNA
aggagaagtggacagtttttcattgggactactatgcgtatcaataatgattgaagaagtgatgagatccagatggagtagaaagatgctgatgactggaacactggctgttttcttcct

SEQ ID NO: 1143 - DNA, 120 bp, synthetic construct
  source 1..120: mol_type = other DNA
gatgagatccagatggagtagaaagatgctgatgactggaacactggctgttttcttccttcttataatgggacaactgacatggaatgatctgatcaggttatgcatcatggttggagc

SEQ ID NO: 1144 - DNA, 120 bp, synthetic construct
  source 1..120: mol_type = other DNA
tcttataatgggacaactgacatggaatgatctgatcaggttatgcatcatggttggagccaatgtctcagacagaatggggatgggaacaacgtacctagccttgatggccacttttaa

SEQ ID NO: 1145 - DNA, 120 bp, synthetic construct
  source 1..120: mol_type = other DNA
caatgtctcagacagaatggggatgggaacaacgtacctagccttgatggccacttttaaaatgagaccgatgttcgctgttgggctattacttcgcagactaacatccagagaggtgct

SEQ ID NO: 1146 - DNA, 120 bp, synthetic construct
  source 1..120: mol_type = other DNA
aatgagaccgatgttcgctgttgggctattacttcgcagactaacatccagagaggtgctccttctcacaattggactaagcctggtggcatccgtggagctaccaaattctttagagga

SEQ ID NO: 1147 - DNA, 120 bp, synthetic construct
  source 1..120: mol_type = other DNA
ccttctcacaattggactaagcctggtggcatccgtggagctaccaaattctttagaggagctaggggacggacttgcgatgggcatcatgatgttaaaattgttgactgattttcagtc

SEQ ID NO: 1148 - DNA, 120 bp, synthetic construct
  source 1..120: mol_type = other DNA
gctaggggacggacttgcgatgggcatcatgatgttaaaattgttgactgattttcagtcacaccagttgtggattaccttactgtctctgacattcatcaaaacaactctctcactgga

SEQ ID NO: 1149 - DNA, 120 bp, synthetic construct
  source 1..120: mol_type = other DNA
acaccagttgtggattaccttactgtctctgacattcatcaaaacaactctctcactggattatgcatggaagacaatggctatggtattgtcaatcgtatctctctttcctctatgtct

SEQ ID NO: 1150 - DNA, 120 bp, synthetic construct
  source 1..120: mol_type = other DNA
ttatgcatggaagacaatggctatggtattgtcaatcgtatctctctttcctctatgtctatccacgacctctcaaaaaacaacatggcttccggtgctgctaggatcctttggatgtaa

SEQ ID NO: 1151 - DNA, 120 bp, synthetic construct
  source 1..120: mol_type = other DNA
atccacgacctctcaaaaaacaacatggcttccggtgctgctaggatcctttggatgtaaaccactaaccatgtttcttataacagaaaacaaaatttggggaaggaaaagttggcccct

SEQ ID NO: 1152 - DNA, 120 bp, synthetic construct
  source 1..120: mol_type = other DNA
accactaaccatgtttcttataacagaaaacaaaatttggggaaggaaaagttggcccctcaatgaaggaattatggctgttggaatagtcagcattttattaagttcactcctcaaaaa

SEQ ID NO: 1153 - DNA, 120 bp, synthetic construct
  source 1..120: mol_type = other DNA
caatgaaggaattatggctgttggaatagtcagcattttattaagttcactcctcaaaaatgacgtgccactagccggcccactaatagctggaggcatgctgatagcatgttacgtcat

SEQ ID NO: 1154 - DNA, 120 bp, synthetic construct
  source 1..120: mol_type = other DNA
tgacgtgccactagccggcccactaatagctggaggcatgctgatagcatgttacgtcatatccggaagctcagccgatttatcattggagagagcggctgaggtctcctgggaagaaga

SEQ ID NO: 1155 - DNA, 120 bp, synthetic construct
  source 1..120: mol_type = other DNA
atccggaagctcagccgatttatcattggagagagcggctgaggtctcctgggaagaagaagcagaacactctggtgcctcacacaacatactagtggaggtccaagatgatggaactat

SEQ ID NO: 1156 - DNA, 120 bp, synthetic construct
  source 1..120: mol_type = other DNA
agcagaacactctggtgcctcacacaacatactagtggaggtccaagatgatggaactatgaaaataaaagatgaagagagagatgatacgctcactatactcctcaaagcaactttgtt

SEQ ID NO: 1157 - DNA, 120 bp, synthetic construct
  source 1..120: mol_type = other DNA
gaaaataaaagatgaagagagagatgatacgctcactatactcctcaaagcaactttgttggcagtttcaggggtgtacccaatgtcaataccagcaaccctttttgtgtggtatttttg

SEQ ID NO: 1158 - DNA, 120 bp, synthetic construct
  source 1..120: mol_type = other DNA
ggcagtttcaggggtgtacccaatgtcaataccagcaaccctttttgtgtggtatttttggcagaaaaagaaacagagatcaggagtcttgtgggacacacccagccctccagaagtaga

SEQ ID NO: 1159 - DNA, 120 bp, synthetic construct
  source 1..120: mol_type = other DNA
gcagaaaaagaaacagagatcaggagtcttgtgggacacacccagccctccagaagtagaaagagcagttcttgatgatggtatctatagaatcttgcaaagaggactgttgggtaggtc

SEQ ID NO: 1160 - DNA, 120 bp, synthetic construct
  source 1..120: mol_type = other DNA
aagagcagttcttgatgatggtatctatagaatcttgcaaagaggactgttgggtaggtcccaggtaggagtgggagtttttcaagacggcgtgttccacacaatgtggcatgtcaccag

SEQ ID NO: 1161 - DNA, 120 bp, synthetic construct
  source 1..120: mol_type = other DNA
ccaggtaggagtgggagtttttcaagacggcgtgttccacacaatgtggcatgtcaccaggggggctgtcctcatgtaccaagggaagaggctggaaccaagttgggccagtgtcaaaaa

SEQ ID NO: 1162 - DNA, 120 bp, synthetic construct
  source 1..120: mol_type = other DNA
gggggctgtcctcatgtaccaagggaagaggctggaaccaagttgggccagtgtcaaaaaagacttgatctcatatggaggaggttggaggtttcaaggatcatggaacacgggagaaga

SEQ ID NO: 1163 - DNA, 120 bp, synthetic construct
  source 1..120: mol_type = other DNA
agacttgatctcatatggaggaggttggaggtttcaaggatcatggaacacgggagaagaagtacaggtgatagctgttgaaccagggaaaaacccaaagaatgtacagacaacgccagg

SEQ ID NO: 1164 - DNA, 120 bp, synthetic construct
  source 1..120: mol_type = other DNA
agtacaggtgatagctgttgaaccagggaaaaacccaaagaatgtacagacaacgccaggcaccttcatgacccctgaaggcgcagttggagccatagccctagatttcaaacctggcac

SEQ ID NO: 1165 - DNA, 120 bp, synthetic construct
  source 1..120: mol_type = other DNA
caccttcatgacccctgaaggcgcagttggagccatagccctagatttcaaacctggcacatctggatctcccatcgtgaacagagagagaaaaatagtaggtctttatggaaatggagt

SEQ ID NO: 1166 - DNA, 120 bp, synthetic construct
  source 1..120: mol_type = other DNA
atctggatctcccatcgtgaacagagagagaaaaatagtaggtctttatggaaatggagtggtgacaacaagtggaacctacgtcagtgccattgcccaagctaaagcgtcacaagaagg

SEQ ID NO: 1167 - DNA, 120 bp, synthetic construct
  source 1..120: mol_type = other DNA
ggtgacaacaagtggaacctacgtcagtgccattgcccaagctaaagcgtcacaagaagggcctctaccagagattgaggacgaggtgttcaagaaaagaaacctaacaataatggacct

SEQ ID NO: 1168 - DNA, 120 bp, synthetic construct
  source 1..120: mol_type = other DNA
gcctctaccagagattgaggacgaggtgttcaagaaaagaaacctaacaataatggacctacatccaggatcaggaaaaacaagaagatatcttccagccatagtccgtgaggccataaa

SEQ ID NO: 1169 - DNA, 120 bp, synthetic construct
  source 1..120: mol_type = other DNA
acatccaggatcaggaaaaacaagaagatatcttccagccatagtccgtgaggccataaaaagaaagctgcgcacgctaatcttggctcccacaagagttgtcgcctctgagatggcaga

SEQ ID NO: 1170 - DNA, 120 bp, synthetic construct
  source 1..120: mol_type = other DNA
aagaaagctgcgcacgctaatcttggctcccacaagagttgtcgcctctgagatggcagaggcgctcaaaggaatgccaataagatatcagacaacagcagtaaagagtgaacacacagg

SEQ ID NO: 1171 - DNA, 120 bp, synthetic construct
  source 1..120: mol_type = other DNA
ggcgctcaaaggaatgccaataagatatcagacaacagcagtaaagagtgaacacacaggaaaggagatagtcgatctcatgtgccacgccactttcaccatgcgtctcctatctccagt

SEQ ID NO: 1172 - DNA, 120 bp, synthetic construct
  source 1..120: mol_type = other DNA
aaaggagatagtcgatctcatgtgccacgccactttcaccatgcgtctcctatctccagtgagagttcccaattacaacatgattatcatggatgaagcacactttaccgatccagctag

SEQ ID NO: 1173 - DNA, 120 bp, synthetic construct
  source 1..120: mol_type = other DNA
gagagttcccaattacaacatgattatcatggatgaagcacactttaccgatccagctagcatagcggccagagggtacatctcaacccgagtgggtatgggtgaagcagctgcgatctt

SEQ ID NO: 1174 - DNA, 120 bp, synthetic construct
  source 1..120: mol_type = other DNA
catagcggccagagggtacatctcaacccgagtgggtatgggtgaagcagctgcgatctttatgacagccactcccccaggatcggtagaggcctttccacagagcaatgcagttattca

SEQ ID NO: 1175 - DNA, 120 bp, synthetic construct
  source 1..120: mol_type = other DNA
tatgacagccactcccccaggatcggtagaggcctttccacagagcaatgcagttattcaagatgaggaaagagacattcctgagagatcatggaactcaggctacgactggatcactga

SEQ ID NO: 1176 - DNA, 120 bp, synthetic construct
  source 1..120: mol_type = other DNA
agatgaggaaagagacattcctgagagatcatggaactcaggctacgactggatcactgatttcccaggaaaaacagtctggtttgttccaagcatcaaatcaggaaatgacattgccaa

SEQ ID NO: 1177 - DNA, 120 bp, synthetic construct
  source 1..120: mol_type = other DNA
tttcccaggaaaaacagtctggtttgttccaagcatcaaatcaggaaatgacattgccaactgtttaagaaaaaacgggaaacgggtgatccaattgagcagaaaaacctttgacactga

SEQ ID NO: 1178 - DNA, 120 bp, synthetic construct
  source 1..120: mol_type = other DNA
ctgtttaagaaaaaacgggaaacgggtgatccaattgagcagaaaaacctttgacactgagtaccagaaaacaaaaaacaatgattgggactatgttgtcacaacagacatttccgaaat

SEQ ID NO: 1179 - DNA, 120 bp, synthetic construct
  source 1..120: mol_type = other DNA
gtaccagaaaacaaaaaacaatgattgggactatgttgtcacaacagacatttccgaaatgggagcaaatttccgggccgacagggtaatagacccaaggcggtgtttgaagccggtaat

SEQ ID NO: 1180 - DNA, 120 bp, synthetic construct
  source 1..120: mol_type = other DNA
gggagcaaatttccgggccgacagggtaatagacccaaggcggtgtttgaagccggtaatactaaaagatggcccagagcgcgtcattctggccggaccaatgccagtgaccgcggccag

SEQ ID NO: 1181 - DNA, 120 bp, synthetic construct
  source 1..120: mol_type = other DNA
actaaaagatggcccagagcgcgtcattctggccggaccaatgccagtgaccgcggccagtgctgcccagagaagaggaagaattggaaggaaccaaaacaaagaaggtgaccagtatat

SEQ ID NO: 1182 - DNA, 120 bp, synthetic construct
  source 1..120: mol_type = other DNA
tgctgcccagagaagaggaagaattggaaggaaccaaaacaaagaaggtgaccagtatatttacatgggacagcctttaaacaatgatgaggaccacgctcattggacagaagcaaaaat

SEQ ID NO: 1183 - DNA, 120 bp, synthetic construct
  source 1..120: mol_type = other DNA
ttacatgggacagcctttaaacaatgatgaggaccacgctcattggacagaagcaaaaatgctccttgacaatataaacacgccagaaggaattatcccagccctctttgagccagagag

SEQ ID NO: 1184 - DNA, 120 bp, synthetic construct
  source 1..120: mol_type = other DNA
gctccttgacaatataaacacgccagaaggaattatcccagccctctttgagccagagagagaaaagagtgcagcaatagacggggagtacagactgcggggagaagcaaggaaaacgtt

SEQ ID NO: 1185 - DNA, 120 bp, synthetic construct
  source 1..120: mol_type = other DNA
agaaaagagtgcagcaatagacggggagtacagactgcggggagaagcaaggaaaacgttcgtggagctaatgagaagaggggatttaccagtttggctatcttacaaagttgcctcaga

SEQ ID NO: 1186 - DNA, 120 bp, synthetic construct
  source 1..120: mol_type = other DNA
cgtggagctaatgagaagaggggatttaccagtttggctatcttacaaagttgcctcagaaggcttccagtactccgacagaagatggtgctttgacggggaaaggaacaaccaggtgtt

SEQ ID NO: 1187 - DNA, 120 bp, synthetic construct
  source 1..120: mol_type = other DNA
aggcttccagtactccgacagaagatggtgctttgacggggaaaggaacaaccaggtgttggaggagaatatggacgtggagatctggacaaaagaaggagaaagaaagaaattgcgacc

SEQ ID NO: 1188 - DNA, 120 bp, synthetic construct
  source 1..120: mol_type = other DNA
ggaggagaatatggacgtggagatctggacaaaagaaggagaaagaaagaaattgcgaccccgctggctggatgccagaacctactctgatccactggccctgcgcgagtttaaagagtt

SEQ ID NO: 1189 - DNA, 120 bp, synthetic construct
  source 1..120: mol_type = other DNA
ccgctggctggatgccagaacctactctgatccactggccctgcgcgagtttaaagagttcgcagcaggaagaagaagtgtctcaggtgacctaatattagaaatagggaaacttccaca

SEQ ID NO: 1190 - DNA, 120 bp, synthetic construct
  source 1..120: mol_type = other DNA
cgcagcaggaagaagaagtgtctcaggtgacctaatattagaaatagggaaacttccacagcatctgacgctaagggcccagaatgctttggacaacttggtcatgttgcacaattccga

SEQ ID NO: 1191 - DNA, 120 bp, synthetic construct
  source 1..120: mol_type = other DNA
gcatctgacgctaagggcccagaatgctttggacaacttggtcatgttgcacaattccgaacaaggaggaaaagcctatagacatgctatggaagaactaccagacaccatagaaacatt

SEQ ID NO: 1192 - DNA, 120 bp, synthetic construct
  source 1..120: mol_type = other DNA
acaaggaggaaaagcctatagacatgctatggaagaactaccagacaccatagaaacattgatgctactagctttgatagctgtgctgactggtggagttacgttgtttttcctatcagg

SEQ ID NO: 1193 - DNA, 120 bp, synthetic construct
  source 1..120: mol_type = other DNA
gatgctactagctttgatagctgtgctgactggtggagttacgttgtttttcctatcaggaaggggtctaggaaaaacatccattggcctactttgtgtaatggcctcaagtgtactgtt

SEQ ID NO: 1194 - DNA, 120 bp, synthetic construct
  source 1..120: mol_type = other DNA
aaggggtctaggaaaaacatccattggcctactttgtgtaatggcctcaagtgtactgttatggatggccagtgtggagccccattggatagcggcctccatcatactagagttttttct

SEQ ID NO: 1195 - DNA, 120 bp, synthetic construct
  source 1..120: mol_type = other DNA
atggatggccagtgtggagccccattggatagcggcctccatcatactagagttttttctgatggtgctgctcattccagagccagacagacagcgtactccacaggacaatcaactagc

SEQ ID NO: 1196 - DNA, 120 bp, synthetic construct
  source 1..120: mol_type = other DNA
gatggtgctgctcattccagagccagacagacagcgtactccacaggacaatcaactagcatatgtggtgataggtttgttattcatgatattgacagtggcagccaatgagatgggatt

SEQ ID NO: 1197 - DNA, 120 bp, synthetic construct
  source 1..120: mol_type = other DNA
atatgtggtgataggtttgttattcatgatattgacagtggcagccaatgagatgggattactggaaaccacaaagaaagacctggggattggccatgtagtcgccgaaaaccaccacca

SEQ ID NO: 1198 - DNA, 120 bp, synthetic construct
  source 1..120: mol_type = other DNA
actggaaaccacaaagaaagacctggggattggccatgtagtcgccgaaaaccaccaccatgccacaatgctagacatagacctacatccagcttcagcctggaccctctatgcagtagc

SEQ ID NO: 1199 - DNA, 120 bp, synthetic construct
  source 1..120: mol_type = other DNA
tgccacaatgctagacatagacctacatccagcttcagcctggaccctctatgcagtagccacaacaatcatcactcccatgatgagacacacaattgaaaacacaacggcaaacatttc

SEQ ID NO: 1200 - DNA, 120 bp, synthetic construct
  source 1..120: mol_type = other DNA
cacaacaatcatcactcccatgatgagacacacaattgaaaacacaacggcaaacatttccctgacagctattgcaaatcaggcggctatattaatgggacttgacaagggatggccaat

SEQ ID NO: 1201 - DNA, 120 bp, synthetic construct
  source 1..120: mol_type = other DNA
cctgacagctattgcaaatcaggcggctatattaatgggacttgacaagggatggccaatatcgaagatggacataggagtgccacttctcgccttagggtgctattcccaggtgaaccc

SEQ ID NO: 1202 - DNA, 120 bp, synthetic construct
  source 1..120: mol_type = other DNA
atcgaagatggacataggagtgccacttctcgccttagggtgctattcccaggtgaacccattgacactgacagcggcggtgttgatgttagtggcccattatgccataatcggacctgg

SEQ ID NO: 1203 - DNA, 120 bp, synthetic construct
  source 1..120: mol_type = other DNA
attgacactgacagcggcggtgttgatgttagtggcccattatgccataatcggacctggactgcaagcgaaagctactagagaagcccaaaaaaggactgcggccggaataatgaaaaa

SEQ ID NO: 1204 - DNA, 120 bp, synthetic construct
  source 1..120: mol_type = other DNA
actgcaagcgaaagctactagagaagcccaaaaaaggactgcggccggaataatgaaaaacccaactgtagacgggattgttgcaatagatttggatcctgtggtttatgatgcaaaatt

SEQ ID NO: 1205 - DNA, 120 bp, synthetic construct
  source 1..120: mol_type = other DNA
cccaactgtagacgggattgttgcaatagatttggatcctgtggtttatgatgcaaaatttgaaaaacagctaggccaaataatgttactaatactctgcacatcacagattctcttgat

SEQ ID NO: 1206 - DNA, 120 bp, synthetic construct
  source 1..120: mol_type = other DNA
tgaaaaacagctaggccaaataatgttactaatactctgcacatcacagattctcttgatgaggactacatgggccttatgtgaatccatcacactggctactggacccttgaccactct

SEQ ID NO: 1207 - DNA, 120 bp, synthetic construct
  source 1..120: mol_type = other DNA
gaggactacatgggccttatgtgaatccatcacactggctactggacccttgaccactctctgggagggatctcctggaagattctggaataccacgatagcagtgtccatggcaaacat

SEQ ID NO: 1208 - DNA, 120 bp, synthetic construct
  source 1..120: mol_type = other DNA
ctgggagggatctcctggaagattctggaataccacgatagcagtgtccatggcaaacatcttcaggggaagttatctagcaggagcaggtctggccttctcattaatgaaatctttagg

SEQ ID NO: 1209 - DNA, 120 bp, synthetic construct
  source 1..120: mol_type = other DNA
cttcaggggaagttatctagcaggagcaggtctggccttctcattaatgaaatctttaggaggaggtaggagaggcacgggagcccaaggggaaacattgggagaaaaatggaaaagaca

SEQ ID NO: 1210 - DNA, 120 bp, synthetic construct
  source 1..120: mol_type = other DNA
aggaggtaggagaggcacgggagcccaaggggaaacattgggagaaaaatggaaaagacaactaaaccaattgagcaagtcagaatttaacacttacaaaaggagtggaattatggaggt

SEQ ID NO: 1211 - DNA, 120 bp, synthetic construct
  source 1..120: mol_type = other DNA
actaaaccaattgagcaagtcagaatttaacacttacaaaaggagtggaattatggaggtggacagatctgaagccaaggaaggactgaaaagaggagaaacaaccaaacatgcagtgtc

SEQ ID NO: 1212 - DNA, 120 bp, synthetic construct
  source 1..120: mol_type = other DNA
ggacagatctgaagccaaggaaggactgaaaagaggagaaacaaccaaacatgcagtgtcgagaggaacagccaaacttaggtggtttgtggagaggaaccttgtgaaaccagaagggaa

SEQ ID NO: 1213 - DNA, 120 bp, synthetic construct
  source 1..120: mol_type = other DNA
gagaggaacagccaaacttaggtggtttgtggagaggaaccttgtgaaaccagaagggaaagtgatagacctcggttgtggaagaggtggctggtcatattactgcgctgggctgaagaa

SEQ ID NO: 1214 - DNA, 120 bp, synthetic construct
  source 1..120: mol_type = other DNA
agtgatagacctcggttgtggaagaggtggctggtcatattactgcgctgggctgaagaaggtcacagaagtgaagggatacacaaaaggaggacccggtcatgaggaacctatcccaat

SEQ ID NO: 1215 - DNA, 120 bp, synthetic construct
  source 1..120: mol_type = other DNA
ggtcacagaagtgaagggatacacaaaaggaggacccggtcatgaggaacctatcccaatggcgacttatggatggaacatagtgaagctacactctggaagggatgtattctttacacc

SEQ ID NO: 1216 - DNA, 120 bp, synthetic construct
  source 1..120: mol_type = other DNA
ggcgacttatggatggaacatagtgaagctacactctggaagggatgtattctttacaccacctgagaaatgtgacacccttttgtgtgatattggtgagtcctctccgaatccaactat

SEQ ID NO: 1217 - DNA, 120 bp, synthetic construct
  source 1..120: mol_type = other DNA
acctgagaaatgtgacacccttttgtgtgatattggtgagtcctctccgaatccaactatagaagaaggaagaacgttacgtgttctaaagatggtggaaccatggctcagaggaaacca

SEQ ID NO: 1218 - DNA, 120 bp, synthetic construct
  source 1..120: mol_type = other DNA
agaagaaggaagaacgttacgtgttctaaagatggtggaaccatggctcagaggaaaccagttttgcataaaaatcctaaatccttacatgccaagtgtggtagaaactctggagcaaat

SEQ ID NO: 1219 - DNA, 120 bp, synthetic construct
  source 1..120: mol_type = other DNA
gttttgcataaaaatcctaaatccttacatgccaagtgtggtagaaactctggagcaaatgcaaagaaaacatggagggatgctagtgcgaaacccactctcaagaaattctacccatga

SEQ ID NO: 1220 - DNA, 120 bp, synthetic construct
  source 1..120: mol_type = other DNA
gcaaagaaaacatggagggatgctagtgcgaaacccactctcaagaaattctacccatgaaatgtactgggtttcatgtggaacaggaaacattgtgtcggcagtgaacatgacatccag

SEQ ID NO: 1221 - DNA, 120 bp, synthetic construct
  source 1..120: mol_type = other DNA
aatgtactgggtttcatgtggaacaggaaacattgtgtcggcagtgaacatgacatccagaatgttgctgaatcggttcacaatgactcacaggaagccaacgtatgaaagagacgtgga

SEQ ID NO: 1222 - DNA, 120 bp, synthetic construct
  source 1..120: mol_type = other DNA
aatgttgctgaatcggttcacaatgactcacaggaagccaacgtatgaaagagacgtggacttgggcgctggaacaagacatgtggcagtggaaccagagatagccaacctagacattat

SEQ ID NO: 1223 - DNA, 120 bp, synthetic construct
  source 1..120: mol_type = other DNA
cttgggcgctggaacaagacatgtggcagtggaaccagagatagccaacctagacattattggccagaggatagagaacataaaaaatgaacataagtcaacatggcattatgatgagga

SEQ ID NO: 1224 - DNA, 120 bp, synthetic construct
  source 1..120: mol_type = other DNA
tggccagaggatagagaacataaaaaatgaacataagtcaacatggcattatgatgaggacaatccatacaaaacatgggcctatcatggatcatatgaggtcaagccatcagggtcagc

SEQ ID NO: 1225 - DNA, 120 bp, synthetic construct
  source 1..120: mol_type = other DNA
caatccatacaaaacatgggcctatcatggatcatatgaggtcaagccatcagggtcagcctcatccatggtgaatggcgtggtgagattgctcaccaagccatgggatgtcatccccat

SEQ ID NO: 1226 - DNA, 120 bp, synthetic construct
  source 1..120: mol_type = other DNA
ctcatccatggtgaatggcgtggtgagattgctcaccaagccatgggatgtcatccccatggtcacacaaatagctatgactgataccacacccttcggacaacagagggttttcaaaga

SEQ ID NO: 1227 - DNA, 120 bp, synthetic construct
  source 1..120: mol_type = other DNA
ggtcacacaaatagctatgactgataccacacccttcggacaacagagggttttcaaagagaaagttgacacacgcacaccaagaccaaaacgaggcacagcacaaattatggaggtgac

SEQ ID NO: 1228 - DNA, 120 bp, synthetic construct
  source 1..120: mol_type = other DNA
gaaagttgacacacgcacaccaagaccaaaacgaggcacagcacaaattatggaggtgacagccaagtggttgtggggattactctctagaaataaaaaacccagaatttgcacaagaga

SEQ ID NO: 1229 - DNA, 120 bp, synthetic construct
  source 1..120: mol_type = other DNA
agccaagtggttgtggggattactctctagaaataaaaaacccagaatttgcacaagagaggagttcacaagaaaagttaggtcaaacgcagcaattggagcagtgtttgttgatgaaaa

SEQ ID NO: 1230 - DNA, 120 bp, synthetic construct
  source 1..120: mol_type = other DNA
ggagttcacaagaaaagttaggtcaaacgcagcaattggagcagtgtttgttgatgaaaaccaatggaactcagcaaaagaagcagtggaagacgaaaggttttgggacctcgtgcacag

SEQ ID NO: 1231 - DNA, 120 bp, synthetic construct
  source 1..120: mol_type = other DNA
ccaatggaactcagcaaaagaagcagtggaagacgaaaggttttgggacctcgtgcacagagagagagagcttcataaacagggaaaatgtgccacgtgtgtctacaatatgatgggtaa

SEQ ID NO: 1232 - DNA, 120 bp, synthetic construct
  source 1..120: mol_type = other DNA
agagagagagcttcataaacagggaaaatgtgccacgtgtgtctacaatatgatgggtaaaagagagaaaaaactaggagagtttggaaaggcaaagggaagtcgtgcaatatggtacat

SEQ ID NO: 1233 - DNA, 120 bp, synthetic construct
  source 1..120: mol_type = other DNA
aagagagaaaaaactaggagagtttggaaaggcaaagggaagtcgtgcaatatggtacatgtggttgggagcacgctttctagagtttgaagcccttggcttcatgaatgaagaccactg

SEQ ID NO: 1234 - DNA, 120 bp, synthetic construct
  source 1..120: mol_type = other DNA
gtggttgggagcacgctttctagagtttgaagcccttggcttcatgaatgaagaccactggttcagtagggagaattcactcagtggagtggaaggagaaggactacataaacttggata

SEQ ID NO: 1235 - DNA, 120 bp, synthetic construct
  source 1..120: mol_type = other DNA
gttcagtagggagaattcactcagtggagtggaaggagaaggactacataaacttggatacatacttagagacatatcaaagattccagggggaaatatgtatgcagacgacacagctgg

SEQ ID NO: 1236 - DNA, 120 bp, synthetic construct
  source 1..120: mol_type = other DNA
catacttagagacatatcaaagattccagggggaaatatgtatgcagacgacacagctggatgggacacgagaataacagaggatgatcttcagaatgaggctaaaatcaccgacatcat

SEQ ID NO: 1237 - DNA, 120 bp, synthetic construct
  source 1..120: mol_type = other DNA
atgggacacgagaataacagaggatgatcttcagaatgaggctaaaatcaccgacatcatggagcccgaacatgctctactggccacgtcaatcttcaagctgacctatcaaaataaagt

SEQ ID NO: 1238 - DNA, 120 bp, synthetic construct
  source 1..120: mol_type = other DNA
ggagcccgaacatgctctactggccacgtcaatcttcaagctgacctatcaaaataaagtggtaagggtgcaaagaccagcaaaaagtggaaccgtgatggacgtcatatccagacgaga

SEQ ID NO: 1239 - DNA, 120 bp, synthetic construct
  source 1..120: mol_type = other DNA
ggtaagggtgcaaagaccagcaaaaagtggaaccgtgatggacgtcatatccagacgagaccagagaggaagtggacaggtcggaacttatggcctaaacactttcactaacatggaggt

SEQ ID NO: 1240 - DNA, 120 bp, synthetic construct
  source 1..120: mol_type = other DNA
ccagagaggaagtggacaggtcggaacttatggcctaaacactttcactaacatggaggtccagctaataagacaaatggaatctgaaggaatcttttcacccagcgaattggaaaattc

SEQ ID NO: 1241 - DNA, 120 bp, synthetic construct
  source 1..120: mol_type = other DNA
ccagctaataagacaaatggaatctgaaggaatcttttcacccagcgaattggaaaattcaaatctagctgagagagttctcgactggttggaaaaacatggcgtcgaaaggttgaaaag

SEQ ID NO: 1242 - DNA, 120 bp, synthetic construct
  source 1..120: mol_type = other DNA
aaatctagctgagagagttctcgactggttggaaaaacatggcgtcgaaaggttgaaaagaatggcaatcagcggagatgactgtgtggtgaaaccaactgatgacaggtttgcaacagc

SEQ ID NO: 1243 - DNA, 120 bp, synthetic construct
  source 1..120: mol_type = other DNA
aatggcaatcagcggagatgactgtgtggtgaaaccaactgatgacaggtttgcaacagctttaacagccctgaatgacatgggaaaggtgagaaaagacataccgcaatgggaaccttc

SEQ ID NO: 1244 - DNA, 120 bp, synthetic construct
  source 1..120: mol_type = other DNA
tttaacagccctgaatgacatgggaaaggtgagaaaagacataccgcaatgggaaccttcaaaaggatggaatgactggcagcaagtgcctttctgttcacaccacttccaccaactgat

SEQ ID NO: 1245 - DNA, 120 bp, synthetic construct
  source 1..120: mol_type = other DNA
aaaaggatggaatgactggcagcaagtgcctttctgttcacaccacttccaccaactgatcatgaaggatgggagggagatagtggtgccatgccgcaaccaagatgaacttgtgggcag

SEQ ID NO: 1246 - DNA, 120 bp, synthetic construct
  source 1..120: mol_type = other DNA
catgaaggatgggagggagatagtggtgccatgccgcaaccaagatgaacttgtgggcagggccagagtatcacaaggcgccgggtggagcctgagagaaactgcttgcctaggcaagtc

SEQ ID NO: 1247 - DNA, 120 bp, synthetic construct
  source 1..120: mol_type = other DNA
ggccagagtatcacaaggcgccgggtggagcctgagagaaactgcttgcctaggcaagtcatatgcacaaatgtggcagctgatgtacttccataggagagacctgagactggcggccaa

SEQ ID NO: 1248 - DNA, 120 bp, synthetic construct
  source 1..120: mol_type = other DNA
atatgcacaaatgtggcagctgatgtacttccataggagagacctgagactggcggccaatgctatctgttcagccgttccagttgattgggtcccaaccagccgcaccacctggtcgat

SEQ ID NO: 1249 - DNA, 120 bp, synthetic construct
  source 1..120: mol_type = other DNA
tgctatctgttcagccgttccagttgattgggtcccaaccagccgcaccacctggtcgatccatgcccaccatcaatggatgacaacagaagacatgttgtcagtatggaatagggtttg

SEQ ID NO: 1250 - DNA, 120 bp, synthetic construct
  source 1..120: mol_type = other DNA
ccatgcccaccatcaatggatgacaacagaagacatgttgtcagtatggaatagggtttggatagaggaaaacccatggatggaggacaaaactcatgtatccagctgggaagatgttcc

SEQ ID NO: 1251 - DNA, 120 bp, synthetic construct
  source 1..120: mol_type = other DNA
gatagaggaaaacccatggatggaggacaaaactcatgtatccagctgggaagatgttccatatttaggaaaaagggaagatcaatggtgtggatctctgataggcttaacagcaagagc

SEQ ID NO: 1252 - DNA, 120 bp, synthetic construct
  source 1..120: mol_type = other DNA
atatttaggaaaaagggaagatcaatggtgtggatctctgataggcttaacagcaagagccacctgggccaccaacatacaagtggccataaaccaagtgagaaggcttattgggaatga

SEQ ID NO: 1253 - DNA, 120 bp, synthetic construct
  source 1..120: mol_type = other DNA
cacctgggccaccaacatacaagtggccataaaccaagtgagaaggcttattgggaatgagaattatttagactacatgacatcaatgaagagattcaagaatgagagtgattccgaagg

SEQ ID NO: 1254 - DNA, 120 bp, synthetic construct
  source 1..120: mol_type = other DNA
gaattatttagactacatgacatcaatgaagagattcaagaatgagagtgattccgaaggagccctctggtaagccaacacactcacaaaataaaggaaaataaaaaatcaaacaaggca

SEQ ID NO: 1255 - DNA, 120 bp, synthetic construct
  source 1..120: mol_type = other DNA
agccctctggtaagccaacacactcacaaaataaaggaaaataaaaaatcaaacaaggcaagaagtcaggccggtttaagccatagtacggtaagagctatgctgcctgtgagccccgtc

SEQ ID NO: 1256 - DNA, 120 bp, synthetic construct
  source 1..120: mol_type = other DNA
agaagtcaggccggtttaagccatagtacggtaagagctatgctgcctgtgagccccgtccaaggacgtaaaatgaagtcaggccgaaagccacggcttgagcaaaccgtgctgcctgtg

SEQ ID NO: 1257 - DNA, 120 bp, synthetic construct
  source 1..120: mol_type = other DNA
caaggacgtaaaatgaagtcaggccgaaagccacggcttgagcaaaccgtgctgcctgtggctccatcgtggggatgtaaaaacccgggaggctgcaacccatggaagctgtacgcatgg

SEQ ID NO: 1258 - DNA, 120 bp, synthetic construct
  source 1..120: mol_type = other DNA
gctccatcgtggggatgtaaaaacccgggaggctgcaacccatggaagctgtacgcatggggtagcagactagtggttagaggagacccctcccaagatacaacgcagcagcggggccca

SEQ ID NO: 1259 - DNA, 120 bp, synthetic construct
  source 1..120: mol_type = other DNA
ggtagcagactagtggttagaggagacccctcccaagatacaacgcagcagcggggcccaacaccaggggaagctgtaccctggtggtaaggactagaggttagaggagaccccccgcac

SEQ ID NO: 1260 - DNA, 120 bp, synthetic construct
  source 1..120: mol_type = other DNA
acaccaggggaagctgtaccctggtggtaaggactagaggttagaggagaccccccgcacaacaataaacagcatattgacgctgggagagaccagagatcctgctgtctccacagcatc

SEQ ID NO: 1261 - DNA, 120 bp, synthetic construct
  source 1..120: mol_type = other DNA
cgcacaacaataaacagcatattgacgctgggagagaccagagatcctgctgtctccacagcatcattccaggcacagaacgccagaaaatggaatggtgctgttgaatcaacaggttct

SEQ ID NO: 1262 - DNA, 120 bp, synthetic construct
  source 1..120: mol_type = other DNA
gttctaacagtttttaattagagcgcagatctctgatgaataaccaacggaaaaaggcgagaagtacgcctttcaatatgctgaaacgcgagagaaaccgcgtgtcaactgtgcaacagc

SEQ ID NO: 1263 - DNA, 120 bp, synthetic construct
  source 1..120: mol_type = other DNA
gaagtacgcctttcaatatgctgaaacgcgagagaaaccgcgtgtcaactgtgcaacagctgacaaagagattctcacttggaatgctgcaaggacgcggaccattaaaactgttcatgg

SEQ ID NO: 1264 - DNA, 120 bp, synthetic construct
  source 1..120: mol_type = other DNA
tgacaaagagattctcacttggaatgctgcaaggacgcggaccattaaaactgttcatggcccttgtggcgttccttcgtttcctaacaatcccaccaacagcagggatactaaaaagat

SEQ ID NO: 1265 - DNA, 120 bp, synthetic construct
  source 1..120: mol_type = other DNA
cccttgtggcgttccttcgtttcctaacaatcccaccaacagcagggatactaaaaagatggggaacgatcaaaaaatcaaaagctatcaatgtcttgagagggttcaggaaagagattg

SEQ ID NO: 1266 - DNA, 120 bp, synthetic construct
  source 1..120: mol_type = other DNA
ggggaacgatcaaaaaatcaaaagctatcaatgtcttgagagggttcaggaaagagattggaaggatgctgaacatcttgaataggagacgcaggacagcaggcgtgattgttatgttga

SEQ ID NO: 1267 - DNA, 120 bp, synthetic construct
  source 1..120: mol_type = other DNA
gaaggatgctgaacatcttgaataggagacgcaggacagcaggcgtgattgttatgttgattccaacagcgatggcgttccatttaaccacacgcaatggagaaccacacatgatcgttg

SEQ ID NO: 1268 - DNA, 120 bp, synthetic construct
  source 1..120: mol_type = other DNA
ttccaacagcgatggcgttccatttaaccacacgcaatggagaaccacacatgatcgttggtaggcaggagaaagggaaaagtcttctgttcaaaacagaggatggtgttaacatgtgta

SEQ ID NO: 1269 - DNA, 120 bp, synthetic construct
  source 1..120: mol_type = other DNA
gtaggcaggagaaagggaaaagtcttctgttcaaaacagaggatggtgttaacatgtgtaccctcatggccatagaccttggtgaattgtgtgaagatacaatcacgtacaagtgtcctc

SEQ ID NO: 1270 - DNA, 120 bp, synthetic construct
  source 1..120: mol_type = other DNA
ccctcatggccatagaccttggtgaattgtgtgaagatacaatcacgtacaagtgtcctctcctcagacaaaatgaaccagaagacatagattgttggtgcaactccacgtccacatggg

SEQ ID NO: 1271 - DNA, 120 bp, synthetic construct
  source 1..120: mol_type = other DNA
tcctcagacaaaatgaaccagaagacatagattgttggtgcaactccacgtccacatgggtaacttatgggacatgtaccaccacaggagaacacagaagagaaaaaagatcagtggcgc

SEQ ID NO: 1272 - DNA, 120 bp, synthetic construct
  source 1..120: mol_type = other DNA
taacttatgggacatgtaccaccacaggagaacacagaagagaaaaaagatcagtggcgctcgttccacatgtgggtatgggactggagacacgaactgaaacatggatgtcatcagaag

SEQ ID NO: 1273 - DNA, 120 bp, synthetic construct
  source 1..120: mol_type = other DNA
tcgttccacatgtgggtatgggactggagacacgaactgaaacatggatgtcatcagaaggggcctggaaacatgtccagagaattgaaacctggatcttaagacatccaggctttacca

SEQ ID NO: 1274 - DNA, 120 bp, synthetic construct
  source 1..120: mol_type = other DNA
gggcctggaaacatgtccagagaattgaaacctggatcttaagacatccaggctttaccataatggcagcaatcctggcatacaccataggaacgacacatttccaaaaggccttgattt

SEQ ID NO: 1275 - DNA, 120 bp, synthetic construct
  source 1..120: mol_type = other DNA
taatggcagcaatcctggcatacaccataggaacgacacatttccaaaaggccttgattttcatcttactgacagctgtcgctccttcaatgacaatgcgctgcataggaatatcaaata

SEQ ID NO: 1276 - DNA, 120 bp, synthetic construct
  source 1..120: mol_type = other DNA
tcatcttactgacagctgtcgctccttcaatgacaatgcgctgcataggaatatcaaatagagacttcgtagaaggggtttcaggaggaagctgggttgacatagtcttggaacatggaa

SEQ ID NO: 1277 - DNA, 120 bp, synthetic construct
  source 1..120: mol_type = other DNA
gagacttcgtagaaggggtttcaggaggaagctgggttgacatagtcttggaacatggaagttgtgtgacgacgatggcaaaaaataaaccaacactggattttgaactgataaaaacag

SEQ ID NO: 1278 - DNA, 120 bp, synthetic construct
  source 1..120: mol_type = other DNA
gttgtgtgacgacgatggcaaaaaataaaccaacactggattttgaactgataaaaacagaagccaaacaacctgccactctaaggaagtactgtatagaagcaaagctgaccaacacaa

SEQ ID NO: 1279 - DNA, 120 bp, synthetic construct
  source 1..120: mol_type = other DNA
aagccaaacaacctgccactctaaggaagtactgtatagaagcaaagctgaccaacacaacaacagaatcgcgttgcccaacacaaggggaacccagtctaaatgaagagcaggacaaaa

SEQ ID NO: 1280 - DNA, 120 bp, synthetic construct
  source 1..120: mol_type = other DNA
caacagaatcgcgttgcccaacacaaggggaacccagtctaaatgaagagcaggacaaaaggttcatctgcaaacactccatggtagacagaggatggggaaatggatgtggattatttg

SEQ ID NO: 1281 - DNA, 120 bp, synthetic construct
  source 1..120: mol_type = other DNA
ggttcatctgcaaacactccatggtagacagaggatggggaaatggatgtggattatttggaaagggaggcattgtgacctgtgctatgtttacatgcaaaaagaacatggaaggaaaag

SEQ ID NO: 1282 - DNA, 120 bp, synthetic construct
  source 1..120: mol_type = other DNA
gaaagggaggcattgtgacctgtgctatgtttacatgcaaaaagaacatggaaggaaaagtcgtgcagccagaaaatttggaatacaccatcgtgataacacctcactcaggagaagagc

SEQ ID NO: 1283 - DNA, 120 bp, synthetic construct
  source 1..120: mol_type = other DNA
tcgtgcagccagaaaatttggaatacaccatcgtgataacacctcactcaggagaagagcacgctgtaggcaatgacacaggaaagcatggcaaggaaattaaaataacaccacagagct

SEQ ID NO: 1284 - DNA, 120 bp, synthetic construct
  source 1..120: mol_type = other DNA
acgctgtaggcaatgacacaggaaagcatggcaaggaaattaaaataacaccacagagctccatcacagaagcagaactgacaggctatggcactgtcacgatggagtgctctccgagaa

SEQ ID NO: 1285 - DNA, 120 bp, synthetic construct
  source 1..120: mol_type = other DNA
ccatcacagaagcagaactgacaggctatggcactgtcacgatggagtgctctccgagaacgggcctcgactttaatgagatggtgctgctgcagatggaagacaaagcttggctggtgc

SEQ ID NO: 1286 - DNA, 120 bp, synthetic construct
  source 1..120: mol_type = other DNA
cgggcctcgactttaatgagatggtgctgctgcagatggaagacaaagcttggctggtgcacaggcaatggttcctagacctgccgttaccatggctacctggagcggatacacaaggat

SEQ ID NO: 1287 - DNA, 120 bp, synthetic construct
  source 1..120: mol_type = other DNA
acaggcaatggttcctagacctgccgttaccatggctacctggagcggatacacaaggatcaaattggatacagaaagagacattggtcactttcaaaaatccccacgcgaagaaacagg

SEQ ID NO: 1288 - DNA, 120 bp, synthetic construct
  source 1..120: mol_type = other DNA
caaattggatacagaaagagacattggtcactttcaaaaatccccacgcgaagaaacaggatgtcgtcgttttagggtctcaagaaggggccatgcacacggcactcacaggggccacag

SEQ ID NO: 1289 - DNA, 120 bp, synthetic construct
  source 1..120: mol_type = other DNA
atgtcgtcgttttagggtctcaagaaggggccatgcacacggcactcacaggggccacagaaatccaaatgtcatcaggaaacttactgttcacaggacatctcaagtgcaggctgagaa

SEQ ID NO: 1290 - DNA, 120 bp, synthetic construct
  source 1..120: mol_type = other DNA
aaatccaaatgtcatcaggaaacttactgttcacaggacatctcaagtgcaggctgagaatggacaaactacagctcaaaggaatgtcatactctatgtgtacaggaaagtttaaaattg

SEQ ID NO: 1291 - DNA, 120 bp, synthetic construct
  source 1..120: mol_type = other DNA
tggacaaactacagctcaaaggaatgtcatactctatgtgtacaggaaagtttaaaattgtgaaggaaatagcagaaacacaacatggaacaatagttatcagagtacaatatgaagggg

SEQ ID NO: 1292 - DNA, 120 bp, synthetic construct
  source 1..120: mol_type = other DNA
tgaaggaaatagcagaaacacaacatggaacaatagttatcagagtacaatatgaaggggacggttctccatgcaagatcccttttgagataacagatttggaaaaaagacacgtcttag

SEQ ID NO: 1293 - DNA, 120 bp, synthetic construct
  source 1..120: mol_type = other DNA
acggttctccatgcaagatcccttttgagataacagatttggaaaaaagacacgtcttaggtcgcttgatcacagttaacccaatcgtaacagaaaaagatagcccagtcaacatagaag

SEQ ID NO: 1294 - DNA, 120 bp, synthetic construct
  source 1..120: mol_type = other DNA
gtcgcttgatcacagttaacccaatcgtaacagaaaaagatagcccagtcaacatagaagcagaacctccatttggagacagctacatcatcataggagtagagccgggacaattgaaac

SEQ ID NO: 1295 - DNA, 120 bp, synthetic construct
  source 1..120: mol_type = other DNA
cagaacctccatttggagacagctacatcatcataggagtagagccgggacaattgaaactcaattggtttaagaagggaagttccatcggccaaatgtttgagacaacaatgagaggag

SEQ ID NO: 1296 - DNA, 120 bp, synthetic construct
  source 1..120: mol_type = other DNA
tcaattggtttaagaagggaagttccatcggccaaatgtttgagacaacaatgagaggagcaaagagaatggccattttaggtgacacagcctgggactttggatccctgggaggagtgt

SEQ ID NO: 1297 - DNA, 120 bp, synthetic construct
  source 1..120: mol_type = other DNA
caaagagaatggccattttaggtgacacagcctgggactttggatccctgggaggagtgtttacatccataggaaaggctctccaccaagttttcggagcaatctatggggctgctttta

SEQ ID NO: 1298 - DNA, 120 bp, synthetic construct
  source 1..120: mol_type = other DNA
ttacatccataggaaaggctctccaccaagttttcggagcaatctatggggctgcttttagtggggtctcatggactatgaaaatcctcataggagtcatcatcacatggataggaatga

SEQ ID NO: 1299 - DNA, 120 bp, synthetic construct
  source 1..120: mol_type = other DNA
gtggggtctcatggactatgaaaatcctcataggagtcatcatcacatggataggaatgaattcacgtagcacctcactgtctgtatcgctagtattggtgggcgtcgtgacattgtacc

SEQ ID NO: 1300 - DNA, 120 bp, synthetic construct
  source 1..120: mol_type = other DNA
attcacgtagcacctcactgtctgtatcgctagtattggtgggcgtcgtgacattgtacctgggagctatggtgcaagctgatagtggttgcgttgtgagctggaaaaacaaagaactga

SEQ ID NO: 1301 - DNA, 120 bp, synthetic construct
  source 1..120: mol_type = other DNA
tgggagctatggtgcaagctgatagtggttgcgttgtgagctggaaaaacaaagaactgaaatgtggcagcgggatcttcattacagataacgtacacacatggacagaacaatacaagt

SEQ ID NO: 1302 - DNA, 120 bp, synthetic construct
  source 1..120: mol_type = other DNA
aatgtggcagcgggatcttcattacagataacgtacacacatggacagaacaatacaagttccaaccagaatccccttcaaaactagcttcagctatccaaaaagctcatgaagagggca

SEQ ID NO: 1303 - DNA, 120 bp, synthetic construct
  source 1..120: mol_type = other DNA
tccaaccagaatccccttcaaaactagcttcagctatccaaaaagctcatgaagagggcatttgtggaatccgctcagtaacaagattggagaatctgatgtggaaacaaataacaccag

SEQ ID NO: 1304 - DNA, 120 bp, synthetic construct
  source 1..120: mol_type = other DNA
tttgtggaatccgctcagtaacaagattggagaatctgatgtggaaacaaataacaccagaattgaatcatattctatcagaaaatgaggtaaagttgaccattatgacaggagacatta

SEQ ID NO: 1305 - DNA, 120 bp, synthetic construct
  source 1..120: mol_type = other DNA
aattgaatcatattctatcagaaaatgaggtaaagttgaccattatgacaggagacattaaaggaatcatgcaggcaggaaaacgatccttgcggccccagcccactgagctgaagtact

SEQ ID NO: 1306 - DNA, 120 bp, synthetic construct
  source 1..120: mol_type = other DNA
aaggaatcatgcaggcaggaaaacgatccttgcggccccagcccactgagctgaagtactcatggaaaacatggggaaaggcgaaaatgctctccacagagtctcacaatcagacctttc

SEQ ID NO: 1307 - DNA, 120 bp, synthetic construct
  source 1..120: mol_type = other DNA
catggaaaacatggggaaaggcgaaaatgctctccacagagtctcacaatcagacctttcttattgatggccctgaaacagcagaatgccccaacacaaacagagcttggaactcgctgg

SEQ ID NO: 1308 - DNA, 120 bp, synthetic construct
  source 1..120: mol_type = other DNA
ttattgatggccctgaaacagcagaatgccccaacacaaacagagcttggaactcgctggaagttgaagactatggttttggagttttcaccaccaatatatggctgaaattgagagaaa

SEQ ID NO: 1309 - DNA, 120 bp, synthetic construct
  source 1..120: mol_type = other DNA
aagttgaagactatggttttggagttttcaccaccaatatatggctgaaattgagagaaaaacaggatgtattttgtgactcaaaactcatgtcagcagccattaaagacaatagagccg

SEQ ID NO: 1310 - DNA, 120 bp, synthetic construct
  source 1..120: mol_type = other DNA
aacaggatgtattttgtgactcaaaactcatgtcagcagccattaaagacaatagagccgttcatgccgatatgggttattggatagaaagtgcactcaatgacacatggaagatggaga

SEQ ID NO: 1311 - DNA, 120 bp, synthetic construct
  source 1..120: mol_type = other DNA
ttcatgccgatatgggttattggatagaaagtgcactcaatgacacatggaagatggagaaagcctccttcattgaagttaaaagctgccactggccaaagtcacacaccctttggagca

SEQ ID NO: 1312 - DNA, 120 bp, synthetic construct
  source 1..120: mol_type = other DNA
aagcctccttcattgaagttaaaagctgccactggccaaagtcacacaccctttggagcaatggagtattagaaagtgagatgataatcccaaaaaattttgccgggccagtgtcacaac

SEQ ID NO: 1313 - DNA, 120 bp, synthetic construct
  source 1..120: mol_type = other DNA
atggagtattagaaagtgagatgataatcccaaaaaattttgccgggccagtgtcacaacacaactacagaccaggctaccatacacaaacagcaggaccttggcatctaggtaagcttg

SEQ ID NO: 1314 - DNA, 120 bp, synthetic construct
  source 1..120: mol_type = other DNA
acaactacagaccaggctaccatacacaaacagcaggaccttggcatctaggtaagcttgagatggactttgatctctgcgaaggaactacagtggtggtgactgaggactgtggaaata

SEQ ID NO: 1315 - DNA, 120 bp, synthetic construct
  source 1..120: mol_type = other DNA
agatggactttgatctctgcgaaggaactacagtggtggtgactgaggactgtggaaatagaggaccctctttaagaacgaccactgcctctggaaaactcataacagaatggtgctgcc

SEQ ID NO: 1316 - DNA, 120 bp, synthetic construct
  source 1..120: mol_type = other DNA
gaggaccctctttaagaacgaccactgcctctggaaaactcataacagaatggtgctgccgatcctgcacactaccacctctaagatacagaggtgaggatggatgctggtacgggatgg

SEQ ID NO: 1317 - DNA, 120 bp, synthetic construct
  source 1..120: mol_type = other DNA
gatcctgcacactaccacctctaagatacagaggtgaggatggatgctggtacgggatggaaatcagaccattgaaagagaaagaggagaatttggtcaactccttggtcacagccggac

SEQ ID NO: 1318 - DNA, 120 bp, synthetic construct
  source 1..120: mol_type = other DNA
aaatcagaccattgaaagagaaagaggagaatttggtcaactccttggtcacagccggacatgggcagattgataacttttcactaggagtcttgggaatggcactgttcctggaagaaa

SEQ ID NO: 1319 - DNA, 120 bp, synthetic construct
  source 1..120: mol_type = other DNA
atgggcagattgataacttttcactaggagtcttgggaatggcactgttcctggaagaaatgctcaggacccgaataggaacgaaacatgcaatactgctagtcgcagtatcttttgtga

SEQ ID NO: 1320 - DNA, 120 bp, synthetic construct
  source 1..120: mol_type = other DNA
tgctcaggacccgaataggaacgaaacatgcaatactgctagtcgcagtatcttttgtgacattgattactgggaacatgtcttttagagacctgggaagagtgatggttatggtgggcg

SEQ ID NO: 1321 - DNA, 120 bp, synthetic construct
  source 1..120: mol_type = other DNA
cattgattactgggaacatgtcttttagagacctgggaagagtgatggttatggtgggcgctaccatgacggatgacataggtatgggagtgacttatcttgccctactagcagctttta

SEQ ID NO: 1322 - DNA, 120 bp, synthetic construct
  source 1..120: mol_type = other DNA
ctaccatgacggatgacataggtatgggagtgacttatcttgccctactagcagcttttaaagttagaccaacttttgcagctggactactcttgagaaaactgacctccaaggaattga

SEQ ID NO: 1323 - DNA, 120 bp, synthetic construct
  source 1..120: mol_type = other DNA
aagttagaccaacttttgcagctggactactcttgagaaaactgacctccaaggaattgatgatggccaccataggaatcgcacttctttcccaaagcaccataccagagaccattcttg

SEQ ID NO: 1324 - DNA, 120 bp, synthetic construct
  source 1..120: mol_type = other DNA
tgatggccaccataggaatcgcacttctttcccaaagcaccataccagagaccattcttgaactgaccgatgcattagccttgggcatgatggtcctcaaaatagtgagaaatatggaaa

SEQ ID NO: 1325 - DNA, 120 bp, synthetic construct
  source 1..120: mol_type = other DNA
aactgaccgatgcattagccttgggcatgatggtcctcaaaatagtgagaaatatggaaaaataccaattggcagtgactatcatggctatttcatgtgtcccaaatgcagtgatactgc

SEQ ID NO: 1326 - DNA, 120 bp, synthetic construct
  source 1..120: mol_type = other DNA
aataccaattggcagtgactatcatggctatttcatgtgtcccaaatgcagtgatactgcaaaacgcatggaaggtgagctgcacaatattggcagcggtgtccgtttcaccactgctct

SEQ ID NO: 1327 - DNA, 120 bp, synthetic construct
  source 1..120: mol_type = other DNA
aaaacgcatggaaggtgagctgcacaatattggcagcggtgtccgtttcaccactgctcttaacatcctcacagcagaaagcggattggataccactggcattgacgataaaaggtctca

SEQ ID NO: 1328 - DNA, 120 bp, synthetic construct
  source 1..120: mol_type = other DNA
taacatcctcacagcagaaagcggattggataccactggcattgacgataaaaggtctcaatccaacagccatttttctaacaactctttcgagaaccagcaaaaaaaggagctggccgc

SEQ ID NO: 1329 - DNA, 120 bp, synthetic construct
  source 1..120: mol_type = other DNA
atccaacagccatttttctaacaactctttcgagaaccagcaaaaaaaggagctggccgctaaatgaagctatcatggcagtcgggatggtgagcattttagccagttctctcctaaaga

SEQ ID NO: 1330 - DNA, 120 bp, synthetic construct
  source 1..120: mol_type = other DNA
taaatgaagctatcatggcagtcgggatggtgagcattttagccagttctctcctaaagaatgatattcccatgacaggtccattagtggctggagggctccttaccgtatgttacgtgc

SEQ ID NO: 1331 - DNA, 120 bp, synthetic construct
  source 1..120: mol_type = other DNA
atgatattcccatgacaggtccattagtggctggagggctccttaccgtatgttacgtgctcactggacgatcggccgatttggaactggagagagctgccgatgtaaaatgggaagatc

SEQ ID NO: 1332 - DNA, 120 bp, synthetic construct
  source 1..120: mol_type = other DNA
tcactggacgatcggccgatttggaactggagagagctgccgatgtaaaatgggaagatcaggcagaaatatcaggaagcagcccaatcctatcaataacaatatcagaagatggcagca

SEQ ID NO: 1333 - DNA, 120 bp, synthetic construct
  source 1..120: mol_type = other DNA
aggcagaaatatcaggaagcagcccaatcctatcaataacaatatcagaagatggcagcatgtcgataaaaaatgaagaggaagaacaaacactgaccatactcatcagaacgggattgt

SEQ ID NO: 1334 - DNA, 120 bp, synthetic construct
  source 1..120: mol_type = other DNA
tgtcgataaaaaatgaagaggaagaacaaacactgaccatactcatcagaacgggattgttggtgatctcaggagtctttccagtatcgataccaattacggcagcagcatggtacctgt

SEQ ID NO: 1335 - DNA, 120 bp, synthetic construct
  source 1..120: mol_type = other DNA
tggtgatctcaggagtctttccagtatcgataccaattacggcagcagcatggtacctgtgggaagtgaagaaacaacgggctggagtattgtgggacgtcccttcacccccaccagtgg

SEQ ID NO: 1336 - DNA, 120 bp, synthetic construct
  source 1..120: mol_type = other DNA
gggaagtgaagaaacaacgggctggagtattgtgggacgtcccttcacccccaccagtggaaaaagccgaactggaggatggagcctacagaatcaagcaaagagggattcttggatatt

SEQ ID NO: 1337 - DNA, 120 bp, synthetic construct
  source 1..120: mol_type = other DNA
aaaaagccgaactggaggatggagcctacagaatcaagcaaagagggattcttggatattctcagatcggagccggagtttacaaagaaggaacattccatacaatgtggcacgtcacac

SEQ ID NO: 1338 - DNA, 120 bp, synthetic construct
  source 1..120: mol_type = other DNA
ctcagatcggagccggagtttacaaagaaggaacattccatacaatgtggcacgtcacacgtggtgctgttctgatgcatagagggaagaggattgaaccatcatgggcagacgtcaaga

SEQ ID NO: 1339 - DNA, 120 bp, synthetic construct
  source 1..120: mol_type = other DNA
gtggtgctgttctgatgcatagagggaagaggattgaaccatcatgggcagacgtcaagaaagacctaatatcatatggaggaggttggaagctagaaggagaatggaaggaaggagagg

SEQ ID NO: 1340 - DNA, 120 bp, synthetic construct
  source 1..120: mol_type = other DNA
aagacctaatatcatatggaggaggttggaagctagaaggagaatggaaggaaggagaggaagtccaagtcctggcactggaacctgggaaaaatccaagagcagtccaaacgaaacctg

SEQ ID NO: 1341 - DNA, 120 bp, synthetic construct
  source 1..120: mol_type = other DNA
aagtccaagtcctggcactggaacctgggaaaaatccaagagcagtccaaacgaaacctggaattttcaaaaccaacaccggaaccataggcgccgtatctctggacttttcccctggaa

SEQ ID NO: 1342 - DNA, 120 bp, synthetic construct
  source 1..120: mol_type = other DNA
gaattttcaaaaccaacaccggaaccataggcgccgtatctctggacttttcccctggaacgtcaggatctccaattgtcgacagaaaaggaaaagttgtgggtctttacggtaatggtg

SEQ ID NO: 1343 - DNA, 120 bp, synthetic construct
  source 1..120: mol_type = other DNA
cgtcaggatctccaattgtcgacagaaaaggaaaagttgtgggtctttacggtaatggtgttgtcacaaggagtggagcatatgtaagtgccatagcccagacagaaaaaagcattgaag

SEQ ID NO: 1344 - DNA, 120 bp, synthetic construct
  source 1..120: mol_type = other DNA
ttgtcacaaggagtggagcatatgtaagtgccatagcccagacagaaaaaagcattgaagacaatccagagatcgaagatgacattttccgaaagaaaagattgaccatcatggacctcc

SEQ ID NO: 1345 - DNA, 120 bp, synthetic construct
  source 1..120: mol_type = other DNA
acaatccagagatcgaagatgacattttccgaaagaaaagattgaccatcatggacctccatccaggagcaggaaagacaaaaagataccttccagccatagttagagaagccataaaac

SEQ ID NO: 1346 - DNA, 120 bp, synthetic construct
  source 1..120: mol_type = other DNA
atccaggagcaggaaagacaaaaagataccttccagccatagttagagaagccataaaacgtggcttgagaacattgatcctggctcccactagagtagtggcagctgaaatggaggaag

SEQ ID NO: 1347 - DNA, 120 bp, synthetic construct
  source 1..120: mol_type = other DNA
gtggcttgagaacattgatcctggctcccactagagtagtggcagctgaaatggaggaagctcttagaggacttccaataagataccaaaccccagccatcaaaacccagcatactgggc

SEQ ID NO: 1348 - DNA, 120 bp, synthetic construct
  source 1..120: mol_type = other DNA
ctcttagaggacttccaataagataccaaaccccagccatcaaaacccagcatactgggcgggagatcgtggacctaatgtgtcatgccacatttactatgaggctactatcaccagtca

SEQ ID NO: 1349 - DNA, 120 bp, synthetic construct
  source 1..120: mol_type = other DNA
gggagatcgtggacctaatgtgtcatgccacatttactatgaggctactatcaccagtcagagtaccaaattacaacctgatcatcatggacgaagcccacttcacagacccagcaagta

SEQ ID NO: 1350 - DNA, 120 bp, synthetic construct
  source 1..120: mol_type = other DNA
gagtaccaaattacaacctgatcatcatggacgaagcccacttcacagacccagcaagtatagcagctagaggatacatttcaactcgagtagagatgggtgaagcagccgggattttca

SEQ ID NO: 1351 - DNA, 120 bp, synthetic construct
  source 1..120: mol_type = other DNA
tagcagctagaggatacatttcaactcgagtagagatgggtgaagcagccgggattttcatgacagccactcctccgggaagtagagacccatttcctcagagcaatgcaccaatcatgg

SEQ ID NO: 1352 - DNA, 120 bp, synthetic construct
  source 1..120: mol_type = other DNA
tgacagccactcctccgggaagtagagacccatttcctcagagcaatgcaccaatcatggatgaggaaagagaaattcctgagcgttcgtggaattcaggacacgaatgggtcacagatt

SEQ ID NO: 1353 - DNA, 120 bp, synthetic construct
  source 1..120: mol_type = other DNA
atgaggaaagagaaattcctgagcgttcgtggaattcaggacacgaatgggtcacagattttaaggggaagactgtttggtttgttccaagtataaaagcaggaaatgatatagcagctt

SEQ ID NO: 1354 - DNA, 120 bp, synthetic construct
  source 1..120: mol_type = other DNA
ttaaggggaagactgtttggtttgttccaagtataaaagcaggaaatgatatagcagcttgtcttaggaaaaatggaaagaaagtgatacaactcagtaggaagacttttgactctgagt

SEQ ID NO: 1355 - DNA, 120 bp, synthetic construct
  source 1..120: mol_type = other DNA
gtcttaggaaaaatggaaagaaagtgatacaactcagtaggaagacttttgactctgagtatgtcaagactagagccaatgattgggactttgtggtcacaactgacatttcagaaatgg

SEQ ID NO: 1356 - DNA, 120 bp, synthetic construct
  source 1..120: mol_type = other DNA
atgtcaagactagagccaatgattgggactttgtggtcacaactgacatttcagaaatgggtgccaactttaaggctgagagggttatagaccccagacgttgcatgaaaccagttatac

SEQ ID NO: 1357 - DNA, 120 bp, synthetic construct
  source 1..120: mol_type = other DNA
gtgccaactttaaggctgagagggttatagaccccagacgttgcatgaaaccagttatactaacagatggcgaagagcgggtgatcttggcaggaccaatgccagtgacccactctagtg

SEQ ID NO: 1358 - DNA, 120 bp, synthetic construct
  source 1..120: mol_type = other DNA
taacagatggcgaagagcgggtgatcttggcaggaccaatgccagtgacccactctagtgcagcgcaaagaagagggagaataggaagaaatccaaagaatgaaaatgaccagtacatat

SEQ ID NO: 1359 - DNA, 120 bp, synthetic construct
  source 1..120: mol_type = other DNA
cagcgcaaagaagagggagaataggaagaaatccaaagaatgaaaatgaccagtacatatatatgggggaacctcttgaaaatgatgaagactgtgcacattggaaagaagctaaaatgc

SEQ ID NO: 1360 - DNA, 120 bp, synthetic construct
  source 1..120: mol_type = other DNA
atatgggggaacctcttgaaaatgatgaagactgtgcacattggaaagaagctaaaatgctcctagataacatcaacacacccgaaggaatcattcctagtatgttcgaaccagagcgtg

SEQ ID NO: 1361 - DNA, 120 bp, synthetic construct
  source 1..120: mol_type = other DNA
tcctagataacatcaacacacccgaaggaatcattcctagtatgttcgaaccagagcgtgaaaaagtggatgccattgatggtgaataccgcttgagaggagaagcaaggaaaacttttg

SEQ ID NO: 1362 - DNA, 120 bp, synthetic construct
  source 1..120: mol_type = other DNA
aaaaagtggatgccattgatggtgaataccgcttgagaggagaagcaaggaaaacttttgtggacctaatgagaagaggggacttaccagtctggttggcctacaaagtggcagctgaag

SEQ ID NO: 1363 - DNA, 120 bp, synthetic construct
  source 1..120: mol_type = other DNA
tggacctaatgagaagaggggacttaccagtctggttggcctacaaagtggcagctgaaggcatcaactacgcagacagaaagtggtgttttgatggaatcaagaacaaccaaatactgg

SEQ ID NO: 1364 - DNA, 120 bp, synthetic construct
  source 1..120: mol_type = other DNA
gcatcaactacgcagacagaaagtggtgttttgatggaatcaagaacaaccaaatactggaagaaaatatagaagtggaaatctggacaaaagaaggggagaggaaaaaattaaaaccca

SEQ ID NO: 1365 - DNA, 120 bp, synthetic construct
  source 1..120: mol_type = other DNA
aagaaaatatagaagtggaaatctggacaaaagaaggggagaggaaaaaattaaaacccagatggttggatgctaggatctactctgacccactggcactaaaagaattcaaggaatttg

SEQ ID NO: 1366 - DNA, 120 bp, synthetic construct
  source 1..120: mol_type = other DNA
gatggttggatgctaggatctactctgacccactggcactaaaagaattcaaggaatttgcagctggaagaaaatctctgaccctgaacctaatcacagaaatgggtaggcttccaactt

SEQ ID NO: 1367 - DNA, 120 bp, synthetic construct
  source 1..120: mol_type = other DNA
cagctggaagaaaatctctgaccctgaacctaatcacagaaatgggtaggcttccaactttcatgactcagaaagcaagaaacgcactggacaacttggctgtgctgcatacggctgagg

SEQ ID NO: 1368 - DNA, 120 bp, synthetic construct
  source 1..120: mol_type = other DNA
tcatgactcagaaagcaagaaacgcactggacaacttggctgtgctgcatacggctgaggcaggtggaagggcgtacaatcatgctctcagtgaactgccggagaccctggaaacactgc

SEQ ID NO: 1369 - DNA, 120 bp, synthetic construct
  source 1..120: mol_type = other DNA
caggtggaagggcgtacaatcatgctctcagtgaactgccggagaccctggaaacactgcttctactgacactcctggcaacagtcacaggaggaatcttcttattcttaatgagcggaa

SEQ ID NO: 1370 - DNA, 120 bp, synthetic construct
  source 1..120: mol_type = other DNA
ttctactgacactcctggcaacagtcacaggaggaatcttcttattcttaatgagcggaaaaggtgtagggaagatgaccctgggaatgtgttgcataatcacggctagtatcctcctat

SEQ ID NO: 1371 - DNA, 120 bp, synthetic construct
  source 1..120: mol_type = other DNA
aaggtgtagggaagatgaccctgggaatgtgttgcataatcacggctagtatcctcctatggtatgcacagatacaaccacactggatagcagcttcaataatactggagttttttctca

SEQ ID NO: 1372 - DNA, 120 bp, synthetic construct
  source 1..120: mol_type = other DNA
ggtatgcacagatacaaccacactggatagcagcttcaataatactggagttttttctcatagttttgctcattccagaaccagaaaaacagagaacaccccaagacaaccaattgacct

SEQ ID NO: 1373 - DNA, 120 bp, synthetic construct
  source 1..120: mol_type = other DNA
tagttttgctcattccagaaccagaaaaacagagaacaccccaagacaaccaattgacctacgttgtcatagctattctcacagtggtggccgcaaccatggcaaacgagatgggttttc

SEQ ID NO: 1374 - DNA, 120 bp, synthetic construct
  source 1..120: mol_type = other DNA
acgttgtcatagctattctcacagtggtggccgcaaccatggcaaacgagatgggttttctagaaaaaaccaagaaagacctcggattgggaagcatcacaacccaggaacctgagagca

SEQ ID NO: 1375 - DNA, 120 bp, synthetic construct
  source 1..120: mol_type = other DNA
tagaaaaaaccaagaaagacctcggattgggaagcatcacaacccaggaacctgagagcaatatcctggacatagatctacgccctgcatcagcatggacgctgtatgccgtggctacaa

SEQ ID NO: 1376 - DNA, 120 bp, synthetic construct
  source 1..120: mol_type = other DNA
atatcctggacatagatctacgccctgcatcagcatggacgctgtatgccgtggctacaacatttgtcacaccaatgttgagacatagcattgaaaattcctcagtgaatgtctccctaa

SEQ ID NO: 1377 - DNA, 120 bp, synthetic construct
  source 1..120: mol_type = other DNA
catttgtcacaccaatgttgagacatagcattgaaaattcctcagtgaatgtctccctaacagccattgctaaccaagctacagtgctaatgggtcttgggaaaggatggccattgtcaa

SEQ ID NO: 1378 - DNA, 120 bp, synthetic construct
  source 1..120: mol_type = other DNA
cagccattgctaaccaagctacagtgctaatgggtcttgggaaaggatggccattgtcaaagatggacattggagttcccctccttgccattggatgctattcacaagtcaaccctataa

SEQ ID NO: 1379 - DNA, 120 bp, synthetic construct
  source 1..120: mol_type = other DNA
agatggacattggagttcccctccttgccattggatgctattcacaagtcaaccctataactctcacagcagctcttcttttattggtagcacattatgccattatagggccaggacttc

SEQ ID NO: 1380 - DNA, 120 bp, synthetic construct
  source 1..120: mol_type = other DNA
ctctcacagcagctcttcttttattggtagcacattatgccattatagggccaggacttcaagcaaaagcaaccagagaagctcagaaaagagcagcagcaggcatcatgaaaaacccaa

SEQ ID NO: 1381 - DNA, 120 bp, synthetic construct
  source 1..120: mol_type = other DNA
aagcaaaagcaaccagagaagctcagaaaagagcagcagcaggcatcatgaaaaacccaacagtagatggaataacagtgattgacctagaaccaataccctatgatccaaaatttgaaa

SEQ ID NO: 1382 - DNA, 120 bp, synthetic construct
  source 1..120: mol_type = other DNA
cagtagatggaataacagtgattgacctagaaccaataccctatgatccaaaatttgaaaagcagttaggacaagtaatgctcctaattctctgcgtgactcaagtattaatgatgagga

SEQ ID NO: 1383 - DNA, 120 bp, synthetic construct
  source 1..120: mol_type = other DNA
agcagttaggacaagtaatgctcctaattctctgcgtgactcaagtattaatgatgaggactacatgggctctatgtgaggctctaaccttagcgaccgggcctatctccacactgtggg

SEQ ID NO: 1384 - DNA, 120 bp, synthetic construct
  source 1..120: mol_type = other DNA
ctacatgggctctatgtgaggctctaaccttagcgaccgggcctatctccacactgtgggaaggaaatccagggaggttttggaacactaccattgcagtgtcaatggctaacatcttta

SEQ ID NO: 1385 - DNA, 120 bp, synthetic construct
  source 1..120: mol_type = other DNA
aaggaaatccagggaggttttggaacactaccattgcagtgtcaatggctaacatctttagggggagctacttggccggagctggacttctcttttccatcatgaaaaacacaacaaaca

SEQ ID NO: 1386 - DNA, 120 bp, synthetic construct
  source 1..120: mol_type = other DNA
gggggagctacttggccggagctggacttctcttttccatcatgaaaaacacaacaaacacaagaagaggaactggcaacataggagagacacttggagaaaaatggaaaagtcgattaa

SEQ ID NO: 1387 - DNA, 120 bp, synthetic construct
  source 1..120: mol_type = other DNA
caagaagaggaactggcaacataggagagacacttggagaaaaatggaaaagtcgattaaacgcattgggaaaaagtgaatttcaagtctacaagaaaagtggaatccaggaagtggata

SEQ ID NO: 1388 - DNA, 120 bp, synthetic construct
  source 1..120: mol_type = other DNA
acgcattgggaaaaagtgaatttcaagtctacaagaaaagtggaatccaggaagtggatagaaccctagcaaaagaaggtatcaaaagaggagaaacggaccaccatgctgtgtcgcgag

SEQ ID NO: 1389 - DNA, 120 bp, synthetic construct
  source 1..120: mol_type = other DNA
gaaccctagcaaaagaaggtatcaaaagaggagaaacggaccaccatgctgtgtcgcgaggttcagctaaactgagatggttcgtcgagagaaatatggtcacaccggaagggaaggtgg

SEQ ID NO: 1390 - DNA, 120 bp, synthetic construct
  source 1..120: mol_type = other DNA
gttcagctaaactgagatggttcgtcgagagaaatatggtcacaccggaagggaaggtggtggatctcggttgcggcagagggggctggtcatactattgtgggggactaaagaatgtaa

SEQ ID NO: 1391 - DNA, 120 bp, synthetic construct
  source 1..120: mol_type = other DNA
tggatctcggttgcggcagagggggctggtcatactattgtgggggactaaagaatgtaagagaagtcaaaggcctaacaaaaggaggaccaggacatgaagaacccatccccatgtcaa

SEQ ID NO: 1392 - DNA, 120 bp, synthetic construct
  source 1..120: mol_type = other DNA
gagaagtcaaaggcctaacaaaaggaggaccaggacatgaagaacccatccccatgtcaacatatgggtggaatctagtgcgtttgcaaagtggagttgacgttttcttcaccccgccag

SEQ ID NO: 1393 - DNA, 120 bp, synthetic construct
  source 1..120: mol_type = other DNA
catatgggtggaatctagtgcgtttgcaaagtggagttgacgttttcttcaccccgccagaaaagtgtgatacattgttgtgtgacataggggagtcgtcgccaaatcccacgatagaag

SEQ ID NO: 1394 - DNA, 120 bp, synthetic construct
  source 1..120: mol_type = other DNA
aaaagtgtgatacattgttgtgtgacataggggagtcgtcgccaaatcccacgatagaagcaggacgaacactcagagtcctcaacttagtggaaaattggttgaataataacacccaat

SEQ ID NO: 1395 - DNA, 120 bp, synthetic construct
  source 1..120: mol_type = other DNA
caggacgaacactcagagtcctcaacttagtggaaaattggttgaataataacacccaattttgcataaaggtcctcaacccatatatgccttcagtcatagaaaaaatggaagcattac

SEQ ID NO: 1396 - DNA, 120 bp, synthetic construct
  source 1..120: mol_type = other DNA
tttgcataaaggtcctcaacccatatatgccttcagtcatagaaaaaatggaagcattacaaaggaaatatggaggagccttagtgaggaatccactctcacgaaactccacgcatgaaa

SEQ ID NO: 1397 - DNA, 120 bp, synthetic construct
  source 1..120: mol_type = other DNA
aaaggaaatatggaggagccttagtgaggaatccactctcacgaaactccacgcatgaaatgtactgggtatctaatgccaccgggaacatagtgtcatcagtgaacatgatttcaagga

SEQ ID NO: 1398 - DNA, 120 bp, synthetic construct
  source 1..120: mol_type = other DNA
tgtactgggtatctaatgccaccgggaacatagtgtcatcagtgaacatgatttcaaggatgttgattaacagattcacaatgaaacacaagaaagccacttacgagccagatgttgacc

SEQ ID NO: 1399 - DNA, 120 bp, synthetic construct
  source 1..120: mol_type = other DNA
tgttgattaacagattcacaatgaaacacaagaaagccacttacgagccagatgttgacctaggaagtggaacccgcaacattggagttgaaagtgagataccaaatctagacataatag

SEQ ID NO: 1400 - DNA, 120 bp, synthetic construct
  source 1..120: mol_type = other DNA
taggaagtggaacccgcaacattggagttgaaagtgagataccaaatctagacataataggaaagagaatagagaaaataaaacaagagcatgaaacatcatggcactatgatcaagatc

SEQ ID NO: 1401 - DNA, 120 bp, synthetic construct
  source 1..120: mol_type = other DNA
gaaagagaatagagaaaataaaacaagagcatgaaacatcatggcactatgatcaagatcacccatacaaaacgtgggcttaccacggcagctatgaaacaaaacaaactggatcagcat

SEQ ID NO: 1402 - DNA, 120 bp, synthetic construct
  source 1..120: mol_type = other DNA
acccatacaaaacgtgggcttaccacggcagctatgaaacaaaacaaactggatcagcatcatctatggtgaacggagtggtcagattgctgacaaaaccttgggacgtcgtccctatgg

SEQ ID NO: 1403 - DNA, 120 bp, synthetic construct
  source 1..120: mol_type = other DNA
catctatggtgaacggagtggtcagattgctgacaaaaccttgggacgtcgtccctatggtgacacagatggcaatgacggacacgactccatttggacaacagcgcgttttcaaagaga

SEQ ID NO: 1404 - DNA, 120 bp, synthetic construct
  source 1..120: mol_type = other DNA
tgacacagatggcaatgacggacacgactccatttggacaacagcgcgttttcaaagagaaagtagacacgagaacccaggaaccgaaggaaggcacaaagaaactgatgaaaattacgg

SEQ ID NO: 1405 - DNA, 120 bp, synthetic construct
  source 1..120: mol_type = other DNA
aagtagacacgagaacccaggaaccgaaggaaggcacaaagaaactgatgaaaattacggcagagtggctttggaaagaactaggaaagaaaaagacacctaggatgtgtaccagagaag

SEQ ID NO: 1406 - DNA, 120 bp, synthetic construct
  source 1..120: mol_type = other DNA
cagagtggctttggaaagaactaggaaagaaaaagacacctaggatgtgtaccagagaagaattcacaagaaaagtgagaagcaatgcagccttgggggccatattcactgatgagaaca

SEQ ID NO: 1407 - DNA, 120 bp, synthetic construct
  source 1..120: mol_type = other DNA
aattcacaagaaaagtgagaagcaatgcagccttgggggccatattcactgatgagaacaaatggaaatcggcacgtgaggctgttgaagatggtaggttttgggagctggttgacaggg

SEQ ID NO: 1408 - DNA, 120 bp, synthetic construct
  source 1..120: mol_type = other DNA
aatggaaatcggcacgtgaggctgttgaagatggtaggttttgggagctggttgacagggaaagaaatctccatcttgaagggaagtgtgaaacatgtgtgtacaacatgatgggaaaaa

SEQ ID NO: 1409 - DNA, 120 bp, synthetic construct
  source 1..120: mol_type = other DNA
aaagaaatctccatcttgaagggaagtgtgaaacatgtgtgtacaacatgatgggaaaaagagagaagaaactaggggagttcggcaaggcaaaaggtagcagagccatatggtacatgt

SEQ ID NO: 1410 - DNA, 120 bp, synthetic construct
  source 1..120: mol_type = other DNA
gagagaagaaactaggggagttcggcaaggcaaaaggtagcagagccatatggtacatgtggcttggagcacgcttcttagagtttgaagccctaggattcctgaatgaagatcactggt

SEQ ID NO: 1411 - DNA, 120 bp, synthetic construct
  source 1..120: mol_type = other DNA
ggcttggagcacgcttcttagagtttgaagccctaggattcctgaatgaagatcactggttctccagagggaactccctgagtggagtggaaggagaagggctgcacagactaggctata

SEQ ID NO: 1412 - DNA, 120 bp, synthetic construct
  source 1..120: mol_type = other DNA
tctccagagggaactccctgagtggagtggaaggagaagggctgcacagactaggctatattttaagagacgtgggcaagaaggaagggggagcaatgtacgccgatgatacagcaggat

SEQ ID NO: 1413 - DNA, 120 bp, synthetic construct
  source 1..120: mol_type = other DNA
ttttaagagacgtgggcaagaaggaagggggagcaatgtacgccgatgatacagcaggatgggacacaagaatcacactagaagacttaaaaaatgaagaaatggtaacaaaccacatga

SEQ ID NO: 1414 - DNA, 120 bp, synthetic construct
  source 1..120: mol_type = other DNA
gggacacaagaatcacactagaagacttaaaaaatgaagaaatggtaacaaaccacatgaaaggagaacacaagaaactagccgaggccatattcaaactaacgtaccaaaacaaggtgg

SEQ ID NO: 1415 - DNA, 120 bp, synthetic construct
  source 1..120: mol_type = other DNA
aaggagaacacaagaaactagccgaggccatattcaaactaacgtaccaaaacaaggtggtgcgtgtgcaaagaccaacgccaagaggcacagtaatggatatcatatcgagaagagacc

SEQ ID NO: 1416 - DNA, 120 bp, synthetic construct
  source 1..120: mol_type = other DNA
tgcgtgtgcaaagaccaacgccaagaggcacagtaatggatatcatatcgagaagagaccaaagaggcagtgggcaagtcggcacctatggccttaatactttcaccaatatggaagccc

SEQ ID NO: 1417 - DNA, 120 bp, synthetic construct
  source 1..120: mol_type = other DNA
aaagaggcagtgggcaagtcggcacctatggccttaatactttcaccaatatggaagcccaattaattagacagatggagggagaaggaatcttcaaaagcattcagcacctgacagcca

SEQ ID NO: 1418 - DNA, 120 bp, synthetic construct
  source 1..120: mol_type = other DNA
aattaattagacagatggagggagaaggaatcttcaaaagcattcagcacctgacagccacagaagaaatcgctgtacagaactggttagcaagagtggggcgtgaaaggctatcgagaa

SEQ ID NO: 1419 - DNA, 120 bp, synthetic construct
  source 1..120: mol_type = other DNA
cagaagaaatcgctgtacagaactggttagcaagagtggggcgtgaaaggctatcgagaatggcaatcagtggggatgattgtgttgtaaagcctatagatgatagatttgcaagtgctt

SEQ ID NO: 1420 - DNA, 120 bp, synthetic construct
  source 1..120: mol_type = other DNA
tggcaatcagtggggatgattgtgttgtaaagcctatagatgatagatttgcaagtgctttaacagctctaaatgacatgggaaaagttagaaaagatatacaacaatgggaaccttcaa

SEQ ID NO: 1421 - DNA, 120 bp, synthetic construct
  source 1..120: mol_type = other DNA
taacagctctaaatgacatgggaaaagttagaaaagatatacaacaatgggaaccttcaagaggatggaacgattggacacaagtgcctttctgttcacaccattttcatgagttagtca

SEQ ID NO: 1422 - DNA, 120 bp, synthetic construct
  source 1..120: mol_type = other DNA
gaggatggaacgattggacacaagtgcctttctgttcacaccattttcatgagttagtcatgaaagatggtcgcgtgctcgtagtcccatgcagaaaccaagatgaactgattggtagag

SEQ ID NO: 1423 - DNA, 120 bp, synthetic construct
  source 1..120: mol_type = other DNA
tgaaagatggtcgcgtgctcgtagtcccatgcagaaaccaagatgaactgattggtagagcccgaatttcccagggagctgggtggtctttgaaggagacggcctgtttggggaagtctt

SEQ ID NO: 1424 - DNA, 120 bp, synthetic construct
  source 1..120: mol_type = other DNA
cccgaatttcccagggagctgggtggtctttgaaggagacggcctgtttggggaagtcttacgcccaaatgtggaccctgatgtacttccacagacgtgacctcagactggcggcaaatg

SEQ ID NO: 1425 - DNA, 120 bp, synthetic construct
  source 1..120: mol_type = other DNA
acgcccaaatgtggaccctgatgtacttccacagacgtgacctcagactggcggcaaatgccatttgctcggcagtcccgccacattgggttccaacaagtcgaacaacctggtccatac

SEQ ID NO: 1426 - DNA, 120 bp, synthetic construct
  source 1..120: mol_type = other DNA
ccatttgctcggcagtcccgccacattgggttccaacaagtcgaacaacctggtccatacacgccaagcatgaatggatgacgacggaagacatgctggcagtctggaacagggtgtgga

SEQ ID NO: 1427 - DNA, 120 bp, synthetic construct
  source 1..120: mol_type = other DNA
acgccaagcatgaatggatgacgacggaagacatgctggcagtctggaacagggtgtggatccaagaaaacccgtggatggaagataaaactccagtggaatcatgggaagaagtcccat

SEQ ID NO: 1428 - DNA, 120 bp, synthetic construct
  source 1..120: mol_type = other DNA
tccaagaaaacccgtggatggaagataaaactccagtggaatcatgggaagaagtcccatacttgggaaaaagagaagaccaatggtgcggctcattgattgggctaacaagcagggcta

SEQ ID NO: 1429 - DNA, 120 bp, synthetic construct
  source 1..120: mol_type = other DNA
acttgggaaaaagagaagaccaatggtgcggctcattgattgggctaacaagcagggctacctgggcaaagaacatccaaacagcaataaatcaagtcagatcccttataggcaatgagg

SEQ ID NO: 1430 - DNA, 120 bp, synthetic construct
  source 1..120: mol_type = other DNA
cctgggcaaagaacatccaaacagcaataaatcaagtcagatcccttataggcaatgaggaatacacagactacatgccatccatgaagagattcagaagggaagaggaagaggcaggtg

SEQ ID NO: 1431 - DNA, 120 bp, synthetic construct
  source 1..120: mol_type = other DNA
aatacacagactacatgccatccatgaagagattcagaagggaagaggaagaggcaggtgtcctgtggtaaaaggcaaaactaacatgaaacaaggctaaaagtcaggtcggattaagcc

SEQ ID NO: 1432 - DNA, 120 bp, synthetic construct
  source 1..120: mol_type = other DNA
tcctgtggtaaaaggcaaaactaacatgaaacaaggctaaaagtcaggtcggattaagccatagtacgggaaaaactatgctacctgtgagccccgtccaaggacgttaaaagaagtcag

SEQ ID NO: 1433 - DNA, 120 bp, synthetic construct
  source 1..120: mol_type = other DNA
atagtacgggaaaaactatgctacctgtgagccccgtccaaggacgttaaaagaagtcaggccatcacaaaatgccacagcttgagtaaactgtgcagcctgtagctccacctgaggagg

SEQ ID NO: 1434 - DNA, 120 bp, synthetic construct
  source 1..120: mol_type = other DNA
gccatcacaaaatgccacagcttgagtaaactgtgcagcctgtagctccacctgaggaggtgtaaaaaacctgggaggccacaaaccatggaagctgtacgcatggtgtagtggactagc

SEQ ID NO: 1435 - DNA, 120 bp, synthetic construct
  source 1..120: mol_type = other DNA
tgtaaaaaacctgggaggccacaaaccatggaagctgtacgcatggtgtagtggactagcggttagaggagacccctcccttacaaatcgcagcaaacaacgggggcccaaggtgagatg

SEQ ID NO: 1436 - DNA, 120 bp, synthetic construct
  source 1..120: mol_type = other DNA
ggttagaggagacccctcccttacaaatcgcagcaaacaacgggggcccaaggtgagatgaagctgtaatctcaccggaaggactagaggttagaggagacccccccaaaacaaaaaaca

SEQ ID NO: 1437 - DNA, 120 bp, synthetic construct
  source 1..120: mol_type = other DNA
atgaagctgtaatctcaccggaaggactagaggttagaggagacccccccaaaacaaaaaacagcatattgacgctgggaaagaccagagatcctgctgtctcctcagcatcattccagg

SEQ ID NO: 1438 - DNA, 120 bp, synthetic construct
  source 1..120: mol_type = other DNA
agttgttagtctacgtggaccgacaagaacagtttcgactcggaagcttgcttaacgtagtgctaacagttttttattagagagcagatctctgatgaacaaccaacggaagaagacggg

SEQ ID NO: 1439 - DNA, 120 bp, synthetic construct
  source 1..120: mol_type = other DNA
tgctaacagttttttattagagagcagatctctgatgaacaaccaacggaagaagacgggaaaaccgtctatcaatatgctgaaacgcgtgagaaaccgtgtgtcaactggatcacagtt

SEQ ID NO: 1440 - DNA, 120 bp, synthetic construct
  source 1..120: mol_type = other DNA
aaaaccgtctatcaatatgctgaaacgcgtgagaaaccgtgtgtcaactggatcacagttggcgaagagattctcaaaaggattgctgaacggccagggaccaatgaaattggtcatggc

SEQ ID NO: 1441 - DNA, 120 bp, synthetic construct
  source 1..120: mol_type = other DNA
ggcgaagagattctcaaaaggattgctgaacggccagggaccaatgaaattggtcatggcgttcatagccttccttagatttctggccattccaccaacagcaggagttttggccagatg

SEQ ID NO: 1442 - DNA, 120 bp, synthetic construct
  source 1..120: mol_type = other DNA
gttcatagccttccttagatttctggccattccaccaacagcaggagttttggccagatggggaaccttcaagaagtcgggtgccattaaggttctgaaaggcttcaagaaggagatttc

SEQ ID NO: 1443 - DNA, 120 bp, synthetic construct
  source 1..120: mol_type = other DNA
gggaaccttcaagaagtcgggtgccattaaggttctgaaaggcttcaagaaggagatttcaaacatgctgagcataatcaacaaacggaaaaagacatcgctctgtctcatgatgatatt

SEQ ID NO: 1444 - DNA, 120 bp, synthetic construct
  source 1..120: mol_type = other DNA
aaacatgctgagcataatcaacaaacggaaaaagacatcgctctgtctcatgatgatattgccagcagcacttgctttccacttgacttcacgagatggagagccgcggatgattgtagg

SEQ ID NO: 1445 - DNA, 120 bp, synthetic construct
  source 1..120: mol_type = other DNA
gccagcagcacttgctttccacttgacttcacgagatggagagccgcggatgattgtagggaagaatgaaagagggaaatccctactttttaagacagcctctggaatcaacatgtgcac

SEQ ID NO: 1446 - DNA, 120 bp, synthetic construct
  source 1..120: mol_type = other DNA
gaagaatgaaagagggaaatccctactttttaagacagcctctggaatcaacatgtgcacactcatagccatggacttgggagaaatgtgtgatgacacggtcacttacaaatgccccca

SEQ ID NO: 1447 - DNA, 120 bp, synthetic construct
  source 1..120: mol_type = other DNA
actcatagccatggacttgggagaaatgtgtgatgacacggtcacttacaaatgcccccacattaccgaagtggaacctgaagacattgactgctggtgcaaccttacatcaacatgggt

SEQ ID NO: 1448 - DNA, 120 bp, synthetic construct
  source 1..120: mol_type = other DNA
cattaccgaagtggaacctgaagacattgactgctggtgcaaccttacatcaacatgggtgacttatggaacgtgtaaccaagctggagagcatagacgcgacaagagatcagtggcgtt

SEQ ID NO: 1449 - DNA, 120 bp, synthetic construct
  source 1..120: mol_type = other DNA
gacttatggaacgtgtaaccaagctggagagcatagacgcgacaagagatcagtggcgttagctccccatgtcggcatgggactggacacacgcacccaaacctggatgtcggctgaagg

SEQ ID NO: 1450 - DNA, 120 bp, synthetic construct
  source 1..120: mol_type = other DNA
agctccccatgtcggcatgggactggacacacgcacccaaacctggatgtcggctgaaggagcttggagacaagtcgagaaggtagagacatgggcccttaggcatccagggttcaccat

SEQ ID NO: 1451 - DNA, 120 bp, synthetic construct
  source 1..120: mol_type = other DNA
agcttggagacaagtcgagaaggtagagacatgggcccttaggcatccagggttcaccatactagccctatttcttgcccattacataggcacctccttgacccagaaggtggttatttt

SEQ ID NO: 1452 - DNA, 120 bp, synthetic construct
  source 1..120: mol_type = other DNA
actagccctatttcttgcccattacataggcacctccttgacccagaaggtggttatttttacactactaatgctggtcaccccatccatgacaatgagatgtgtgggagtgggaaatag

SEQ ID NO: 1453 - DNA, 120 bp, synthetic construct
  source 1..120: mol_type = other DNA
tacactactaatgctggtcaccccatccatgacaatgagatgtgtgggagtgggaaatagagattttgtggaaggtctgtcaggagctacgtgggttgacgtggtgctagagcacggggg

SEQ ID NO: 1454 - DNA, 120 bp, synthetic construct
  source 1..120: mol_type = other DNA
agattttgtggaaggtctgtcaggagctacgtgggttgacgtggtgctagagcacggggggtgtgtgaccaccatggctaagaacaagcccacgctggatatagagcttcagaagaccga

SEQ ID NO: 1455 - DNA, 120 bp, synthetic construct
  source 1..120: mol_type = other DNA
gtgtgtgaccaccatggctaagaacaagcccacgctggatatagagcttcagaagaccgaggccacccaactggcgaccctaaggaagctatgcattgaggggaaaattaccaacataac

SEQ ID NO: 1456 - DNA, 120 bp, synthetic construct
  source 1..120: mol_type = other DNA
ggccacccaactggcgaccctaaggaagctatgcattgaggggaaaattaccaacataacaactgactcaagatgtcctacccaaggggaagcggttttgcctgaggagcaggaccagaa

SEQ ID NO: 1457 - DNA, 120 bp, synthetic construct
  source 1..120: mol_type = other DNA
aactgactcaagatgtcctacccaaggggaagcggttttgcctgaggagcaggaccagaactacgtgtgtaagcacacatacgtagatagaggctgggggaacggttgtggtttgtttgg

SEQ ID NO: 1458 - DNA, 120 bp, synthetic construct
  source 1..120: mol_type = other DNA
ctacgtgtgtaagcacacatacgtagatagaggctgggggaacggttgtggtttgtttggcaagggaagcttggtaacatgtgcgaaatttcaatgcctggaaccgatagagggaaaagt

SEQ ID NO: 1459 - DNA, 120 bp, synthetic construct
  source 1..120: mol_type = other DNA
caagggaagcttggtaacatgtgcgaaatttcaatgcctggaaccgatagagggaaaagtagtgcaatatgagaacctcaaatacaccgtcatcattacagtgcacacaggagaccaaca

SEQ ID NO: 1460 - DNA, 120 bp, synthetic construct
  source 1..120: mol_type = other DNA
agtgcaatatgagaacctcaaatacaccgtcatcattacagtgcacacaggagaccaacaccaggtgggaaatgaaacgcagggaatcacggctgagataacgcctcaggcatcaactac

SEQ ID NO: 1461 - DNA, 120 bp, synthetic construct
  source 1..120: mol_type = other DNA
ccaggtgggaaatgaaacgcagggaatcacggctgagataacgcctcaggcatcaactactgaagccatcttgcctgaatatggaacccttgggctagaatgctcaccacggacaggttt

SEQ ID NO: 1462 - DNA, 120 bp, synthetic construct
  source 1..120: mol_type = other DNA
tgaagccatcttgcctgaatatggaacccttgggctagaatgctcaccacggacaggtttggatttcaatgaaatgatcttactaacaatgaagaacaaagcatggatggtacacagaca

SEQ ID NO: 1463 - DNA, 120 bp, synthetic construct
  source 1..120: mol_type = other DNA
ggatttcaatgaaatgatcttactaacaatgaagaacaaagcatggatggtacacagacaatggttttttgatctacctctaccatggacatcaggagccacgacagaaacaccaacttg

SEQ ID NO: 1464 - DNA, 120 bp, synthetic construct
  source 1..120: mol_type = other DNA
atggttttttgatctacctctaccatggacatcaggagccacgacagaaacaccaacttggaacaggaaggagctccttgtgacattcaaaaatgcacatgcgaaaaaacaagaagtagt

SEQ ID NO: 1465 - DNA, 120 bp, synthetic construct
  source 1..120: mol_type = other DNA
gaacaggaaggagctccttgtgacattcaaaaatgcacatgcgaaaaaacaagaagtagttgtccttggatcgcaagagggagcaatgcataccgcactgacaggagccacagaaatcca

SEQ ID NO: 1466 - DNA, 120 bp, synthetic construct
  source 1..120: mol_type = other DNA
tgtccttggatcgcaagagggagcaatgcataccgcactgacaggagccacagaaatccaaaactcaggaggcacaagcatttttgcggggcacttaaagtgtagacttaagatggacaa

SEQ ID NO: 1467 - DNA, 120 bp, synthetic construct
  source 1..120: mol_type = other DNA
aaactcaggaggcacaagcatttttgcggggcacttaaagtgtagacttaagatggacaaattggaactcaaggggatgagctatgcaatgtgcacgaacacctttgtgttgaagaaaga

SEQ ID NO: 1468 - DNA, 120 bp, synthetic construct
  source 1..120: mol_type = other DNA
attggaactcaaggggatgagctatgcaatgtgcacgaacacctttgtgttgaagaaagaagtctcagaaacgcagcatgggacaatactcattaaggtcgagtacaaaggggaagacgc

SEQ ID NO: 1469 - DNA, 120 bp, synthetic construct
  source 1..120: mol_type = other DNA
agtctcagaaacgcagcatgggacaatactcattaaggtcgagtacaaaggggaagacgcaccttgcaagattcctttctccacagaggatggacaagggaaagctcacaatggcagact

SEQ ID NO: 1470 - DNA, 120 bp, synthetic construct
  source 1..120: mol_type = other DNA
accttgcaagattcctttctccacagaggatggacaagggaaagctcacaatggcagactgatcacagccaacccagtggtgactaagaaggaggagcctgtcaacattgaggctgaacc

SEQ ID NO: 1471 - DNA, 120 bp, synthetic construct
  source 1..120: mol_type = other DNA
gatcacagccaacccagtggtgactaagaaggaggagcctgtcaacattgaggctgaacctccttttggggaaagtaatatagtaattggaactggagacaatgccttgaaaatcaattg

SEQ ID NO: 1472 - DNA, 120 bp, synthetic construct
  source 1..120: mol_type = other DNA
tccttttggggaaagtaatatagtaattggaactggagacaatgccttgaaaatcaattggtacaagaagggaagctctattgggaagatgttcgaggccactgccagaggtgcaaggcg

SEQ ID NO: 1473 - DNA, 120 bp, synthetic construct
  source 1..120: mol_type = other DNA
gtacaagaagggaagctctattgggaagatgttcgaggccactgccagaggtgcaaggcgcatggccatcttgggagacacagcttgggactttggatcagtgggtggtgttctgaactc

SEQ ID NO: 1474 - DNA, 120 bp, synthetic construct
  source 1..120: mol_type = other DNA
catggccatcttgggagacacagcttgggactttggatcagtgggtggtgttctgaactcattaggcaaaatggtgcaccaaatattcggaagtgcttacacagccctattcagtggagt

SEQ ID NO: 1475 - DNA, 120 bp, synthetic construct
  source 1..120: mol_type = other DNA
attaggcaaaatggtgcaccaaatattcggaagtgcttacacagccctattcagtggagtctcttgggtgatgaaaattggaataggtgttctcttaacttggatagggttgaattcaaa

SEQ ID NO: 1476 - DNA, 120 bp, synthetic construct
  source 1..120: mol_type = other DNA
ctcttgggtgatgaaaattggaataggtgttctcttaacttggatagggttgaattcaaaaaacacatccatgtcattttcatgcattgcaattggaatcatcacactctatttgggagc

SEQ ID NO: 1477 - DNA, 120 bp, synthetic construct
  source 1..120: mol_type = other DNA
aaacacatccatgtcattttcatgcattgcaattggaatcatcacactctatttgggagctgtagtacaagctgacatggggtgtgtcataaactggaaaggcaaagaactcaaatgcgg

SEQ ID NO: 1478 - DNA, 120 bp, synthetic construct
  source 1..120: mol_type = other DNA
tgtagtacaagctgacatggggtgtgtcataaactggaaaggcaaagaactcaaatgcggaagtggaattttcgtcaccaacgaggtccatacctggacagagcagtacaaattccaagc

SEQ ID NO: 1479 - DNA, 120 bp, synthetic construct
  source 1..120: mol_type = other DNA
aagtggaattttcgtcaccaacgaggtccatacctggacagagcagtacaaattccaagcggattccccaaaaagattggcgacagccattgcaggcgcttgggaaaatggagtgtgtgg

SEQ ID NO: 1480 - DNA, 120 bp, synthetic construct
  source 1..120: mol_type = other DNA
ggattccccaaaaagattggcgacagccattgcaggcgcttgggaaaatggagtgtgtggaattaggtcaacaaccagaatggagaatctcttgtggaagcaagtagccaatgaactgaa

SEQ ID NO: 1481 - DNA, 120 bp, synthetic construct
  source 1..120: mol_type = other DNA
aattaggtcaacaaccagaatggagaatctcttgtggaagcaagtagccaatgaactgaactacatattatgggaaaacaacatcaaattaacggtagttgtgggcgacacaatcggggt

SEQ ID NO: 1482 - DNA, 120 bp, synthetic construct
  source 1..120: mol_type = other DNA
ctacatattatgggaaaacaacatcaaattaacggtagttgtgggcgacacaatcggggttttagagcaaggaaaaagaacactaacaccacaacccatggagctaaaatactcatggaa

SEQ ID NO: 1483 - DNA, 120 bp, synthetic construct
  source 1..120: mol_type = other DNA
tttagagcaaggaaaaagaacactaacaccacaacccatggagctaaaatactcatggaaaacgtggggaaaggcaaaaatagtgacagcagaaacacaaaattcctctttcataataga

SEQ ID NO: 1484 - DNA, 120 bp, synthetic construct
  source 1..120: mol_type = other DNA
aacgtggggaaaggcaaaaatagtgacagcagaaacacaaaattcctctttcataatagacgggccaaacacaccggagtgtccaagtgcctcaagagcatggaatgtgtgggaggtaga

SEQ ID NO: 1485 - DNA, 120 bp, synthetic construct
  source 1..120: mol_type = other DNA
cgggccaaacacaccggagtgtccaagtgcctcaagagcatggaatgtgtgggaggtagaagattacggattcggagtcttcacaaccaacatatggctgaaactccgagaggtgtacac

SEQ ID NO: 1486 - DNA, 120 bp, synthetic construct
  source 1..120: mol_type = other DNA
agattacggattcggagtcttcacaaccaacatatggctgaaactccgagaggtgtacacccaaatgtgtgaccataggctaatgtcggcagccgtcaaggatgagagggccgtgcatgc

SEQ ID NO: 1487 - DNA, 120 bp, synthetic construct
  source 1..120: mol_type = other DNA
ccaaatgtgtgaccataggctaatgtcggcagccgtcaaggatgagagggccgtgcatgccgacatgggctactggatagaaagccaaaagaatggaagttggaagctagaaaaagcatc

SEQ ID NO: 1488 - DNA, 120 bp, synthetic construct
  source 1..120: mol_type = other DNA
cgacatgggctactggatagaaagccaaaagaatggaagttggaagctagaaaaagcatccctcatagaggtgaaaacctgcacatggccaaaatcacacactctttggagcaacggtgt

SEQ ID NO: 1489 - DNA, 120 bp, synthetic construct
  source 1..120: mol_type = other DNA
cctcatagaggtgaaaacctgcacatggccaaaatcacacactctttggagcaacggtgtgctagagagtgacatgatcattccaaagagtctagctggtcctatctcgcaacacaacta

SEQ ID NO: 1490 - DNA, 120 bp, synthetic construct
  source 1..120: mol_type = other DNA
gctagagagtgacatgatcattccaaagagtctagctggtcctatctcgcaacacaactacaggcccgggtaccacacccaaacggcaggaccctggcacttaggaaaattggagctgga

SEQ ID NO: 1491 - DNA, 120 bp, synthetic construct
  source 1..120: mol_type = other DNA
caggcccgggtaccacacccaaacggcaggaccctggcacttaggaaaattggagctggacttcaactattgtgaaggaacaacagttgtcatcacagaaaattgtgggacaagaggccc

SEQ ID NO: 1492 - DNA, 120 bp, synthetic construct
  source 1..120: mol_type = other DNA
cttcaactattgtgaaggaacaacagttgtcatcacagaaaattgtgggacaagaggcccatcattgagaacgacaacagtgtcaggaaagttgatacatgaatggtgttgccgctcgtg

SEQ ID NO: 1493 - DNA, 120 bp, synthetic construct
  source 1..120: mol_type = other DNA
atcattgagaacgacaacagtgtcaggaaagttgatacatgaatggtgttgccgctcgtgcacacttcctcccctgcgatacatgggagaagacggctgttggtatggcatggaaatcag

SEQ ID NO: 1494 - DNA, 120 bp, synthetic construct
  source 1..120: mol_type = other DNA
cacacttcctcccctgcgatacatgggagaagacggctgttggtatggcatggaaatcaggcccatcagtgagaaagaagagaacatggtaaagtctctagtctcagcgggaagtggaaa

SEQ ID NO: 1495 - DNA, 120 bp, synthetic construct
  source 1..120: mol_type = other DNA
gcccatcagtgagaaagaagagaacatggtaaagtctctagtctcagcgggaagtggaaaggtagacaacttcacaatgggcgtcttgtgtttggcaatcctctttgaagaggtgatgag

SEQ ID NO: 1496 - DNA, 120 bp, synthetic construct
  source 1..120: mol_type = other DNA
ggtagacaacttcacaatgggcgtcttgtgtttggcaatcctctttgaagaggtgatgagaggaaaatttgggaagaaacacatgattgcaggggttttcctcacgtttgtgctccttct

SEQ ID NO: 1497 - DNA, 120 bp, synthetic construct
  source 1..120: mol_type = other DNA
aggaaaatttgggaagaaacacatgattgcaggggttttcctcacgtttgtgctccttctctcagggcaaataacatggagagacatggcgcacacactaataatgattgggtccaacgc

SEQ ID NO: 1498 - DNA, 120 bp, synthetic construct
  source 1..120: mol_type = other DNA
ctcagggcaaataacatggagagacatggcgcacacactaataatgattgggtccaacgcctctgacaggatgggaatgggcgtcacctatctagctttaattgcaacatttaaaatcca

SEQ ID NO: 1499 - DNA, 120 bp, synthetic construct
  source 1..120: mol_type = other DNA
ctctgacaggatgggaatgggcgtcacctatctagctttaattgcaacatttaaaatccagccattcctggctttgggatttttcctaagaaaactgacatctagagaaaatttactgtt

SEQ ID NO: 1500 - DNA, 120 bp, synthetic construct
  source 1..120: mol_type = other DNA
gccattcctggctttgggatttttcctaagaaaactgacatctagagaaaatttactgttaggagttggactggctatggcaacaacgttacaattgccagaggacattgaacaaatggc

SEQ ID NO: 1501 - DNA, 120 bp, synthetic construct
  source 1..120: mol_type = other DNA
aggagttggactggctatggcaacaacgttacaattgccagaggacattgaacaaatggcaaatggaatcgccctggggctcatggctcttaaattgataacacaatttgaaacatacca

SEQ ID NO: 1502 - DNA, 120 bp, synthetic construct
  source 1..120: mol_type = other DNA
aaatggaatcgccctggggctcatggctcttaaattgataacacaatttgaaacataccaattatggacagcattaatctccttaacgtgttcaaatacaatcttcacgttgactgttgc

SEQ ID NO: 1503 - DNA, 120 bp, synthetic construct
  source 1..120: mol_type = other DNA
attatggacagcattaatctccttaacgtgttcaaatacaatcttcacgttgactgttgcttggagaacagccaccctgattttggctggagtttcacttttaccagtgtgccagtcttc

SEQ ID NO: 1504 - DNA, 120 bp, synthetic construct
  source 1..120: mol_type = other DNA
ttggagaacagccaccctgattttggctggagtttcacttttaccagtgtgccagtcttcgagcatgagaaaaacagactggcttccaatgacagtggcagctatgggagtcccacccct

SEQ ID NO: 1505 - DNA, 120 bp, synthetic construct
  source 1..120: mol_type = other DNA
gagcatgagaaaaacagactggcttccaatgacagtggcagctatgggagtcccacccctaccactctttatttttagcttgaaagacacactcaaaaggagaagctggccactgaatga

SEQ ID NO: 1506 - DNA, 120 bp, synthetic construct
  source 1..120: mol_type = other DNA
accactctttatttttagcttgaaagacacactcaaaaggagaagctggccactgaatgaaggggtgatggctgttggacttgtgagcattctggccagttctctccttaggaatgacgt

SEQ ID NO: 1507 - DNA, 120 bp, synthetic construct
  source 1..120: mol_type = other DNA
aggggtgatggctgttggacttgtgagcattctggccagttctctccttaggaatgacgtgcccatggctggaccattagtggccgggggcttgctgatagcgtgctacgtcataactgg

SEQ ID NO: 1508 - DNA, 120 bp, synthetic construct
  source 1..120: mol_type = other DNA
gcccatggctggaccattagtggccgggggcttgctgatagcgtgctacgtcataactggcacgtcagcagaccttacagtagaaaaagcagcagatgtaacatgggaggaagaggctga

SEQ ID NO: 1509 - DNA, 120 bp, synthetic construct
  source 1..120: mol_type = other DNA
cacgtcagcagaccttacagtagaaaaagcagcagatgtaacatgggaggaagaggctgagcaaacaggagtgtcccacaacttaatgatcacagttgatgatgatggaacaatgagaat

SEQ ID NO: 1510 - DNA, 120 bp, synthetic construct
  source 1..120: mol_type = other DNA
gcaaacaggagtgtcccacaacttaatgatcacagttgatgatgatggaacaatgagaataaaagatgatgagactgagaatattctaacagtgcttttgaagacagcattattaatagt

SEQ ID NO: 1511 - DNA, 120 bp, synthetic construct
  source 1..120: mol_type = other DNA
aaaagatgatgagactgagaatattctaacagtgcttttgaagacagcattattaatagtatcaggtatctttccatactccatacctgcaacattgttggtctggcatacttggcaaaa

SEQ ID NO: 1512 - DNA, 120 bp, synthetic construct
  source 1..120: mol_type = other DNA
atcaggtatctttccatactccatacctgcaacattgttggtctggcatacttggcaaaagcaaacccaaagatccggtgttctatgggacgtacccagccccccagagacacagaaagc

SEQ ID NO: 1513 - DNA, 120 bp, synthetic construct
  source 1..120: mol_type = other DNA
gcaaacccaaagatccggtgttctatgggacgtacccagccccccagagacacagaaagcagaactggaagaaggggtctataggatcaaacagcaaggaatttttgggaaaacccaagt

SEQ ID NO: 1514 - DNA, 120 bp, synthetic construct
  source 1..120: mol_type = other DNA
agaactggaagaaggggtctataggatcaaacagcaaggaatttttgggaaaacccaagtaggggttggagtacaaaaagacggagtcttccacaccatgtggcacgtcacaagaggggc

SEQ ID NO: 1515 - DNA, 120 bp, synthetic construct
  source 1..120: mol_type = other DNA
aggggttggagtacaaaaagacggagtcttccacaccatgtggcacgtcacaagaggggcagtgttgacacataatgggaaaagactggaaccaaattgggctagcgtgaaaaaagatct

SEQ ID NO: 1516 - DNA, 120 bp, synthetic construct
  source 1..120: mol_type = other DNA
agtgttgacacataatgggaaaagactggaaccaaattgggctagcgtgaaaaaagatctgatttcatacggaggaggatggagattgagcgcacaatggcaaaagggggaggaggtgca

SEQ ID NO: 1517 - DNA, 120 bp, synthetic construct
  source 1..120: mol_type = other DNA
gatttcatacggaggaggatggagattgagcgcacaatggcaaaagggggaggaggtgcaggtcattgccgtagagcctgggaagaatccaaagaacttccaaaccatgccaggcacatt

SEQ ID NO: 1518 - DNA, 120 bp, synthetic construct
  source 1..120: mol_type = other DNA
ggtcattgccgtagagcctgggaagaatccaaagaacttccaaaccatgccaggcacattccagactacaacaggggaaataggagcaattgcactggatttcaagcctggaacttcagg

SEQ ID NO: 1519 - DNA, 120 bp, synthetic construct
  source 1..120: mol_type = other DNA
ccagactacaacaggggaaataggagcaattgcactggatttcaagcctggaacttcagggtctcctatcataaacagagagggaaaggtagtgggactatatggcaatggagtggttac

SEQ ID NO: 1520 - DNA, 120 bp, synthetic construct
  source 1..120: mol_type = other DNA
gtctcctatcataaacagagagggaaaggtagtgggactatatggcaatggagtggttacaaagaatggcggctacgtcagtggaatagcgcaaacaaatgcagaaccagatggaccgac

SEQ ID NO: 1521 - DNA, 120 bp, synthetic construct
  source 1..120: mol_type = other DNA
aaagaatggcggctacgtcagtggaatagcgcaaacaaatgcagaaccagatggaccgacgccagagttggaagaagagatgttcaaaaagcgaaatctaaccataatggatcttcatcc

SEQ ID NO: 1522 - DNA, 120 bp, synthetic construct
  source 1..120: mol_type = other DNA
gccagagttggaagaagagatgttcaaaaagcgaaatctaaccataatggatcttcatcctgggtcaggaaagacacggaaataccttccagccattgttagagaggcaatcaagagacg

SEQ ID NO: 1523 - DNA, 120 bp, synthetic construct
  source 1..120: mol_type = other DNA
tgggtcaggaaagacacggaaataccttccagccattgttagagaggcaatcaagagacgtttaagaactctgattttggcaccgacaagggtggttgcagctgagatggaagaagcatt

SEQ ID NO: 1524 - DNA, 120 bp, synthetic construct
  source 1..120: mol_type = other DNA
tttaagaactctgattttggcaccgacaagggtggttgcagctgagatggaagaagcattgaaagggctcccaataaggtaccaaacaacagcaacaaaatctgaacatacgggaagaga

SEQ ID NO: 1525 - DNA, 120 bp, synthetic construct
  source 1..120: mol_type = other DNA
gaaagggctcccaataaggtaccaaacaacagcaacaaaatctgaacatacgggaagagagattgttgatctaatgtgccacgcaacgttcacaatgcgcttgctgtcaccagttagggt

SEQ ID NO: 1526 - DNA, 120 bp, synthetic construct
  source 1..120: mol_type = other DNA
gattgttgatctaatgtgccacgcaacgttcacaatgcgcttgctgtcaccagttagggttccaaattacaacttgataataatggatgaggcccatttcacagacccagccagtatagc

SEQ ID NO: 1527 - DNA, 120 bp, synthetic construct
  source 1..120: mol_type = other DNA
tccaaattacaacttgataataatggatgaggcccatttcacagacccagccagtatagcggccagagggtacatatcaactcgcgttggaatgggagaggcagccgcaatcttcatgac

SEQ ID NO: 1528 - DNA, 120 bp, synthetic construct
  source 1..120: mol_type = other DNA
ggccagagggtacatatcaactcgcgttggaatgggagaggcagccgcaatcttcatgacggcaacaccccctggaacagctgatgcctttcctcagagcaacgctccaattcaagatga

SEQ ID NO: 1529 - DNA, 120 bp, synthetic construct
  source 1..120: mol_type = other DNA
ggcaacaccccctggaacagctgatgcctttcctcagagcaacgctccaattcaagatgaagaaagggacataccagaacgctcatggaattcaggcaatgaatggattaccgacttcgc

SEQ ID NO: 1530 - DNA, 120 bp, synthetic construct
  source 1..120: mol_type = other DNA
agaaagggacataccagaacgctcatggaattcaggcaatgaatggattaccgacttcgccgggaaaacggtgtggtttgtccccagcatcaaagccggaaatgacatagcaaactgctt

SEQ ID NO: 1531 - DNA, 120 bp, synthetic construct
  source 1..120: mol_type = other DNA
cgggaaaacggtgtggtttgtccccagcatcaaagccggaaatgacatagcaaactgcttgcgaaagaacgggaaaaaggtcattcaacttagtaggaagacttttgaaacagaatatca

SEQ ID NO: 1532 - DNA, 120 bp, synthetic construct
  source 1..120: mol_type = other DNA
gcgaaagaacgggaaaaaggtcattcaacttagtaggaagacttttgaaacagaatatcagaagactaaactaaatgactgggactttgtggtgacaactgacatttcagaaatgggggc

SEQ ID NO: 1533 - DNA, 120 bp, synthetic construct
  source 1..120: mol_type = other DNA
gaagactaaactaaatgactgggactttgtggtgacaactgacatttcagaaatgggggccaatttcaaagcagatagagtgatcgacccaagaagatgtctaaaaccagtgatcctgac

SEQ ID NO: 1534 - DNA, 120 bp, synthetic construct
  source 1..120: mol_type = other DNA
caatttcaaagcagatagagtgatcgacccaagaagatgtctaaaaccagtgatcctgacagatggaccagagcgggtgatcctggctggaccaatgccagtcaccgcggcgagtgctgc

SEQ ID NO: 1535 - DNA, 120 bp, synthetic construct
  source 1..120: mol_type = other DNA
agatggaccagagcgggtgatcctggctggaccaatgccagtcaccgcggcgagtgctgcgcaaaggagagggagagttggcaggaacccacaaaaagaaaatgaccagtacatattcac

SEQ ID NO: 1536 - DNA, 120 bp, synthetic construct
  source 1..120: mol_type = other DNA
gcaaaggagagggagagttggcaggaacccacaaaaagaaaatgaccagtacatattcacgggtcagcctctcaacaatgatgaagaccatgctcactggacagaagcaaaaatgctgct

SEQ ID NO: 1537 - DNA, 120 bp, synthetic construct
  source 1..120: mol_type = other DNA
gggtcagcctctcaacaatgatgaagaccatgctcactggacagaagcaaaaatgctgctggacaacatcaacactccagaaggaatcataccagctctctttgaaccagaaagggagaa

SEQ ID NO: 1538 - DNA, 120 bp, synthetic construct
  source 1..120: mol_type = other DNA
ggacaacatcaacactccagaaggaatcataccagctctctttgaaccagaaagggagaagtcagccgccatagacggtgaatatcgcctgaagggtgaatccaggaagactttcgtgga

SEQ ID NO: 1539 - DNA, 120 bp, synthetic construct
  source 1..120: mol_type = other DNA
gtcagccgccatagacggtgaatatcgcctgaagggtgaatccaggaagactttcgtggaactcatgaggaggggtgacctcccagtttggttagcccacaaagtagcatcagaagggat

SEQ ID NO: 1540 - DNA, 120 bp, synthetic construct
  source 1..120: mol_type = other DNA
actcatgaggaggggtgacctcccagtttggttagcccacaaagtagcatcagaagggatcaaatatacagataggaaatggtgctttgatggacagcgcaacaaccaaattttagagga

SEQ ID NO: 1541 - DNA, 120 bp, synthetic construct
  source 1..120: mol_type = other DNA
caaatatacagataggaaatggtgctttgatggacagcgcaacaaccaaattttagaggaaaacatggacgtggaaatctggacaaaggaaggagaaaagaaaaaattaagacctaggtg

SEQ ID NO: 1542 - DNA, 120 bp, synthetic construct
  source 1..120: mol_type = other DNA
aaacatggacgtggaaatctggacaaaggaaggagaaaagaaaaaattaagacctaggtggcttgatgcccgcacttattcagatcccttagcactcaaggaattcaaggactttgcggc

SEQ ID NO: 1543 - DNA, 120 bp, synthetic construct
  source 1..120: mol_type = other DNA
gcttgatgcccgcacttattcagatcccttagcactcaaggaattcaaggactttgcggctggcagaaagtcaatcgcccttgatcttgtgacagaaataggaagagtgccttcacacct

SEQ ID NO: 1544 - DNA, 120 bp, synthetic construct
  source 1..120: mol_type = other DNA
tggcagaaagtcaatcgcccttgatcttgtgacagaaataggaagagtgccttcacacctagcccacagaacgagaaacgctctggacaatctggtgatgctgcacacgtcagaacatgg

SEQ ID NO: 1545 - DNA, 120 bp, synthetic construct
  source 1..120: mol_type = other DNA
agcccacagaacgagaaacgctctggacaatctggtgatgctgcacacgtcagaacatggcggtagggcctacaggcatgcggtggaggaactaccagaaacaatggaaacactcctact

SEQ ID NO: 1546 - DNA, 120 bp, synthetic construct
  source 1..120: mol_type = other DNA
cggtagggcctacaggcatgcggtggaggaactaccagaaacaatggaaacactcctactcttaggactcatgatcttactgacaggtggagcaatgcttttcttgatatcaggtaaagg

SEQ ID NO: 1547 - DNA, 120 bp, synthetic construct
  source 1..120: mol_type = other DNA
cttaggactcatgatcttactgacaggtggagcaatgcttttcttgatatcaggtaaagggattggaaagacttcaataggacttatttgtgtgattgcttccagcggcatgctgtggat

SEQ ID NO: 1548 - DNA, 120 bp, synthetic construct
  source 1..120: mol_type = other DNA
gattggaaagacttcaataggacttatttgtgtgattgcttccagcggcatgctgtggatggccgaaattccactccaatggatcgcgtcggctatagtcctggagttttttatgatggt

SEQ ID NO: 1549 - DNA, 120 bp, synthetic construct
  source 1..120: mol_type = other DNA
ggccgaaattccactccaatggatcgcgtcggctatagtcctggagttttttatgatggtgttgcttataccagaaccagaaaagcagagaaccccccaagacaaccaactcgcatatgt

SEQ ID NO: 1550 - DNA, 120 bp, synthetic construct
  source 1..120: mol_type = other DNA
gttgcttataccagaaccagaaaagcagagaaccccccaagacaaccaactcgcatatgtcgtgataggcatacttacaatggctgcaataatagcggccaatgaaatgggactattgga

SEQ ID NO: 1551 - DNA, 120 bp, synthetic construct
  source 1..120: mol_type = other DNA
cgtgataggcatacttacaatggctgcaataatagcggccaatgaaatgggactattggaaactacaaagagagatctaggaatgtctaaggaaccaggtgttgtttctccaactagcta

SEQ ID NO: 1552 - DNA, 120 bp, synthetic construct
  source 1..120: mol_type = other DNA
aactacaaagagagatctaggaatgtctaaggaaccaggtgttgtttctccaactagctatttggatgtggatttgcacccagcatcagcctggacattgtacgctgtggccactacagt

SEQ ID NO: 1553 - DNA, 120 bp, synthetic construct
  source 1..120: mol_type = other DNA
tttggatgtggatttgcacccagcatcagcctggacattgtacgctgtggccactacagtaataacaccaatgttaagacataccatagagaattctacagcaaatgtgtccctggcagc

SEQ ID NO: 1554 - DNA, 120 bp, synthetic construct
  source 1..120: mol_type = other DNA
aataacaccaatgttaagacataccatagagaattctacagcaaatgtgtccctggcagctatagccaaccaggcggtggttctgatgggtttggacaaaggatggccaatatcaaaaat

SEQ ID NO: 1555 - DNA, 120 bp, synthetic construct
  source 1..120: mol_type = other DNA
tatagccaaccaggcggtggttctgatgggtttggacaaaggatggccaatatcaaaaatggacttaggcgtaccactactggcattgggttgctattcacaagtgaacccactaactct

SEQ ID NO: 1556 - DNA, 120 bp, synthetic construct
  source 1..120: mol_type = other DNA
ggacttaggcgtaccactactggcattgggttgctattcacaagtgaacccactaactctaacagcggcagtacttttgctagttacgcattatgctattataggtccaggactgcaggc

SEQ ID NO: 1557 - DNA, 120 bp, synthetic construct
  source 1..120: mol_type = other DNA
aacagcggcagtacttttgctagttacgcattatgctattataggtccaggactgcaggcaaaagccactcgtgaagctcaaaaaaggacagctgctggaataatgaagaatccaacggt

SEQ ID NO: 1558 - DNA, 120 bp, synthetic construct
  source 1..120: mol_type = other DNA
aaaagccactcgtgaagctcaaaaaaggacagctgctggaataatgaagaatccaacggtggatgggataataacaatagacctagaccctgtaatatatgattcaaaatttgaaaagca

SEQ ID NO: 1559 - DNA, 120 bp, synthetic construct
  source 1..120: mol_type = other DNA
ggatgggataataacaatagacctagaccctgtaatatatgattcaaaatttgaaaagcaactgggacaggtcatgctcctggttttgtgtgcagttcaactgttgttaatgagaacatc

SEQ ID NO: 1560 - DNA, 120 bp, synthetic construct
  source 1..120: mol_type = other DNA
actgggacaggtcatgctcctggttttgtgtgcagttcaactgttgttaatgagaacatcatgggccttgtgtgaagctttaactttagctacaggaccaataacaacactctgggaagg

SEQ ID NO: 1561 - DNA, 120 bp, synthetic construct
  source 1..120: mol_type = other DNA
atgggccttgtgtgaagctttaactttagctacaggaccaataacaacactctgggaaggatcacctgggaagttttggaataccacgatagctgtttccatggcgaacatttttagagg

SEQ ID NO: 1562 - DNA, 120 bp, synthetic construct
  source 1..120: mol_type = other DNA
atcacctgggaagttttggaataccacgatagctgtttccatggcgaacatttttagagggagctatttagcaggagctgggcttgccttttctattatgaaatcagttggaacaggaaa

SEQ ID NO: 1563 - DNA, 120 bp, synthetic construct
  source 1..120: mol_type = other DNA
gagctatttagcaggagctgggcttgccttttctattatgaaatcagttggaacaggaaaaagaggaacaggctctcaaggtgaaactttaggagaaaaatggaaaaagaaattgaatca

SEQ ID NO: 1564 - DNA, 120 bp, synthetic construct
  source 1..120: mol_type = other DNA
aagaggaacaggctctcaaggtgaaactttaggagaaaaatggaaaaagaaattgaatcaattatcccggaaagagtttgacctttacaagaagtctggaatcactgaagtggatagaac

SEQ ID NO: 1565 - DNA, 120 bp, synthetic construct
  source 1..120: mol_type = other DNA
attatcccggaaagagtttgacctttacaagaagtctggaatcactgaagtggatagaacagaagccaaagaagggttgaaaagaggagaaacaacacatcatgccgtgtccaggggtag

SEQ ID NO: 1566 - DNA, 120 bp, synthetic construct
  source 1..120: mol_type = other DNA
agaagccaaagaagggttgaaaagaggagaaacaacacatcatgccgtgtccaggggtagtgcaaaacttcaatggtttgtggaaaggaacatggtcattcccgagggaagagtcataga

SEQ ID NO: 1567 - DNA, 120 bp, synthetic construct
  source 1..120: mol_type = other DNA
tgcaaaacttcaatggtttgtggaaaggaacatggtcattcccgagggaagagtcatagacctgggctgtggaagaggaggctggtcatattactgtgcaggactgaaaaaagtcacaga

SEQ ID NO: 1568 - DNA, 120 bp, synthetic construct
  source 1..120: mol_type = other DNA
cctgggctgtggaagaggaggctggtcatattactgtgcaggactgaaaaaagtcacagaagtgcgaggatacacaaaaggcggcccaggacacgaagaaccagtgcctatgtcaacata

SEQ ID NO: 1569 - DNA, 120 bp, synthetic construct
  source 1..120: mol_type = other DNA
agtgcgaggatacacaaaaggcggcccaggacacgaagaaccagtgcctatgtcaacatatggatggaacatagttaaattaatgagtggaaaggatgtgttttatcttccgcctgaaaa

SEQ ID NO: 1570 - DNA, 120 bp, synthetic construct
  source 1..120: mol_type = other DNA
tggatggaacatagttaaattaatgagtggaaaggatgtgttttatcttccgcctgaaaagtgtgacaccctgttgtgcgacattggagaatcttcaccaagcccaacagtggaagaaag

SEQ ID NO: 1571 - DNA, 120 bp, synthetic construct
  source 1..120: mol_type = other DNA
gtgtgacaccctgttgtgcgacattggagaatcttcaccaagcccaacagtggaagaaagcagaactataagagttttgaagatggttgaaccatggctgaaaaacaaccagttttgcat

SEQ ID NO: 1572 - DNA, 120 bp, synthetic construct
  source 1..120: mol_type = other DNA
cagaactataagagttttgaagatggttgaaccatggctgaaaaacaaccagttttgcattaaagtattgaacccttacatgccagccgtgattgagcacctagaaagactgcaaaggaa

SEQ ID NO: 1573 - DNA, 120 bp, synthetic construct
  source 1..120: mol_type = other DNA
taaagtattgaacccttacatgccagccgtgattgagcacctagaaagactgcaaaggaaacacggaggaatgcttgtgagaaatccactttcacgaaactccacgcacgaaatgtactg

SEQ ID NO: 1574 - DNA, 120 bp, synthetic construct
  source 1..120: mol_type = other DNA
acacggaggaatgcttgtgagaaatccactttcacgaaactccacgcacgaaatgtactggatatctaatggtacaggtaacattgtctcttcagtcaacatgatatccagattgctact

SEQ ID NO: 1575 - DNA, 120 bp, synthetic construct
  source 1..120: mol_type = other DNA
gatatctaatggtacaggtaacattgtctcttcagtcaacatgatatccagattgctactgaacaggttcacgatgacacacaggagacctaccatagagaaagatgtggatttaggagc

SEQ ID NO: 1576 - DNA, 120 bp, synthetic construct
  source 1..120: mol_type = other DNA
gaacaggttcacgatgacacacaggagacctaccatagagaaagatgtggatttaggagcaggaactcgacatgtcaatgcggaaccagaaacacccaacatggatgtcattggggaaag

SEQ ID NO: 1577 - DNA, 120 bp, synthetic construct
  source 1..120: mol_type = other DNA
aggaactcgacatgtcaatgcggaaccagaaacacccaacatggatgtcattggggaaagaataaaaaggatcaaggaggagcataattcaacatggcactatgatgacgaaaaccccta

SEQ ID NO: 1578 - DNA, 120 bp, synthetic construct
  source 1..120: mol_type = other DNA
aataaaaaggatcaaggaggagcataattcaacatggcactatgatgacgaaaacccctacaaaacgtgggcttaccacggatcttatgaagtcaaggccacaggctcagcctcctccat

SEQ ID NO: 1579 - DNA, 120 bp, synthetic construct
  source 1..120: mol_type = other DNA
caaaacgtgggcttaccacggatcttatgaagtcaaggccacaggctcagcctcctccatgataaacggagtcgtgaaacttctcactaaaccatgggatgtagtgcccatggtgacaca

SEQ ID NO: 1580 - DNA, 120 bp, synthetic construct
  source 1..120: mol_type = other DNA
gataaacggagtcgtgaaacttctcactaaaccatgggatgtagtgcccatggtgacacagatggcaatgacagatacaactccatttggccagcagagagtttttaaagagaaggtgga

SEQ ID NO: 1581 - DNA, 120 bp, synthetic construct
  source 1..120: mol_type = other DNA
gatggcaatgacagatacaactccatttggccagcagagagtttttaaagagaaggtggacaccaggacacccaggcccatgccagggacaagaaaggttatggagatcacagcggagtg

SEQ ID NO: 1582 - DNA, 120 bp, synthetic construct
  source 1..120: mol_type = other DNA
caccaggacacccaggcccatgccagggacaagaaaggttatggagatcacagcggagtggctctggagaaccctgggaaggaacaaaagacccaggttatgcacaagggaagagttcac

SEQ ID NO: 1583 - DNA, 120 bp, synthetic construct
  source 1..120: mol_type = other DNA
gctctggagaaccctgggaaggaacaaaagacccaggttatgcacaagggaagagttcacaaaaaaggtcagaaccaacgcagccatgggcgccgttttcacagaggagaaccaatggga

SEQ ID NO: 1584 - DNA, 120 bp, synthetic construct
  source 1..120: mol_type = other DNA
aaaaaaggtcagaaccaacgcagccatgggcgccgttttcacagaggagaaccaatgggacagtgcgaaagccgctgttgaggatgaagatttttggaaacttgtggacagagaacgtga

SEQ ID NO: 1585 - DNA, 120 bp, synthetic construct
  source 1..120: mol_type = other DNA
cagtgcgaaagccgctgttgaggatgaagatttttggaaacttgtggacagagaacgtgaactccacaaattgggcaagtgtggaagctgtgtttacaacatgatgggcaagagagagaa

SEQ ID NO: 1586 - DNA, 120 bp, synthetic construct
  source 1..120: mol_type = other DNA
actccacaaattgggcaagtgtggaagctgtgtttacaacatgatgggcaagagagagaagaaacttggagagtttggcaaagcaaaaggcagtagagctatatggtacatgtggttggg

SEQ ID NO: 1587 - DNA, 120 bp, synthetic construct
  source 1..120: mol_type = other DNA
gaaacttggagagtttggcaaagcaaaaggcagtagagctatatggtacatgtggttgggagccaggtaccttgagttcgaagcccttggattcttaaatgaagatcactggttctcgcg

SEQ ID NO: 1588 - DNA, 120 bp, synthetic construct
  source 1..120: mol_type = other DNA
agccaggtaccttgagttcgaagcccttggattcttaaatgaagatcactggttctcgcgtgaaaactcttacagtggagtagaaggagaaggactgcacaagctaggctacatattaag

SEQ ID NO: 1589 - DNA, 120 bp, synthetic construct
  source 1..120: mol_type = other DNA
tgaaaactcttacagtggagtagaaggagaaggactgcacaagctaggctacatattaagggacatttccaagatacccggaggagccatgtatgctgatgacacagctggttgggacac

SEQ ID NO: 1590 - DNA, 120 bp, synthetic construct
  source 1..120: mol_type = other DNA
ggacatttccaagatacccggaggagccatgtatgctgatgacacagctggttgggacacaagaataacagaagatgacctgcacaatgaggaaaagatcacacagcaaatggaccctga

SEQ ID NO: 1591 - DNA, 120 bp, synthetic construct
  source 1..120: mol_type = other DNA
aagaataacagaagatgacctgcacaatgaggaaaagatcacacagcaaatggaccctgaacacaggctgttagcgaacgctatatttaagctcacataccaaaacaaagtggtcaaagt

SEQ ID NO: 1592 - DNA, 120 bp, synthetic construct
  source 1..120: mol_type = other DNA
acacaggctgttagcgaacgctatatttaagctcacataccaaaacaaagtggtcaaagttcaacgaccgactccaacaggcacggtaatggacattatatctaggaaagaccaaagagg

SEQ ID NO: 1593 - DNA, 120 bp, synthetic construct
  source 1..120: mol_type = other DNA
tcaacgaccgactccaacaggcacggtaatggacattatatctaggaaagaccaaagaggtagtggacaggtgggaacttatggtctgaacacatttactaacatggaagcccagttagt

SEQ ID NO: 1594 - DNA, 120 bp, synthetic construct
  source 1..120: mol_type = other DNA
tagtggacaggtgggaacttatggtctgaacacatttactaacatggaagcccagttagtcagacaaatggaaggagaaggtgtgctgtcaaaggcagacctcgagaaccctcatctgcc

SEQ ID NO: 1595 - DNA, 120 bp, synthetic construct
  source 1..120: mol_type = other DNA
cagacaaatggaaggagaaggtgtgctgtcaaaggcagacctcgagaaccctcatctgccagaaaagaaaattacacaatggctggaaaccaaaggagtggagaggttaaaaagaatggc

SEQ ID NO: 1596 - DNA, 120 bp, synthetic construct
  source 1..120: mol_type = other DNA
agaaaagaaaattacacaatggctggaaaccaaaggagtggagaggttaaaaagaatggccattagcggggatgattgcgtagtgaaaccaatcgatgacaggttcgctaacgccctgct

SEQ ID NO: 1597 - DNA, 120 bp, synthetic construct
  source 1..120: mol_type = other DNA
cattagcggggatgattgcgtagtgaaaccaatcgatgacaggttcgctaacgccctgcttgctctgaacgatatgggaaaggttcggaaagacatacctcaatggcagccatcaaaagg

SEQ ID NO: 1598 - DNA, 120 bp, synthetic construct
  source 1..120: mol_type = other DNA
tgctctgaacgatatgggaaaggttcggaaagacatacctcaatggcagccatcaaaaggatggcatgactggcagcaggttcctttctgctcccaccactttcatgaattgatcatgaa

SEQ ID NO: 1599 - DNA, 120 bp, synthetic construct
  source 1..120: mol_type = other DNA
atggcatgactggcagcaggttcctttctgctcccaccactttcatgaattgatcatgaaagatggaagaaagttggtggttccctgcagaccccaggacgaactaataggaagagcaag

SEQ ID NO: 1600 - DNA, 120 bp, synthetic construct
  source 1..120: mol_type = other DNA
agatggaagaaagttggtggttccctgcagaccccaggacgaactaataggaagagcaagaatctctcaaggagcgggatggagccttagagaaaccgcatgtttagggaaagcctacgc

SEQ ID NO: 1601 - DNA, 120 bp, synthetic construct
  source 1..120: mol_type = other DNA
aatctctcaaggagcgggatggagccttagagaaaccgcatgtttagggaaagcctacgcccaaatgtggagtctcatgtattttcacagaagagatctcagactagcgtccaatgccat

SEQ ID NO: 1602 - DNA, 120 bp, synthetic construct
  source 1..120: mol_type = other DNA
ccaaatgtggagtctcatgtattttcacagaagagatctcagactagcgtccaatgccatatgttcagcagtaccagtccactgggtccctacaagtagaacgacatggtctattcatgc

SEQ ID NO: 1603 - DNA, 120 bp, synthetic construct
  source 1..120: mol_type = other DNA
atgttcagcagtaccagtccactgggtccctacaagtagaacgacatggtctattcatgctcaccatcagtggatgaccacagaggacatgcttactgtttggaacagggtgtggattga

SEQ ID NO: 1604 - DNA, 120 bp, synthetic construct
  source 1..120: mol_type = other DNA
tcaccatcagtggatgaccacagaggacatgcttactgtttggaacagggtgtggattgaggacaatccatggatggaagacaaaactccaattacaacctgggaaaatgttccatacct

SEQ ID NO: 1605 - DNA, 120 bp, synthetic construct
  source 1..120: mol_type = other DNA
ggacaatccatggatggaagacaaaactccaattacaacctgggaaaatgttccatacctagggaagagggaagaccaatggtgtggatcacttattggtctcacttccagagcaacctg

SEQ ID NO: 1606 - DNA, 120 bp, synthetic construct
  source 1..120: mol_type = other DNA
agggaagagggaagaccaatggtgtggatcacttattggtctcacttccagagcaacctgggcccagaacatacccacagcaattcaacaggtgagaagccttataggcaatgaagagtt

SEQ ID NO: 1607 - DNA, 120 bp, synthetic construct
  source 1..120: mol_type = other DNA
ggcccagaacatacccacagcaattcaacaggtgagaagccttataggcaatgaagagtttctggactacatgccttcaatgaagagattcaggaaggaggaggagtcggagggagccat

SEQ ID NO: 1608 - DNA, 120 bp, synthetic construct
  source 1..120: mol_type = other DNA
tctggactacatgccttcaatgaagagattcaggaaggaggaggagtcggagggagccatttggtaaacgtaggaagtgaaaaagaggctgactgtcaggccaccttaagccacagtacg

SEQ ID NO: 1609 - DNA, 120 bp, synthetic construct
  source 1..120: mol_type = other DNA
ttggtaaacgtaggaagtgaaaaagaggctgactgtcaggccaccttaagccacagtacggaagaagctgtgctgcctgtgagccccgtccaaggacgttaaaagaagaagtcaggcccc

SEQ ID NO: 1610 - DNA, 120 bp, synthetic construct
  source 1..120: mol_type = other DNA
gaagaagctgtgctgcctgtgagccccgtccaaggacgttaaaagaagaagtcaggccccaaagccacggtttgagcaaaccgtgctgcctgtagctccgtcgtggggacgtaaaacctg

SEQ ID NO: 1611 - DNA, 120 bp, synthetic construct
  source 1..120: mol_type = other DNA
aaagccacggtttgagcaaaccgtgctgcctgtagctccgtcgtggggacgtaaaacctgggaggctgcaaactgtggaagctgtacgcacggtgtagcagactagtggttagaggagac

SEQ ID NO: 1612 - DNA, 120 bp, synthetic construct
  source 1..120: mol_type = other DNA
ggaggctgcaaactgtggaagctgtacgcacggtgtagcagactagtggttagaggagacccctcccatgacacaacgcagcagcggggcccgagcactgagggaagctgtacctccttg

SEQ ID NO: 1613 - DNA, 120 bp, synthetic construct
  source 1..120: mol_type = other DNA
ccctcccatgacacaacgcagcagcggggcccgagcactgagggaagctgtacctccttgcaaaggactagaggttagaggagaccccccgcaaacaaaaacagcatattgacgctggga

SEQ ID NO: 1614 - DNA, 120 bp, synthetic construct
  source 1..120: mol_type = other DNA
caaaggactagaggttagaggagaccccccgcaaacaaaaacagcatattgacgctgggagagaccagagatcctgctgtctcctcagcatcattccaggcacagaacgccagaaaatgg

SEQ ID NO: 1615 - DNA, 120 bp, synthetic construct
  source 1..120: mol_type = other DNA
cccgcaaacaaaaacagcatattgacgctgggagagaccagagatcctgctgtctcctcagcatcattccaggcacagaacgccagaaaatggaatggtgctgttgaatcaacaggttct

SEQ ID NO: 1616 - DNA, 120 bp, synthetic construct
  source 1..120: mol_type = other DNA
agttgttagtctgtgtggaccgacaaggacagttccaaatcggaagcttgcttaacacagttctaacagtttgtttaaatagagagcagatctctggaaaaatgaaccaacgaaaaaagg

SEQ ID NO: 1617 - DNA, 120 bp, synthetic construct
  source 1..120: mol_type = other DNA
ttctaacagtttgtttaaatagagagcagatctctggaaaaatgaaccaacgaaaaaaggtggtcagaccacctttcaatatgctgaaacgcgagagaaaccgcgtatctacccctcaag

SEQ ID NO: 1618 - DNA, 120 bp, synthetic construct
  source 1..120: mol_type = other DNA
tggtcagaccacctttcaatatgctgaaacgcgagagaaaccgcgtatctacccctcaagggttgggaaagagattctcaaccggacttttctccgggaaaggacccttgcggatggtgc

SEQ ID NO: 1619 - DNA, 120 bp, synthetic construct
  source 1..120: mol_type = other DNA
ggttgggaaagagattctcaaccggacttttctccgggaaaggacccttgcggatggtgctagcattcatcacgtttttgcgggtcctttccatcccaccaacagcagggattctgaaaa

SEQ ID NO: 1620 - DNA, 120 bp, synthetic construct
  source 1..120: mol_type = other DNA
tagcattcatcacgtttttgcgggtcctttccatcccaccaacagcagggattctgaaaagatggggacagttgaaaaagaacaaggccgtcaaaatactgattggattcaggaaggaga

SEQ ID NO: 1621 - DNA, 120 bp, synthetic construct
  source 1..120: mol_type = other DNA
gatggggacagttgaaaaagaacaaggccgtcaaaatactgattggattcaggaaggagataggtcgcatgttaaacatcttgaataggagaagaaggtcaacaatgacattgctgtgtt

SEQ ID NO: 1622 - DNA, 120 bp, synthetic construct
  source 1..120: mol_type = other DNA
taggtcgcatgttaaacatcttgaataggagaagaaggtcaacaatgacattgctgtgtttgattcccaccgtaatggcgtttcacctgtcaacaagagatggcgaacccctcatgatag

SEQ ID NO: 1623 - DNA, 120 bp, synthetic construct
  source 1..120: mol_type = other DNA
tgattcccaccgtaatggcgtttcacctgtcaacaagagatggcgaacccctcatgatagtggcaaaacacgaaagggggggacctcttttgtttaagataacagaaggaatcaacaaat

SEQ ID NO: 1624 - DNA, 120 bp, synthetic construct
  source 1..120: mol_type = other DNA
tggcaaaacacgaaagggggggacctcttttgtttaagataacagaaggaatcaacaaatgtacccttattgctatggacctgggtgaaatgtgcgaagacactgtcacgtataagtgtc

SEQ ID NO: 1625 - DNA, 120 bp, synthetic construct
  source 1..120: mol_type = other DNA
gtacccttattgctatggacctgggtgaaatgtgcgaagacactgtcacgtataagtgtcctctactggttaacaccgaacctgaggacattgactgctggtgcaatctcacgtccacct

SEQ ID NO: 1626 - DNA, 120 bp, synthetic construct
  source 1..120: mol_type = other DNA
ctctactggttaacaccgaacctgaggacattgactgctggtgcaatctcacgtccacctgggtcatgtacgggacatgcacccagaacggagaacggagacgagagaagcgctcagtag

SEQ ID NO: 1627 - DNA, 120 bp, synthetic construct
  source 1..120: mol_type = other DNA
gggtcatgtacgggacatgcacccagaacggagaacggagacgagagaagcgctcagtagctttaacaccacattcaggaatgggattggaaacaagagctgagacatggatgtcatcgg

SEQ ID NO: 1628 - DNA, 120 bp, synthetic construct
  source 1..120: mol_type = other DNA
ctttaacaccacattcaggaatgggattggaaacaagagctgagacatggatgtcatcggaaggggcttggaaacatgctcagagagtagaaagctggatactcagaaacccaggattcg

SEQ ID NO: 1629 - DNA, 120 bp, synthetic construct
  source 1..120: mol_type = other DNA
aaggggcttggaaacatgctcagagagtagaaagctggatactcagaaacccaggattcgcgctcttggccggatttatggcttacatgattgggcaaacaggaatccagcgaactgttt

SEQ ID NO: 1630 - DNA, 120 bp, synthetic construct
  source 1..120: mol_type = other DNA
cgctcttggccggatttatggcttacatgattgggcaaacaggaatccagcgaactgttttctttgtcctgatgatgctagtcgccccatcctacggaatgcgatgcgtaggggtaggga

SEQ ID NO: 1631 - DNA, 120 bp, synthetic construct
  source 1..120: mol_type = other DNA
tctttgtcctgatgatgctagtcgccccatcctacggaatgcgatgcgtaggggtagggaacagagactttgtggaaggagtctcgggtggagcatgggtcgacttggtgctagaacatg

SEQ ID NO: 1632 - DNA, 120 bp, synthetic construct
  source 1..120: mol_type = other DNA
acagagactttgtggaaggagtctcgggtggagcatgggtcgacttggtgctagaacatggaggatgcgtcacaaccatggcccagggaaaaccaaccctggattttgaattgaccaaga

SEQ ID NO: 1633 - DNA, 120 bp, synthetic construct
  source 1..120: mol_type = other DNA
gaggatgcgtcacaaccatggcccagggaaaaccaaccctggattttgaattgaccaagacaacagccaaggaagtggctctgttaagaacctattgcattgaagcctcgatatcaaaca

SEQ ID NO: 1634 - DNA, 120 bp, synthetic construct
  source 1..120: mol_type = other DNA
caacagccaaggaagtggctctgttaagaacctattgcattgaagcctcgatatcaaacataaccacggcaacaagatgtccaacgcaacgcaatcaccgactcgacccattgcaagacc

SEQ ID NO: 1635 - DNA, 120 bp, synthetic construct
  source 1..120: mol_type = other DNA
taaccacggcaacaagatgtccaacgcaacgcaatcaccgactcgacccattgcaagaccaacagtacatttgccgtagagacgtggtagacagagggtggggcaatggctgtggcttat

SEQ ID NO: 1636 - DNA, 120 bp, synthetic construct
  source 1..120: mol_type = other DNA
aacagtacatttgccgtagagacgtggtagacagagggtggggcaatggctgtggcttatttggaaaaggaggagttgtgacatgtgcgaagtttttatgctcggggaaaataacaggca

SEQ ID NO: 1637 - DNA, 120 bp, synthetic construct
  source 1..120: mol_type = other DNA
ttggaaaaggaggagttgtgacatgtgcgaagtttttatgctcggggaaaataacaggcaatctggtccaagttgaaaaccttgaatatacagtagtagtaacagtccacaatggagaca

SEQ ID NO: 1638 - DNA, 120 bp, synthetic construct
  source 1..120: mol_type = other DNA
atctggtccaagttgaaaaccttgaatatacagtagtagtaacagtccacaatggagacacccatgcagtaggaaatgacacgtccaaccatggagtgacagccacgataactcctaggt

SEQ ID NO: 1639 - DNA, 120 bp, synthetic construct
  source 1..120: mol_type = other DNA
cccatgcagtaggaaatgacacgtccaaccatggagtgacagccacgataactcctaggtcaccatcggtagaagttaaattgccggactatggagaactaacactcgactgcgaaccca

SEQ ID NO: 1640 - DNA, 120 bp, synthetic construct
  source 1..120: mol_type = other DNA
caccatcggtagaagttaaattgccggactatggagaactaacactcgactgcgaacccaggtccggaattgattttaatgagatgatcctgatgaaaatgaaaaagaaaacgtggcttg

SEQ ID NO: 1641 - DNA, 120 bp, synthetic construct
  source 1..120: mol_type = other DNA
ggtccggaattgattttaatgagatgatcctgatgaaaatgaaaaagaaaacgtggcttgtgcataagcaatggtttttagacctacctctaccatggacggcaggagcagacacatcag

SEQ ID NO: 1642 - DNA, 120 bp, synthetic construct
  source 1..120: mol_type = other DNA
tgcataagcaatggtttttagacctacctctaccatggacggcaggagcagacacatcagaagttcattggaatcataaagagagaatggtgacatttaaggttcctcatgccaagagac

SEQ ID NO: 1643 - DNA, 120 bp, synthetic construct
  source 1..120: mol_type = other DNA
aagttcattggaatcataaagagagaatggtgacatttaaggttcctcatgccaagagacaggatgtgacagtgctaggatctcaggagggagctatgcactctgccctcgccggagcca

SEQ ID NO: 1644 - DNA, 120 bp, synthetic construct
  source 1..120: mol_type = other DNA
aggatgtgacagtgctaggatctcaggagggagctatgcactctgccctcgccggagccacagaagtggattctggtgatggaaatcacatgtttgcgggacatctcaagtgcaaagaac

SEQ ID NO: 1645 - DNA, 120 bp, synthetic construct
  source 1..120: mol_type = other DNA
cagaagtggattctggtgatggaaatcacatgtttgcgggacatctcaagtgcaaagaacaatggctaaaattgagaattaaaggaatgtcatacacgatgtgttcaggaaagttctcaa

SEQ ID NO: 1646 - DNA, 120 bp, synthetic construct
  source 1..120: mol_type = other DNA
aatggctaaaattgagaattaaaggaatgtcatacacgatgtgttcaggaaagttctcaattgacaaagagatggcagaaacacagcatggaacaacagtggtgaaagtcaagtatgaag

SEQ ID NO: 1647 - DNA, 120 bp, synthetic construct
  source 1..120: mol_type = other DNA
ttgacaaagagatggcagaaacacagcatggaacaacagtggtgaaagtcaagtatgaaggcgctggagctccgtgtaaagtccccatagagataagagatgtgaacaaggaaaaagtgg

SEQ ID NO: 1648 - DNA, 120 bp, synthetic construct
  source 1..120: mol_type = other DNA
gcgctggagctccgtgtaaagtccccatagagataagagatgtgaacaaggaaaaagtggtcgggcgtatcatctcatctaccccttttgctgagaataccaacagcgtaaccaacatag

SEQ ID NO: 1649 - DNA, 120 bp, synthetic construct
  source 1..120: mol_type = other DNA
tcgggcgtatcatctcatctaccccttttgctgagaataccaacagcgtaaccaacatagaattagaacccccttttggggacagctacatagtgataggtgttggggagagtgcattaa

SEQ ID NO: 1650 - DNA, 120 bp, synthetic construct
  source 1..120: mol_type = other DNA
aattagaacccccttttggggacagctacatagtgataggtgttggggagagtgcattaacactccattggttcagaaaagggagctccattggcaagatgtttgagtccacatacagag

SEQ ID NO: 1651 - DNA, 120 bp, synthetic construct
  source 1..120: mol_type = other DNA
cactccattggttcagaaaagggagctccattggcaagatgtttgagtccacatacagaggtgcaaaacgaatggccattctaggtgaaacagcttgggattttggttctgttggtggac

SEQ ID NO: 1652 - DNA, 120 bp, synthetic construct
  source 1..120: mol_type = other DNA
gtgcaaaacgaatggccattctaggtgaaacagcttgggattttggttctgttggtggactgttcacatcattgggaaaggctgtacaccaggtttttggaagtgtgtatacaaccatgt

SEQ ID NO: 1653 - DNA, 120 bp, synthetic construct
  source 1..120: mol_type = other DNA
tgttcacatcattgggaaaggctgtacaccaggtttttggaagtgtgtatacaaccatgtttggaggggtctcatggatggttagaatcctaattgggttcttagtattgtggattggca

SEQ ID NO: 1654 - DNA, 120 bp, synthetic construct
  source 1..120: mol_type = other DNA
ttggaggggtctcatggatggttagaatcctaattgggttcttagtattgtggattggcacgaattcaagaaacacttcaatggcaatgacgtgcatagctgttggaggaatcactctgt

SEQ ID NO: 1655 - DNA, 120 bp, synthetic construct
  source 1..120: mol_type = other DNA
cgaattcaagaaacacttcaatggcaatgacgtgcatagctgttggaggaatcactctgtttctaggcttcacagttcaagcagacatgggttgtgtggtgtcatggaatgggaaggaat

SEQ ID NO: 1656 - DNA, 120 bp, synthetic construct
  source 1..120: mol_type = other DNA
ttctaggcttcacagttcaagcagacatgggttgtgtggtgtcatggaatgggaaggaattaaaatgtggaagcggaatctttgtggttgacaacgtgcacacttggacagaacagtaca

SEQ ID NO: 1657 - DNA, 120 bp, synthetic construct
  source 1..120: mol_type = other DNA
taaaatgtggaagcggaatctttgtggttgacaacgtgcacacttggacagaacagtacaaatttcaaccagagtccccagcgagactagcgtctgcaatattgaatgcccacaaagatg

SEQ ID NO: 1658 - DNA, 120 bp, synthetic construct
  source 1..120: mol_type = other DNA
aatttcaaccagagtccccagcgagactagcgtctgcaatattgaatgcccacaaagatggggtctgtggaattagatcaaccacgaggctggaaaatgtcatgtggaagcaaataacca

SEQ ID NO: 1659 - DNA, 120 bp, synthetic construct
  source 1..120: mol_type = other DNA
gggtctgtggaattagatcaaccacgaggctggaaaatgtcatgtggaagcaaataaccaacgagctaaactatgttctctgggaaggaggacatgacctcactgttgtggctggggacg

SEQ ID NO: 1660 - DNA, 120 bp, synthetic construct
  source 1..120: mol_type = other DNA
acgagctaaactatgttctctgggaaggaggacatgacctcactgttgtggctggggacgtgaagggggtgttgaccaaaggcaagagagcactcacacctccagtgaatgatctgaaat

SEQ ID NO: 1661 - DNA, 120 bp, synthetic construct
  source 1..120: mol_type = other DNA
tgaagggggtgttgaccaaaggcaagagagcactcacacctccagtgaatgatctgaaatattcatggaaaacatgggggaaagcaaaaatctttaccccagaagcaagaaatagtacgt

SEQ ID NO: 1662 - DNA, 120 bp, synthetic construct
  source 1..120: mol_type = other DNA
attcatggaaaacatgggggaaagcaaaaatctttaccccagaagcaagaaatagtacgtttttaatagacggaccagacacccccgaatgccccaatgagcgaagagcatggaactttt

SEQ ID NO: 1663 - DNA, 120 bp, synthetic construct
  source 1..120: mol_type = other DNA
ttttaatagacggaccagacacccccgaatgccccaatgagcgaagagcatggaactttttggaggtagaagactatggatttggcatgttcacgaccaacatatggatgaaattccgag

SEQ ID NO: 1664 - DNA, 120 bp, synthetic construct
  source 1..120: mol_type = other DNA
tggaggtagaagactatggatttggcatgttcacgaccaacatatggatgaaattccgagaaggaagttcagaagtgtgtgaccatagattaatgtcggcggcaatcaaagaccagaaag

SEQ ID NO: 1665 - DNA, 120 bp, synthetic construct
  source 1..120: mol_type = other DNA
aaggaagttcagaagtgtgtgaccatagattaatgtcggcggcaatcaaagaccagaaagctgtgcatgccgacatgggttattggatagagagctcaaaaaaccagacctggcagatag

SEQ ID NO: 1666 - DNA, 120 bp, synthetic construct
  source 1..120: mol_type = other DNA
ctgtgcatgccgacatgggttattggatagagagctcaaaaaaccagacctggcagatagagaaagcatcccttattgaagtgaaaacatgtctgtggcccaaaacccacacgctgtgga

SEQ ID NO: 1667 - DNA, 120 bp, synthetic construct
  source 1..120: mol_type = other DNA
agaaagcatcccttattgaagtgaaaacatgtctgtggcccaaaacccacacgctgtggagcaatggagtgctggaaagtcagatgctcattccaagatcatatgcaggccccttttcac

SEQ ID NO: 1668 - DNA, 120 bp, synthetic construct
  source 1..120: mol_type = other DNA
gcaatggagtgctggaaagtcagatgctcattccaagatcatatgcaggccccttttcacagcacaattaccgtcagggctatgccacgcaaaccgtgggcccatggcacctaggcaaat

SEQ ID NO: 1669 - DNA, 120 bp, synthetic construct
  source 1..120: mol_type = other DNA
agcacaattaccgtcagggctatgccacgcaaaccgtgggcccatggcacctaggcaaattagagatagactttggagaatgccccgggacaacagtcgcaattcgggaggattgtgacc

SEQ ID NO: 1670 - DNA, 120 bp, synthetic construct
  source 1..120: mol_type = other DNA
tagagatagactttggagaatgccccgggacaacagtcgcaattcgggaggattgtgaccacagaggcccatctttgagaaccaccaccgcatctggaaaactggtcacgcaatggtgct

SEQ ID NO: 1671 - DNA, 120 bp, synthetic construct
  source 1..120: mol_type = other DNA
acagaggcccatctttgagaaccaccaccgcatctggaaaactggtcacgcaatggtgctgccgctcctgcacgatgcctcccttaaggtttttgggagaagatggatgttggtatggga

SEQ ID NO: 1672 - DNA, 120 bp, synthetic construct
  source 1..120: mol_type = other DNA
gccgctcctgcacgatgcctcccttaaggtttttgggagaagatggatgttggtatgggatggagatcaggcctttgagtgaaaaagaagagaacatggtaaaatcacaggtaacggccg

SEQ ID NO: 1673 - DNA, 120 bp, synthetic construct
  source 1..120: mol_type = other DNA
tggagatcaggcctttgagtgaaaaagaagagaacatggtaaaatcacaggtaacggccggacagggcacatcagaaactttttctatggggctgctatgcctgaccttgtttgtggagg

SEQ ID NO: 1674 - DNA, 120 bp, synthetic construct
  source 1..120: mol_type = other DNA
gacagggcacatcagaaactttttctatggggctgctatgcctgaccttgtttgtggaggaatgcttgaggagaagagtcactaggaaacacatgatattggttgtggtaatcacctttt

SEQ ID NO: 1675 - DNA, 120 bp, synthetic construct
  source 1..120: mol_type = other DNA
aatgcttgaggagaagagtcactaggaaacacatgatattggttgtggtaatcaccttttgtgctatcatcctaggaggtcttacatggatggatttactacgagcccttatcatgttag

SEQ ID NO: 1676 - DNA, 120 bp, synthetic construct
  source 1..120: mol_type = other DNA
gtgctatcatcctaggaggtcttacatggatggatttactacgagcccttatcatgttaggggatactatgtctggtagaataggaggacagattcacctagccatcatggcagtgttca

SEQ ID NO: 1677 - DNA, 120 bp, synthetic construct
  source 1..120: mol_type = other DNA
gggatactatgtctggtagaataggaggacagattcacctagccatcatggcagtgttcaagatgtcaccaggatatgtgctgggtgtgtttttaaggaaactcacttcaagagagacag

SEQ ID NO: 1678 - DNA, 120 bp, synthetic construct
  source 1..120: mol_type = other DNA
agatgtcaccaggatatgtgctgggtgtgtttttaaggaaactcacttcaagagagacagcactaatggtaataggaatggccatgacaacggtgttttcaatcccacatgacctcatgg

SEQ ID NO: 1679 - DNA, 120 bp, synthetic construct
  source 1..120: mol_type = other DNA
cactaatggtaataggaatggccatgacaacggtgttttcaatcccacatgacctcatggaactcattgatggaatatcattggggttgatattactaaaaatagtaacacattttgata

SEQ ID NO: 1680 - DNA, 120 bp, synthetic construct
  source 1..120: mol_type = other DNA
aactcattgatggaatatcattggggttgatattactaaaaatagtaacacattttgataacacccaagtgggaaccctagccctttccttgacttttttaagatcaacaataccattag

SEQ ID NO: 1681 - DNA, 120 bp, synthetic construct
  source 1..120: mol_type = other DNA
acacccaagtgggaaccctagccctttccttgacttttttaagatcaacaataccattagtcatggcttggaggaccatcatggctgtgttctttgtggtcacactcattcctttgtgca

SEQ ID NO: 1682 - DNA, 120 bp, synthetic construct
  source 1..120: mol_type = other DNA
tcatggcttggaggaccatcatggctgtgttctttgtggtcacactcattcctttgtgcaggacaagctgtctccaaaaacagtcccattgggtagaaataacagcactcatcctgggag

SEQ ID NO: 1683 - DNA, 120 bp, synthetic construct
  source 1..120: mol_type = other DNA
ggacaagctgtctccaaaaacagtcccattgggtagaaataacagcactcatcctgggagcccaggctttgccagtgtacctaatgactctcatgaaaggagcctcaaggagatcttggc

SEQ ID NO: 1684 - DNA, 120 bp, synthetic construct
  source 1..120: mol_type = other DNA
cccaggctttgccagtgtacctaatgactctcatgaaaggagcctcaaggagatcttggcctcttaatgagggcataatggcagtaggtttggtaagcctcttaggaagcgccctcttga

SEQ ID NO: 1685 - DNA, 120 bp, synthetic construct
  source 1..120: mol_type = other DNA
ctcttaatgagggcataatggcagtaggtttggtaagcctcttaggaagcgccctcttgaagaatgatgttcctttggctggcccaatggtggcaggaggcttgcttctagcggcttacg

SEQ ID NO: 1686 - DNA, 120 bp, synthetic construct
  source 1..120: mol_type = other DNA
agaatgatgttcctttggctggcccaatggtggcaggaggcttgcttctagcggcttacgtaatgagtggtagctcagcagacctgtcactagagaaagctgccaacgtgcagtgggatg

SEQ ID NO: 1687 - DNA, 120 bp, synthetic construct
  source 1..120: mol_type = other DNA
taatgagtggtagctcagcagacctgtcactagagaaagctgccaacgtgcagtgggatgaaatggcggacataactggctcaagcccaatcatagaagtgaagcaggatgaagatggct

SEQ ID NO: 1688 - DNA, 120 bp, synthetic construct
  source 1..120: mol_type = other DNA
aaatggcggacataactggctcaagcccaatcatagaagtgaagcaggatgaagatggctctttctccatacgggacgtcgaggaaaccaatatgataactctcttggtgaaactggcac

SEQ ID NO: 1689 - DNA, 120 bp, synthetic construct
  source 1..120: mol_type = other DNA
ctttctccatacgggacgtcgaggaaaccaatatgataactctcttggtgaaactggcactgataacagtatcaggtctttaccccttggcaattccagtcacaatggcattatggtata

SEQ ID NO: 1690 - DNA, 120 bp, synthetic construct
  source 1..120: mol_type = other DNA
tgataacagtatcaggtctttaccccttggcaattccagtcacaatggcattatggtatatttggcaagtgaagacacaaagatcaggagctctgtgggacgtcccctcacccgctgcca

SEQ ID NO: 1691 - DNA, 120 bp, synthetic construct
  source 1..120: mol_type = other DNA
tttggcaagtgaagacacaaagatcaggagctctgtgggacgtcccctcacccgctgccacccagaaagccacactgtctgaaggagtgtacaggatcatgcaaagagggctgtttggga

SEQ ID NO: 1692 - DNA, 120 bp, synthetic construct
  source 1..120: mol_type = other DNA
cccagaaagccacactgtctgaaggagtgtacaggatcatgcaaagagggctgtttgggaagactcaggttggagtaggaatacacatggaaggcgtatttcacacaatgtggcatgtga

SEQ ID NO: 1693 - DNA, 120 bp, synthetic construct
  source 1..120: mol_type = other DNA
agactcaggttggagtaggaatacacatggaaggcgtatttcacacaatgtggcatgtgacaagaggatcagtgatctgtcatgagacagggagattagagccatcttgggctgacgtca

SEQ ID NO: 1694 - DNA, 120 bp, synthetic construct
  source 1..120: mol_type = other DNA
caagaggatcagtgatctgtcatgagacagggagattagagccatcttgggctgacgtcaggagcgacatgatatcatacggtgggggatggaggcttggagacaaatgggacaaagaag

SEQ ID NO: 1695 - DNA, 120 bp, synthetic construct
  source 1..120: mol_type = other DNA
ggagcgacatgatatcatacggtgggggatggaggcttggagacaaatgggacaaagaagaagatgttcaggtcttagccatagaaccagggaaaaatcccaaacatgtccaaacgaaac

SEQ ID NO: 1696 - DNA, 120 bp, synthetic construct
  source 1..120: mol_type = other DNA
aagatgttcaggtcttagccatagaaccagggaaaaatcccaaacatgtccaaacgaaacctggccttttcaagaccctaactggagaaattggagcagtaactctggatttcaaacccg

SEQ ID NO: 1697 - DNA, 120 bp, synthetic construct
  source 1..120: mol_type = other DNA
ctggccttttcaagaccctaactggagaaattggagcagtaactctggatttcaaacccggaacgtctggctctcctatcattaacaagaaagggaaagttattggactctatggaaatg

SEQ ID NO: 1698 - DNA, 120 bp, synthetic construct
  source 1..120: mol_type = other DNA
gaacgtctggctctcctatcattaacaagaaagggaaagttattggactctatggaaatggagtagttaccaaatcaggtgattatgtcagtgccataacgcaagccgaaaaaattggtg

SEQ ID NO: 1699 - DNA, 120 bp, synthetic construct
  source 1..120: mol_type = other DNA
gagtagttaccaaatcaggtgattatgtcagtgccataacgcaagccgaaaaaattggtgagccagattatgaagtagatgaggacatttttcgaaaaaaaagaaaaaccataatggatt

SEQ ID NO: 1700 - DNA, 120 bp, synthetic construct
  source 1..120: mol_type = other DNA
agccagattatgaagtagatgaggacatttttcgaaaaaaaagaaaaaccataatggatttacaccccggagctggaaagacaaaaagaattctcccatctatagtcagagaggctttaa

SEQ ID NO: 1701 - DNA, 120 bp, synthetic construct
  source 1..120: mol_type = other DNA
tacaccccggagctggaaagacaaaaagaattctcccatctatagtcagagaggctttaaaaaggaggctgcgaacactgattttggctcccacgagagtggtggcggccgagatggaag

SEQ ID NO: 1702 - DNA, 120 bp, synthetic construct
  source 1..120: mol_type = other DNA
aaaggaggctgcgaacactgattttggctcccacgagagtggtggcggccgagatggaagaggcactacgtggattgccaatccgttatcagactccagctgtgaaatcagagcacacag

SEQ ID NO: 1703 - DNA, 120 bp, synthetic construct
  source 1..120: mol_type = other DNA
aggcactacgtggattgccaatccgttatcagactccagctgtgaaatcagagcacacaggaagagagattgtagacctcatgtgtcatgcaaccttcacaacaagacttttgtcatcga

SEQ ID NO: 1704 - DNA, 120 bp, synthetic construct
  source 1..120: mol_type = other DNA
gaagagagattgtagacctcatgtgtcatgcaaccttcacaacaagacttttgtcatcgaccagagttccagcttgcaacctcatagtgatggatgaagcacatttcactgacccttgca

SEQ ID NO: 1705 - DNA, 120 bp, synthetic construct
  source 1..120: mol_type = other DNA
ccagagttccagcttgcaacctcatagtgatggatgaagcacatttcactgacccttgcagtgttgcggctagaggatacatttcaaccagggtggaaatgggagaggcagcagctatct

SEQ ID NO: 1706 - DNA, 120 bp, synthetic construct
  source 1..120: mol_type = other DNA
gtgttgcggctagaggatacatttcaaccagggtggaaatgggagaggcagcagctatcttcatgactgcaacccctcctggagcgacagatcccttcccccagagtaacagcccaatag

SEQ ID NO: 1707 - DNA, 120 bp, synthetic construct
  source 1..120: mol_type = other DNA
tcatgactgcaacccctcctggagcgacagatcccttcccccagagtaacagcccaatagaagacattgagagggaaattccagaaaggtcatggaatacagggttcgactggataacag

SEQ ID NO: 1708 - DNA, 120 bp, synthetic construct
  source 1..120: mol_type = other DNA
aagacattgagagggaaattccagaaaggtcatggaatacagggttcgactggataacagactaccaagggaaaactgtgtggtttgttcccagcataaaagctggaaatgacattgcaa

SEQ ID NO: 1709 - DNA, 120 bp, synthetic construct
  source 1..120: mol_type = other DNA
actaccaagggaaaactgtgtggtttgttcccagcataaaagctggaaatgacattgcaaattgtttgagaaagtcgggaaagagagtgatccagatgctgtggtggtcctttgacacag

SEQ ID NO: 1710 - DNA, 120 bp, synthetic construct
  source 1..120: mol_type = other DNA
attgtttgagaaagtcgggaaagagagtgatccagatgctgtggtggtcctttgacacagagtatccaaagacgaaactcacggactgggattttgtggtcaccacagacatatctgaaa

SEQ ID NO: 1711 - DNA, 120 bp, synthetic construct
  source 1..120: mol_type = other DNA
agtatccaaagacgaaactcacggactgggattttgtggtcaccacagacatatctgaaatgggggccaatttcagagctgggagagtgatagaccccaggagatgcctcaagccagtta

SEQ ID NO: 1712 - DNA, 120 bp, synthetic construct
  source 1..120: mol_type = other DNA
tgggggccaatttcagagctgggagagtgatagaccccaggagatgcctcaagccagttatcctaacagatgggccagagagagttattctagcaggtccaatcccagtaactccagcaa

SEQ ID NO: 1713 - DNA, 120 bp, synthetic construct
  source 1..120: mol_type = other DNA
tcctaacagatgggccagagagagttattctagcaggtccaatcccagtaactccagcaagtgccgctcagagaagagggcgaataggtaggaatccagcacaggaagatgaccaatatg

SEQ ID NO: 1714 - DNA, 120 bp, synthetic construct
  source 1..120: mol_type = other DNA
gtgccgctcagagaagagggcgaataggtaggaatccagcacaggaagatgaccaatatgttttctccggagacccactaaaaaatgatgaagatcatgctcactggacagaagcaaaga

SEQ ID NO: 1715 - DNA, 120 bp, synthetic construct
  source 1..120: mol_type = other DNA
ttttctccggagacccactaaaaaatgatgaagatcatgctcactggacagaagcaaagatgctgcttgacaacatctacacccctgaagggataattccaacactgtttggtccggaaa

SEQ ID NO: 1716 - DNA, 120 bp, synthetic construct
  source 1..120: mol_type = other DNA
tgctgcttgacaacatctacacccctgaagggataattccaacactgtttggtccggaaagggaaaaaacccaagccattgatggagagtttcgcctcagagggaacaaaaggaagactt

SEQ ID NO: 1717 - DNA, 120 bp, synthetic construct
  source 1..120: mol_type = other DNA
gggaaaaaacccaagccattgatggagagtttcgcctcagagggaacaaaaggaagacttttgtggaattaatgaggagaggagaccttccggtgtggctgagctacaaggtagcttctg

SEQ ID NO: 1718 - DNA, 120 bp, synthetic construct
  source 1..120: mol_type = other DNA
ttgtggaattaatgaggagaggagaccttccggtgtggctgagctacaaggtagcttctgccggtatctcttacaaagatcgagaatggtgcttcacaggagaaaggaataaccaaattt

SEQ ID NO: 1719 - DNA, 120 bp, synthetic construct
  source 1..120: mol_type = other DNA
ccggtatctcttacaaagatcgagaatggtgcttcacaggagaaaggaataaccaaattttagaagaaaacatggaggttgaaatttggaccaaagagggagaaaagaaaaagctaaggc

SEQ ID NO: 1720 - DNA, 120 bp, synthetic construct
  source 1..120: mol_type = other DNA
tagaagaaaacatggaggttgaaatttggaccaaagagggagaaaagaaaaagctaaggccaaaatggttagatgcacgtgtgtacgctgatcccatggctttgaaagatttcaaggagt

SEQ ID NO: 1721 - DNA, 120 bp, synthetic construct
  source 1..120: mol_type = other DNA
caaaatggttagatgcacgtgtgtacgctgatcccatggctttgaaagatttcaaggagtttgccagtggaagaaagagcataactctcgacattctaacagagattgccagtctgccaa

SEQ ID NO: 1722 - DNA, 120 bp, synthetic construct
  source 1..120: mol_type = other DNA
ttgccagtggaagaaagagcataactctcgacattctaacagagattgccagtctgccaacttacctttcctctaaggccaagctggcccttgacaacatagtcatgctccacacaacag

SEQ ID NO: 1723 - DNA, 120 bp, synthetic construct
  source 1..120: mol_type = other DNA
cttacctttcctctaaggccaagctggcccttgacaacatagtcatgctccacacaacagaaaaaggagggagggcctaccaacacgccctgaatgaactcccggagtcactggaaacac

SEQ ID NO: 1724 - DNA, 120 bp, synthetic construct
  source 1..120: mol_type = other DNA
aaaaaggagggagggcctaccaacacgccctgaatgaactcccggagtcactggaaacactcatgcttgtagctctactaggagccatgggatcaggcatcttcctgtttttcatgcagg

SEQ ID NO: 1725 - DNA, 120 bp, synthetic construct
  source 1..120: mol_type = other DNA
tcatgcttgtagctctactaggagccatgggatcaggcatcttcctgtttttcatgcaggggaaaggaataggaaaattgtcaatgggtctaatagctatagctgtggctagtggcttgc

SEQ ID NO: 1726 - DNA, 120 bp, synthetic construct
  source 1..120: mol_type = other DNA
ggaaaggaataggaaaattgtcaatgggtctaatagctatagctgtggctagtggcttgctctgggtagcagaaattcagccccagtggatagcagcttcaatcatactggagttctttc

SEQ ID NO: 1727 - DNA, 120 bp, synthetic construct
  source 1..120: mol_type = other DNA
tctgggtagcagaaattcagccccagtggatagcagcttcaatcatactggagttctttctgatggtgctgttgataccagaaccagaaaaacagaggaccccacaagacaatcaattta

SEQ ID NO: 1728 - DNA, 120 bp, synthetic construct
  source 1..120: mol_type = other DNA
tgatggtgctgttgataccagaaccagaaaaacagaggaccccacaagacaatcaatttatctatgtcatattgaccattctcaccatcatcggtcttatagcagccaatgagatggggc

SEQ ID NO: 1729 - DNA, 120 bp, synthetic construct
  source 1..120: mol_type = other DNA
tctatgtcatattgaccattctcaccatcatcggtcttatagcagccaatgagatggggctgattgaaaaaacaaaaactgactttgggttttaccaggtaaaaacagaaaccactattc

SEQ ID NO: 1730 - DNA, 120 bp, synthetic construct
  source 1..120: mol_type = other DNA
tgattgaaaaaacaaaaactgactttgggttttaccaggtaaaaacagaaaccactattcttgatgtggatttgagaccagcctcagcatggacactctatgcggtagccaccaccattc

SEQ ID NO: 1731 - DNA, 120 bp, synthetic construct
  source 1..120: mol_type = other DNA
ttgatgtggatttgagaccagcctcagcatggacactctatgcggtagccaccaccattctgactcccatgctgagacacaccatagaaaacacgtctgccaacctatctctagcagcca

SEQ ID NO: 1732 - DNA, 120 bp, synthetic construct
  source 1..120: mol_type = other DNA
tgactcccatgctgagacacaccatagaaaacacgtctgccaacctatctctagcagccattgccaatcaagcagctgtcctaatgggacttggaaaaggatggccgctccacagaatgg

SEQ ID NO: 1733 - DNA, 120 bp, synthetic construct
  source 1..120: mol_type = other DNA
ttgccaatcaagcagctgtcctaatgggacttggaaaaggatggccgctccacagaatggaccttggtgtgccgctgttagcaataggatgttattctcaagtgaacccaacaacctcga

SEQ ID NO: 1734 - DNA, 120 bp, synthetic construct
  source 1..120: mol_type = other DNA
accttggtgtgccgctgttagcaataggatgttattctcaagtgaacccaacaacctcgacagcatctttagtcagtcttttacgccattatgccataataggtccgggattgcaggcaa

SEQ ID NO: 1735 - DNA, 120 bp, synthetic construct
  source 1..120: mol_type = other DNA
cagcatctttagtcagtcttttacgccattatgccataataggtccgggattgcaggcaaaagccacacgagaggcccagaaaaggacagctgctgggatcatgaagaaccccacggtgg

SEQ ID NO: 1736 - DNA, 120 bp, synthetic construct
  source 1..120: mol_type = other DNA
aagccacacgagaggcccagaaaaggacagctgctgggatcatgaagaaccccacggtggacgggataacagtaatagatctagaaccaatatcctatgacccaaaatttgaaaagcaat

SEQ ID NO: 1737 - DNA, 120 bp, synthetic construct
  source 1..120: mol_type = other DNA
acgggataacagtaatagatctagaaccaatatcctatgacccaaaatttgaaaagcaattagggcaagtcatgctactagtcctgtgtgttggacaattacttttgatgagaacaacat

SEQ ID NO: 1738 - DNA, 120 bp, synthetic construct
  source 1..120: mol_type = other DNA
tagggcaagtcatgctactagtcctgtgtgttggacaattacttttgatgagaacaacatgggctctctgcgaagtcttgactttggccacaggaccagccttgaccttgtgggagggca

SEQ ID NO: 1739 - DNA, 120 bp, synthetic construct
  source 1..120: mol_type = other DNA
gggctctctgcgaagtcttgactttggccacaggaccagccttgaccttgtgggagggcaggggggcaacccgggggaggaagaccatagctgtatccacagccaacattttcagaggaa

SEQ ID NO: 1740 - DNA, 120 bp, synthetic construct
  source 1..120: mol_type = other DNA
ggggggcaacccgggggaggaagaccatagctgtatccacagccaacattttcagaggaagctacttggcaggagctggactagctttttcgctcataaagaatgcacaaacccctagga

SEQ ID NO: 1741 - DNA, 120 bp, synthetic construct
  source 1..120: mol_type = other DNA
gctacttggcaggagctggactagctttttcgctcataaagaatgcacaaacccctaggaggggaactgggaccacaggagagacactgggagagaagtggaagagacagctaaactcat

SEQ ID NO: 1742 - DNA, 120 bp, synthetic construct
  source 1..120: mol_type = other DNA
ggggaactgggaccacaggagagacactgggagagaagtggaagagacagctaaactcattagacagaaaagagtttgaagagtacaaaagaagtggaatacaagaagtggataggactg

SEQ ID NO: 1743 - DNA, 120 bp, synthetic construct
  source 1..120: mol_type = other DNA
tagacagaaaagagtttgaagagtacaaaagaagtggaatacaagaagtggataggactgaagccaagtctgccctaaaagatggatctaaaatcaagcatgcagtgtccagagggtcta

SEQ ID NO: 1744 - DNA, 120 bp, synthetic construct
  source 1..120: mol_type = other DNA
aagccaagtctgccctaaaagatggatctaaaatcaagcatgcagtgtccagagggtctagtaagatcagatggattgttgaaagagggatggtaaagccaaaagggaaggtcgtggatc

SEQ ID NO: 1745 - DNA, 120 bp, synthetic construct
  source 1..120: mol_type = other DNA
gtaagatcagatggattgttgaaagagggatggtaaagccaaaagggaaggtcgtggatcttggttgcgggaggggaggatggtcctattacatggcgacactcaagaacgtgactgaag

SEQ ID NO: 1746 - DNA, 120 bp, synthetic construct
  source 1..120: mol_type = other DNA
ttggttgcgggaggggaggatggtcctattacatggcgacactcaagaacgtgactgaagtgaaaggatatacaaaaggaggtccaggacatgaggaaccaatccccatggctacttatg

SEQ ID NO: 1747 - DNA, 120 bp, synthetic construct
  source 1..120: mol_type = other DNA
tgaaaggatatacaaaaggaggtccaggacatgaggaaccaatccccatggctacttatggctggaacttggtcaaactccattcaggggttgatgtgttttacaaacccactgaacagg

SEQ ID NO: 1748 - DNA, 120 bp, synthetic construct
  source 1..120: mol_type = other DNA
gctggaacttggtcaaactccattcaggggttgatgtgttttacaaacccactgaacaggtggacaccttgctctgtgatattggggagtcgtcctccaatccgacaatagaggaaggaa

SEQ ID NO: 1749 - DNA, 120 bp, synthetic construct
  source 1..120: mol_type = other DNA
tggacaccttgctctgtgatattggggagtcgtcctccaatccgacaatagaggaaggaagaacattgagagccttatctaaagaggagacatggctctcatcaaaacctgagttctgca

SEQ ID NO: 1750 - DNA, 120 bp, synthetic construct
  source 1..120: mol_type = other DNA
gaacattgagagccttatctaaagaggagacatggctctcatcaaaacctgagttctgcatcaaaatcctcaacccctacatgccaacagttatagaagagctggagaaactccagagaa

SEQ ID NO: 1751 - DNA, 120 bp, synthetic construct
  source 1..120: mol_type = other DNA
tcaaaatcctcaacccctacatgccaacagttatagaagagctggagaaactccagagaagatatggtggaagcctcatcagatgccctctatctaggaattctacccatgagatgtatt

SEQ ID NO: 1752 - DNA, 120 bp, synthetic construct
  source 1..120: mol_type = other DNA
gatatggtggaagcctcatcagatgccctctatctaggaattctacccatgagatgtattgggtgtcaggtgcgtcgggaaacatcgtgagttctgtaaacacagtgtcaaagatgctgt

SEQ ID NO: 1753 - DNA, 120 bp, synthetic construct
  source 1..120: mol_type = other DNA
gggtgtcaggtgcgtcgggaaacatcgtgagttctgtaaacacagtgtcaaagatgctgttgaacaggttcacaacaaggcataggaaacctacttatgagaaggacgtggatcttgggg

SEQ ID NO: 1754 - DNA, 120 bp, synthetic construct
  source 1..120: mol_type = other DNA
tgaacaggttcacaacaaggcataggaaacctacttatgagaaggacgtggatcttggggcaggaacaagaagtgtctccactgaaacagaaaaaccagacatgacagttattgggacaa

SEQ ID NO: 1755 - DNA, 120 bp, synthetic construct
  source 1..120: mol_type = other DNA
caggaacaagaagtgtctccactgaaacagaaaaaccagacatgacagttattgggacaatggattggagattgcaagaagagcacaaagaaacctggcactatgaccaggaaaatccat

SEQ ID NO: 1756 - DNA, 120 bp, synthetic construct
  source 1..120: mol_type = other DNA
tggattggagattgcaagaagagcacaaagaaacctggcactatgaccaggaaaatccatacagaacctgggcgtatcatggaagctatgaagctccttcgacaggctcagcatcctcca

SEQ ID NO: 1757 - DNA, 120 bp, synthetic construct
  source 1..120: mol_type = other DNA
acagaacctgggcgtatcatggaagctatgaagctccttcgacaggctcagcatcctccatggtgaacggggtagtaaaactgctgacaaaaccctgggatgtgattccaatggtgaccc

SEQ ID NO: 1758 - DNA, 120 bp, synthetic construct
  source 1..120: mol_type = other DNA
tggtgaacggggtagtaaaactgctgacaaaaccctgggatgtgattccaatggtgacccagctggcaatgacagacacaaccccttttgggcaacaaagagtgttcaaggagaaggtgg

SEQ ID NO: 1759 - DNA, 120 bp, synthetic construct
  source 1..120: mol_type = other DNA
agctggcaatgacagacacaaccccttttgggcaacaaagagtgttcaaggagaaggtggataccagaacaccacaaccaaaacccggcacacgaatgattatgaccacgacagctaatt

SEQ ID NO: 1760 - DNA, 120 bp, synthetic construct
  source 1..120: mol_type = other DNA
ataccagaacaccacaaccaaaacccggcacacgaatgattatgaccacgacagctaattggctgtgggctctcctcgggaagaagaaaaatcccagattgtgtacaagggaagagttca

SEQ ID NO: 1761 - DNA, 120 bp, synthetic construct
  source 1..120: mol_type = other DNA
ggctgtgggctctcctcgggaagaagaaaaatcccagattgtgtacaagggaagagttcatctcaaaagttaggtcaaacgcagccataggcgcagtctttcaggaagagcagggatgga

SEQ ID NO: 1762 - DNA, 120 bp, synthetic construct
  source 1..120: mol_type = other DNA
tctcaaaagttaggtcaaacgcagccataggcgcagtctttcaggaagagcagggatggacatctgccagtgaagctgtgagtgacagccggttctgggaactggttgacaaagaaaggg

SEQ ID NO: 1763 - DNA, 120 bp, synthetic construct
  source 1..120: mol_type = other DNA
catctgccagtgaagctgtgagtgacagccggttctgggaactggttgacaaagaaagggctctgcaccaggaaggaaaatgtgaatcgtgtgtctacaacatgatgggaaaacgtgaga

SEQ ID NO: 1764 - DNA, 120 bp, synthetic construct
  source 1..120: mol_type = other DNA
ctctgcaccaggaaggaaaatgtgaatcgtgtgtctacaacatgatgggaaaacgtgagaaaaaactaggagagtttggtagggccaagggaagccgagcaatctggtacatgtggctgg

SEQ ID NO: 1765 - DNA, 120 bp, synthetic construct
  source 1..120: mol_type = other DNA
aaaaactaggagagtttggtagggccaagggaagccgagcaatctggtacatgtggctgggggcgcgcttcctggaatttgaagccctgggtttcttgaatgaagatcactggtttagca

SEQ ID NO: 1766 - DNA, 120 bp, synthetic construct
  source 1..120: mol_type = other DNA
gggcgcgcttcctggaatttgaagccctgggtttcttgaatgaagatcactggtttagcagagaaaactcatggagtggagtggaaggggaaggtctgcatagattgggatatatcttgg

SEQ ID NO: 1767 - DNA, 120 bp, synthetic construct
  source 1..120: mol_type = other DNA
gagaaaactcatggagtggagtggaaggggaaggtctgcatagattgggatatatcttggaggatatagacaagcaggatggagatctaatatatgctgacgacacagcaggctgggaca

SEQ ID NO: 1768 - DNA, 120 bp, synthetic construct
  source 1..120: mol_type = other DNA
aggatatagacaagcaggatggagatctaatatatgctgacgacacagcaggctgggacacaagaatcactgaggatgaccttttaaatgaagaactgatcacagaacagatggcccccc

SEQ ID NO: 1769 - DNA, 120 bp, synthetic construct
  source 1..120: mol_type = other DNA
caagaatcactgaggatgaccttttaaatgaagaactgatcacagaacagatggccccccatcacaagaccctagccaaagccatattcaaactaacctatcaaaacaaagtggtgaaag

SEQ ID NO: 1770 - DNA, 120 bp, synthetic construct
  source 1..120: mol_type = other DNA
atcacaagaccctagccaaagccatattcaaactaacctatcaaaacaaagtggtgaaagttctcagacccacaccgaaaggagcggtgatggacatcatatccaggaaagaccaaagag

SEQ ID NO: 1771 - DNA, 120 bp, synthetic construct
  source 1..120: mol_type = other DNA
ttctcagacccacaccgaaaggagcggtgatggacatcatatccaggaaagaccaaagaggtagtggacaggttggaacatatggtttaaacacattcactaacatggaagttcaactca

SEQ ID NO: 1772 - DNA, 120 bp, synthetic construct
  source 1..120: mol_type = other DNA
gtagtggacaggttggaacatatggtttaaacacattcactaacatggaagttcaactcatccgtcaaatggaagctgaaggagtcatcacacaagacgacatgcagaacccaaaagggt

SEQ ID NO: 1773 - DNA, 120 bp, synthetic construct
  source 1..120: mol_type = other DNA
tccgtcaaatggaagctgaaggagtcatcacacaagacgacatgcagaacccaaaagggttgaaagaaagagttgagaaatggctgacagagtgtggcgtcgacaggttgaagaggatgg

SEQ ID NO: 1774 - DNA, 120 bp, synthetic construct
  source 1..120: mol_type = other DNA
tgaaagaaagagttgagaaatggctgacagagtgtggcgtcgacaggttgaagaggatggcaatcagtggagatgattgcgtggtgaagcccctagatgagaggttcagcacctccctcc

SEQ ID NO: 1775 - DNA, 120 bp, synthetic construct
  source 1..120: mol_type = other DNA
caatcagtggagatgattgcgtggtgaagcccctagatgagaggttcagcacctccctcctcttcttgaacgacatgggaaaggtgaggaaagacatcccgcagtgggaaccatccaagg

SEQ ID NO: 1776 - DNA, 120 bp, synthetic construct
  source 1..120: mol_type = other DNA
tcttcttgaacgacatgggaaaggtgaggaaagacatcccgcagtgggaaccatccaagggatggaaaaactggcaagaggttcctttttgctcccaccattttcataagatctttatga

SEQ ID NO: 1777 - DNA, 120 bp, synthetic construct
  source 1..120: mol_type = other DNA
gatggaaaaactggcaagaggttcctttttgctcccaccattttcataagatctttatgaaagatggccgctcactagttgttccatgcagaaaccaggatgaactgataggaagagcca

SEQ ID NO: 1778 - DNA, 120 bp, synthetic construct
  source 1..120: mol_type = other DNA
aagatggccgctcactagttgttccatgcagaaaccaggatgaactgataggaagagccagaatctcgcagggggctggatggagcctaagagaaacagcctgttcgggcaaagcttacg

SEQ ID NO: 1779 - DNA, 120 bp, synthetic construct
  source 1..120: mol_type = other DNA
gaatctcgcagggggctggatggagcctaagagaaacagcctgttcgggcaaagcttacgcccaaatgtggtcgcttatgtatttccatagaagggacctgcgtttggcctccatggcca

SEQ ID NO: 1780 - DNA, 120 bp, synthetic construct
  source 1..120: mol_type = other DNA
cccaaatgtggtcgcttatgtatttccatagaagggacctgcgtttggcctccatggccatatgttcagcagttccaacggaatggtttccaacaagcaggacaacatggtcaatccacg

SEQ ID NO: 1781 - DNA, 120 bp, synthetic construct
  source 1..120: mol_type = other DNA
tatgttcagcagttccaacggaatggtttccaacaagcaggacaacatggtcaatccacgctcaccaccagtggatgaccactgaagacatgctcaaagtgtggaacagggtgtggatag

SEQ ID NO: 1782 - DNA, 120 bp, synthetic construct
  source 1..120: mol_type = other DNA
ctcaccaccagtggatgaccactgaagacatgctcaaagtgtggaacagggtgtggatagaagacaaccccaatatgactgacaagactccagtccgttcgtgggaggacataccttacc

SEQ ID NO: 1783 - DNA, 120 bp, synthetic construct
  source 1..120: mol_type = other DNA
aagacaaccccaatatgactgacaagactccagtccgttcgtgggaggacataccttacctagggaaaagagaggatctgtggtgtggatccctgattggactctcttccagagccacct

SEQ ID NO: 1784 - DNA, 120 bp, synthetic construct
  source 1..120: mol_type = other DNA
tagggaaaagagaggatctgtggtgtggatccctgattggactctcttccagagccacctgggcgaagaacattcacacggccataacccaggtcaggaatctgatcggaaaagaggaat

SEQ ID NO: 1785 - DNA, 120 bp, synthetic construct
  source 1..120: mol_type = other DNA
gggcgaagaacattcacacggccataacccaggtcaggaatctgatcggaaaagaggaatacgtggattacatgccagtcatgagaagatacagcgctccttccgaaagtgaaggagttc

SEQ ID NO: 1786 - DNA, 120 bp, synthetic construct
  source 1..120: mol_type = other DNA
acgtggattacatgccagtcatgagaagatacagcgctccttccgaaagtgaaggagttctgtaattactaataacaaacaccaaagagaccattgaagtcaggccacttgtgccacggc

SEQ ID NO: 1787 - DNA, 120 bp, synthetic construct
  source 1..120: mol_type = other DNA
tgtaattactaataacaaacaccaaagagaccattgaagtcaggccacttgtgccacggcttgagcaaaccgtgctgcctgtagctccgccaataatgggaggcgtaaaattcccaggga

SEQ ID NO: 1788 - DNA, 120 bp, synthetic construct
  source 1..120: mol_type = other DNA
ttgagcaaaccgtgctgcctgtagctccgccaataatgggaggcgtaaaattcccagggaggccatgcgccacggaagctgtacgcgtggcatattggactagcggttagaggagacccc

SEQ ID NO: 1789 - DNA, 120 bp, synthetic construct
  source 1..120: mol_type = other DNA
ggccatgcgccacggaagctgtacgcgtggcatattggactagcggttagaggagacccctcccatcaccgacaaaacgcagcaaaaaagggggcccgaagccaggaggaagctgtactt

SEQ ID NO: 1790 - DNA, 120 bp, synthetic construct
  source 1..120: mol_type = other DNA
tcccatcaccgacaaaacgcagcaaaaaagggggcccgaagccaggaggaagctgtacttctggtagaaggactagaggttagaggagacccccccaacacaaaaacagcatattgacgc

SEQ ID NO: 1791 - DNA, 120 bp, synthetic construct
  source 1..120: mol_type = other DNA
ctggtagaaggactagaggttagaggagacccccccaacacaaaaacagcatattgacgctgggacagaccagagatcctgctgtctctgcaacatcaatccaggcacagagcgccgcga

SEQ ID NO: 1792 - DNA, 120 bp, synthetic construct
  source 1..120: mol_type = other DNA
ccccaacacaaaaacagcatattgacgctgggacagaccagagatcctgctgtctctgcaacatcaatccaggcacagagcgccgcgagatggattggtgttgttgatccaacaggttct

SEQ ID NO: 1793 - DNA, 120 bp, synthetic construct
  source 1..120: mol_type = other DNA
tttccatacagcctctgtaaatagttgtgtggggactgagaatatgtgagaattgtcttgtataaattcttaattactgtactgtaataaaaaatatcgtataagttgttgttcagtata

SEQ ID NO: 1794 - DNA, 120 bp, synthetic construct
  source 1..120: mol_type = other DNA
tataaattcttaattactgtactgtaataaaaaatatcgtataagttgttgttcagtataaaattgtgtcatagtcacaatttagaaaaatgcagcttgatacatcatgaacatttaggt

SEQ ID NO: 1795 - DNA, 120 bp, synthetic construct
  source 1..120: mol_type = other DNA
aaattgtgtcatagtcacaatttagaaaaatgcagcttgatacatcatgaacatttaggtcggtatagatttgctaatagcaagtttatattacatagaaagcgtaatgctattcactta

SEQ ID NO: 1796 - DNA, 120 bp, synthetic construct
  source 1..120: mol_type = other DNA
cggtatagatttgctaatagcaagtttatattacatagaaagcgtaatgctattcacttaaattttcatcaaaataaataaacttattttttgtgtacttgtgggattctgcgtctgaat

SEQ ID NO: 1797 - DNA, 120 bp, synthetic construct
  source 1..120: mol_type = other DNA
aattttcatcaaaataaataaacttattttttgtgtacttgtgggattctgcgtctgaatatggaggtttagcagaagttatgttgttccattctttagagaattttttatttatttcat

SEQ ID NO: 1798 - DNA, 120 bp, synthetic construct
  source 1..120: mol_type = other DNA
atggaggtttagcagaagttatgttgttccattctttagagaattttttatttatttcataaaactttttaaggtttttctgttcttcgtttaatgcgctatcattgcattctaatacgt

SEQ ID NO: 1799 - DNA, 120 bp, synthetic construct
  source 1..120: mol_type = other DNA
aaaactttttaaggtttttctgttcttcgtttaatgcgctatcattgcattctaatacgtctcttataaaatcatctgggacgattgcatcgatgggacattctgggacacacacaccac

SEQ ID NO: 1800 - DNA, 120 bp, synthetic construct
  source 1..120: mol_type = other DNA
ctcttataaaatcatctgggacgattgcatcgatgggacattctgggacacacacaccacagtctatacattgatcaggatctattactaacatattagctccttcatagaaacaatcta

SEQ ID NO: 1801 - DNA, 120 bp, synthetic construct
  source 1..120: mol_type = other DNA
agtctatacattgatcaggatctattactaacatattagctccttcatagaaacaatctaccgggcatacttcaacacaatcagtgtatttgcatcttatgcacctatccgttataaagt

SEQ ID NO: 1802 - DNA, 120 bp, synthetic construct
  source 1..120: mol_type = other DNA
ccgggcatacttcaacacaatcagtgtatttgcatcttatgcacctatccgttataaagtgtgtcattacagggttattaataataatgtaacggtttttattgtaatgttttttcttgc

SEQ ID NO: 1803 - DNA, 120 bp, synthetic construct
  source 1..120: mol_type = other DNA
gtgtcattacagggttattaataataatgtaacggtttttattgtaatgttttttcttgccaagttcaattagtatttattattttacaaggtatagatgtggagttgtagttaaactta

SEQ ID NO: 1804 - DNA, 120 bp, synthetic construct
  source 1..120: mol_type = other DNA
caagttcaattagtatttattattttacaaggtatagatgtggagttgtagttaaacttatacatcgtagagttaagtagtttggttaatgtttaggtaacatcctaatacgtatatgag

SEQ ID NO: 1805 - DNA, 120 bp, synthetic construct
  source 1..120: mol_type = other DNA
tacatcgtagagttaagtagtttggttaatgtttaggtaacatcctaatacgtatatgagctatcaattctatagagtatgttattttatgatagagaattgattgtggagttggatttg

SEQ ID NO: 1806 - DNA, 120 bp, synthetic construct
  source 1..120: mol_type = other DNA
ctatcaattctatagagtatgttattttatgatagagaattgattgtggagttggatttggcaatacgtttaaaattaaaggagatttttatggatattgataatagtaacataagtaca

SEQ ID NO: 1807 - DNA, 120 bp, synthetic construct
  source 1..120: mol_type = other DNA
gcaatacgtttaaaattaaaggagatttttatggatattgataatagtaacataagtacagccgatatacggagtaatactgatggcttgatagacataattatgcgtatattaggtttt

SEQ ID NO: 1808 - DNA, 120 bp, synthetic construct
  source 1..120: mol_type = other DNA
gccgatatacggagtaatactgatggcttgatagacataattatgcgtatattaggttttggtaataagaatattgtgcaaccacaggatctgggttctgaaatttatcagcaagagcaa

SEQ ID NO: 1809 - DNA, 120 bp, synthetic construct
  source 1..120: mol_type = other DNA
ggtaataagaatattgtgcaaccacaggatctgggttctgaaatttatcagcaagagcaagaagatgacacagtctctcaaccttcattagagccatttgttgcagaaagtgaagtttct

SEQ ID NO: 1810 - DNA, 120 bp, synthetic construct
  source 1..120: mol_type = other DNA
gaagatgacacagtctctcaaccttcattagagccatttgttgcagaaagtgaagtttctaaagttgaacaagaaaaaactaaccctgaggttttaataaaagatttgcaagatgttgcg

SEQ ID NO: 1811 - DNA, 120 bp, synthetic construct
  source 1..120: mol_type = other DNA
aaagttgaacaagaaaaaactaaccctgaggttttaataaaagatttgcaagatgttgcgagtcatgaatctggtgtatcagatcagccagctcaagttgttacagaaagagaaaatgaa

SEQ ID NO: 1812 - DNA, 120 bp, synthetic construct
  source 1..120: mol_type = other DNA
agtcatgaatctggtgtatcagatcagccagctcaagttgttacagaaagagaaaatgaaattgaatcccatcaaggagaaacagaaaaagaaagtggaataactgaatctcatcagaaa

SEQ ID NO: 1813 - DNA, 120 bp, synthetic construct
  source 1..120: mol_type = other DNA
attgaatcccatcaaggagaaacagaaaaagaaagtggaataactgaatctcatcagaaagaagatgaaatagtatctcaatcttcatcagagccatttgttgcagaaagtgaagtttct

SEQ ID NO: 1814 - DNA, 120 bp, synthetic construct
  source 1..120: mol_type = other DNA
gaagatgaaatagtatctcaatcttcatcagagccatttgttgcagaaagtgaagtttctaaagttgaacaagaagaaactaaccctgaagttttaataaaagatttgcaagatgttgcg

SEQ ID NO: 1815 - DNA, 120 bp, synthetic construct
  source 1..120: mol_type = other DNA
aaagttgaacaagaagaaactaaccctgaagttttaataaaagatttgcaagatgttgcgagtcatgaatctggtgtatcagatcagccagctcaagttgttacagagagagaaagtgaa

SEQ ID NO: 1816 - DNA, 120 bp, synthetic construct
  source 1..120: mol_type = other DNA
agtcatgaatctggtgtatcagatcagccagctcaagttgttacagagagagaaagtgaaattgaatcccatcaaggagaaacagaaaaagaaagtggaataactgaatctcatcagaaa

SEQ ID NO: 1817 - DNA, 120 bp, synthetic construct
  source 1..120: mol_type = other DNA
attgaatcccatcaaggagaaacagaaaaagaaagtggaataactgaatctcatcagaaagaagatgaaatagtatctcaaccttcatcagagccatttgttgcagaaagtgaagtttct

SEQ ID NO: 1818 - DNA, 120 bp, synthetic construct
  source 1..120: mol_type = other DNA
gaagatgaaatagtatctcaaccttcatcagagccatttgttgcagaaagtgaagtttctaaagttgaacaagaagaaactaaccctgaagttttaataaaagatttgcaagatgttgcg

SEQ ID NO: 1819 - DNA, 120 bp, synthetic construct
  source 1..120: mol_type = other DNA
gaagatgaaatagtatctcaaccttcatcagagccatttgttgcagaaagtgaagtttctaaagttgaacaagaaaaaactaaccctgaaattctagtagaagatttgccattaggtcaa

SEQ ID NO: 1820 - DNA, 120 bp, synthetic construct
  source 1..120: mol_type = other DNA
aaagttgaacaagaaaaaactaaccctgaaattctagtagaagatttgccattaggtcaagtgattccggttgttgtagagaaagatgaaatgtttgcaccttcatttaatccaatcgtt

SEQ ID NO: 1821 - DNA, 120 bp, synthetic construct
  source 1..120: mol_type = other DNA
gtgattccggttgttgtagagaaagatgaaatgtttgcaccttcatttaatccaatcgttataaaggaggaagataaagtttgtgaaacttgcgaacaagaatttgagattgtaaaggat

SEQ ID NO: 1822 - DNA, 120 bp, synthetic construct
  source 1..120: mol_type = other DNA
ataaaggaggaagataaagtttgtgaaacttgcgaacaagaatttgagattgtaaaggattcacagactgtaaaaggtagtgaagatataatatcacctatcgaatgcttagaaagtatg

SEQ ID NO: 1823 - DNA, 120 bp, synthetic construct
  source 1..120: mol_type = other DNA
tcacagactgtaaaaggtagtgaagatataatatcacctatcgaatgcttagaaagtatggattctatagtttcaacaatatttgaaagtggaatgttatgtcctatgtcaaaacctgga

SEQ ID NO: 1824 - DNA, 120 bp, synthetic construct
  source 1..120: mol_type = other DNA
gattctatagtttcaacaatatttgaaagtggaatgttatgtcctatgtcaaaacctggacagtatgtttgtgggtatgaaatgtatatgtatggatttcaagatgtgaaagacttatta

SEQ ID NO: 1825 - DNA, 120 bp, synthetic construct
  source 1..120: mol_type = other DNA
cagtatgtttgtgggtatgaaatgtatatgtatggatttcaagatgtgaaagacttattaggtggtttattaagtaatgttcctgtgtgttgtaatgttagcctttattttatggaacat

SEQ ID NO: 1826 - DNA, 120 bp, synthetic construct
  source 1..120: mol_type = other DNA
ggtggtttattaagtaatgttcctgtgtgttgtaatgttagcctttattttatggaacataattactttactaaccatgagaatattaatcacaatgtagtaaatgatattgtataattg

SEQ ID NO: 1827 - DNA, 120 bp, synthetic construct
  source 1..120: mol_type = other DNA
aattactttactaaccatgagaatattaatcacaatgtagtaaatgatattgtataattgtaaggtttagtcttgagatagcaagtgatgcttttattaagtattgcttgctattttttt

SEQ ID NO: 1828 - DNA, 120 bp, synthetic construct
  source 1..120: mol_type = other DNA
taaggtttagtcttgagatagcaagtgatgcttttattaagtattgcttgctatttttttgtttatttacctgctttttatatgggagaaatcatatattaagtgattgaaagtaaaagt

SEQ ID NO: 1829 - DNA, 120 bp, synthetic construct
  source 1..120: mol_type = other DNA
gtttatttacctgctttttatatgggagaaatcatatattaagtgattgaaagtaaaagtggaattttgctgatattataggttataagcaattttttgaagtaaaaatgtatatagtta

SEQ ID NO: 1830 - DNA, 120 bp, synthetic construct
  source 1..120: mol_type = other DNA
ggaattttgctgatattataggttataagcaattttttgaagtaaaaatgtatatagttagtgatatgtactaaaaagtagctgaattttattagtgagttagccattagtcttttgcct

SEQ ID NO: 1831 - DNA, 120 bp, synthetic construct
  source 1..120: mol_type = other DNA
gtgatatgtactaaaaagtagctgaattttattagtgagttagccattagtcttttgcctttttcagaagaactttgctgaaatgattaaaacagagtgatagttgttgttaatgtaatt

SEQ ID NO: 1832 - DNA, 120 bp, synthetic construct
  source 1..120: mol_type = other DNA
ttttcagaagaactttgctgaaatgattaaaacagagtgatagttgttgttaatgtaattgataataaacggtgataggaatataagtcttcgtatatagctattcaatttagtataaag

SEQ ID NO: 1833 - DNA, 120 bp, synthetic construct
  source 1..120: mol_type = other DNA
gataataaacggtgataggaatataagtcttcgtatatagctattcaatttagtataaaggcggaaaattggtgtgtgcataatatctaagtgtttgcttaaggtttgagttttggtaat

SEQ ID NO: 1834 - DNA, 120 bp, synthetic construct
  source 1..120: mol_type = other DNA
gcggaaaattggtgtgtgcataatatctaagtgtttgcttaaggtttgagttttggtaattaagaattaagtgctatcctgcgctattgtaatatgtttacgtatgtaaaagtggacaaa

SEQ ID NO: 1835 - DNA, 120 bp, synthetic construct
  source 1..120: mol_type = other DNA
taagaattaagtgctatcctgcgctattgtaatatgtttacgtatgtaaaagtggacaaagtagacttacctatagcgtggttgggaattaaaaataaaaagctgttctgcgctattgta

SEQ ID NO: 1836 - DNA, 120 bp, synthetic construct
  source 1..120: mol_type = other DNA
gtagacttacctatagcgtggttgggaattaaaaataaaaagctgttctgcgctattgtaatatatttatgtatgtaaaagtatacaaagtaaacttacctatggtgcggttagtaatta

SEQ ID NO: 1837 - DNA, 120 bp, synthetic construct
  source 1..120: mol_type = other DNA
atatatttatgtatgtaaaagtatacaaagtaaacttacctatggtgcggttagtaattaagaattaagtgctatcctgcgctgtaatatgtttacgtatgtaaaagtggacaaagtaga

SEQ ID NO: 1838 - DNA, 120 bp, synthetic construct
  source 1..120: mol_type = other DNA
agaattaagtgctatcctgcgctgtaatatgtttacgtatgtaaaagtggacaaagtagacctacctatggcgtggttgggaattaagaataaaaagctattctacgctgttataatata

SEQ ID NO: 1839 - DNA, 120 bp, synthetic construct
  source 1..120: mol_type = other DNA
cctacctatggcgtggttgggaattaagaataaaaagctattctacgctgttataatatatttatgtatgtaaaagtgtacaaagtaaacttacctatgatgtagttgggaattaagaat

SEQ ID NO: 1840 - DNA, 120 bp, synthetic construct
  source 1..120: mol_type = other DNA
tttatgtatgtaaaagtgtacaaagtaaacttacctatgatgtagttgggaattaagaataaaaagctattctacgctgttataatatatttatgtatgtaaaagtatacaaagtaaact

SEQ ID NO: 1841 - DNA, 120 bp, synthetic construct
  source 1..120: mol_type = other DNA
aaaaagctattctacgctgttataatatatttatgtatgtaaaagtatacaaagtaaacttacctatggtgtagttggtaattaagaattaaatgctattctgcgctgttataatgtatt

SEQ ID NO: 1842 - DNA, 120 bp, synthetic construct
  source 1..120: mol_type = other DNA
tacctatggtgtagttggtaattaagaattaaatgctattctgcgctgttataatgtatttacgtatgttaaaagtgacaaagtaaacttacctatggtgtgaattgaatgttggttaat

SEQ ID NO: 1843 - DNA, 120 bp, synthetic construct
  source 1..120: mol_type = other DNA
tacgtatgttaaaagtgacaaagtaaacttacctatggtgtgaattgaatgttggttaattacactttaatcacagcttgcgtcttataagaaaattactgtttatcattttttatatct

SEQ ID NO: 1844 - DNA, 120 bp, synthetic construct
  source 1..120: mol_type = other DNA
tacactttaatcacagcttgcgtcttataagaaaattactgtttatcattttttatatcttgatccttgacaggtttttcattgtgattgtcaaaatcattttcatggtgtgagttgctt

SEQ ID NO: 1845 - DNA, 120 bp, synthetic construct
  source 1..120: mol_type = other DNA
tgatccttgacaggtttttcattgtgattgtcaaaatcattttcatggtgtgagttgcttatattattattttcatagtcatcatcttcattactattgttgtaatcgttgtcttcttca

SEQ ID NO: 1846 - DNA, 120 bp, synthetic construct
  source 1..120: mol_type = other DNA
atattattattttcatagtcatcatcttcattactattgttgtaatcgttgtcttcttcatcttcttcttcatcttcatcttcttcatcggtatagtcatagtcttcttcaggctgttcg

SEQ ID NO: 1847 - DNA, 120 bp, synthetic construct
  source 1..120: mol_type = other DNA
tcttcttcttcatcttcatcttcttcatcggtatagtcatagtcttcttcaggctgttcgctgtactcttcatcttcatctatgtactcatctaaatcatcgaagttaaaatcatcatct

SEQ ID NO: 1848 - DNA, 120 bp, synthetic construct
  source 1..120: mol_type = other DNA
ctgtactcttcatcttcatctatgtactcatctaaatcatcgaagttaaaatcatcatcttcgtcttcatcatcttcataatttgtttctgtactgttatatatagcaccttcttctgtt

SEQ ID NO: 1849 - DNA, 120 bp, synthetic construct
  source 1..120: mol_type = other DNA
tcgtcttcatcatcttcataatttgtttctgtactgttatatatagcaccttcttctgttagattattttcagtgttgttaggtttgttttcaggaatatcactttcaatactagggata

SEQ ID NO: 1850 - DNA, 120 bp, synthetic construct
  source 1..120: mol_type = other DNA
agattattttcagtgttgttaggtttgttttcaggaatatcactttcaatactagggatagggtcttcattttctttttttgttatttttacattattaggatcgtaaggttcttgagta

SEQ ID NO: 1851 - DNA, 120 bp, synthetic construct
  source 1..120: mol_type = other DNA
gggtcttcattttctttttttgttatttttacattattaggatcgtaaggttcttgagtaggtacgaaagtgcttttcaataatttttttgtaaagtttttgtcttcataatattttatt

SEQ ID NO: 1852 - DNA, 120 bp, synthetic construct
  source 1..120: mol_type = other DNA
ggtacgaaagtgcttttcaataatttttttgtaaagtttttgtcttcataatattttattttttttgattttataggataagtagactctattaaaagtatttgttcatctctaggtaac

SEQ ID NO: 1853 - DNA, 120 bp, synthetic construct
  source 1..120: mol_type = other DNA
ttttttgattttataggataagtagactctattaaaagtatttgttcatctctaggtaacattataacttcttgaggtaataataacgctctttgtgtttctgatatgtgtaatgaacga

SEQ ID NO: 1854 - DNA, 120 bp, synthetic construct
  source 1..120: mol_type = other DNA
attataacttcttgaggtaataataacgctctttgtgtttctgatatgtgtaatgaacgagaggcagggtttaaatctaaaaatttaggtctatttaaagattcctgattaactgtttta

SEQ ID NO: 1855 - DNA, 120 bp, synthetic construct
  source 1..120: mol_type = other DNA
gaggcagggtttaaatctaaaaatttaggtctatttaaagattcctgattaactgttttattgcctattagctgtgatattaggtttgcagtttcaatattgtttgctgcaaaagtaatt

SEQ ID NO: 1856 - DNA, 120 bp, synthetic construct
  source 1..120: mol_type = other DNA
ttgcctattagctgtgatattaggtttgcagtttcaatattgtttgctgcaaaagtaattctataagtagaatttgacagaaatgagttcattcctgcttcctcatatatacctttaagc

SEQ ID NO: 1857 - DNA, 120 bp, synthetic construct
  source 1..120: mol_type = other DNA
ctataagtagaatttgacagaaatgagttcattcctgcttcctcatatatacctttaagctgttcagtgtcttggataatcaaaaataatctaactctatatccacggaaatatgcaata

SEQ ID NO: 1858 - DNA, 120 bp, synthetic construct
  source 1..120: mol_type = other DNA
tgttcagtgtcttggataatcaaaaataatctaactctatatccacggaaatatgcaataccagtttgaaattgctccatctttcctaatgttggaaactcatccattaaaaacaataca

SEQ ID NO: 1859 - DNA, 120 bp, synthetic construct
  source 1..120: mol_type = other DNA
ccagtttgaaattgctccatctttcctaatgttggaaactcatccattaaaaacaatacaccgtaaggttcatcatccgatggtaaagttcgacataaaaactctgttgcttgctgatag

SEQ ID NO: 1860 - DNA, 120 bp, synthetic construct
  source 1..120: mol_type = other DNA
ccgtaaggttcatcatccgatggtaaagttcgacataaaaactctgttgcttgctgatagaatacctgcattaaaggcctaagacgagttaagttgtctggtgttaatccaacatatact

SEQ ID NO: 1861 - DNA, 120 bp, synthetic construct
  source 1..120: mol_type = other DNA
aatacctgcattaaaggcctaagacgagttaagttgtctggtgttaatccaacatatactgttactttttttcttttaaattcttgaatattaaaatcacttgaagctgttgctgtatct

SEQ ID NO: 1862 - DNA, 120 bp, synthetic construct
  source 1..120: mol_type = other DNA
gttactttttttcttttaaattcttgaatattaaaatcacttgaagctgttgctgtatctattaacgggtttgcccataattctaaagatgagttcatagttgatactacacctgaacgc

SEQ ID NO: 1863 - DNA, 120 bp, synthetic construct
  source 1..120: mol_type = other DNA
attaacgggtttgcccataattctaaagatgagttcatagttgatactacacctgaacgctctttatcagctttttgtaagaatgcagctatattcatatatgcaactgggtgaattttt

SEQ ID NO: 1864 - DNA, 120 bp, synthetic construct
  source 1..120: mol_type = other DNA
tctttatcagctttttgtaagaatgcagctatattcatatatgcaactgggtgaatttttttccctatagtgtctaatacaactgccaagttgtagactacgtcatcactacgcattgtt

SEQ ID NO: 1865 - DNA, 120 bp, synthetic construct
  source 1..120: mol_type = other DNA
ttccctatagtgtctaatacaactgccaagttgtagactacgtcatcactacgcattgttcgtacaacttctccaaaggattttactttttctggtactgctagtagatataatactact

SEQ ID NO: 1866 - DNA, 120 bp, synthetic construct
  source 1..120: mol_type = other DNA
cgtacaacttctccaaaggattttactttttctggtactgctagtagatataatactactcctacaaataaactacgtgcttcgttgtaccaaaagtcttgttcaggcattattagattg

SEQ ID NO: 1867 - DNA, 120 bp, synthetic construct
  source 1..120: mol_type = other DNA
cctacaaataaactacgtgcttcgttgtaccaaaagtcttgttcaggcattattagattggcgattttttgtacatcatccaccatttgtcctggtttagagcttatccaatccaatgga

SEQ ID NO: 1868 - DNA, 120 bp, synthetic construct
  source 1..120: mol_type = other DNA
gcgattttttgtacatcatccaccatttgtcctggtttagagcttatccaatccaatggattgtaacagtgacttaccccatcaggttgagctggattccacacaaatacttcttgtcct

SEQ ID NO: 1869 - DNA, 120 bp, synthetic construct
  source 1..120: mol_type = other DNA
ttgtaacagtgacttaccccatcaggttgagctggattccacacaaatacttcttgtcctctttttttcctccatccacttgtgagatcatagttttctaattttatgtcatgtactatt

SEQ ID NO: 1870 - DNA, 120 bp, synthetic construct
  source 1..120: mol_type = other DNA
ctttttttcctccatccacttgtgagatcatagttttctaattttatgtcatgtactattacagagtcttcccaaaacaataagtttggtattacaaaacctacacctttcccagatccg

SEQ ID NO: 1871 - DNA, 120 bp, synthetic construct
  source 1..120: mol_type = other DNA
acagagtcttcccaaaacaataagtttggtattacaaaacctacacctttcccagatccggttggtgcaaatagtaaagcatgttgaaatccatcagcaataagataacctcttttgtct

SEQ ID NO: 1872 - DNA, 120 bp, synthetic construct
  source 1..120: mol_type = other DNA
gttggtgcaaatagtaaagcatgttgaaatccatcagcaataagataacctcttttgtcttttcctagtagtataccttttctactacgtaatcctatttttcgaatatctttttctgtt

SEQ ID NO: 1873 - DNA, 120 bp, synthetic construct
  source 1..120: mol_type = other DNA
tttcctagtagtataccttttctactacgtaatcctatttttcgaatatctttttctgttgcccatcttgaatctccatgtaatgattctttctttttaaatggtctccaatcgaatagt

SEQ ID NO: 1874 - DNA, 120 bp, synthetic construct
  source 1..120: mol_type = other DNA
gcccatcttgaatctccatgtaatgattctttctttttaaatggtctccaatcgaatagtatgtttcttaaattccacaatactatacttaggatacctattggtatacatagtgatgat

SEQ ID NO: 1875 - DNA, 120 bp, synthetic construct
  source 1..120: mol_type = other DNA
atgtttcttaaattccacaatactatacttaggatacctattggtatacatagtgatgatattaactttactaatagtattgcatcgtatgaagaaggattatgccaccagtgttctacg

SEQ ID NO: 1876 - DNA, 120 bp, synthetic construct
  source 1..120: mol_type = other DNA
attaactttactaatagtattgcatcgtatgaagaaggattatgccaccagtgttctacgtaattaaaaacagtaggccaaattctgtctggaaagtcgctgaaactaggatttatagcg

SEQ ID NO: 1877 - DNA, 120 bp, synthetic construct
  source 1..120: mol_type = other DNA
taattaaaaacagtaggccaaattctgtctggaaagtcgctgaaactaggatttatagcgttgaaatctagatagtctggtccccataccattaagataaataaaacccctgatagataa

SEQ ID NO: 1878 - DNA, 120 bp, synthetic construct
  source 1..120: mol_type = other DNA
ttgaaatctagatagtctggtccccataccattaagataaataaaacccctgatagataaaagcaaaattccaacccgaagaatgctcctaagaccaggaataaaatattacgtatgtgg

SEQ ID NO: 1879 - DNA, 120 bp, synthetic construct
  source 1..120: mol_type = other DNA
aagcaaaattccaacccgaagaatgctcctaagaccaggaataaaatattacgtatgtggtttgcacttacactatccataaaaataacaacttaattataaaacttacgtatcatttaa

SEQ ID NO: 1880 - DNA, 120 bp, synthetic construct
  source 1..120: mol_type = other DNA
tttgcacttacactatccataaaaataacaacttaattataaaacttacgtatcatttaaccatttttctgtaaagatttagtgaataatatttctgatacataccttttaccctctgat

SEQ ID NO: 1881 - DNA, 120 bp, synthetic construct
  source 1..120: mol_type = other DNA
ccatttttctgtaaagatttagtgaataatatttctgatacataccttttaccctctgatcctctttttaactgtattacaatatctactatattagtgatgtaattaattatttgatct

SEQ ID NO: 1882 - DNA, 120 bp, synthetic construct
  source 1..120: mol_type = other DNA
cctctttttaactgtattacaatatctactatattagtgatgtaattaattatttgatctggaggtatgccaagtcctgcttgcataaccattaattttaattgttctagtgccatcatt

SEQ ID NO: 1883 - DNA, 120 bp, synthetic construct
  source 1..120: mol_type = other DNA
actgtattacaatatctactatattagtgatgtaattaattatttgatctggaggtatgccaagtcctgcttgcataaccattaattttaattgttctagtgccatcattggtgtgtcag

SEQ ID NO: 1884 - DNA, 120 bp, synthetic construct
  source 1..120: mol_type = other DNA
tgtttgcgctagttttagcggtggtaattcttcctctttggaccacggctaataaatcttacgtaacaccaacccctgcgactcgctctatcggacatatgtctgctcttctacgagaat

SEQ ID NO: 1885 - DNA, 120 bp, synthetic construct
  source 1..120: mol_type = other DNA
acgtaacaccaacccctgcgactcgctctatcggacatatgtctgctcttctacgagaatattccgaccgtaatatgtctctgaaattagaagccttttatcctactggtttcgatgaag

SEQ ID NO: 1886 - DNA, 120 bp, synthetic construct
  source 1..120: mol_type = other DNA
attccgaccgtaatatgtctctgaaattagaagccttttatcctactggtttcgatgaagaactcattaaatcacttcactggggaaatgatagaaaacacgttttcttggttattgtta

SEQ ID NO: 1887 - DNA, 120 bp, synthetic construct
  source 1..120: mol_type = other DNA
aactcattaaatcacttcactggggaaatgatagaaaacacgttttcttggttattgttaaggttaaccctacaacacacgaaggagacgtcgggctggttatatttccaaaatacttgt

SEQ ID NO: 1888 - DNA, 120 bp, synthetic construct
  source 1..120: mol_type = other DNA
aggttaaccctacaacacacgaaggagacgtcgggctggttatatttccaaaatacttgttatcgccataccatttcaaagcagaacatcgagcaccgtttcctgctggacgttttggat

SEQ ID NO: 1889 - DNA, 120 bp, synthetic construct
  source 1..120: mol_type = other DNA
tatcgccataccatttcaaagcagaacatcgagcaccgtttcctgctggacgttttggatttcttagtcaccctgtgacacccgacgtgagcttctttgacagttcgtttgcgccgtatt

SEQ ID NO: 1890 - DNA, 120 bp, synthetic construct
  source 1..120: mol_type = other DNA
ttcttagtcaccctgtgacacccgacgtgagcttctttgacagttcgtttgcgccgtatttaactacgcaacatcttgttgcgtttactacgttcccaccaaacccccttgtatggcatt

SEQ ID NO: 1891 - DNA, 120 bp, synthetic construct
  source 1..120: mol_type = other DNA
taactacgcaacatcttgttgcgtttactacgttcccaccaaacccccttgtatggcatttggaaagagctgagaccgcagcaactgcagaaaggccgtttggggtaagtcttttacccg

SEQ ID NO: 1892 - DNA, 120 bp, synthetic construct
  source 1..120: mol_type = other DNA
tggaaagagctgagaccgcagcaactgcagaaaggccgtttggggtaagtcttttacccgctcgcccaacagtccccaagaatactattctggaacataaagcgcattttgctacatggg

SEQ ID NO: 1893 - DNA, 120 bp, synthetic construct
  source 1..120: mol_type = other DNA
ctcgcccaacagtccccaagaatactattctggaacataaagcgcattttgctacatgggatgcccttgcccgacatacttttttttctgccgaagcaattatcaccaactcaacgttga

SEQ ID NO: 1894 - DNA, 120 bp, synthetic construct
  source 1..120: mol_type = other DNA
atgcccttgcccgacatacttttttttctgccgaagcaattatcaccaactcaacgttgagaatacacgttcccctttttgggtcggtatggccaattcgatactgggccaccggttcgg

SEQ ID NO: 1895 - DNA, 120 bp, synthetic construct
  source 1..120: mol_type = other DNA
gaatacacgttcccctttttgggtcggtatggccaattcgatactgggccaccggttcggtgcttctcacaagcgactcgggtcgtgtggaagtaaatattggtgtaggatttatgagct

SEQ ID NO: 1896 - DNA, 120 bp, synthetic construct
  source 1..120: mol_type = other DNA
tgcttctcacaagcgactcgggtcgtgtggaagtaaatattggtgtaggatttatgagctcgctcatttctttatcctctggaccaccgatagaattaattgttgtaccacatacagtaa

SEQ ID NO: 1897 - DNA, 120 bp, synthetic construct
  source 1..120: mol_type = other DNA
cgctcatttctttatcctctggaccaccgatagaattaattgttgtaccacatacagtaaaactgaacgcggttacaagcgacaccacatggttccagctaaatccaccgggtccggatc

SEQ ID NO: 1898 - DNA, 120 bp, synthetic construct
  source 1..120: mol_type = other DNA
aactgaacgcggttacaagcgacaccacatggttccagctaaatccaccgggtccggatccggggccatcttatcgagtttatttacttggacgtgggttggatatgaatttttcaaagc

SEQ ID NO: 1899 - DNA, 120 bp, synthetic construct
  source 1..120: mol_type = other DNA
cggggccatcttatcgagtttatttacttggacgtgggttggatatgaatttttcaaagcatgctacggtcgatatatgcgcatatcccgaagagagtttggattaccgctatcatttat

SEQ ID NO: 1900 - DNA, 120 bp, synthetic construct
  source 1..120: mol_type = other DNA
atgctacggtcgatatatgcgcatatcccgaagagagtttggattaccgctatcatttatccatggcccacacggaggctctgcggatgacaacgaaggcggatcaacatgacataaacg

SEQ ID NO: 1901 - DNA, 120 bp, synthetic construct
  source 1..120: mol_type = other DNA
ccatggcccacacggaggctctgcggatgacaacgaaggcggatcaacatgacataaacgaggaaagctattaccatatcgccgcaagaatagccacatcaatttttgcgttgtcggaaa

SEQ ID NO: 1902 - DNA, 120 bp, synthetic construct
  source 1..120: mol_type = other DNA
aggaaagctattaccatatcgccgcaagaatagccacatcaatttttgcgttgtcggaaatgggccgtaccacagaatattttctgttagatgagatcgtagatgttcagtatcaattaa

SEQ ID NO: 1903 - DNA, 120 bp, synthetic construct
  source 1..120: mol_type = other DNA
tgggccgtaccacagaatattttctgttagatgagatcgtagatgttcagtatcaattaaaattccttaattacattttaatgcggataggagcaggagctcatcccaacactatatccg

SEQ ID NO: 1904 - DNA, 120 bp, synthetic construct
  source 1..120: mol_type = other DNA
aattccttaattacattttaatgcggataggagcaggagctcatcccaacactatatccggaacctcggatctgatctttgccgatccatcgcagcttcatgacgaactttcacttcttt

SEQ ID NO: 1905 - DNA, 120 bp, synthetic construct
  source 1..120: mol_type = other DNA
gaacctcggatctgatctttgccgatccatcgcagcttcatgacgaactttcacttctttttggtcaggtaaaacccgcaaatgtcgattattttatttcatatgatgaagcccgtgatc

SEQ ID NO: 1906 - DNA, 120 bp, synthetic construct
  source 1..120: mol_type = other DNA
ttggtcaggtaaaacccgcaaatgtcgattattttatttcatatgatgaagcccgtgatcaactaaagaccgcatacgcgctttcccgtggtcaagaccatgtgaatgcactttctctcg

SEQ ID NO: 1907 - DNA, 120 bp, synthetic construct
  source 1..120: mol_type = other DNA
aactaaagaccgcatacgcgctttcccgtggtcaagaccatgtgaatgcactttctctcgccaggcgtgttataatgagcatatacaaggggctgcttgtgaagcaaaatttaaatgcta

SEQ ID NO: 1908 - DNA, 120 bp, synthetic construct
  source 1..120: mol_type = other DNA
ccaggcgtgttataatgagcatatacaaggggctgcttgtgaagcaaaatttaaatgctacagagaggcaggctttattttttgcctcaatgattttattaaatttccgcgaaggactag

SEQ ID NO: 1909 - DNA, 120 bp, synthetic construct
  source 1..120: mol_type = other DNA
cagagaggcaggctttattttttgcctcaatgattttattaaatttccgcgaaggactagaaaattcatctcgggtattagacggtcgcacaactttgcttttaatgacatccatgtgta

SEQ ID NO: 1910 - DNA, 120 bp, synthetic construct
  source 1..120: mol_type = other DNA
aaaattcatctcgggtattagacggtcgcacaactttgcttttaatgacatccatgtgtacggcagctcacgccacgcaagcagcacttaacatacaagaaggcctggcatacttaaatc

SEQ ID NO: 1911 - DNA, 120 bp, synthetic construct
  source 1..120: mol_type = other DNA
cggcagctcacgccacgcaagcagcacttaacatacaagaaggcctggcatacttaaatccttcaaaacacatgtttacaataccaaacgtatacagtccttgtatgggttcccttcgta

SEQ ID NO: 1912 - DNA, 120 bp, synthetic construct
  source 1..120: mol_type = other DNA
cttcaaaacacatgtttacaataccaaacgtatacagtccttgtatgggttcccttcgtacagacctcacggaagagattcatgttatgaatctcctgtcggcaataccaacacgcccag

SEQ ID NO: 1913 - DNA, 120 bp, synthetic construct
  source 1..120: mol_type = other DNA
cagacctcacggaagagattcatgttatgaatctcctgtcggcaataccaacacgcccaggacttaacgaggtattgcatacccaactagacgaatctgaaatattcgacgcggcattta

SEQ ID NO: 1914 - DNA, 120 bp, synthetic construct
  source 1..120: mol_type = other DNA
gacttaacgaggtattgcatacccaactagacgaatctgaaatattcgacgcggcatttaaaaccatgatgatttttaccacatggactgccaaagatttgcatatactccacacccatg

SEQ ID NO: 1915 - DNA, 120 bp, synthetic construct
  source 1..120: mol_type = other DNA
aaaccatgatgatttttaccacatggactgccaaagatttgcatatactccacacccatgtaccagaagtatttacgtgtcaagatgcagccgcgcgtaacggagaatatgtgctcattc

SEQ ID NO: 1916 - DNA, 120 bp, synthetic construct
  source 1..120: mol_type = other DNA
taccagaagtatttacgtgtcaagatgcagccgcgcgtaacggagaatatgtgctcattcttccagctgtccagggacacagttatgtgattacacgaaacaaacctcaaaggggtttgg

SEQ ID NO: 1917 - DNA, 120 bp, synthetic construct
  source 1..120: mol_type = other DNA
ttccagctgtccagggacacagttatgtgattacacgaaacaaacctcaaaggggtttggtatattccctggcagatgtggatgtatataaccccatatccgttgtttatttaagcaggg

SEQ ID NO: 1918 - DNA, 120 bp, synthetic construct
  source 1..120: mol_type = other DNA
tatattccctggcagatgtggatgtatataaccccatatccgttgtttatttaagcagggatacttgcgtgtctgaacatggtgtcatagagacggtcgcactgccccatccggacaatt

SEQ ID NO: 1919 - DNA, 120 bp, synthetic construct
  source 1..120: mol_type = other DNA
atacttgcgtgtctgaacatggtgtcatagagacggtcgcactgccccatccggacaatttaaaagaatgtttgtattgcggaagtgtttttcttaggtatctaaccacgggggcgatta

SEQ ID NO: 1920 - DNA, 120 bp, synthetic construct
  source 1..120: mol_type = other DNA
taaaagaatgtttgtattgcggaagtgtttttcttaggtatctaaccacgggggcgattatggatataattattattgacagcaaagatacagaacgacaactagccgctatgggaaact

SEQ ID NO: 1921 - DNA, 120 bp, synthetic construct
  source 1..120: mol_type = other DNA
tggatataattattattgacagcaaagatacagaacgacaactagccgctatgggaaactccacaattccacccttcaatccagacatgcacggggatgactctaaggctgtgttgttgt

SEQ ID NO: 1922 - DNA, 120 bp, synthetic construct
  source 1..120: mol_type = other DNA
ccacaattccacccttcaatccagacatgcacggggatgactctaaggctgtgttgttgtttccaaacggaactgtggtaacgcttctaggattcgaacgacgacaagccatacgaatgt

SEQ ID NO: 1923 - DNA, 120 bp, synthetic construct
  source 1..120: mol_type = other DNA
ttccaaacggaactgtggtaacgcttctaggattcgaacgacgacaagccatacgaatgtcgggacaataccttggggcctctttaggaggggcgtttctggcggtagtggggtttggta

SEQ ID NO: 1924 - DNA, 120 bp, synthetic construct
  source 1..120: mol_type = other DNA
cgggacaataccttggggcctctttaggaggggcgtttctggcggtagtggggtttggtattatcggatggatgttatgtggaaattcccgccttcgagaatataataaaatacctctga

SEQ ID NO: 1925 - DNA, 120 bp, synthetic construct
  source 1..120: mol_type = other DNA
ttatcggatggatgttatgtggaaattcccgccttcgagaatataataaaatacctctgacataaaaaacatgtataataaaaagtcactataaacgtattctctacaatactttattcg

SEQ ID NO: 1926 - DNA, 120 bp, synthetic construct
  source 1..120: mol_type = other DNA
cataaaaaacatgtataataaaaagtcactataaacgtattctctacaatactttattcgcgaataatacacactacctttgggtttttttcccgtccccaaatggtgtttggtgcactc

SEQ ID NO: 1927 - DNA, 120 bp, synthetic construct
  source 1..120: mol_type = other DNA
cgaataatacacactacctttgggtttttttcccgtccccaaatggtgtttggtgcactctaccaaaaaatagagcgcctaaatatgctatataacgcctcccagcaaaatacggttcaa

SEQ ID NO: 1928 - DNA, 120 bp, synthetic construct
  source 1..120: mol_type = other DNA
taccaaaaaatagagcgcctaaatatgctatataacgcctcccagcaaaatacggttcaaaggcattacccgatattgtattgtagtacagggcaatgggaattgatgatcccaataaac

SEQ ID NO: 1929 - DNA, 120 bp, synthetic construct
  source 1..120: mol_type = other DNA
aggcattacccgatattgtattgtagtacagggcaatgggaattgatgatcccaataaacggcatagacgcacagcgccgttatagcaggggtctccagagtacagggtatctaagtacc

SEQ ID NO: 1930 - DNA, 120 bp, synthetic construct
  source 1..120: mol_type = other DNA
ggcatagacgcacagcgccgttatagcaggggtctccagagtacagggtatctaagtaccgggatatctcatactcatgcctttccgtgacagaaacatcaaccggaacagtatccgata

SEQ ID NO: 1931 - DNA, 120 bp, synthetic construct
  source 1..120: mol_type = other DNA
gggatatctcatactcatgcctttccgtgacagaaacatcaaccggaacagtatccgataaaccaactcctgtttttgcaaggcgtaaaattcgcacaccttccttttttgcaagatgtg

SEQ ID NO: 1932 - DNA, 120 bp, synthetic construct
  source 1..120: mol_type = other DNA
aaccaactcctgtttttgcaaggcgtaaaattcgcacaccttccttttttgcaagatgtgacgtttccttgtaacagggaagctgggggagtggtaagaacaacaaagtttcagccaacg

SEQ ID NO: 1933 - DNA, 120 bp, synthetic construct
  source 1..120: mol_type = other DNA
acgtttccttgtaacagggaagctgggggagtggtaagaacaacaaagtttcagccaacgtgccaataaagcccacttccctcaagaggctgtttgctgtatccacaatggtccgtatta

SEQ ID NO: 1934 - DNA, 120 bp, synthetic construct
  source 1..120: mol_type = other DNA
tgccaataaagcccacttccctcaagaggctgtttgctgtatccacaatggtccgtattaaatcttgagcaacttgatccgtgtcatcatcactgggtaacgcgttaacataactacgcg

SEQ ID NO: 1935 - DNA, 120 bp, synthetic construct
  source 1..120: mol_type = other DNA
aatcttgagcaacttgatccgtgtcatcatcactgggtaacgcgttaacataactacgcgttaaatcttcaataacggcataacaattaaacgcttcccaccgagacagtatatattgaa

SEQ ID NO: 1936 - DNA, 120 bp, synthetic construct
  source 1..120: mol_type = other DNA
ttaaatcttcaataacggcataacaattaaacgcttcccaccgagacagtatatattgaacaatcacgaaccgttgacaggacgtcagatcacgtccgtaagcatgcccgaaaaatggaa

SEQ ID NO: 1937 - DNA, 120 bp, synthetic construct
  source 1..120: mol_type = other DNA
caatcacgaaccgttgacaggacgtcagatcacgtccgtaagcatgcccgaaaaatggaagttccccccgttcgccatataccgcaacaactgcagtatatatcgtctcacgggcttcat

SEQ ID NO: 1938 - DNA, 120 bp, synthetic construct
  source 1..120: mol_type = other DNA
gttccccccgttcgccatataccgcaacaactgcagtatatatcgtctcacgggcttcattaagttcatcttcaagtccaggccattttctggctttaaatataacctcgtccgcaaaaa

SEQ ID NO: 1939 - DNA, 120 bp, synthetic construct
  source 1..120: mol_type = other DNA
taagttcatcttcaagtccaggccattttctggctttaaatataacctcgtccgcaaaaaaaaccgcacatgataacgcgcggatacaatgagtagtggctttatggcgaggatcccaaa

SEQ ID NO: 1940 - DNA, 120 bp, synthetic construct
  source 1..120: mol_type = other DNA
aaaccgcacatgataacgcgcggatacaatgagtagtggctttatggcgaggatcccaaatgtccattacccgggggatggtcctaatctgtacaaagttacttagtgtaatatgatcgg

SEQ ID NO: 1941 - DNA, 120 bp, synthetic construct
  source 1..120: mol_type = other DNA
tgtccattacccgggggatggtcctaatctgtacaaagttacttagtgtaatatgatcggacttcttacgccgtctaggctgtttctcagaatacggttcacccgaaatcggcacatcat

SEQ ID NO: 1942 - DNA, 120 bp, synthetic construct
  source 1..120: mol_type = other DNA
acttcttacgccgtctaggctgtttctcagaatacggttcacccgaaatcggcacatcatctgcttttacgtcttccgtaaccacatcagcagcgcgccgactaacaattatacttgttt

SEQ ID NO: 1943 - DNA, 120 bp, synthetic construct
  source 1..120: mol_type = other DNA
ctgcttttacgtcttccgtaaccacatcagcagcgcgccgactaacaattatacttgttttttcatcgtcgttacttccgttaagcgcgtctcgtatctcgggcgtcccgtcgaataatc

SEQ ID NO: 1944 - DNA, 120 bp, synthetic construct
  source 1..120: mol_type = other DNA
tttcatcgtcgttacttccgttaagcgcgtctcgtatctcgggcgtcccgtcgaataatccactcactagctcctgcaaactttctggtaactccaacatacgcatatacaccaatgaaa

SEQ ID NO: 1945 - DNA, 120 bp, synthetic construct
  source 1..120: mol_type = other DNA
cactcactagctcctgcaaactttctggtaactccaacatacgcatatacaccaatgaaaaactggcttcgtttggtacgtacataaagccatttgtggtattaatggcggtgggtgttg

SEQ ID NO: 1946 - DNA, 120 bp, synthetic construct
  source 1..120: mol_type = other DNA
aactggcttcgtttggtacgtacataaagccatttgtggtattaatggcggtgggtgttggaaacaattttagcttattctcgcgcgtaacatctacccccgccaccaatgttaaatgcg

SEQ ID NO: 1947 - DNA, 120 bp, synthetic construct
  source 1..120: mol_type = other DNA
gaaacaattttagcttattctcgcgcgtaacatctacccccgccaccaatgttaaatgcgtcacggggagggacacgagataatctgcgagcgtagggtcctccacttcaacatcaaatg

SEQ ID NO: 1948 - DNA, 120 bp, synthetic construct
  source 1..120: mol_type = other DNA
tcacggggagggacacgagataatctgcgagcgtagggtcctccacttcaacatcaaatgttccgcaaaggtcgcgatccaccgcccccgatcccgctgcaagtaaggccactcgatcca

SEQ ID NO: 1949 - DNA, 120 bp, synthetic construct
  source 1..120: mol_type = other DNA
ttccgcaaaggtcgcgatccaccgcccccgatcccgctgcaagtaaggccactcgatccaaaaacacgcagttattattggatgataccgcccatgtcttcccggtgcgattgagctcac

SEQ ID NO: 1950 - DNA, 120 bp, synthetic construct
  source 1..120: mol_type = other DNA
aaaacacgcagttattattggatgataccgcccatgtcttcccggtgcgattgagctcacttcgaacgtaactggcaacagatctgtcaccgggtccgaccccgcgaacaacatgtccaa

SEQ ID NO: 1951 - DNA, 120 bp, synthetic construct
  source 1..120: mol_type = other DNA
ttcgaacgtaactggcaacagatctgtcaccgggtccgaccccgcgaacaacatgtccaaattttgcgatctcgcctccatgtttgcggggtatggaaattaagcatcccccgcatataa

SEQ ID NO: 1952 - DNA, 120 bp, synthetic construct
  source 1..120: mol_type = other DNA
attttgcgatctcgcctccatgtttgcggggtatggaaattaagcatcccccgcatataaaatacgccctggtagcacgctcgttaaaataaaacgttacgccgttataagatacggttg

SEQ ID NO: 1953 - DNA, 120 bp, synthetic construct
  source 1..120: mol_type = other DNA
aatacgccctggtagcacgctcgttaaaataaaacgttacgccgttataagatacggttgaatgatatggaaattccatattaaagcgtttatcggaacattaacctcgaacttgccgtc

SEQ ID NO: 1954 - DNA, 120 bp, synthetic construct
  source 1..120: mol_type = other DNA
aatgatatggaaattccatattaaagcgtttatcggaacattaacctcgaacttgccgtcccgtgatcgtgtgatcgccaaccttaggtccacaccgaatatgagaaatatataactaca

SEQ ID NO: 1955 - DNA, 120 bp, synthetic construct
  source 1..120: mol_type = other DNA
ccgtgatcgtgtgatcgccaaccttaggtccacaccgaatatgagaaatatataactacacgcaaacattcaaaacaccgtggtatcattaacgtcatatgaaaagatccaatcaatcca

SEQ ID NO: 1956 - DNA, 120 bp, synthetic construct
  source 1..120: mol_type = other DNA
cgcaaacattcaaaacaccgtggtatcattaacgtcatatgaaaagatccaatcaatccaatcaaccacacctcctaccgtttagcacgtcagctatgtgacatgctccaaacatacgta

SEQ ID NO: 1957 - DNA, 120 bp, synthetic construct
  source 1..120: mol_type = other DNA
atcaaccacacctcctaccgtttagcacgtcagctatgtgacatgctccaaacatacgtaaacatttagagagggtgttataacagtctgtcaggcggggtatattctacataatacaag

SEQ ID NO: 1958 - DNA, 120 bp, synthetic construct
  source 1..120: mol_type = other DNA
aacatttagagagggtgttataacagtctgtcaggcggggtatattctacataatacaaggatcggctttaactttgtcaacatttttactttggactataaactgcgactgaacgttat

SEQ ID NO: 1959 - DNA, 120 bp, synthetic construct
  source 1..120: mol_type = other DNA
gatcggctttaactttgtcaacatttttactttggactataaactgcgactgaacgttatgaacccaccccaagcccgcgtctcggaacagacaaaggacttgcttagcgttatggttaa

SEQ ID NO: 1960 - DNA, 120 bp, synthetic construct
  source 1..120: mol_type = other DNA
gaacccaccccaagcccgcgtctcggaacagacaaaggacttgcttagcgttatggttaaccagcaccccgaagaggacgcaaaagtgtgtaaatccagtgataattcaccgctttataa

SEQ ID NO: 1961 - DNA, 120 bp, synthetic construct
  source 1..120: mol_type = other DNA
ccagcaccccgaagaggacgcaaaagtgtgtaaatccagtgataattcaccgctttataacaccatggttatgttatcgtatgggggtgatacggacttactattaagctctgcatgtac

SEQ ID NO: 1962 - DNA, 120 bp, synthetic construct
  source 1..120: mol_type = other DNA
caccatggttatgttatcgtatgggggtgatacggacttactattaagctctgcatgtacccgcacatctaccgtaaacaggtcggcgtttacgcaacactccgtgttttatattatatc

SEQ ID NO: 1963 - DNA, 120 bp, synthetic construct
  source 1..120: mol_type = other DNA
ccgcacatctaccgtaaacaggtcggcgtttacgcaacactccgtgttttatattatatccacggtgttgattcaaccaatatgttgtatcttcttttttttttactataaagcgacacg

SEQ ID NO: 1964 - DNA, 120 bp, synthetic construct
  source 1..120: mol_type = other DNA
cacggtgttgattcaaccaatatgttgtatcttcttttttttttactataaagcgacacgctgtatgctcttattcacagccgggttacttctgacgattctacatcactttcgacttat

SEQ ID NO: 1965 - DNA, 120 bp, synthetic construct
  source 1..120: mol_type = other DNA
ctgtatgctcttattcacagccgggttacttctgacgattctacatcactttcgacttattattatgttattgtgtgtctacagaaatatacgatcagacctgctacccttatctacatc

SEQ ID NO: 1966 - DNA, 120 bp, synthetic construct
  source 1..120: mol_type = other DNA
tattatgttattgtgtgtctacagaaatatacgatcagacctgctacccttatctacatcccagcaactgctgcttggaattattgttgtgactcgaacaatgctattttgtattacggc

SEQ ID NO: 1967 - DNA, 120 bp, synthetic construct
  source 1..120: mol_type = other DNA
ccagcaactgctgcttggaattattgttgtgactcgaacaatgctattttgtattacggcgtattatactctttttatagacacccgggtgttctttttgattaccggacacttgcaaag

SEQ ID NO: 1968 - DNA, 120 bp, synthetic construct
  source 1..120: mol_type = other DNA
gtattatactctttttatagacacccgggtgttctttttgattaccggacacttgcaaagtgaggttatttttccagatagcgtttcaaaaatacttcctgtgtcgtggggtccaagtcc

SEQ ID NO: 1969 - DNA, 120 bp, synthetic construct
  source 1..120: mol_type = other DNA
tgaggttatttttccagatagcgtttcaaaaatacttcctgtgtcgtggggtccaagtccagccgtgttactggtaatggcggcagttatttacgctatggactgtttggtggacacggt

SEQ ID NO: 1970 - DNA, 120 bp, synthetic construct
  source 1..120: mol_type = other DNA
agccgtgttactggtaatggcggcagttatttacgctatggactgtttggtggacacggtatcctttattgggccaagggtgtgggtccgtgttatgttaaaaacatctatttcgtttta

SEQ ID NO: 1971 - DNA, 120 bp, synthetic construct
  source 1..120: mol_type = other DNA
aatggcggcagttatttacgctatggactgtttggtggacacggtatcctttattgggccaagggtgtgggtccgtgttatgttaaaaacatctatttcgttttagtccatttcaataaa

SEQ ID NO: 1972 - DNA, 120 bp, synthetic construct
  source 1..120: mol_type = other DNA
accaaacaaagttgggtaaggatagatcaatcaatgatcatattctagtgcacttaggattcaagatcctatcatcagggacaggagcagggttagggacatccgagatggccacacttt

SEQ ID NO: 1973 - DNA, 120 bp, synthetic construct
  source 1..120: mol_type = other DNA
tcaagatcctatcatcagggacaggagcagggttagggacatccgagatggccacacttttaaggagcttagcattgttcaaaagaaacaaggacaaaccacccattacatcaggatccg

SEQ ID NO: 1974 - DNA, 120 bp, synthetic construct
  source 1..120: mol_type = other DNA
taaggagcttagcattgttcaaaagaaacaaggacaaaccacccattacatcaggatccggtggagccatcagaggaatcaaacacattattatagtaccaatccctggagattcctcaa

SEQ ID NO: 1975 - DNA, 120 bp, synthetic construct
  source 1..120: mol_type = other DNA
gtggagccatcagaggaatcaaacacattattatagtaccaatccctggagattcctcaattaccactcgatccagactcctggaccggttggtcaggttaattggaaacccggatgtga

SEQ ID NO: 1976 - DNA, 120 bp, synthetic construct
  source 1..120: mol_type = other DNA
ttaccactcgatccagactcctggaccggttggtcaggttaattggaaacccggatgtgagcgggcccaaactaacaggagcactaataggtatattatccttatttgtggagtctccag

SEQ ID NO: 1977 - DNA, 120 bp, synthetic construct
  source 1..120: mol_type = other DNA
gcgggcccaaactaacaggagcactaataggtatattatccttatttgtggagtctccaggtcaattgattcagaggatcactgatgaccctgacgttagcataaggctgttggaggttg

SEQ ID NO: 1978 - DNA, 120 bp, synthetic construct
  source 1..120: mol_type = other DNA
gtcaattgattcagaggatcactgatgaccctgacgttagcataaggctgttggaggttgtccagagcgaccagtcacaatctggccttaccttcgcatcgagaggtactaatatggagg

SEQ ID NO: 1979 - DNA, 120 bp, synthetic construct
  source 1..120: mol_type = other DNA
tccagagcgaccagtcacaatctggccttaccttcgcatcgagaggtactaatatggaggatgaggcggaccagtacttttcacatgatgatccaagtagtagtgatcaatccaggttcg

SEQ ID NO: 1980 - DNA, 120 bp, synthetic construct
  source 1..120: mol_type = other DNA
atgaggcggaccagtacttttcacatgatgatccaagtagtagtgatcaatccaggttcgggtggtttgagaacaaggaaatctcagatattgaagtgcaagaccctgagggcttcaaca

SEQ ID NO: 1981 - DNA, 120 bp, synthetic construct
  source 1..120: mol_type = other DNA
ggtggtttgagaacaaggaaatctcagatattgaagtgcaagaccctgagggcttcaacatgattctgggtaccatcctagctcagatttgggtcttgctcgcaaaggcggttacggctc

SEQ ID NO: 1982 - DNA, 120 bp, synthetic construct
  source 1..120: mol_type = other DNA
tgattctgggtaccatcctagctcagatttgggtcttgctcgcaaaggcggttacggctccagacacagcagctgattcagagctaagaagatggatcaaatacacccaacaaagaagag

SEQ ID NO: 1983 - DNA, 120 bp, synthetic construct
  source 1..120: mol_type = other DNA
cagacacagcagctgattcagagctaagaagatggatcaaatacacccaacaaagaagagtagttggtgaatttagattggagagaaaatggttggatgtggtgagaaacaggattgccg

SEQ ID NO: 1984 - DNA, 120 bp, synthetic construct
  source 1..120: mol_type = other DNA
tagttggtgaatttagattggagagaaaatggttggatgtggtgagaaacaggattgccgaggacctctccttacgccgattcatggtcgctctaatcctggatatcaagagaacacccg

SEQ ID NO: 1985 - DNA, 120 bp, synthetic construct
  source 1..120: mol_type = other DNA
aggacctctccttacgccgattcatggtcgctctaatcctggatatcaagagaacacccggaaacaaacccaggattgctgaaatgatatgtgacattgatacatatatcgtagaggcag

SEQ ID NO: 1986 - DNA, 120 bp, synthetic construct
  source 1..120: mol_type = other DNA
gaaacaaacccaggattgctgaaatgatatgtgacattgatacatatatcgtagaggcaggattagccagttttatcctgactattaagtttgggatagaaaccatgtatcctgctcttg

SEQ ID NO: 1987 - DNA, 120 bp, synthetic construct
  source 1..120: mol_type = other DNA
gattagccagttttatcctgactattaagtttgggatagaaaccatgtatcctgctcttggactgcatgaatttgctggtgaattatccacacttgagtccttgatgaatctttaccagc

SEQ ID NO: 1988 - DNA, 120 bp, synthetic construct
  source 1..120: mol_type = other DNA
gactgcatgaatttgctggtgaattatccacacttgagtccttgatgaatctttaccagcaaatgggggaaactgcaccctatatggtaatcctggagaactcaattcagaacaagttta

SEQ ID NO: 1989 - DNA, 120 bp, synthetic construct
  source 1..120: mol_type = other DNA
aaatgggggaaactgcaccctatatggtaatcctggagaactcaattcagaacaagtttagtgcaggatcataccctctgctctggagctatgccatgggagtaggagtggaacttgaaa

SEQ ID NO: 1990 - DNA, 120 bp, synthetic construct
  source 1..120: mol_type = other DNA
gtgcaggatcataccctctgctctggagctatgccatgggagtaggagtggaacttgaaaactccatgggaggtttgaacttcggccgatcttactttgatccggcatattttagattag

SEQ ID NO: 1991 - DNA, 120 bp, synthetic construct
  source 1..120: mol_type = other DNA
actccatgggaggtttgaacttcggccgatcttactttgatccggcatattttagattagggcaagagatggtaaggaggtcagctggaaaggtcagttccacattggcatctgaactcg

SEQ ID NO: 1992 - DNA, 120 bp, synthetic construct
  source 1..120: mol_type = other DNA
ggcaagagatggtaaggaggtcagctggaaaggtcagttccacattggcatctgaactcggtataactgccgaggatgcaaggcttgtttcagagattgcaatgcatactactgaggaca

SEQ ID NO: 1993 - DNA, 120 bp, synthetic construct
  source 1..120: mol_type = other DNA
gtataactgccgaggatgcaaggcttgtttcagagattgcaatgcatactactgaggacaggatcagcagagcagttggacccagacaagcccaagtgtcatttctacacggtgatcaaa

SEQ ID NO: 1994 - DNA, 120 bp, synthetic construct
  source 1..120: mol_type = other DNA
ggatcagcagagcagttggacccagacaagcccaagtgtcatttctacacggtgatcaaagtgagaatgagctgccgagattggggggtaaggaggacaggagggtcaaacagaaccgag

SEQ ID NO: 1995 - DNA, 120 bp, synthetic construct
  source 1..120: mol_type = other DNA
gtgagaatgagctgccgagattggggggtaaggaggacaggagggtcaaacagaaccgaggagaagcccgggagagccacagagaaaccgagcccagcagagcaagtgatgcgagagctg

SEQ ID NO: 1996 - DNA, 120 bp, synthetic construct
  source 1..120: mol_type = other DNA
gagaagcccgggagagccacagagaaaccgagcccagcagagcaagtgatgcgagagctgcccatcctccaaccggcacacccctagacattgacactgcatcggagttcagccaagatc

SEQ ID NO: 1997 - DNA, 120 bp, synthetic construct
  source 1..120: mol_type = other DNA
cccatcctccaaccggcacacccctagacattgacactgcatcggagttcagccaagatccgcaggacagtcgaaggtcagccgatgccctgcttaggctgcaagccatggcaggaatct

SEQ ID NO: 1998 - DNA, 120 bp, synthetic construct
  source 1..120: mol_type = other DNA
cgcaggacagtcgaaggtcagccgatgccctgcttaggctgcaagccatggcaggaatctcggaagaacaagactcagacacggacacccctagagtgtacaatgatagagaccttctag

SEQ ID NO: 1999 - DNA, 120 bp, synthetic construct
  source 1..120: mol_type = other DNA
cggaagaacaagactcagacacggacacccctagagtgtacaatgatagagaccttctagactaggtgcgaggggtcgaggaccagaacaacatctgcctaccctccatcattgttataa

SEQ ID NO: 2000 - DNA, 120 bp, synthetic construct
  source 1..120: mol_type = other DNA
actaggtgcgaggggtcgaggaccagaacaacatctgcctaccctccatcattgttataaaaaacttaggaaccaggtccacacagccgccagcccatcaaccatccactcccacgatcg

SEQ ID NO: 2001 - DNA, 120 bp, synthetic construct
  source 1..120: mol_type = other DNA
aaaacttaggaaccaggtccacacagccgccagcccatcaaccatccactcccacgatcggagccgatggcagaggagcaggcacgccatgtcaaaaacggactggaatgcatccgggct

SEQ ID NO: 2002 - DNA, 120 bp, synthetic construct
  source 1..120: mol_type = other DNA
gagccgatggcagaggagcaggcacgccatgtcaaaaacggactggaatgcatccgggctctcaaagccgagcccatcggcacactggccatcgaggaagccatggcagcatggtcagaa

SEQ ID NO: 2003 - DNA, 120 bp, synthetic construct
  source 1..120: mol_type = other DNA
ctcaaagccgagcccatcggcacactggccatcgaggaagccatggcagcatggtcagaaatatcagacaacccaggacaggagcgagccacctgcaagaaagagaaggcaggcagttcg

SEQ ID NO: 2004 - DNA, 120 bp, synthetic construct
  source 1..120: mol_type = other DNA
atatcagacaacccaggacaggagcgagccacctgcaagaaagagaaggcaggcagttcgggtctcagcaaaccatgcctctcagcaattggatcaactgaaggcagtgcacctcgcatc

SEQ ID NO: 2005 - DNA, 120 bp, synthetic construct
  source 1..120: mol_type = other DNA
ggtctcagcaaaccatgcctctcagcaattggatcaactgaaggcagtgcacctcgcatccgcggtcagggatctggagagagcgatgacgacgctgaaactttgggagccccctcagga

SEQ ID NO: 2006 - DNA, 120 bp, synthetic construct
  source 1..120: mol_type = other DNA
cgcggtcagggatctggagagagcgatgacgacgctgaaactttgggagccccctcaggaaatctccaggcatcaagcgctgggttacagcgttattatgtttatgatcacagcggtgaa

SEQ ID NO: 2007 - DNA, 120 bp, synthetic construct
  source 1..120: mol_type = other DNA
aatctccaggcatcaagcgctgggttacagcgttattatgtttatgatcacagcggtgaagcgattaagggaatccaagatgctgactctatcatggttcaatcaggccttgaaggtgat

SEQ ID NO: 2008 - DNA, 120 bp, synthetic construct
  source 1..120: mol_type = other DNA
gcgattaagggaatccaagatgctgactctatcatggttcaatcaggccttgaaggtgatagcaccttctcaggaggagacaatgaatctgaaaacagcgatgtggatattggcgaacct

SEQ ID NO: 2009 - DNA, 120 bp, synthetic construct
  source 1..120: mol_type = other DNA
agcaccttctcaggaggagacaatgaatctgaaaacagcgatgtggatattggcgaacctgataccgagggatatgctatcactgaccggggatctgctcccatctctatggggttcaga

SEQ ID NO: 2010 - DNA, 120 bp, synthetic construct
  source 1..120: mol_type = other DNA
gataccgagggatatgctatcactgaccggggatctgctcccatctctatggggttcagagcttctgatgttgaaactgcagaaggaggggagatccacgagctcctgagactccaatcc

SEQ ID NO: 2011 - DNA, 120 bp, synthetic construct
  source 1..120: mol_type = other DNA
gcttctgatgttgaaactgcagaaggaggggagatccacgagctcctgagactccaatccagaggcaacaactttctgaagcctgggaagactctcaatgttcccccgcctccggacccc

SEQ ID NO: 2012 - DNA, 120 bp, synthetic construct
  source 1..120: mol_type = other DNA
agaggcaacaactttctgaagcctgggaagactctcaatgttcccccgcctccggaccccggtagagccgacacttctgagacacccattaaaaagggcacagacgcgagattagcctca

SEQ ID NO: 2013 - DNA, 120 bp, synthetic construct
  source 1..120: mol_type = other DNA
ggtagagccgacacttctgagacacccattaaaaagggcacagacgcgagattagcctcatttggaacggagatcgcgtctttattgacaggtggtgcaacccaatgtgctcgaaagtcg

SEQ ID NO: 2014 - DNA, 120 bp, synthetic construct
  source 1..120: mol_type = other DNA
tttggaacggagatcgcgtctttattgacaggtggtgcaacccaatgtgctcgaaagtcgccctcggaaccatcagggccaggtgcacctgcggagaatgtccccgagtatgtgagcaat

SEQ ID NO: 2015 - DNA, 120 bp, synthetic construct
  source 1..120: mol_type = other DNA
ccctcggaaccatcagggccaggtgcacctgcggagaatgtccccgagtatgtgagcaatgccgcactgatacaggagtggacacccgaatctggtaccacaatctccccgagatcccag

SEQ ID NO: 2016 - DNA, 120 bp, synthetic construct
  source 1..120: mol_type = other DNA
gccgcactgatacaggagtggacacccgaatctggtaccacaatctccccgagatcccagaataatgaagaagggggagaatactatgatgatgagctgttctctgatgtccaagatatc

SEQ ID NO: 2017 - DNA, 120 bp, synthetic construct
  source 1..120: mol_type = other DNA
aataatgaagaagggggagaatactatgatgatgagctgttctctgatgtccaagatatcaaaacagccctggccaaaatacacgaggacaaccagaagataatctccaagctagaatca

SEQ ID NO: 2018 - DNA, 120 bp, synthetic construct
  source 1..120: mol_type = other DNA
aaaacagccctggccaaaatacacgaggacaaccagaagataatctccaagctagaatcactgctgttattgaaaggagaagttgagtcaatcaagaagcagatcaacaagcaaaatatc

SEQ ID NO: 2019 - DNA, 120 bp, synthetic construct
  source 1..120: mol_type = other DNA
ctgctgttattgaaaggagaagttgagtcaatcaagaagcagatcaacaagcaaaatatcagcatatccaccctagaagggcacctctcaagcatcatgatagccattcctggatttggg

SEQ ID NO: 2020 - DNA, 120 bp, synthetic construct
  source 1..120: mol_type = other DNA
agcatatccaccctagaagggcacctctcaagcatcatgatagccattcctggatttgggaaggatcccaacgaccctactgcagatgtcgaaatcaatcccgacttgaaacccatcata

SEQ ID NO: 2021 - DNA, 120 bp, synthetic construct
  source 1..120: mol_type = other DNA
aaggatcccaacgaccctactgcagatgtcgaaatcaatcccgacttgaaacccatcataagtagagattcaggccgagcactggccgaagttctcaagaaacccattgccagccgacaa

SEQ ID NO: 2022 - DNA, 120 bp, synthetic construct
  source 1..120: mol_type = other DNA
agtagagattcaggccgagcactggccgaagttctcaagaaacccattgccagccgacaactccaaggaatgacaaatggacggaccagttccagaggacagctacttaaggaatttcaa

SEQ ID NO: 2023 - DNA, 120 bp, synthetic construct
  source 1..120: mol_type = other DNA
ctccaaggaatgacaaatggacggaccagttccagaggacagctacttaaggaatttcaactaaagccgatcgggaaaaagatgagctcagccgtcgggtttgttcctgacaccggccct

SEQ ID NO: 2024 - DNA, 120 bp, synthetic construct
  source 1..120: mol_type = other DNA
ctaaagccgatcgggaaaaagatgagctcagccgtcgggtttgttcctgacaccggccctgcatcacgcagtgtaatccgctccattataaaatctagccggctagaggaggatcggaag

SEQ ID NO: 2025 - DNA, 120 bp, synthetic construct
  source 1..120: mol_type = other DNA
gcatcacgcagtgtaatccgctccattataaaatctagccggctagaggaggatcggaagcgttacctgatgactctccttgatgatatcaaaggagccaacgatcttgccaagttccac

SEQ ID NO: 2026 - DNA, 120 bp, synthetic construct
  source 1..120: mol_type = other DNA
cgttacctgatgactctccttgatgatatcaaaggagccaacgatcttgccaagttccaccagatgctgatgaaaataataatgaagtagctacagctcaacttacctgccaaccccatg

SEQ ID NO: 2027 - DNA, 120 bp, synthetic construct
  source 1..120: mol_type = other DNA
cagatgctgatgaaaataataatgaagtagctacagctcaacttacctgccaaccccatgccagtcgacccaaccagtacaacctaagtccattataaaaaacttaggagcaaagtgatt

SEQ ID NO: 2028 - DNA, 120 bp, synthetic construct
  source 1..120: mol_type = other DNA
ccagtcgacccaaccagtacaacctaagtccattataaaaaacttaggagcaaagtgattgcctcccaagctccacaatgacagagatctacgacttcgacaagtcggcatgggacatca

SEQ ID NO: 2029 - DNA, 120 bp, synthetic construct
  source 1..120: mol_type = other DNA
gcctcccaagctccacaatgacagagatctacgacttcgacaagtcggcatgggacatcaaagggtcgatcgctccgattcaacccaccacatacagtgatgggaggctggtgccccagg

SEQ ID NO: 2030 - DNA, 120 bp, synthetic construct
  source 1..120: mol_type = other DNA
aagggtcgatcgctccgattcaacccaccacatacagtgatgggaggctggtgccccaggtcagagtcatagatcctggtctaggcgacaggaaggatgaatgctttatgtacatgtttc

SEQ ID NO: 2031 - DNA, 120 bp, synthetic construct
  source 1..120: mol_type = other DNA
tcagagtcatagatcctggtctaggcgacaggaaggatgaatgctttatgtacatgtttctgctgggggttgttgaggacagcgatcccctagggcccccaatcgggcgagcatttgggt

SEQ ID NO: 2032 - DNA, 120 bp, synthetic construct
  source 1..120: mol_type = other DNA
tgctgggggttgttgaggacagcgatcccctagggcccccaatcgggcgagcatttgggtccctgcccctaggtgttggcagatccacagcaaaacccgaagaactcctcaaggaggcca

SEQ ID NO: 2033 - DNA, 120 bp, synthetic construct
  source 1..120: mol_type = other DNA
ccctgcccctaggtgttggcagatccacagcaaaacccgaagaactcctcaaggaggccactgagcttgacatagttgttagacgtacagcagggctcaatgaaaaactggtgttctaca

SEQ ID NO: 2034 - DNA, 120 bp, synthetic construct
  source 1..120: mol_type = other DNA
ctgagcttgacatagttgttagacgtacagcagggctcaatgaaaaactggtgttctacaacaacactccactaaccctcctcacaccttggagaaaggtcctgacaacagggagtgtct

SEQ ID NO: 2035 - DNA, 120 bp, synthetic construct
  source 1..120: mol_type = other DNA
acaacactccactaaccctcctcacaccttggagaaaggtcctgacaacagggagtgtcttcaacgcaaatcaagtgtgcaatgcggttaatctgataccgctggataccccgcagaggt

SEQ ID NO: 2036 - DNA, 120 bp, synthetic construct
  source 1..120: mol_type = other DNA
tcaacgcaaatcaagtgtgcaatgcggttaatctgataccgctggataccccgcagaggttccgtgttgtttatatgagcatcacccgtctttcagataacgggtattacactgttccta

SEQ ID NO: 2037 - DNA, 120 bp, synthetic construct
  source 1..120: mol_type = other DNA
tccgtgttgtttatatgagcatcacccgtctttcagataacgggtattacactgttcctagaagaatgctggaattcagatcagtcaatgcagtggccttcaacctgctggtgaccctta

SEQ ID NO: 2038 - DNA, 120 bp, synthetic construct
  source 1..120: mol_type = other DNA
gaagaatgctggaattcagatcagtcaatgcagtggccttcaacctgctggtgacccttaggattgacaaggcaattggccctgggaagatcatcgacaatacagagcaacttcctgagg

SEQ ID NO: 2039 - DNA, 120 bp, synthetic construct
  source 1..120: mol_type = other DNA
ggattgacaaggcaattggccctgggaagatcatcgacaatacagagcaacttcctgaggcaacatttatggttcacatcgggaacttcaggagaaagaagaatgaagtctactctgccg

SEQ ID NO: 2040 - DNA, 120 bp, synthetic construct
  source 1..120: mol_type = other DNA
caacatttatggttcacatcgggaacttcaggagaaagaagaatgaagtctactctgccgattattgcaaaatgaagatcgaaaagatgggtctagtttttgcacttggcgggatagggg

SEQ ID NO: 2041 - DNA, 120 bp, synthetic construct
  source 1..120: mol_type = other DNA
attattgcaaaatgaagatcgaaaagatgggtctagtttttgcacttggcgggatagggggcaccagtcttcacattagaagcacaggcaaaatgagcaagaccctccatgcacaactcg

SEQ ID NO: 2042 - DNA, 120 bp, synthetic construct
  source 1..120: mol_type = other DNA
gcaccagtcttcacattagaagcacaggcaaaatgagcaagaccctccatgcacaactcgggttcaagaagaccttatgttacccactgatggatatcaatgaagaccttaatcgattac

SEQ ID NO: 2043 - DNA, 120 bp, synthetic construct
  source 1..120: mol_type = other DNA
ggttcaagaagaccttatgttacccactgatggatatcaatgaagaccttaatcgattactctggaggagcagatgcaagatagtaagaatccaggcagtcttgcagccatcagttcctc

SEQ ID NO: 2044 - DNA, 120 bp, synthetic construct
  source 1..120: mol_type = other DNA
tctggaggagcagatgcaagatagtaagaatccaggcagtcttgcagccatcagttcctcaagaattccgcatttacgatgacgtgatcataaatgatgatcaaggactcttcaaagttc

SEQ ID NO: 2045 - DNA, 120 bp, synthetic construct
  source 1..120: mol_type = other DNA
aagaattccgcatttacgatgacgtgatcataaatgatgatcaaggactcttcaaagttctgtagaccgtagtgctcagcagtgcccaaaaacaacccccctcacaatgacagtcagaat

SEQ ID NO: 2046 - DNA, 120 bp, synthetic construct
  source 1..120: mol_type = other DNA
tgtagaccgtagtgctcagcagtgcccaaaaacaacccccctcacaatgacagtcagaattcccggacaaaaaagccccctccgagagactccacggactaagcgagaggccaactagca

SEQ ID NO: 2047 - DNA, 120 bp, synthetic construct
  source 1..120: mol_type = other DNA
tcccggacaaaaaagccccctccgagagactccacggactaagcgagaggccaactagcagccgacggcaagcgcgaacaccaggtggccccagcataggagagtcccgacccagggcca

SEQ ID NO: 2048 - DNA, 120 bp, synthetic construct
  source 1..120: mol_type = other DNA
gccgacggcaagcgcgaacaccaggtggccccagcataggagagtcccgacccagggccaccaccagctatcccaatccgcatcatcctcgtgtgacccccgaggaccagcctccaaggt

SEQ ID NO: 2049 - DNA, 120 bp, synthetic construct
  source 1..120: mol_type = other DNA
ccaccagctatcccaatccgcatcatcctcgtgtgacccccgaggaccagcctccaaggttgcccccgacccaaaccaccaaccacatccccaccacccccgggaaagaaacccccagca

SEQ ID NO: 2050 - DNA, 120 bp, synthetic construct
  source 1..120: mol_type = other DNA
tgcccccgacccaaaccaccaaccacatccccaccacccccgggaaagaaacccccagcagctggaaggcccctctccccctctcccaacacaagaaccccacaaccggatcgcacaagc

SEQ ID NO: 2051 - DNA, 120 bp, synthetic construct
  source 1..120: mol_type = other DNA
gctggaaggcccctctccccctctcccaacacaagaaccccacaaccggatcgcacaagcgaccgaggtgacccaaccacaggcacccgactccccaggcaaatcctctccccccggcaa

SEQ ID NO: 2052 - DNA, 120 bp, synthetic construct
  source 1..120: mol_type = other DNA
gaccgaggtgacccaaccacaggcacccgactccccaggcaaatcctctccccccggcaaactaaacaaaacttagggccaaggaacacacacacccaacagaacccagaccccggccca

SEQ ID NO: 2053 - DNA, 120 bp, synthetic construct
  source 1..120: mol_type = other DNA
actaaacaaaacttagggccaaggaacacacacacccaacagaacccagaccccggcccacggcaccgcgcccccaacccccgacaaccagagggagcccccaaccaatcccgccggctc

SEQ ID NO: 2054 - DNA, 120 bp, synthetic construct
  source 1..120: mol_type = other DNA
cggcaccgcgcccccaacccccgacaaccagagggagcccccaaccaatcccgccggctcccccggcgcccacaggcaggcacaccaacccccgaacagactcagcacccagccacctac

SEQ ID NO: 2055 - DNA, 120 bp, synthetic construct
  source 1..120: mol_type = other DNA
ccccggcgcccacaggcaggcacaccaacccccgaacagactcagcacccagccacctacaatccaagacgggggggcccccccaaaaaagggcccccaggggccgacaaccagggcagc

SEQ ID NO: 2056 - DNA, 120 bp, synthetic construct
  source 1..120: mol_type = other DNA
aatccaagacgggggggcccccccaaaaaagggcccccaggggccgacaaccagggcagcgaggaagcccacccacaccacacaccatcacggcaaccagatcagaacccagaccaccct

SEQ ID NO: 2057 - DNA, 120 bp, synthetic construct
  source 1..120: mol_type = other DNA
gaggaagcccacccacaccacacaccatcacggcaaccagatcagaacccagaccaccctgggccaccaactcccagacccggccaccaccccgcggaaagggacggccacaacccgcac

SEQ ID NO: 2058 - DNA, 120 bp, synthetic construct
  source 1..120: mol_type = other DNA
gggccaccaactcccagacccggccaccaccccgcggaaagggacggccacaacccgcacaccccagccccgatccggcgggcagccacccaacccgaaccagcacccaagagcgacccc

SEQ ID NO: 2059 - DNA, 120 bp, synthetic construct
  source 1..120: mol_type = other DNA
accccagccccgatccggcgggcagccacccaacccgaaccagcacccaagagcgacccccgaaggacccccaaaccgcaaaggacatcagcatcccacagcctctccaagtcccccggt

SEQ ID NO: 2060 - DNA, 120 bp, synthetic construct
  source 1..120: mol_type = other DNA
cgaaggacccccaaaccgcaaaggacatcagcatcccacagcctctccaagtcccccggtctcccccccttctcgaagggacaaaaagatcaacccactatatccgacgtcactcaactc

SEQ ID NO: 2061 - DNA, 120 bp, synthetic construct
  source 1..120: mol_type = other DNA
ctcccccccttctcgaagggacaaaaagatcaacccactatatccgacgtcactcaactccccacccctagagaagacaccagggatcccagaatcaagactcatccaatatccatcatg

SEQ ID NO: 2062 - DNA, 120 bp, synthetic construct
  source 1..120: mol_type = other DNA
cccacccctagagaagacaccagggatcccagaatcaagactcatccaatatccatcatgggtctcaaggtgaacgtctctgccgtattcatggcagtactgttaactctccaaacaccc

SEQ ID NO: 2063 - DNA, 120 bp, synthetic construct
  source 1..120: mol_type = other DNA
ggtctcaaggtgaacgtctctgccgtattcatggcagtactgttaactctccaaacacccgccggtcaaattcattggggcaatctctctaagataggggtagtaggaataggaagtgca

SEQ ID NO: 2064 - DNA, 120 bp, synthetic construct
  source 1..120: mol_type = other DNA
gccggtcaaattcattggggcaatctctctaagataggggtagtaggaataggaagtgcaagctacaaagttatgactcgttccagccatcaatcattagtcataaaattaatgcccaat

SEQ ID NO: 2065 - DNA, 120 bp, synthetic construct
  source 1..120: mol_type = other DNA
agctacaaagttatgactcgttccagccatcaatcattagtcataaaattaatgcccaatataactctcctcaataactgcacgagggtagagattgcagaatacaggaggctactaaga

SEQ ID NO: 2066 - DNA, 120 bp, synthetic construct
  source 1..120: mol_type = other DNA
ataactctcctcaataactgcacgagggtagagattgcagaatacaggaggctactaagaacagttttggaaccaattagagatgcacttaatgcaatgacccagaacataaggccggtt

SEQ ID NO: 2067 - DNA, 120 bp, synthetic construct
  source 1..120: mol_type = other DNA
acagttttggaaccaattagagatgcacttaatgcaatgacccagaacataaggccggttcagagcgtagcttcaagtaggagacacaagagatttgcgggagtagtcctggcaggtgcg

SEQ ID NO: 2068 - DNA, 120 bp, synthetic construct
  source 1..120: mol_type = other DNA
cagagcgtagcttcaagtaggagacacaagagatttgcgggagtagtcctggcaggtgcggccctaggtgttgccacatctgctcagataacagccggcattgcacttcaccggtccatg

SEQ ID NO: 2069 - DNA, 120 bp, synthetic construct
  source 1..120: mol_type = other DNA
gccctaggtgttgccacatctgctcagataacagccggcattgcacttcaccggtccatgctgaactctcaggccatcgacaatctgagagcgagcctggaaactactaatcaggcaatt

SEQ ID NO: 2070 - DNA, 120 bp, synthetic construct
  source 1..120: mol_type = other DNA
ctgaactctcaggccatcgacaatctgagagcgagcctggaaactactaatcaggcaattgaggcaatcagacaagcagggcaggagatgatattggctgttcagggtgtccaagactac

SEQ ID NO: 2071 - DNA, 120 bp, synthetic construct
  source 1..120: mol_type = other DNA
gaggcaatcagacaagcagggcaggagatgatattggctgttcagggtgtccaagactacatcaataatgagctgataccgtctatgaaccagctgtcttgtgatctaatcggtcagaag

SEQ ID NO: 2072 - DNA, 120 bp, synthetic construct
  source 1..120: mol_type = other DNA
atcaataatgagctgataccgtctatgaaccagctgtcttgtgatctaatcggtcagaagctcgggctcaaattgcttagatactatacagaaatcctgtcactatttggccccagccta

SEQ ID NO: 2073 - DNA, 120 bp, synthetic construct
  source 1..120: mol_type = other DNA
ctcgggctcaaattgcttagatactatacagaaatcctgtcactatttggccccagcctacgggaccccatatctgcggagatatctatccaggctttgagctatgcacttggaggagat

SEQ ID NO: 2074 - DNA, 120 bp, synthetic construct
  source 1..120: mol_type = other DNA
cgggaccccatatctgcggagatatctatccaggctttgagctatgcacttggaggagatatcaataaggtgttagaaaagctcggatacagtggaggcgatttactaggcatcttagag

SEQ ID NO: 2075 - DNA, 120 bp, synthetic construct
  source 1..120: mol_type = other DNA
atcaataaggtgttagaaaagctcggatacagtggaggcgatttactaggcatcttagagagcagaggaataaaggctcggataactcacgtcgacacagagtcctacttcatagtcctc

SEQ ID NO: 2076 - DNA, 120 bp, synthetic construct
  source 1..120: mol_type = other DNA
agcagaggaataaaggctcggataactcacgtcgacacagagtcctacttcatagtcctcagtatagcctatccgacgctgtccgagattaagggggtgattgtccaccggctagagggg

SEQ ID NO: 2077 - DNA, 120 bp, synthetic construct
  source 1..120: mol_type = other DNA
agtatagcctatccgacgctgtccgagattaagggggtgattgtccaccggctagagggggtctcgtataacataggctctcaagagtggtataccactgtgcccaagtatgttgcaacc

SEQ ID NO: 2078 - DNA, 120 bp, synthetic construct
  source 1..120: mol_type = other DNA
gtctcgtataacataggctctcaagagtggtataccactgtgcccaagtatgttgcaacccaagggtaccttatctcgaattttgatgagtcgtcatgtactttcatgccagaggggact

SEQ ID NO: 2079 - DNA, 120 bp, synthetic construct
  source 1..120: mol_type = other DNA
caagggtaccttatctcgaattttgatgagtcgtcatgtactttcatgccagaggggactgtgtgcagccaaaatgccttgtacccgatgagtcctctgctccaagaatgcctccggggg

SEQ ID NO: 2080 - DNA, 120 bp, synthetic construct
  source 1..120: mol_type = other DNA
gtgtgcagccaaaatgccttgtacccgatgagtcctctgctccaagaatgcctccgggggtccaccaagtcctgtgctcgtacacttgtatccgggtcttttgggaaccggttcatttta

SEQ ID NO: 2081 - DNA, 120 bp, synthetic construct
  source 1..120: mol_type = other DNA
tccaccaagtcctgtgctcgtacacttgtatccgggtcttttgggaaccggttcattttatcacaagggaacctaatagccaattgtgcatcaattctctgtaagtgttacacaacaggt

SEQ ID NO: 2082 - DNA, 120 bp, synthetic construct
  source 1..120: mol_type = other DNA
tcacaagggaacctaatagccaattgtgcatcaattctctgtaagtgttacacaacaggtacgattattaatcaagaccctgacaagatcctaacatacattgctgccgatcgctgcccg

SEQ ID NO: 2083 - DNA, 120 bp, synthetic construct
  source 1..120: mol_type = other DNA
acgattattaatcaagaccctgacaagatcctaacatacattgctgccgatcgctgcccggtagtcgaggtgaacggcgtgaccatccaagtcgggagcaggaggtatccagatgctgtg

SEQ ID NO: 2084 - DNA, 120 bp, synthetic construct
  source 1..120: mol_type = other DNA
gtagtcgaggtgaacggcgtgaccatccaagtcgggagcaggaggtatccagatgctgtgtacttgcacagaattgacctcggtcctcccatatcattggagagattggacgtagggaca

SEQ ID NO: 2085 - DNA, 120 bp, synthetic construct
  source 1..120: mol_type = other DNA
tacttgcacagaattgacctcggtcctcccatatcattggagagattggacgtagggacaaatctggggaatgcaattgccaaactggaggatgccaaggaattgttggaatcatcggac

SEQ ID NO: 2086 - DNA, 120 bp, synthetic construct
  source 1..120: mol_type = other DNA
aatctggggaatgcaattgccaaactggaggatgccaaggaattgttggaatcatcggaccagatattgagaagtatgaaaggtttatcgagcactagcatagtctacatcctgattgca

SEQ ID NO: 2087 - DNA, 120 bp, synthetic construct
  source 1..120: mol_type = other DNA
cagatattgagaagtatgaaaggtttatcgagcactagcatagtctacatcctgattgcagtgtgtcttggagggttgatagggatccccactttaatatgttgctgcagggggcgttgt

SEQ ID NO: 2088 - DNA, 120 bp, synthetic construct
  source 1..120: mol_type = other DNA
gtgtgtcttggagggttgatagggatccccactttaatatgttgctgcagggggcgttgtaacaaaaagggagaacaagttggtatgtcaagaccaggcctaaagcctgaccttacggga

SEQ ID NO: 2089 - DNA, 120 bp, synthetic construct
  source 1..120: mol_type = other DNA
aacaaaaagggagaacaagttggtatgtcaagaccaggcctaaagcctgaccttacgggaacatcaaaatcctatgtaagatcgctttgatcctctacaactcttgaaacacaagtgtcc

SEQ ID NO: 2090 - DNA, 120 bp, synthetic construct
  source 1..120: mol_type = other DNA
acatcaaaatcctatgtaagatcgctttgatcctctacaactcttgaaacacaagtgtcccagaattctcctcttagtcatcaagcaaccaccgtgcccgacatcaagccaccctgaaat

SEQ ID NO: 2091 - DNA, 120 bp, synthetic construct
  source 1..120: mol_type = other DNA
cagaattctcctcttagtcatcaagcaaccaccgtgcccgacatcaagccaccctgaaattttctccggcttccctctagccgaacaatatcgataattaattaaaacttagggtgcaag

SEQ ID NO: 2092 - DNA, 120 bp, synthetic construct
  source 1..120: mol_type = other DNA
tttctccggcttccctctagccgaacaatatcgataattaattaaaacttagggtgcaagaccatccacaatgtcaccgcaacgagaccggataaatgccttttacaaagataaccctta

SEQ ID NO: 2093 - DNA, 120 bp, synthetic construct
  source 1..120: mol_type = other DNA
accatccacaatgtcaccgcaacgagaccggataaatgccttttacaaagataacccttatcccaagggaagtaggatagttattaacagagaacatcttatgattgacagaccctatgt

SEQ ID NO: 2094 - DNA, 120 bp, synthetic construct
  source 1..120: mol_type = other DNA
tcccaagggaagtaggatagttattaacagagaacatcttatgattgacagaccctatgttctgctggctgttctgttcgtcatgtttctgagcttgatcggattgctggcaattgcagg

SEQ ID NO: 2095 - DNA, 120 bp, synthetic construct
  source 1..120: mol_type = other DNA
tctgctggctgttctgttcgtcatgtttctgagcttgatcggattgctggcaattgcaggcattagacttcatcgagcagccatctacaccgcggagatccataaaagcctcagtaccaa

SEQ ID NO: 2096 - DNA, 120 bp, synthetic construct
  source 1..120: mol_type = other DNA
cattagacttcatcgagcagccatctacaccgcggagatccataaaagcctcagtaccaatctagatgtgactaactcaatcgagcatcaagtcaaggacgtgctgacaccactctttaa

SEQ ID NO: 2097 - DNA, 120 bp, synthetic construct
  source 1..120: mol_type = other DNA
tctagatgtgactaactcaatcgagcatcaagtcaaggacgtgctgacaccactctttaagatcatcggggatgaagtgggcctgagaacacctcagagattcactgacctagtgaaatt

SEQ ID NO: 2098 - DNA, 120 bp, synthetic construct
  source 1..120: mol_type = other DNA
gatcatcggggatgaagtgggcctgagaacacctcagagattcactgacctagtgaaattcatctcggacaagattaaattccttaatccggatagggagtacgacttcagagatctcac

SEQ ID NO: 2099 - DNA, 120 bp, synthetic construct
  source 1..120: mol_type = other DNA
catctcggacaagattaaattccttaatccggatagggagtacgacttcagagatctcacttggtgcatcaatccgccagagaggatcaaactagattatgatcaatactgtgcagatgt

SEQ ID NO: 2100 - DNA, 120 bp, synthetic construct
  source 1..120: mol_type = other DNA
ttggtgcatcaatccgccagagaggatcaaactagattatgatcaatactgtgcagatgtggctgctgaagagctcatgaatacattggtgaactcaactctactggagaccagaacaac

SEQ ID NO: 2101 - DNA, 120 bp, synthetic construct
  source 1..120: mol_type = other DNA
ggctgctgaagagctcatgaatacattggtgaactcaactctactggagaccagaacaaccaatcagttcctagctgtctcaaagggaaactgctcagggcccactacaatcagaggtca

SEQ ID NO: 2102 - DNA, 120 bp, synthetic construct
  source 1..120: mol_type = other DNA
caatcagttcctagctgtctcaaagggaaactgctcagggcccactacaatcagaggtcaattctcaaacatgtcgctgtccttgttggacttgtacttaggtcgaggttacaatgtgtc

SEQ ID NO: 2103 - DNA, 120 bp, synthetic construct
  source 1..120: mol_type = other DNA
attctcaaacatgtcgctgtccttgttggacttgtacttaggtcgaggttacaatgtgtcatctatagtcactataacatcccagggaatgtatgggggaacctacctagttgaaaagcc

SEQ ID NO: 2104 - DNA, 120 bp, synthetic construct
  source 1..120: mol_type = other DNA
atctatagtcactataacatcccagggaatgtatgggggaacctacctagttgaaaagcctaatctgaacagcaaagggtcagagttgtcacaactgagcatgtaccgagtgtttgaagt

SEQ ID NO: 2105 - DNA, 120 bp, synthetic construct
  source 1..120: mol_type = other DNA
taatctgaacagcaaagggtcagagttgtcacaactgagcatgtaccgagtgtttgaagtaggtgttatcagaaacccgggtttgggggctccggtgttccatatgacaaactattttga

SEQ ID NO: 2106 - DNA, 120 bp, synthetic construct
  source 1..120: mol_type = other DNA
aggtgttatcagaaacccgggtttgggggctccggtgttccatatgacaaactattttgagcaaccagtcagtgatggtctcggcaactgtatggtggctttgggggagctcaaactcgc

SEQ ID NO: 2107 - DNA, 120 bp, synthetic construct
  source 1..120: mol_type = other DNA
gcaaccagtcagtgatggtctcggcaactgtatggtggctttgggggagctcaaactcgcagccctttgtcacggggacgattctatcacaattccctatcggggatcagggaaaggtgt

SEQ ID NO: 2108 - DNA, 120 bp, synthetic construct
  source 1..120: mol_type = other DNA
agccctttgtcacggggacgattctatcacaattccctatcggggatcagggaaaggtgtcagcttccagctcgtcaagctgggtgtctggaaatccccaaccgacatgcaatcctgggt

SEQ ID NO: 2109 - DNA, 120 bp, synthetic construct
  source 1..120: mol_type = other DNA
cagcttccagctcgtcaagctgggtgtctggaaatccccaaccgacatgcaatcctgggtccccttatcaacggatgatccagtagtagacaggctttacctctcatctcacagaggtgt

SEQ ID NO: 2110 - DNA, 120 bp, synthetic construct
  source 1..120: mol_type = other DNA
ccccttatcaacggatgatccagtagtagacaggctttacctctcatctcacagaggtgtcatcgctgacaatcaagcaaaatgggctgtcccgacaacacgaacagatgacaagttgcg

SEQ ID NO: 2111 - DNA, 120 bp, synthetic construct
  source 1..120: mol_type = other DNA
catcgctgacaatcaagcaaaatgggctgtcccgacaacacgaacagatgacaagttgcgaatggagacatgcttccagcaggcgtgtaaaggtaaaatccaagcactctgcgagaatcc

SEQ ID NO: 2112 - DNA, 120 bp, synthetic construct
  source 1..120: mol_type = other DNA
aatggagacatgcttccagcaggcgtgtaaaggtaaaatccaagcactctgcgagaatcccgagtgggtaccattgaaggataacaggattccttcatacggggtcctgtctgttgatct

SEQ ID NO: 2113 - DNA, 120 bp, synthetic construct
  source 1..120: mol_type = other DNA
cgagtgggtaccattgaaggataacaggattccttcatacggggtcctgtctgttgatctgagtttgacagttgagcttaaaatcaaaattgcttcgggattcgggccattgatcacaca

SEQ ID NO: 2114 - DNA, 120 bp, synthetic construct
  source 1..120: mol_type = other DNA
gagtttgacagttgagcttaaaatcaaaattgcttcgggattcgggccattgatcacacacggctcagggatggacctatacaaatccaaccgcaacaatgtgtattggctgactattcc

SEQ ID NO: 2115 - DNA, 120 bp, synthetic construct
  source 1..120: mol_type = other DNA
cggctcagggatggacctatacaaatccaaccgcaacaatgtgtattggctgactattccgccaatgagaaatctagccttaggcgtaatcaacacattggagtggataccgagattcaa

SEQ ID NO: 2116 - DNA, 120 bp, synthetic construct
  source 1..120: mol_type = other DNA
gccaatgagaaatctagccttaggcgtaatcaacacattggagtggataccgagattcaaagttagtcccaacctcttcactgtcccaattaaggaagcaggcgaagactgccatgcccc

SEQ ID NO: 2117 - DNA, 120 bp, synthetic construct
  source 1..120: mol_type = other DNA
agttagtcccaacctcttcactgtcccaattaaggaagcaggcgaagactgccatgccccaacatacctacctgcggaggtggacggtgatgtcaaactcagttccaacctggtgattct

SEQ ID NO: 2118 - DNA, 120 bp, synthetic construct
  source 1..120: mol_type = other DNA
aacatacctacctgcggaggtggacggtgatgtcaaactcagttccaacctggtgattctacctggtcaagatctccaatatgttttggcaacctacgacacctccagggttgagcatgc

SEQ ID NO: 2119 - DNA, 120 bp, synthetic construct
  source 1..120: mol_type = other DNA
acctggtcaagatctccaatatgttttggcaacctacgacacctccagggttgagcatgctgtggtttattacgtttacagcccaagccgctcattttcctacttttatccttttaggtt

SEQ ID NO: 2120 - DNA, 120 bp, synthetic construct
  source 1..120: mol_type = other DNA
tgtggtttattacgtttacagcccaagccgctcattttcctacttttatccttttaggttgcctataaagggggtcccaatcgaactacaagtggaatgcttcacatgggaccaaaaact

SEQ ID NO: 2121 - DNA, 120 bp, synthetic construct
  source 1..120: mol_type = other DNA
gcctataaagggggtcccaatcgaactacaagtggaatgcttcacatgggaccaaaaactctggtgccgtcacttctgtgtgcttgcggactcagaatccggtggacatatcactcactc

SEQ ID NO: 2122 - DNA, 120 bp, synthetic construct
  source 1..120: mol_type = other DNA
ctggtgccgtcacttctgtgtgcttgcggactcagaatccggtggacatatcactcactctgggatggttggcatgggagtcagctgcacagctacccgggaagatggaaccaatcgcag

SEQ ID NO: 2123 - DNA, 120 bp, synthetic construct
  source 1..120: mol_type = other DNA
tgggatggttggcatgggagtcagctgcacagctacccgggaagatggaaccaatcgcagataaggctgttagtgaaccaatcacatgatgtcgcccagacatcaggcatacccactagt

SEQ ID NO: 2124 - DNA, 120 bp, synthetic construct
  source 1..120: mol_type = other DNA
ataaggctgttagtgaaccaatcacatgatgtcgcccagacatcaggcatacccactagtgtgaaatagacatcagaattaagaaaaacgtagggtccaagtagttccccattatggact

SEQ ID NO: 2125 - DNA, 120 bp, synthetic construct
  source 1..120: mol_type = other DNA
gtgaaatagacatcagaattaagaaaaacgtagggtccaagtagttccccattatggactcgctatctgtcaaccagatcttataccctgaagttcatctggatagtccgatagtcacca

SEQ ID NO: 2126 - DNA, 120 bp, synthetic construct
  source 1..120: mol_type = other DNA
cgctatctgtcaaccagatcttataccctgaagttcatctggatagtccgatagtcaccaataagatagtagccatcctggagtatgctagactccctcacgcttacagcttggaggacc

SEQ ID NO: 2127 - DNA, 120 bp, synthetic construct
  source 1..120: mol_type = other DNA
ataagatagtagccatcctggagtatgctagactccctcacgcttacagcttggaggaccctacattgtgtcagaacatcaagcaccgcctaaaaaccggattttccaaccaaatgatta

SEQ ID NO: 2128 - DNA, 120 bp, synthetic construct
  source 1..120: mol_type = other DNA
ctacattgtgtcagaacatcaagcaccgcctaaaaaccggattttccaaccaaatgattataaacaatgtggaagttgggaatgtcatcaagtccaagcttaggagttatccgacccact

SEQ ID NO: 2129 - DNA, 120 bp, synthetic construct
  source 1..120: mol_type = other DNA
taaacaatgtggaagttgggaatgtcatcaagtccaagcttaggagttatccgacccactctcatattccatatccaaattgtaatcaggatttatttaacatagaagacaaagagtcaa

SEQ ID NO: 2130 - DNA, 120 bp, synthetic construct
  source 1..120: mol_type = other DNA
ctcatattccatatccaaattgtaatcaggatttatttaacatagaagacaaagagtcaacgaggaagatccgtgaacttctcaaaaagggaaatttgctgtactccaaagtcagtgata

SEQ ID NO: 2131 - DNA, 120 bp, synthetic construct
  source 1..120: mol_type = other DNA
cgaggaagatccgtgaacttctcaaaaagggaaatttgctgtactccaaagtcagtgataaggttttccaatgcttgagggacattaactcacggcttggcctaggctccgaattgaggg

SEQ ID NO: 2132 - DNA, 120 bp, synthetic construct
  source 1..120: mol_type = other DNA
aggttttccaatgcttgagggacattaactcacggcttggcctaggctccgaattgagggaggacatcaaggagaaagttactaacttgggagtttacatgcacagctcccaatggtttg

SEQ ID NO: 2133 - DNA, 120 bp, synthetic construct
  source 1..120: mol_type = other DNA
aggacatcaaggagaaagttactaacttgggagtttacatgcacagctcccaatggtttgagccctttctgttttggtttacagtcaagaccgagatgaggtcagtgattaaatcacaaa

SEQ ID NO: 2134 - DNA, 120 bp, synthetic construct
  source 1..120: mol_type = other DNA
agccctttctgttttggtttacagtcaagaccgagatgaggtcagtgattaaatcacaaacccatacttgccataggaggagacacacacctgtattcttcactggtagttcagttgagt

SEQ ID NO: 2135 - DNA, 120 bp, synthetic construct
  source 1..120: mol_type = other DNA
cccatacttgccataggaggagacacacacctgtattcttcactggtagttcagttgagttgctaatctctcgtgaccttgttgctataataagtagagagtctcaacatgtatattacc

SEQ ID NO: 2136 - DNA, 120 bp, synthetic construct
  source 1..120: mol_type = other DNA
tgctaatctctcgtgaccttgttgctataataagtagagagtctcaacatgtatattacctgacatttgagctggttttgatgtattgtgatgtcatagaggggaggttaatgacagata

SEQ ID NO: 2137 - DNA, 120 bp, synthetic construct
  source 1..120: mol_type = other DNA
tgacatttgagctggttttgatgtattgtgatgtcatagaggggaggttaatgacagataccgctatgaccattgatgctaggtatactgagcttctaggaagagtcaggtacatgtgga

SEQ ID NO: 2138 - DNA, 120 bp, synthetic construct
  source 1..120: mol_type = other DNA
ccgctatgaccattgatgctaggtatactgagcttctaggaagagtcaggtacatgtggaaactgatagatggtttcttccctgcactcggtaatccaacttatcaaattgtagccatgc

SEQ ID NO: 2139 - DNA, 120 bp, synthetic construct
  source 1..120: mol_type = other DNA
aactgatagatggtttcttccctgcactcggtaatccaacttatcaaattgtagccatgctggagccactttcacttgcttacctgcaactgagggatataacagtagaactcagaggtg

SEQ ID NO: 2140 - DNA, 120 bp, synthetic construct
  source 1..120: mol_type = other DNA
tggagccactttcacttgcttacctgcaactgagggatataacagtagaactcagaggtgctttccttaaccactgctttactgaaatacatgatgttcttgaccaaaacgggttttctg

SEQ ID NO: 2141 - DNA, 120 bp, synthetic construct
  source 1..120: mol_type = other DNA
ctttccttaaccactgctttactgaaatacatgatgttcttgaccaaaacgggttttctgatgaaggtacttatcatgagttaattgaagctctagattacatcttcataactgatgata

SEQ ID NO: 2142 - DNA, 120 bp, synthetic construct
  source 1..120: mol_type = other DNA
atgaaggtacttatcatgagttaattgaagctctagattacatcttcataactgatgatatacatctgacaggggagattttttcattttttagaagtttcggccaccccagacttgaag

SEQ ID NO: 2143 - DNA, 120 bp, synthetic construct
  source 1..120: mol_type = other DNA
tacatctgacaggggagattttttcattttttagaagtttcggccaccccagacttgaagcagtaacggctgctgaaaatgttaggaaatacatgaatcagcccaaagtcattgtgtatg

SEQ ID NO: 2144 - DNA, 120 bp, synthetic construct
  source 1..120: mol_type = other DNA
cagtaacggctgctgaaaatgttaggaaatacatgaatcagcccaaagtcattgtgtatgagacactgatgaaaggtcatgccatattttgtggaatcataatcaatggctatcgtgaca

SEQ ID NO: 2145 - DNA, 120 bp, synthetic construct
  source 1..120: mol_type = other DNA
agacactgatgaaaggtcatgccatattttgtggaatcataatcaatggctatcgtgacaggcacggaggcagttggccgccgctgaccctccccctacatgctgctgacacaatccgaa

SEQ ID NO: 2146 - DNA, 120 bp, synthetic construct
  source 1..120: mol_type = other DNA
ggcacggaggcagttggccgccgctgaccctccccctacatgctgctgacacaatccgaaatgctcaagcttcaggtgaagggttaacacatgagcagtgcgttgataactggagatcct

SEQ ID NO: 2147 - DNA, 120 bp, synthetic construct
  source 1..120: mol_type = other DNA
atgctcaagcttcaggtgaagggttaacacatgagcagtgcgttgataactggagatcctttgctggagtgaaatttggctgctttatgcctcttagcctggatagtgatctgacaatgt

SEQ ID NO: 2148 - DNA, 120 bp, synthetic construct
  source 1..120: mol_type = other DNA
ttgctggagtgaaatttggctgctttatgcctcttagcctggatagtgatctgacaatgtacctaaaggataaggcacttgctgctctccaaagagaatgggattcagtttacccgaaag

SEQ ID NO: 2149 - DNA, 120 bp, synthetic construct
  source 1..120: mol_type = other DNA
acctaaaggataaggcacttgctgctctccaaagagaatgggattcagtttacccgaaagagttcctgcgttacgaccctcccaagggaaccgggtcccggaggcttgtagatgttttcc

SEQ ID NO: 2150 - DNA, 120 bp, synthetic construct
  source 1..120: mol_type = other DNA
agttcctgcgttacgaccctcccaagggaaccgggtcccggaggcttgtagatgttttccttaatgattcgagctttgacccatatgatatgataatgtatgttgtgagtggagcttacc

SEQ ID NO: 2151 - DNA, 120 bp, synthetic construct
  source 1..120: mol_type = other DNA
ttaatgattcgagctttgacccatatgatatgataatgtatgttgtgagtggagcttacctccatgaccctgagttcaacttgtcctacagtctgaaggagaaggagatcaaggagacag

SEQ ID NO: 2152 - DNA, 120 bp, synthetic construct
  source 1..120: mol_type = other DNA
tccatgaccctgagttcaacttgtcctacagtctgaaggagaaggagatcaaggagacaggtagactttttgctaaaatgacttacaaaatgagagcatgccaagtgattgctgaaaatc

SEQ ID NO: 2153 - DNA, 120 bp, synthetic construct
  source 1..120: mol_type = other DNA
gtagactttttgctaaaatgacttacaaaatgagagcatgccaagtgattgctgaaaatctaatctcaaacggcattggcaaatattttaaggacaatgggatggccaaggatgaacatg

SEQ ID NO: 2154 - DNA, 120 bp, synthetic construct
  source 1..120: mol_type = other DNA
taatctcaaacggcattggcaaatattttaaggacaatgggatggccaaggatgaacatgatttgactaaggcactccacactctagctgtctcaggaatccccaaagatctcaaagaaa

SEQ ID NO: 2155 - DNA, 120 bp, synthetic construct
  source 1..120: mol_type = other DNA
atttgactaaggcactccacactctagctgtctcaggaatccccaaagatctcaaagaaagtcacagaggggggccaatcttaaaaacctactcccgaaactcagttcacacaagtacca

SEQ ID NO: 2156 - DNA, 120 bp, synthetic construct
  source 1..120: mol_type = other DNA
gtcacagaggggggccaatcttaaaaacctactcccgaaactcagttcacacaagtaccaggaacgtgagagcagcaaaagggtttatagggttccctcaagtaattcagcagggccaag

SEQ ID NO: 2157 - DNA, 120 bp, synthetic construct
  source 1..120: mol_type = other DNA
ggaacgtgagagcagcaaaagggtttatagggttccctcaagtaattcagcagggccaagacactgatcatccggagaatgtggaagcctacgagacagtcagtgcatttatcacgactg

SEQ ID NO: 2158 - DNA, 120 bp, synthetic construct
  source 1..120: mol_type = other DNA
acactgatcatccggagaatgtggaagcctacgagacagtcagtgcatttatcacgactgatctcaagaagtactgccttaattggagatatgagaccatcagcctgtttgcacagaggc

SEQ ID NO: 2159 - DNA, 120 bp, synthetic construct
  source 1..120: mol_type = other DNA
atctcaagaagtactgccttaattggagatatgagaccatcagcctgtttgcacagaggctaaatgagatttacggattaccctcattttttcagtggctgcataagaggctcgagacct

SEQ ID NO: 2160 - DNA, 120 bp, synthetic construct
  source 1..120: mol_type = other DNA
taaatgagatttacggattaccctcattttttcagtggctgcataagaggctcgagacctctgttctgtatgtaagtgatcctcattgcccccctgaccttgacgcccatatcccgttat

SEQ ID NO: 2161 - DNA, 120 bp, synthetic construct
  source 1..120: mol_type = other DNA
ctgttctgtatgtaagtgatcctcattgcccccctgaccttgacgcccatatcccgttatgcaaagtcccgaatgaccaaatcttcattaagtaccctatgggaggtatagaagggtatt

SEQ ID NO: 2162 - DNA, 120 bp, synthetic construct
  source 1..120: mol_type = other DNA
gcaaagtcccgaatgaccaaatcttcattaagtaccctatgggaggtatagaagggtattgtcagaagctgtggaccatcagcaccatcccctatttatacctggctgcttatgagagcg

SEQ ID NO: 2163 - DNA, 120 bp, synthetic construct
  source 1..120: mol_type = other DNA
gtcagaagctgtggaccatcagcaccatcccctatttatacctggctgcttatgagagcggagtaaggattgcttcgttagtgcagggggacaatcagaccatagccgtaacaaaaaggg

SEQ ID NO: 2164 - DNA, 120 bp, synthetic construct
  source 1..120: mol_type = other DNA
gagtaaggattgcttcgttagtgcagggggacaatcagaccatagccgtaacaaaaagggtacccagcacatggccttacaacctcaagaaacgggaagctgctagagtaactagagact

SEQ ID NO: 2165 - DNA, 120 bp, synthetic construct
  source 1..120: mol_type = other DNA
tacccagcacatggccttacaacctcaagaaacgggaagctgctagagtaactagagactactttgtaattcttaggcaaaggctacatgacattggtcatcacctcaaggcaaatgaga

SEQ ID NO: 2166 - DNA, 120 bp, synthetic construct
  source 1..120: mol_type = other DNA
actttgtaattcttaggcaaaggctacatgacattggtcatcacctcaaggcaaatgagacaattgtctcatcacatttttttgtctattcaaaaggaatatattatgatgggctacttg

SEQ ID NO: 2167 - DNA, 120 bp, synthetic construct
  source 1..120: mol_type = other DNA
caattgtctcatcacatttttttgtctattcaaaaggaatatattatgatgggctacttgtgtcccaatcactcaagagcatcgcaagatgtgtattctggtcagagactatagttgatg

SEQ ID NO: 2168 - DNA, 120 bp, synthetic construct
  source 1..120: mol_type = other DNA
tgtcccaatcactcaagagcatcgcaagatgtgtattctggtcagagactatagttgatgagacaagggcagcatgcagcaatattgccacaacgatggctaagagcatcgagagaggtt

SEQ ID NO: 2169 - DNA, 120 bp, synthetic construct
  source 1..120: mol_type = other DNA
agacaagggcagcatgcagcaatattgccacaacgatggctaagagcatcgagagaggttatgaccgttaccttgcatattctctgaatgtcctaaaagtgatacagcaaattctgatct

SEQ ID NO: 2170 - DNA, 120 bp, synthetic construct
  source 1..120: mol_type = other DNA
atgaccgttaccttgcatattctctgaatgtcctaaaagtgatacagcaaattctgatctcccttggcttcacaatcaattcaaccatgacccgggatgtagtcataccactcctcacaa

SEQ ID NO: 2171 - DNA, 120 bp, synthetic construct
  source 1..120: mol_type = other DNA
cccttggcttcacaatcaattcaaccatgacccgggatgtagtcataccactcctcacaaacaacgacctcttaataaggatggcactattgcccgcccctattggggggatgaattatt

SEQ ID NO: 2172 - DNA, 120 bp, synthetic construct
  source 1..120: mol_type = other DNA
acaacgacctcttaataaggatggcactattgcccgcccctattggggggatgaattatttgaatatgagcaggctgtttgtcagaaacatcggtgatccagtaacatcatcaattgctg

SEQ ID NO: 2173 - DNA, 120 bp, synthetic construct
  source 1..120: mol_type = other DNA
tgaatatgagcaggctgtttgtcagaaacatcggtgatccagtaacatcatcaattgctgatctcaagagaatgattctcgcctcgctaatgcctgaagagaccctccatcaagtaatga

SEQ ID NO: 2174 - DNA, 120 bp, synthetic construct
  source 1..120: mol_type = other DNA
atctcaagagaatgattctcgcctcgctaatgcctgaagagaccctccatcaagtaatgacacaacaaccaggagactcttcattcctagactgggctagcgacccttactcagcgaatc

SEQ ID NO: 2175 - DNA, 120 bp, synthetic construct
  source 1..120: mol_type = other DNA
cacaacaaccaggagactcttcattcctagactgggctagcgacccttactcagcgaatcttgtatgtgtccaaagcatcactagactcctcaagaacataactgcaaggtttgtcctga

SEQ ID NO: 2176 - DNA, 120 bp, synthetic construct
  source 1..120: mol_type = other DNA
ttgtatgtgtccaaagcatcactagactcctcaagaacataactgcaaggtttgtcctgatccatagtccaaacccaatgttaaaaggattattccatgatgacagcaaagaagaggacg

SEQ ID NO: 2177 - DNA, 120 bp, synthetic construct
  source 1..120: mol_type = other DNA
tccatagtccaaacccaatgttaaaaggattattccatgatgacagcaaagaagaggacgagggactggcggcgttcctcatggacaggcatattatagtacctagggcagctcatgaaa

SEQ ID NO: 2178 - DNA, 120 bp, synthetic construct
  source 1..120: mol_type = other DNA
agggactggcggcgttcctcatggacaggcatattatagtacctagggcagctcatgaaatcctggatcatagtgtcacaggggcaagagagtctatcgcaggcatgctggacaccacaa

SEQ ID NO: 2179 - DNA, 120 bp, synthetic construct
  source 1..120: mol_type = other DNA
tcctggatcatagtgtcacaggggcaagagagtctatcgcaggcatgctggacaccacaaagggcctgattcgagccagcatgaggaagggggggttaacctctcgagtgataactagat

SEQ ID NO: 2180 - DNA, 120 bp, synthetic construct
  source 1..120: mol_type = other DNA
agggcctgattcgagccagcatgaggaagggggggttaacctctcgagtgataactagattgtccaattatgactatgaacaattcagggcagggatggtgctattgacaggaagaagga

SEQ ID NO: 2181 - DNA, 120 bp, synthetic construct
  source 1..120: mol_type = other DNA
tgtccaattatgactatgaacaattcagggcagggatggtgctattgacaggaagaaggagaaatatcctcattgacaaagagtcatgttcagtgcagctggcgagagctctaagaagcc

SEQ ID NO: 2182 - DNA, 120 bp, synthetic construct
  source 1..120: mol_type = other DNA
gaaatatcctcattgacaaagagtcatgttcagtgcagctggcgagagctctaagaagccatatgtgggcgaggctagctcgaggacggcctatttacggccttgaggtccctgatgtac

SEQ ID NO: 2183 - DNA, 120 bp, synthetic construct
  source 1..120: mol_type = other DNA
atatgtgggcgaggctagctcgaggacggcctatttacggccttgaggtccctgatgtactagaatctatgcgaggccaccttattcggcgtcacgagacatgtgtcatctgcgagtgtg

SEQ ID NO: 2184 - DNA, 120 bp, synthetic construct
  source 1..120: mol_type = other DNA
tagaatctatgcgaggccaccttattcggcgtcacgagacatgtgtcatctgcgagtgtggatcagtcaattacggatggttttttgtcccctcgagttgccaactggatgatattgaca

SEQ ID NO: 2185 - DNA, 120 bp, synthetic construct
  source 1..120: mol_type = other DNA
gatcagtcaattacggatggttttttgtcccctcgagttgccaactggatgatattgacaaggaaacatcatccttgagagtcccctatattggttctaccactgatgagagaacagaca

SEQ ID NO: 2186 - DNA, 120 bp, synthetic construct
  source 1..120: mol_type = other DNA
aggaaacatcatccttgagagtcccctatattggttctaccactgatgagagaacagacatgaagcttgccttcgtaagagccccaagtcgatccttgcgatctgctgttagaatagcaa

SEQ ID NO: 2187 - DNA, 120 bp, synthetic construct
  source 1..120: mol_type = other DNA
tgaagcttgccttcgtaagagccccaagtcgatccttgcgatctgctgttagaatagcaacagtgtactcatgggcttacggtgatgatgatagctcctggaacgaagcttggttgttgg

SEQ ID NO: 2188 - DNA, 120 bp, synthetic construct
  source 1..120: mol_type = other DNA
cagtgtactcatgggcttacggtgatgatgatagctcctggaacgaagcttggttgttggcaaaacaaagggccaatgtgagcctggaggagctaagggtgatcactcccatctcaactt

SEQ ID NO: 2189 - DNA, 120 bp, synthetic construct
  source 1..120: mol_type = other DNA
caaaacaaagggccaatgtgagcctggaggagctaagggtgatcactcccatctcaacttcgactaatttagcgcataggttgagggatcgtagtactcaagtgaaatactcaggtacat

SEQ ID NO: 2190 - DNA, 120 bp, synthetic construct
  source 1..120: mol_type = other DNA
cgactaatttagcgcataggttgagggatcgtagtactcaagtgaaatactcaggtacatcccttgtccgagtggcgaggtataccacaatctccaacgacaatctttcatttgtcatat

SEQ ID NO: 2191 - DNA, 120 bp, synthetic construct
  source 1..120: mol_type = other DNA
cccttgtccgagtggcgaggtataccacaatctccaacgacaatctttcatttgtcatatcagataagaaggttgatactaactttatataccaacaaggaatgcttctaggattgggtg

SEQ ID NO: 2192 - DNA, 120 bp, synthetic construct
  source 1..120: mol_type = other DNA
cagataagaaggttgatactaactttatataccaacaaggaatgcttctaggattgggtgttttagaaacattgttccgacttgagaaaaacaccggaccatccaacacggtactacatc

SEQ ID NO: 2193 - DNA, 120 bp, synthetic construct
  source 1..120: mol_type = other DNA
ttttagaaacattgttccgacttgagaaaaacaccggaccatccaacacggtactacatcttcacgtcgaaacagattgttgcgtgatcccgatgatagatcatcccagaatacccagct

SEQ ID NO: 2194 - DNA, 120 bp, synthetic construct
  source 1..120: mol_type = other DNA
ttcacgtcgaaacagattgttgcgtgatcccgatgatagatcatcccagaatacccagctcccgcaagctagagctgagagcagagctatgtaccaacccattgatatatgataatgctc

SEQ ID NO: 2195 - DNA, 120 bp, synthetic construct
  source 1..120: mol_type = other DNA
cccgcaagctagagctgagagcagagctatgtaccaacccattgatatatgataatgctcctttaattgacagagatgcaacaaggctatacacccagagccataggaggcaccttgtgg

SEQ ID NO: 2196 - DNA, 120 bp, synthetic construct
  source 1..120: mol_type = other DNA
ctttaattgacagagatgcaacaaggctatacacccagagccataggaggcaccttgtggaatttgttacgtggtccacaccccaactatatcacattctagctaagtccacagcactat

SEQ ID NO: 2197 - DNA, 120 bp, synthetic construct
  source 1..120: mol_type = other DNA
aatttgttacgtggtccacaccccaactatatcacattctagctaagtccacagcactatctatgattgacctgataacaaaatttgagaaggaccatatgaatgaaatttcagctctta

SEQ ID NO: 2198 - DNA, 120 bp, synthetic construct
  source 1..120: mol_type = other DNA
ctatgattgacctgataacaaaatttgagaaggaccatatgaatgaaatttcagctcttataggagatgatgatattaatagtttcataactgaatttctgcttatagagccaagactgt

SEQ ID NO: 2199 - DNA, 120 bp, synthetic construct
  source 1..120: mol_type = other DNA
taggagatgatgatattaatagtttcataactgaatttctgcttatagagccaagactgttcactatctacttgggccagtgtgcggccattaattgggcatttgatgtgcattatcata

SEQ ID NO: 2200 - DNA, 120 bp, synthetic construct
  source 1..120: mol_type = other DNA
tcactatctacttgggccagtgtgcggccattaattgggcatttgatgtgcattatcatagaccatcaggaaaatatcagatgggtgagctgttgtcatcgttcctttctagaatgagca

SEQ ID NO: 2201 - DNA, 120 bp, synthetic construct
  source 1..120: mol_type = other DNA
gaccatcaggaaaatatcagatgggtgagctgttgtcatcgttcctttctagaatgagcaaaggagtgtttaaggtgcttgtcaatgctctaagccacccaaagatctacaagaaattct

SEQ ID NO: 2202 - DNA, 120 bp, synthetic construct
  source 1..120: mol_type = other DNA
aaggagtgtttaaggtgcttgtcaatgctctaagccacccaaagatctacaagaaattctggcattgtggtattatagagcctatccatggtccgtcacttgatgctcaaaacttgcaca

SEQ ID NO: 2203 - DNA, 120 bp, synthetic construct
  source 1..120: mol_type = other DNA
ggcattgtggtattatagagcctatccatggtccgtcacttgatgctcaaaacttgcacacaactgtgtgcaacatgatttacacatgctatatgacctacctagacctgttgttgaatg

SEQ ID NO: 2204 - DNA, 120 bp, synthetic construct
  source 1..120: mol_type = other DNA
caactgtgtgcaacatgatttacacatgctatatgacctacctagacctgttgttgaatgaagagttagacgagttcacatttcttttgtgtgaaagtgacgaggatgtagtaccggaca

SEQ ID NO: 2205 - DNA, 120 bp, synthetic construct
  source 1..120: mol_type = other DNA
aagagttagacgagttcacatttcttttgtgtgaaagtgacgaggatgtagtaccggacagatttgacaacatccaggcaaaacacttgtgtgttctagcagatttgtactgtcaaccag

SEQ ID NO: 2206 - DNA, 120 bp, synthetic construct
  source 1..120: mol_type = other DNA
gatttgacaacatccaggcaaaacacttgtgtgttctagcagatttgtactgtcaaccagggacctgcccaccaattcgaggtctaagaccggtggagaaatgtgcagttctaaccaacc

SEQ ID NO: 2207 - DNA, 120 bp, synthetic construct
  source 1..120: mol_type = other DNA
ggacctgcccaccaattcgaggtctaagaccggtggagaaatgtgcagttctaaccaaccatatcaaggcagaggctagattatctccagcaggatcttcgtggaacataaacccaatta

SEQ ID NO: 2208 - DNA, 120 bp, synthetic construct
  source 1..120: mol_type = other DNA
atatcaaggcagaggctagattatctccagcaggatcttcgtggaacataaacccaattattgtagaccactactcatgctccctgacttatctccggcgaggctcgatcaaacagataa

SEQ ID NO: 2209 - DNA, 120 bp, synthetic construct
  source 1..120: mol_type = other DNA
ttgtagaccactactcatgctccctgacttatctccggcgaggctcgatcaaacagataagattgagagttgatccaggattcatcttcgacgccctcgctgaggcaaatgtcagtcagc

SEQ ID NO: 2210 - DNA, 120 bp, synthetic construct
  source 1..120: mol_type = other DNA
gattgagagttgatccaggattcatcttcgacgccctcgctgaggcaaatgtcagtcagccaaaaataggcagcaacaacatctcaaatatgagtatcaaggatttcagacccccacacg

SEQ ID NO: 2211 - DNA, 120 bp, synthetic construct
  source 1..120: mol_type = other DNA
caaaaataggcagcaacaacatctcaaatatgagtatcaaggatttcagacccccacacgatgatgttgccaaattgctcaaagatatcaacacaagcaagcacaaccttcctatttcag

SEQ ID NO: 2212 - DNA, 120 bp, synthetic construct
  source 1..120: mol_type = other DNA
atgatgttgccaaattgctcaaagatatcaacacaagcaagcacaaccttcctatttcagggggcagtctcgccaattatgaaatccatgctttccgcagaatcgggttgaactcatctg

SEQ ID NO: 2213 - DNA, 120 bp, synthetic construct
  source 1..120: mol_type = other DNA
ggggcagtctcgccaattatgaaatccatgctttccgcagaatcgggttgaactcatctgcttgctacaaagctgttgagatatcaacattaattaggagatgccttgagccaggggaag

SEQ ID NO: 2214 - DNA, 120 bp, synthetic construct
  source 1..120: mol_type = other DNA
cttgctacaaagctgttgagatatcaacattaattaggagatgccttgagccaggggaagacggcttgttcttgggtgagggatcgggttctatgttggtcacttataaggagatactta

SEQ ID NO: 2215 - DNA, 120 bp, synthetic construct
  source 1..120: mol_type = other DNA
acggcttgttcttgggtgagggatcgggttctatgttggtcacttataaggagatacttaaactaaacaagtgcttctataatagtggggtttccgccaattctagatctggtcaaaggg

SEQ ID NO: 2216 - DNA, 120 bp, synthetic construct
  source 1..120: mol_type = other DNA
aactaaacaagtgcttctataatagtggggtttccgccaattctagatctggtcaaagggaattagcaccctacccctccgaagtcggccttgtcgaacacagaatgggagtgggcaata

SEQ ID NO: 2217 - DNA, 120 bp, synthetic construct
  source 1..120: mol_type = other DNA
aattagcaccctacccctccgaagtcggccttgtcgaacacagaatgggagtgggcaatattgtcaaggtgctctttaacgggaggcccgaagtcacgtggataggcagtgtagattgct

SEQ ID NO: 2218 - DNA, 120 bp, synthetic construct
  source 1..120: mol_type = other DNA
ttgtcaaggtgctctttaacgggaggcccgaagtcacgtggataggcagtgtagattgcttcaatttcatagtcagtaatatccctacctctagtgtggggtttatccattcagatatag

SEQ ID NO: 2219 - DNA, 120 bp, synthetic construct
  source 1..120: mol_type = other DNA
tcaatttcatagtcagtaatatccctacctctagtgtggggtttatccattcagatatagagaccttacctaacaaagatactatagagaagctagaggaattggcagccatcttgtcgc

SEQ ID NO: 2220 - DNA, 120 bp, synthetic construct
  source 1..120: mol_type = other DNA
agaccttacctaacaaagatactatagagaagctagaggaattggcagccatcttgtcgctggctctgctcctgggcaaaataggatcaatattggtgattaagcttatgcctttcagcg

SEQ ID NO: 2221 - DNA, 120 bp, synthetic construct
  source 1..120: mol_type = other DNA
tggctctgctcctgggcaaaataggatcaatattggtgattaagcttatgcctttcagcggggattttgttcaaggatttataagttatgtagggtctcattatagggaagtgaaccttg

SEQ ID NO: 2222 - DNA, 120 bp, synthetic construct
  source 1..120: mol_type = other DNA
gggattttgttcaaggatttataagttatgtagggtctcattatagggaagtgaaccttgtataccctagatacagcaacttcatatctactgaatcttatttggttatggcagatctca

SEQ ID NO: 2223 - DNA, 120 bp, synthetic construct
  source 1..120: mol_type = other DNA
tataccctagatacagcaacttcatatctactgaatcttatttggttatggcagatctcaaggctaaccggctaatgaatcctgaaaagattaagcagcagataattgaatcatctgtgc

SEQ ID NO: 2224 - DNA, 120 bp, synthetic construct
  source 1..120: mol_type = other DNA
aggctaaccggctaatgaatcctgaaaagattaagcagcagataattgaatcatctgtgcggacttcacctggacttataggtcacatcctatccattaagcaactaagctgcatacaag

SEQ ID NO: 2225 - DNA, 120 bp, synthetic construct
  source 1..120: mol_type = other DNA
ggacttcacctggacttataggtcacatcctatccattaagcaactaagctgcatacaagcaattgtgggaggcgcagttattagaggtgatatcaaccctactctgaaaaaacttacac

SEQ ID NO: 2226 - DNA, 120 bp, synthetic construct
  source 1..120: mol_type = other DNA
caattgtgggaggcgcagttattagaggtgatatcaaccctactctgaaaaaacttacacctatagagcaggtgctgatcaattgcgggttggcgattaacggacccaaactgtgcaaag

SEQ ID NO: 2227 - DNA, 120 bp, synthetic construct
  source 1..120: mol_type = other DNA
ctatagagcaggtgctgatcaattgcgggttggcgattaacggacccaaactgtgcaaagaattgatccaccatgatgttgcctcagggcaagatggattgcttaattctatactcatcc

SEQ ID NO: 2228 - DNA, 120 bp, synthetic construct
  source 1..120: mol_type = other DNA
aattgatccaccatgatgttgcctcagggcaagatggattgcttaattctatactcatcctctacagggaattggcaagattcaaggacaaccaaagaagtcaacaggggatgttccacg

SEQ ID NO: 2229 - DNA, 120 bp, synthetic construct
  source 1..120: mol_type = other DNA
tctacagggaattggcaagattcaaggacaaccaaagaagtcaacaggggatgttccacgcttaccccgtattggtaagtagcagacaacgagaacttatatctaggatcgcccgcaaat

SEQ ID NO: 2230 - DNA, 120 bp, synthetic construct
  source 1..120: mol_type = other DNA
cttaccccgtattggtaagtagcagacaacgagaacttatatctaggatcgcccgcaaattctgggggcacattcttctttactccgggaacagaaagttgataaataagtttatccaga

SEQ ID NO: 2231 - DNA, 120 bp, synthetic construct
  source 1..120: mol_type = other DNA
tctgggggcacattcttctttactccgggaacagaaagttgataaataagtttatccagaatctcaagtccggttatctgatactggacttacaccagaatatcttcgttaagaatctat

SEQ ID NO: 2232 - DNA, 120 bp, synthetic construct
  source 1..120: mol_type = other DNA
atctcaagtccggttatctgatactggacttacaccagaatatcttcgttaagaatctatccaagtcagagaaacagattatcctgtcggggggtctgaaacgtgagtgggtctttaagg

SEQ ID NO: 2233 - DNA, 120 bp, synthetic construct
  source 1..120: mol_type = other DNA
ccaagtcagagaaacagattatcctgtcggggggtctgaaacgtgagtgggtctttaaggtaacagtcaaggagaccaaagaatggtataagttactcggatacagtgctctgattaagg

SEQ ID NO: 2234 - DNA, 120 bp, synthetic construct
  source 1..120: mol_type = other DNA
taacagtcaaggagaccaaagaatggtataagttactcggatacagtgctctgattaaggactagatggttgaactccggaaccctgaaccttcccaaggtagttgggcattatttgcaa

SEQ ID NO: 2235 - DNA, 120 bp, synthetic construct
  source 1..120: mol_type = other DNA
ttaaggactagatggttgaactccggaaccctgaaccttcccaaggtagttgggcattatttgcaatatattaaagaaaactttgaaaatacgaagtttctattcccagctttgtctggt

SEQ ID NO: 2236 - DNA, 120 bp, synthetic construct
  source 1..120: mol_type = other DNA
taaaatacaattatatctttttcgatattaataaatccgtgtctcccgggttttttatctctttcagtatgtgaatagataggtattttatctctattcatcatcgaatttaagagatcc

SEQ ID NO: 2237 - DNA, 120 bp, synthetic construct
  source 1..120: mol_type = other DNA
ctttcagtatgtgaatagataggtattttatctctattcatcatcgaatttaagagatccgataaacattgtttgtattctccagatgtcagcatctgatacaacaatatatgtgcacat

SEQ ID NO: 2238 - DNA, 120 bp, synthetic construct
  source 1..120: mol_type = other DNA
gataaacattgtttgtattctccagatgtcagcatctgatacaacaatatatgtgcacataaacctctggcacttatttcatgtaccttccccttatcactaaggagaatagtatttgag

SEQ ID NO: 2239 - DNA, 120 bp, synthetic construct
  source 1..120: mol_type = other DNA
aaacctctggcacttatttcatgtaccttccccttatcactaaggagaatagtatttgagaaatatgtatacatgatattatcatgtattagatatacagaatttgtaacactctcgaaa

SEQ ID NO: 2240 - DNA, 120 bp, synthetic construct
  source 1..120: mol_type = other DNA
aaatatgtatacatgatattatcatgtattagatatacagaatttgtaacactctcgaaatcacacgatgtgtcggcgttaagatctaatatatcactcgataacacattttcatctaga

SEQ ID NO: 2241 - DNA, 120 bp, synthetic construct
  source 1..120: mol_type = other DNA
tcacacgatgtgtcggcgttaagatctaatatatcactcgataacacattttcatctagatacactagacattttttaaagctaaaatagtctttagtagtaacagtaactatgcgatta

SEQ ID NO: 2242 - DNA, 120 bp, synthetic construct
  source 1..120: mol_type = other DNA
tacactagacattttttaaagctaaaatagtctttagtagtaacagtaactatgcgattattttcatcgatgatacatttcatcggcatattattacgcgtaccatcaaagactatacca

SEQ ID NO: 2243 - DNA, 120 bp, synthetic construct
  source 1..120: mol_type = other DNA
ttttcatcgatgatacatttcatcggcatattattacgcgtaccatcaaagactataccatgtgtatatctaacgtattctagcatagttgccatacgtacattaaacttttcaggatct

SEQ ID NO: 2244 - DNA, 120 bp, synthetic construct
  source 1..120: mol_type = other DNA
tgtgtatatctaacgtattctagcatagttgccatacgtacattaaacttttcaggatctttggatagatcttccaatctatctatttgagaaaacatttttatcatgttcaatagttga

SEQ ID NO: 2245 - DNA, 120 bp, synthetic construct
  source 1..120: mol_type = other DNA
ttggatagatcttccaatctatctatttgagaaaacatttttatcatgttcaatagttgaaacgtcggatccactatatagatattatctataaagattttaggaactatgttcatggta

SEQ ID NO: 2246 - DNA, 120 bp, synthetic construct
  source 1..120: mol_type = other DNA
aacgtcggatccactatatagatattatctataaagattttaggaactatgttcatggtatcctggcgaatattaaaactatcaatgatatgattatcgttttcatcttttatcaccata

SEQ ID NO: 2247 - DNA, 120 bp, synthetic construct
  source 1..120: mol_type = other DNA
tcctggcgaatattaaaactatcaatgatatgattatcgttttcatcttttatcaccatatagtttctaagatatgggattttacttaatataatattatttcccgtaataaattttatt

SEQ ID NO: 2248 - DNA, 120 bp, synthetic construct
  source 1..120: mol_type = other DNA
tagtttctaagatatgggattttacttaatataatattatttcccgtaataaattttattagaaatgccaaatctataagaaaagtcctagaattagtctgaagaatatctatatcaccg

SEQ ID NO: 2249 - DNA, 120 bp, synthetic construct
  source 1..120: mol_type = other DNA
agaaatgccaaatctataagaaaagtcctagaattagtctgaagaatatctatatcaccgtaccgtatatttggattaattagatatagagaatatgatccgtaacatatacaactttta

SEQ ID NO: 2250 - DNA, 120 bp, synthetic construct
  source 1..120: mol_type = other DNA
taccgtatatttggattaattagatatagagaatatgatccgtaacatatacaacttttattatgacgtctaagatattcttccatcaacttattaacatttttgactagggaagataca

SEQ ID NO: 2251 - DNA, 120 bp, synthetic construct
  source 1..120: mol_type = other DNA
ttatgacgtctaagatattcttccatcaacttattaacatttttgactagggaagatacattatgacgtcccattacttttgccttgtctattacagcgacgttcatagaatttagcata

SEQ ID NO: 2252 - DNA, 120 bp, synthetic construct
  source 1..120: mol_type = other DNA
ttatgacgtcccattacttttgccttgtctattacagcgacgttcatagaatttagcatatctcttgccaattcttccattgatgttacattataagaaattttagatgaaattacattt

SEQ ID NO: 2253 - DNA, 120 bp, synthetic construct
  source 1..120: mol_type = other DNA
tctcttgccaattcttccattgatgttacattataagaaattttagatgaaattacatttggagctttaatagtaagaactcctaatatatccgtgtatgtggtcactaatacagattgt

SEQ ID NO: 2254 - DNA, 120 bp, synthetic construct
  source 1..120: mol_type = other DNA
ggagctttaatagtaagaactcctaatatatccgtgtatgtggtcactaatacagattgtagttctataatcgtaaataatttacctatattatatgtttgagtttgtttagaaaagtag

SEQ ID NO: 2255 - DNA, 120 bp, synthetic construct
  source 1..120: mol_type = other DNA
agttctataatcgtaaataatttacctatattatatgtttgagtttgtttagaaaagtagctaagtatacgatcttttatttctgatgccgatgtatcaacatcgaaaaaaaatcttttt

SEQ ID NO: 2256 - DNA, 120 bp, synthetic construct
  source 1..120: mol_type = other DNA
ctaagtatacgatcttttatttctgatgccgatgtatcaacatcgaaaaaaaatctttttttattcttttttactaacgatacgaatatgtctttgttaaaaacagttattttctgaata

SEQ ID NO: 2257 - DNA, 120 bp, synthetic construct
  source 1..120: mol_type = other DNA
ttattcttttttactaacgatacgaatatgtctttgttaaaaacagttattttctgaatatttctagcttgtaattttaacatatgatattcgttcacactaggtactctgcctaaatag

SEQ ID NO: 2258 - DNA, 120 bp, synthetic construct
  source 1..120: mol_type = other DNA
tttctagcttgtaattttaacatatgatattcgttcacactaggtactctgcctaaataggtttctataatctttaatgtaatattaggaagagtattctgatcaggattcctattcatt

SEQ ID NO: 2259 - DNA, 120 bp, synthetic construct
  source 1..120: mol_type = other DNA
gtttctataatctttaatgtaatattaggaagagtattctgatcaggattcctattcattttgaggatttaaaactctgattattgtctaatatggtctcaacacaaactttttcacaga

SEQ ID NO: 2260 - DNA, 120 bp, synthetic construct
  source 1..120: mol_type = other DNA
ttgaggatttaaaactctgattattgtctaatatggtctcaacacaaactttttcacagagtgatagagtttttgataactcgtttttcttaagaaatataaaactactgtctccagagc

SEQ ID NO: 2261 - DNA, 120 bp, synthetic construct
  source 1..120: mol_type = other DNA
gtgatagagtttttgataactcgtttttcttaagaaatataaaactactgtctccagagctcgctctatcttttattttatctaattcgatacaaactcctgatactggttcagaaagta

SEQ ID NO: 2262 - DNA, 120 bp, synthetic construct
  source 1..120: mol_type = other DNA
tcgctctatcttttattttatctaattcgatacaaactcctgatactggttcagaaagtaattcattaattttcagtcctttatagaagatatttaatatagataatacaaaatcttcag

SEQ ID NO: 2263 - DNA, 120 bp, synthetic construct
  source 1..120: mol_type = other DNA
attcattaattttcagtcctttatagaagatatttaatatagataatacaaaatcttcagttcttgatatcgatctgattgatcctagaactagatatattaataacgtgctcattaggc

SEQ ID NO: 2264 - DNA, 120 bp, synthetic construct
  source 1..120: mol_type = other DNA
ttcttgatatcgatctgattgatcctagaactagatatattaataacgtgctcattaggcagtttatggcagcttgataattagatatagtatattccagttcatatttattagataccg

SEQ ID NO: 2265 - DNA, 120 bp, synthetic construct
  source 1..120: mol_type = other DNA
agtttatggcagcttgataattagatatagtatattccagttcatatttattagataccgcattgcccagattttgatattctatgaattcctctgaaaataaatccaaaataactagac

SEQ ID NO: 2266 - DNA, 120 bp, synthetic construct
  source 1..120: mol_type = other DNA
cattgcccagattttgatattctatgaattcctctgaaaataaatccaaaataactagacattctattttttgtggattagtgtactctcttccctctatcatgttcactactggtgtcc

SEQ ID NO: 2267 - DNA, 120 bp, synthetic construct
  source 1..120: mol_type = other DNA
attctattttttgtggattagtgtactctcttccctctatcatgttcactactggtgtccacaatgataaatatctagagggaatataatatagtccatatgatgccaatctagcaatgt

SEQ ID NO: 2268 - DNA, 120 bp, synthetic construct
  source 1..120: mol_type = other DNA
acaatgataaatatctagagggaatataatatagtccatatgatgccaatctagcaatgtcgaataactgtaattttattcttcgctcttcattatgaattgaatcttgaggtataaacc

SEQ ID NO: 2269 - DNA, 120 bp, synthetic construct
  source 1..120: mol_type = other DNA
cgaataactgtaattttattcttcgctcttcattatgaattgaatcttgaggtataaacctaacacaaattatatcattagacttttcgtatgtaatgtctttcatgttataagttttta

SEQ ID NO: 2270 - DNA, 120 bp, synthetic construct
  source 1..120: mol_type = other DNA
taacacaaattatatcattagacttttcgtatgtaatgtctttcatgttataagtttttaatcctggaatagaatctattttaatgaggcttttaaacgcagcgttctccaacgagtcaa

SEQ ID NO: 2271 - DNA, 120 bp, synthetic construct
  source 1..120: mol_type = other DNA
atcctggaatagaatctattttaatgaggcttttaaacgcagcgttctccaacgagtcaaagcataatactctgttggttttcttatattcaatattacgattttcttctttgaatggaa

SEQ ID NO: 2272 - DNA, 120 bp, synthetic construct
  source 1..120: mol_type = other DNA
agcataatactctgttggttttcttatattcaatattacgattttcttctttgaatggaataggtttttgaattagtttataattacaacataatagataaggaagtgtgtaaatagtac

SEQ ID NO: 2273 - DNA, 120 bp, synthetic construct
  source 1..120: mol_type = other DNA
taggtttttgaattagtttataattacaacataatagataaggaagtgtgtaaatagtacgcggaaaaaacataatagctcccctgttttcatccatggttttaagtaaatgatcactgg

SEQ ID NO: 2274 - DNA, 120 bp, synthetic construct
  source 1..120: mol_type = other DNA
gcggaaaaaacataatagctcccctgttttcatccatggttttaagtaaatgatcactggcttctttagtcaatggatattcgaacattaaccgtttcatcatcattggacagaatccat

SEQ ID NO: 2275 - DNA, 120 bp, synthetic construct
  source 1..120: mol_type = other DNA
cttctttagtcaatggatattcgaacattaaccgtttcatcatcattggacagaatccatatttcttaatgtaaagagtgatcaaatcattgtgtttattgtaccatcttgttgtaaatg

SEQ ID NO: 2276 - DNA, 120 bp, synthetic construct
  source 1..120: mol_type = other DNA
atttcttaatgtaaagagtgatcaaatcattgtgtttattgtaccatcttgttgtaaatgtgtattcggttatcggatctgctcctttttctattaaagtatcgatatcgatctcgtcta

SEQ ID NO: 2277 - DNA, 120 bp, synthetic construct
  source 1..120: mol_type = other DNA
tgtattcggttatcggatctgctcctttttctattaaagtatcgatatcgatctcgtctaagaattcaactatatcgacatatttcatttgtatacacataaccattactaacgtagaat

SEQ ID NO: 2278 - DNA, 120 bp, synthetic construct
  source 1..120: mol_type = other DNA
agaattcaactatatcgacatatttcatttgtatacacataaccattactaacgtagaatgtataggaagagatgtaacgggaacagggtttgttgattcgcaaactattctaatacata

SEQ ID NO: 2279 - DNA, 120 bp, synthetic construct
  source 1..120: mol_type = other DNA
gtataggaagagatgtaacgggaacagggtttgttgattcgcaaactattctaatacataattcttctgttaatacgtcttgcacgtaatctattatagatgccaagatatctatataat

SEQ ID NO: 2280 - DNA, 120 bp, synthetic construct
  source 1..120: mol_type = other DNA
attcttctgttaatacgtcttgcacgtaatctattatagatgccaagatatctatataattattttgtaagatgatgttaacaatgtgatctatataagtagtgtaataattcatgtatt

SEQ ID NO: 2281 - DNA, 120 bp, synthetic construct
  source 1..120: mol_type = other DNA
tattttgtaagatgatgttaacaatgtgatctatataagtagtgtaataattcatgtatttcgatatatgttccaactctgtctttgtgatgtctagtttcgtaatatctatagcgtcct

SEQ ID NO: 2282 - DNA, 120 bp, synthetic construct
  source 1..120: mol_type = other DNA
tcgatatatgttccaactctgtctttgtgatgtctagtttcgtaatatctatagcgtcctcaaaaaatatattcgcatatattcccaagtcttcagttctatcttctaaaaaatcttcaa

SEQ ID NO: 2283 - DNA, 120 bp, synthetic construct
  source 1..120: mol_type = other DNA
caaaaaatatattcgcatatattcccaagtcttcagttctatcttctaaaaaatcttcaacgtatggaatataataatctattttacctcttctgatgtcattaatgatatagtttttga

SEQ ID NO: 2284 - DNA, 120 bp, synthetic construct
  source 1..120: mol_type = other DNA
cgtatggaatataataatctattttacctcttctgatgtcattaatgatatagtttttgacactattttccgtcaattgattcttattcactatgtctaaaaaccggatagcgtccctag

SEQ ID NO: 2285 - DNA, 120 bp, synthetic construct
  source 1..120: mol_type = other DNA
cactattttccgtcaattgattcttattcactatgtctaaaaaccggatagcgtccctaggacgaactactgccattaatatctctattatagcttctggacataaatcatctattatac

SEQ ID NO: 2286 - DNA, 120 bp, synthetic construct
  source 1..120: mol_type = other DNA
gacgaactactgccattaatatctctattatagcttctggacataaatcatctattataccagaattaatgggaactattccgtatctatctaacatagttttaagaaagtcagaatcta

SEQ ID NO: 2287 - DNA, 120 bp, synthetic construct
  source 1..120: mol_type = other DNA
cagaattaatgggaactattccgtatctatctaacatagttttaagaaagtcagaatctaagacctgatgttcatatattggttcatacatgaaatgatctctattgatgatagtgacta

SEQ ID NO: 2288 - DNA, 120 bp, synthetic construct
  source 1..120: mol_type = other DNA
agacctgatgttcatatattggttcatacatgaaatgatctctattgatgatagtgactatttcattctctgaaaattggtaactcattctatacacgctttccttgttgataaaggata

SEQ ID NO: 2289 - DNA, 120 bp, synthetic construct
  source 1..120: mol_type = other DNA
tttcattctctgaaaattggtaactcattctatacacgctttccttgttgataaaggatagtatatactcaatggaatttgtaccaacaaactgttctcttatgaatcgtatatcatcat

SEQ ID NO: 2290 - DNA, 120 bp, synthetic construct
  source 1..120: mol_type = other DNA
gtatatactcaatggaatttgtaccaacaaactgttctcttatgaatcgtatatcatcatctgaaatgatcatgtaaggcatacatttaacaataagagacttgtctcctgttatcaata

SEQ ID NO: 2291 - DNA, 120 bp, synthetic construct
  source 1..120: mol_type = other DNA
ctgaaatgatcatgtaaggcatacatttaacaataagagacttgtctcctgttatcaatatactattcttgtgataatttatgtgtgcggcaaatttgtccacgttctttaattttgtta

SEQ ID NO: 2292 - DNA, 120 bp, synthetic construct
  source 1..120: mol_type = other DNA
tactattcttgtgataatttatgtgtgcggcaaatttgtccacgttctttaattttgttatagtagatatcaaatccaatggagatacagttcttggcttaaacagatatagtttttctg

SEQ ID NO: 2293 - DNA, 120 bp, synthetic construct
  source 1..120: mol_type = other DNA
tagtagatatcaaatccaatggagatacagttcttggcttaaacagatatagtttttctggaacgaattctacaacattattataaaggactttgggtatataagtgggatgaaatccta

SEQ ID NO: 2294 - DNA, 120 bp, synthetic construct
  source 1..120: mol_type = other DNA
gaacgaattctacaacattattataaaggactttgggtatataagtgggatgaaatcctattttaattaatgcgatagccttgtcctcgtgcagatatccaaacgcttttgtgatagtat

SEQ ID NO: 2295 - DNA, 120 bp, synthetic construct
  source 1..120: mol_type = other DNA
ttttaattaatgcgatagccttgtcctcgtgcagatatccaaacgcttttgtgatagtatggcattcattgtctagaaacgctctacgaatatctgtaacagatatcatctttagagaat

SEQ ID NO: 2296 - DNA, 120 bp, synthetic construct
  source 1..120: mol_type = other DNA
ggcattcattgtctagaaacgctctacgaatatctgtaacagatatcatctttagagaatactagtcgcgttaatagtactaaaatttgtattttttaatctatctcaataaaaaattaa

SEQ ID NO: 2297 - DNA, 120 bp, synthetic construct
  source 1..120: mol_type = other DNA
actagtcgcgttaatagtactaaaatttgtattttttaatctatctcaataaaaaattaatatgtatgattcaatgtataactaaactactaactgttattgataactagaatcagaatc

SEQ ID NO: 2298 - DNA, 120 bp, synthetic construct
  source 1..120: mol_type = other DNA
tatgtatgattcaatgtataactaaactactaactgttattgataactagaatcagaatctaatgatgacataactaagaagtttatctacagccaatttagctgcattatttttagcat

SEQ ID NO: 2299 - DNA, 120 bp, synthetic construct
  source 1..120: mol_type = other DNA
taatgatgacataactaagaagtttatctacagccaatttagctgcattatttttagcatctcgtttagattttccatctgccttatcgaatactcttccgtcaatgtctacacaggcat

SEQ ID NO: 2300 - DNA, 120 bp, synthetic construct
  source 1..120: mol_type = other DNA
ctcgtttagattttccatctgccttatcgaatactcttccgtcaatgtctacacaggcataaaatgtaggagagttactaggccccactgattcaatacgaaaagaccaatctctcctag

SEQ ID NO: 2301 - DNA, 120 bp, synthetic construct
  source 1..120: mol_type = other DNA
aaaatgtaggagagttactaggccccactgattcaatacgaaaagaccaatctctcctagttatttgacagtactcattaataacggtgacagggttaacacctttccaataaataattt

SEQ ID NO: 2302 - DNA, 120 bp, synthetic construct
  source 1..120: mol_type = other DNA
ttatttgacagtactcattaataacggtgacagggttaacacctttccaataaataatttttttaaccggaataacatcatcaaaagacttatgatcctctctcattgatttttcgcggg

SEQ ID NO: 2303 - DNA, 120 bp, synthetic construct
  source 1..120: mol_type = other DNA
ttttaaccggaataacatcatcaaaagacttatgatcctctctcattgatttttcgcgggatacatcatctattatagcatcagcatcagaatctgtaggccgtgtatcagcatccattg

SEQ ID NO: 2304 - DNA, 120 bp, synthetic construct
  source 1..120: mol_type = other DNA
atacatcatctattatagcatcagcatcagaatctgtaggccgtgtatcagcatccattgtcgtagaccaacgaggaggagtatcgttggagctgtaaaccatagcactacgttgaagat

SEQ ID NO: 2305 - DNA, 120 bp, synthetic construct
  source 1..120: mol_type = other DNA
tcgtagaccaacgaggaggagtatcgttggagctgtaaaccatagcactacgttgaagatcatacagagctttattaacttctcgcttctccatattaagttgtttagttagttgtacag

SEQ ID NO: 2306 - DNA, 120 bp, synthetic construct
  source 1..120: mol_type = other DNA
catacagagctttattaacttctcgcttctccatattaagttgtttagttagttgtacagcagtagctccttagtccaatgtttttaataaccgcacacaatctctgtgtcagaacgctc

SEQ ID NO: 2307 - DNA, 120 bp, synthetic construct
  source 1..120: mol_type = other DNA
cagtagctccttagtccaatgtttttaataaccgcacacaatctctgtgtcagaacgctcgtcaatatagatcttagaaatttttttagagagaactaacgcaactagcaataaaactga

SEQ ID NO: 2308 - DNA, 120 bp, synthetic construct
  source 1..120: mol_type = other DNA
gtcaatatagatcttagaaatttttttagagagaactaacgcaactagcaataaaactgatcttattttatcattttttttattcatcatcctctggtggttcgtcgttcctatcgaatg

SEQ ID NO: 2309 - DNA, 120 bp, synthetic construct
  source 1..120: mol_type = other DNA
tcttattttatcattttttttattcatcatcctctggtggttcgtcgttcctatcgaatgtagctctgattaacccgtcatctataggtgatgctggttctggagattctggaggagatg

SEQ ID NO: 2310 - DNA, 120 bp, synthetic construct
  source 1..120: mol_type = other DNA
tagctctgattaacccgtcatctataggtgatgctggttctggagattctggaggagatggattattatctggaagaatctctgttatttccttgttttcatgtatcgattgcgttgtaa

SEQ ID NO: 2311 - DNA, 120 bp, synthetic construct
  source 1..120: mol_type = other DNA
gattattatctggaagaatctctgttatttccttgttttcatgtatcgattgcgttgtaacattaagattgcgaaatgctctaaatttgggaggcttaaagtgttgtttacaatctctac

SEQ ID NO: 2312 - DNA, 120 bp, synthetic construct
  source 1..120: mol_type = other DNA
cattaagattgcgaaatgctctaaatttgggaggcttaaagtgttgtttacaatctctacacgcgtgtctaactaatggaggttcatcagcggctctagtttgaatcatcatcggtgtag

SEQ ID NO: 2313 - DNA, 120 bp, synthetic construct
  source 1..120: mol_type = other DNA
acgcgtgtctaactaatggaggttcatcagcggctctagtttgaatcatcatcggtgtagtattcctacttttacagttaggacacggtgtattgtatttctcgtcgagaacgttaaaat

SEQ ID NO: 2314 - DNA, 120 bp, synthetic construct
  source 1..120: mol_type = other DNA
tattcctacttttacagttaggacacggtgtattgtatttctcgtcgagaacgttaaaataatcgttgtaactcacatcctttattttatctatattgtattctactcctttcttaatgc

SEQ ID NO: 2315 - DNA, 120 bp, synthetic construct
  source 1..120: mol_type = other DNA
aatcgttgtaactcacatcctttattttatctatattgtattctactcctttcttaatgcattttataccgaacaagagatagcgaaggaattctttttcggtaccgctagtacccttaa

SEQ ID NO: 2316 - DNA, 120 bp, synthetic construct
  source 1..120: mol_type = other DNA
attttataccgaacaagagatagcgaaggaattctttttcggtaccgctagtacccttaatcatatcacatagtgttttatattctaaatgtgtggcaatggacggtttatttctatacg

SEQ ID NO: 2317 - DNA, 120 bp, synthetic construct
  source 1..120: mol_type = other DNA
tcatatcacatagtgttttatattctaaatgtgtggcaatggacggtttatttctatacgatagtttgtttttggaatcctttgagtattctataccaatattattctttgattcgaatt

SEQ ID NO: 2318 - DNA, 120 bp, synthetic construct
  source 1..120: mol_type = other DNA
atagtttgtttttggaatcctttgagtattctataccaatattattctttgattcgaatttagtttcttcgatattagattttgtattacctatattcttgatgtagtactttgatgatt

SEQ ID NO: 2319 - DNA, 120 bp, synthetic construct
  source 1..120: mol_type = other DNA
tagtttcttcgatattagattttgtattacctatattcttgatgtagtactttgatgatttttccatggcccattctattaagttttccaagttggcatcatccacatattgtgatagta

SEQ ID NO: 2320 - DNA, 120 bp, synthetic construct
  source 1..120: mol_type = other DNA
tttccatggcccattctattaagttttccaagttggcatcatccacatattgtgatagtaattctcggatatcagtagtgactaccgccattgatatttgttcatttgatgagtaactac

SEQ ID NO: 2321 - DNA, 120 bp, synthetic construct
  source 1..120: mol_type = other DNA
taagttttccaagttggcatcatccacatattgtgatagtaattctcggatatcagtagtgactaccgccattgatatttgttcatttgatgagtaactactaatgtatacattttccat

SEQ ID NO: 2322 - DNA, 120 bp, synthetic construct
  source 1..120: mol_type = other DNA
taatattccaactactttaccatctagtaaagcaacctgtagctctctacccttgatatattgctcaactaaaaccttattaccaaattgaaatttataatccttaaatagaaatttatc

SEQ ID NO: 2323 - DNA, 120 bp, synthetic construct
  source 1..120: mol_type = other DNA
ttgctcaactaaaaccttattaccaaattgaaatttataatccttaaatagaaatttatcttctaaatgtacaatttttacacctatacttgacccctgctgtagtggctttataacata

SEQ ID NO: 2324 - DNA, 120 bp, synthetic construct
  source 1..120: mol_type = other DNA
ttctaaatgtacaatttttacacctatacttgacccctgctgtagtggctttataacatatggtcttaaaataggatcatttattacattatcattactattgatagttatactggcagg

SEQ ID NO: 2325 - DNA, 120 bp, synthetic construct
  source 1..120: mol_type = other DNA
tggtcttaaaataggatcatttattacattatcattactattgatagttatactggcaggagttttaatcttatagcattgtaatatagttttagcaatttgtttatcaaatgcagcagc

SEQ ID NO: 2326 - DNA, 120 bp, synthetic construct
  source 1..120: mol_type = other DNA
agttttaatcttatagcattgtaatatagttttagcaatttgtttatcaaatgcagcagcagaagtttttacaccagaatgagtatatggtatattcataatatttaataaaccaggaat

SEQ ID NO: 2327 - DNA, 120 bp, synthetic construct
  source 1..120: mol_type = other DNA
agaagtttttacaccagaatgagtatatggtatattcataatatttaataaaccaggaatacatccatcctctccatatgtaccaactagacaattaaatactgtatatggtggtgtaat

SEQ ID NO: 2328 - DNA, 120 bp, synthetic construct
  source 1..120: mol_type = other DNA
acatccatcctctccatatgtaccaactagacaattaaatactgtatatggtggtgtaatttcagatagtttaactgcaatatcttgcccaacatctatacgagtcacctgatatccatt

SEQ ID NO: 2329 - DNA, 120 bp, synthetic construct
  source 1..120: mol_type = other DNA
ttcagatagtttaactgcaatatcttgcccaacatctatacgagtcacctgatatccattagagataagagcagcttgtacattatcattagacatcaatgatacttctctttctgctga

SEQ ID NO: 2330 - DNA, 120 bp, synthetic construct
  source 1..120: mol_type = other DNA
agagataagagcagcttgtacattatcattagacatcaatgatacttctctttctgctgacataccaccatataagattactacatgctttttgcctgaactagttatactttcaacaac

SEQ ID NO: 2331 - DNA, 120 bp, synthetic construct
  source 1..120: mol_type = other DNA
cataccaccatataagattactacatgctttttgcctgaactagttatactttcaacaacagaattgcgtctttgaacactataggctttttttaccaacaattttaatctcccattcta

SEQ ID NO: 2332 - DNA, 120 bp, synthetic construct
  source 1..120: mol_type = other DNA
agaattgcgtctttgaacactataggctttttttaccaacaattttaatctcccattctaatgttataccagtatggtcaaaaacatttttacgaatcaactcccctagattttcaatat

SEQ ID NO: 2333 - DNA, 120 bp, synthetic construct
  source 1..120: mol_type = other DNA
atgttataccagtatggtcaaaaacatttttacgaatcaactcccctagattttcaatatcgctagctgtagcatttccattattaattaaaaaattgcaatgtagatttgacacttgag

SEQ ID NO: 2334 - DNA, 120 bp, synthetic construct
  source 1..120: mol_type = other DNA
cgctagctgtagcatttccattattaattaaaaaattgcaatgtagatttgacacttgagcaccaccaatactatgcccacgtaatcctaccttatctatcaactgccaagctttatagt

SEQ ID NO: 2335 - DNA, 120 bp, synthetic construct
  source 1..120: mol_type = other DNA
caccaccaatactatgcccacgtaatcctaccttatctatcaactgccaagctttatagttgttagtattacgaaaagcgctaccagcagttttttggttaattggctgcgttaatttac

SEQ ID NO: 2336 - DNA, 120 bp, synthetic construct
  source 1..120: mol_type = other DNA
tgttagtattacgaaaagcgctaccagcagttttttggttaattggctgcgttaatttacgaactgtttgtattttttgtagcttttgactaatacttgttttactgtcattataacaaa

SEQ ID NO: 2337 - DNA, 120 bp, synthetic construct
  source 1..120: mol_type = other DNA
gaactgtttgtattttttgtagcttttgactaatacttgttttactgtcattataacaaatgagattagtttttgtaaagattaaaaagccattcacgatacattgcctatattcaaagt

SEQ ID NO: 2338 - DNA, 120 bp, synthetic construct
  source 1..120: mol_type = other DNA
tgagattagtttttgtaaagattaaaaagccattcacgatacattgcctatattcaaagtttaaatctttagataaaaatatatgcttattacctaatctatctaaagcctcaacagaat

SEQ ID NO: 2339 - DNA, 120 bp, synthetic construct
  source 1..120: mol_type = other DNA
ttaaatctttagataaaaatatatgcttattacctaatctatctaaagcctcaacagaataaacaacatctttaaattcctgtccataagctccagcattcatagcaatccccccaccta

SEQ ID NO: 2340 - DNA, 120 bp, synthetic construct
  source 1..120: mol_type = other DNA
aaacaacatctttaaattcctgtccataagctccagcattcatagcaatccccccacctattgtgccaggtattcctactaaaaattctaaaccacctaagttatgttgtagacaaaatt

SEQ ID NO: 2341 - DNA, 120 bp, synthetic construct
  source 1..120: mol_type = other DNA
ttgtgccaggtattcctactaaaaattctaaaccacctaagttatgttgtagacaaaattttgcaacatcatagtttaaagttccagctccaacactaataatattatagtgattatttt

SEQ ID NO: 2342 - DNA, 120 bp, synthetic construct
  source 1..120: mol_type = other DNA
ttgcaacatcatagtttaaagttccagctccaacactaataatattatagtgattatttttaacaaaattaatctcattgaaacttctacctaatttaattgttacaccatcaataccat

SEQ ID NO: 2343 - DNA, 120 bp, synthetic construct
  source 1..120: mol_type = other DNA
taacaaaattaatctcattgaaacttctacctaatttaattgttacaccatcaataccattatctctgataagtaaatttgatcctgctcctaatactgtaatttgaatatcaaattgta

SEQ ID NO: 2344 - DNA, 120 bp, synthetic construct
  source 1..120: mol_type = other DNA
tatctctgataagtaaatttgatcctgctcctaatactgtaatttgaatatcaaattgtaaattttttaaaaagcaagacagatcctcctcatctttaggtttataaaaaacttgactaa

SEQ ID NO: 2345 - DNA, 120 bp, synthetic construct
  source 1..120: mol_type = other DNA
aattttttaaaaagcaagacagatcctcctcatctttaggtttataaaaaacttgactaattccaccaaccttaaaccaagtcagttgagatagtttgaaattttttctatattcaccgt

SEQ ID NO: 2346 - DNA, 120 bp, synthetic construct
  source 1..120: mol_type = other DNA
ttccaccaaccttaaaccaagtcagttgagatagtttgaaattttttctatattcaccgttaatttttggtagtgatatcactgtagacatgctgctttaataatttctgtaattgctgt

SEQ ID NO: 2347 - DNA, 120 bp, synthetic construct
  source 1..120: mol_type = other DNA
taatttttggtagtgatatcactgtagacatgctgctttaataatttctgtaattgctgtggcaatattgctgcaaatttagtaatatctccagctcccattagtagaataatatcacat

SEQ ID NO: 2348 - DNA, 120 bp, synthetic construct
  source 1..120: mol_type = other DNA
ggcaatattgctgcaaatttagtaatatctccagctcccattagtagaataatatcacatggtttgacttgcctataaataatttgtggcaaatcatctaaattatttataggcataaca

SEQ ID NO: 2349 - DNA, 120 bp, synthetic construct
  source 1..120: mol_type = other DNA
ggtttgacttgcctataaataatttgtggcaaatcatctaaattatttataggcataacatatacgctatgataataactcttaatagcattaactaaagaaatatgagataagttatat

SEQ ID NO: 2350 - DNA, 120 bp, synthetic construct
  source 1..120: mol_type = other DNA
tatacgctatgataataactcttaatagcattaactaaagaaatatgagataagttatatgtttcttgttctccagcatcgtatatttgcgaaatatataattgatctacacgttgaaag

SEQ ID NO: 2351 - DNA, 120 bp, synthetic construct
  source 1..120: mol_type = other DNA
gtttcttgttctccagcatcgtatatttgcgaaatatataattgatctacacgttgaaagcaatgagtaaactctgaaaataactgttttaatctagagtaacgatgcggttgaaataca

SEQ ID NO: 2352 - DNA, 120 bp, synthetic construct
  source 1..120: mol_type = other DNA
caatgagtaaactctgaaaataactgttttaatctagagtaacgatgcggttgaaatacagctataacccttccctgctgcttatctgcaatacatcttgctgtatcaattgttgctata

SEQ ID NO: 2353 - DNA, 120 bp, synthetic construct
  source 1..120: mol_type = other DNA
gctataacccttccctgctgcttatctgcaatacatcttgctgtatcaattgttgctataatttctgcaggatggtgagcatagtcatcaataacggtaatgttattatactctccgatc

SEQ ID NO: 2354 - DNA, 120 bp, synthetic construct
  source 1..120: mol_type = other DNA
atttctgcaggatggtgagcatagtcatcaataacggtaatgttattatactctccgatctttgtaaagcgcctcgcaatacctttaaaatttttaaatccatccttaataatatttaag

SEQ ID NO: 2355 - DNA, 120 bp, synthetic construct
  source 1..120: mol_type = other DNA
tttgtaaagcgcctcgcaatacctttaaaatttttaaatccatccttaataatatttaagtctaagtttagctctacagcaatagctattgcagctagtgaattgagaatgttatgctta

SEQ ID NO: 2356 - DNA, 120 bp, synthetic construct
  source 1..120: mol_type = other DNA
tctaagtttagctctacagcaatagctattgcagctagtgaattgagaatgttatgcttacctaaagctggtaaagtaacttgcgtaattatgacttcattatgaaaattatatgcttta

SEQ ID NO: 2357 - DNA, 120 bp, synthetic construct
  source 1..120: mol_type = other DNA
cctaaagctggtaaagtaacttgcgtaattatgacttcattatgaaaattatatgctttaattctaacatcataggttgaataaccattatcagtattaatattaaatgcctgaatatgt

SEQ ID NO: 2358 - DNA, 120 bp, synthetic construct
  source 1..120: mol_type = other DNA
attctaacatcataggttgaataaccattatcagtattaatattaaatgcctgaatatgtgcattcttagaatcaataccataagtaataatctttctagatgtaattttagctattaaa

SEQ ID NO: 2359 - DNA, 120 bp, synthetic construct
  source 1..120: mol_type = other DNA
gcattcttagaatcaataccataagtaataatctttctagatgtaattttagctattaaattttgtactgtaatatcatcaatacaagctactgcaaaaccgtcatatggtaaattaata

SEQ ID NO: 2360 - DNA, 120 bp, synthetic construct
  source 1..120: mol_type = other DNA
ttttgtactgtaatatcatcaatacaagctactgcaaaaccgtcatatggtaaattaataataaatttacgaaaagcactaatcaaattatcaaaatttttataaaaatctaaatgctca

SEQ ID NO: 2361 - DNA, 120 bp, synthetic construct
  source 1..120: mol_type = other DNA
ataaatttacgaaaagcactaatcaaattatcaaaatttttataaaaatctaaatgctcaacatcaatattagtaataacagcaatcgttgcaggaattttaataaaagttgcatctgat

SEQ ID NO: 2362 - DNA, 120 bp, synthetic construct
  source 1..120: mol_type = other DNA
acatcaatattagtaataacagcaatcgttgcaggaattttaataaaagttgcatctgattcatcagcttcagcaatgaaataatcaccatcacctaaataagcatttgtggccctatta

SEQ ID NO: 2363 - DNA, 120 bp, synthetic construct
  source 1..120: mol_type = other DNA
tcatcagcttcagcaatgaaataatcaccatcacctaaataagcatttgtggccctattattcataattccaccagtaataactgtaggatgtaacccacatgcttcaaatatgcaagca

SEQ ID NO: 2364 - DNA, 120 bp, synthetic construct
  source 1..120: mol_type = other DNA
ttcataattccaccagtaataactgtaggatgtaacccacatgcttcaaatatgcaagcaatcaatgctgttgtagtagttttgccgtgagatcctgaaattgctatagcaacctttgat

SEQ ID NO: 2365 - DNA, 120 bp, synthetic construct
  source 1..120: mol_type = other DNA
atcaatgctgttgtagtagttttgccgtgagatcctgaaattgctatagcaacctttgatctcattagctcagctaacatctctgctctagatattattggtatttttgctaagattgca

SEQ ID NO: 2366 - DNA, 120 bp, synthetic construct
  source 1..120: mol_type = other DNA
ctcattagctcagctaacatctctgctctagatattattggtatttttgctaagattgcagcctgatattcagggttattgtgttttatagcagaagatataactacaattcctgctcca

SEQ ID NO: 2367 - DNA, 120 bp, synthetic construct
  source 1..120: mol_type = other DNA
gcctgatattcagggttattgtgttttatagcagaagatataactacaattcctgctccattaatattattagcattatggccatgtaatacttcaatgcctaataatctcaatctttca

SEQ ID NO: 2368 - DNA, 120 bp, synthetic construct
  source 1..120: mol_type = other DNA
ttaatattattagcattatggccatgtaatacttcaatgcctaataatctcaatctttcagtattaacattactagtaagatctgaccctctaatcttataacctagattgtacattatt

SEQ ID NO: 2369 - DNA, 120 bp, synthetic construct
  source 1..120: mol_type = other DNA
gtattaacattactagtaagatctgaccctctaatcttataacctagattgtacattatttctgcaataccactcatacctatgccaccgataccaataatatgcacaataccaaaatta

SEQ ID NO: 2370 - DNA, 120 bp, synthetic construct
  source 1..120: mol_type = other DNA
tctgcaataccactcatacctatgccaccgataccaataatatgcacaataccaaaattacttttaagtcttcgatttgctaacaatgtcatgcaaataatacttatataagcatgcctt

SEQ ID NO: 2371 - DNA, 120 bp, synthetic construct
  source 1..120: mol_type = other DNA
cttttaagtcttcgatttgctaacaatgtcatgcaaataatacttatataagcatgcctttttgacatgctattttttttaaaatatacagccgtcttccatttatcagcttatcagcat

SEQ ID NO: 2372 - DNA, 120 bp, synthetic construct
  source 1..120: mol_type = other DNA
tttgacatgctattttttttaaaatatacagccgtcttccatttatcagcttatcagcattgcttaagcataagctgcaactcaatattaactaaataagcagctaaaattagaaaaaga

SEQ ID NO: 2373 - DNA, 120 bp, synthetic construct
  source 1..120: mol_type = other DNA
tgcttaagcataagctgcaactcaatattaactaaataagcagctaaaattagaaaaagaaattaatcaaaatttttacataatttttcataatttcttttttttctataatgttataag

SEQ ID NO: 2374 - DNA, 120 bp, synthetic construct
  source 1..120: mol_type = other DNA
aattaatcaaaatttttacataatttttcataatttcttttttttctataatgttataagaacttaaaagctaaatctaacactacatgataaagtatggccattaagatcatacgtctt

SEQ ID NO: 2375 - DNA, 120 bp, synthetic construct
  source 1..120: mol_type = other DNA
aacttaaaagctaaatctaacactacatgataaagtatggccattaagatcatacgtcttaaagttatcatatggcttatctttcacatcttcgcctgtaatgcttcctatccacatata

SEQ ID NO: 2376 - DNA, 120 bp, synthetic construct
  source 1..120: mol_type = other DNA
aaagttatcatatggcttatctttcacatcttcgcctgtaatgcttcctatccacatatacctatattcaacatctaagtgcacttcatcaattacttcagccgatataccagccatagc

SEQ ID NO: 2377 - DNA, 120 bp, synthetic construct
  source 1..120: mol_type = other DNA
cctatattcaacatctaagtgcacttcatcaattacttcagccgatataccagccatagcttctttataaaaaccaactttataacctatcttatgctgttctattgtaccaccagtata

SEQ ID NO: 2378 - DNA, 120 bp, synthetic construct
  source 1..120: mol_type = other DNA
ttctttataaaaaccaactttataacctatcttatgctgttctattgtaccaccagtatatgaagcaccaacccctccaccagcaaaaattgacactggccctaatttaattaaattaag

SEQ ID NO: 2379 - DNA, 120 bp, synthetic construct
  source 1..120: mol_type = other DNA
tgaagcaccaacccctccaccagcaaaaattgacactggccctaatttaattaaattaagataacaccttaatgccagaactccagagttaagagataacaaactgctatctagcttatg

SEQ ID NO: 2380 - DNA, 120 bp, synthetic construct
  source 1..120: mol_type = other DNA
ataacaccttaatgccagaactccagagttaagagataacaaactgctatctagcttatgattaggattattattattatctaagtcattaccgctagcttgttgctcttcctgtgaatt

SEQ ID NO: 2381 - DNA, 120 bp, synthetic construct
  source 1..120: mol_type = other DNA
attaggattattattattatctaagtcattaccgctagcttgttgctcttcctgtgaattacttacactttgctctggtttagttgtaatatcaaagagccacatagccccaacttctgt

SEQ ID NO: 2382 - DNA, 120 bp, synthetic construct
  source 1..120: mol_type = other DNA
acttacactttgctctggtttagttgtaatatcaaagagccacatagccccaacttctgtcctaaaatatcgatttacataagcccctaaacttccacctattccaaatgaaaatttgtt

SEQ ID NO: 2383 - DNA, 120 bp, synthetic construct
  source 1..120: mol_type = other DNA
cctaaaatatcgatttacataagcccctaaacttccacctattccaaatgaaaatttgttaaactcaagctctttatttttaaaatgagattcccaattggttggcattaatccaaccgc

SEQ ID NO: 2384 - DNA, 120 bp, synthetic construct
  source 1..120: mol_type = other DNA
aaactcaagctctttatttttaaaatgagattcccaattggttggcattaatccaaccgcactaaccttagcataataattatattctaaatagtctaaatattctgatgaattattagc

SEQ ID NO: 2385 - DNA, 120 bp, synthetic construct
  source 1..120: mol_type = other DNA
actaaccttagcataataattatattctaaatagtctaaatattctgatgaattattagcatgtaccaaagatgaacttgataatgcagaaagcgcagtaatagcatttattattacttt

SEQ ID NO: 2386 - DNA, 120 bp, synthetic construct
  source 1..120: mol_type = other DNA
atgtaccaaagatgaacttgataatgcagaaagcgcagtaatagcatttattattactttttttattttactcatgaacttttacttattttttatgactgttgttattgatttaaatgc

SEQ ID NO: 2387 - DNA, 120 bp, synthetic construct
  source 1..120: mol_type = other DNA
ttttattttactcatgaacttttacttattttttatgactgttgttattgatttaaatgcttcctaattacaaaaacttctccattttaggagtatatttctatatataatccaacaagc

SEQ ID NO: 2388 - DNA, 120 bp, synthetic construct
  source 1..120: mol_type = other DNA
ttcctaattacaaaaacttctccattttaggagtatatttctatatataatccaacaagctttaagttaattaaatagcaaagaataaagttaatttttattattataaaaactctgaaa

SEQ ID NO: 2389 - DNA, 120 bp, synthetic construct
  source 1..120: mol_type = other DNA
tttaagttaattaaatagcaaagaataaagttaatttttattattataaaaactctgaaaaagtagctaaaaaacctgcaaaggacttttagctgctttttttttataattttaaagaaa

SEQ ID NO: 2390 - DNA, 120 bp, synthetic construct
  source 1..120: mol_type = other DNA
aagtagctaaaaaacctgcaaaggacttttagctgctttttttttataattttaaagaaaaactagaagttatagcgcacacatgcacttgcaataaacgcgtttacttggtacttatct

SEQ ID NO: 2391 - DNA, 120 bp, synthetic construct
  source 1..120: mol_type = other DNA
aactagaagttatagcgcacacatgcacttgcaataaacgcgtttacttggtacttatcttctactttactgaatgagtgcatataaccagcctctaagtccacacatacaccctcagca

SEQ ID NO: 2392 - DNA, 120 bp, synthetic construct
  source 1..120: mol_type = other DNA
tctactttactgaatgagtgcatataaccagcctctaagtccacacatacaccctcagcagcattaattgctacaccaagtgctcctgatgcaaccatgcctgtataccctttaacatcc

SEQ ID NO: 2393 - DNA, 120 bp, synthetic construct
  source 1..120: mol_type = other DNA
gcattaattgctacaccaagtgctcctgatgcaaccatgcctgtataccctttaacatccttattatctatttttccataagtataagctaaccctgcaccaacaccaccgtatattgag

SEQ ID NO: 2394 - DNA, 120 bp, synthetic construct
  source 1..120: mol_type = other DNA
ttattatctatttttccataagtataagctaaccctgcaccaacaccaccgtatattgagaatgattcagttgtaactaggtcagcatagagtttaacttggccaacaaccatactcaga

SEQ ID NO: 2395 - DNA, 120 bp, synthetic construct
  source 1..120: mol_type = other DNA
aatgattcagttgtaactaggtcagcatagagtttaacttggccaacaaccatactcagatcaaactctgtttctttgacttttccttctttagatttttcagatgctccttgttgctgc

SEQ ID NO: 2396 - DNA, 120 bp, synthetic construct
  source 1..120: mol_type = other DNA
tcaaactctgtttctttgacttttccttctttagatttttcagatgctccttgttgctgcttgcagtcacctttaccttgattctttgcatcttcttcttgttgggcagctaatttttcc

SEQ ID NO: 2397 - DNA, 120 bp, synthetic construct
  source 1..120: mol_type = other DNA
ttgcagtcacctttaccttgattctttgcatcttcttcttgttgggcagctaatttttccatggctttcctaattcctgcatgacgctgcaatttaacaagatctttatataactgcgca

SEQ ID NO: 2398 - DNA, 120 bp, synthetic construct
  source 1..120: mol_type = other DNA
atggctttcctaattcctgcatgacgctgcaatttaacaagatctttatataactgcgcaatctgatcactgccatttaaaagcctaacagctgctgctgctactgcttcttgcgctgta

SEQ ID NO: 2399 - DNA, 120 bp, synthetic construct
  source 1..120: mol_type = other DNA
atctgatcactgccatttaaaagcctaacagctgctgctgctactgcttcttgcgctgtagcttgagcttgctgttgctgcccttgcccctgctgttgctgtgcttgcggcggcatgaca

SEQ ID NO: 2400 - DNA, 120 bp, synthetic construct
  source 1..120: mol_type = other DNA
gcttgagcttgctgttgctgcccttgcccctgctgttgctgtgcttgcggcggcatgacaaaattcaagtgtatctgattaacaaaagcattattaatatacccatcaaaagaatctctg

SEQ ID NO: 2401 - DNA, 120 bp, synthetic construct
  source 1..120: mol_type = other DNA
aaattcaagtgtatctgattaacaaaagcattattaatatacccatcaaaagaatctctgagttcttccaatgtatcacctaattcttggattttactctgtatctgttcgatagatgca

SEQ ID NO: 2402 - DNA, 120 bp, synthetic construct
  source 1..120: mol_type = other DNA
agttcttccaatgtatcacctaattcttggattttactctgtatctgttcgatagatgcactattaggcaaaccagtatcaggaacattaataccagctatatcagcaaatggctttata

SEQ ID NO: 2403 - DNA, 120 bp, synthetic construct
  source 1..120: mol_type = other DNA
ctattaggcaaaccagtatcaggaacattaataccagctatatcagcaaatggctttatatcactatatatctgaataattttgtcactcaaaactttgacaggagaagcgctaggttta

SEQ ID NO: 2404 - DNA, 120 bp, synthetic construct
  source 1..120: mol_type = other DNA
tcactatatatctgaataattttgtcactcaaaactttgacaggagaagcgctaggtttattagcatttgataatgcagcaagaccaactaccaaactcctccattgctcatggttatgt

SEQ ID NO: 2405 - DNA, 120 bp, synthetic construct
  source 1..120: mol_type = other DNA
ttagcatttgataatgcagcaagaccaactaccaaactcctccattgctcatggttatgtatcgcaaaatttgcaggctgatttgctcgctgcggtggctgtccaacaggattagggttg

SEQ ID NO: 2406 - DNA, 120 bp, synthetic construct
  source 1..120: mol_type = other DNA
atcgcaaaatttgcaggctgatttgctcgctgcggtggctgtccaacaggattagggttgccctgtggaatatttaacaacaccggatttaccatcatatgcccaggattattaggatcc

SEQ ID NO: 2407 - DNA, 120 bp, synthetic construct
  source 1..120: mol_type = other DNA
ccctgtggaatatttaacaacaccggatttaccatcatatgcccaggattattaggatccttcaccatatagtcaataccagcacaattctttaaccaagcgatcctagctgcagcacgc

SEQ ID NO: 2408 - DNA, 120 bp, synthetic construct
  source 1..120: mol_type = other DNA
ttcaccatatagtcaataccagcacaattctttaaccaagcgatcctagctgcagcacgcttctgatcattaagcggaggctgtgcagcttgcgcttgcgcctgaggtatgttaggaata

SEQ ID NO: 2409 - DNA, 120 bp, synthetic construct
  source 1..120: mol_type = other DNA
ttctgatcattaagcggaggctgtgcagcttgcgcttgcgcctgaggtatgttaggaatatcaatcccaaagtcacgatcagctatacttataggcatcatagtaggctgaggtggtgta

SEQ ID NO: 2410 - DNA, 120 bp, synthetic construct
  source 1..120: mol_type = other DNA
tcaatcccaaagtcacgatcagctatacttataggcatcatagtaggctgaggtggtgtaagtttaaacggcttacgtataggagcatctgtcccacctccagaatctgcctttatctca

SEQ ID NO: 2411 - DNA, 120 bp, synthetic construct
  source 1..120: mol_type = other DNA
agtttaaacggcttacgtataggagcatctgtcccacctccagaatctgcctttatctcacctttagaatctacctcgcctttacctacttcaacctcagcgcttatatttctaaggtac

SEQ ID NO: 2412 - DNA, 120 bp, synthetic construct
  source 1..120: mol_type = other DNA
cctttagaatctacctcgcctttacctacttcaacctcagcgcttatatttctaaggtacataacacctagctctgctctaaatcctggtgcaattgtcatacccgcagctaatgtacca

SEQ ID NO: 2413 - DNA, 120 bp, synthetic construct
  source 1..120: mol_type = other DNA
ataacacctagctctgctctaaatcctggtgcaattgtcatacccgcagctaatgtaccaccaaatggcagtccagttgttaatgacaaatgtttttttccctcagaatcagttgaatcc

SEQ ID NO: 2414 - DNA, 120 bp, synthetic construct
  source 1..120: mol_type = other DNA
ccaaatggcagtccagttgttaatgacaaatgtttttttccctcagaatcagttgaatccaagcgagtagattctgcaccagtaatcattcctccaacaactccaactttagcataagga

SEQ ID NO: 2415 - DNA, 120 bp, synthetic construct
  source 1..120: mol_type = other DNA
aagcgagtagattctgcaccagtaatcattcctccaacaactccaactttagcataaggaccacactctaatcctacttcatcctccaattctatcgcactagctgaaaacggcaacgac

SEQ ID NO: 2416 - DNA, 120 bp, synthetic construct
  source 1..120: mol_type = other DNA
ccacactctaatcctacttcatcctccaattctatcgcactagctgaaaacggcaacgacaacgcagacattgcactagcaattaacataatttttttcattctaatctccttaaaagaa

SEQ ID NO: 2417 - DNA, 120 bp, synthetic construct
  source 1..120: mol_type = other DNA
aacgcagacattgcactagcaattaacataatttttttcattctaatctccttaaaagaattaaatttattttttagtggtaaccattctaaactaattatttagccacactaacttagt

SEQ ID NO: 2418 - DNA, 120 bp, synthetic construct
  source 1..120: mol_type = other DNA
ttaaatttattttttagtggtaaccattctaaactaattatttagccacactaacttagttttatatcaaaaaactattatttagtatactaatatttaatagtacttgtaaaataattt

SEQ ID NO: 2419 - DNA, 120 bp, synthetic construct
  source 1..120: mol_type = other DNA
tttatatcaaaaaactattatttagtatactaatatttaatagtacttgtaaaataatttaaacaatctataaaacactgtgttaaaaatatcgcttcaaagcgttttatccattgtaaa

SEQ ID NO: 2420 - DNA, 120 bp, synthetic construct
  source 1..120: mol_type = other DNA
aaacaatctataaaacactgtgttaaaaatatcgcttcaaagcgttttatccattgtaaaatttatttttattttttatatataacttaaagacaacattcaatagaacactgctcttat

SEQ ID NO: 2421 - DNA, 120 bp, synthetic construct
  source 1..120: mol_type = other DNA
atttatttttattttttatatataacttaaagacaacattcaatagaacactgctcttatatatatgtttaaagacacgttcgaaaatacattaattatctattagcaccttgttacagt

SEQ ID NO: 2422 - DNA, 120 bp, synthetic construct
  source 1..120: mol_type = other DNA
atatatgtttaaagacacgttcgaaaatacattaattatctattagcaccttgttacagttaaccttagatagcataacactactttttacgcaacaactaccttcaattattaataatt

SEQ ID NO: 2423 - DNA, 120 bp, synthetic construct
  source 1..120: mol_type = other DNA
taaccttagatagcataacactactttttacgcaacaactaccttcaattattaataatttttcttgcctaaaagtttatttttagctaaaatagcaacagtttttcaagctaaataatc

SEQ ID NO: 2424 - DNA, 120 bp, synthetic construct
  source 1..120: mol_type = other DNA
tttcttgcctaaaagtttatttttagctaaaatagcaacagtttttcaagctaaataatcaagccctgtcttaattattattttatataaaatcttaaatcaagatacattaatttaacc

SEQ ID NO: 2425 - DNA, 120 bp, synthetic construct
  source 1..120: mol_type = other DNA
aagccctgtcttaattattattttatataaaatcttaaatcaagatacattaatttaaccacataattatactaacattgtattatctaaaattagcccacataaaaaatgaacaaactt

SEQ ID NO: 2426 - DNA, 120 bp, synthetic construct
  source 1..120: mol_type = other DNA
acataattatactaacattgtattatctaaaattagcccacataaaaaatgaacaaactttcttttcaacaaataataatgcacctgcagcaattctggtgcaatcaaggctgtgctata

SEQ ID NO: 2427 - DNA, 120 bp, synthetic construct
  source 1..120: mol_type = other DNA
tcttttcaacaaataataatgcacctgcagcaattctggtgcaatcaaggctgtgctatattgcaaccatatgacgttgaaattggcgcaggaacttttcatcctgcaacagcaataaaa

SEQ ID NO: 2428 - DNA, 120 bp, synthetic construct
  source 1..120: mol_type = other DNA
ttgcaaccatatgacgttgaaattggcgcaggaacttttcatcctgcaacagcaataaaattgctagggcaagccaaatggcgtgcagcatatgttcagccatccaggcgaccaactgat

SEQ ID NO: 2429 - DNA, 120 bp, synthetic construct
  source 1..120: mol_type = other DNA
ttgctagggcaagccaaatggcgtgcagcatatgttcagccatccaggcgaccaactgatagtagatatggcagccaccctaatcgtttacagcaatactaccagtttcaagtcataatt

SEQ ID NO: 2430 - DNA, 120 bp, synthetic construct
  source 1..120: mol_type = other DNA
agtagatatggcagccaccctaatcgtttacagcaatactaccagtttcaagtcataattaagccatctccagataatattcaagctctttacttacatagcttagaatatctcaacata

SEQ ID NO: 2431 - DNA, 120 bp, synthetic construct
  source 1..120: mol_type = other DNA
aagccatctccagataatattcaagctctttacttacatagcttagaatatctcaacataaaaactcaaactaatgatattagatttgtagaagatgactggcaatcccctaccctagga

SEQ ID NO: 2432 - DNA, 120 bp, synthetic construct
  source 1..120: mol_type = other DNA
aaaactcaaactaatgatattagatttgtagaagatgactggcaatcccctaccctaggagcctcaggcttaggctgggaagtatggtgtaatggaatggaaatttctcagattacttac

SEQ ID NO: 2433 - DNA, 120 bp, synthetic construct
  source 1..120: mol_type = other DNA
gcctcaggcttaggctgggaagtatggtgtaatggaatggaaatttctcagattacttacttacaacaaatagctagcatagaatgcaatccagtacctatagaaatcacttatggactt

SEQ ID NO: 2434 - DNA, 120 bp, synthetic construct
  source 1..120: mol_type = other DNA
ttacaacaaatagctagcatagaatgcaatccagtacctatagaaatcacttatggacttgaacgattagcaatgtacatacaggaagtcgatgatattaaactactaaattggaataat

SEQ ID NO: 2435 - DNA, 120 bp, synthetic construct
  source 1..120: mol_type = other DNA
gaacgattagcaatgtacatacaggaagtcgatgatattaaactactaaattggaataatcaatcaggagaactagctttaacatatcaaatggttaacatagagaatgaacggcaattt

SEQ ID NO: 2436 - DNA, 120 bp, synthetic construct
  source 1..120: mol_type = other DNA
caatcaggagaactagctttaacatatcaaatggttaacatagagaatgaacggcaattttctgcttataaccttgaatacgccaacacaaatatattgtttaaacaatttgaagacgct

SEQ ID NO: 2437 - DNA, 120 bp, synthetic construct
  source 1..120: mol_type = other DNA
tctgcttataaccttgaatacgccaacacaaatatattgtttaaacaatttgaagacgctgaacaacaatgccaagatttagtcaagcaaaatcttcctctaccagcatatgatttctgt

SEQ ID NO: 2438 - DNA, 120 bp, synthetic construct
  source 1..120: mol_type = other DNA
gaacaacaatgccaagatttagtcaagcaaaatcttcctctaccagcatatgatttctgtttaaaagctagccacttatttaatctacttgatagcagaggagtaatcggagttactcaa

SEQ ID NO: 2439 - DNA, 120 bp, synthetic construct
  source 1..120: mol_type = other DNA
ttaaaagctagccacttatttaatctacttgatagcagaggagtaatcggagttactcaacgcactaattatatcgctagaatacgaacactagctcaaacagtatgtaatcaatatata

SEQ ID NO: 2440 - DNA, 120 bp, synthetic construct
  source 1..120: mol_type = other DNA
cgcactaattatatcgctagaatacgaacactagctcaaacagtatgtaatcaatatataaaaaatcttaatatatcaaatgcatagttacagtttaatattagaactctactctgagga

SEQ ID NO: 2441 - DNA, 120 bp, synthetic construct
  source 1..120: mol_type = other DNA
aaaaatcttaatatatcaaatgcatagttacagtttaatattagaactctactctgaggaaattccagctaaaatgcaaaaaaaagctgaattagcatttcaagaaatttttactaaaaa

SEQ ID NO: 2442 - DNA, 120 bp, synthetic construct
  source 1..120: mol_type = other DNA
aattccagctaaaatgcaaaaaaaagctgaattagcatttcaagaaatttttactaaaaatttcaaattagctaatattagttttaatcacttaaaagtatatataggcccatgcagagt

SEQ ID NO: 2443 - DNA, 120 bp, synthetic construct
  source 1..120: mol_type = other DNA
tttcaaattagctaatattagttttaatcacttaaaagtatatataggcccatgcagagtggttctacatacagtctttagcagcaaagaactagccgctaaagcaattgaacataaagg

SEQ ID NO: 2444 - DNA, 120 bp, synthetic construct
  source 1..120: mol_type = other DNA
ggttctacatacagtctttagcagcaaagaactagccgctaaagcaattgaacataaaggccctaaagtcggagcaaaaaaatcagctgttgaaggattttgcaaagctaagtctatttt

SEQ ID NO: 2445 - DNA, 120 bp, synthetic construct
  source 1..120: mol_type = other DNA
ccctaaagtcggagcaaaaaaatcagctgttgaaggattttgcaaagctaagtctattttaagcaaggacttaaccataaaaacatttaataatcagcagttctacgtttatactcatgt

SEQ ID NO: 2446 - DNA, 120 bp, synthetic construct
  source 1..120: mol_type = other DNA
aagcaaggacttaaccataaaaacatttaataatcagcagttctacgtttatactcatgttactccaactcaacctattaaagatctattaccagaaatcatattaaattccattaaaga

SEQ ID NO: 2447 - DNA, 120 bp, synthetic construct
  source 1..120: mol_type = other DNA
tactccaactcaacctattaaagatctattaccagaaatcatattaaattccattaaagaatacacttggccaaaatcaatgaaatgggggaattatcagattaattgggttagaccact

SEQ ID NO: 2448 - DNA, 120 bp, synthetic construct
  source 1..120: mol_type = other DNA
atacacttggccaaaatcaatgaaatgggggaattatcagattaattgggttagaccacttagaaacattttatgcatgttcaatggcgaagaattaaaaatcagctggcatcatctaac

SEQ ID NO: 2449 - DNA, 120 bp, synthetic construct
  source 1..120: mol_type = other DNA
tagaaacattttatgcatgttcaatggcgaagaattaaaaatcagctggcatcatctaacatcaaataataaaagctttgggcataaattcatgagtccaaatagctttaccgtaagcac

SEQ ID NO: 2450 - DNA, 120 bp, synthetic construct
  source 1..120: mol_type = other DNA
atcaaataataaaagctttgggcataaattcatgagtccaaatagctttaccgtaagcacatggaaagattatactaataatttaagagataattttgtcatattagacagatcagaacg

SEQ ID NO: 2451 - DNA, 120 bp, synthetic construct
  source 1..120: mol_type = other DNA
atggaaagattatactaataatttaagagataattttgtcatattagacagatcagaacgacaagctattatacttaattccttagaaaaaacatgccaaactctaggcatcaccttaaa

SEQ ID NO: 2452 - DNA, 120 bp, synthetic construct
  source 1..120: mol_type = other DNA
acaagctattatacttaattccttagaaaaaacatgccaaactctaggcatcaccttaaattacaataataaattacttgatgaagttactggtttagttgaataccctatcgtattata

SEQ ID NO: 2453 - DNA, 120 bp, synthetic construct
  source 1..120: mol_type = other DNA
ttacaataataaattacttgatgaagttactggtttagttgaataccctatcgtattatatggcacaatacctaatgagtttcttagcttaccagaagaaatcatcatcacttctgtaca

SEQ ID NO: 2454 - DNA, 120 bp, synthetic construct
  source 1..120: mol_type = other DNA
tggcacaatacctaatgagtttcttagcttaccagaagaaatcatcatcacttctgtacaaactcatcaaaaatatttcactacaaaagatcatagcaataaactagctccatatttttt

SEQ ID NO: 2455 - DNA, 120 bp, synthetic construct
  source 1..120: mol_type = other DNA
aactcatcaaaaatatttcactacaaaagatcatagcaataaactagctccatattttttatttgttaccaatatcaatactgaagattacagcaatattatcaaaggaaatgaaaaagt

SEQ ID NO: 2456 - DNA, 120 bp, synthetic construct
  source 1..120: mol_type = other DNA
atttgttaccaatatcaatactgaagattacagcaatattatcaaaggaaatgaaaaagtcttatcatctcgtctaactgatgctatatacttttttaatcaagactgtcaacttacatt

SEQ ID NO: 2457 - DNA, 120 bp, synthetic construct
  source 1..120: mol_type = other DNA
cttatcatctcgtctaactgatgctatatacttttttaatcaagactgtcaacttacattgcttagtaaattagaaaaattaaaaaaagtagtctttcacactaaaattggtagtatatt

SEQ ID NO: 2458 - DNA, 120 bp, synthetic construct
  source 1..120: mol_type = other DNA
gcttagtaaattagaaaaattaaaaaaagtagtctttcacactaaaattggtagtatatttgataaagttcagagaataaaaaaaatatgccataagcttgcacctgatgatcaagaact

SEQ ID NO: 2459 - DNA, 120 bp, synthetic construct
  source 1..120: mol_type = other DNA
tgataaagttcagagaataaaaaaaatatgccataagcttgcacctgatgatcaagaactagctattgcagctgaactgtgtaaatcagatttagtctcagaagtggtacaagaattccc

SEQ ID NO: 2460 - DNA, 120 bp, synthetic construct
  source 1..120: mol_type = other DNA
agctattgcagctgaactgtgtaaatcagatttagtctcagaagtggtacaagaattccctaatctacaaggaataatgggaaaatactatgctttaaatgacaaactcagccctgcagt

SEQ ID NO: 2461 - DNA, 120 bp, synthetic construct
  source 1..120: mol_type = other DNA
taatctacaaggaataatgggaaaatactatgctttaaatgacaaactcagccctgcagtcgctaatataatcggcaaccactactatcctaccagaattgaagatgaagtacctaatgg

SEQ ID NO: 2462 - DNA, 120 bp, synthetic construct
  source 1..120: mol_type = other DNA
cgctaatataatcggcaaccactactatcctaccagaattgaagatgaagtacctaatggtaaggcagcaattcttgctttagctgacaagcttgataatttaactagcctatatttagc

SEQ ID NO: 2463 - DNA, 120 bp, synthetic construct
  source 1..120: mol_type = other DNA
taaggcagcaattcttgctttagctgacaagcttgataatttaactagcctatatttagcaggagagcgcgctactagttcaaaagatccatttgcattacgtagatgcgctttttctat

SEQ ID NO: 2464 - DNA, 120 bp, synthetic construct
  source 1..120: mol_type = other DNA
aggagagcgcgctactagttcaaaagatccatttgcattacgtagatgcgctttttctatcgctagaataattttaactaataaaatacaagtaaaattattagatttattaactttcat

SEQ ID NO: 2465 - DNA, 120 bp, synthetic construct
  source 1..120: mol_type = other DNA
cgctagaataattttaactaataaaatacaagtaaaattattagatttattaactttcatttatcaacttcatgatatttatactaatgagctagcaaccgaagtactactattcataaa

SEQ ID NO: 2466 - DNA, 120 bp, synthetic construct
  source 1..120: mol_type = other DNA
ttatcaacttcatgatatttatactaatgagctagcaaccgaagtactactattcataaaagataaaacaaaaaatttacttaatgcaaaatttaatcatttgttagtcgaagctatatt

SEQ ID NO: 2467 - DNA, 120 bp, synthetic construct
  source 1..120: mol_type = other DNA
agataaaacaaaaaatttacttaatgcaaaatttaatcatttgttagtcgaagctatatttcagcaaaacaactatgatgatcttactgagttagaattaagaatgaatattcttgatca

SEQ ID NO: 2468 - DNA, 120 bp, synthetic construct
  source 1..120: mol_type = other DNA
tcagcaaaacaactatgatgatcttactgagttagaattaagaatgaatattcttgatcattttttaacctcaactaaaggtcaaaactttatacaatcatataaaagagcgtataatat

SEQ ID NO: 2469 - DNA, 120 bp, synthetic construct
  source 1..120: mol_type = other DNA
ttttttaacctcaactaaaggtcaaaactttatacaatcatataaaagagcgtataatatcattaaagatgaagaaattcgtcaagcaaaaatagatggttacaaattattaactaaaca

SEQ ID NO: 2470 - DNA, 120 bp, synthetic construct
  source 1..120: mol_type = other DNA
cattaaagatgaagaaattcgtcaagcaaaaatagatggttacaaattattaactaaacaagaaaccatcctatatcagcaagctatgaattcaaaagttagccaattatctactcaatt

SEQ ID NO: 2471 - DNA, 120 bp, synthetic construct
  source 1..120: mol_type = other DNA
agaaaccatcctatatcagcaagctatgaattcaaaagttagccaattatctactcaattctcagctgaaagttttactttagctcttgatcaattatcaaatcttagcatacaaattgc

SEQ ID NO: 2472 - DNA, 120 bp, synthetic construct
  source 1..120: mol_type = other DNA
ctcagctgaaagttttactttagctcttgatcaattatcaaatcttagcatacaaattgcagaatttttagacaatgtcactgttaacactactgatcagtatcttactgatactcgcaa

SEQ ID NO: 2473 - DNA, 120 bp, synthetic construct
  source 1..120: mol_type = other DNA
agaatttttagacaatgtcactgttaacactactgatcagtatcttactgatactcgcaagcttatattacaatatgtagtacagttttgcaataatatagcaccatttgacaaagtaat

SEQ ID NO: 2474 - DNA, 120 bp, synthetic construct
  source 1..120: mol_type = other DNA
gcttatattacaatatgtagtacagttttgcaataatatagcaccatttgacaaagtaataaaacattatgttagcaaatatgaacagtaataataatgatataaatgttgctgcacaat

SEQ ID NO: 2475 - DNA, 120 bp, synthetic construct
  source 1..120: mol_type = other DNA
aaaacattatgttagcaaatatgaacagtaataataatgatataaatgttgctgcacaatttattgaacaagggaaattagttatattccctactgaaacagtgtatggcataggagctg

SEQ ID NO: 2476 - DNA, 120 bp, synthetic construct
  source 1..120: mol_type = other DNA
ttattgaacaagggaaattagttatattccctactgaaacagtgtatggcataggagctgatgcaactaatgacaatgcttgtcaaagcatttataaaatcaaaaacagaccaatgaata

SEQ ID NO: 2477 - DNA, 120 bp, synthetic construct
  source 1..120: mol_type = other DNA
atgcaactaatgacaatgcttgtcaaagcatttataaaatcaaaaacagaccaatgaataatccattaattattcatgtcagcaatatacaagctgctcaaactataggcatatttaaca

SEQ ID NO: 2478 - DNA, 120 bp, synthetic construct
  source 1..120: mol_type = other DNA
atccattaattattcatgtcagcaatatacaagctgctcaaactataggcatatttaacaatcttgctattaaactagcaaccttatggccaggcccaattagcttagttgtaccactta

SEQ ID NO: 2479 - DNA, 120 bp, synthetic construct
  source 1..120: mol_type = other DNA
atcttgctattaaactagcaaccttatggccaggcccaattagcttagttgtaccacttaatcaatcagcaggaattagcagaacagcaacagcaaatcttgatactgtagcaattagaa

SEQ ID NO: 2480 - DNA, 120 bp, synthetic construct
  source 1..120: mol_type = other DNA
atcaatcagcaggaattagcagaacagcaacagcaaatcttgatactgtagcaattagaattccatctcataaggtagctctcatgttgctacagttaacacaaaaacctatagctgctc

SEQ ID NO: 2481 - DNA, 120 bp, synthetic construct
  source 1..120: mol_type = other DNA
ttccatctcataaggtagctctcatgttgctacagttaacacaaaaacctatagctgctccaagcgcaaacccatcaggctatctcagccctactacctatcaacatgccaatatccatt

SEQ ID NO: 2482 - DNA, 120 bp, synthetic construct
  source 1..120: mol_type = other DNA
caagcgcaaacccatcaggctatctcagccctactacctatcaacatgccaatatccatttccaaaattctccagacatattcattcttaagggcgctcaatcaacttatggattagaat

SEQ ID NO: 2483 - DNA, 120 bp, synthetic construct
  source 1..120: mol_type = other DNA
tccaaaattctccagacatattcattcttaagggcgctcaatcaacttatggattagaatctactataattgatactactgctgatagaccaacaatattacgccatggattcattacaa

SEQ ID NO: 2484 - DNA, 120 bp, synthetic construct
  source 1..120: mol_type = other DNA
ctactataattgatactactgctgatagaccaacaatattacgccatggattcattacaacagaaataataaagactattactgggcaaaaccctattatagcagaaaaacataacaagc

SEQ ID NO: 2485 - DNA, 120 bp, synthetic construct
  source 1..120: mol_type = other DNA
cagaaataataaagactattactgggcaaaaccctattatagcagaaaaacataacaagcttttaaaagctccaggaatgatgttaaagcattattctcctattactaaaattaggttaa

SEQ ID NO: 2486 - DNA, 120 bp, synthetic construct
  source 1..120: mol_type = other DNA
ttttaaaagctccaggaatgatgttaaagcattattctcctattactaaaattaggttaaatgcaacaaagcttcttccaaaagaagtaggattaaattatgggcctaatactctaactg

SEQ ID NO: 2487 - DNA, 120 bp, synthetic construct
  source 1..120: mol_type = other DNA
atgcaacaaagcttcttccaaaagaagtaggattaaattatgggcctaatactctaactggaaaatactgcctaaatcttagcccaaacagtaatttaatgaatgcagcagcaaacttat

SEQ ID NO: 2488 - DNA, 120 bp, synthetic construct
  source 1..120: mol_type = other DNA
gaaaatactgcctaaatcttagcccaaacagtaatttaatgaatgcagcagcaaacttatatcatatgcttcatcaacttgacaactatgcacaaaatcctatcaatgaggttgagacta

SEQ ID NO: 2489 - DNA, 120 bp, synthetic construct
  source 1..120: mol_type = other DNA
atcatatgcttcatcaacttgacaactatgcacaaaatcctatcaatgaggttgagactatcgctatagctcaaataccaaatataggcataggaattgctatcaatgacaagcttaatc

SEQ ID NO: 2490 - DNA, 120 bp, synthetic construct
  source 1..120: mol_type = other DNA
tcgctatagctcaaataccaaatataggcataggaattgctatcaatgacaagcttaatcgcgcaagctcatattaaccccagaataagacaagagaaagtataaaaggtatagaataaa

SEQ ID NO: 2491 - DNA, 120 bp, synthetic construct
  source 1..120: mol_type = other DNA
gcgcaagctcatattaaccccagaataagacaagagaaagtataaaaggtatagaataaaagatatacaaagataaaatgttgagttacaaagaaaatttaaataaaaataaaataactc

SEQ ID NO: 2492 - DNA, 120 bp, synthetic construct
  source 1..120: mol_type = other DNA
agatatacaaagataaaatgttgagttacaaagaaaatttaaataaaaataaaataactcaacatgaaaaaatgtattataacagtatactatttaatagataattcttgcaagatatat

SEQ ID NO: 2493 - DNA, 120 bp, synthetic construct
  source 1..120: mol_type = other DNA
aacatgaaaaaatgtattataacagtatactatttaatagataattcttgcaagatatatcaagagtgagaaagaaagagattaataccaagtaataatcaaaaaaaaacaaagatggaa

SEQ ID NO: 2494 - DNA, 120 bp, synthetic construct
  source 1..120: mol_type = other DNA
caagagtgagaaagaaagagattaataccaagtaataatcaaaaaaaaacaaagatggaaagttatttttaactgagttattaacaatactgatatattagacctctttcgaaactggtt

SEQ ID NO: 2495 - DNA, 120 bp, synthetic construct
  source 1..120: mol_type = other DNA
agttatttttaactgagttattaacaatactgatatattagacctctttcgaaactggttgacgttgttcaaaattatgaatgccagagatcaaattaaatctaagacctaatcttttac

SEQ ID NO: 2496 - DNA, 120 bp, synthetic construct
  source 1..120: mol_type = other DNA
gacgttgttcaaaattatgaatgccagagatcaaattaaatctaagacctaatcttttacgtctattttgatatttatcagcaataattttgaactacgtcaaccagtttcgaaagagat

SEQ ID NO: 2497 - DNA, 120 bp, synthetic construct
  source 1..120: mol_type = other DNA
gtctattttgatatttatcagcaataattttgaactacgtcaaccagtttcgaaagagatctatttttatttatctcaatgtaaggattttaaaaattattatctatattacttgtgtca

SEQ ID NO: 2498 - DNA, 120 bp, synthetic construct
  source 1..120: mol_type = other DNA
ctatttttatttatctcaatgtaaggattttaaaaattattatctatattacttgtgtcattaagtataaaaaagaaagctagtatacagtgcatgaccttaggataatagcctgaattt

SEQ ID NO: 2499 - DNA, 120 bp, synthetic construct
  source 1..120: mol_type = other DNA
aaaaattattatctatattacttgtgtcattaagtataaaaaagaaagctagtatacagtgcatgaccttaggataatagcctgaattttagataagtacctagcttttttgaaaactaa

SEQ ID NO: 2500 - DNA, 120 bp, synthetic construct
  source 1..120: mol_type = other DNA
aacccgcattataaaactatcggcagtttttctaatattatctaacataattttttgtctaagtttttaagtgagaatatgtcacacccgcggggcaatgcatcctcagcattacggaat

SEQ ID NO: 2501 - DNA, 120 bp, synthetic construct
  source 1..120: mol_type = other DNA
aagtttttaagtgagaatatgtcacacccgcggggcaatgcatcctcagcattacggaatgacatttaagcagcttctcaagactgcattataaagcaaaaaagcctatatagtcaaact

SEQ ID NO: 2502 - DNA, 120 bp, synthetic construct
  source 1..120: mol_type = other DNA
gacatttaagcagcttctcaagactgcattataaagcaaaaaagcctatatagtcaaactatataggcttttttattatttttgtagatgttcgatgtcatttctgtatggttcagtttt

SEQ ID NO: 2503 - DNA, 120 bp, synthetic construct
  source 1..120: mol_type = other DNA
atataggcttttttattatttttgtagatgttcgatgtcatttctgtatggttcagtttttctgtcattgcaatgaaattacaaagtaattgacgcagcaatctcagaagtttgttatta

SEQ ID NO: 2504 - DNA, 120 bp, synthetic construct
  source 1..120: mol_type = other DNA
tctgtcattgcaatgaaattacaaagtaattgacgcagcaatctcagaagtttgttattatttcatgagattgccacgcagcctatggcttgctcgcaatgacgacctagagcatattag

SEQ ID NO: 2505 - DNA, 120 bp, synthetic construct
  source 1..120: mol_type = other DNA
tttcatgagattgccacgcagcctatggcttgctcgcaatgacgacctagagcatattagaagtttatacgaacttttacactaccttgctgagtaaaatacttacttccgatattggta

SEQ ID NO: 2506 - DNA, 120 bp, synthetic construct
  source 1..120: mol_type = other DNA
aagtttatacgaacttttacactaccttgctgagtaaaatacttacttccgatattggtatcgtagttaataccgtattccatcatttgatgcttagcagtaataccaacaccgatatca

SEQ ID NO: 2507 - DNA, 120 bp, synthetic construct
  source 1..120: mol_type = other DNA
tcgtagttaataccgtattccatcatttgatgcttagcagtaataccaacaccgatatcaaagcttgttttgctttgcttaaagctgttggttgggaaaggagcaatcataccttgtaat

SEQ ID NO: 2508 - DNA, 120 bp, synthetic construct
  source 1..120: mol_type = other DNA
aagcttgttttgctttgcttaaagctgttggttgggaaaggagcaatcataccttgtaatctcgcatcaatcgccggaactttattcttgaatgcataatcaaccattgcgtacagctca

SEQ ID NO: 2509 - DNA, 120 bp, synthetic construct
  source 1..120: mol_type = other DNA
ctcgcatcaatcgccggaactttattcttgaatgcataatcaaccattgcgtacagctcaggagttaacactacttcacctacatttatattacttaataccttagcaccgagtaaacca

SEQ ID NO: 2510 - DNA, 120 bp, synthetic construct
  source 1..120: mol_type = other DNA
ggagttaacactacttcacctacatttatattacttaataccttagcaccgagtaaaccatcgaaagtgttatagttcttgcctttaactgtaagatttttgttagtagtaccggtttct

SEQ ID NO: 2511 - DNA, 120 bp, synthetic construct
  source 1..120: mol_type = other DNA
tcgaaagtgttatagttcttgcctttaactgtaagatttttgttagtagtaccggtttctttataacccttatctttgatagccgaatatctaagcccaactagaggtgttaagctaatg

SEQ ID NO: 2512 - DNA, 120 bp, synthetic construct
  source 1..120: mol_type = other DNA
ttataacccttatctttgatagccgaatatctaagcccaactagaggtgttaagctaatgttttcacgcaccatataggtataaccagccattaactaacctgtatagctttctgattta

SEQ ID NO: 2513 - DNA, 120 bp, synthetic construct
  source 1..120: mol_type = other DNA
ttttcacgcaccatataggtataaccagccattaactaacctgtatagctttctgatttatacttaccgcttgcggtttgatagccgacagtctctagtgccgtcgcaataacacatctt

SEQ ID NO: 2514 - DNA, 120 bp, synthetic construct
  source 1..120: mol_type = other DNA
tacttaccgcttgcggtttgatagccgacagtctctagtgccgtcgcaataacacatcttgatttgcttcttatcttgttatcagagtaagatgctatagctttaacgcaaagatttgca

SEQ ID NO: 2515 - DNA, 120 bp, synthetic construct
  source 1..120: mol_type = other DNA
gatttgcttcttatcttgttatcagagtaagatgctatagctttaacgcaaagatttgcataaggtacgttatataaaccgtataaagagtaaatattactctctacctcattcttatca

SEQ ID NO: 2516 - DNA, 120 bp, synthetic construct
  source 1..120: mol_type = other DNA
taaggtacgttatataaaccgtataaagagtaaatattactctctacctcattcttatcacctgtcttattatttttcagtttgatatcagtatcggctccagctcttgtatatgcaagt

SEQ ID NO: 2517 - DNA, 120 bp, synthetic construct
  source 1..120: mol_type = other DNA
cctgtcttattatttttcagtttgatatcagtatcggctccagctcttgtatatgcaagtccgagtgctaaatcatccttaactaagccatcaaaacctatagtaccaccgattgtatca

SEQ ID NO: 2518 - DNA, 120 bp, synthetic construct
  source 1..120: mol_type = other DNA
ccgagtgctaaatcatccttaactaagccatcaaaacctatagtaccaccgattgtatcagacttataaccgcttatattgttatgcatcttctgcattgcattaccgacaaatgagctc

SEQ ID NO: 2519 - DNA, 120 bp, synthetic construct
  source 1..120: mol_type = other DNA
gacttataaccgcttatattgttatgcatcttctgcattgcattaccgacaaatgagctccaaacttagcatctctgccctcatcacaagcagctacagcaaccggctctattgcatcca

SEQ ID NO: 2520 - DNA, 120 bp, synthetic construct
  source 1..120: mol_type = other DNA
caaacttagcatctctgccctcatcacaagcagctacagcaaccggctctattgcatccattctagcatttagattaattaagctacttgagatattactgagtataacttgattattaa

SEQ ID NO: 2521 - DNA, 120 bp, synthetic construct
  source 1..120: mol_type = other DNA
ttctagcatttagattaattaagctacttgagatattactgagtataacttgattattaatagcagctatagtatcgctaagctttacaacgtcttgcatgagctgagttacagtatctg

SEQ ID NO: 2522 - DNA, 120 bp, synthetic construct
  source 1..120: mol_type = other DNA
tagcagctatagtatcgctaagctttacaacgtcttgcatgagctgagttacagtatctgcttcttggattggactcagtttaccccaattatcgaaagctcaacatgcatctgaacctc

SEQ ID NO: 2523 - DNA, 120 bp, synthetic construct
  source 1..120: mol_type = other DNA
cttcttggattggactcagtttaccccaattatcgaaagctcaacatgcatctgaacctctttgtgcttgctccattaactcaagcgatttctttacatttgcagcatttgtgatatttg

SEQ ID NO: 2524 - DNA, 120 bp, synthetic construct
  source 1..120: mol_type = other DNA
tttgtgcttgctccattaactcaagcgatttctttacatttgcagcatttgtgatatttgcaagcggcccaccaggtttaaaatatgcttctatcacttcttccgccatatcctctgcaa

SEQ ID NO: 2525 - DNA, 120 bp, synthetic construct
  source 1..120: mol_type = other DNA
caagcggcccaccaggtttaaaatatgcttctatcacttcttccgccatatcctctgcaaataacgtcaaagtcgattcatcaaaagtaaagttgacaaagcggttgtaattattaacgg

SEQ ID NO: 2526 - DNA, 120 bp, synthetic construct
  source 1..120: mol_type = other DNA
ataacgtcaaagtcgattcatcaaaagtaaagttgacaaagcggttgtaattattaacggttactttaacattacctgcgggagtaggctttcatccgcctgctgtttctgaagatatta

SEQ ID NO: 2527 - DNA, 120 bp, synthetic construct
  source 1..120: mol_type = other DNA
ttactttaacattacctgcgggagtaggctttcatccgcctgctgtttctgaagatattaccgtatattttgtatccgggcttatattattaatgtcaaaattagtagcagtaacaacaa

SEQ ID NO: 2528 - DNA, 120 bp, synthetic construct
  source 1..120: mol_type = other DNA
ccgtatattttgtatccgggcttatattattaatgtcaaaattagtagcagtaacaacaagttctaaagttgaaactcctgataaatcaagagtactacctgatttaattaagatattac

SEQ ID NO: 2529 - DNA, 120 bp, synthetic construct
  source 1..120: mol_type = other DNA
gttctaaagttgaaactcctgataaatcaagagtactacctgatttaattaagatattaccgtctaacttatctgcaccatcaaaagtagtatttaaggttagtgtatcggtaaagctac

SEQ ID NO: 2530 - DNA, 120 bp, synthetic construct
  source 1..120: mol_type = other DNA
cgtctaacttatctgcaccatcaaaagtagtatttaaggttagtgtatcggtaaagctaccggtaccggtatatgttatttggcttgcacctaaagtaagtgtagtaccgctacctgtta

SEQ ID NO: 2531 - DNA, 120 bp, synthetic construct
  source 1..120: mol_type = other DNA
cggtaccggtatatgttatttggcttgcacctaaagtaagtgtagtaccgctacctgttatattactattaaaagctaggctattaccgaaattaatagtagcattgttaactgcaaagc

SEQ ID NO: 2532 - DNA, 120 bp, synthetic construct
  source 1..120: mol_type = other DNA
tattactattaaaagctaggctattaccgaaattaatagtagcattgttaactgcaaagctggtagccgttacatttttagcaaaattagtgatagaagctttagctaaagtaactgcac

SEQ ID NO: 2533 - DNA, 120 bp, synthetic construct
  source 1..120: mol_type = other DNA
tggtagccgttacatttttagcaaaattagtgatagaagctttagctaaagtaactgcaccagtgttagtaaatgtatcggcaaaacttgtagtaccgcagagcgtcgccgtaccttttg

SEQ ID NO: 2534 - DNA, 120 bp, synthetic construct
  source 1..120: mol_type = other DNA
cagtgttagtaaatgtatcggcaaaacttgtagtaccgcagagcgtcgccgtaccttttgcattaacactgcttgcaaagtttattatgcctgccgttgtgatatcacccaccgaattag

SEQ ID NO: 2535 - DNA, 120 bp, synthetic construct
  source 1..120: mol_type = other DNA
cattaacactgcttgcaaagtttattatgcctgccgttgtgatatcacccaccgaattagccacagtccctacaacaccactaacactgccgccattcgtgaagtttaacttcagagcct

SEQ ID NO: 2536 - DNA, 120 bp, synthetic construct
  source 1..120: mol_type = other DNA
ccacagtccctacaacaccactaacactgccgccattcgtgaagtttaacttcagagcctgaccaccggttttatttatgctgcctgttaagttaaagtttgcaggtaatgtgaagagtg

SEQ ID NO: 2537 - DNA, 120 bp, synthetic construct
  source 1..120: mol_type = other DNA
gaccaccggttttatttatgctgcctgttaagttaaagtttgcaggtaatgtgaagagtgcagtaccgttaccttggatttcagtgatgctagcattaccgccttgggttatgcttacag

SEQ ID NO: 2538 - DNA, 120 bp, synthetic construct
  source 1..120: mol_type = other DNA
cagtaccgttaccttggatttcagtgatgctagcattaccgccttgggttatgcttacagccccggcacctacttttaacatagcaatattattaatagtacttgcaacagttgcgatga

SEQ ID NO: 2539 - DNA, 120 bp, synthetic construct
  source 1..120: mol_type = other DNA
ccccggcacctacttttaacatagcaatattattaatagtacttgcaacagttgcgatgattgtaccattaactctgttactgcttgtaatactaccggttatatttttatttgcaccaa

SEQ ID NO: 2540 - DNA, 120 bp, synthetic construct
  source 1..120: mol_type = other DNA
ttgtaccattaactctgttactgcttgtaatactaccggttatatttttatttgcaccaagtattataactgctgcttgattattgaaatctacactatcgttaatattaccgttttgag

SEQ ID NO: 2541 - DNA, 120 bp, synthetic construct
  source 1..120: mol_type = other DNA
gtattataactgctgcttgattattgaaatctacactatcgttaatattaccgttttgagttaaagcagtagcagcaccgaatgataaattagagttgatatccttattatagccggcac

SEQ ID NO: 2542 - DNA, 120 bp, synthetic construct
  source 1..120: mol_type = other DNA
ttaaagcagtagcagcaccgaatgataaattagagttgatatccttattatagccggcactgataattctaaattgttagcaaatatatcagtatctatttagaatgtgctgtttcctct

SEQ ID NO: 2543 - DNA, 120 bp, synthetic construct
  source 1..120: mol_type = other DNA
tgataattctaaattgttagcaaatatatcagtatctatttagaatgtgctgtttcctctaaattctaatgcttttaatttatttactacagtaccgtaagtagcatttccgacatttgt

SEQ ID NO: 2544 - DNA, 120 bp, synthetic construct
  source 1..120: mol_type = other DNA
aaattctaatgcttttaatttatttactacagtaccgtaagtagcatttccgacatttgtaagaattacttgcccgcccgcagctcctgaatctacagcaagtttacctttatttggatc

SEQ ID NO: 2545 - DNA, 120 bp, synthetic construct
  source 1..120: mol_type = other DNA
aagaattacttgcccgcccgcagctcctgaatctacagcaagtttacctttatttggatctccaggatcaagtgtggcatttaatgttattgtactatcaccggctgcactattttgtaa

SEQ ID NO: 2546 - DNA, 120 bp, synthetic construct
  source 1..120: mol_type = other DNA
tccaggatcaagtgtggcatttaatgttattgtactatcaccggctgcactattttgtaatactaactctgcatcttcatggacaaaattgatagtctgaccgtttgcgaaaattcctac

SEQ ID NO: 2547 - DNA, 120 bp, synthetic construct
  source 1..120: mol_type = other DNA
tactaactctgcatcttcatggacaaaattgatagtctgaccgtttgcgaaaattcctacattagcgccatttgcatcaatcgtataagaaccagcagcggcaggaagtccaagactcgc

SEQ ID NO: 2548 - DNA, 120 bp, synthetic construct
  source 1..120: mol_type = other DNA
attagcgccatttgcatcaatcgtataagaaccagcagcggcaggaagtccaagactcgcatttgctgcacctatatttattacattaatttggttagtaataccgcatacatcaacaaa

SEQ ID NO: 2549 - DNA, 120 bp, synthetic construct
  source 1..120: mol_type = other DNA
atttgctgcacctatatttattacattaatttggttagtaataccgcatacatcaacaaactgcatagtatttatgatattaaatgcgagaacatttgtagtatctatattattaaaggc

SEQ ID NO: 2550 - DNA, 120 bp, synthetic construct
  source 1..120: mol_type = other DNA
ctgcatagtatttatgatattaaatgcgagaacatttgtagtatctatattattaaaggctacattccctaaaacatttaatgatgctagttcatttcctgccgtacatattgctttagc

SEQ ID NO: 2551 - DNA, 120 bp, synthetic construct
  source 1..120: mol_type = other DNA
tacattccctaaaacatttaatgatgctagttcatttcctgccgtacatattgctttagctgcacaatcatcttgtaaggttataaggttttctgtaccaagaagaagtaacataccacc

SEQ ID NO: 2552 - DNA, 120 bp, synthetic construct
  source 1..120: mol_type = other DNA
tgcacaatcatcttgtaaggttataaggttttctgtaccaagaagaagtaacataccaccaccggttgtaaacgccggtaaatcatttttaatacaactctatcatctgtagcactattg

SEQ ID NO: 2553 - DNA, 120 bp, synthetic construct
  source 1..120: mol_type = other DNA
accggttgtaaacgccggtaaatcatttttaatacaactctatcatctgtagcactattgttaactaaaaaaagctttgagtttgcacctttaaaatcaataacttgagcgtttaatatc

SEQ ID NO: 2554 - DNA, 120 bp, synthetic construct
  source 1..120: mol_type = other DNA
ttaactaaaaaaagctttgagtttgcacctttaaaatcaataacttgagcgtttaatatctcaatatcagcgttcttaacatttattgcaaaagtcttattatcttgaatgttaatttgt

SEQ ID NO: 2555 - DNA, 120 bp, synthetic construct
  source 1..120: mol_type = other DNA
tcaatatcagcgttcttaacatttattgcaaaagtcttattatcttgaatgttaatttgtgcaaccgtcccgatactagcattatctgcagtaaccaaaccgagagtattaatattaatt

SEQ ID NO: 2556 - DNA, 120 bp, synthetic construct
  source 1..120: mol_type = other DNA
gcaaccgtcccgatactagcattatctgcagtaaccaaaccgagagtattaatattaattgtagcattattactgtttgctatagttctgcttaatgtataactcttaccgacaggaccg

SEQ ID NO: 2557 - DNA, 120 bp, synthetic construct
  source 1..120: mol_type = other DNA
gtagcattattactgtttgctatagttctgcttaatgtataactcttaccgacaggaccgttcaattctaaagtacccccctgagcattcacaccgaaattgatatttgtagctatcaaa

SEQ ID NO: 2558 - DNA, 120 bp, synthetic construct
  source 1..120: mol_type = other DNA
ttcaattctaaagtacccccctgagcattcacaccgaaattgatatttgtagctatcaaattaccgccgacttgtatcgtaccgactgctccaccaccggcaatatcatcaaaatttacg

SEQ ID NO: 2559 - DNA, 120 bp, synthetic construct
  source 1..120: mol_type = other DNA
ttaccgccgacttgtatcgtaccgactgctccaccaccggcaatatcatcaaaatttacgatttgtgcataaatatcacttgtaaaacaagatccgcagcaccattatcaactttagcat

SEQ ID NO: 2560 - DNA, 120 bp, synthetic construct
  source 1..120: mol_type = other DNA
atttgtgcataaatatcacttgtaaaacaagatccgcagcaccattatcaactttagcattcagaacttttagagatgctgcatttgtacctaccgagccggtaacccatactccagcgt

SEQ ID NO: 2561 - DNA, 120 bp, synthetic construct
  source 1..120: mol_type = other DNA
tcagaacttttagagatgctgcatttgtacctaccgagccggtaacccatactccagcgttgttgcacttattgctcctactgtacttactccgcctgcattaccgttattaaacgttac

SEQ ID NO: 2562 - DNA, 120 bp, synthetic construct
  source 1..120: mol_type = other DNA
tgttgcacttattgctcctactgtacttactccgcctgcattaccgttattaaacgttacggcatacaaagttttggtccaagcgattgctccggtaaaacttgttcgagtattaacagt

SEQ ID NO: 2563 - DNA, 120 bp, synthetic construct
  source 1..120: mol_type = other DNA
ggcatacaaagttttggtccaagcgattgctccggtaaaacttgttcgagtattaacagttatttcactatgatcatgatcatcactatctatagctactgcaatctttattaatgctag

SEQ ID NO: 2564 - DNA, 120 bp, synthetic construct
  source 1..120: mol_type = other DNA
tatttcactatgatcatgatcatcactatctatagctactgcaatctttattaatgctagagttgcagattgtatagttaagcctgcagtggcaccgcctatggtaatagctcctcaacc

SEQ ID NO: 2565 - DNA, 120 bp, synthetic construct
  source 1..120: mol_type = other DNA
agttgcagattgtatagttaagcctgcagtggcaccgcctatggtaatagctcctcaacctatataatcagcagcagcatcaaaaccatgatttgcagcaactgcttcagtaccggttaa

SEQ ID NO: 2566 - DNA, 120 bp, synthetic construct
  source 1..120: mol_type = other DNA
tatataatcagcagcagcatcaaaaccatgatttgcagcaactgcttcagtaccggttaaaattaagcttttgccgtcagtgatagtaacaggcaacaagttatcacatgtaacaataga

SEQ ID NO: 2567 - DNA, 120 bp, synthetic construct
  source 1..120: mol_type = other DNA
aattaagcttttgccgtcagtgatagtaacaggcaacaagttatcacatgtaacaatagaactgacgctagtattttgagtaatatttagagctacttgaatagtacctgcaacatttat

SEQ ID NO: 2568 - DNA, 120 bp, synthetic construct
  source 1..120: mol_type = other DNA
actgacgctagtattttgagtaatatttagagctacttgaatagtacctgcaacatttatagcagtaataatacgatctgcttcatctgcagtgatagtatgatcaccaccgtaagtaaa

SEQ ID NO: 2569 - DNA, 120 bp, synthetic construct
  source 1..120: mol_type = other DNA
agcagtaataatacgatctgcttcatctgcagtgatagtatgatcaccaccgtaagtaaatgcatcatcgtcttgaggaccgtcagaaggatgaccattagcggctcctccagccgttat

SEQ ID NO: 2570 - DNA, 120 bp, synthetic construct
  source 1..120: mol_type = other DNA
tgcatcatcgtcttgaggaccgtcagaaggatgaccattagcggctcctccagccgttatatcattcaaattattggcaacagcaaaatcactaaatactgcatcattaacagaaataaa

SEQ ID NO: 2571 - DNA, 120 bp, synthetic construct
  source 1..120: mol_type = other DNA
atcattcaaattattggcaacagcaaaatcactaaatactgcatcattaacagaaataaaaccagaagcgacaccacatgccacgctaccactcagcattatcgctgcggttgaggtagt

SEQ ID NO: 2572 - DNA, 120 bp, synthetic construct
  source 1..120: mol_type = other DNA
accagaagcgacaccacatgccacgctaccactcagcattatcgctgcggttgaggtagtgaataaagctgttttaagacttttttgaattgctttttgaaataattttggagaaatatt

SEQ ID NO: 2573 - DNA, 120 bp, synthetic construct
  source 1..120: mol_type = other DNA
gaataaagctgttttaagacttttttgaattgctttttgaaataattttggagaaatattcaccataatgtaaactttaataaaaattaaataatttaataattaaatataagtgtttaa

SEQ ID NO: 2574 - DNA, 120 bp, synthetic construct
  source 1..120: mol_type = other DNA
caccataatgtaaactttaataaaaattaaataatttaataattaaatataagtgtttaaatatgtctattataattaataattatatacaatattttacaaatttatatgcggcatttg

SEQ ID NO: 2575 - DNA, 120 bp, synthetic construct
  source 1..120: mol_type = other DNA
atatgtctattataattaataattatatacaatattttacaaatttatatgcggcatttgcattctgcaggggcggtagctttgttgcatagatcggtaaaacctactcaatgtcattcc

SEQ ID NO: 2576 - DNA, 120 bp, synthetic construct
  source 1..120: mol_type = other DNA
cattctgcaggggcggtagctttgttgcatagatcggtaaaacctactcaatgtcattcccgcgtaagcagaaccttgttgcatggttcgagaaatctactgagtagtagaccgtgctca

SEQ ID NO: 2577 - DNA, 120 bp, synthetic construct
  source 1..120: mol_type = other DNA
cgcgtaagcagaaccttgttgcatggttcgagaaatctactgagtagtagaccgtgctcaaaccacggggtgacagctaaaagtactggatccacactttcactgggataacattaagaa

SEQ ID NO: 2578 - DNA, 120 bp, synthetic construct
  source 1..120: mol_type = other DNA
aaccacggggtgacagctaaaagtactggatccacactttcactgggataacattaagaatacgagaataacatttacctctcaggcagtaatatctccctcttacctgtatgattcggt

SEQ ID NO: 2579 - DNA, 120 bp, synthetic construct
  source 1..120: mol_type = other DNA
tacgagaataacatttacctctcaggcagtaatatctccctcttacctgtatgattcggtggtgagactattccatctttctccatcttctcaactaagttggcagctttgttatagccg

SEQ ID NO: 2580 - DNA, 120 bp, synthetic construct
  source 1..120: mol_type = other DNA
ggtgagactattccatctttctccatcttctcaactaagttggcagctttgttatagccgattctaagcgacctttggatatagctaatggaagatttacgttcgtcacgcactatctga

SEQ ID NO: 2581 - DNA, 120 bp, synthetic construct
  source 1..120: mol_type = other DNA
attctaagcgacctttggatatagctaatggaagatttacgttcgtcacgcactatctgaacagcttttttgtaaagcactgcatcagacgtgccatcaacgatatcaattctactatcg

SEQ ID NO: 2582 - DNA, 120 bp, synthetic construct
  source 1..120: mol_type = other DNA
acagcttttttgtaaagcactgcatcagacgtgccatcaacgatatcaattctactatcgtcttcttcaggctgctcggtaacggcagagatatattcaggcgcaccggtctctttcaaa

SEQ ID NO: 2583 - DNA, 120 bp, synthetic construct
  source 1..120: mol_type = other DNA
tcttcttcaggctgctcggtaacggcagagatatattcaggcgcaccggtctctttcaaatatcctgtaattttctcgatttcaacttcattaacaaacggtccatgtaccctacttatc

SEQ ID NO: 2584 - DNA, 120 bp, synthetic construct
  source 1..120: mol_type = other DNA
tatcctgtaattttctcgatttcaacttcattaacaaacggtccatgtaccctacttatctttgcagtattccccataaatagcatatcacccatacctagtaactgctcggagccttgc

SEQ ID NO: 2585 - DNA, 120 bp, synthetic construct
  source 1..120: mol_type = other DNA
tttgcagtattccccataaatagcatatcacccatacctagtaactgctcggagccttgctcgcctaaaatcgttcggctatcgattttagatgtaactttaaagctaatacgacttggg

SEQ ID NO: 2586 - DNA, 120 bp, synthetic construct
  source 1..120: mol_type = other DNA
tcgcctaaaatcgttcggctatcgattttagatgtaactttaaagctaatacgacttgggaaattggctttaatgacaccggtaataacgtctacagaaggtctttgcgttgccatgata

SEQ ID NO: 2587 - DNA, 120 bp, synthetic construct
  source 1..120: mol_type = other DNA
aaattggctttaatgacaccggtaataacgtctacagaaggtctttgcgttgccatgataatatggatacctgccgctcttgccatttgagcaagcctttgaatcagcatttcaatatcc

SEQ ID NO: 2588 - DNA, 120 bp, synthetic construct
  source 1..120: mol_type = other DNA
atatggatacctgccgctcttgccatttgagcaagcctttgaatcagcatttcaatatccttaccggcaactagcattaaatcagccatctcatcaacaataaccacaatgtaaggtagt

SEQ ID NO: 2589 - DNA, 120 bp, synthetic construct
  source 1..120: mol_type = other DNA
ttaccggcaactagcattaaatcagccatctcatcaacaataaccacaatgtaaggtagtttctccatattcatcgtaacggtttcgtaaataggcttacctgtttcaggatcaaaaccc

SEQ ID NO: 2590 - DNA, 120 bp, synthetic construct
  source 1..120: mol_type = other DNA
ttctccatattcatcgtaacggtttcgtaaataggcttacctgtttcaggatcaaaacccgtttgaatcgaacgctcaattactctattctctttcaccgcttctaagatttttgcattg

SEQ ID NO: 2591 - DNA, 120 bp, synthetic construct
  source 1..120: mol_type = other DNA
gtttgaatcgaacgctcaattactctattctctttcaccgcttctaagatttttgcattgtaacctgcaatattcttaacaccgatattgctcataattctatagcggttttccatttcc

SEQ ID NO: 2592 - DNA, 120 bp, synthetic construct
  source 1..120: mol_type = other DNA
taacctgcaatattcttaacaccgatattgctcataattctatagcggttttccatttccttaaccgcccatttaagagcaactacagccttagaaggttcagttactacaggagtgagt

SEQ ID NO: 2593 - DNA, 120 bp, synthetic construct
  source 1..120: mol_type = other DNA
ttaaccgcccatttaagagcaactacagccttagaaggttcagttactacaggagtgagtaaatggggtattccgtcataagcggataattcaagcattttcgggtcaatcatgataaag

SEQ ID NO: 2594 - DNA, 120 bp, synthetic construct
  source 1..120: mol_type = other DNA
aaatggggtattccgtcataagcggataattcaagcattttcgggtcaatcatgataaagcggcattcttcaggagtatagcggtataagagcgaaactatcatcgcgttaatcccaact

SEQ ID NO: 2595 - DNA, 120 bp, synthetic construct
  source 1..120: mol_type = other DNA
cggcattcttcaggagtatagcggtataagagcgaaactatcatcgcgttaatcccaactgatttaccagaaccggttgttcctgcaacaagcaagtgaggcatcttcgcaagatcggca

SEQ ID NO: 2596 - DNA, 120 bp, synthetic construct
  source 1..120: mol_type = other DNA
gatttaccagaaccggttgttcctgcaacaagcaagtgaggcatcttcgcaagatcggcaatcagtggcttaccgactaaatctttacctaagactaacggtaataaagttgatttgtct

SEQ ID NO: 2597 - DNA, 120 bp, synthetic construct
  source 1..120: mol_type = other DNA
atcagtggcttaccgactaaatctttacctaagactaacggtaataaagttgatttgtcttggtattcaggcgtctctatcaactctttcacacaaaagaattcacgctgcttattaggg

SEQ ID NO: 2598 - DNA, 120 bp, synthetic construct
  source 1..120: mol_type = other DNA
tggtattcaggcgtctctatcaactctttcacacaaaagaattcacgctgcttattagggagctcaataccaagtacgtttttgccgggtattaccgctatccttgttgataaagcagat

SEQ ID NO: 2599 - DNA, 120 bp, synthetic construct
  source 1..120: mol_type = other DNA
agctcaataccaagtacgtttttgccgggtattaccgctatccttgttgataaagcagatagtgagcgtgctatatcgtcagataatcctactactcttgatgttttagtaccagctgcc

SEQ ID NO: 2600 - DNA, 120 bp, synthetic construct
  source 1..120: mol_type = other DNA
agtgagcgtgctatatcgtcagataatcctactactcttgatgttttagtaccagctgccggctcaaactcatattgagttaccaccggtccttgattgatattaattatatgcccttta

SEQ ID NO: 2601 - DNA, 120 bp, synthetic construct
  source 1..120: mol_type = other DNA
gatgttttagtaccagctgccggctcaaactcatattgagttaccaccggtccttgattgatattaattatatgccctttaactccaaaatcattcagcacggttagtagctcctcggct

SEQ ID NO: 2602 - DNA, 120 bp, synthetic construct
  source 1..120: mol_type = other DNA
gaagcaatctcaggatatttgacgagattgccacgttgcttcgctcctcgcaatgacgcttctcaaaactacattataaagcaaaaaagcctatatagtcaaactatataggcttttttt

SEQ ID NO: 2603 - DNA, 120 bp, synthetic construct
  source 1..120: mol_type = other DNA
tctcaaaactacattataaagcaaaaaagcctatatagtcaaactatataggctttttttatgattatagaacggttaattaaaaattaacacgaactttcacactaccttgctgagcga

SEQ ID NO: 2604 - DNA, 120 bp, synthetic construct
  source 1..120: mol_type = other DNA
atgattatagaacggttaattaaaaattaacacgaactttcacactaccttgctgagcgaaatacttacttccgatattggtatcgtagttaatcccgtattccatcattttatgcttag

SEQ ID NO: 2605 - DNA, 120 bp, synthetic construct
  source 1..120: mol_type = other DNA
aatacttacttccgatattggtatcgtagttaatcccgtattccatcattttatgcttagcagtaacaccgacaccaacatcaaaacttgttttgctttgcttaaagctgttggttggaa

SEQ ID NO: 2606 - DNA, 120 bp, synthetic construct
  source 1..120: mol_type = other DNA
cagtaacaccgacaccaacatcaaaacttgttttgctttgcttaaagctgttggttggaagaggagcagtcataccttgtaatcttgcatcaatcgccgaaactttattcttgaatgcat

SEQ ID NO: 2607 - DNA, 120 bp, synthetic construct
  source 1..120: mol_type = other DNA
gaggagcagtcataccttgtaatcttgcatcaatcgccgaaactttattcttgaatgcataatcgaccattgcgtaaagctcaggtgttagcactatttcattgacattgatattacttg

SEQ ID NO: 2608 - DNA, 120 bp, synthetic construct
  source 1..120: mol_type = other DNA
aatcgaccattgcgtaaagctcaggtgttagcactatttcattgacattgatattacttgatactttagcaccgagtaaaccgtcgaaagtattatagttcttgcctttaacggtaagat

SEQ ID NO: 2609 - DNA, 120 bp, synthetic construct
  source 1..120: mol_type = other DNA
atactttagcaccgagtaaaccgtcgaaagtattatagttcttgcctttaacggtaagattttggtaagtagtaccggtttccttatagctcttatctttgatagtcgaatatctaagcc

SEQ ID NO: 2610 - DNA, 120 bp, synthetic construct
  source 1..120: mol_type = other DNA
tttggtaagtagtaccggtttccttatagctcttatctttgatagtcgaatatctaagcccagctaacggtgttaagttaatgttctcagacatcatataggtataaccagccattaact

SEQ ID NO: 2611 - DNA, 120 bp, synthetic construct
  source 1..120: mol_type = other DNA
cagctaacggtgttaagttaatgttctcagacatcatataggtataaccagccattaactgacctgtatagctttcggatttatacttaccgtttgcagtttgataaccgacagtctcta

SEQ ID NO: 2612 - DNA, 120 bp, synthetic construct
  source 1..120: mol_type = other DNA
gacctgtatagctttcggatttatacttaccgtttgcagtttgataaccgacagtctctagtgttgttgcaataacacgtcttgatttgcttcttatcttattatctgagtaagatgcta

SEQ ID NO: 2613 - DNA, 120 bp, synthetic construct
  source 1..120: mol_type = other DNA
gtgttgttgcaataacacgtcttgatttgcttcttatcttattatctgagtaagatgctatagcttcaacgaagagattttcataaggtacactatataaaccgtataaagaatagatgt

SEQ ID NO: 2614 - DNA, 120 bp, synthetic construct
  source 1..120: mol_type = other DNA
tagcttcaacgaagagattttcataaggtacactatataaaccgtataaagaatagatgttgctctctaccttattcttatcgcccgttttattattttttagcttaatgtcagtatcgg

SEQ ID NO: 2615 - DNA, 120 bp, synthetic construct
  source 1..120: mol_type = other DNA
tgctctctaccttattcttatcgcccgttttattattttttagcttaatgtcagtatcggctcttgtatatgcaagtccgagtactagatcatcgctaacgaagccgtcaaaacctatag

SEQ ID NO: 2616 - DNA, 120 bp, synthetic construct
  source 1..120: mol_type = other DNA
ctcttgtatatgcaagtccgagtactagatcatcgctaacgaagccgtcaaaacctatagtgccaccagttgtatcagacttataaccacttatactattacacatcttctgcgttgcat

SEQ ID NO: 2617 - DNA, 120 bp, synthetic construct
  source 1..120: mol_type = other DNA
tgccaccagttgtatcagacttataaccacttatactattacacatcttctgcgttgcattaccgacaaacgggcttatccacgcaccaaacttagcatccatatcttcatcaccagaag

SEQ ID NO: 2618 - DNA, 120 bp, synthetic construct
  source 1..120: mol_type = other DNA
taccgacaaacgggcttatccacgcaccaaacttagcatccatatcttcatcaccagaagaaacaggacctttattccctgcttgtactttatccattctagcatttagagcagttatat

SEQ ID NO: 2619 - DNA, 120 bp, synthetic construct
  source 1..120: mol_type = other DNA
aaacaggacctttattccctgcttgtactttatccattctagcatttagagcagttatattacttgatatattactcgctacaacttgattattaacggcagctatagtgtcgctaggtt

SEQ ID NO: 2620 - DNA, 120 bp, synthetic construct
  source 1..120: mol_type = other DNA
tacttgatatattactcgctacaacttgattattaacggcagctatagtgtcgctaggttttacaacatcttgcatgagatgagttgtagcatctgcttcctgtagcggtgtcattagac

SEQ ID NO: 2621 - DNA, 120 bp, synthetic construct
  source 1..120: mol_type = other DNA
ttacaacatcttgcatgagatgagttgtagcatctgcttcctgtagcggtgtcattagaccaaagttattgaaagcttgacgtgcatctgaaccattgggagcatcctccattaactcaa

SEQ ID NO: 2622 - DNA, 120 bp, synthetic construct
  source 1..120: mol_type = other DNA
caaagttattgaaagcttgacgtgcatctgaaccattgggagcatcctccattaactcaagcgatttctttatatttgcagcatttgggatatttgcaagcggtccacccggtgcaaaat

SEQ ID NO: 2623 - DNA, 120 bp, synthetic construct
  source 1..120: mol_type = other DNA
gcgatttctttatatttgcagcatttgggatatttgcaagcggtccacccggtgcaaaatcttcatctataacacctgcagctatatcctctgcaaataacgttaaagtcgatgcatcaa

SEQ ID NO: 2624 - DNA, 120 bp, synthetic construct
  source 1..120: mol_type = other DNA
cttcatctataacacctgcagctatatcctctgcaaataacgttaaagtcgatgcatcaaaagtaaagtcaacaaaacggttgtcattattaatagttattttaacattctctttaggag

SEQ ID NO: 2625 - DNA, 120 bp, synthetic construct
  source 1..120: mol_type = other DNA
aagtaaagtcaacaaaacggttgtcattattaatagttattttaacattctctttaggagtaggctttaaaccacctgctgtttctgcagatattaccgtatattttgtatctgggctta

SEQ ID NO: 2626 - DNA, 120 bp, synthetic construct
  source 1..120: mol_type = other DNA
taggctttaaaccacctgctgtttctgcagatattaccgtatattttgtatctgggcttatattattcatgtcgaaattagtagcagtaacaacaagtgctaaatttgaaacccctgata

SEQ ID NO: 2627 - DNA, 120 bp, synthetic construct
  source 1..120: mol_type = other DNA
tattattcatgtcgaaattagtagcagtaacaacaagtgctaaatttgaaacccctgataaatcaagagtactacctgatttaattaagatattaccacctgacttagctgctccgtcaa

SEQ ID NO: 2628 - DNA, 120 bp, synthetic construct
  source 1..120: mol_type = other DNA
aatcaagagtactacctgatttaattaagatattaccacctgacttagctgctccgtcaaaagtagtatttaaggttagcgtatcggtaaagctaccggtaccagtatatgttacttgat

SEQ ID NO: 2629 - DNA, 120 bp, synthetic construct
  source 1..120: mol_type = other DNA
aagtagtatttaaggttagcgtatcggtaaagctaccggtaccagtatatgttacttgatttgcacctaaagtaagtgtagtaccgctacctgttatattactattaaaggctaggctat

SEQ ID NO: 2630 - DNA, 120 bp, synthetic construct
  source 1..120: mol_type = other DNA
ttgcacctaaagtaagtgtagtaccgctacctgttatattactattaaaggctaggctattgccgaaattaatagtagcactgttagctacaaagctggtagccgttacatttttagcaa

SEQ ID NO: 2631 - DNA, 120 bp, synthetic construct
  source 1..120: mol_type = other DNA
tgccgaaattaatagtagcactgttagctacaaagctggtagccgttacatttttagcaaaactagtgatagaacctttggctaaagtaaccgcacctgtattagtgaatgtatgggcaa

SEQ ID NO: 2632 - DNA, 120 bp, synthetic construct
  source 1..120: mol_type = other DNA
aactagtgatagaacctttggctaaagtaaccgcacctgtattagtgaatgtatgggcaaaacttgtagtaccgccaagtgtcgccgtaccttttgcgttaacactgcttgcaaaacttg

SEQ ID NO: 2633 - DNA, 120 bp, synthetic construct
  source 1..120: mol_type = other DNA
aacttgtagtaccgccaagtgtcgccgtaccttttgcgttaacactgcttgcaaaacttgtagcacctgccgttgtgatatcaccaaccgaattagccgcagtccctacaacaccgctaa

SEQ ID NO: 2634 - DNA, 120 bp, synthetic construct
  source 1..120: mol_type = other DNA
tagcacctgccgttgtgatatcaccaaccgaattagccgcagtccctacaacaccgctaacactaccgccattcatgaagtttagcttcagagcctgaccaccggttttatttatgctgc

SEQ ID NO: 2635 - DNA, 120 bp, synthetic construct
  source 1..120: mol_type = other DNA
cactaccgccattcatgaagtttagcttcagagcctgaccaccggttttatttatgctgcctgttaacttaaagtgtgcaggtaatgttaaagtatttgtacctgtaccttggatttcgc

SEQ ID NO: 2636 - DNA, 120 bp, synthetic construct
  source 1..120: mol_type = other DNA
ctgttaacttaaagtgtgcaggtaatgttaaagtatttgtacctgtaccttggatttcgccaattttaacgttaccgcctttggcaatagttacatttcctgcacctacttttaacatag

SEQ ID NO: 2637 - DNA, 120 bp, synthetic construct
  source 1..120: mol_type = other DNA
caattttaacgttaccgcctttggcaatagttacatttcctgcacctacttttaacatagcaatcccgtttactctattaagattacttgcacctaaaactattaacgtaccgttattag

SEQ ID NO: 2638 - DNA, 120 bp, synthetic construct
  source 1..120: mol_type = other DNA
caatcccgtttactctattaagattacttgcacctaaaactattaacgtaccgttattagtaccaccggtatttttgactgttcccgcaacatttacattgttatttaatgttaccgtac

SEQ ID NO: 2639 - DNA, 120 bp, synthetic construct
  source 1..120: mol_type = other DNA
taccaccggtatttttgactgttcccgcaacatttacattgttatttaatgttaccgtaccgttttttgcattaaaatctaaaaaacctccaatattaccggtttgagttaattgaacag

SEQ ID NO: 2640 - DNA, 120 bp, synthetic construct
  source 1..120: mol_type = other DNA
cgttttttgcattaaaatctaaaaaacctccaatattaccggtttgagttaattgaacagcatccttaaataaaactacatttgccgtagtagctccaagttctaattgacctgtaatat

SEQ ID NO: 2641 - DNA, 120 bp, synthetic construct
  source 1..120: mol_type = other DNA
catccttaaataaaactacatttgccgtagtagctccaagttctaattgacctgtaatatcaagcactatatttgttgtattaaaagtggtacctgccgtgccaaaatctccctctcctt

SEQ ID NO: 2642 - DNA, 120 bp, synthetic construct
  source 1..120: mol_type = other DNA
caagcactatatttgttgtattaaaagtggtacctgccgtgccaaaatctccctctcctttgaaaactatatcttgtaacttatgagctccaccaaacgtcttgcctccggctattgtta

SEQ ID NO: 2643 - DNA, 120 bp, synthetic construct
  source 1..120: mol_type = other DNA
tgaaaactatatcttgtaacttatgagctccaccaaacgtcttgcctccggctattgttaatttttttcctgcagttacagaatttaatattactataccctcatcgtcattatcagggt

SEQ ID NO: 2644 - DNA, 120 bp, synthetic construct
  source 1..120: mol_type = other DNA
atttttttcctgcagttacagaatttaatattactataccctcatcgtcattatcagggtctatattcgcacctagtgtgatcgtacggtcgtttcctgaactattttgtaatattaatt

SEQ ID NO: 2645 - DNA, 120 bp, synthetic construct
  source 1..120: mol_type = other DNA
ctatattcgcacctagtgtgatcgtacggtcgtttcctgaactattttgtaatattaattgagcatccgcatgtgcaaatttaatatttcctgccggtatatttaaattaccattatttg

SEQ ID NO: 2646 - DNA, 120 bp, synthetic construct
  source 1..120: mol_type = other DNA
gagcatccgcatgtgcaaatttaatatttcctgccggtatatttaaattaccattatttgcatcaatcgtataagtagcatcgtttatttgtatagtaccagcattaaatgctgtactac

SEQ ID NO: 2647 - DNA, 120 bp, synthetic construct
  source 1..120: mol_type = other DNA
catcaatcgtataagtagcatcgtttatttgtatagtaccagcattaaatgctgtactactagtaaaatctgcattattgttaataagcacgttctgtataccttctaaatttacatcgt

SEQ ID NO: 2648 - DNA, 120 bp, synthetic construct
  source 1..120: mol_type = other DNA
tagtaaaatctgcattattgttaataagcacgttctgtataccttctaaatttacatcgtcagttattgtaacggcattataaataagtaaagtgttaaatttattaccgcctacatcac

SEQ ID NO: 2649 - DNA, 120 bp, synthetic construct
  source 1..120: mol_type = other DNA
cagttattgtaacggcattataaataagtaaagtgttaaatttattaccgcctacatcaccgatatttctagcggcacctgctacattactcccaatattcagaccattaaccccaccat

SEQ ID NO: 2650 - DNA, 120 bp, synthetic construct
  source 1..120: mol_type = other DNA
cgatatttctagcggcacctgctacattactcccaatattcagaccattaaccccaccatcaaagactaccgtaccttcatcaacaccgggagctactaaatcagctgctaataatatat

SEQ ID NO: 2651 - DNA, 120 bp, synthetic construct
  source 1..120: mol_type = other DNA
caaagactaccgtaccttcatcaacaccgggagctactaaatcagctgctaataatatattatttactccgactccggttaagttagaaagtactaaagcagaatctagagctctaaaat

SEQ ID NO: 2652 - DNA, 120 bp, synthetic construct
  source 1..120: mol_type = other DNA
tatttactccgactccggttaagttagaaagtactaaagcagaatctagagctctaaaatgaatatcttgagcatttaatatagtaacatcaccagcacttgcatcaattgcaaaaagat

SEQ ID NO: 2653 - DNA, 120 bp, synthetic construct
  source 1..120: mol_type = other DNA
gaatatcttgagcatttaatatagtaacatcaccagcacttgcatcaattgcaaaaagattaccggctccaatattgatttctgcaactgttcctatagttaaatgatatgccgtaagta

SEQ ID NO: 2654 - DNA, 120 bp, synthetic construct
  source 1..120: mol_type = other DNA
taccggctccaatattgatttctgcaactgttcctatagttaaatgatatgccgtaagtaactttgtattaacatttaatatagcattattgccgtttgctatagctcctttaaaataat

SEQ ID NO: 2655 - DNA, 120 bp, synthetic construct
  source 1..120: mol_type = other DNA
actttgtattaacatttaatatagcattattgccgtttgctatagctcctttaaaataataagggattgcgttaccaccaccatcaagaggtccgttaaactctaaagtactcctagctc

SEQ ID NO: 2656 - DNA, 120 bp, synthetic construct
  source 1..120: mol_type = other DNA
aagggattgcgttaccaccaccatcaagaggtccgttaaactctaaagtactcctagctccaaaatctatattattcgcatctagacttcctccagcttgtaatgttacacctgctccta

SEQ ID NO: 2657 - DNA, 120 bp, synthetic construct
  source 1..120: mol_type = other DNA
caaaatctatattattcgcatctagacttcctccagcttgtaatgttacacctgctcctacattcactgttgctaatgcatttgtattacctatattgccagttactgtactatcaccgg

SEQ ID NO: 2658 - DNA, 120 bp, synthetic construct
  source 1..120: mol_type = other DNA
cattcactgttgctaatgcatttgtattacctatattgccagttactgtactatcaccggtaaacgttactataccattatttgcattaccggtattatctatcgctccggtcaccacta

SEQ ID NO: 2659 - DNA, 120 bp, synthetic construct
  source 1..120: mol_type = other DNA
taaacgttactataccattatttgcattaccggtattatctatcgctccggtcaccactacaggattcgtaaatgtcactgctgacgcattatctgttaacttagtcgtagtagctttaa

SEQ ID NO: 2660 - DNA, 120 bp, synthetic construct
  source 1..120: mol_type = other DNA
caggattcgtaaatgtcactgctgacgcattatctgttaacttagtcgtagtagctttaataatcgctccccctaacgtggctttacctgctcctacacttatcgtggctaatgcatttg

SEQ ID NO: 2661 - DNA, 120 bp, synthetic construct
  source 1..120: mol_type = other DNA
taatcgctccccctaacgtggctttacctgctcctacacttatcgtggctaatgcatttgtattacctatattgccagttactgtactatcaccggtaaacgttactataccattatttg

SEQ ID NO: 2662 - DNA, 120 bp, synthetic construct
  source 1..120: mol_type = other DNA
tattacctatattgccagttactgtactatcaccggtaaacgttactataccattatttgcattaccggtattatctatcgctccggtcaccactacaggattcgtaaatgtcactgctg

SEQ ID NO: 2663 - DNA, 120 bp, synthetic construct
  source 1..120: mol_type = other DNA
cattaccggtattatctatcgctccggtcaccactacaggattcgtaaatgtcactgctgacgcattatccgttaagtttattgtattcgattttaccactccgccttgtactcgtagca

SEQ ID NO: 2664 - DNA, 120 bp, synthetic construct
  source 1..120: mol_type = other DNA
acgcattatccgttaagtttattgtattcgattttaccactccgccttgtactcgtagcaaacctgctcctacattcactgttgctaatgcatttgtattacctatattgccagttactg

SEQ ID NO: 2665 - DNA, 120 bp, synthetic construct
  source 1..120: mol_type = other DNA
aacctgctcctacattcactgttgctaatgcatttgtattacctatattgccagttactgtactatcaccggtaaacgtcgctataccattatttgcattaccggtattatctatcgctc

SEQ ID NO: 2666 - DNA, 120 bp, synthetic construct
  source 1..120: mol_type = other DNA
tactatcaccggtaaacgtcgctataccattatttgcattaccggtattatctatcgctccggtcaccactacaggattcgtaaatgtcactgctgacgcattatctgttaacttagtcg

SEQ ID NO: 2667 - DNA, 120 bp, synthetic construct
  source 1..120: mol_type = other DNA
cggtcaccactacaggattcgtaaatgtcactgctgacgcattatctgttaacttagtcgtagtagctttaataaccgctccccctaacgtggctttacctgctcctacacttatcgtgg

SEQ ID NO: 2668 - DNA, 120 bp, synthetic construct
  source 1..120: mol_type = other DNA
tagtagctttaataaccgctccccctaacgtggctttacctgctcctacacttatcgtggctaatgcatttgtattacctatattcccggttacttgacttaatgcaccatttaaattta

SEQ ID NO: 2669 - DNA, 120 bp, synthetic construct
  source 1..120: mol_type = other DNA
ctaatgcatttgtattacctatattcccggttacttgacttaatgcaccatttaaatttaagacacctacattatcaacgcctgtggtgttatcaatcgcacctgttaatactgcattta

SEQ ID NO: 2670 - DNA, 120 bp, synthetic construct
  source 1..120: mol_type = other DNA
agacacctacattatcaacgcctgtggtgttatcaatcgcacctgttaatactgcatttacatttgtaagggttaataccgacgcagcattcgttaatttagtcgtagtagctttaataa

SEQ ID NO: 2671 - DNA, 120 bp, synthetic construct
  source 1..120: mol_type = other DNA
catttgtaagggttaataccgacgcagcattcgttaatttagtcgtagtagctttaataaccgctccctctaacgtggctatacctgctcctacattcactgttgctaatgcatttgtat

SEQ ID NO: 2672 - DNA, 120 bp, synthetic construct
  source 1..120: mol_type = other DNA
ccgctccctctaacgtggctatacctgctcctacattcactgttgctaatgcatttgtattacctatattgccagttactgtactattaccggtaaacgttactataccattatttgcat

SEQ ID NO: 2673 - DNA, 120 bp, synthetic construct
  source 1..120: mol_type = other DNA
tacctatattgccagttactgtactattaccggtaaacgttactataccattatttgcattaccggtattatctatcgctccggtcaccactacaggattcgtaaatgtcactgctgacg

SEQ ID NO: 2674 - DNA, 120 bp, synthetic construct
  source 1..120: mol_type = other DNA
taccggtattatctatcgctccggtcaccactacaggattcgtaaatgtcactgctgacgcattatctgttaacttagtcgtagtagctttaataatcgctccccctaacgtggctttac

SEQ ID NO: 2675 - DNA, 120 bp, synthetic construct
  source 1..120: mol_type = other DNA
cattatctgttaacttagtcgtagtagctttaataatcgctccccctaacgtggctttacctgctcctacacttatcgtggctaatgcatttgtattacctatattgccagttactgtac

SEQ ID NO: 2676 - DNA, 120 bp, synthetic construct
  source 1..120: mol_type = other DNA
ctgctcctacacttatcgtggctaatgcatttgtattacctatattgccagttactgtactatcaccggtaaacgttactataccattatttgcattaccggtattatctatcgctccgg

SEQ ID NO: 2677 - DNA, 120 bp, synthetic construct
  source 1..120: mol_type = other DNA
tatcaccggtaaacgttactataccattatttgcattaccggtattatctatcgctccggtcaccactacaggattcgtaaatgtcactgctgacgcattatccgttaacttagtcgtag

SEQ ID NO: 2678 - DNA, 120 bp, synthetic construct
  source 1..120: mol_type = other DNA
tcaccactacaggattcgtaaatgtcactgctgacgcattatccgttaacttagtcgtagtagctttaataatcgctccccctaacgtggctttacctgctcctacacttatcgtggcta

SEQ ID NO: 2679 - DNA, 120 bp, synthetic construct
  source 1..120: mol_type = other DNA
tagctttaataatcgctccccctaacgtggctttacctgctcctacacttatcgtggctaatgcatttgtattacctatattgccagttactgtactatcaccggtaaacgttactatac

SEQ ID NO: 2680 - DNA, 120 bp, synthetic construct
  source 1..120: mol_type = other DNA
atgcatttgtattacctatattgccagttactgtactatcaccggtaaacgttactataccattatttgcattaccggtattatctatcgctccggtcaccactacaggattcgtaaatg

SEQ ID NO: 2681 - DNA, 120 bp, synthetic construct
  source 1..120: mol_type = other DNA
cattatttgcattaccggtattatctatcgctccggtcaccactacaggattcgtaaatgtcactgctgacgcattatccgttaacttagtcgtagtagctttaataatcgctcccccta

SEQ ID NO: 2682 - DNA, 120 bp, synthetic construct
  source 1..120: mol_type = other DNA
tcactgctgacgcattatccgttaacttagtcgtagtagctttaataatcgctccccctaacgtggctttacctgctcctacacttatcgtggctaatgcatttgtattacctatattgc

SEQ ID NO: 2683 - DNA, 120 bp, synthetic construct
  source 1..120: mol_type = other DNA
acgtggctttacctgctcctacacttatcgtggctaatgcatttgtattacctatattgccagttactgtactatcaccggtaaacgttactataccattatttgcattaccggtattat

SEQ ID NO: 2684 - DNA, 120 bp, synthetic construct
  source 1..120: mol_type = other DNA
cagttactgtactatcaccggtaaacgttactataccattatttgcattaccggtattatctatcgctccggtcaccactacaggattcgtaaatgtcactgctgacgcattatccgtta

SEQ ID NO: 2685 - DNA, 120 bp, synthetic construct
  source 1..120: mol_type = other DNA
ctatcgctccggtcaccactacaggattcgtaaatgtcactgctgacgcattatccgttaacttagtcgtagtagctttaataatcgctccccctaacgtggctttacctgctcctacac

SEQ ID NO: 2686 - DNA, 120 bp, synthetic construct
  source 1..120: mol_type = other DNA
acttagtcgtagtagctttaataatcgctccccctaacgtggctttacctgctcctacacttatcgtggctaatgcatttgtattacctatattgccagttactgtactatcaccggtaa

SEQ ID NO: 2687 - DNA, 120 bp, synthetic construct
  source 1..120: mol_type = other DNA
ttatcgtggctaatgcatttgtattacctatattgccagttactgtactatcaccggtaaacgttactataccattatttgcattaccggtattatctatcgctccggtcaccactacag

SEQ ID NO: 2688 - DNA, 120 bp, synthetic construct
  source 1..120: mol_type = other DNA
acgttactataccattatttgcattaccggtattatctatcgctccggtcaccactacaggattcgtaaatgtcactgctgacgcattatctgttaacttagtcgtagtagctttaataa

SEQ ID NO: 2689 - DNA, 120 bp, synthetic construct
  source 1..120: mol_type = other DNA
gattcgtaaatgtcactgctgacgcattatctgttaacttagtcgtagtagctttaataaccgctccccctaacgtggctttacctgctcctacacttatcgtggctaatgcatttgtat

SEQ ID NO: 2690 - DNA, 120 bp, synthetic construct
  source 1..120: mol_type = other DNA
ccgctccccctaacgtggctttacctgctcctacacttatcgtggctaatgcatttgtattacctatattcccggttacttgacttaatgcaccatttaaatttaagacacctacattat

SEQ ID NO: 2691 - DNA, 120 bp, synthetic construct
  source 1..120: mol_type = other DNA
tacctatattcccggttacttgacttaatgcaccatttaaatttaagacacctacattatcaacgcctgtggtgttatcaatcgcacctgttaatactgcatttacatttgtaagggtta

SEQ ID NO: 2692 - DNA, 120 bp, synthetic construct
  source 1..120: mol_type = other DNA
caacgcctgtggtgttatcaatcgcacctgttaatactgcatttacatttgtaagggttaataccgacgcagcattcgttaatttagtcgtagtagctttaataatcgctccctctaacg

SEQ ID NO: 2693 - DNA, 120 bp, synthetic construct
  source 1..120: mol_type = other DNA
ataccgacgcagcattcgttaatttagtcgtagtagctttaataatcgctccctctaacgtggctatacctgctcctacattcactgttgctaacgcatttgtattacctattgttccgt

SEQ ID NO: 2694 - DNA, 120 bp, synthetic construct
  source 1..120: mol_type = other DNA
tggctatacctgctcctacattcactgttgctaacgcatttgtattacctattgttccgttaatggcagcatctgtcttgacagttattatacctcctccatttatattgcctgcaagtg

SEQ ID NO: 2695 - DNA, 120 bp, synthetic construct
  source 1..120: mol_type = other DNA
taatggcagcatctgtcttgacagttattatacctcctccatttatattgcctgcaagtgttatctttgccggggctgcagattgtataattagtgcagcattcgctccccctaaagcta

SEQ ID NO: 2696 - DNA, 120 bp, synthetic construct
  source 1..120: mol_type = other DNA
ttatctttgccggggctgcagattgtataattagtgcagcattcgctccccctaaagctatatttcctaaacctgtataattatcggcaggagcaccaaaaccatgatttgcagcatcag

SEQ ID NO: 2697 - DNA, 120 bp, synthetic construct
  source 1..120: mol_type = other DNA
tatttcctaaacctgtataattatcggcaggagcaccaaaaccatgatttgcagcatcagcattattaccgtttaaagttaagcttttgccggcagtaatagtaacaggcaacaagttac

SEQ ID NO: 2698 - DNA, 120 bp, synthetic construct
  source 1..120: mol_type = other DNA
cattattaccgtttaaagttaagcttttgccggcagtaatagtaacaggcaacaagttacctcccgttacaatcgaaccaacgacggtattttgagcaatatttagacctatgggagtag

SEQ ID NO: 2699 - DNA, 120 bp, synthetic construct
  source 1..120: mol_type = other DNA
ctcccgttacaatcgaaccaacgacggtattttgagcaatatttagacctatgggagtagtatccgcaacatttatagccgtaataatatgatcggctacatctgcagtgatagtataat

SEQ ID NO: 2700 - DNA, 120 bp, synthetic construct
  source 1..120: mol_type = other DNA
tatccgcaacatttatagccgtaataatatgatcggctacatctgcagtgatagtataatcaccaccgtaagtaaatgcccaattgttttgaggaccgcgagcaggagtaccattagcta

SEQ ID NO: 2701 - DNA, 120 bp, synthetic construct
  source 1..120: mol_type = other DNA
caccaccgtaagtaaatgcccaattgttttgaggaccgcgagcaggagtaccattagctacccctgcagccgttatctcattccaattattgccaacattatcactaaatgctgcattat

SEQ ID NO: 2702 - DNA, 120 bp, synthetic construct
  source 1..120: mol_type = other DNA
cccctgcagccgttatctcattccaattattgccaacattatcactaaatgctgcattattattagtagcaataacacctgaaacagcaataccgagtgccccgctactactcagcatta

SEQ ID NO: 2703 - DNA, 120 bp, synthetic construct
  source 1..120: mol_type = other DNA
tattagtagcaataacacctgaaacagcaataccgagtgccccgctactactcagcattatcgctgcggttgaggtggtgaataaagcggctttaagaccttgttgtattgctttttgaa

SEQ ID NO: 2704 - DNA, 120 bp, synthetic construct
  source 1..120: mol_type = other DNA
tcgctgcggttgaggtggtgaataaagcggctttaagaccttgttgtattgctttttgaaataattttggagaaatattcgccatatacgtaaaccttaataaaaattaactcacttaaa

SEQ ID NO: 2705 - DNA, 120 bp, synthetic construct
  source 1..120: mol_type = other DNA
ataattttggagaaatattcgccatatacgtaaaccttaataaaaattaactcacttaaaaagtgttataacgcaacttttttagtatgtctattataattaataacatagatgatattt

SEQ ID NO: 2706 - DNA, 120 bp, synthetic construct
  source 1..120: mol_type = other DNA
attaactcacttaaaaagtgttataacgcaacttttttagtatgtctattataattaataacatagatgatatttttatgtatagattgtcattccgtagcgacgttggccttgttgcat

SEQ ID NO: 2707 - DNA, 120 bp, synthetic construct
  source 1..120: mol_type = other DNA
tttttatgattatagaacggttaattaaaaattaacacgaacttttacactaccttgctgagcgaaatacttacttccgatattggtatcgtagttaatcccatattccatcattttatg

SEQ ID NO: 2708 - DNA, 120 bp, synthetic construct
  source 1..120: mol_type = other DNA
agcgaaatacttacttccgatattggtatcgtagttaatcccatattccatcattttatgcttagcagtaacaccgacaccgacatcaaaacttgttttgctttgcttaaagctgttggt

SEQ ID NO: 2709 - DNA, 120 bp, synthetic construct
  source 1..120: mol_type = other DNA
cttagcagtaacaccgacaccgacatcaaaacttgttttgctttgcttaaagctgttggttgggagaggagcagtcataccttgtaatcttgcatcaatcgccgaaactttattcttgaa

SEQ ID NO: 2710 - DNA, 120 bp, synthetic construct
  source 1..120: mol_type = other DNA
tgggagaggagcagtcataccttgtaatcttgcatcaatcgccgaaactttattcttgaatgcataatcgaccattgcgtaaagctcaggtgttagcactatttcattgacattgatatt

SEQ ID NO: 2711 - DNA, 120 bp, synthetic construct
  source 1..120: mol_type = other DNA
tgcataatcgaccattgcgtaaagctcaggtgttagcactatttcattgacattgatattacttgatactttagcaccgagtaaaccgtcgaaagtattatagtgcttgcctttaacggt

SEQ ID NO: 2712 - DNA, 120 bp, synthetic construct
  source 1..120: mol_type = other DNA
acttgatactttagcaccgagtaaaccgtcgaaagtattatagtgcttgcctttaacggtaagattttggtaagtagtaccggtttccttatagcccttatctttgatagtcgaatatct

SEQ ID NO: 2713 - DNA, 120 bp, synthetic construct
  source 1..120: mol_type = other DNA
aagattttggtaagtagtaccggtttccttatagcccttatctttgatagtcgaatatctaagcccagctagcggtgttaagttaatgttctcaggcatcatataggtataaccagccat

SEQ ID NO: 2714 - DNA, 120 bp, synthetic construct
  source 1..120: mol_type = other DNA
aagcccagctagcggtgttaagttaatgttctcaggcatcatataggtataaccagccattaactgacctgtatagctttcggatttataattaccgtttgcagtttgataaccgacagt

SEQ ID NO: 2715 - DNA, 120 bp, synthetic construct
  source 1..120: mol_type = other DNA
taactgacctgtatagctttcggatttataattaccgtttgcagtttgataaccgacagtctctagtgccgttgcaataacacgtcttgatttgcttcttatcttattatctgagtaaga

SEQ ID NO: 2716 - DNA, 120 bp, synthetic construct
  source 1..120: mol_type = other DNA
ctctagtgccgttgcaataacacgtcttgatttgcttcttatcttattatctgagtaagatgctatagcttcaacgaagagattttcataaggtacattatataaaccgtataaagaata

SEQ ID NO: 2717 - DNA, 120 bp, synthetic construct
  source 1..120: mol_type = other DNA
tgctatagcttcaacgaagagattttcataaggtacattatataaaccgtataaagaatagatgttgctctctaccttattcttatcgcccgttttattattttttagcttaatgtcagt

SEQ ID NO: 2718 - DNA, 120 bp, synthetic construct
  source 1..120: mol_type = other DNA
gatgttgctctctaccttattcttatcgcccgttttattattttttagcttaatgtcagtatcggatcttgtatatgcaagtccgagtgctagatcatcgctaacgaagccgtcaaaacc

SEQ ID NO: 2719 - DNA, 120 bp, synthetic construct
  source 1..120: mol_type = other DNA
atcggatcttgtatatgcaagtccgagtgctagatcatcgctaacgaagccgtcaaaacctatagtgccaccagttgtatcagacttataaccacttatattgttacacatcttctgctt

SEQ ID NO: 2720 - DNA, 120 bp, synthetic construct
  source 1..120: mol_type = other DNA
tatagtgccaccagttgtatcagacttataaccacttatattgttacacatcttctgctttgcattaccgacaaacgggcttatccacgcaccaaacttagcatccatatcttcatcacc

SEQ ID NO: 2721 - DNA, 120 bp, synthetic construct
  source 1..120: mol_type = other DNA
tgcattaccgacaaacgggcttatccacgcaccaaacttagcatccatatcttcatcaccggaagaaacaggacctttattcgctacttgtactttatccattctagcatttagagcagt

SEQ ID NO: 2722 - DNA, 120 bp, synthetic construct
  source 1..120: mol_type = other DNA
ggaagaaacaggacctttattcgctacttgtactttatccattctagcatttagagcagttatattacttgatatattacttgctacaacttgattattaacggcagctatagtatcgct

SEQ ID NO: 2723 - DNA, 120 bp, synthetic construct
  source 1..120: mol_type = other DNA
tatattacttgatatattacttgctacaacttgattattaacggcagctatagtatcgctaggttttacaacatcttgaatgagatgagttgtagcatctgcttcctgtagcggtgtcat

SEQ ID NO: 2724 - DNA, 120 bp, synthetic construct
  source 1..120: mol_type = other DNA
aggttttacaacatcttgaatgagatgagttgtagcatctgcttcctgtagcggtgtcattagaccaaagttattgaaagcttgacgtgcatctgaaccattgggagcatcctccattaa

SEQ ID NO: 2725 - DNA, 120 bp, synthetic construct
  source 1..120: mol_type = other DNA
tagaccaaagttattgaaagcttgacgtgcatctgaaccattgggagcatcctccattaactcaagcgatttctttatatttgcagcatttgggatacttacaagcggtccacccggtgc

SEQ ID NO: 2726 - DNA, 120 bp, synthetic construct
  source 1..120: mol_type = other DNA
ctcaagcgatttctttatatttgcagcatttgggatacttacaagcggtccacccggtgcaaaatcttcatctataacatctgcagctatatcctctgcaaataacgttaaagtcgatgc

SEQ ID NO: 2727 - DNA, 120 bp, synthetic construct
  source 1..120: mol_type = other DNA
aaaatcttcatctataacatctgcagctatatcctctgcaaataacgttaaagtcgatgcatcaaaagtaaaatcaacaaaacggttgtcattattaatagttattttaacattctcttt

SEQ ID NO: 2728 - DNA, 120 bp, synthetic construct
  source 1..120: mol_type = other DNA
atcaaaagtaaaatcaacaaaacggttgtcattattaatagttattttaacattctctttaggagtaggctttaaatcacctgctgtttctgcagatattaccgtatattttgtatctgg

SEQ ID NO: 2729 - DNA, 120 bp, synthetic construct
  source 1..120: mol_type = other DNA
aggagtaggctttaaatcacctgctgtttctgcagatattaccgtatattttgtatctgggcttatattattcatgtcgaaattagtagcagtaacaacaagtgctaaagttgaaacccc

SEQ ID NO: 2730 - DNA, 120 bp, synthetic construct
  source 1..120: mol_type = other DNA
gcttatattattcatgtcgaaattagtagcagtaacaacaagtgctaaagttgaaacccctgataaatcaagagtactacctgatttaattaagatattaccacctgacttagctgctcc

SEQ ID NO: 2731 - DNA, 120 bp, synthetic construct
  source 1..120: mol_type = other DNA
tgataaatcaagagtactacctgatttaattaagatattaccacctgacttagctgctccatcaaaagtagtatttaaggttagcgtatcggtaaagctaccggtgccagtatatgttac

SEQ ID NO: 2732 - DNA, 120 bp, synthetic construct
  source 1..120: mol_type = other DNA
atcaaaagtagtatttaaggttagcgtatcggtaaagctaccggtgccagtatatgttacgtgatttgcacctaaagtaattgtagtaccgctacctgttatattactattaaaggctag

SEQ ID NO: 2733 - DNA, 120 bp, synthetic construct
  source 1..120: mol_type = other DNA
gtgatttgcacctaaagtaattgtagtaccgctacctgttatattactattaaaggctaggctattgccgaaattaatagtagcactgttagctacaaagctggtagctgttacattttt

SEQ ID NO: 2734 - DNA, 120 bp, synthetic construct
  source 1..120: mol_type = other DNA
gctattgccgaaattaatagtagcactgttagctacaaagctggtagctgttacatttttagcaaaactagtgatagaacctttggctaaagtaaccgcacctgtattagtgaatgtatt

SEQ ID NO: 2735 - DNA, 120 bp, synthetic construct
  source 1..120: mol_type = other DNA
agcaaaactagtgatagaacctttggctaaagtaaccgcacctgtattagtgaatgtattggcaaaacttgtagtaccgccaagtgtcgctgtaccttttgcgttaacactgcttgcaaa

SEQ ID NO: 2736 - DNA, 120 bp, synthetic construct
  source 1..120: mol_type = other DNA
ggcaaaacttgtagtaccgccaagtgtcgctgtaccttttgcgttaacactgcttgcaaaacttgtagcacctgccgttgtgatatcaccaaccgaattagccgcagtccctacaacacc

SEQ ID NO: 2737 - DNA, 120 bp, synthetic construct
  source 1..120: mol_type = other DNA
acttgtagcacctgccgttgtgatatcaccaaccgaattagccgcagtccctacaacacctttaacactaccgccattcgtgaagtttagcttcagagcctgaccaccggttttatttat

SEQ ID NO: 2738 - DNA, 120 bp, synthetic construct
  source 1..120: mol_type = other DNA
tttaacactaccgccattcgtgaagtttagcttcagagcctgaccaccggttttatttatgctgcctgttaagttaaagtttgcaggtaatgttaaagtatttgtgcctgtaccttggat

SEQ ID NO: 2739 - DNA, 120 bp, synthetic construct
  source 1..120: mol_type = other DNA
gctgcctgttaagttaaagtttgcaggtaatgttaaagtatttgtgcctgtaccttggatttcgccgattttaacgttaccgcctttggcaatagttacatttcctgcacctacttttaa

SEQ ID NO: 2740 - DNA, 120 bp, synthetic construct
  source 1..120: mol_type = other DNA
ttcgccgattttaacgttaccgcctttggcaatagttacatttcctgcacctacttttaacatagcaatcccgtttactctattaagattacttgcacctaaaactattaacgtaccgtt

SEQ ID NO: 2741 - DNA, 120 bp, synthetic construct
  source 1..120: mol_type = other DNA
catagcaatcccgtttactctattaagattacttgcacctaaaactattaacgtaccgttattagtaccgccggtattttggactgctcccgcaacacttacattgttatttaatattac

SEQ ID NO: 2742 - DNA, 120 bp, synthetic construct
  source 1..120: mol_type = other DNA
attagtaccgccggtattttggactgctcccgcaacacttacattgttatttaatattaccgtaccgttttttgcattaaaatctaagaaaccgccaatatgaccggtttgagttaattg

SEQ ID NO: 2743 - DNA, 120 bp, synthetic construct
  source 1..120: mol_type = other DNA
cgtaccgttttttgcattaaaatctaagaaaccgccaatatgaccggtttgagttaattgaacagcatcattaaataaaactacatttgccttagcagctccaagttctaatttacctgt

SEQ ID NO: 2744 - DNA, 120 bp, synthetic construct
  source 1..120: mol_type = other DNA
aacagcatcattaaataaaactacatttgccttagcagctccaagttctaatttacctgtaatatcaagctctatatttgttgtattaaaagtggtacctgccgcgctgcaatctcccgc

SEQ ID NO: 2745 - DNA, 120 bp, synthetic construct
  source 1..120: mol_type = other DNA
aatatcaagctctatatttgttgtattaaaagtggtacctgccgcgctgcaatctcccgctcctttgaaaactatagtttgtaacttatgagctccaccaaacgtcttgcctccggctat

SEQ ID NO: 2746 - DNA, 120 bp, synthetic construct
  source 1..120: mol_type = other DNA
tcctttgaaaactatagtttgtaacttatgagctccaccaaacgtcttgcctccggctatcgttaatttttttcctgcagttacagaatttaatattactacaccctcattgtcattatc

SEQ ID NO: 2747 - DNA, 120 bp, synthetic construct
  source 1..120: mol_type = other DNA
cgttaatttttttcctgcagttacagaatttaatattactacaccctcattgtcattatcagggtctatattcgcacctagtgtgatcgtacggtcgtttcctgaactattttgtaatat

SEQ ID NO: 2748 - DNA, 120 bp, synthetic construct
  source 1..120: mol_type = other DNA
agggtctatattcgcacctagtgtgatcgtacggtcgtttcctgaactattttgtaatattaattgagcatccgcatgtgcaaattgaatatttcctgccggtatatttaaattaccatt

SEQ ID NO: 2749 - DNA, 120 bp, synthetic construct
  source 1..120: mol_type = other DNA
taattgagcatccgcatgtgcaaattgaatatttcctgccggtatatttaaattaccattatttgcatcaatcgtataagtagcatcgtttatttgtataataccagcattaaatgctgt

SEQ ID NO: 2750 - DNA, 120 bp, synthetic construct
  source 1..120: mol_type = other DNA
atttgcatcaatcgtataagtagcatcgtttatttgtataataccagcattaaatgctgtactactagtaaaatctgcattattttcaatacgcacgttctgtataccttctaaatttac

SEQ ID NO: 2751 - DNA, 120 bp, synthetic construct
  source 1..120: mol_type = other DNA
actactagtaaaatctgcattattttcaatacgcacgttctgtataccttctaaatttacatcgtcagttattgtaacggcattataaataagtaaagtgttaaatttattaccgcctcc

SEQ ID NO: 2752 - DNA, 120 bp, synthetic construct
  source 1..120: mol_type = other DNA
atcgtcagttattgtaacggcattataaataagtaaagtgttaaatttattaccgcctccatcaccgatatttctagcggtacctgctacattactcccaatattcaggccattaacccc

SEQ ID NO: 2753 - DNA, 120 bp, synthetic construct
  source 1..120: mol_type = other DNA
atcaccgatatttctagcggtacctgctacattactcccaatattcaggccattaaccccaccatcaaagactacattaccttcatcagcaccgggagctactaaatcagctgctaataa

SEQ ID NO: 2754 - DNA, 120 bp, synthetic construct
  source 1..120: mol_type = other DNA
accatcaaagactacattaccttcatcagcaccgggagctactaaatcagctgctaataatatattttttgctccgactccggtgaagttagaaagtactaaagcagaatctggaactct

SEQ ID NO: 2755 - DNA, 120 bp, synthetic construct
  source 1..120: mol_type = other DNA
tatattttttgctccgactccggtgaagttagaaagtactaaagcagaatctggaactctaaaattaatatcttgagcatttaatatagtaacatcaccagcacttgcatcaattgtaaa

SEQ ID NO: 2756 - DNA, 120 bp, synthetic construct
  source 1..120: mol_type = other DNA
aaaattaatatcttgagcatttaatatagtaacatcaccagcacttgcatcaattgtaaaaagattaccggctccaatattaatttctgcaactgttcctatagttgaatgatatgccgt

SEQ ID NO: 2757 - DNA, 120 bp, synthetic construct
  source 1..120: mol_type = other DNA
aagattaccggctccaatattaatttctgcaactgttcctatagttgaatgatatgccgtaagtgactttgtattaacatttaatatagcgttattgccgtttgctatagctcctttaaa

SEQ ID NO: 2758 - DNA, 120 bp, synthetic construct
  source 1..120: mol_type = other DNA
aagtgactttgtattaacatttaatatagcgttattgccgtttgctatagctcctttaaaataataagggattatgttaccaccaccatcaagaggtccgttaaactctaaaatactcct

SEQ ID NO: 2759 - DNA, 120 bp, synthetic construct
  source 1..120: mol_type = other DNA
ataataagggattatgttaccaccaccatcaagaggtccgttaaactctaaaatactcctggctccaaaatctatattattcgcagctaggcttcctccagcttttaatgttactcctgc

SEQ ID NO: 2760 - DNA, 120 bp, synthetic construct
  source 1..120: mol_type = other DNA
ggctccaaaatctatattattcgcagctaggcttcctccagcttttaatgttactcctgctcctacattcactgttgctaatgcatttgtattacctatattgccagttactgtactatt

SEQ ID NO: 2761 - DNA, 120 bp, synthetic construct
  source 1..120: mol_type = other DNA
tcctacattcactgttgctaatgcatttgtattacctatattgccagttactgtactattaccggtaaacgttgctataccattatttgcattaccggtattatctagcgccccggtcac

SEQ ID NO: 2762 - DNA, 120 bp, synthetic construct
  source 1..120: mol_type = other DNA
accggtaaacgttgctataccattatttgcattaccggtattatctagcgccccggtcaccactacaggattcgtaaatgtcactgctgacgcattatccgttaagtttattgcattcgc

SEQ ID NO: 2763 - DNA, 120 bp, synthetic construct
  source 1..120: mol_type = other DNA
cactacaggattcgtaaatgtcactgctgacgcattatccgttaagtttattgcattcgcttttaccactccgccttgtacttgtagcaaacctgctcctacattcactgttgctaatgc

SEQ ID NO: 2764 - DNA, 120 bp, synthetic construct
  source 1..120: mol_type = other DNA
ttttaccactccgccttgtacttgtagcaaacctgctcctacattcactgttgctaatgcatttgtattacctatattgccagttactgtactattaccggtaaacgttgctataccatt

SEQ ID NO: 2765 - DNA, 120 bp, synthetic construct
  source 1..120: mol_type = other DNA
atttgtattacctatattgccagttactgtactattaccggtaaacgttgctataccattatttgcattaccggtattatctagcgctccggtcaccactacaggattcgtaaatgtcac

SEQ ID NO: 2766 - DNA, 120 bp, synthetic construct
  source 1..120: mol_type = other DNA
atttgcattaccggtattatctagcgctccggtcaccactacaggattcgtaaatgtcactgctgacgcattatccgttaagtttattgcattcgcttttaccactccgccttgtacttg

SEQ ID NO: 2767 - DNA, 120 bp, synthetic construct
  source 1..120: mol_type = other DNA
tgctgacgcattatccgttaagtttattgcattcgcttttaccactccgccttgtacttgtagcaaacctgctcctacattcactgttgctaatgcatttgtattacctatattgccagt

SEQ ID NO: 2768 - DNA, 120 bp, synthetic construct
  source 1..120: mol_type = other DNA
tagcaaacctgctcctacattcactgttgctaatgcatttgtattacctatattgccagttactgtactattaccggtaaacgttgctataccattatttgcattaccggtattatctag

SEQ ID NO: 2769 - DNA, 120 bp, synthetic construct
  source 1..120: mol_type = other DNA
tactgtactattaccggtaaacgttgctataccattatttgcattaccggtattatctagcgccccggtcaccactacaggattcgtaaatgtcactgctgacgcagcatttgttaattt

SEQ ID NO: 2770 - DNA, 120 bp, synthetic construct
  source 1..120: mol_type = other DNA
cgccccggtcaccactacaggattcgtaaatgtcactgctgacgcagcatttgttaatttagtcgtagtagctttaataaccgccccccctaacgtggctgtacctgctcctacatttat

SEQ ID NO: 2771 - DNA, 120 bp, synthetic construct
  source 1..120: mol_type = other DNA
agtcgtagtagctttaataaccgccccccctaacgtggctgtacctgctcctacatttatcgtggctaatgcatttgtattacctatattcccgcttacttgacttaatgcaccatttaa

SEQ ID NO: 2772 - DNA, 120 bp, synthetic construct
  source 1..120: mol_type = other DNA
cgtggctaatgcatttgtattacctatattcccgcttacttgacttaatgcaccatttaaatttaagacacctacattatcaccgcctgtggtgttatcaatctcacctgttaatactgc

SEQ ID NO: 2773 - DNA, 120 bp, synthetic construct
  source 1..120: mol_type = other DNA
atttaagacacctacattatcaccgcctgtggtgttatcaatctcacctgttaatactgcatttgcatttgtaagggttaataccgacgcagcatttgttaatttagtcgtagtagcttt

SEQ ID NO: 2774 - DNA, 120 bp, synthetic construct
  source 1..120: mol_type = other DNA
atttgcatttgtaagggttaataccgacgcagcatttgttaatttagtcgtagtagctttaataaccgctccctctaacgtggctgtacctgctcctacatttatcgtggctaatgcatt

SEQ ID NO: 2775 - DNA, 120 bp, synthetic construct
  source 1..120: mol_type = other DNA
aataaccgctccctctaacgtggctgtacctgctcctacatttatcgtggctaatgcatttgtattacctatattcccgcttacttgacttaatgcaccatttaaatttaagacacctac

SEQ ID NO: 2776 - DNA, 120 bp, synthetic construct
  source 1..120: mol_type = other DNA
tgtattacctatattcccgcttacttgacttaatgcaccatttaaatttaagacacctacattatcaccgcctgtggtgttatcaatctcacctgttaatactgcatttgcatttgtaag

SEQ ID NO: 2777 - DNA, 120 bp, synthetic construct
  source 1..120: mol_type = other DNA
attatcaccgcctgtggtgttatcaatctcacctgttaatactgcatttgcatttgtaagggttaataccgacgcagcatttgttaatttagtcgtagtagctttaataaccgctccctc

SEQ ID NO: 2778 - DNA, 120 bp, synthetic construct
  source 1..120: mol_type = other DNA
ggttaataccgacgcagcatttgttaatttagtcgtagtagctttaataaccgctccctctaacgtggctgtacctgctcctacatttatcgtggctaatgcatttgtattacctatatt

SEQ ID NO: 2779 - DNA, 120 bp, synthetic construct
  source 1..120: mol_type = other DNA
taacgtggctgtacctgctcctacatttatcgtggctaatgcatttgtattacctatattcccgcttacttgacttaatgcaccatttaaatttaagacacctacattatcaccgcctgt

SEQ ID NO: 2780 - DNA, 120 bp, synthetic construct
  source 1..120: mol_type = other DNA
cccgcttacttgacttaatgcaccatttaaatttaagacacctacattatcaccgcctgtggtgttatcaatctcacctgttaatactgcatttgcatttgtaagggttaataccgacgc

SEQ ID NO: 2781 - DNA, 120 bp, synthetic construct
  source 1..120: mol_type = other DNA
ggtgttatcaatctcacctgttaatactgcatttgcatttgtaagggttaataccgacgcagcatttgttaatttagtcgtagtagctttaataaccgctccctctaacgtggctgtacc

SEQ ID NO: 2782 - DNA, 120 bp, synthetic construct
  source 1..120: mol_type = other DNA
agcatttgttaatttagtcgtagtagctttaataaccgctccctctaacgtggctgtacctgctcctacatttatcgtggctaatgcatttgtattacctatattgccagttactgtact

SEQ ID NO: 2783 - DNA, 120 bp, synthetic construct
  source 1..120: mol_type = other DNA
tgctcctacatttatcgtggctaatgcatttgtattacctatattgccagttactgtactattaccggtaaacgttgctataccattatttgcattaccggtattatctagcgctccggt

SEQ ID NO: 2784 - DNA, 120 bp, synthetic construct
  source 1..120: mol_type = other DNA
attaccggtaaacgttgctataccattatttgcattaccggtattatctagcgctccggttaccactacaggattcgtaaatgtcactgctgacgcattatccgttaagtttattgcatt

SEQ ID NO: 2785 - DNA, 120 bp, synthetic construct
  source 1..120: mol_type = other DNA
taccactacaggattcgtaaatgtcactgctgacgcattatccgttaagtttattgcattcgcttttaccactccgccttgtacttgtagcaaacctgctcctacattcactgttgctaa

SEQ ID NO: 2786 - DNA, 120 bp, synthetic construct
  source 1..120: mol_type = other DNA
cgcttttaccactccgccttgtacttgtagcaaacctgctcctacattcactgttgctaatgcatttgtattacctatattgccagttactgtactattaccggtaaacgttgctatacc

SEQ ID NO: 2787 - DNA, 120 bp, synthetic construct
  source 1..120: mol_type = other DNA
tgcatttgtattacctatattgccagttactgtactattaccggtaaacgttgctataccattatttgcattaccggtattatctagcgctccggtcaccactacaggattcgtaaatgt

SEQ ID NO: 2788 - DNA, 120 bp, synthetic construct
  source 1..120: mol_type = other DNA
attatttgcattaccggtattatctagcgctccggtcaccactacaggattcgtaaatgtcactgctgacgcattatccgttaagtttattgcattcgcttttaccactccgccttgtac

SEQ ID NO: 2789 - DNA, 120 bp, synthetic construct
  source 1..120: mol_type = other DNA
cactgctgacgcattatccgttaagtttattgcattcgcttttaccactccgccttgtacttgtagcaaacctgctcctacattcactgttgctaatgcatttgtattacctatattgcc

SEQ ID NO: 2790 - DNA, 120 bp, synthetic construct
  source 1..120: mol_type = other DNA
ttgtagcaaacctgctcctacattcactgttgctaatgcatttgtattacctatattgccagttactgtactattaccggtaaacgttgctataccattatttgcattaccggtattatc

SEQ ID NO: 2791 - DNA, 120 bp, synthetic construct
  source 1..120: mol_type = other DNA
agttactgtactattaccggtaaacgttgctataccattatttgcattaccggtattatctagcgccccggtcaccactacaggattcgtaaatgtcactgctgacgcattatccgttaa

SEQ ID NO: 2792 - DNA, 120 bp, synthetic construct
  source 1..120: mol_type = other DNA
tagcgccccggtcaccactacaggattcgtaaatgtcactgctgacgcattatccgttaagtttattgcattcgcttttaccactccgccttgtacttgtagcaaacctgctcctacatt

SEQ ID NO: 2793 - DNA, 120 bp, synthetic construct
  source 1..120: mol_type = other DNA
gtttattgcattcgcttttaccactccgccttgtacttgtagcaaacctgctcctacattcactgttgctaatgcatttgtattacctatattgccagttactgtactattaccggtaaa

SEQ ID NO: 2794 - DNA, 120 bp, synthetic construct
  source 1..120: mol_type = other DNA
cactgttgctaatgcatttgtattacctatattgccagttactgtactattaccggtaaacgttgctataccattatttgcattaccggtattatctagcgctccggtcaccactacagg

SEQ ID NO: 2795 - DNA, 120 bp, synthetic construct
  source 1..120: mol_type = other DNA
cgttgctataccattatttgcattaccggtattatctagcgctccggtcaccactacaggattcgtaaatgtcactgctgacgcattatccgttaagtttattgcattcgcttttaccac

SEQ ID NO: 2796 - DNA, 120 bp, synthetic construct
  source 1..120: mol_type = other DNA
attcgtaaatgtcactgctgacgcattatccgttaagtttattgcattcgcttttaccactccgccttgtacttgtagcaaacctgctcctacattcactgttgctaatgcatttgtatt

SEQ ID NO: 2797 - DNA, 120 bp, synthetic construct
  source 1..120: mol_type = other DNA
tccgccttgtacttgtagcaaacctgctcctacattcactgttgctaatgcatttgtattacctatattgccagttactgtactattaccggtaaacgttgctataccattatttgcatt

SEQ ID NO: 2798 - DNA, 120 bp, synthetic construct
  source 1..120: mol_type = other DNA
acctatattgccagttactgtactattaccggtaaacgttgctataccattatttgcattaccggtattatctagcgccccggtcaccactacaggattcgtaaatgtcactgctgacgc

SEQ ID NO: 2799 - DNA, 120 bp, synthetic construct
  source 1..120: mol_type = other DNA
accggtattatctagcgccccggtcaccactacaggattcgtaaatgtcactgctgacgcattatccgttaagtttattgcattcgcttttaccactccgccttgtacttgtagcaaacc

SEQ ID NO: 2800 - DNA, 120 bp, synthetic construct
  source 1..120: mol_type = other DNA
attatccgttaagtttattgcattcgcttttaccactccgccttgtacttgtagcaaacctgctcctacattcactgttgctaatgcatttgtattacctatattcccgcttacttgact

SEQ ID NO: 2801 - DNA, 120 bp, synthetic construct
  source 1..120: mol_type = other DNA
tgctcctacattcactgttgctaatgcatttgtattacctatattcccgcttacttgacttaatgcaccatttaaatttaagacacctacattatcaccgcctgtggtgttatcaatctc

SEQ ID NO: 2802 - DNA, 120 bp, synthetic construct
  source 1..120: mol_type = other DNA
taatgcaccatttaaatttaagacacctacattatcaccgcctgtggtgttatcaatctcacctgttaatactgcatttgcatttgtaagggttaataccgacgcagcatttgttaattt

SEQ ID NO: 2803 - DNA, 120 bp, synthetic construct
  source 1..120: mol_type = other DNA
acctgttaatactgcatttgcatttgtaagggttaataccgacgcagcatttgttaatttagtcgtagtagctttaataaccgctccctctaacgtggctttacctgctcctacatttat

SEQ ID NO: 2804 - DNA, 120 bp, synthetic construct
  source 1..120: mol_type = other DNA
agtcgtagtagctttaataaccgctccctctaacgtggctttacctgctcctacatttatcgtggctaatgtatttgtattacctatattcccgcttacttgacttaatgcaccatttaa

SEQ ID NO: 2805 - DNA, 120 bp, synthetic construct
  source 1..120: mol_type = other DNA
cgtggctaatgtatttgtattacctatattcccgcttacttgacttaatgcaccatttaaatttaagacacctacattatcaccgcctgtggtgttatcaatctcacctgttaatactgc

SEQ ID NO: 2806 - DNA, 120 bp, synthetic construct
  source 1..120: mol_type = other DNA
atttgcatttgtaagggttaataccgacgcagcatttgttaatttagtcgtagtagctttaataaccgctccctctaacgtggctttacctgctcctacatttatcgtggctaatgtatt

SEQ ID NO: 2807 - DNA, 120 bp, synthetic construct
  source 1..120: mol_type = other DNA
aataaccgctccctctaacgtggctttacctgctcctacatttatcgtggctaatgtatttgtattacctatattcccgcttacttgacttaatgcaccatttaaatttaagacacctac

SEQ ID NO: 2808 - DNA, 120 bp, synthetic construct
  source 1..120: mol_type = other DNA
attatcaccgcctgtggtgttatcaatctcacctgttaatactgcatttgcatttgtaagggttaataccgacgcagcatttgttaatttagtcgtagtagctttaataaccgctccccc

SEQ ID NO: 2809 - DNA, 120 bp, synthetic construct
  source 1..120: mol_type = other DNA
ggttaataccgacgcagcatttgttaatttagtcgtagtagctttaataaccgctccccctaacgtggctttacctgctcctacatttatcgtggctaatgcatttgtattacctattgt

SEQ ID NO: 2810 - DNA, 120 bp, synthetic construct
  source 1..120: mol_type = other DNA
taacgtggctttacctgctcctacatttatcgtggctaatgcatttgtattacctattgttccgttaatggcagcatctgtcttgacagttattatacctcctccatctatatttcctgc

SEQ ID NO: 2811 - DNA, 120 bp, synthetic construct
  source 1..120: mol_type = other DNA
tccgttaatggcagcatctgtcttgacagttattatacctcctccatctatatttcctgcaagtgttatatttgccggggttgcagattgtataattagttcagcattcactccccctaa

SEQ ID NO: 2812 - DNA, 120 bp, synthetic construct
  source 1..120: mol_type = other DNA
aagtgttatatttgccggggttgcagattgtataattagttcagcattcactccccctaaagttatatttcctaaacctgtataattatcggcaggagcattaaaaccatgatttgcagc

SEQ ID NO: 2813 - DNA, 120 bp, synthetic construct
  source 1..120: mol_type = other DNA
agttatatttcctaaacctgtataattatcggcaggagcattaaaaccatgatttgcagcaacagcattattaccatttaaagttaagcttttgccggcagtaatagtaacaggcaacaa

SEQ ID NO: 2814 - DNA, 120 bp, synthetic construct
  source 1..120: mol_type = other DNA
aacagcattattaccatttaaagttaagcttttgccggcagtaatagtaacaggcaacaagttacctcccgttataatcgaaccaacgacggtattttgagcaatatttagacctacggg

SEQ ID NO: 2815 - DNA, 120 bp, synthetic construct
  source 1..120: mol_type = other DNA
gttacctcccgttataatcgaaccaacgacggtattttgagcaatatttagacctacgggattagtattcgcaacatttatagccttaataatacaattgactacatctgcagtgatagt

SEQ ID NO: 2816 - DNA, 120 bp, synthetic construct
  source 1..120: mol_type = other DNA
attagtattcgcaacatttatagccttaataatacaattgactacatctgcagtgatagtataatcaccaccgtaagtaaatgcccaattgttttgaggaccaccagcaggattaccatc

SEQ ID NO: 2817 - DNA, 120 bp, synthetic construct
  source 1..120: mol_type = other DNA
ataatcaccaccgtaagtaaatgcccaattgttttgaggaccaccagcaggattaccatcagcttcccctctagccgttatctgattccaattattggcagcagcatcattactaaatgc

SEQ ID NO: 2818 - DNA, 120 bp, synthetic construct
  source 1..120: mol_type = other DNA
agcttcccctctagccgttatctgattccaattattggcagcagcatcattactaaatgctgcatcattattagtagcaataacacctgcagcaacaccgagtgccccactactactcag

SEQ ID NO: 2819 - DNA, 120 bp, synthetic construct
  source 1..120: mol_type = other DNA
tgcatcattattagtagcaataacacctgcagcaacaccgagtgccccactactactcagcattatcgctgcggttgaggtggtgaataaagcggctttaagaccttgttgtattgcttt

SEQ ID NO: 2820 - DNA, 120 bp, synthetic construct
  source 1..120: mol_type = other DNA
cattatcgctgcggttgaggtggtgaataaagcggctttaagaccttgttgtattgctttttgaaataattttggagaaatatttgccatatgtaaaccttaataaaaattaaatcactt

SEQ ID NO: 2821 - DNA, 120 bp, synthetic construct
  source 1..120: mol_type = other DNA
taatcggttatgatctcttgcatatctcttggtagttcacaagaaaatgccataatatcattactagttggatgtgtaaaacttaaataccaagaatgaagagcttggcgtttaaaagct

SEQ ID NO: 2822 - DNA, 120 bp, synthetic construct
  source 1..120: mol_type = other DNA
ttactagttggatgtgtaaaacttaaataccaagaatgaagagcttggcgtttaaaagctattaatttagcttttagtttaggtggtgaattaataattttacggttgttattaccataa

SEQ ID NO: 2823 - DNA, 120 bp, synthetic construct
  source 1..120: mol_type = other DNA
attaatttagcttttagtttaggtggtgaattaataattttacggttgttattaccataagtttggtcaccaactactgaatgctttaaattacttaactgtactctgatttggtgcgtt

SEQ ID NO: 2824 - DNA, 120 bp, synthetic construct
  source 1..120: mol_type = other DNA
gtttggtcaccaactactgaatgctttaaattacttaactgtactctgatttggtgcgttctcccggtactaagcttgcattccaccatactaagagtaccgccgtaaaatagctctaaa

SEQ ID NO: 2825 - DNA, 120 bp, synthetic construct
  source 1..120: mol_type = other DNA
ctcccggtactaagcttgcattccaccatactaagagtaccgccgtaaaatagctctaaagtcttgtaatacgtaacagcttttttgccgccgtattttaatattgtcattttttttcga

SEQ ID NO: 2826 - DNA, 120 bp, synthetic construct
  source 1..120: mol_type = other DNA
gtcttgtaatacgtaacagcttttttgccgccgtattttaatattgtcattttttttcgattatttctattacgacctacattattcttaattattccttctagtggattaattactccc

SEQ ID NO: 2827 - DNA, 120 bp, synthetic construct
  source 1..120: mol_type = other DNA
ttatttctattacgacctacattattcttaattattccttctagtggattaattactccccaaactaatgctttatatttccgtattacctgcctttgttttatctgattggcaagcaga

SEQ ID NO: 2828 - DNA, 120 bp, synthetic construct
  source 1..120: mol_type = other DNA
caaactaatgctttatatttccgtattacctgcctttgttttatctgattggcaagcagaatatgtgttttattatttttagcaacaaccattaaacctgtagtgtctttatctaaacga

SEQ ID NO: 2829 - DNA, 120 bp, synthetic construct
  source 1..120: mol_type = other DNA
atatgtgttttattatttttagcaacaaccattaaacctgtagtgtctttatctaaacgatgtactatgcctggtctttctgctgaaccaatatctgatagatactttgtatggtgcagt

SEQ ID NO: 2830 - DNA, 120 bp, synthetic construct
  source 1..120: mol_type = other DNA
tgtactatgcctggtctttctgctgaaccaatatctgatagatactttgtatggtgcagtaatgcgttaacaagagtattatcgtgatgtcttatacctggatgtacagtcatacctgct

SEQ ID NO: 2831 - DNA, 120 bp, synthetic construct
  source 1..120: mol_type = other DNA
aatgcgttaacaagagtattatcgtgatgtcttatacctggatgtacagtcatacctgctgctttgttaattactatcaaatcatcatcttcataaattatatcaagtgttatatttgct

SEQ ID NO: 2832 - DNA, 120 bp, synthetic construct
  source 1..120: mol_type = other DNA
gctttgttaattactatcaaatcatcatcttcataaattatatcaagtgttatatttgctgctgtaatttttagctcttcaggctctttaaaagaaaataatatagtatcattctccttg

SEQ ID NO: 2833 - DNA, 120 bp, synthetic construct
  source 1..120: mol_type = other DNA
gctgtaatttttagctcttcaggctctttaaaagaaaataatatagtatcattctccttgaccaaaacatcagaatcagaaataatcacaccattaacttgtacacaataattcttaata

SEQ ID NO: 2834 - DNA, 120 bp, synthetic construct
  source 1..120: mol_type = other DNA
accaaaacatcagaatcagaaataatcacaccattaacttgtacacaataattcttaatagctttttgaacttgatttcttgagacctttttcaggagtaatgataaagctttatcaagc

SEQ ID NO: 2835 - DNA, 120 bp, synthetic construct
  source 1..120: mol_type = other DNA
gctttttgaacttgatttcttgagacctttttcaggagtaatgataaagctttatcaagccttgtgttgtttagttcctttggtacattataggttaacatattttattttaagataatg

SEQ ID NO: 2836 - DNA, 120 bp, synthetic construct
  source 1..120: mol_type = other DNA
cttgtgttgtttagttcctttggtacattataggttaacatattttattttaagataatgaatgatatgtttaaatggttaaatgcaatcggtgttgaatattattgctacgaacacaca

SEQ ID NO: 2837 - DNA, 120 bp, synthetic construct
  source 1..120: mol_type = other DNA
aatgatatgtttaaatggttaaatgcaatcggtgttgaatattattgctacgaacacacaccacaattaaaaatatctcacaatactgcaatcactgaaaaaaaacaagttaaactgatg

SEQ ID NO: 2838 - DNA, 120 bp, synthetic construct
  source 1..120: mol_type = other DNA
ccacaattaaaaatatctcacaatactgcaatcactgaaaaaaaacaagttaaactgatgcatacaacagaagcggtatttaataataatgttcatgataatataacgttatcaagatct

SEQ ID NO: 2839 - DNA, 120 bp, synthetic construct
  source 1..120: mol_type = other DNA
catacaacagaagcggtatttaataataatgttcatgataatataacgttatcaagatctcttgcagacaaagctaataatatcgtagaactaagagaatctctactaaattttaatggt

SEQ ID NO: 2840 - DNA, 120 bp, synthetic construct
  source 1..120: mol_type = other DNA
cttgcagacaaagctaataatatcgtagaactaagagaatctctactaaattttaatggttgtgaacttaagaagtttgctactaatacagttttcggtgatggtaatccacaagctaac

SEQ ID NO: 2841 - DNA, 120 bp, synthetic construct
  source 1..120: mol_type = other DNA
tgtgaacttaagaagtttgctactaatacagttttcggtgatggtaatccacaagctaacattatgttaataggcgaagctccagggaatactgaggatttaaaaggaatacctttttgc

SEQ ID NO: 2842 - DNA, 120 bp, synthetic construct
  source 1..120: mol_type = other DNA
attatgttaataggcgaagctccagggaatactgaggatttaaaaggaatacctttttgcggtgaaagtggtaatttacttgataatatgttgtatgctataggtatttcacggaataat

SEQ ID NO: 2843 - DNA, 120 bp, synthetic construct
  source 1..120: mol_type = other DNA
ggtgaaagtggtaatttacttgataatatgttgtatgctataggtatttcacggaataatttttatattactaatatggtattttggcgtcctcctgctaatagacaaccaactctagaa

SEQ ID NO: 2844 - DNA, 120 bp, synthetic construct
  source 1..120: mol_type = other DNA
ttttatattactaatatggtattttggcgtcctcctgctaatagacaaccaactctagaagaagttgatatttgcagacctttcgtagaaaaacatattgctctaattaatcctaagttg

SEQ ID NO: 2845 - DNA, 120 bp, synthetic construct
  source 1..120: mol_type = other DNA
gaagttgatatttgcagacctttcgtagaaaaacatattgctctaattaatcctaagttgcttattttagtcggtagcactgctgcaacgagtttacttggaaaaaatgcatgtattact

SEQ ID NO: 2846 - DNA, 120 bp, synthetic construct
  source 1..120: mol_type = other DNA
cttattttagtcggtagcactgctgcaacgagtttacttggaaaaaatgcatgtattactaaaattagacaagaatattatttttatacaaataaatatatatcaactcctattcaaact

SEQ ID NO: 2847 - DNA, 120 bp, synthetic construct
  source 1..120: mol_type = other DNA
aaaattagacaagaatattatttttatacaaataaatatatatcaactcctattcaaactactgcaatctttcaccctgcatacttacttagacaacctatgcaaaaacgtacctcttgg

SEQ ID NO: 2848 - DNA, 120 bp, synthetic construct
  source 1..120: mol_type = other DNA
actgcaatctttcaccctgcatacttacttagacaacctatgcaaaaacgtacctcttggtatgatctactaaagattaaggaatatttggtgaataatagagtcattgcataacttgta

SEQ ID NO: 2849 - DNA, 120 bp, synthetic construct
  source 1..120: mol_type = other DNA
tatgatctactaaagattaaggaatatttggtgaataatagagtcattgcataacttgtatatctaatactattatatgttttctatgtatttaagcttaatatgtgtatgacaaataca

SEQ ID NO: 2850 - DNA, 120 bp, synthetic construct
  source 1..120: mol_type = other DNA
tatctaatactattatatgttttctatgtatttaagcttaatatgtgtatgacaaatacaatttttataacagcaaactgtatttaagatttgttagaaattagatctcataacactgag

SEQ ID NO: 2851 - DNA, 120 bp, synthetic construct
  source 1..120: mol_type = other DNA
atttttataacagcaaactgtatttaagatttgttagaaattagatctcataacactgagattagtgcacttagaatatgaattttttaaataaaatgaatgtcatatgagcttatgttt

SEQ ID NO: 2852 - DNA, 120 bp, synthetic construct
  source 1..120: mol_type = other DNA
attagtgcacttagaatatgaattttttaaataaaatgaatgtcatatgagcttatgttttttgttaaaggttatattaaatgcatataataaagatacacaagaagaaatttatcaatg

SEQ ID NO: 2853 - DNA, 120 bp, synthetic construct
  source 1..120: mol_type = other DNA
tttgttaaaggttatattaaatgcatataataaagatacacaagaagaaatttatcaatgaaattgtttgtgttatgtggtaaagtttacagattctttaaaagaaaaattgatagtatg

SEQ ID NO: 2854 - DNA, 120 bp, synthetic construct
  source 1..120: mol_type = other DNA
aaattgtttgtgttatgtggtaaagtttacagattctttaaaagaaaaattgatagtatggtatattgaagtgttagtgcaatatttcatggatcaaaataaggagttattttttgttac

SEQ ID NO: 2855 - DNA, 120 bp, synthetic construct
  source 1..120: mol_type = other DNA
gtatattgaagtgttagtgcaatatttcatggatcaaaataaggagttattttttgttactgtttgttattgttaataaagctaatataaaaatgtaatctgaactttaacaataatctt

SEQ ID NO: 2856 - DNA, 120 bp, synthetic construct
  source 1..120: mol_type = other DNA
tgtttgttattgttaataaagctaatataaaaatgtaatctgaactttaacaataatctttatcaaagcttttaacttatagatgaaagtagaagagtatgcgtttttaattttcatgaa

SEQ ID NO: 2857 - DNA, 120 bp, synthetic construct
  source 1..120: mol_type = other DNA
tatcaaagcttttaacttatagatgaaagtagaagagtatgcgtttttaattttcatgaaccttacacgttgagcaagatatcaaaaaaatttataaatcgtaattcatttctaatttcc

SEQ ID NO: 2858 - DNA, 120 bp, synthetic construct
  source 1..120: mol_type = other DNA
ccttacacgttgagcaagatatcaaaaaaatttataaatcgtaattcatttctaatttcctaaaattagggttatactgactgaatgaggtatatacattatgactaatggcaataataa

SEQ ID NO: 2859 - DNA, 120 bp, synthetic construct
  source 1..120: mol_type = other DNA
taaaattagggttatactgactgaatgaggtatatacattatgactaatggcaataataataacttagaatttgcagaattaaaaattagaggtaaactatttaagttacctatacttaa

SEQ ID NO: 2860 - DNA, 120 bp, synthetic construct
  source 1..120: mol_type = other DNA
taacttagaatttgcagaattaaaaattagaggtaaactatttaagttacctatacttaaagcaagtatcggtaaagatgtaatcgatataagtagggtatctgcggaagccgattactt

SEQ ID NO: 2861 - DNA, 120 bp, synthetic construct
  source 1..120: mol_type = other DNA
agcaagtatcggtaaagatgtaatcgatataagtagggtatctgcggaagccgattactttacttatgatccgggttttatgtctactgcttcttgtcaatctactatcacatatataga

SEQ ID NO: 2862 - DNA, 120 bp, synthetic construct
  source 1..120: mol_type = other DNA
tacttatgatccgggttttatgtctactgcttcttgtcaatctactatcacatatatagacggtgataaaggcatattatggtatcgaggatatgatattaaagacttagctgagaaaag

SEQ ID NO: 2863 - DNA, 120 bp, synthetic construct
  source 1..120: mol_type = other DNA
cggtgataaaggcatattatggtatcgaggatatgatattaaagacttagctgagaaaagtgattttttagaagtggcatatttgatgatttatggggagctaccaagtagtgatcagta

SEQ ID NO: 2864 - DNA, 120 bp, synthetic construct
  source 1..120: mol_type = other DNA
tgattttttagaagtggcatatttgatgatttatggggagctaccaagtagtgatcagtattgtaattttactaaaaaggttgctcatcattcattagtgaatgaaagattacactattt

SEQ ID NO: 2865 - DNA, 120 bp, synthetic construct
  source 1..120: mol_type = other DNA
ttgtaattttactaaaaaggttgctcatcattcattagtgaatgaaagattacactatttatttcaaaccttttgtagttcttctcatcctatggctattatgcttgcagctgttggttc

SEQ ID NO: 2866 - DNA, 120 bp, synthetic construct
  source 1..120: mol_type = other DNA
atttcaaaccttttgtagttcttctcatcctatggctattatgcttgcagctgttggttctctttcagcattctatcctgatttattaaattttaatgaaacagactatgaacttaccgc

SEQ ID NO: 2867 - DNA, 120 bp, synthetic construct
  source 1..120: mol_type = other DNA
tctttcagcattctatcctgatttattaaattttaatgaaacagactatgaacttaccgctattagaatgattgctaagatacctactatcgctgcaatgtcttataaatattctatagg

SEQ ID NO: 2868 - DNA, 120 bp, synthetic construct
  source 1..120: mol_type = other DNA
tattagaatgattgctaagatacctactatcgctgcaatgtcttataaatattctatagggcaaccgtttatttatcctgataattcattagattttaccgaaaattttctacatatgat

SEQ ID NO: 2869 - DNA, 120 bp, synthetic construct
  source 1..120: mol_type = other DNA
gcaaccgtttatttatcctgataattcattagattttaccgaaaattttctacatatgatgtttgcaactccttgtactaaatataaagtaaatccaataataaaaaatgctcttaataa

SEQ ID NO: 2870 - DNA, 120 bp, synthetic construct
  source 1..120: mol_type = other DNA
gtttgcaactccttgtactaaatataaagtaaatccaataataaaaaatgctcttaataagatatttatcttacatgcagaccatgagcagaatgcttctacttcaacagttcggattgc

SEQ ID NO: 2871 - DNA, 120 bp, synthetic construct
  source 1..120: mol_type = other DNA
gatatttatcttacatgcagaccatgagcagaatgcttctacttcaacagttcggattgctggctcatcaggagctaatccttttgcatgtattagcactggtattgcatcactttgggg

SEQ ID NO: 2872 - DNA, 120 bp, synthetic construct
  source 1..120: mol_type = other DNA
tggctcatcaggagctaatccttttgcatgtattagcactggtattgcatcactttgggggcctgctcacggcggggctaatgaagcagtgataaatatgcttaaagaaattggcagttc

SEQ ID NO: 2873 - DNA, 120 bp, synthetic construct
  source 1..120: mol_type = other DNA
gcctgctcacggcggggctaatgaagcagtgataaatatgcttaaagaaattggcagttctgagaatattcctaaatatgtagctaaagctaaagataagaatgatccatttaggttaat

SEQ ID NO: 2874 - DNA, 120 bp, synthetic construct
  source 1..120: mol_type = other DNA
tgagaatattcctaaatatgtagctaaagctaaagataagaatgatccatttaggttaatgggttttggtcatcgagtatataaaagctatgacccgcgtgccgcagtacttaaagaaac

SEQ ID NO: 2875 - DNA, 120 bp, synthetic construct
  source 1..120: mol_type = other DNA
gggttttggtcatcgagtatataaaagctatgacccgcgtgccgcagtacttaaagaaacttgtaaagaagtattaaatgaattaggtcagttagacaataatccgctgttacaaatagc

SEQ ID NO: 2876 - DNA, 120 bp, synthetic construct
  source 1..120: mol_type = other DNA
ttgtaaagaagtattaaatgaattaggtcagttagacaataatccgctgttacaaatagcaatagaacttgaagctctcgctcttaaagatgaatattttattgaaagaaaattatatcc

SEQ ID NO: 2877 - DNA, 120 bp, synthetic construct
  source 1..120: mol_type = other DNA
aatagaacttgaagctctcgctcttaaagatgaatattttattgaaagaaaattatatccaaatgttgatttttattcaggcattatctataaagctatgggtataccgtcgcaaatgtt

SEQ ID NO: 2878 - DNA, 120 bp, synthetic construct
  source 1..120: mol_type = other DNA
aaatgttgatttttattcaggcattatctataaagctatgggtataccgtcgcaaatgttcactgtactttttgcaatagcaagaaccgtaggttggatggcacaatggaaagaaatgca

SEQ ID NO: 2879 - DNA, 120 bp, synthetic construct
  source 1..120: mol_type = other DNA
cactgtactttttgcaatagcaagaaccgtaggttggatggcacaatggaaagaaatgcacgaagatcctgaacaaaaaatcagtagacctagacagctttacactggttatctacatag

SEQ ID NO: 2880 - DNA, 120 bp, synthetic construct
  source 1..120: mol_type = other DNA
cgaagatcctgaacaaaaaatcagtagacctagacagctttacactggttatctacatagagagtataagtgtattgtagaaagaaagtgacgcattaaaattgtatgcattagcaattt

SEQ ID NO: 2881 - DNA, 120 bp, synthetic construct
  source 1..120: mol_type = other DNA
agagtataagtgtattgtagaaagaaagtgacgcattaaaattgtatgcattagcaatttagtgatttagatgaagcattaagaaaatctaattaattcatctaaaattttttaggaaca

SEQ ID NO: 2882 - DNA, 120 bp, synthetic construct
  source 1..120: mol_type = other DNA
agtgatttagatgaagcattaagaaaatctaattaattcatctaaaattttttaggaacatatattaataaaaagatgttttttatactatcattgtccaatgtactataatttttattt

SEQ ID NO: 2883 - DNA, 120 bp, synthetic construct
  source 1..120: mol_type = other DNA
tatattaataaaaagatgttttttatactatcattgtccaatgtactataatttttatttttcaaacattccaaaacctagtaaaattataatatgaaggttgaatactattcaataaat

SEQ ID NO: 2884 - DNA, 120 bp, synthetic construct
  source 1..120: mol_type = other DNA
ttcaaacattccaaaacctagtaaaattataatatgaaggttgaatactattcaataaattcacatctgtggttctttcagaaaattaagaagaaatttatattataactaacaactttt

SEQ ID NO: 2885 - DNA, 120 bp, synthetic construct
  source 1..120: mol_type = other DNA
tcacatctgtggttctttcagaaaattaagaagaaatttatattataactaacaacttttaaatttttaaacacttatacgactaacaaagaaattaaaatgcattttattgatgaagtt

SEQ ID NO: 2886 - DNA, 120 bp, synthetic construct
  source 1..120: mol_type = other DNA
aaatttttaaacacttatacgactaacaaagaaattaaaatgcattttattgatgaagttaaaatatatataaaaggtggaaacggcggcaatggttgtattagttttcatcgtgagaaa

SEQ ID NO: 2887 - DNA, 120 bp, synthetic construct
  source 1..120: mol_type = other DNA
aaaatatatataaaaggtggaaacggcggcaatggttgtattagttttcatcgtgagaaatttattgatagaggtggaccagatggtggagatggtggatttggtggcagtgttattttt

SEQ ID NO: 2888 - DNA, 120 bp, synthetic construct
  source 1..120: mol_type = other DNA
tttattgatagaggtggaccagatggtggagatggtggatttggtggcagtgttatttttagaagtaatcaccatattaatacactagtgaattatcgatatcaacaacattttaccgca

SEQ ID NO: 2889 - DNA, 120 bp, synthetic construct
  source 1..120: mol_type = other DNA
agaagtaatcaccatattaatacactagtgaattatcgatatcaacaacattttaccgcagaaaacggcgaaaacggtaaagggtcaaatcgaagtggaaaatcaggaaaatcattaatt

SEQ ID NO: 2890 - DNA, 120 bp, synthetic construct
  source 1..120: mol_type = other DNA
gaaaacggcgaaaacggtaaagggtcaaatcgaagtggaaaatcaggaaaatcattaattcttgatgttccagtcggcactcaaattttttctcaggatggcgatatattattgtatgat

SEQ ID NO: 2891 - DNA, 120 bp, synthetic construct
  source 1..120: mol_type = other DNA
cttgatgttccagtcggcactcaaattttttctcaggatggcgatatattattgtatgatttcactgaagatgaaaaaagttttgaaataattaaaggaggatgtggtggtcttggtaac

SEQ ID NO: 2892 - DNA, 120 bp, synthetic construct
  source 1..120: mol_type = other DNA
ttcactgaagatgaaaaaagttttgaaataattaaaggaggatgtggtggtcttggtaacagccatttcaaaacatctgttaatcaagcaccaagaaagagtacagaaggggaaattgct

SEQ ID NO: 2893 - DNA, 120 bp, synthetic construct
  source 1..120: mol_type = other DNA
agccatttcaaaacatctgttaatcaagcaccaagaaagagtacagaaggggaaattgctgaagaaatgtggattcatttgagactaaaactactctctgatgtcggacttattggatta

SEQ ID NO: 2894 - DNA, 120 bp, synthetic construct
  source 1..120: mol_type = other DNA
gaagaaatgtggattcatttgagactaaaactactctctgatgtcggacttattggattacccaatgccggtaaatctacttttttatctgttgtaacggcagcaaaacctaagattgct

SEQ ID NO: 2895 - DNA, 120 bp, synthetic construct
  source 1..120: mol_type = other DNA
cccaatgccggtaaatctacttttttatctgttgtaacggcagcaaaacctaagattgctgattatccatttactactttagtgccgaatcttggagttgtatatattgatgatgaagag

SEQ ID NO: 2896 - DNA, 120 bp, synthetic construct
  source 1..120: mol_type = other DNA
gattatccatttactactttagtgccgaatcttggagttgtatatattgatgatgaagagtttgtgatagctgatattccaggtttgattgccggagctcatcaagggtacggactagga

SEQ ID NO: 2897 - DNA, 120 bp, synthetic construct
  source 1..120: mol_type = other DNA
tttgtgatagctgatattccaggtttgattgccggagctcatcaagggtacggactaggagataaattcttaaagcatatagaaagatgtaatgtattaatacatttaatagatggtgct

SEQ ID NO: 2898 - DNA, 120 bp, synthetic construct
  source 1..120: mol_type = other DNA
gataaattcttaaagcatatagaaagatgtaatgtattaatacatttaatagatggtgctagtaataatgtaattgcagattataatacggtacgttttgaacttgagtcatattctgat

SEQ ID NO: 2899 - DNA, 120 bp, synthetic construct
  source 1..120: mol_type = other DNA
agtaataatgtaattgcagattataatacggtacgttttgaacttgagtcatattctgattatctaaaaaataaaatcgaaattatatgtcttaataaatgtgatgttcttgttgatgaa

SEQ ID NO: 2900 - DNA, 120 bp, synthetic construct
  source 1..120: mol_type = other DNA
tatctaaaaaataaaatcgaaattatatgtcttaataaatgtgatgttcttgttgatgaagaaatacaaaaaaaaataaaaaagcttcaaaaagttactaataaagtagtgcaccctatc

SEQ ID NO: 2901 - DNA, 120 bp, synthetic construct
  source 1..120: mol_type = other DNA
gaaatacaaaaaaaaataaaaaagcttcaaaaagttactaataaagtagtgcaccctatctctacttataataatcaaggtgtgaataaaatagttaaacttgctttagagattataaaa

SEQ ID NO: 2902 - DNA, 120 bp, synthetic construct
  source 1..120: mol_type = other DNA
tctacttataataatcaaggtgtgaataaaatagttaaacttgctttagagattataaaaaatcaaaaatactaatatagtattagctaatctacgattactaatcatgacttagttgta

SEQ ID NO: 2903 - DNA, 120 bp, synthetic construct
  source 1..120: mol_type = other DNA
aatcaaaaatactaatatagtattagctaatctacgattactaatcatgacttagttgtattatacagtaatgaaaattaataaattttaaattaagctaatacgttgttcttcggtttc

SEQ ID NO: 2904 - DNA, 120 bp, synthetic construct
  source 1..120: mol_type = other DNA
ttatacagtaatgaaaattaataaattttaaattaagctaatacgttgttcttcggtttcaagatatttctctagttcttccttagtatatctcttttctttaagttgtatttcattatt

SEQ ID NO: 2905 - DNA, 120 bp, synthetic construct
  source 1..120: mol_type = other DNA
aagatatttctctagttcttccttagtatatctcttttctttaagttgtatttcattattaaatatatattgtacagttttatcttctaatgcaggacctttaagtccctcaatcgctct

SEQ ID NO: 2906 - DNA, 120 bp, synthetic construct
  source 1..120: mol_type = other DNA
aaatatatattgtacagttttatcttctaatgcaggacctttaagtccctcaatcgctctaggattatttttataaaaatcaaatatcatattttcttgtcctggaaaattacgtgcttg

SEQ ID NO: 2907 - DNA, 120 bp, synthetic construct
  source 1..120: mol_type = other DNA
aggattatttttataaaaatcaaatatcatattttcttgtcctggaaaattacgtgcttgctgcataataatttttttgaaatcatcaggctctagttgcaaatttttaaattttgcgta

SEQ ID NO: 2908 - DNA, 120 bp, synthetic construct
  source 1..120: mol_type = other DNA
ctgcataataatttttttgaaatcatcaggctctagttgcaaatttttaaattttgcgtattcagcaagtaataaacctattcgtacacgacgtagagctaatttattataatattctgt

SEQ ID NO: 2909 - DNA, 120 bp, synthetic construct
  source 1..120: mol_type = other DNA
ttcagcaagtaataaacctattcgtacacgacgtagagctaatttattataatattctgttatttctttagaggatttaccgtttaataatgatccatcatgtttatttttatcagtttc

SEQ ID NO: 2910 - DNA, 120 bp, synthetic construct
  source 1..120: mol_type = other DNA
tatttctttagaggatttaccgtttaataatgatccatcatgtttatttttatcagtttcagactttaaaatatttttttcttgctctaataaagattcaggtacatcaaaatctaacaa

SEQ ID NO: 2911 - DNA, 120 bp, synthetic construct
  source 1..120: mol_type = other DNA
agactttaaaatatttttttcttgctctaataaagattcaggtacatcaaaatctaacaatttttctaacttatcaaataagttcattttcattatagtattaatagcttcttctgattc

SEQ ID NO: 2912 - DNA, 120 bp, synthetic construct
  source 1..120: mol_type = other DNA
tttttctaacttatcaaataagttcattttcattatagtattaatagcttcttctgattcgttttctatttgtttagcaaaatgtgtacgtaattcttcaaggctattactttggaattt

SEQ ID NO: 2913 - DNA, 120 bp, synthetic construct
  source 1..120: mol_type = other DNA
gttttctatttgtttagcaaaatgtgtacgtaattcttcaaggctattactttggaattttttagcaaactcctcatcaataatagtaggttctgcagtatgtactgctttaatttgtac

SEQ ID NO: 2914 - DNA, 120 bp, synthetic construct
  source 1..120: mol_type = other DNA
tttagcaaactcctcatcaataatagtaggttctgcagtatgtactgctttaatttgtactacaaaatgagcatctttacctgataaatttttatcatgataattttcaggaaaagtaac

SEQ ID NO: 2915 - DNA, 120 bp, synthetic construct
  source 1..120: mol_type = other DNA
tacaaaatgagcatctttacctgataaatttttatcatgataattttcaggaaaagtaacgttaacatctacttcattacctgttttagaacctattaattgttgttcaaaaccttgaat

SEQ ID NO: 2916 - DNA, 120 bp, synthetic construct
  source 1..120: mol_type = other DNA
gttaacatctacttcattacctgttttagaacctattaattgttgttcaaaaccttgaataagggtattactacctattactaccttaaaatcatttaatttgccaccatcaaaagctct

SEQ ID NO: 2917 - DNA, 120 bp, synthetic construct
  source 1..120: mol_type = other DNA
aagggtattactacctattactaccttaaaatcatttaatttgccaccatcaaaagctctatccttaatatatccaattgcatcaatagtaacctgatcaccatcttttatttttgtttt

SEQ ID NO: 2918 - DNA, 120 bp, synthetic construct
  source 1..120: mol_type = other DNA
atccttaatatatccaattgcatcaatagtaacctgatcaccatcttttatttttgttttactttctttagtataacattttgttaatgcagcaagtttttctaattgtatttcaacatc

SEQ ID NO: 2919 - DNA, 120 bp, synthetic construct
  source 1..120: mol_type = other DNA
actttctttagtataacattttgttaatgcagcaagtttttctaattgtatttcaacatcttgagagtttactgctaattttggacgatctagtgaaattttctttaaatccggaatggt

SEQ ID NO: 2920 - DNA, 120 bp, synthetic construct
  source 1..120: mol_type = other DNA
ttgagagtttactgctaattttggacgatctagtgaaattttctttaaatccggaatggtaattttaggcaacaactctatttttactgtaaattctaaatctttatcgggttcgttttg

SEQ ID NO: 2921 - DNA, 120 bp, synthetic construct
  source 1..120: mol_type = other DNA
aattttaggcaacaactctatttttactgtaaattctaaatctttatcgggttcgttttgtaattcttcaatttttggtctacctattatatttagattatactctttaataatgtgatt

SEQ ID NO: 2922 - DNA, 120 bp, synthetic construct
  source 1..120: mol_type = other DNA
taattcttcaatttttggtctacctattatatttagattatactctttaataatgtgatttactaaattgttaattcttttttctattatatcatgcctaacagaagtaccgtatttctt

SEQ ID NO: 2923 - DNA, 120 bp, synthetic construct
  source 1..120: mol_type = other DNA
tactaaattgttaattcttttttctattatatcatgcctaacagaagtaccgtatttcttcttaacaattgaaacaggtactttaccagctctaaaaccagctactttaacttttttggt

SEQ ID NO: 2924 - DNA, 120 bp, synthetic construct
  source 1..120: mol_type = other DNA
cttaacaattgaaacaggtactttaccagctctaaaaccagctactttaacttttttggttaaatcaagtaattctttttgtatgtcatcatctatctcacttaaaggagtagagattct

SEQ ID NO: 2925 - DNA, 120 bp, synthetic construct
  source 1..120: mol_type = other DNA
tttaacttttttggttaaatcaagtaattctttttgtatgtcatcatctatctcacttaaaggagtagagattcttgcatgaaaattcaatccttcgttttttaatacgataattcccat

SEQ ID NO: 2926 - DNA, 120 bp, synthetic construct
  source 1..120: mol_type = other DNA
attacgtacacattttgctaaacaaatagaaaatgagtcagaagaagctattaatactataatgaaaatgaacttatttgataagttagaaaaattgttagattttgatgtaccagaatc

SEQ ID NO: 2927 - DNA, 120 bp, synthetic construct
  source 1..120: mol_type = other DNA
aatgaaaatgaacttatttgataagttagaaaaattgttagattttgatgtaccagaatctttattagagcaagaaaaaaatattttaaaatccgaaaccgataaaaataaacatgatgg

SEQ ID NO: 2928 - DNA, 120 bp, synthetic construct
  source 1..120: mol_type = other DNA
tttattagagcaagaaaaaaatattttaaaatccgaaaccgataaaaataaacatgatggatcattattaaatgggaaatcctctaaagaaataatagaatattataataaattagcact

SEQ ID NO: 2929 - DNA, 120 bp, synthetic construct
  source 1..120: mol_type = other DNA
atcattattaaatgggaaatcctctaaagaaataatagaatattataataaattagcactacgacgtgtacgcataggcttattacttgctgagtacgcaaaatttaaaaatttacaact

SEQ ID NO: 2930 - DNA, 120 bp, synthetic construct
  source 1..120: mol_type = other DNA
acgacgtgtacgcataggcttattacttgctgagtacgcaaaatttaaaaatttacaactagagcctgatgatttgaaaaaagttattatgcagcaagcacgtaattttcctggacaaga

SEQ ID NO: 2931 - DNA, 120 bp, synthetic construct
  source 1..120: mol_type = other DNA
agagcctgatgatttgaaaaaagttattatgcagcaagcacgtaattttcctggacaagaaaatatgatatttgatttttacaaaaataatcctagagccattgaagggcttagaggtcc

SEQ ID NO: 2932 - DNA, 120 bp, synthetic construct
  source 1..120: mol_type = other DNA
aaatatgatatttgatttttacaaaaataatcctagagccattgaagggcttagaggtcctgcattagaagataaaactgtacaatatatatttaataatgaaatacaacttaaagaaaa

SEQ ID NO: 2933 - DNA, 120 bp, synthetic construct
  source 1..120: mol_type = other DNA
tgcattagaagataaaactgtacaatatatatttaataatgaaatacaacttaaagaaaagagatattctaaggaagagctagaaaaatatcttgaaaccgaagaacagcaacgtattag

SEQ ID NO: 2934 - DNA, 120 bp, synthetic construct
  source 1..120: mol_type = other DNA
gagatattctaaggaagagctagaaaaatatcttgaaaccgaagaacagcaacgtattagtttaatttaaagttaattaattgtcattgctataatacaacgtagaacaattaagtcatg

SEQ ID NO: 2935 - DNA, 120 bp, synthetic construct
  source 1..120: mol_type = other DNA
tttaatttaaagttaattaattgtcattgctataatacaacgtagaacaattaagtcatgattagtaatcgtagatttaggtagaaataataaatttaaatcagattttcttatttacta

SEQ ID NO: 2936 - DNA, 120 bp, synthetic construct
  source 1..120: mol_type = other DNA
attagtaatcgtagatttaggtagaaataataaatttaaatcagattttcttatttactatagttttactttacaaaaattggtgcacgtagttaatacttaaatattactatatttgat

SEQ ID NO: 2937 - DNA, 120 bp, synthetic construct
  source 1..120: mol_type = other DNA
tagttttactttacaaaaattggtgcacgtagttaatacttaaatattactatatttgattttttataatctctaaagcaagtttaactattttattcacacctagattagtataagtag

SEQ ID NO: 2938 - DNA, 120 bp, synthetic construct
  source 1..120: mol_type = other DNA
tttttataatctctaaagcaagtttaactattttattcacacctagattagtataagtagaaatagggtgcactactttattagtaactctctgaagcttctttatttttttttgtattt

SEQ ID NO: 2939 - DNA, 120 bp, synthetic construct
  source 1..120: mol_type = other DNA
aaatagggtgcactactttattagtaactctctgaagcttctttatttttttttgtatttcctcatcagtaagaacatcacatttattaatacatatgatttcgattttattttttaaat

SEQ ID NO: 2940 - DNA, 120 bp, synthetic construct
  source 1..120: mol_type = other DNA
cctcatcagtaagaacatcacatttattaatacatatgatttcgattttattttttaaataatccgaatatgattcaagttcaaaacgtacagtatcataatctgcgattacattatgac

SEQ ID NO: 2941 - DNA, 120 bp, synthetic construct
  source 1..120: mol_type = other DNA
aatccgaatatgattcaagttcaaaacgtacagtatcataatctgcgattacattatgactagaaccatctattaaatgtattaatacattacatctttctatatgctttaagaatttat

SEQ ID NO: 2942 - DNA, 120 bp, synthetic construct
  source 1..120: mol_type = other DNA
tagaaccatctattaaatgtattaatacattacatctttctatatgctttaagaatttatctccaagtccgtgtccttggtgagctcctgcaatcaaacctggaatatcagctattacaa

SEQ ID NO: 2943 - DNA, 120 bp, synthetic construct
  source 1..120: mol_type = other DNA
ctccaagtccgtgtccttggtgagctcctgcaatcaaacctggaatatcagctattacaaactcttcatcattaatatatacaactccaagatttggcactaaagtagtaaatggataat

SEQ ID NO: 2944 - DNA, 120 bp, synthetic construct
  source 1..120: mol_type = other DNA
actcttcatcattaatatatacaactccaagatttggcactaaagtagtaaatggataatcagcaatcttaggtttcgctgctgttacaacagataaaaaagtagatttacctgcattgg

SEQ ID NO: 2945 - DNA, 120 bp, synthetic construct
  source 1..120: mol_type = other DNA
cagcaatcttaggtttcgctgctgttacaacagataaaaaagtagatttacctgcattgggtaacccaacaagcccaacatcagaaagtagttttagtctcaaatgaatccacatttctt

SEQ ID NO: 2946 - DNA, 120 bp, synthetic construct
  source 1..120: mol_type = other DNA
gtaacccaacaagcccaacatcagaaagtagttttagtctcaaatgaatccacatttcttgcgcaatttctccttctgtacgctttcttggcgcttgattaacagatgttttgaaatggc

SEQ ID NO: 2947 - DNA, 120 bp, synthetic construct
  source 1..120: mol_type = other DNA
gcgcaatttctccttctgtacgctttcttggcgcttgattaacagatgttttgaaatggctgttaccaagaccaccacatcctcctttaattatttcaaaacttttttcatcttccgtga

SEQ ID NO: 2948 - DNA, 120 bp, synthetic construct
  source 1..120: mol_type = other DNA
tgttaccaagaccaccacatcctcctttaattatttcaaaacttttttcatcttccgtgaaatcatgcaataatatattgccgtcctcagaaaaaatttgagtaccgattggaacatcaa

SEQ ID NO: 2949 - DNA, 120 bp, synthetic construct
  source 1..120: mol_type = other DNA
aatcatgcaataatatattgccgtcctcagaaaaaatttgagtaccgattggaacatcaagaattaatgattttcctgatttaccactgcgatttgaacctttgccgtttccaccgtttt

SEQ ID NO: 2950 - DNA, 120 bp, synthetic construct
  source 1..120: mol_type = other DNA
gaattaatgattttcctgatttaccactgcgatttgaacctttgccgtttccaccgttttctgcgataaaatgctgttgatatcgatagttcactaatgtattaatatggtgattacttc

SEQ ID NO: 2951 - DNA, 120 bp, synthetic construct
  source 1..120: mol_type = other DNA
ctgcgataaaatgctgttgatatcgatagttcactaatgtattaatatggtgattacttctaaaaataacactgccaccaaatccaccatctccaccatccggtccacctctgtcaacaa

SEQ ID NO: 2952 - DNA, 120 bp, synthetic construct
  source 1..120: mol_type = other DNA
taaaaataacactgccaccaaatccaccatctccaccatccggtccacctctgtcaacaaatttctcacgatgaaaactaatacaaccattgccgccgtttccaccttttatatatattt

SEQ ID NO: 2953 - DNA, 120 bp, synthetic construct
  source 1..120: mol_type = other DNA
atttctcacgatgaaaactaatacaaccattgccgccgtttccaccttttatatatattttaacttcatcaataaaatgcattttactttcttgttagtgatataagtgttttaaaattt

SEQ ID NO: 2954 - DNA, 120 bp, synthetic construct
  source 1..120: mol_type = other DNA
taacttcatcaataaaatgcattttactttcttgttagtgatataagtgttttaaaatttaaaagttgttagtaagctttaattattataatataaattataaatttcctcttaatcttc

SEQ ID NO: 2955 - DNA, 120 bp, synthetic construct
  source 1..120: mol_type = other DNA
aaaagttgttagtaagctttaattattataatataaattataaatttcctcttaatcttctgattaatcttccaaaaggattgcagatgtgaatttatttaatggtattctatcttgatt

SEQ ID NO: 2956 - DNA, 120 bp, synthetic construct
  source 1..120: mol_type = other DNA
tgattaatcttccaaaaggattgcagatgtgaatttatttaatggtattctatcttgattatagaatgtgatattattctaatttttctaggtttccgtaatatttaaaaaataaaaatt

SEQ ID NO: 2957 - DNA, 120 bp, synthetic construct
  source 1..120: mol_type = other DNA
atagaatgtgatattattctaatttttctaggtttccgtaatatttaaaaaataaaaattatcgcgcattggacaacacataatacaaaaagcatcttttttattaaaatgatgattttt

SEQ ID NO: 2958 - DNA, 120 bp, synthetic construct
  source 1..120: mol_type = other DNA
atcgcgcattggacaacacataatacaaaaagcatcttttttattaaaatgatgatttttgctaaaaaattttagatgaagtaattatatttctaattcatcatctaaatcactaaattt

SEQ ID NO: 2959 - DNA, 120 bp, synthetic construct
  source 1..120: mol_type = other DNA
gctaaaaaattttagatgaagtaattatatttctaattcatcatctaaatcactaaatttatcacctttatatctcatataattttagtttgactttatgagacaaatttattaataacc

SEQ ID NO: 2960 - DNA, 120 bp, synthetic construct
  source 1..120: mol_type = other DNA
atcacctttatatctcatataattttagtttgactttatgagacaaatttattaataacctagtaaatagaattttaattcgtcactttctttctacaatacacttatattctctatgta

SEQ ID NO: 2961 - DNA, 120 bp, synthetic construct
  source 1..120: mol_type = other DNA
tagtaaatagaattttaattcgtcactttctttctacaatacacttatattctctatgtacataaccagtgtaaagttgtctaggtctactgattttttgttcaggatcttcgtgcattt

SEQ ID NO: 2962 - DNA, 120 bp, synthetic construct
  source 1..120: mol_type = other DNA
cataaccagtgtaaagttgtctaggtctactgattttttgttcaggatcttcgtgcatttctttccattgcgccatccaacctacggttcttgctattgcaaaaagtacagtgaacattt

SEQ ID NO: 2963 - DNA, 120 bp, synthetic construct
  source 1..120: mol_type = other DNA
ctttccattgcgccatccaacctacggttcttgctattgcaaaaagtacagtgaacatttgcgacggtatacccatagctttatagataatgcctgaataaaaatcaacatttggatata

SEQ ID NO: 2964 - DNA, 120 bp, synthetic construct
  source 1..120: mol_type = other DNA
gcgacggtatacccatagctttatagataatgcctgaataaaaatcaacatttggatataattttctctcaataaaatattcatctttaagagcaagagcttcaagttctattgctattt

SEQ ID NO: 2965 - DNA, 120 bp, synthetic construct
  source 1..120: mol_type = other DNA
attttctctcaataaaatattcatctttaagagcaagagcttcaagttctattgctatttgtaacaacggattattttctaactgccctagttcatttaatacttctttacaagtttctt

SEQ ID NO: 2966 - DNA, 120 bp, synthetic construct
  source 1..120: mol_type = other DNA
gtaacaacggattattttctaactgccctagttcatttaatacttctttacaagtttctttaagtactgcagcacgcgggtcataacttttatatactcgatgaccaaaacccattaacc

SEQ ID NO: 2967 - DNA, 120 bp, synthetic construct
  source 1..120: mol_type = other DNA
taagtactgcagcacgcgggtcataacttttatatactcgatgaccaaaacccattaacctaaatggatcatttttgtctttagctttagctacatatttaggaatattctcagaactac

SEQ ID NO: 2968 - DNA, 120 bp, synthetic construct
  source 1..120: mol_type = other DNA
taaatggatcatttttgtctttagctttagctacatatttaggaatattctcagaactaccaatttctttaagcatatttatcactgcttcattagctccaccgtgagcaggcccccaaa

SEQ ID NO: 2969 - DNA, 120 bp, synthetic construct
  source 1..120: mol_type = other DNA
caatttctttaagcatatttatcactgcttcattagctccaccgtgagcaggcccccaaagtgatgcaataccagtgctaatacatgcaaaaggattagctcctgatgagccagcaattc

SEQ ID NO: 2970 - DNA, 120 bp, synthetic construct
  source 1..120: mol_type = other DNA
gtgatgcaataccagtgctaatacatgcaaaaggattagctcctgatgagccagcaattcgtactgttgaagtagaagcattctgctcatggtctgcatgtaagataaatatcttattaa

SEQ ID NO: 2971 - DNA, 120 bp, synthetic construct
  source 1..120: mol_type = other DNA
gtactgttgaagtagaagcattctgctcatggtctgcatgtaagataaatatcttattaagcgcattttttattattggatttactttatatttagtacaaggagttgcaaacatcatat

SEQ ID NO: 2972 - DNA, 120 bp, synthetic construct
  source 1..120: mol_type = other DNA
gcgcattttttattattggatttactttatatttagtacaaggagttgcaaacatcatatgtagaaaattttcggtaaaatctaatgaattatcaggataaataaatggctgccctatag

SEQ ID NO: 2973 - DNA, 120 bp, synthetic construct
  source 1..120: mol_type = other DNA
gtagaaaattttcggtaaaatctaatgaattatcaggataaataaatggctgccctatagaatatttataagacattgcagcgatagtaggtatcttagcaatcattctaatagcggtaa

SEQ ID NO: 2974 - DNA, 120 bp, synthetic construct
  source 1..120: mol_type = other DNA
aatatttataagacattgcagcgatagtaggtatcttagcaatcattctaatagcggtaagttcatagtctgtttcattaaaattcaataaatcaggataaaatgctgaaagagaaccaa

SEQ ID NO: 2975 - DNA, 120 bp, synthetic construct
  source 1..120: mol_type = other DNA
gttcatagtctgtttcattaaaattcaataaatcaggataaaatgctgaaagagaaccaacagctgcaagcataatagccataggatgagaagaactacaaaaggtttgaaataaatagt

SEQ ID NO: 2976 - DNA, 120 bp, synthetic construct
  source 1..120: mol_type = other DNA
cagctgcaagcataatagccataggatgagaagaactacaaaaggtttgaaataaatagtgtaatctttcatttactaatgcatgatgagcaatctttgtagtaaaattatgatactgct

SEQ ID NO: 2977 - DNA, 120 bp, synthetic construct
  source 1..120: mol_type = other DNA
gtaatctttcatttactaatgcatgatgagcaatctttgtagtaaaattatgatactgctcactacttggtagttccccataaatcatcaaatatgccacttctaaaaaatcacttttct

SEQ ID NO: 2978 - DNA, 120 bp, synthetic construct
  source 1..120: mol_type = other DNA
cactacttggtagttccccataaatcatcaaatatgccacttctaaaaaatcacttttctcagctaagtctttaatatcatatcctcgatgccataagattcctttatcaccgtctatat

SEQ ID NO: 2979 - DNA, 120 bp, synthetic construct
  source 1..120: mol_type = other DNA
cagctaagtctttaatatcatatcctcgatgccataagattcctttatcaccgtctatatatgtgatggtagattgacaagaagcagtagacataaaacctggatcgtaagtaaagcaat

SEQ ID NO: 2980 - DNA, 120 bp, synthetic construct
  source 1..120: mol_type = other DNA
atgtgatggtagattgacaagaagcagtagacataaaacctggatcgtaagtaaagcaatcggcttccgcagataccctacttatatctattacatctttacctatacttgctttaagta

SEQ ID NO: 2981 - DNA, 120 bp, synthetic construct
  source 1..120: mol_type = other DNA
cggcttccgcagataccctacttatatctattacatctttacctatacttgctttaagtataggtaatttaaacattttacctctaatttttaattccgcaaattctaaattattattat

SEQ ID NO: 2982 - DNA, 120 bp, synthetic construct
  source 1..120: mol_type = other DNA
taggtaatttaaacattttacctctaatttttaattccgcaaattctaaattattattatttccattagtcataatgtatataccttattttacatcagtaagtataaccctaattatag

SEQ ID NO: 2983 - DNA, 120 bp, synthetic construct
  source 1..120: mol_type = other DNA
ttccattagtcataatgtatataccttattttacatcagtaagtataaccctaattataggaaattagaaatgaattatgatttataaattttctttgatatcttactcaacgtgtaagg

SEQ ID NO: 2984 - DNA, 120 bp, synthetic construct
  source 1..120: mol_type = other DNA
gaaattagaaatgaattatgatttataaattttctttgatatcttactcaacgtgtaaggttaatgaaaattaaaaacacatacacctctattttcgctataagttaaaagcttttttga

SEQ ID NO: 2985 - DNA, 120 bp, synthetic construct
  source 1..120: mol_type = other DNA
ttaatgaaaattaaaaacacatacacctctattttcgctataagttaaaagcttttttgaataaaaatgcaattttctagataatatttttatattagctttattatatgctatacctcc

SEQ ID NO: 2986 - DNA, 120 bp, synthetic construct
  source 1..120: mol_type = other DNA
ataaaaatgcaattttctagataatatttttatattagctttattatatgctatacctcctcctcttcttactatatcttttacagaaaaaataactccttattgtgatccataaaatat

SEQ ID NO: 2987 - DNA, 120 bp, synthetic construct
  source 1..120: mol_type = other DNA
tcctcttcttactatatcttttacagaaaaaataactccttattgtgatccataaaatattacgctaacacttcaatataccatactaatatttttttcttttaaaaaatctgtaaccac

SEQ ID NO: 2988 - DNA, 120 bp, synthetic construct
  source 1..120: mol_type = other DNA
tacgctaacacttcaatataccatactaatatttttttcttttaaaaaatctgtaaccacataatacaaacaatttcagtgataaatttcttttactatttctaaagtatttttatactt

SEQ ID NO: 2989 - DNA, 120 bp, synthetic construct
  source 1..120: mol_type = other DNA
ataatacaaacaatttcagtgataaatttcttttactatttctaaagtatttttatactttatttatcttatattacatgcatttaataacagaataattttataaaaaatatgagctgc

SEQ ID NO: 2990 - DNA, 120 bp, synthetic construct
  source 1..120: mol_type = other DNA
tatttatcttatattacatgcatttaataacagaataattttataaaaaatatgagctgcatttgatttaataaatttcaagtacactaatctagtgtcatgatatctaattttctaaca

SEQ ID NO: 2991 - DNA, 120 bp, synthetic construct
  source 1..120: mol_type = other DNA
atttgatttaataaatttcaagtacactaatctagtgtcatgatatctaattttctaacaaaaatatttactgtttgctgctataaacattgtatttgttacacatatattacgcttaaa

SEQ ID NO: 2992 - DNA, 120 bp, synthetic construct
  source 1..120: mol_type = other DNA
aaaatatttactgtttgctgctataaacattgtatttgttacacatatattacgcttaaatatatggtacgcttaaatatatggaaaaatatatatagtattagatgtacaagttatgca

SEQ ID NO: 2993 - DNA, 120 bp, synthetic construct
  source 1..120: mol_type = other DNA
tatatggtacgcttaaatatatggaaaaatatatatagtattagatgtacaagttatgcaataactctattattcactaaatattccttaatctttagtagatcataccaggaggtgcgt

SEQ ID NO: 2994 - DNA, 120 bp, synthetic construct
  source 1..120: mol_type = other DNA
ataactctattattcactaaatattccttaatctttagtagatcataccaggaggtgcgtttttgcataggttgtctcagtaaatatgcagggtgaaagattgcagtagtttgaatagga

SEQ ID NO: 2995 - DNA, 120 bp, synthetic construct
  source 1..120: mol_type = other DNA
ttttgcataggttgtctcagtaaatatgcagggtgaaagattgcagtagtttgaataggagttgatatatatttatttgtataaaagtaatattcttgtctaattttagtaatacatgaa

SEQ ID NO: 2996 - DNA, 120 bp, synthetic construct
  source 1..120: mol_type = other DNA
gttgatatatatttatttgtataaaagtaatattcttgtctaattttagtaatacatgaattttttccaagtaaactagttgcagcagtgctaccaactagaataagtaacttaggatta

SEQ ID NO: 2997 - DNA, 120 bp, synthetic construct
  source 1..120: mol_type = other DNA
ttttttccaagtaaactagttgcagcagtgctaccaactagaataagtaacttaggattaattagggcaatatgtttttctacaaaaggtctacaaatatcaacttcttccagagtcggt

SEQ ID NO: 2998 - DNA, 120 bp, synthetic construct
  source 1..120: mol_type = other DNA
attagggcaatatgtttttctacaaaaggtctacaaatatcaacttcttccagagtcggttgtctattagcaggaggacgccaaaataccatattagtaatataaaaattatttttccgt

SEQ ID NO: 2999 - DNA, 120 bp, synthetic construct
  source 1..120: mol_type = other DNA
tgtctattagcaggaggacgccaaaataccatattagtaatataaaaattatttttccgtgaaatccctatagcatacaacatattatcaagtaaattaccactttcaccacaaaaaggt

SEQ ID NO: 3000 - DNA, 120 bp, synthetic construct
  source 1..120: mol_type = other DNA
gaaatccctatagcatacaacatattatcaagtaaattaccactttcaccacaaaaaggtatcccttttaaatcttcagtattccctggagcttcacctattaacataattttagcttgt

SEQ ID NO: 3001 - DNA, 120 bp, synthetic construct
  source 1..120: mol_type = other DNA
atcccttttaaatcttcagtattccctggagcttcacctattaacataattttagcttgtggattaccatcaccgaaaactgtattagtagcaaatttcttaagttcgcaaccattaaaa

SEQ ID NO: 3002 - DNA, 120 bp, synthetic construct
  source 1..120: mol_type = other DNA
ggattaccatcaccgaaaactgtattagtagcaaatttcttaagttcgcaaccattaaaatttagtagagattctcgtagttctgcgatattattagctttatctgcaagagatcttgat

SEQ ID NO: 3003 - DNA, 120 bp, synthetic construct
  source 1..120: mol_type = other DNA
tttagtagagattctcgtagttctgcgatattattagctttatctgcaagagatcttgataaagtgatattatcatgaacattattattacatgccgcttctgttgtatgcataagttct

SEQ ID NO: 3004 - DNA, 120 bp, synthetic construct
  source 1..120: mol_type = other DNA
aaagtgatattatcatgaacattattattacatgccgcttctgttgtatgcataagttctacttgttgcttttcagtgagttcagtattattaggtattttttgtggtgtgtgttcgtag

SEQ ID NO: 3005 - DNA, 120 bp, synthetic construct
  source 1..120: mol_type = other DNA
acttgttgcttttcagtgagttcagtattattaggtattttttgtggtgtgtgttcgtagcaataatattcaacaccgattgcatttaaccatttaaaaatatcattcattatcttacaa

SEQ ID NO: 3006 - DNA, 120 bp, synthetic construct
  source 1..120: mol_type = other DNA
caataatattcaacaccgattgcatttaaccatttaaaaatatcattcattatcttacaataaaatatgttaacatatcatataccaaaggaactaaacaacacaaggcttgataaagct

SEQ ID NO: 3007 - DNA, 120 bp, synthetic construct
  source 1..120: mol_type = other DNA
taaaatatgttaacatatcatataccaaaggaactaaacaacacaaggcttgataaagctttatcatcactccttgaaaaggtctcaagaaatcaagttcaaaaagctattaagaattct

SEQ ID NO: 3008 - DNA, 120 bp, synthetic construct
  source 1..120: mol_type = other DNA
ttatcatcactccttgaaaaggtctcaagaaatcaagttcaaaaagctattaagaattcttgtgtacaaattaatgatgtgattatttctgattctgatgttttggtcaaggagaatgat

SEQ ID NO: 3009 - DNA, 120 bp, synthetic construct
  source 1..120: mol_type = other DNA
tgtgtacaaattaatgatgtgattatttctgattctgatgttttggtcaaggagaatgatactatattattttcttttaaagagcctgaagaactaaaaattacatcagcaaatataaca

SEQ ID NO: 3010 - DNA, 120 bp, synthetic construct
  source 1..120: mol_type = other DNA
actatattattttcttttaaagagcctgaagaactaaaaattacatcagcaaatataacacttgatataatttatgaagatgatgatttgatagtaattaacaaagcagcaggtataact

SEQ ID NO: 3011 - DNA, 120 bp, synthetic construct
  source 1..120: mol_type = other DNA
cttgatataatttatgaagatgatgatttgatagtaattaacaaagcagcaggtataactgtacatccaggtgcaaaacatcatgataatactcttgttaatgcattactgcaccataca

SEQ ID NO: 3012 - DNA, 120 bp, synthetic construct
  source 1..120: mol_type = other DNA
gtacatccaggtgcaaaacatcatgataatactcttgttaatgcattactgcaccatacaaagaatttatcagatattggttcagcagaaaggccaggaatagtacatcgtttagataaa

SEQ ID NO: 3013 - DNA, 120 bp, synthetic construct
  source 1..120: mol_type = other DNA
aagaatttatcagatattggttcagcagaaaggccaggaatagtacatcgtttagataaagaaactacaggtttgatggttgttgctaaaaataataaagctcatatgctacttgccaaa

SEQ ID NO: 3014 - DNA, 120 bp, synthetic construct
  source 1..120: mol_type = other DNA
gaaactacaggtttgatggttgttgctaaaaataataaagctcatatgctacttgccaaacagatagaacaaaggcaggtgatacgaaaatataaagcattagtttggggggtaattaat

SEQ ID NO: 3015 - DNA, 120 bp, synthetic construct
  source 1..120: mol_type = other DNA
cagatagaacaaaggcaggtgatacgaaaatataaagcattagtttggggggtaattaatccactagaaggaataattaataataatataggtcgtaatagaaataaccgcaaaaaaatg

SEQ ID NO: 3016 - DNA, 120 bp, synthetic construct
  source 1..120: mol_type = other DNA
ccactagaaggaataattaataataatataggtcgtaatagaaataaccgcaaaaaaatgacaatattaaaatacggtggaaaaaaagctgttacgcattacaagactttagagctattt

SEQ ID NO: 3017 - DNA, 120 bp, synthetic construct
  source 1..120: mol_type = other DNA
gaaataaccgcaaaaaaatgacaatattaaaatacggtggaaaaaaagctgttacgcattacaagactttagagctattttacggcggcactcttagtatggtggaatgcaagcttagta

SEQ ID NO: 3018 - DNA, 120 bp, synthetic construct
  source 1..120: mol_type = other DNA
caatgggagctatcggacctcgcttaggactcctaatcccatggagaaactcctagatgaggttcttgcccccggtgggccttacaacttaaccgtcggcagttgggtaagagaccacgt

SEQ ID NO: 3019 - DNA, 120 bp, synthetic construct
  source 1..120: mol_type = other DNA
ggttcttgcccccggtgggccttacaacttaaccgtcggcagttgggtaagagaccacgtccgctcaattgtcgagggcgcgtgggaagtgcgcgatgttgttaccgctgcccaaaagcg

SEQ ID NO: 3020 - DNA, 120 bp, synthetic construct
  source 1..120: mol_type = other DNA
ccgctcaattgtcgagggcgcgtgggaagtgcgcgatgttgttaccgctgcccaaaagcgggccatcgtagccgtgatacccagacctgtgttcacgcagatgcaggttagcgatcaccc

SEQ ID NO: 3021 - DNA, 120 bp, synthetic construct
  source 1..120: mol_type = other DNA
ggccatcgtagccgtgatacccagacctgtgttcacgcagatgcaggttagcgatcacccagcactccacgcaatttcgcggtacacccgccgccattggatcgagtggggccctaaaga

SEQ ID NO: 3022 - DNA, 120 bp, synthetic construct
  source 1..120: mol_type = other DNA
agcactccacgcaatttcgcggtacacccgccgccattggatcgagtggggccctaaagaagccctacacgtcctcatcgacccaagcccgggcttgctccgcgaggtcgctcgcgttga

SEQ ID NO: 3023 - DNA, 120 bp, synthetic construct
  source 1..120: mol_type = other DNA
agccctacacgtcctcatcgacccaagcccgggcttgctccgcgaggtcgctcgcgttgagcgccgttgggtcgcactgtgcctccacaggacggcacgcaaactcgccaccgccctggc

SEQ ID NO: 3024 - DNA, 120 bp, synthetic construct
  source 1..120: mol_type = other DNA
gcgccgttgggtcgcactgtgcctccacaggacggcacgcaaactcgccaccgccctggccgagacggccagcgaggcgtggcacgccgactacgtgtgcgcgctgcgtggcgcaccgag

SEQ ID NO: 3025 - DNA, 120 bp, synthetic construct
  source 1..120: mol_type = other DNA
cgagacggccagcgaggcgtggcacgccgactacgtgtgcgcgctgcgtggcgcaccgagcggccccttctacgtccaccctgaggacgtcccgcacggcggccgcgccgtggcggacag

SEQ ID NO: 3026 - DNA, 120 bp, synthetic construct
  source 1..120: mol_type = other DNA
cggccccttctacgtccaccctgaggacgtcccgcacggcggccgcgccgtggcggacagatgcctgctctactacacacccatgcagatgtgcgagctgatgcgcaccattgacgccac

SEQ ID NO: 3027 - DNA, 120 bp, synthetic construct
  source 1..120: mol_type = other DNA
atgcctgctctactacacacccatgcagatgtgcgagctgatgcgcaccattgacgccaccttgctcgtggcggttgacttgtggccggtcgcccttgcggcccacgtcggcgacgactg

SEQ ID NO: 3028 - DNA, 120 bp, synthetic construct
  source 1..120: mol_type = other DNA
cttgctcgtggcggttgacttgtggccggtcgcccttgcggcccacgtcggcgacgactgggacgacctgggcatcgcctggcatctcgaccatgacggcggctgccccgccgattgccg

SEQ ID NO: 3029 - DNA, 120 bp, synthetic construct
  source 1..120: mol_type = other DNA
ggacgacctgggcatcgcctggcatctcgaccatgacggcggctgccccgccgattgccgcggagccggcgctgggcccacgcccggctacacccgcccctgcaccacacgcatctacca

SEQ ID NO: 3030 - DNA, 120 bp, synthetic construct
  source 1..120: mol_type = other DNA
cggagccggcgctgggcccacgcccggctacacccgcccctgcaccacacgcatctaccaagtcttgccggacaccgcccaccccgggcgcctctaccgatgcgggccccgcctgtggac

SEQ ID NO: 3031 - DNA, 120 bp, synthetic construct
  source 1..120: mol_type = other DNA
agtcttgccggacaccgcccaccccgggcgcctctaccgatgcgggccccgcctgtggacgcgcgattgcgccgtggccgaactctcatgggaggttgcccaacactgcgggcaccaggc

SEQ ID NO: 3032 - DNA, 120 bp, synthetic construct
  source 1..120: mol_type = other DNA
gcgcgattgcgccgtggccgaactctcatgggaggttgcccaacactgcgggcaccaggcgcgcgtgcgcgccgtgcgatgcaccctccccatccgccacgtgcgcagcctccaacccag

SEQ ID NO: 3033 - DNA, 120 bp, synthetic construct
  source 1..120: mol_type = other DNA
gcgcgtgcgcgccgtgcgatgcaccctccccatccgccacgtgcgcagcctccaacccagcgcgcgggtccgactcccggacctcgtccatctcgccgaggtgggccggtggcggtggtt

SEQ ID NO: 3034 - DNA, 120 bp, synthetic construct
  source 1..120: mol_type = other DNA
cgcgcgggtccgactcccggacctcgtccatctcgccgaggtgggccggtggcggtggttcagcctcccccgccccgtgttccagcgcatgctgtcctactgcaagaccctgagccccga

SEQ ID NO: 3035 - DNA, 120 bp, synthetic construct
  source 1..120: mol_type = other DNA
cagcctcccccgccccgtgttccagcgcatgctgtcctactgcaagaccctgagccccgacgcgtactacagcgagcgcgtgttcaagtttaagaacgctctgagccacagcatcacgct

SEQ ID NO: 3036 - DNA, 120 bp, synthetic construct
  source 1..120: mol_type = other DNA
cgcgtactacagcgagcgcgtgttcaagtttaagaacgctctgagccacagcatcacgctcgcgggcaatgtgctgcaagaagggtggaagggcacgtgcgccgaggaagacgcgctgtg

SEQ ID NO: 3037 - DNA, 120 bp, synthetic construct
  source 1..120: mol_type = other DNA
cgcgggcaatgtgctgcaagaagggtggaagggcacgtgcgccgaggaagacgcgctgtgcgcatacgtggccttccgcgcgtggcagtctaacgccaggttggcggggatcatgaaagg

SEQ ID NO: 3038 - DNA, 120 bp, synthetic construct
  source 1..120: mol_type = other DNA
cgcatacgtggccttccgcgcgtggcagtctaacgccaggttggcggggatcatgaaaggcgccaagcgctgcgccgccgactctttgagcgtggccggctggctggacaccatttggga

SEQ ID NO: 3039 - DNA, 120 bp, synthetic construct
  source 1..120: mol_type = other DNA
cgccaagcgctgcgccgccgactctttgagcgtggccggctggctggacaccatttgggacgccattaagcgattcttcggcagcgtgcccctcgccgagcgcatggaggagtgggaaca

SEQ ID NO: 3040 - DNA, 120 bp, synthetic construct
  source 1..120: mol_type = other DNA
cgccattaagcgattcttcggcagcgtgcccctcgccgagcgcatggaggagtgggaacaggacgccgcggtcgccgccttcgaccgcggccccctcgaggacggcgggcgccacttgga

SEQ ID NO: 3041 - DNA, 120 bp, synthetic construct
  source 1..120: mol_type = other DNA
ggacgccgcggtcgccgccttcgaccgcggccccctcgaggacggcgggcgccacttggacaccgtgcaacccccaaaatcgccgccccgccctgagatcgccgcgacctggatcgttca

SEQ ID NO: 3042 - DNA, 120 bp, synthetic construct
  source 1..120: mol_type = other DNA
caccgtgcaacccccaaaatcgccgccccgccctgagatcgccgcgacctggatcgttcacgcagccagcgcagaccgccattgcgcgtgcgctccccgctgcgacgccccgcgcgaacg

SEQ ID NO: 3043 - DNA, 120 bp, synthetic construct
  source 1..120: mol_type = other DNA
cgcagccagcgcagaccgccattgcgcgtgcgctccccgctgcgacgccccgcgcgaacgtccttccgcgcccgccggcccgcccgatgacgaggcgctcatcccgccgtggctgttcgc

SEQ ID NO: 3044 - DNA, 120 bp, synthetic construct
  source 1..120: mol_type = other DNA
tccttccgcgcccgccggcccgcccgatgacgaggcgctcatcccgccgtggctgttcgccgagcgccgtgccctccgctgccgcgagtgggacttcgaggctctccgcgcgcgcgccga

SEQ ID NO: 3045 - DNA, 120 bp, synthetic construct
  source 1..120: mol_type = other DNA
cgagcgccgtgccctccgctgccgcgagtgggacttcgaggctctccgcgcgcgcgccgatacggcggccgcgcccgccccgctggccccacgccctgcgcggtaccccactgtgctcta

SEQ ID NO: 3046 - DNA, 120 bp, synthetic construct
  source 1..120: mol_type = other DNA
tacggcggccgcgcccgccccgctggccccacgccctgcgcggtaccccactgtgctctaccgccaccccgcccaccacggcccgtggctcacccttgacgagccgggcgaggctgacgc

SEQ ID NO: 3047 - DNA, 120 bp, synthetic construct
  source 1..120: mol_type = other DNA
ccgccaccccgcccaccacggcccgtggctcacccttgacgagccgggcgaggctgacgcggccctggtcttatgcgacccgctcggccagccgctccggggccccgaacgccatttcgc

SEQ ID NO: 3048 - DNA, 120 bp, synthetic construct
  source 1..120: mol_type = other DNA
ggccctggtcttatgcgacccgctcggccagccgctccggggccccgaacgccatttcgccgccggcgcgcatatgtgcgcgcaggcgcgggggctccaggctttcgtccgtgtcgtgcc

SEQ ID NO: 3049 - DNA, 120 bp, synthetic construct
  source 1..120: mol_type = other DNA
cgccggcgcgcatatgtgcgcgcaggcgcgggggctccaggctttcgtccgtgtcgtgcctccacccgagcgcccctgggccgacgggggcgccagagcgtgggcaaagttcttccgcgg

SEQ ID NO: 3050 - DNA, 120 bp, synthetic construct
  source 1..120: mol_type = other DNA
tccacccgagcgcccctgggccgacgggggcgccagagcgtgggcaaagttcttccgcggctgcgcctgggcgcagcgcttgctcggcgagccggcagtcatgcacctcccatacaccga

SEQ ID NO: 3051 - DNA, 120 bp, synthetic construct
  source 1..120: mol_type = other DNA
ctgcgcctgggcgcagcgcttgctcggcgagccggcagtcatgcacctcccatacaccgatggcgatgtgccacagctgatcgcgctggccttgcgcacgctggcccaacagggggccgc

SEQ ID NO: 3052 - DNA, 120 bp, synthetic construct
  source 1..120: mol_type = other DNA
tggcgatgtgccacagctgatcgcgctggccttgcgcacgctggcccaacagggggccgccttggcactctccgtgcgtgacctgcccgggggtgcagcgttcgacgcaaatgcggtcac

SEQ ID NO: 3053 - DNA, 120 bp, synthetic construct
  source 1..120: mol_type = other DNA
cttggcactctccgtgcgtgacctgcccgggggtgcagcgttcgacgcaaatgcggtcaccgccgctgtgcgcgctggccccggccagtccgcggccacgtcaccgccacctggcgaccc

SEQ ID NO: 3054 - DNA, 120 bp, synthetic construct
  source 1..120: mol_type = other DNA
cgccgctgtgcgcgctggccccggccagtccgcggccacgtcaccgccacctggcgaccccccgccgccgcgccgcgcacggcgttcgcaacggcactcggacgcccgcggcactccgcc

SEQ ID NO: 3055 - DNA, 120 bp, synthetic construct
  source 1..120: mol_type = other DNA
cccgccgccgcgccgcgcacggcgttcgcaacggcactcggacgcccgcggcactccgccccccgcgcctgcgcccgacccgccgccgcccgcccccagcccgcccgcgccaccccgcgc

SEQ ID NO: 3056 - DNA, 120 bp, synthetic construct
  source 1..120: mol_type = other DNA
ccccgcgcctgcgcccgacccgccgccgcccgcccccagcccgcccgcgccaccccgcgcgggtgactcggcccctcccacccctgcggggccggcggatcgcgcgcgcgacgccgagct

SEQ ID NO: 3057 - DNA, 120 bp, synthetic construct
  source 1..120: mol_type = other DNA
gggtgactcggcccctcccacccctgcggggccggcggatcgcgcgcgcgacgccgagctggaggtcgcctgcgaaccgagcggcccccccgcggcagccaaggcagacccagacagcga

SEQ ID NO: 3058 - DNA, 120 bp, synthetic construct; identical to SEQ ID NO: 3057
  source 1..120: mol_type = other DNA

SEQ ID NO: 3059 - DNA, 120 bp, synthetic construct
  source 1..120: mol_type = other DNA
catcgttgagagttacgcccgcgccgccggacccgtgcacctccgagtccgcgacatcatggacccaccgcccggctgcaaggttgtggtcaacgccgccaacgaggggctgctggccgg

SEQ ID NO: 3060 - DNA, 120 bp, synthetic construct
  source 1..120: mol_type = other DNA
ggacccaccgcccggctgcaaggttgtggtcaacgccgccaacgaggggctgctggccggctctggcgtgtgtggcgccatctttgccaacgccacggcggccctcgctgcagactgccg

SEQ ID NO: 3061 - DNA, 120 bp, synthetic construct
  source 1..120: mol_type = other DNA
ctctggcgtgtgtggcgccatctttgccaacgccacggcggccctcgctgcagactgccggcgcctcgccccatgccccaccggcgaggcagtggcgacacccggccatggctgcgggta

SEQ ID NO: 3062 - DNA, 120 bp, synthetic construct
  source 1..120: mol_type = other DNA
gcgcctcgccccatgccccaccggcgaggcagtggcgacacccggccatggctgcgggtacacccacatcatccacgccgttgcgccgcggcgtcctcgggaccccgccgccctcgagga

SEQ ID NO: 3063 - DNA, 120 bp, synthetic construct
  source 1..120: mol_type = other DNA
cacccacatcatccacgccgttgcgccgcggcgtcctcgggaccccgccgccctcgaggagggcgaagcactgctcgagcgcgcctaccgcagcatcgtcgcgctggccgctgcgcgcag

SEQ ID NO: 3064 - DNA, 120 bp, synthetic construct
  source 1..120: mol_type = other DNA
gggcgaagcactgctcgagcgcgcctaccgcagcatcgtcgcgctggccgctgcgcgcaggtgggcgtgtgtcgcgtgccccctcctcggcgctggcgtctacggctggtctgctgcgga

SEQ ID NO: 3065 - DNA, 120 bp, synthetic construct
  source 1..120: mol_type = other DNA
gtgggcgtgtgtcgcgtgccccctcctcggcgctggcgtctacggctggtctgctgcggagtccctccgagccgcgcttgcggctacgcgcgccgagcccgccgagcgcgtgagcctgca

SEQ ID NO: 3066 - DNA, 120 bp, synthetic construct
  source 1..120: mol_type = other DNA
gtccctccgagccgcgcttgcggctacgcgcgccgagcccgccgagcgcgtgagcctgcacatctgccaccccgaccgcgccacgctgacgcacgcctccgtgctcgtcggcgcggggct

SEQ ID NO: 3067 - DNA, 120 bp, synthetic construct
  source 1..120: mol_type = other DNA
catctgccaccccgaccgcgccacgctgacgcacgcctccgtgctcgtcggcgcggggctcgctgccaggcgcgttagtcctcccccggccgagcccctcgcaccttgccccgccggtgc

SEQ ID NO: 3068 - DNA, 120 bp, synthetic construct
  source 1..120: mol_type = other DNA
cgctgccaggcgcgttagtcctcccccggccgagcccctcgcaccttgccccgccggtgctccgggcccgccggctcagcgcagctcgtcgcctccagcggcaccccttggggatgccac

SEQ ID NO: 3069 - DNA, 120 bp, synthetic construct
  source 1..120: mol_type = other DNA
tccgggcccgccggctcagcgcagctcgtcgcctccagcggcaccccttggggatgccaccgcgcccgagcctcgcggatgccaggggtgcgaactctgccggtacacgcgcgtcaccaa

SEQ ID NO: 3070 - DNA, 120 bp, synthetic construct
  source 1..120: mol_type = other DNA
cgcgcccgagcctcgcggatgccaggggtgcgaactctgccggtacacgcgcgtcaccaacgaccgcgcctatgtcaacctgtggctcgaacgcgaccgcggcgccaccagctgggcgat

SEQ ID NO: 3071 - DNA, 120 bp, synthetic construct
  source 1..120: mol_type = other DNA
cgaccgcgcctatgtcaacctgtggctcgaacgcgaccgcggcgccaccagctgggcgatgcgcattcccgaggtggtcgtctacggcccggagcacctcgccacgcatttcccattaaa

SEQ ID NO: 3072 - DNA, 120 bp, synthetic construct
  source 1..120: mol_type = other DNA
gcgcattcccgaggtggtcgtctacggcccggagcacctcgccacgcatttcccattaaaccactacagtgtgctcaagcccgcggaggttaggcccccgcgaggcatgtgcgggagtga

SEQ ID NO: 3073 - DNA, 120 bp, synthetic construct
  source 1..120: mol_type = other DNA
ccactacagtgtgctcaagcccgcggaggttaggcccccgcgaggcatgtgcgggagtgacatgtggcgctgccgcggctggcagggcatgccgcaagtgcgctgcaccccctccaacgc

SEQ ID NO: 3074 - DNA, 120 bp, synthetic construct
  source 1..120: mol_type = other DNA
catgtggcgctgccgcggctggcagggcatgccgcaagtgcgctgcaccccctccaacgctcacgccgccctgtgccgcacaggcgtgccccctcgagtgagcacgcgaggcagcgagct

SEQ ID NO: 3075 - DNA, 120 bp, synthetic construct
  source 1..120: mol_type = other DNA
tcacgccgccctgtgccgcacaggcgtgccccctcgagtgagcacgcgaggcagcgagctagacccaaacacctgctggctccgcgccgccgccaacgttgcgcaggctgcgcgcgcctg

SEQ ID NO: 3076 - DNA, 120 bp, synthetic construct
  source 1..120: mol_type = other DNA
agacccaaacacctgctggctccgcgccgccgccaacgttgcgcaggctgcgcgcgcctgcggcgcctacacgagtgccgggtgccccaagtgcgcctacggccgcgccctgagcgaagc

SEQ ID NO: 3077 - DNA, 120 bp, synthetic construct
  source 1..120: mol_type = other DNA
cggcgcctacacgagtgccgggtgccccaagtgcgcctacggccgcgccctgagcgaagcccgcactcacgaggactttgccgccctgagccagcggtggagcgctagccacgccgatgc

SEQ ID NO: 3078 - DNA, 120 bp, synthetic construct
  source 1..120: mol_type = other DNA
ccgcactcacgaggactttgccgccctgagccagcggtggagcgctagccacgccgatgcctcccctgacggcaccggagatcccctcgaccccctgatggagaccgtgggatgcgcctg

SEQ ID NO: 3079 - DNA, 120 bp, synthetic construct
  source 1..120: mol_type = other DNA
ctcccctgacggcaccggagatcccctcgaccccctgatggagaccgtgggatgcgcctgttcgcgcgtgtgggtcggctccgagcatgaggccccgcccgaccacctcctcgtgtccct

SEQ ID NO: 3080 - DNA, 120 bp, synthetic construct
  source 1..120: mol_type = other DNA
ttcgcgcgtgtgggtcggctccgagcatgaggccccgcccgaccacctcctcgtgtccctccaccgtgcccccaacggcccctggggcgtagtgctcgaggtgcgcgcgcgccccgaagg

SEQ ID NO: 3081 - DNA, 120 bp, synthetic construct
  source 1..120: mol_type = other DNA
ccaccgtgcccccaacggcccctggggcgtagtgctcgaggtgcgcgcgcgccccgaagggggcaaccccaccggccatttcgtctgcgcggttggcggtggcccacgccgcgtctcgga

SEQ ID NO: 3082 - DNA, 120 bp, synthetic construct
  source 1..120: mol_type = other DNA
gggcaaccccaccggccatttcgtctgcgcggttggcggtggcccacgccgcgtctcggaccgtccccacctttggctcgcggtccccctgtctcggggcggcggcacctgtgccgcgac

SEQ ID NO: 3083 - DNA, 120 bp, synthetic construct
  source 1..120: mol_type = other DNA
ccgtccccacctttggctcgcggtccccctgtctcggggcggcggcacctgtgccgcgaccgacgaggggctggcccaggcgtactacgacgacctcgaggtgcgtcgcctcggggatga

SEQ ID NO: 3084 - DNA, 120 bp, synthetic construct
  source 1..120: mol_type = other DNA
cgacgaggggctggcccaggcgtactacgacgacctcgaggtgcgtcgcctcggggatgacgccatggcccgggcggccctcgcatcagtccaacgccctcgcaaaggcccctacaacat

SEQ ID NO: 3085 - DNA, 120 bp, synthetic construct
  source 1..120: mol_type = other DNA
cgccatggcccgggcggccctcgcatcagtccaacgccctcgcaaaggcccctacaacatcagagtatggaacatggccgcgggcgctggcaagaccacccgcatcctcgctgccttcac

SEQ ID NO: 3086 - DNA, 120 bp, synthetic construct
  source 1..120: mol_type = other DNA
cagagtatggaacatggccgcgggcgctggcaagaccacccgcatcctcgctgccttcacgcgcgaagacctttacgtctgccccaccaatgcgctcctgcacgagattcaggccaaact

SEQ ID NO: 3087 - DNA, 120 bp, synthetic construct
  source 1..120: mol_type = other DNA
gcgcgaagacctttacgtctgccccaccaatgcgctcctgcacgagattcaggccaaactccgcgcgcgcgacatcgacatcaagaacgccgccacctacgaacgcgcgctgaccaaacc

SEQ ID NO: 3088 - DNA, 120 bp, synthetic construct
  source 1..120: mol_type = other DNA
ccgcgcgcgcgacatcgacatcaagaacgccgccacctacgaacgcgcgctgaccaaaccgctcgccgcctaccgccgcatctacatcgatgaggcgttcaccctcggcggtgagtactg

SEQ ID NO: 3089 - DNA, 120 bp, synthetic construct
  source 1..120: mol_type = other DNA
gctcgccgcctaccgccgcatctacatcgatgaggcgttcaccctcggcggtgagtactgcgcgttcgttgccagtcaaaccaccgcggaggtgatctgcgtcggtgaccgagaccagtg

SEQ ID NO: 3090 - DNA, 120 bp, synthetic construct
  source 1..120: mol_type = other DNA
cgcgttcgttgccagtcaaaccaccgcggaggtgatctgcgtcggtgaccgagaccagtgcggcccacattacgccaacaactgccgcacccccgtccctgaccgctggcctaccgagcg

SEQ ID NO: 3091 - DNA, 120 bp, synthetic construct
  source 1..120: mol_type = other DNA
cggcccacattacgccaacaactgccgcacccccgtccctgaccgctggcctaccgagcgctcacgacacacttggcgcttccccgactgctgggccgcccgcctgcgcgcggggctcga

SEQ ID NO: 3092 - DNA, 120 bp, synthetic construct
  source 1..120: mol_type = other DNA
ctcacgacacacttggcgcttccccgactgctgggccgcccgcctgcgcgcggggctcgattacgacatcgagggcgagcgcgccggcaccttcgcctgcaacctttgggacggccgcca

SEQ ID NO: 3093 - DNA, 120 bp, synthetic construct
  source 1..120: mol_type = other DNA
ttacgacatcgagggcgagcgcgccggcaccttcgcctgcaacctttgggacggccgccaggtcgaccttcacctcgccttctcgcgcgaaaccgtgcgccgccttcacgaagctggcat

SEQ ID NO: 3094 - DNA, 120 bp, synthetic construct
  source 1..120: mol_type = other DNA
ggtcgaccttcacctcgccttctcgcgcgaaaccgtgcgccgccttcacgaagctggcatacgcgcgtacaccgtgcgcgaggcccagggtatgagcgttagcaccgcctgcatccacgt

SEQ ID NO: 3095 - DNA, 120 bp, synthetic construct
  source 1..120: mol_type = other DNA
acgcgcgtacaccgtgcgcgaggcccagggtatgagcgttagcaccgcctgcatccacgtaggcagagacggcacagacgttgccctggcgctgacacgcgacctcgccatcgtcagcct

SEQ ID NO: 3096 - DNA, 120 bp, synthetic construct
  source 1..120: mol_type = other DNA
aggcagagacggcacagacgttgccctggcgctgacacgcgacctcgccatcgtcagcctgacccgggcctccgacgcactctacctccacgagctcgaggacggctcactgcgcgctgc

SEQ ID NO: 3097 - DNA, 120 bp, synthetic construct
  source 1..120: mol_type = other DNA
gacccgggcctccgacgcactctacctccacgagctcgaggacggctcactgcgcgctgcggggctcagcgcgttccttgacgccggggcactggcggagctcaaggaggttcccgccgg

SEQ ID NO: 3098 - DNA, 120 bp, synthetic construct
  source 1..120: mol_type = other DNA
ggggctcagcgcgttccttgacgccggggcactggcggagctcaaggaggttcccgccggcatcgaccgcgttgtcgccgtcgaacaggcaccaccaccgttgccgcccgccgacggcat

SEQ ID NO: 3099 - DNA, 120 bp, synthetic construct
  source 1..120: mol_type = other DNA
catcgaccgcgttgtcgccgtcgaacaggcaccaccaccgttgccgcccgccgacggcatccccgaggcccaagacgtgccgcccttctgcccccgcactctggaggagctcgtcttcgg

SEQ ID NO: 3100 - DNA, 120 bp, synthetic construct
  source 1..120: mol_type = other DNA
ccccgaggcccaagacgtgccgcccttctgcccccgcactctggaggagctcgtcttcggccgtgctggccacccccactacgcggacctcaaccgcgtcactgagggcgagcgggaagt

SEQ ID NO: 3101 - DNA, 120 bp, synthetic construct
  source 1..120: mol_type = other DNA
ccgtgctggccacccccactacgcggacctcaaccgcgtcactgagggcgagcgggaagtgcggtatatgcgcatctcgcgtcacctgctcaacaagaatcacaccgagatgcccgggac

SEQ ID NO: 3102 - DNA, 120 bp, synthetic construct
  source 1..120: mol_type = other DNA
gcggtatatgcgcatctcgcgtcacctgctcaacaagaatcacaccgagatgcccgggacggaacgcgtcctcagtgccgtttgcgccgtgcggcgctaccgcgcgggcgaggatgggtc

SEQ ID NO: 3103 - DNA, 120 bp, synthetic construct
  source 1..120: mol_type = other DNA
ggaacgcgtcctcagtgccgtttgcgccgtgcggcgctaccgcgcgggcgaggatgggtcgacccttcgcactgctgtggcccgccagcacccgcgccctttccgccagatcccaccccc

SEQ ID NO: 3104 - DNA, 120 bp, synthetic construct
  source 1..120: mol_type = other DNA
gacccttcgcactgctgtggcccgccagcacccgcgccctttccgccagatcccacccccgcgcgtcaccgccggggtcgctcaggagtggcgcatgacgtacttgcgggaacggatcga

SEQ ID NO: 3105 - DNA, 120 bp, synthetic construct
  source 1..120: mol_type = other DNA
gcgcgtcaccgccggggtcgctcaggagtggcgcatgacgtacttgcgggaacggatcgacctcactgatgtctacacgcagatgggcgtggccgcgcgggagctgaccgaccgctacgc

SEQ ID NO: 3106 - DNA, 120 bp, synthetic construct
  source 1..120: mol_type = other DNA
cctcactgatgtctacacgcagatgggcgtggccgcgcgggagctgaccgaccgctacgcgcgccgctaccccgagattttcgccggcatgtgtaccgcccagagcctgagcgtccccgc

SEQ ID NO: 3107 - DNA, 120 bp, synthetic construct
  source 1..120: mol_type = other DNA
gcgccgctaccccgagattttcgccggcatgtgtaccgcccagagcctgagcgtccccgccttcctcaaggccaccctgaagtgcgtagacgccgccctcggccccagggacaccgagga

SEQ ID NO: 3108 - DNA, 120 bp, synthetic construct
  source 1..120: mol_type = other DNA
cttcctcaaggccaccctgaagtgcgtagacgccgccctcggccccagggacaccgaggactgccacgccgctcaggggaaagccggccttgagattcgggcgtgggccaaggagtgggt

SEQ ID NO: 3109 - DNA, 120 bp, synthetic construct
  source 1..120: mol_type = other DNA
ctgccacgccgctcaggggaaagccggccttgagattcgggcgtgggccaaggagtgggttcaggtcatgtccccgcatttccgtgcgatccagaagatcatcatgcgcgccctgcgccc

SEQ ID NO: 3110 - DNA, 120 bp, synthetic construct
  source 1..120: mol_type = other DNA
tcaggtcatgtccccgcatttccgtgcgatccagaagatcatcatgcgcgccctgcgcccgcaattccttgtggccgctggccatacggagcccgaggtcgatgcgtggtggcaggctca

SEQ ID NO: 3111 - DNA, 120 bp, synthetic construct
  source 1..120: mol_type = other DNA
gcaattccttgtggccgctggccatacggagcccgaggtcgatgcgtggtggcaggctcactacaccaccaatgccatcgaagtcgacttcaccgagttcgacatgaaccagaccctcgc

SEQ ID NO: 3112 - DNA, 120 bp, synthetic construct
  source 1..120: mol_type = other DNA
ctacaccaccaatgccatcgaagtcgacttcaccgagttcgacatgaaccagaccctcgccactcgggacgtcgagctcgagattagcgccgctctcttgggcctcccctgcgccgaaga

SEQ ID NO: 3113 - DNA, 120 bp, synthetic construct
  source 1..120: mol_type = other DNA
cactcgggacgtcgagctcgagattagcgccgctctcttgggcctcccctgcgccgaagactaccgcgcgctccgcgccggcagctactgcaccttgcgcgaactgggcaccactgagac

SEQ ID NO: 3114 - DNA, 120 bp, synthetic construct
  source 1..120: mol_type = other DNA
ctaccgcgcgctccgcgccggcagctactgcaccttgcgcgaactgggcaccactgagaccggctgcgagcgcacaagcggcgagcccgccacgctgctgcacaacaccaccgtggccat

SEQ ID NO: 3115 - DNA, 120 bp, synthetic construct
  source 1..120: mol_type = other DNA
cggctgcgagcgcacaagcggcgagcccgccacgctgctgcacaacaccaccgtggccatgtgcatggctatgcgcatggtccccaaaggcgtgcgctgggctgggatcttccagggcga

SEQ ID NO: 3116 - DNA, 120 bp, synthetic construct
  source 1..120: mol_type = other DNA
gtgcatggctatgcgcatggtccccaaaggcgtgcgctgggctgggatcttccagggcgacgatatggtcatcttcctccctgagggcgcgcgcagcgcggcactcaagtggacccccgc

SEQ ID NO: 3117 - DNA, 120 bp, synthetic construct
  source 1..120: mol_type = other DNA
cgatatggtcatcttcctccctgagggcgcgcgcagcgcggcactcaagtggacccccgccgaggtgggcttgttcggcttccacatcccggtgaagcatgtgagcacccctacccccag

SEQ ID NO: 3118 - DNA, 120 bp, synthetic construct
  source 1..120: mol_type = other DNA
cgaggtgggcttgttcggcttccacatcccggtgaagcatgtgagcacccctacccccagtttctgcgggcacgtcggcactgcggccggcctcttccatgatgtcatgcaccaggcgat

SEQ ID NO: 3119 - DNA, 120 bp, synthetic construct
  source 1..120: mol_type = other DNA
tttctgcgggcacgtcggcactgcggccggcctcttccatgatgtcatgcaccaggcgattaaggtgctttgccgccgtttcgacccggacgtgcttgaagaacagcaggtggccctcct

SEQ ID NO: 3120 - DNA, 120 bp, synthetic construct
  source 1..120: mol_type = other DNA
taaggtgctttgccgccgtttcgacccggacgtgcttgaagaacagcaggtggccctcctcgaccgcctccggggggtctacgcggccttgcctgacaccgttgccgccaatgctgcgta

SEQ ID NO: 3121 - DNA, 120 bp, synthetic construct
  source 1..120: mol_type = other DNA
cgaccgcctccggggggtctacgcggccttgcctgacaccgttgccgccaatgctgcgtactacgactacagtgcggagcgcgtcctcgccatcgtgcgcgaactcaccgcgtacgcgcg

SEQ ID NO: 3122 - DNA, 120 bp, synthetic construct
  source 1..120: mol_type = other DNA
ctacgactacagtgcggagcgcgtcctcgccatcgtgcgcgaactcaccgcgtacgcgcgggggcgcggcctcgaccacccggccaccatcggcgcgctcgaggagatccagacccccta

SEQ ID NO: 3123 - DNA, 120 bp, synthetic construct
  source 1..120: mol_type = other DNA
ggggcgcggcctcgaccacccggccaccatcggcgcgctcgaggagatccagaccccctacgcgcgcgccaacctccacgacgctgactaacgcccctgtacgtggggcctttaatctta

SEQ ID NO: 3124 - DNA, 120 bp, synthetic construct
  source 1..120: mol_type = other DNA
cgcgcgcgccaacctccacgacgctgactaacgcccctgtacgtggggcctttaatcttacctactccaaccaggtcatcacccaccgttgtttcgccgcatctggtgggtaccgcactc

SEQ ID NO: 3125 - DNA, 120 bp, synthetic construct
  source 1..120: mol_type = other DNA
cctactccaaccaggtcatcacccaccgttgtttcgccgcatctggtgggtaccgcactcttgccattcgggagagccccagggtgcccgaatggcttccactacccccatcaccatgga

SEQ ID NO: 3126 - DNA, 120 bp, synthetic construct
  source 1..120: mol_type = other DNA
ttgccattcgggagagccccagggtgcccgaatggcttccactacccccatcaccatggaggacctccagaaggccctcgaggcacaatcacgcgccctgcgcgcggaactcgctgccgg

SEQ ID NO: 3127 - DNA, 120 bp, synthetic construct
  source 1..120: mol_type = other DNA
ggacctccagaaggccctcgaggcacaatcacgcgccctgcgcgcggaactcgctgccggcgcctcgcagacgcgccggccgcggccgccgcgacagcgcgactccagcacctccggaga

SEQ ID NO: 3128 - DNA, 120 bp, synthetic construct
  source 1..120: mol_type = other DNA
cgcctcgcagacgcgccggccgcggccgccgcgacagcgcgactccagcacctccggagatgactccggccgtgactccggagggccccgccgccgccgcggcaaccggggccgtggcca

SEQ ID NO: 3129 - DNA, 120 bp, synthetic construct
  source 1..120: mol_type = other DNA
tgactccggccgtgactccggagggccccgccgccgccgcggcaaccggggccgtggccagcgcggggactggtccagggccccgccccccccggaagagcggcaagaaagtcgctccca

SEQ ID NO: 3130 - DNA, 120 bp, synthetic construct
  source 1..120: mol_type = other DNA
gcgcggggactggtccagggccccgccccccccggaagagcggcaagaaagtcgctcccagactccggctccgaagccaccgcgggcgccgccacagcagcctcaacccccgcgtatgca

SEQ ID NO: 3131 - DNA, 120 bp, synthetic construct
  source 1..120: mol_type = other DNA
gactccggctccgaagccaccgcgggcgccgccacagcagcctcaacccccgcgtatgcaaaccgggcgtgggggctctgccccgcgccccgagctggggccgccgaccaacccgttcca

SEQ ID NO: 3132 - DNA, 120 bp, synthetic construct
  source 1..120: mol_type = other DNA
aaccgggcgtgggggctctgccccgcgccccgagctggggccgccgaccaacccgttccaagcagccgtggcgcgtggcctgcgcccgccgctccacgaccctgacaccgaggcacccac

SEQ ID NO: 3133 - DNA, 120 bp, synthetic construct
  source 1..120: mol_type = other DNA
agcagccgtggcgcgtggcctgcgcccgccgctccacgaccctgacaccgaggcacccaccgaggcctgcgtaacctcatggctttggagcgaaggcgaaggcgcggtcttctaccgcgt

SEQ ID NO: 3134 - DNA, 120 bp, synthetic construct
  source 1..120: mol_type = other DNA
cgaggcctgcgtaacctcatggctttggagcgaaggcgaaggcgcggtcttctaccgcgtcgacctacacttcaccaacctgggcaccccccccctcgacgaggacggccgctgggaccc

SEQ ID NO: 3135 - DNA, 120 bp, synthetic construct
  source 1..120: mol_type = other DNA
cgacctacacttcaccaacctgggcaccccccccctcgacgaggacggccgctgggaccccgcgctcatgtacaacccctgcgggcccgagccgcccgctcacgtcgtacgcgcgtacaa

SEQ ID NO: 3136 - DNA, 120 bp, synthetic construct
  source 1..120: mol_type = other DNA
cgcgctcatgtacaacccctgcgggcccgagccgcccgctcacgtcgtacgcgcgtacaatcaacccgccggcgacgtcaggggcgtttggggtaaaggcgagcgcacttacgccgagca

SEQ ID NO: 3137 - DNA, 120 bp, synthetic construct
  source 1..120: mol_type = other DNA
tcaacccgccggcgacgtcaggggcgtttggggtaaaggcgagcgcacttacgccgagcaggatttccgcgtcggtggcacgcgctggcaccgactgctgcgcatgccagtgcgcggcct

SEQ ID NO: 3138 - DNA, 120 bp, synthetic construct
  source 1..120: mol_type = other DNA
ggatttccgcgtcggtggcacgcgctggcaccgactgctgcgcatgccagtgcgcggcctcgacggcgacagcgccccgcttcccccccacaccaccgagcgcattgagacccgctcggc

SEQ ID NO: 3139 - DNA, 120 bp, synthetic construct
  source 1..120: mol_type = other DNA
cgacggcgacagcgccccgcttcccccccacaccaccgagcgcattgagacccgctcggcgcgccatccttggcgcatccgctttggcgctccccaggccttccttgccgggctcttgct

SEQ ID NO: 3140 - DNA, 120 bp, synthetic construct
  source 1..120: mol_type = other DNA
gcgccatccttggcgcatccgctttggcgctccccaggccttccttgccgggctcttgctcgccgcggtcgccgtcggcaccgcgcgcgccgggctccagccccgcgctgacatggcggc

SEQ ID NO: 3141 - DNA, 120 bp, synthetic construct
  source 1..120: mol_type = other DNA
cgccgcggtcgccgtcggcaccgcgcgcgccgggctccagccccgcgctgacatggcggccccgcctgcgccgccgcagcccccccgtgcgcacgggcagcactacggccatcaccacca

SEQ ID NO: 3142 - DNA, 120 bp, synthetic construct
  source 1..120: mol_type = other DNA
cccgcctgcgccgccgcagcccccccgtgcgcacgggcagcactacggccatcaccaccatcagctgccgttcctcgggcacgacggccatcacggcggcaccctgcgcgtcggccagca

SEQ ID NO: 3143 - DNA, 120 bp, synthetic construct
  source 1..120: mol_type = other DNA
tcagctgccgttcctcgggcacgacggccatcacggcggcaccctgcgcgtcggccagcatcaccgaaacgccagcgacgtgctgcccggccactggctccaaggcggctggggctgcta

SEQ ID NO: 3144 - DNA, 120 bp, synthetic construct
  source 1..120: mol_type = other DNA
tcaccgaaacgccagcgacgtgctgcccggccactggctccaaggcggctggggctgctacaacctgagcgactggcaccagggcactcatgtctgtcacaccaagcacatggacttctg

SEQ ID NO: 3145 - DNA, 120 bp, synthetic construct
  source 1..120: mol_type = other DNA
caacctgagcgactggcaccagggcactcatgtctgtcacaccaagcacatggacttctggtgtgtggagcacgaccgaccgccgcctgcgaccccgacgcctctcaccaccgcggcgaa

SEQ ID NO: 3146 - DNA, 120 bp, synthetic construct
  source 1..120: mol_type = other DNA
gtgtgtggagcacgaccgaccgccgcctgcgaccccgacgcctctcaccaccgcggcgaacgccacgaccgccgccacccccaccactgtgccggccccttgccacgccggcctcaatga

SEQ ID NO: 3147 - DNA, 120 bp, synthetic construct
  source 1..120: mol_type = other DNA
cgccacgaccgccgccacccccaccactgtgccggccccttgccacgccggcctcaatgacagctgcggcggcttcttgtcagggtgcgggccgatgcgcctgcgccacggcgccgacac

SEQ ID NO: 3148 - DNA, 120 bp, synthetic construct
  source 1..120: mol_type = other DNA
cagctgcggcggcttcttgtcagggtgcgggccgatgcgcctgcgccacggcgccgacacccggtgcggtcggctgatctgcgggctgtccaccaccgcccagtacccgcctacccggtt

SEQ ID NO: 3149 - DNA, 120 bp, synthetic construct
  source 1..120: mol_type = other DNA
ccggtgcggtcggctgatctgcgggctgtccaccaccgcccagtacccgcctacccggttcggctgcgttatgcggtggggccttcccccttgggaactggtcgtccttaccgcccgccc

SEQ ID NO: 3150 - DNA, 120 bp, synthetic construct
  source 1..120: mol_type = other DNA
cggctgcgttatgcggtggggccttcccccttgggaactggtcgtccttaccgcccgccccgaagacggctggacttgccgcggcgtgcccgcccatccaggtacccgctgccccaaact

SEQ ID NO: 3151 - DNA, 120 bp, synthetic construct
  source 1..120: mol_type = other DNA
cgaagacggctggacttgccgcggcgtgcccgcccatccaggtacccgctgccccaaactggtgagccccatgggacgcgcgacctgctccccagcctcggccctctggctcgccacagc

SEQ ID NO: 3152 - DNA, 120 bp, synthetic construct
  source 1..120: mol_type = other DNA
ggtgagccccatgggacgcgcgacctgctccccagcctcggccctctggctcgccacagccaatgcgctgtctcttgatcacgcccttgcggccgccgtcctgctggtcccgtgggtcct

SEQ ID NO: 3153 - DNA, 120 bp, synthetic construct
  source 1..120: mol_type = other DNA
caatgcgctgtctcttgatcacgcccttgcggccgccgtcctgctggtcccgtgggtcctgatatttatggtgtgccgccgcgcctgccgccgccgcggcgccgccgccgcccttaccgc

SEQ ID NO: 3154 - DNA, 120 bp, synthetic construct
  source 1..120: mol_type = other DNA
gatatttatggtgtgccgccgcgcctgccgccgccgcggcgccgccgccgcccttaccgcggtcgtcctgcagggttacaacccccccgcctacggcgaggaggctttcacctacctctg

SEQ ID NO: 3155 - DNA, 120 bp, synthetic construct
  source 1..120: mol_type = other DNA
ggtcgtcctgcagggttacaacccccccgcctacggcgaggaggctttcacctacctctgtactgcaccggggtgcgccacgcaaacacctgtccctgtgcgcctcgctggcgtccgctt

SEQ ID NO: 3156 - DNA, 120 bp, synthetic construct
  source 1..120: mol_type = other DNA
tactgcaccggggtgcgccacgcaaacacctgtccctgtgcgcctcgctggcgtccgctttgagtccaagattgtggacggcggctgctttgccccatgggacctcgaggccactggagc

SEQ ID NO: 3157 - DNA, 120 bp, synthetic construct
  source 1..120: mol_type = other DNA
tgagtccaagattgtggacggcggctgctttgccccatgggacctcgaggccactggagcctgcatttgcgagatccccactgacgtctcgtgcgagggcttgggggcctgggtacccac

SEQ ID NO: 3158 - DNA, 120 bp, synthetic construct
  source 1..120: mol_type = other DNA
ctgcatttgcgagatccccactgacgtctcgtgcgagggcttgggggcctgggtacccacagccccttgcgcgcgcatttggaacggcacacagcgcgcgtgcaccttttgggccgtcaa

SEQ ID NO: 3159 - DNA, 120 bp, synthetic construct
  source 1..120: mol_type = other DNA
agccccttgcgcgcgcatttggaacggcacacagcgcgcgtgcaccttttgggccgtcaacgcctactcttctggtgggtacgcgcagctggcctcttacttcaaccctggcggtagcta

SEQ ID NO: 3160 - DNA, 120 bp, synthetic construct
  source 1..120: mol_type = other DNA
cgcctactcttctggtgggtacgcgcagctggcctcttacttcaaccctggcggtagctactacaagcagtaccatcctaccgcgtgcgaggttgagcccgccttcggacacagcgacgc

SEQ ID NO: 3161 - DNA, 120 bp, synthetic construct
  source 1..120: mol_type = other DNA
ctacaagcagtaccatcctaccgcgtgcgaggttgagcccgccttcggacacagcgacgcggcctgctggggcttccccaccgacactgtgatgagcgtgttcgcccttgccagctacgt

SEQ ID NO: 3162 - DNA, 120 bp, synthetic construct
  source 1..120: mol_type = other DNA
ggcctgctggggcttccccaccgacactgtgatgagcgtgttcgcccttgccagctacgtccagcaccctcacaagaccgtccgggtcaagttccatacagagaccaggaccgtctggca

SEQ ID NO: 3163 - DNA, 120 bp, synthetic construct
  source 1..120: mol_type = other DNA
ccagcaccctcacaagaccgtccgggtcaagttccatacagagaccaggaccgtctggcaactctccgttgccggcgtgtcgtgcaatgtcaccactgaacacccattctgcaacacgcc

SEQ ID NO: 3164 - DNA, 120 bp, synthetic construct
  source 1..120: mol_type = other DNA
actctccgttgccggcgtgtcgtgcaatgtcaccactgaacacccattctgcaacacgccgcacggacaactcgaggtccaggtcccgcccgaccccggggacctggttgagtacattat

SEQ ID NO: 3165 - DNA, 120 bp, synthetic construct
  source 1..120: mol_type = other DNA
gcacggacaactcgaggtccaggtcccgcccgaccccggggacctggttgagtacattatgaattacaccggcaatcagcagtcccggtggggccttgggagcccgaattgccacggccc

SEQ ID NO: 3166 - DNA, 120 bp, synthetic construct
  source 1..120: mol_type = other DNA
gaattacaccggcaatcagcagtcccggtggggccttgggagcccgaattgccacggccccgactgggcctccccggtttgtcagcgccattcccctgactgctcgcggcttgtgggggc

SEQ ID NO: 3167 - DNA, 120 bp, synthetic construct
  source 1..120: mol_type = other DNA
cgactgggcctccccggtttgtcagcgccattcccctgactgctcgcggcttgtgggggccacgccagagcgtccccggcttcgcctggtcgacgccgacgaccccctgctgcgcactgc

SEQ ID NO: 3168 - DNA, 120 bp, synthetic construct
  source 1..120: mol_type = other DNA
cacgccagagcgtccccggcttcgcctggtcgacgccgacgaccccctgctgcgcactgcccctgggcccggcgaggtgtgggtcacgcctgtcataggctctcaggcgcgcaagtgcgg

SEQ ID NO: 3169 - DNA, 120 bp, synthetic construct
  source 1..120: mol_type = other DNA
ccctgggcccggcgaggtgtgggtcacgcctgtcataggctctcaggcgcgcaagtgcggactccacatacgcgctggaccgtacggccatgctaccgtcgaaatgcccgagtggatcca

SEQ ID NO: 3170 - DNA, 120 bp, synthetic construct
  source 1..120: mol_type = other DNA
actccacatacgcgctggaccgtacggccatgctaccgtcgaaatgcccgagtggatccacgcccacaccaccagcgacccctggcacccaccgggccccttggggctgaaattcaagac

SEQ ID NO: 3171 - DNA, 120 bp, synthetic construct
  source 1..120: mol_type = other DNA
cgcccacaccaccagcgacccctggcacccaccgggccccttggggctgaaattcaagaccgttcgcccggttgccctgccacgcgcgttagcgccaccccgcaatgtgcgtgtgaccgg

SEQ ID NO: 3172 - DNA, 120 bp, synthetic construct
  source 1..120: mol_type = other DNA
cgttcgcccggttgccctgccacgcgcgttagcgccaccccgcaatgtgcgtgtgaccgggtgttaccagtgcggtactcccgcgctggtggaaggccttgcccccggggggggcaattg

SEQ ID NO: 3173 - DNA, 120 bp, synthetic construct
  source 1..120: mol_type = other DNA
gtgttaccagtgcggtactcccgcgctggtggaaggccttgcccccggggggggcaattgccatctcactgtcaatggcgaggacgtcggcgccttcccccctgggaagttcgtcaccgc

SEQ ID NO: 3174 - DNA, 120 bp, synthetic construct
  source 1..120: mol_type = other DNA
ccatctcactgtcaatggcgaggacgtcggcgccttcccccctgggaagttcgtcaccgccgccctcctcaacacccccccgccctaccaagtcagctgcgggggcgagagcgatcgcgc

SEQ ID NO: 3175 - DNA, 120 bp, synthetic construct
  source 1..120: mol_type = other DNA
cgccctcctcaacacccccccgccctaccaagtcagctgcgggggcgagagcgatcgcgcgagcgcgcgggttattgaccccgccgcgcaatcgtttaccggcgtggtgtatggcacaca

SEQ ID NO: 3176 - DNA, 120 bp, synthetic construct
  source 1..120: mol_type = other DNA
gagcgcgcgggttattgaccccgccgcgcaatcgtttaccggcgtggtgtatggcacacacaccaccgctgtgtcggagacccggcagacctgggcggagtgggctgctgcccattggtg

SEQ ID NO: 3177 - DNA, 120 bp, synthetic construct
  source 1..120: mol_type = other DNA
caccaccgctgtgtcggagacccggcagacctgggcggagtgggctgctgcccattggtggcagctcactctgggcgccatctgcaccctcctatttgctggcttacttgcttgctgtgc

SEQ ID NO: 3178 - DNA, 120 bp, synthetic construct
  source 1..120: mol_type = other DNA
gcagctcactctgggcgccatctgcaccctcctatttgctggcttacttgcttgctgtgccaaatgcttgtactacttgcgcggcgctatagcgccgcgctagtgggcccccgcgcgaaa

SEQ ID NO: 3179 - DNA, 120 bp, synthetic construct
  source 1..120: mol_type = other DNA
cttacttgcttgctgtgccaaatgcttgtactacttgcgcggcgctatagcgccgcgctagtgggcccccgcgcgaaacccgcatcagcccactagattcccgcacctgttgctgcatag

SEQ ID NO: 3180 - DNA, 120 bp, synthetic construct
  source 1..120: mol_type = other DNA
tgtataaaaaactaataacgtttttatttgtaataggtgcagtagcatcctattcgaataatgagtacactccgtttaataaactgagtgtaaaactctatatagatggagtagataata

SEQ ID NO: 3181 - DNA, 120 bp, synthetic construct
  source 1..120: mol_type = other DNA
atgagtacactccgtttaataaactgagtgtaaaactctatatagatggagtagataatatagaaaattcatatactgatgataataatgaattggtgttaaattttaaagagtacacaa

SEQ ID NO: 3182 - DNA, 120 bp, synthetic construct
  source 1..120: mol_type = other DNA
tagaaaattcatatactgatgataataatgaattggtgttaaattttaaagagtacacaatttctattattacagagtcatgcgacgtcggatttgattccatagatatagatgttataa

SEQ ID NO: 3183 - DNA, 120 bp, synthetic construct
  source 1..120: mol_type = other DNA
tttctattattacagagtcatgcgacgtcggatttgattccatagatatagatgttataaacgactataaaattattgatatgtataccattgactcgtctactattcaacgcagaggtc

SEQ ID NO: 3184 - DNA, 120 bp, synthetic construct
  source 1..120: mol_type = other DNA
acgactataaaattattgatatgtataccattgactcgtctactattcaacgcagaggtcacacgtgtagaatatctaccaaattatcatgccattatgataagtacccttatattcaca

SEQ ID NO: 3185 - DNA, 120 bp, synthetic construct
  source 1..120: mol_type = other DNA
acacgtgtagaatatctaccaaattatcatgccattatgataagtacccttatattcacaaatatgatggtgatgagcgacaatattctattactgcagagggaaaatgctataaaggaa

SEQ ID NO: 3186 - DNA, 120 bp, synthetic construct
  source 1..120: mol_type = other DNA
aatatgatggtgatgagcgacaatattctattactgcagagggaaaatgctataaaggaataaaatatgaaataagtatgatcaacgatgatactctattgagaaaacatactcttaaaa

SEQ ID NO: 3187 - DNA, 120 bp, synthetic construct
  source 1..120: mol_type = other DNA
taaaatatgaaataagtatgatcaacgatgatactctattgagaaaacatactcttaaaattggatctacttatatatttgatcgtcatggacatagtaatacatattattcaaaatatg

SEQ ID NO: 3188 - DNA, 120 bp, synthetic construct
  source 1..120: mol_type = other DNA
ttggatctacttatatatttgatcgtcatggacatagtaatacatattattcaaaatatgatttttaaaaatttaaaatatattatcacttcagtgacagtagtcaaataacaaacaaca

SEQ ID NO: 3189 - DNA, 120 bp, synthetic construct
  source 1..120: mol_type = other DNA
atttttaaaaatttaaaatatattatcacttcagtgacagtagtcaaataacaaacaacaccatgagatatattataattctcgcagttttgttcattaatagtatacatgctaaaataa

SEQ ID NO: 3190 - DNA, 120 bp, synthetic construct
  source 1..120: mol_type = other DNA
ccatgagatatattataattctcgcagttttgttcattaatagtatacatgctaaaataactagttataagtttgaatccgtcaattttgattccaaaattgaatggactggggatggtc

SEQ ID NO: 3191 - DNA, 120 bp, synthetic construct
  source 1..120: mol_type = other DNA
ctagttataagtttgaatccgtcaattttgattccaaaattgaatggactggggatggtctatacaatatatcccttaaaaattatggcatcaagacgtggcaaacaatgtatacaaatg

SEQ ID NO: 3192 - DNA, 120 bp, synthetic construct
  source 1..120: mol_type = other DNA
tatacaatatatcccttaaaaattatggcatcaagacgtggcaaacaatgtatacaaatgtaccagaaggaacatacgacatatccgcatttccaaagaatgatttcgtatctttctggg

SEQ ID NO: 3193 - DNA, 120 bp, synthetic construct
  source 1..120: mol_type = other DNA
taccagaaggaacatacgacatatccgcatttccaaagaatgatttcgtatctttctgggttaaatttgaacaaggcgattataaagtggaagagtattgtacgggactatgcgtcgaag

SEQ ID NO: 3194 - DNA, 120 bp, synthetic construct
  source 1..120: mol_type = other DNA
ttaaatttgaacaaggcgattataaagtggaagagtattgtacgggactatgcgtcgaagtaaaaattggaccaccgactgtaacattaactgaatacgacgaccatatcaatttgtaca

SEQ ID NO: 3195 - DNA, 120 bp, synthetic construct
  source 1..120: mol_type = other DNA
taaaaattggaccaccgactgtaacattaactgaatacgacgaccatatcaatttgtacatcgagcatccgtatgctactagaggtagcaaaaagattcctatttacaaacgcggtgaca

SEQ ID NO: 3196 - DNA, 120 bp, synthetic construct
  source 1..120: mol_type = other DNA
tcgagcatccgtatgctactagaggtagcaaaaagattcctatttacaaacgcggtgacatgtgtgatatctacttgttgtatacggctaacttcacattcggagattctaaagaaccag

SEQ ID NO: 3197 - DNA, 120 bp, synthetic construct
  source 1..120: mol_type = other DNA
tgtgtgatatctacttgttgtatacggctaacttcacattcggagattctaaagaaccagtaccatatgatatcgatgactacgattgcacgtctacaggttgcagcatagactttgtca

SEQ ID NO: 3198 - DNA, 120 bp, synthetic construct
  source 1..120: mol_type = other DNA
taccatatgatatcgatgactacgattgcacgtctacaggttgcagcatagactttgtcacaacagaaaaagtgtgcgtgacagcacagggagccacagaagggtttctcgaaaaaatta

SEQ ID NO: 3199 - DNA, 120 bp, synthetic construct
  source 1..120: mol_type = other DNA
caacagaaaaagtgtgcgtgacagcacagggagccacagaagggtttctcgaaaaaattactccatggagttcggaagtatgtctgacacctaaaaagagtgtatatacatgcgcaatta

SEQ ID NO: 3200 - DNA, 120 bp, synthetic construct
  source 1..120: mol_type = other DNA
ctccatggagttcggaagtatgtctgacacctaaaaagagtgtatatacatgcgcaattagatccaaagaagatgttcccaatttcaaggacaaaatggccagagttatcaagagaaaat

SEQ ID NO: 3201 - DNA, 120 bp, synthetic construct
  source 1..120: mol_type = other DNA
gatccaaagaagatgttcccaatttcaaggacaaaatggccagagttatcaagagaaaatttaataaacagtctcaatcttatttaactaaatttctcggtagcacatcaaatgatgtta

SEQ ID NO: 3202 - DNA, 120 bp, synthetic construct
  source 1..120: mol_type = other DNA
ttaataaacagtctcaatcttatttaactaaatttctcggtagcacatcaaatgatgttaccacttttcttagcatgcttaacttgactaaatattcataactaatttttattaatgata

SEQ ID NO: 3203 - DNA, 120 bp, synthetic construct
  source 1..120: mol_type = other DNA
ccacttttcttagcatgcttaacttgactaaatattcataactaatttttattaatgatacaaaaacgaaataaaactgcatattatacactggttaacgcccttataggctctaaccat

SEQ ID NO: 3204 - DNA, 120 bp, synthetic construct
  source 1..120: mol_type = other DNA
caaaaacgaaataaaactgcatattatacactggttaacgcccttataggctctaaccattttcaagatgaggtccctgattatagtccttctgttcccctctatcatctactccatgtc

SEQ ID NO: 3205 - DNA, 120 bp, synthetic construct
  source 1..120: mol_type = other DNA
tttcaagatgaggtccctgattatagtccttctgttcccctctatcatctactccatgtctattagacgatgtgagaagactgaagaggaaacatggggattgaaaatagggttgtgtat

SEQ ID NO: 3206 - DNA, 120 bp, synthetic construct
  source 1..120: mol_type = other DNA
tattagacgatgtgagaagactgaagaggaaacatggggattgaaaatagggttgtgtataattgccaaagatttttatcccgaaagaactgattgcagtgttcatctcccaactgcaag

SEQ ID NO: 3207 - DNA, 120 bp, synthetic construct
  source 1..120: mol_type = other DNA
aattgccaaagatttttatcccgaaagaactgattgcagtgttcatctcccaactgcaagtgaaggattgataactgaaggcaatggattcagggatatacgaaacaccgataaattata

SEQ ID NO: 3208 - DNA, 120 bp, synthetic construct
  source 1..120: mol_type = other DNA
tgaaggattgataactgaaggcaatggattcagggatatacgaaacaccgataaattataaaaaaagcaatgtgtccgctgtttccgttaataatactattttcgtaactggcggattat

SEQ ID NO: 3209 - DNA, 120 bp, synthetic construct
  source 1..120: mol_type = other DNA
aaaaaagcaatgtgtccgctgtttccgttaataatactattttcgtaactggcggattattcataaataactctaatagcacgatcgtggttaacaatatggaaaaacttgacatttata

SEQ ID NO: 3210 - DNA, 120 bp, synthetic construct
  source 1..120: mol_type = other DNA
tcataaataactctaatagcacgatcgtggttaacaatatggaaaaacttgacatttataaagacaaacaatggtcgattatagaaatgcctatggctagggtatatcacggcatcgact

SEQ ID NO: 3211 - DNA, 120 bp, synthetic construct
  source 1..120: mol_type = other DNA
aagacaaacaatggtcgattatagaaatgcctatggctagggtatatcacggcatcgactcgacatttggaatgttatattttgccggaggtctatccgttaccgaacaatatggtaatt

SEQ ID NO: 3212 - DNA, 120 bp, synthetic construct
  source 1..120: mol_type = other DNA
cgacatttggaatgttatattttgccggaggtctatccgttaccgaacaatatggtaatttagagaaaaacaacgagatatcttgttacaatcctagaacgaataagtggtttgatattt

SEQ ID NO: 3213 - DNA, 120 bp, synthetic construct
  source 1..120: mol_type = other DNA
tagagaaaaacaacgagatatcttgttacaatcctagaacgaataagtggtttgatatttcatatactatttataagatatccatatcatcattgtgtaaactaaataacgtcttctatg

SEQ ID NO: 3214 - DNA, 120 bp, synthetic construct
  source 1..120: mol_type = other DNA
catatactatttataagatatccatatcatcattgtgtaaactaaataacgtcttctatgtatttagtaaggacattggatatgtggaaaagtatgatggtgcatggaagttagtacatg

SEQ ID NO: 3215 - DNA, 120 bp, synthetic construct
  source 1..120: mol_type = other DNA
tatttagtaaggacattggatatgtggaaaagtatgatggtgcatggaagttagtacatgatcgtctccccgctataaaggcattatcaacttctccttattgattgaaaatgaaaatat

SEQ ID NO: 3216 - DNA, 120 bp, synthetic construct
  source 1..120: mol_type = other DNA
atcgtctccccgctataaaggcattatcaacttctccttattgattgaaaatgaaaatataaatagtttttatgtatagcagtattaccctatagttttattgcttactactaacatgga

SEQ ID NO: 3217 - DNA, 120 bp, synthetic construct
  source 1..120: mol_type = other DNA
aaatagtttttatgtatagcagtattaccctatagttttattgcttactactaacatggatacagatgttacaaatgtagaagatatcataaatgaaatagatagagagaaagaagaaat

SEQ ID NO: 3218 - DNA, 120 bp, synthetic construct
  source 1..120: mol_type = other DNA
tacagatgttacaaatgtagaagatatcataaatgaaatagatagagagaaagaagaaatactaaaaaatgtagaaattgaaaataataaaaacattaacaagaatcatcccaatgaata

SEQ ID NO: 3219 - DNA, 120 bp, synthetic construct
  source 1..120: mol_type = other DNA
actaaaaaatgtagaaattgaaaataataaaaacattaacaagaatcatcccaatgaatatattagagaagcactcgttattaataccagtagtaatagtgattccattgataaagaagt

SEQ ID NO: 3220 - DNA, 120 bp, synthetic construct
  source 1..120: mol_type = other DNA
tattagagaagcactcgttattaataccagtagtaatagtgattccattgataaagaagttatagaatgtatctgtcacgatgtaggaatatagatcatatctactaatttttataatcg

SEQ ID NO: 3221 - DNA, 120 bp, synthetic construct
  source 1..120: mol_type = other DNA
tatagaatgtatctgtcacgatgtaggaatatagatcatatctactaatttttataatcgatacaaaacataaaaaacaactcgttattacatagcaggcatggaatccttcaagtattg

SEQ ID NO: 3222 - DNA, 120 bp, synthetic construct
  source 1..120: mol_type = other DNA
atacaaaacataaaaaacaactcgttattacatagcaggcatggaatccttcaagtattgttttgataacgatggcaagaaatggattatcggaaatactttatattctggtaattcaat

SEQ ID NO: 3223 - DNA, 120 bp, synthetic construct
  source 1..120: mol_type = other DNA
ttttgataacgatggcaagaaatggattatcggaaatactttatattctggtaattcaatactatataaggtcagaaaaaatttcactagttcgttctacaattacgtaatgaagataga

SEQ ID NO: 3224 - DNA, 120 bp, synthetic construct
  source 1..120: mol_type = other DNA
actatataaggtcagaaaaaatttcactagttcgttctacaattacgtaatgaagatagatcacaaatcacacaagccattgttgtctgaaatacgattctatatatctgtattggatcc

SEQ ID NO: 3225 - DNA, 120 bp, synthetic construct
  source 1..120: mol_type = other DNA
tcacaaatcacacaagccattgttgtctgaaatacgattctatatatctgtattggatcctttgactatcgacaactggacacgggaacgtggtataaagtatttggctattccagatct

SEQ ID NO: 3226 - DNA, 120 bp, synthetic construct
  source 1..120: mol_type = other DNA
tttgactatcgacaactggacacgggaacgtggtataaagtatttggctattccagatctgtatggaattggagaaaccgatgattatatgttcttcgttataaaaaattcgggaagagt

SEQ ID NO: 3227 - DNA, 120 bp, synthetic construct
  source 1..120: mol_type = other DNA
gtatggaattggagaaaccgatgattatatgttcttcgttataaaaaattcgggaagagtattcgccccaaaggatactgaatcagtcttcgaagcatgtgtcactatgataaacacgtt

SEQ ID NO: 3228 - DNA, 120 bp, synthetic construct
  source 1..120: mol_type = other DNA
attcgccccaaaggatactgaatcagtcttcgaagcatgtgtcactatgataaacacgttagagtttatacactctcgaggatttacccatggaaaaatagaaccgaggaatatactgat

SEQ ID NO: 3229 - DNA, 120 bp, synthetic construct
  source 1..120: mol_type = other DNA
agagtttatacactctcgaggatttacccatggaaaaatagaaccgaggaatatactgattagaaataaacgtctttcactaattgactattctagaactaacaaactatacaagagtgg

SEQ ID NO: 3230 - DNA, 120 bp, synthetic construct
  source 1..120: mol_type = other DNA
tagaaataaacgtctttcactaattgactattctagaactaacaaactatacaagagtggaaactcacatatagattacaacgaggacatgataacttcaggaaatatcaattatatgtg

SEQ ID NO: 3231 - DNA, 120 bp, synthetic construct
  source 1..120: mol_type = other DNA
aaactcacatatagattacaacgaggacatgataacttcaggaaatatcaattatatgtgtgtagacaatcatcttggagcaacagtttcaaaacgaggagatttagaaatgttgggata

SEQ ID NO: 3232 - DNA, 120 bp, synthetic construct
  source 1..120: mol_type = other DNA
tgtagacaatcatcttggagcaacagtttcaaaacgaggagatttagaaatgttgggatattgcatgatagaatggttcggtggcaaacttccatggaaaaacgaaagtagtataaaagt

SEQ ID NO: 3233 - DNA, 120 bp, synthetic construct
  source 1..120: mol_type = other DNA
ttgcatgatagaatggttcggtggcaaacttccatggaaaaacgaaagtagtataaaagtaataaaacaaaaaaaagaatataaaaaatttatagctactttctttgaggactgttttcc

SEQ ID NO: 3234 - DNA, 120 bp, synthetic construct
  source 1..120: mol_type = other DNA
aataaaacaaaaaaaagaatataaaaaatttatagctactttctttgaggactgttttcctgaaggaaatgaacctctggaattagttagatatatagaattagtatacacgttagatta

SEQ ID NO: 3235 - DNA, 120 bp, synthetic construct
  source 1..120: mol_type = other DNA
tgaaggaaatgaacctctggaattagttagatatatagaattagtatacacgttagattattctcaaactcctaattatgacagactacgtaaactgtttatacaagattgaaattatat

SEQ ID NO: 3236 - DNA, 120 bp, synthetic construct
  source 1..120: mol_type = other DNA
ttctcaaactcctaattatgacagactacgtaaactgtttatacaagattgaaattatattctttttttatagagtgtggtagtgttacggatatctaatattaatattagactatctct

SEQ ID NO: 3237 - DNA, 120 bp, synthetic construct
  source 1..120: mol_type = other DNA
tctttttttatagagtgtggtagtgttacggatatctaatattaatattagactatctctatcgcgctacacgaccaatatcgattactatggatatcttcagggaaatcgcatcttcta

SEQ ID NO: 3238 - DNA, 120 bp, synthetic construct
  source 1..120: mol_type = other DNA
atcgcgctacacgaccaatatcgattactatggatatcttcagggaaatcgcatcttctatgaaaggagagaatgtatttatttctccagcgtcaatctcgtcagtattgacaatactgt

SEQ ID NO: 3239 - DNA, 120 bp, synthetic construct
  source 1..120: mol_type = other DNA
tgaaaggagagaatgtatttatttctccagcgtcaatctcgtcagtattgacaatactgtattatggagctaatggatccactgctgaacagctatcaaaatatgtagaaacggaggaga

SEQ ID NO: 3240 - DNA, 120 bp, synthetic construct
  source 1..120: mol_type = other DNA
attatggagctaatggatccactgctgaacagctatcaaaatatgtagaaacggaggagaacacggataaggttagcgctcagaatatctcattcaaatccatgaataaagtatatgggc

SEQ ID NO: 3241 - DNA, 120 bp, synthetic construct
  source 1..120: mol_type = other DNA
acacggataaggttagcgctcagaatatctcattcaaatccatgaataaagtatatgggcgatattctgccgtgtttaaagattcctttttgagaaaaattggcgataagtttcaaactg

SEQ ID NO: 3242 - DNA, 120 bp, synthetic construct
  source 1..120: mol_type = other DNA
gatattctgccgtgtttaaagattcctttttgagaaaaattggcgataagtttcaaactgttgacttcactgattgtcgcactatagatgcaatcaacaagtgtgtagatatctttactg

SEQ ID NO: 3243 - DNA, 120 bp, synthetic construct
  source 1..120: mol_type = other DNA
ttgacttcactgattgtcgcactatagatgcaatcaacaagtgtgtagatatctttactgaggggaaaatcaatccactattggatgaaccattgtctcctagcaattagtgccgtatac

SEQ ID NO: 3244 - DNA, 120 bp, synthetic construct
  source 1..120: mol_type = other DNA
aggggaaaatcaatccactattggatgaaccattgtctcctagcaattagtgccgtatactttaaagcaaaatggttgacgccattcgaaaaggaatttaccagtgattatcccttttac

SEQ ID NO: 3245 - DNA, 120 bp, synthetic construct
  source 1..120: mol_type = other DNA
tttaaagcaaaatggttgacgccattcgaaaaggaatttaccagtgattatcccttttacgtatctccgacggaaatggtagatgtaagtatgatgtctatgtacggcaaggcatttaat

SEQ ID NO: 3246 - DNA, 120 bp, synthetic construct
  source 1..120: mol_type = other DNA
gtatctccgacggaaatggtagatgtaagtatgatgtctatgtacggcaaggcatttaatcacgcatctgtaaaggaatcattcggcaacttttcaatcatagaactgccatatgttgga

SEQ ID NO: 3247 - DNA, 120 bp, synthetic construct
  source 1..120: mol_type = other DNA
cacgcatctgtaaaggaatcattcggcaacttttcaatcatagaactgccatatgttggagatactagtatgatggtcattcttccagacaagattgatggattagaatccatagaacaa

SEQ ID NO: 3248 - DNA, 120 bp, synthetic construct
  source 1..120: mol_type = other DNA
gatactagtatgatggtcattcttccagacaagattgatggattagaatccatagaacaaaatctaacagatacaaattttaagaaatggtgtgactttatggatgctatgtttatagat

SEQ ID NO: 3249 - DNA, 120 bp, synthetic construct
  source 1..120: mol_type = other DNA
aatctaacagatacaaattttaagaaatggtgtgactttatggatgctatgtttatagatgttcacattcccaagtttaaggtaacaggctcgtataatctggtggatactctagtaaag

SEQ ID NO: 3250 - DNA, 120 bp, synthetic construct
  source 1..120: mol_type = other DNA
gttcacattcccaagtttaaggtaacaggctcgtataatctggtggatactctagtaaagtcaggactgacagaggtgttcggttcaactggagattatagcaatatgtgtaattcagat

SEQ ID NO: 3251 - DNA, 120 bp, synthetic construct
  source 1..120: mol_type = other DNA
tcaggactgacagaggtgttcggttcaactggagattatagcaatatgtgtaattcagatgtgagtgtcgacgctatgatccacaaaacgtatatagatgtcaatgaagagtatacagaa

SEQ ID NO: 3252 - DNA, 120 bp, synthetic construct
  source 1..120: mol_type = other DNA
gtgagtgtcgacgctatgatccacaaaacgtatatagatgtcaatgaagagtatacagaagcagctgcagcaacttgtgcactggtgtcagactgtgcatcaacaattacaaatgagttc

SEQ ID NO: 3253 - DNA, 120 bp, synthetic construct
  source 1..120: mol_type = other DNA
gcagctgcagcaacttgtgcactggtgtcagactgtgcatcaacaattacaaatgagttctgtgtagatcatccgttcatctatgtgattaggcatgttgatggcaaaattcttttcgtt

SEQ ID NO: 3254 - DNA, 120 bp, synthetic construct
  source 1..120: mol_type = other DNA
tgtgtagatcatccgttcatctatgtgattaggcatgttgatggcaaaattcttttcgttggtagatattgctctccaacaactaattgttaaccattttttttaaaaaaatagaaaaaa

SEQ ID NO: 3255 - DNA, 120 bp, synthetic construct
  source 1..120: mol_type = other DNA
ggtagatattgctctccaacaactaattgttaaccattttttttaaaaaaatagaaaaaacatgtggtattagtgcaggtcgttattcttccaattgcaattggtaagatgacggccaac

SEQ ID NO: 3256 - DNA, 120 bp, synthetic construct
  source 1..120: mol_type = other DNA
catgtggtattagtgcaggtcgttattcttccaattgcaattggtaagatgacggccaactttagtacccacgtcttttcaccacagcactgtggatgtgacagactgaccagtattgat

SEQ ID NO: 3257 - DNA, 120 bp, synthetic construct
  source 1..120: mol_type = other DNA
tttagtacccacgtcttttcaccacagcactgtggatgtgacagactgaccagtattgatgacgtcaaacaatgtttgactgaatatatttattggtcgtcctatgcataccgcaacagg

SEQ ID NO: 3258 - DNA, 120 bp, synthetic construct
  source 1..120: mol_type = other DNA
gacgtcaaacaatgtttgactgaatatatttattggtcgtcctatgcataccgcaacaggcaatgcgctggacagttgtattccacactcctctcttttagagatgatgcggaattagtg

SEQ ID NO: 3259 - DNA, 120 bp, synthetic construct
  source 1..120: mol_type = other DNA
caatgcgctggacagttgtattccacactcctctcttttagagatgatgcggaattagtgttcatcgacattcgcgagctggtaaaacatatgccgtgggatgatgtcaaagattgtgca

SEQ ID NO: 3260 - DNA, 120 bp, synthetic construct
  source 1..120: mol_type = other DNA
ttcatcgacattcgcgagctggtaaaacatatgccgtgggatgatgtcaaagattgtgcagaaatcatccgttgttatataccggatgagcaaaaaaccatcagagagatttcggccatc

SEQ ID NO: 3261 - DNA, 120 bp, synthetic construct
  source 1..120: mol_type = other DNA
gaaatcatccgttgttatataccggatgagcaaaaaaccatcagagagatttcggccatcatcggactttgtgcatatgctgctacttactggggaggtgaagaccatcccactagtaac

SEQ ID NO: 3262 - DNA, 120 bp, synthetic construct
  source 1..120: mol_type = other DNA
atcggactttgtgcatatgctgctacttactggggaggtgaagaccatcccactagtaacagtctgaacgcattgtttgtgatgcttgagatgctaaattacgtggattataacatcata

SEQ ID NO: 3263 - DNA, 120 bp, synthetic construct
  source 1..120: mol_type = other DNA
gctgctacttactggggaggtgaagaccatcccactagtaacagtctgaacgcattgtttgtgatgcttgagatgctaaattacgtggattataacatcatattccggcgtatgaattga

SEQ ID NO: 3264 - DNA, 120 bp, synthetic construct
  source 1..120: mol_type = other DNA
tggatattaccgcgttttatcagacgttttttgatgaagcagatgaactgttggcagatatggaacagcatttgttattgctggacccgctgacacctgacaatgaacagcttaatgcta

SEQ ID NO: 3265 - DNA, 120 bp, synthetic construct
  source 1..120: mol_type = other DNA
tggaacagcatttgttattgctggacccgctgacacctgacaatgaacagcttaatgctattttccgtgctgcacattcgatcaagggcggtgccgctacttttggttttacggtattgc

SEQ ID NO: 3266 - DNA, 120 bp, synthetic construct
  source 1..120: mol_type = other DNA
ttttccgtgctgcacattcgatcaagggcggtgccgctacttttggttttacggtattgcaagagacaactcatctattggaaaacctgttggatggtgctcgccgcgacgagatgcgct

SEQ ID NO: 3267 - DNA, 120 bp, synthetic construct
  source 1..120: mol_type = other DNA
aagagacaactcatctattggaaaacctgttggatggtgctcgccgcgacgagatgcgcttaagcactgagatcatcaacctgtttttggaaacgaaagatattatgcaggaacagttgg

SEQ ID NO: 3268 - DNA, 120 bp, synthetic construct
  source 1..120: mol_type = other DNA
taagcactgagatcatcaacctgtttttggaaacgaaagatattatgcaggaacagttggacgcctacaaaacctctcaggaacctcattcggaaagctttgagtacatttgtcaggcgt

SEQ ID NO: 3269 - DNA, 120 bp, synthetic construct
  source 1..120: mol_type = other DNA
acgcctacaaaacctctcaggaacctcattcggaaagctttgagtacatttgtcaggcgttgcgccaattggcacttgatgctttagatcaacctacaaccgaagatcaacctacaaccg

SEQ ID NO: 3270 - DNA, 120 bp, synthetic construct
  source 1..120: mol_type = other DNA
tgcgccaattggcacttgatgctttagatcaacctacaaccgaagatcaacctacaaccgaaaatcaatccgctaccgatcagcacagtacggccgccaatacgcaagcaacggcttcca

SEQ ID NO: 3271 - DNA, 120 bp, synthetic construct
  source 1..120: mol_type = other DNA
aaaatcaatccgctaccgatcagcacagtacggccgccaatacgcaagcaacggcttccacccgcgtatcatcttctctcgctggcaacacatcacccgcgttgcttcaaggcgggatgc

SEQ ID NO: 3272 - DNA, 120 bp, synthetic construct
  source 1..120: mol_type = other DNA
cccgcgtatcatcttctctcgctggcaacacatcacccgcgttgcttcaaggcgggatgcgtattcgtttgtctggcctgaaagcgccagaaatctctctgatgctggaggaactgggta

SEQ ID NO: 3273 - DNA, 120 bp, synthetic construct
  source 1..120: mol_type = other DNA
gtattcgtttgtctggcctgaaagcgccagaaatctctctgatgctggaggaactgggtaatctgggcgaggtgcaagatccccatcagggcgctgatagccttgaggccaccttaataa

SEQ ID NO: 3274 - DNA, 120 bp, synthetic construct
  source 1..120: mol_type = other DNA
atctgggcgaggtgcaagatccccatcagggcgctgatagccttgaggccaccttaataacctccgtcagtgaagaggatattagcgcggtattgtgctttgttctggaacctgagcaga

SEQ ID NO: 3275 - DNA, 120 bp, synthetic construct
  source 1..120: mol_type = other DNA
cctccgtcagtgaagaggatattagcgcggtattgtgctttgttctggaacctgagcagattagctttgtgtccgcaggggacaccgagcagatttatgctgagcagaccgttgaatcag

SEQ ID NO: 3276 - DNA, 120 bp, synthetic construct
  source 1..120: mol_type = other DNA
ttagctttgtgtccgcaggggacaccgagcagatttatgctgagcagaccgttgaatcagaacaatcatctgagccagaacgcttgtttgagccagcaataaccgaggcatcggtgatcg

SEQ ID NO: 3277 - DNA, 120 bp, synthetic construct
  source 1..120: mol_type = other DNA
aacaatcatctgagccagaacgcttgtttgagccagcaataaccgaggcatcggtgatcgcagaatcggttcagccggtggcaacacctgccgcaacacctgccgttgaagtccaaagca

SEQ ID NO: 3278 - DNA, 120 bp, synthetic construct
  source 1..120: mol_type = other DNA
cagaatcggttcagccggtggcaacacctgccgcaacacctgccgttgaagtccaaagcacgctgaaagctgatgtgcatgctgcaccagctaacgcagaacaggtcaggcctaaagcga

SEQ ID NO: 3279 - DNA, 120 bp, synthetic construct
  source 1..120: mol_type = other DNA
cgctgaaagctgatgtgcatgctgcaccagctaacgcagaacaggtcaggcctaaagcgaaagccagtgaatcgaccagtatccgtgtagcggtagaaaaagtggaccagctgattaacc

SEQ ID NO: 3280 - DNA, 120 bp, synthetic construct
  source 1..120: mol_type = other DNA
aagccagtgaatcgaccagtatccgtgtagcggtagaaaaagtggaccagctgattaacctggtcggcgaattggttattacccaatcgatgctcgctcagcgctcaagttcgctggatc

SEQ ID NO: 3281 - DNA, 120 bp, synthetic construct
  source 1..120: mol_type = other DNA
tggtcggcgaattggttattacccaatcgatgctcgctcagcgctcaagttcgctggatccggtgatcaacggtgatttactgaatagcatggggcagttggaacgtaacgcccgcgatt

SEQ ID NO: 3282 - DNA, 120 bp, synthetic construct
  source 1..120: mol_type = other DNA
cggtgatcaacggtgatttactgaatagcatggggcagttggaacgtaacgcccgcgatttgcaagaatccgtcatgtctatccggatgatgccaatggagtatgtatttagccgcttcc

SEQ ID NO: 3283 - DNA, 120 bp, synthetic construct
  source 1..120: mol_type = other DNA
tgcaagaatccgtcatgtctatccggatgatgccaatggagtatgtatttagccgcttcccacgtttggtccgtgatttagccagcaagctcaacaaacaagttgaattgacgctgttag

SEQ ID NO: 3284 - DNA, 120 bp, synthetic construct
  source 1..120: mol_type = other DNA
cacgtttggtccgtgatttagccagcaagctcaacaaacaagttgaattgacgctgttaggcagttcgacagaactggataagagtttgattgagcgcattatcgatcctctgacccact

SEQ ID NO: 3285 - DNA, 120 bp, synthetic construct
  source 1..120: mol_type = other DNA
gcagttcgacagaactggataagagtttgattgagcgcattatcgatcctctgacccacttggtgcgcaacagtctggaccacggtattgaagagccggctactcgtattgctgcgggga

SEQ ID NO: 3286 - DNA, 120 bp, synthetic construct
  source 1..120: mol_type = other DNA
tggtgcgcaacagtctggaccacggtattgaagagccggctactcgtattgctgcggggaaatcgccagtgggcaacctgacactgtcagctgaacatcagggcggaaatatttgtatcg

SEQ ID NO: 3287 - DNA, 120 bp, synthetic construct
  source 1..120: mol_type = other DNA
aatcgccagtgggcaacctgacactgtcagctgaacatcagggcggaaatatttgtatcgaagtcattgatgatggtgctggcctgaatcgacagagaattttggcgaaagcacagtctc

SEQ ID NO: 3288 - DNA, 120 bp, synthetic construct
  source 1..120: mol_type = other DNA
aagtcattgatgatggtgctggcctgaatcgacagagaattttggcgaaagcacagtctcaagggctggcagtcaacgaaaacatgagcgatgaagacgttgggatgcttatttttgcac

SEQ ID NO: 3289 - DNA, 120 bp, synthetic construct
  source 1..120: mol_type = other DNA
aagggctggcagtcaacgaaaacatgagcgatgaagacgttgggatgcttatttttgcacaaggattctctactgccgaacaagtcacggatgtgtcagggcgtggtgtcgggatggatg

SEQ ID NO: 3290 - DNA, 120 bp, synthetic construct
  source 1..120: mol_type = other DNA
aaggattctctactgccgaacaagtcacggatgtgtcagggcgtggtgtcgggatggatgtggtcaaacgtaacatccaggaaatgggcggccatgtacaggtcagttttcaggccggtt

SEQ ID NO: 3291 - DNA, 120 bp, synthetic construct
  source 1..120: mol_type = other DNA
tggtcaaacgtaacatccaggaaatgggcggccatgtacaggtcagttttcaggccggtttaggtacctcaatccgtatcctgctgccattaacgctggctatccttgatggcatgtcgg

SEQ ID NO: 3292 - DNA, 120 bp, synthetic construct
  source 1..120: mol_type = other DNA
taggtacctcaatccgtatcctgctgccattaacgctggctatccttgatggcatgtcggttaaagtcagcaatgaagtctttatcttgccattgaatgccgtgatggagtcactgcaac

SEQ ID NO: 3293 - DNA, 120 bp, synthetic construct
  source 1..120: mol_type = other DNA
ttaaagtcagcaatgaagtctttatcttgccattgaatgccgtgatggagtcactgcaacccttggccgaagacctacatccattagccggtggtgagcgcgtgctgcaagttcgcggtg

SEQ ID NO: 3294 - DNA, 120 bp, synthetic construct
  source 1..120: mol_type = other DNA
ccttggccgaagacctacatccattagccggtggtgagcgcgtgctgcaagttcgcggtgaatttctaccattggttgaattgtaccgcgtctttgatgttaaaaatgccaagacggaag

SEQ ID NO: 3295 - DNA, 120 bp, synthetic construct
  source 1..120: mol_type = other DNA
aatttctaccattggttgaattgtaccgcgtctttgatgttaaaaatgccaagacggaagccacgcaaggcatcgttgtgattctacaaagtgccgggcgccgctatgcactgctggtag

SEQ ID NO: 3296 - DNA, 120 bp, synthetic construct
  source 1..120: mol_type = other DNA
ccacgcaaggcatcgttgtgattctacaaagtgccgggcgccgctatgcactgctggtagaccaactgattggtcagcatcaggtggtcgtgaaaaatctggaaagtaactatcggaaag

SEQ ID NO: 3297 - DNA, 120 bp, synthetic construct
  source 1..120: mol_type = other DNA
accaactgattggtcagcatcaggtggtcgtgaaaaatctggaaagtaactatcggaaagtgccgggtatttctgccgccaccattttgggtgatggtagcgtcgcgctaatcgttgatg

SEQ ID NO: 3298 - DNA, 120 bp, synthetic construct
  source 1..120: mol_type = other DNA
tgccgggtatttctgccgccaccattttgggtgatggtagcgtcgcgctaatcgttgatgtgtcagcgttgcaggccttaaaccgtgaaaaacgcgtcgcggctgatgaggtggttaccg

SEQ ID NO: 3299 - DNA, 120 bp, synthetic construct
  source 1..120: mol_type = other DNA
tgtcagcgttgcaggccttaaaccgtgaaaaacgcgtcgcggctgatgaggtggttaccgcatagcgcacaggaatttttccttataaaaacaggtaataccctaaataatttgagtgca

SEQ ID NO: 3300 - DNA, 120 bp, synthetic construct
  source 1..120: mol_type = other DNA
catagcgcacaggaatttttccttataaaaacaggtaataccctaaataatttgagtgcagcaagccaccaccggccactttaaatatgacgggtatccagggcggtgaaatatgtttcc

SEQ ID NO: 3301 - DNA, 120 bp, synthetic construct
  source 1..120: mol_type = other DNA
gcaagccaccaccggccactttaaatatgacgggtatccagggcggtgaaatatgtttccggtcctgaaaaacataaattcaacctattgattgaagggtaaaaaacatggcaggactag

SEQ ID NO: 3302 - DNA, 120 bp, synthetic construct
  source 1..120: mol_type = other DNA
ggtcctgaaaaacataaattcaacctattgattgaagggtaaaaaacatggcaggactagcaaccgtcacgaaactggctggcgaaacggtaggacaagaattcctgatttttacgctgg

SEQ ID NO: 3303 - DNA, 120 bp, synthetic construct
  source 1..120: mol_type = other DNA
caaccgtcacgaaactggctggcgaaacggtaggacaagaattcctgatttttacgctgggcgatgaagagtacggcatcgatattctgaaagtacaagagatccgaggctatgatcagg

SEQ ID NO: 3304 - DNA, 120 bp, synthetic construct
  source 1..120: mol_type = other DNA
gcgatgaagagtacggcatcgatattctgaaagtacaagagatccgaggctatgatcaggtgactcgtattgctaacactcctgcgtttattaaaggtgtgaccaacttacgcggcgtca

SEQ ID NO: 3305 - DNA, 120 bp, synthetic construct
  source 1..120: mol_type = other DNA
tgactcgtattgctaacactcctgcgtttattaaaggtgtgaccaacttacgcggcgtcattgtgcctatcattgatctgcgggttaaattcgcccagcaaggtgtcacttataacgaaa

SEQ ID NO: 3306 - DNA, 120 bp, synthetic construct
  source 1..120: mol_type = other DNA
ttgtgcctatcattgatctgcgggttaaattcgcccagcaaggtgtcacttataacgaaaataccgtggtgattgtgctgaattttggtcaacgcgtggtgggtattgtcgttgatggtg

SEQ ID NO: 3307 - DNA, 120 bp, synthetic construct
  source 1..120: mol_type = other DNA
ataccgtggtgattgtgctgaattttggtcaacgcgtggtgggtattgtcgttgatggtgtgtcagatgtcctgtcgttgaccaacgagcagatccgtccggcacctgaatttgctgtga

SEQ ID NO: 3308 - DNA, 120 bp, synthetic construct
  source 1..120: mol_type = other DNA
tgtcagatgtcctgtcgttgaccaacgagcagatccgtccggcacctgaatttgctgtgactctcgcaacagaatatctgaccggtttaggctcgcttggcgaaagaatgttgatcctgg

SEQ ID NO: 3309 - DNA, 120 bp, synthetic construct
  source 1..120: mol_type = other DNA
ctctcgcaacagaatatctgaccggtttaggctcgcttggcgaaagaatgttgatcctggttgatatcgaaaaactgctgagcagtgaagagatgtcgttgattgatagtgtttctaagg

SEQ ID NO: 3310 - DNA, 120 bp, synthetic construct
  source 1..120: mol_type = other DNA
ttgatatcgaaaaactgctgagcagtgaagagatgtcgttgattgatagtgtttctaaggcgtgataatagtctttttaatatgtgacaatagtgttgctaaggtgtgattgaagcgtgg

SEQ ID NO: 3311 - DNA, 120 bp, synthetic construct
  source 1..120: mol_type = other DNA
cgtgataatagtctttttaatatgtgacaatagtgttgctaaggtgtgattgaagcgtggagtttacgcacgttgagtgatcacctgagccaatcggccttaaccaagcaggggaggcgg

SEQ ID NO: 3312 - DNA, 120 bp, synthetic construct
  source 1..120: mol_type = other DNA
agtttacgcacgttgagtgatcacctgagccaatcggccttaaccaagcaggggaggcggtcctcctgcccctacggcttgcgcgaaatattgccctacgggtaaagcgtcagcgtcttt

SEQ ID NO: 3313 - DNA, 120 bp, synthetic construct
  source 1..120: mol_type = other DNA
tcctcctgcccctacggcttgcgcgaaatattgccctacgggtaaagcgtcagcgtctttcgggctgatgaatagaggactattcaatgactcctgaaataaagaactgaaccgccattg

SEQ ID NO: 3314 - DNA, 120 bp, synthetic construct
  source 1..120: mol_type = other DNA
cgggctgatgaatagaggactattcaatgactcctgaaataaagaactgaaccgccattgcatattgctcgggcggttctttatgacaagtcatgatgttgagatagtcattttatttag

SEQ ID NO: 3315 - DNA, 120 bp, synthetic construct
  source 1..120: mol_type = other DNA
catattgctcgggcggttctttatgacaagtcatgatgttgagatagtcattttatttaggctacagctactgcacgcattctttttgttaaaatagtggcacaaataaaaccaagaaga

SEQ ID NO: 3316 - DNA, 120 bp, synthetic construct
  source 1..120: mol_type = other DNA
gctacagctactgcacgcattctttttgttaaaatagtggcacaaataaaaccaagaagactaaacgctaccatgagtgaaaatatgtagttgtacccctgaatcccctcaaaattatct

SEQ ID NO: 3317 - DNA, 120 bp, synthetic construct
  source 1..120: mol_type = other DNA
ctaaacgctaccatgagtgaaaatatgtagttgtacccctgaatcccctcaaaattatctaataatgagccataaagtgcgtaggcaaacatggacggcatatagccgataatacacccg

SEQ ID NO: 3318 - DNA, 120 bp, synthetic construct
  source 1..120: mol_type = other DNA
aataatgagccataaagtgcgtaggcaaacatggacggcatatagccgataatacacccgaaggccattgccgaacctgcatgttcacgagaagtaccaatttcatccatcggggcgaag

SEQ ID NO: 3319 - DNA, 120 bp, synthetic construct
  source 1..120: mol_type = other DNA
aaggccattgccgaacctgcatgttcacgagaagtaccaatttcatccatcggggcgaagaagattgcgcgctgagagaagataatggctccgaagccgagtgttgccatcatacccaag

SEQ ID NO: 3320 - DNA, 120 bp, synthetic construct
  source 1..120: mol_type = other DNA
aagattgcgcgctgagagaagataatggctccgaagccgagtgttgccatcatacccaagtatacgttcatcgaatcatggggtaattggatgaataagatcatcgctatggccgaaatt

SEQ ID NO: 3321 - DNA, 120 bp, synthetic construct
  source 1..120: mol_type = other DNA
tatacgttcatcgaatcatggggtaattggatgaataagatcatcgctatggccgaaattaaaaatgtccatttcaggtaaactgtcggtgattttgcgactttgtcagcgaggaatccc

SEQ ID NO: 3322 - DNA, 120 bp, synthetic construct
  source 1..120: mol_type = other DNA
aaaaatgtccatttcaggtaaactgtcggtgattttgcgactttgtcagcgaggaatcccccaacaggtcctcctaccattttgagaccgtactgattaatgatcccgtaagcgccaata

SEQ ID NO: 3323 - DNA, 120 bp, synthetic construct
  source 1..120: mol_type = other DNA
ccaacaggtcctcctaccattttgagaccgtactgattaatgatcccgtaagcgccaataagagcgactggcaatccataaatatctttgaggaatggtatgaaataggttaagccgcaa

SEQ ID NO: 3324 - DNA, 120 bp, synthetic construct
  source 1..120: mol_type = other DNA
agagcgactggcaatccataaatatctttgaggaatggtatgaaataggttaagccgcaataggcggaatagacaaagaagatacagaaagaagccaaccacaagttagggcttttaata

SEQ ID NO: 3325 - DNA, 120 bp, synthetic construct
  source 1..120: mol_type = other DNA
taggcggaatagacaaagaagatacagaaagaagccaaccacaagttagggcttttaataacatctttgatccccgccaaaacatgtttattaactttatctgcattatctaccttaatc

SEQ ID NO: 3326 - DNA, 120 bp, synthetic construct
  source 1..120: mol_type = other DNA
acatctttgatccccgccaaaacatgtttattaactttatctgcattatctaccttaatcttgtcatcactgtctacgataaaccaagtaatgacgccaaccaatatcgtggctatcgtg

SEQ ID NO: 3327 - DNA, 120 bp, synthetic construct
  source 1..120: mol_type = other DNA
ttgtcatcactgtctacgataaaccaagtaatgacgccaaccaatatcgtggctatcgtgtaatagattagcccggcctgcatccccgctttaccttcaccaaactgaacaaaaacaaac

SEQ ID NO: 3328 - DNA, 120 bp, synthetic construct
  source 1..120: mol_type = other DNA
taatagattagcccggcctgcatccccgctttaccttcaccaaactgaacaaaaacaaacagggcaccagaagcgataagtacatcaatcacaccgcgacccgcttccagaaaaccaaac

SEQ ID NO: 3329 - DNA, 120 bp, synthetic construct
  source 1..120: mol_type = other DNA
agggcaccagaagcgataagtacatcaatcacaccgcgacccgcttccagaaaaccaaacatgcgtccttgttcttctttggttcccagcaaccttactgctttcaacagtacaggccag

SEQ ID NO: 3330 - DNA, 120 bp, synthetic construct
  source 1..120: mol_type = other DNA
atgcgtccttgttcttctttggttcccagcaaccttactgctttcaacagtacaggccagtaaaccacttccccaaaaaatgccatagcaccaaaggcgatgagataaccggtaaacggt

SEQ ID NO: 3331 - DNA, 120 bp, synthetic construct
  source 1..120: mol_type = other DNA
taaaccacttccccaaaaaatgccatagcaccaaaggcgatgagataaccggtaaacggtggaagcgtggctaagtatgcgccacagaggcccacaccgatcaaccctacgggcagtaag

SEQ ID NO: 3332 - DNA, 120 bp, synthetic construct
  source 1..120: mol_type = other DNA
ggaagcgtggctaagtatgcgccacagaggcccacaccgatcaaccctacgggcagtaagatctttttcgaaaaacgatcagcaatataaagagaactgaataagccaacggtctgaatg

SEQ ID NO: 3333 - DNA, 120 bp, synthetic construct
  source 1..120: mol_type = other DNA
atctttttcgaaaaacgatcagcaatataaagagaactgaataagccaacggtctgaatgatggcatatacggtaaaaccaaaaccaatctgtgtattcgttagcccccagtcttgttgc

SEQ ID NO: 3334 - DNA, 120 bp, synthetic construct
  source 1..120: mol_type = other DNA
atggcatatacggtaaaaccaaaaccaatctgtgtattcgttagcccccagtcttgttgcatagggatgtaaaacacatctttcatactggagagtttgaaaatcgtccctccacccaaa

SEQ ID NO: 3335 - DNA, 120 bp, synthetic construct
  source 1..120: mol_type = other DNA
atagggatgtaaaacacatctttcatactggagagtttgaaaatcgtccctccacccaaaatgaggaagcaaagctttgtccatttattcacaatattcctaccttattttagagagaca

SEQ ID NO: 3336 - DNA, 120 bp, synthetic construct
  source 1..120: mol_type = other DNA
atgaggaagcaaagctttgtccatttattcacaatattcctaccttattttagagagacaatagcctctacttcaatgagaacgtcttttggtagccgagcgacttcaacacatgaacgg

SEQ ID NO: 3337 - DNA, 120 bp, synthetic construct
  source 1..120: mol_type = other DNA
atagcctctacttcaatgagaacgtcttttggtagccgagcgacttcaacacatgaacgggcagggaatgtccctgatgggaaatagcccgcgtaaatggtattgaatgactgaaaattg

SEQ ID NO: 3338 - DNA, 120 bp, synthetic construct
  source 1..120: mol_type = other DNA
gcagggaatgtccctgatgggaaatagcccgcgtaaatggtattgaatgactgaaaattgttcatatcactgataaagcaagtggttttaaccacgtcattcatataactaccggtggct

SEQ ID NO: 3339 - DNA, 120 bp, synthetic construct
  source 1..120: mol_type = other DNA
ttcatatcactgataaagcaagtggttttaaccacgtcattcatataactaccggtggcttccacaatagcctttaggtttttcatggcttgaatggtttgctctgtaatatcaatacct

SEQ ID NO: 3340 - DNA, 120 bp, synthetic construct
  source 1..120: mol_type = other DNA
tccacaatagcctttaggtttttcatggcttgaatggtttgctctgtaatatcaatacctacgactgatccatctttttcactgaaagggcagcaaccggaaataaaaagcaaattaccg

SEQ ID NO: 3341 - DNA, 120 bp, synthetic construct
  source 1..120: mol_type = other DNA
acgactgatccatctttttcactgaaagggcagcaaccggaaataaaaagcaaattaccggcgacaacgccttgggagtatggtccgatagctgctggtgcgttttgagttttaataatc

SEQ ID NO: 3342 - DNA, 120 bp, synthetic construct
  source 1..120: mol_type = other DNA
gcgacaacgccttgggagtatggtccgatagctgctggtgcgttttgagttttaataatcattcgacgattcctgttgtggtgttggggcaatatttatcacgcagtgctttgagcactt

SEQ ID NO: 3343 - DNA, 120 bp, synthetic construct
  source 1..120: mol_type = other DNA
attcgacgattcctgttgtggtgttggggcaatatttatcacgcagtgctttgagcacttgaaccgatgtataaacacagtggtcctgagcttgcataagctcttgtagtaactctggcg

SEQ ID NO: 3344 - DNA, 120 bp, synthetic construct
  source 1..120: mol_type = other DNA
gaaccgatgtataaacacagtggtcctgagcttgcataagctcttgtagtaactctggcgatattttgtcggggtagtaatattccagtggtttaattcggctggagtcaaaaggagggg

SEQ ID NO: 3345 - DNA, 120 bp, synthetic construct
  source 1..120: mol_type = other DNA
atattttgtcggggtagtaatattccagtggtttaattcggctggagtcaaaaggaggggtttttacttcaaaagtcccttttagtgtactgacttcattggggttgcaaggtcgagaaa

SEQ ID NO: 3346 - DNA, 120 bp, synthetic construct
  source 1..120: mol_type = other DNA
tttttacttcaaaagtcccttttagtgtactgacttcattggggttgcaaggtcgagaaaatgcagaggcataaggaaagcaggtttcaatattgacccgagttatgcctgatttttcaa

SEQ ID NO: 3347 - DNA, 120 bp, synthetic construct
  source 1..120: mol_type = other DNA
atgcagaggcataaggaaagcaggtttcaatattgacccgagttatgcctgatttttcaaccaatattctgaagcaattatcaatatcgatactcccttcaccgataggaacgccacata

SEQ ID NO: 3348 - DNA, 120 bp, synthetic construct
  source 1..120: mol_type = other DNA
ccaatattctgaagcaattatcaatatcgatactcccttcaccgataggaacgccacataccactaattgctcgtcatgttgagtaacaatgtgatctttaaaatgggtactgtaagtaa

SEQ ID NO: 3349 - DNA, 120 bp, synthetic construct
  source 1..120: mol_type = other DNA
ccactaattgctcgtcatgttgagtaacaatgtgatctttaaaatgggtactgtaagtaaagggggcaagttggctgacagtgacaacgggctcttcccaagccatcatgccatttccta

SEQ ID NO: 3350 - DNA, 120 bp, synthetic construct
  source 1..120: mol_type = other DNA
agggggcaagttggctgacagtgacaacgggctcttcccaagccatcatgccatttcctatatcgcaatgtgccccgacccatagggagtctaccgcttttacaatttggataatctcgt

SEQ ID NO: 3351 - DNA, 120 bp, synthetic construct
  source 1..120: mol_type = other DNA
tatcgcaatgtgccccgacccatagggagtctaccgcttttacaatttggataatctcgtcggcagtttcatcttcatgattttcaacggccagacgaattcgatttgcctgaagtagag

SEQ ID NO: 3352 - DNA, 120 bp, synthetic construct
  source 1..120: mol_type = other DNA
cggcagtttcatcttcatgattttcaacggccagacgaattcgatttgcctgaagtagaggaaccagtgatttcaactcatgaataatgcgtggatattctaggggctcatactgaccac

SEQ ID NO: 3353 - DNA, 120 bp, synthetic construct
  source 1..120: mol_type = other DNA
gaaccagtgatttcaactcatgaataatgcgtggatattctaggggctcatactgaccacgacggaacatgtaggttcgaataacatccgcacccagtgcagatgcaaattgcacggctt

SEQ ID NO: 3354 - DNA, 120 bp, synthetic construct
  source 1..120: mol_type = other DNA
gacggaacatgtaggttcgaataacatccgcacccagtgcagatgcaaattgcacggctttactaatcgctttaaccgacgtaaaacgggtatcgatttcacaataaagattgcgttgtt

SEQ ID NO: 3355 - DNA, 120 bp, synthetic construct
  source 1..120: mol_type = other DNA
tactaatcgctttaaccgacgtaaaacgggtatcgatttcacaataaagattgcgttgttcgatagcgtgtctcacccgtgcaagatatgttgggtcatcgctactcaacacaccaaatt

SEQ ID NO: 3356 - DNA, 120 bp, synthetic construct
  source 1..120: mol_type = other DNA
cgatagcgtgtctcacccgtgcaagatatgttgggtcatcgctactcaacacaccaaattcagggtgaaggccctcatctggaatgatatttatttctacgccatccagtcctaaactcc

SEQ ID NO: 3357 - DNA, 120 bp, synthetic construct
  source 1..120: mol_type = other DNA
cagggtgaaggccctcatctggaatgatatttatttctacgccatccagtcctaaactccaggctttatcaatgaaatcaaaaatatccattttcccctgctggaaaaaaagatgatagg

SEQ ID NO: 3358 - DNA, 120 bp, synthetic construct
  source 1..120: mol_type = other DNA
aggctttatcaatgaaatcaaaaatatccattttcccctgctggaaaaaaagatgataggactcagtctctaaaccaattttcataggattatctccattaatgactaatttggagttta

SEQ ID NO: 3359 - DNA, 120 bp, synthetic construct
  source 1..120: mol_type = other DNA
actcagtctctaaaccaattttcataggattatctccattaatgactaatttggagtttagggtttaaagaaagtcataaccgtgacaaaggtaatgtttttgtattcttagtataaata

SEQ ID NO: 3360 - DNA, 120 bp, synthetic construct
  source 1..120: mol_type = other DNA
gggtttaaagaaagtcataaccgtgacaaaggtaatgtttttgtattcttagtataaatatattttactaagtgtactgtttagatactgtattggacagagggcagcgagaggtgtagc

SEQ ID NO: 3361 - DNA, 120 bp, synthetic construct
  source 1..120: mol_type = other DNA
tattttactaagtgtactgtttagatactgtattggacagagggcagcgagaggtgtagcatgatacacacgacaatttttcttgggtaacatcatgagagatatattaaataaagcatt

SEQ ID NO: 3362 - DNA, 120 bp, synthetic construct
  source 1..120: mol_type = other DNA
atgatacacacgacaatttttcttgggtaacatcatgagagatatattaaataaagcatttactgatgatgatcggagattattacagtcttatattcccttcatagagtgcttgggaca

SEQ ID NO: 3363 - DNA, 120 bp, synthetic construct
  source 1..120: mol_type = other DNA
tactgatgatgatcggagattattacagtcttatattcccttcatagagtgcttgggacagttttttggtgagtactgtgaaattgtactgcacagttttgaagatcttcatcgttccgt

SEQ ID NO: 3364 - DNA, 120 bp, synthetic construct
  source 1..120: mol_type = other DNA
gttttttggtgagtactgtgaaattgtactgcacagttttgaagatcttcatcgttccgtgatccacattgtgaatgggcatgttactggcagagagttaggtgcgccggtcaccaatat

SEQ ID NO: 3365 - DNA, 120 bp, synthetic construct
  source 1..120: mol_type = other DNA
gatccacattgtgaatgggcatgttactggcagagagttaggtgcgccggtcaccaatatagccttggaaaaactgacagaattcaaatcatcaaaagagatgtgggatgtttatttcag

SEQ ID NO: 3366 - DNA, 120 bp, synthetic construct
  source 1..120: mol_type = other DNA
agccttggaaaaactgacagaattcaaatcatcaaaagagatgtgggatgtttatttcagcaataaagatacgcgtccttttaagtcttcatccactctgatagttaacaaacagggcga

SEQ ID NO: 3367 - DNA, 120 bp, synthetic construct
  source 1..120: mol_type = other DNA
caataaagatacgcgtccttttaagtcttcatccactctgatagttaacaaacagggcgatccaataggaatgatatgcatgaatatggcgatggatatgccaatgaatgcttttatcga

SEQ ID NO: 3368 - DNA, 120 bp, synthetic construct
  source 1..120: mol_type = other DNA
tccaataggaatgatatgcatgaatatggcgatggatatgccaatgaatgcttttatcgatatattcatgaaagccaataatagttgtagaaatgagagttttacacaggatgtcaataa

SEQ ID NO: 3369 - DNA, 120 bp, synthetic construct
  source 1..120: mol_type = other DNA
tatattcatgaaagccaataatagttgtagaaatgagagttttacacaggatgtcaataacctggtccaaagccaccttgaaccggttaagagtatggtttatgcgaataaagacatccc

SEQ ID NO: 3370 - DNA, 120 bp, synthetic construct
  source 1..120: mol_type = other DNA
cctggtccaaagccaccttgaaccggttaagagtatggtttatgcgaataaagacatccctagtaagaacaaaaatttcgaaataatcaaagaattaaatgaaacgggtttatttgaact

SEQ ID NO: 3371 - DNA, 120 bp, synthetic construct
  source 1..120: mol_type = other DNA
tagtaagaacaaaaatttcgaaataatcaaagaattaaatgaaacgggtttatttgaactccccgtaacaaataaaattgtctccgcaagtctggggattagtccggtgaccatttataa

SEQ ID NO: 3372 - DNA, 120 bp, synthetic construct
  source 1..120: mol_type = other DNA
ccccgtaacaaataaaattgtctccgcaagtctggggattagtccggtgaccatttataaacatttaagaacgctaaatgcacaaaaagtcagtgagtgaggtcctcgactttggctatg

SEQ ID NO: 3373 - DNA, 120 bp, synthetic construct
  source 1..120: mol_type = other DNA
acatttaagaacgctaaatgcacaaaaagtcagtgagtgaggtcctcgactttggctatgatagtgccttccctgatgttcggttggccgaatagtatcgccataaattttatggcgaag

SEQ ID NO: 3374 - DNA, 120 bp, synthetic construct
  source 1..120: mol_type = other DNA
atagtgccttccctgatgttcggttggccgaatagtatcgccataaattttatggcgaagtaacattaatatggagaagtaacattaatatggcaaaataacattaacattgcaaaataa

SEQ ID NO: 3375 - DNA, 120 bp, synthetic construct
  source 1..120: mol_type = other DNA
taacattaatatggagaagtaacattaatatggcaaaataacattaacattgcaaaataacattaaactgacacgattaattaacaattattgttcttggtgatgttaatgtaattattg

SEQ ID NO: 3376 - DNA, 120 bp, synthetic construct
  source 1..120: mol_type = other DNA
cattaaactgacacgattaattaacaattattgttcttggtgatgttaatgtaattattgttggtgttatttgttattcaatttattttaattaatgtgtttaggatatttcctacaaaa

SEQ ID NO: 3377 - DNA, 120 bp, synthetic construct
  source 1..120: mol_type = other DNA
ttggtgttatttgttattcaatttattttaattaatgtgtttaggatatttcctacaaaaaaacagtatggtcctattatccccttccttgagccctgttatcctttttcgaatatattc

SEQ ID NO: 3378 - DNA, 120 bp, synthetic construct
  source 1..120: mol_type = other DNA
aaacagtatggtcctattatccccttccttgagccctgttatcctttttcgaatatattccatctgaatgacttaatcgtcgacagacagcacttccaacgttgatcgaacgcttcaact

SEQ ID NO: 3379 - DNA, 120 bp, synthetic construct
  source 1..120: mol_type = other DNA
catctgaatgacttaatcgtcgacagacagcacttccaacgttgatcgaacgcttcaactctttgctgacaatatttagtgagaaggagagaaaatatttttcaggcgatatgtcgtatc

SEQ ID NO: 3380 - DNA, 120 bp, synthetic construct
  source 1..120: mol_type = other DNA
ctttgctgacaatatttagtgagaaggagagaaaatatttttcaggcgatatgtcgtatcggtaataaactggggcagctaatagggtaattctatgttgaaacatttcagactgggtct

SEQ ID NO: 3381 - DNA, 120 bp, synthetic construct
  source 1..120: mol_type = other DNA
ggtaataaactggggcagctaatagggtaattctatgttgaaacatttcagactgggtctttttaccgcaaatgttcaggcggatacagggagccaacactcctttagccgtgttccagc

SEQ ID NO: 3382 - DNA, 120 bp, synthetic construct
  source 1..120: mol_type = other DNA
ttttaccgcaaatgttcaggcggatacagggagccaacactcctttagccgtgttccagcagccgcgattaatcccataacattagcgattgttgtggcgttttctactattgctttacc

SEQ ID NO: 3383 - DNA, 120 bp, synthetic construct
  source 1..120: mol_type = other DNA
agccgcgattaatcccataacattagcgattgttgtggcgttttctactattgctttaccaccaatggcattagcagcatgcaccagccccggggtgggaacctatgtctgcgaaggtga

SEQ ID NO: 3384 - DNA, 120 bp, synthetic construct
  source 1..120: mol_type = other DNA
accaatggcattagcagcatgcaccagccccggggtgggaacctatgtctgcgaaggtgaaaataccgacggcatcatcctgagcggcacggatattgcggttgagacccaacctggttt

SEQ ID NO: 3385 - DNA, 120 bp, synthetic construct
  source 1..120: mol_type = other DNA
aaataccgacggcatcatcctgagcggcacggatattgcggttgagacccaacctggtttcagcataatagttcctgaaaatggagaccctgcactctcgctagtcggttctggcaccat

SEQ ID NO: 3386 - DNA, 120 bp, synthetic construct
  source 1..120: mol_type = other DNA
cagcataatagttcctgaaaatggagaccctgcactctcgctagtcggttctggcaccatcagctaccttgataccaacagttctgcgcttgataccacgggtgccgattctttgtatat

SEQ ID NO: 3387 - DNA, 120 bp, synthetic construct
  source 1..120: mol_type = other DNA
cagctaccttgataccaacagttctgcgcttgataccacgggtgccgattctttgtatatccagaatgatacgcacaccactgggcaatcgtcgtccattaatgttcagacaaacggttc

SEQ ID NO: 3388 - DNA, 120 bp, synthetic construct
  source 1..120: mol_type = other DNA
ccagaatgatacgcacaccactgggcaatcgtcgtccattaatgttcagacaaacggttcaatgggtagcggtatcaatattagcaaccatagcggtgccgactcgacagtacaggtgga

SEQ ID NO: 3389 - DNA, 120 bp, synthetic construct
  source 1..120: mol_type = other DNA
aatgggtagcggtatcaatattagcaaccatagcggtgccgactcgacagtacaggtggatgtttccggcacattatttggtgatctaaatggttctcccgcccttttaatctattcatc

SEQ ID NO: 3390 - DNA, 120 bp, synthetic construct
  source 1..120: mol_type = other DNA
tgtttccggcacattatttggtgatctaaatggttctcccgcccttttaatctattcatcggcggagaataattccactattctcatgaatatcaatactattttcggcgacgtgggtat

SEQ ID NO: 3391 - DNA, 120 bp, synthetic construct
  source 1..120: mol_type = other DNA
ggcggagaataattccactattctcatgaatatcaatactattttcggcgacgtgggtattcgaagcgataacacttcattcaatggaacagccatcactaacgttgatattgctaatga

SEQ ID NO: 3392 - DNA, 120 bp, synthetic construct
  source 1..120: mol_type = other DNA
tcgaagcgataacacttcattcaatggaacagccatcactaacgttgatattgctaatgatattaatgctacatattcgggtgccactatcaacaacagcggtagcggcggtaccagtgt

SEQ ID NO: 3393 - DNA, 120 bp, synthetic construct
  source 1..120: mol_type = other DNA
tattaatgctacatattcgggtgccactatcaacaacagcggtagcggcggtaccagtgtggttaatttcaactcaaaaagcatcattacagaattggacgccttaaatatttataatac

SEQ ID NO: 3394 - DNA, 120 bp, synthetic construct
  source 1..120: mol_type = other DNA
ggttaatttcaactcaaaaagcatcattacagaattggacgccttaaatatttataataccaattattcaggggcggttataaccaatgtcgatatcgatggtgatgtcatttcaacgac

SEQ ID NO: 3395 - DNA, 120 bp, synthetic construct
  source 1..120: mol_type = other DNA
caattattcaggggcggttataaccaatgtcgatatcgatggtgatgtcatttcaacgactagccaggcgacctctttttataacgatgcctacaacggctctgcaaactttacgtttcg

SEQ ID NO: 3396 - DNA, 120 bp, synthetic construct
  source 1..120: mol_type = other DNA
tagccaggcgacctctttttataacgatgcctacaacggctctgcaaactttacgtttcgtgcgaacaatgtcactggtgaatattccggcatttctatcaataatagcagtcataacag

SEQ ID NO: 3397 - DNA, 120 bp, synthetic construct
  source 1..120: mol_type = other DNA
tgcgaacaatgtcactggtgaatattccggcatttctatcaataatagcagtcataacagtgctaataacaaccatgataatgcggtgataaccgatatcctgttgacgggggatcttac

SEQ ID NO: 3398 - DNA, 120 bp, synthetic construct
  source 1..120: mol_type = other DNA
tgctaataacaaccatgataatgcggtgataaccgatatcctgttgacgggggatcttacgtctacttcaggatcgggcctccagataaactcttatatggacgatggggatatcaaggt

SEQ ID NO: 3399 - DNA, 120 bp, synthetic construct
  source 1..120: mol_type = other DNA
gtctacttcaggatcgggcctccagataaactcttatatggacgatggggatatcaaggtatcagcccagttggagaacatctattcttactatgaagccctcagtgtgcgtgcggatac

SEQ ID NO: 3400 - DNA, 120 bp, synthetic construct
  source 1..120: mol_type = other DNA
atcagcccagttggagaacatctattcttactatgaagccctcagtgtgcgtgcggataccctaactggcaacctgcagtttaacatcgatgtttcgggcaatattgttgctgaaaatgg

SEQ ID NO: 3401 - DNA, 120 bp, synthetic construct
  source 1..120: mol_type = other DNA
cctaactggcaacctgcagtttaacatcgatgtttcgggcaatattgttgctgaaaatggcctcggtttcatggtgatggggggcgcttccgaaggcaactccactatgatcatcaatgc

SEQ ID NO: 3402 - DNA, 120 bp, synthetic construct
  source 1..120: mol_type = other DNA
cctcggtttcatggtgatggggggcgcttccgaaggcaactccactatgatcatcaatgcgaataacattagttctggtagtcaagcactcaatatttacaactatagcggtttaggttc

SEQ ID NO: 3403 - DNA, 120 bp, synthetic construct
  source 1..120: mol_type = other DNA
gaataacattagttctggtagtcaagcactcaatatttacaactatagcggtttaggttcggcatttactgccgttaccgcaaccgggcatctcgtctctgaacaggggataggggcaat

SEQ ID NO: 3404 - DNA, 120 bp, synthetic construct
  source 1..120: mol_type = other DNA
ggcatttactgccgttaccgcaaccgggcatctcgtctctgaacaggggataggggcaatgttcagtacctatgtcagtcaaggggatgctaccgctgtcatcaatttaaatgacatcac

SEQ ID NO: 3405 - DNA, 120 bp, synthetic construct
  source 1..120: mol_type = other DNA
gttcagtacctatgtcagtcaaggggatgctaccgctgtcatcaatttaaatgacatcactactgcgggcagtggtgtaaagatagacaccatagcgaatggggggaattcaaccaccta

SEQ ID NO: 3406 - DNA, 120 bp, synthetic construct
  source 1..120: mol_type = other DNA
tactgcgggcagtggtgtaaagatagacaccatagcgaatggggggaattcaaccacctatctcaccgtggtgggccagattaactctagtttgtatgatggtattgatcttcgtgcgac

SEQ ID NO: 3407 - DNA, 120 bp, synthetic construct
  source 1..120: mol_type = other DNA
tctcaccgtggtgggccagattaactctagtttgtatgatggtattgatcttcgtgcgacggctactgaaggtaataccctggtcagcattgacgtcaataatatcgccagtgaatacga

SEQ ID NO: 3408 - DNA, 120 bp, synthetic construct
  source 1..120: mol_type = other DNA
ggctactgaaggtaataccctggtcagcattgacgtcaataatatcgccagtgaatacgatgctatccacctcgataacaagaactacaccacaggcgcagacaacggcacctcgaccat

SEQ ID NO: 3409 - DNA, 120 bp, synthetic construct
  source 1..120: mol_type = other DNA
tgctatccacctcgataacaagaactacaccacaggcgcagacaacggcacctcgaccattgatctgatcacccggggcgcgctggtttcgcagcagggctacggaattaatattgaaac

SEQ ID NO: 3410 - DNA, 120 bp, synthetic construct
  source 1..120: mol_type = other DNA
tgatctgatcacccggggcgcgctggtttcgcagcagggctacggaattaatattgaaaccaataccgcagacacctatgtcaccgtgggcggcttggtgcacggcggcaatggcaccgc

SEQ ID NO: 3411 - DNA, 120 bp, synthetic construct
  source 1..120: mol_type = other DNA
caataccgcagacacctatgtcaccgtgggcggcttggtgcacggcggcaatggcaccgcaatcggcattcatcggcttgataacattcaaacatcggccacgttagagctgcaatctgg

SEQ ID NO: 3412 - DNA, 120 bp, synthetic construct
  source 1..120: mol_type = other DNA
aatcggcattcatcggcttgataacattcaaacatcggccacgttagagctgcaatctggctatgcccttgaaggcgttacgcaggcactggtcttcaatggcagttatgcggagatcaa

SEQ ID NO: 3413 - DNA, 120 bp, synthetic construct
  source 1..120: mol_type = other DNA
ctatgcccttgaaggcgttacgcaggcactggtcttcaatggcagttatgcggagatcaatgatgccgcgctggatctggcaaacagccatctggtgctgggcggagcaggagacgccgc

SEQ ID NO: 3414 - DNA, 120 bp, synthetic construct
  source 1..120: mol_type = other DNA
tgatgccgcgctggatctggcaaacagccatctggtgctgggcggagcaggagacgccgctttcgatctcacgcgtattgataaccgtgaagaggccattctggatggcgacccgaaccg

SEQ ID NO: 3415 - DNA, 120 bp, synthetic construct
  source 1..120: mol_type = other DNA
tttcgatctcacgcgtattgataaccgtgaagaggccattctggatggcgacccgaaccggatcatcggcttcggtaccctgaccaaaaccaacaacagcatctggacgttaaccggcgc

SEQ ID NO: 3416 - DNA, 120 bp, synthetic construct
  source 1..120: mol_type = other DNA
gatcatcggcttcggtaccctgaccaaaaccaacaacagcatctggacgttaaccggcgccaatatggccgacggtgacgccaatgccttcctgtcggccaatatcgccggggggatttt

SEQ ID NO: 3417 - DNA, 120 bp, synthetic construct
  source 1..120: mol_type = other DNA
caatatggccgacggtgacgccaatgccttcctgtcggccaatatcgccggggggattttggtgctggataacgccacgctgggcctgacacctgacgctggggcactcactggagccac

SEQ ID NO: 3418 - DNA, 120 bp, synthetic construct
  source 1..120: mol_type = other DNA
ggtgctggataacgccacgctgggcctgacacctgacgctggggcactcactggagccacagtaaaccgcctcagtgctgccgatatcgccgctgacccgacgctagtggctaccgaaac

SEQ ID NO: 3419 - DNA, 120 bp, synthetic construct
  source 1..120: mol_type = other DNA
agtaaaccgcctcagtgctgccgatatcgccgctgacccgacgctagtggctaccgaaaccggtgcattaaccctggctgaaggcggggcgttgtcctcgctcggtgactcggttctgag

SEQ ID NO: 3420 - DNA, 120 bp, synthetic construct
  source 1..120: mol_type = other DNA
cggtgcattaaccctggctgaaggcggggcgttgtcctcgctcggtgactcggttctgagcggtaaccttatcagcgccggtgggatcctgctgtcaaaccactataccggcggcaatgg

SEQ ID NO: 3421 - DNA, 120 bp, synthetic construct
  source 1..120: mol_type = other DNA
cggtaaccttatcagcgccggtgggatcctgctgtcaaaccactataccggcggcaatggtgccgctaccgacgatcggctgaccgtgaccgggacttattttggtgaaaataacggttc

SEQ ID NO: 3422 - DNA, 120 bp, synthetic construct
  source 1..120: mol_type = other DNA
tgccgctaccgacgatcggctgaccgtgaccgggacttattttggtgaaaataacggttccggtgaaggggcctggctggcactcgatacggtgctgggggatgacgattctgccaccga

SEQ ID NO: 3423 - DNA, 120 bp, synthetic construct
  source 1..120: mol_type = other DNA
cggtgaaggggcctggctggcactcgatacggtgctgggggatgacgattctgccaccgaccggttagtgatcaacggcgatgccaccggcaccacctcggtccgggtgaacaatgcggg

SEQ ID NO: 3424 - DNA, 120 bp, synthetic construct
  source 1..120: mol_type = other DNA
ccggttagtgatcaacggcgatgccaccggcaccacctcggtccgggtgaacaatgcgggcggtctgggcgataaaaccctcaatggcatcaacctgatcaccgtggacggtctggcgca

SEQ ID NO: 3425 - DNA, 120 bp, synthetic construct
  source 1..120: mol_type = other DNA
cggtctgggcgataaaaccctcaatggcatcaacctgatcaccgtggacggtctggcgcaggatgacaccttcctactggccggggactatgtcaccacggatggctatcaggcggtggt

SEQ ID NO: 3426 - DNA, 120 bp, synthetic construct
  source 1..120: mol_type = other DNA
ggatgacaccttcctactggccggggactatgtcaccacggatggctatcaggcggtggtgggcggggcgtatgcctacaccttacaggccgacggggaagccgccactgcggggcgcaa

SEQ ID NO: 3427 - DNA, 120 bp, synthetic construct
  source 1..120: mol_type = other DNA
gggcggggcgtatgcctacaccttacaggccgacggggaagccgccactgcggggcgcaactggtatctctcttcagaactgatgttaaccgagggggtacgctatcaggcgggcgtgcc

SEQ ID NO: 3428 - DNA, 120 bp, synthetic construct
  source 1..120: mol_type = other DNA
ctggtatctctcttcagaactgatgttaaccgagggggtacgctatcaggcgggcgtgccgctgtatgaacaatatccgcaggtgctggccgccctgaataccctgccgacgctgcaaca

SEQ ID NO: 3429 - DNA, 120 bp, synthetic construct
  source 1..120: mol_type = other DNA
gctgtatgaacaatatccgcaggtgctggccgccctgaataccctgccgacgctgcaacagcgtgtcggtaaccgttacggggcgccgggcgcgctggcagacctggactttgacaataa

SEQ ID NO: 3430 - DNA, 120 bp, synthetic construct
  source 1..120: mol_type = other DNA
gcgtgtcggtaaccgttacggggcgccgggcgcgctggcagacctggactttgacaataatcaatgggcctggggccgtattgaagggagccaccaggtcaccgacccggcccgctccac

SEQ ID NO: 3431 - DNA, 120 bp, synthetic construct
  source 1..120: mol_type = other DNA
tcaatgggcctggggccgtattgaagggagccaccaggtcaccgacccggcccgctccaccagtggttcacaacgcgagattgatgtgtggaagttgcagaccggcattgatgtgccgct

SEQ ID NO: 3432 - DNA, 120 bp, synthetic construct
  source 1..120: mol_type = other DNA
cagtggttcacaacgcgagattgatgtgtggaagttgcagaccggcattgatgtgccgctgtatcagagccaggacggttcactgctgaccggcggggtaaacttctcctacggtaaagc

SEQ ID NO: 3433 - DNA, 120 bp, synthetic construct
  source 1..120: mol_type = other DNA
gtatcagagccaggacggttcactgctgaccggcggggtaaacttctcctacggtaaagccaaagcggatatccactcattctttggtgatggccgcatcaacagcgcaggttacggtct

SEQ ID NO: 3434 - DNA, 120 bp, synthetic construct
  source 1..120: mol_type = other DNA
caaagcggatatccactcattctttggtgatggccgcatcaacagcgcaggttacggtcttggcaccagcctgacctggtatggcaataacggcgtgtatgtggatggccagttgcagac

SEQ ID NO: 3435 - DNA, 120 bp, synthetic construct
  source 1..120: mol_type = other DNA
tggcaccagcctgacctggtatggcaataacggcgtgtatgtggatggccagttgcagacgatgtggtttgacagcgacctgagctcccgtaccgcagggcatgcagtggccagcggtaa

SEQ ID NO: 3436 - DNA, 120 bp, synthetic construct
  source 1..120: mol_type = other DNA
gatgtggtttgacagcgacctgagctcccgtaccgcagggcatgcagtggccagcggtaacaatggtcgcgggtatacctcggcgatagaagccggtaaaggttacgcactgggtaacgg

SEQ ID NO: 3437 - DNA, 120 bp, synthetic construct
  source 1..120: mol_type = other DNA
caatggtcgcgggtatacctcggcgatagaagccggtaaaggttacgcactgggtaacgggttgtcactgaccccgcagatgcaggtgacctactcgcgggtcgatttcgataccttccg

SEQ ID NO: 3438 - DNA, 120 bp, synthetic construct
  source 1..120: mol_type = other DNA
gttgtcactgaccccgcagatgcaggtgacctactcgcgggtcgatttcgataccttccgcgatccgtttgatagcgaagtttcgctgcaagagggtgacagcctgcggggccgcatcgg

SEQ ID NO: 3439 - DNA, 120 bp, synthetic construct
  source 1..120: mol_type = other DNA
cgatccgtttgatagcgaagtttcgctgcaagagggtgacagcctgcggggccgcatcggtgtctcactggataaggaaacgacctggagcgcgaaagacggcaccacccgccgctcaca

SEQ ID NO: 3440 - DNA, 120 bp, synthetic construct
  source 1..120: mol_type = other DNA
tgtctcactggataaggaaacgacctggagcgcgaaagacggcaccacccgccgctcacacatttacagtcatctcgatctgcacaatgagttcctcaatggcagtaaagtgcaggtctc

SEQ ID NO: 3441 - DNA, 120 bp, synthetic construct
  source 1..120: mol_type = other DNA
catttacagtcatctcgatctgcacaatgagttcctcaatggcagtaaagtgcaggtctcgggggtggagttcgccacccgggatgagcgtcagtcggtggggttaggcgcgggcggcac

SEQ ID NO: 3442 - DNA, 120 bp, synthetic construct
  source 1..120: mol_type = other DNA
gggggtggagttcgccacccgggatgagcgtcagtcggtggggttaggcgcgggcggcacctatgaatggcagaatggtcgctacgcggtttacggcaatgtcaatctgctgggggctac

SEQ ID NO: 3443 - DNA, 120 bp, synthetic construct
  source 1..120: mol_type = other DNA
ctatgaatggcagaatggtcgctacgcggtttacggcaatgtcaatctgctgggggctacacggaatgtcagtgacaactatgccgtcggcggtacgataggtgcacgggtgagctggta

SEQ ID NO: 3444 - DNA, 120 bp, synthetic construct
  source 1..120: mol_type = other DNA
acggaatgtcagtgacaactatgccgtcggcggtacgataggtgcacgggtgagctggtaatacaggacggttttgttatatcggggtatcagtgcgccgagtagggcactgataacgca

SEQ ID NO: 3445 - DNA, 120 bp, synthetic construct
  source 1..120: mol_type = other DNA
atacaggacggttttgttatatcggggtatcagtgcgccgagtagggcactgataacgcatttagtatacttaatattaggtcgtcataccgacggtgtgcagaagaaagtcgagttgct

SEQ ID NO: 3446 - DNA, 120 bp, synthetic construct
  source 1..120: mol_type = other DNA
tttagtatacttaatattaggtcgtcataccgacggtgtgcagaagaaagtcgagttgctgttgaaatcaatgacgaaatagccttgtttcagatctcatttataaaaaaatagttacag

SEQ ID NO: 3447 - DNA, 120 bp, synthetic construct
  source 1..120: mol_type = other DNA
gttgaaatcaatgacgaaatagccttgtttcagatctcatttataaaaaaatagttacagataaattgtaggaaaattcactcaatgaacttccaatattctttgtttaatttttatgat

SEQ ID NO: 3448 - DNA, 120 bp, synthetic construct
  source 1..120: mol_type = other DNA
ataaattgtaggaaaattcactcaatgaacttccaatattctttgtttaatttttatgatgtttataaaagcctttaataatgtgtgcttatattggctttgtaggaaatatcttacgta

SEQ ID NO: 3449 - DNA, 120 bp, synthetic construct
  source 1..120: mol_type = other DNA
gtttataaaagcctttaataatgtgtgcttatattggctttgtaggaaatatcttacgtatcaatatgatgaacggttgcttttgaattttcactgcttacatactgttacatttaaccc

SEQ ID NO: 3450 - DNA, 120 bp, synthetic construct
  source 1..120: mol_type = other DNA
tcaatatgatgaacggttgcttttgaattttcactgcttacatactgttacatttaacccattggtgttagctggctaacttttctacactgccgccggcgagtatttaattggtagatt

SEQ ID NO: 3451 - DNA, 120 bp, synthetic construct
  source 1..120: mol_type = other DNA
attggtgttagctggctaacttttctacactgccgccggcgagtatttaattggtagattaaggcgtgtgaaaaatacctgtcagatactgtttcatgctatccgatgaatggatagggt

SEQ ID NO: 3452 - DNA, 120 bp, synthetic construct
  source 1..120: mol_type = other DNA
aaggcgtgtgaaaaatacctgtcagatactgtttcatgctatccgatgaatggatagggttatctcatagagaattttttacttaataaacgctgagttggatacataatggagtattgg

SEQ ID NO: 3453 - DNA, 120 bp, synthetic construct
  source 1..120: mol_type = other DNA
tatctcatagagaattttttacttaataaacgctgagttggatacataatggagtattggctgttaatttttttacttatcttcttgtttgtcatctatatgcaaataagtgcgttatcc

SEQ ID NO: 3454 - DNA, 120 bp, synthetic construct
  source 1..120: mol_type = other DNA
ctgttaatttttttacttatcttcttgtttgtcatctatatgcaaataagtgcgttatccaactcggtaaaatatatacgagaagagataggcaggctgcgcaatgagcttgctccacgc

SEQ ID NO: 3455 - DNA, 120 bp, synthetic construct
  source 1..120: mol_type = other DNA
aactcggtaaaatatatacgagaagagataggcaggctgcgcaatgagcttgctccacgcttgcctgaacctaccgtggctactgttgtggccactgttaaggaagagatcacgccaacg

SEQ ID NO: 3456 - DNA, 120 bp, synthetic construct
  source 1..120: mol_type = other DNA
ttgcctgaacctaccgtggctactgttgtggccactgttaaggaagagatcacgccaacgaatttggcagatgatgtggccgcatccgaggtatggacccctgattacgcaacctatcag

SEQ ID NO: 3457 - DNA, 120 bp, synthetic construct
  source 1..120: mol_type = other DNA
aatttggcagatgatgtggccgcatccgaggtatggacccctgattacgcaacctatcagaattatctactcaccaaacagcaaagccagattaaagagatggctctagcctatgccgca

SEQ ID NO: 3458 - DNA, 120 bp, synthetic construct
  source 1..120: mol_type = other DNA
aattatctactcaccaaacagcaaagccagattaaagagatggctctagcctatgccgcaaaaaaagaacccgctcggccaatagaatataggattgctgaccgtcaggtggtgcttgag

SEQ ID NO: 3459 - DNA, 120 bp, synthetic construct
  source 1..120: mol_type = other DNA
aaaaaagaacccgctcggccaatagaatataggattgctgaccgtcaggtggtgcttgagccacaggatggggctcctcaagaatcgccgaaaatggatgcaggtcctgccagtggtcat

SEQ ID NO: 3460 - DNA, 120 bp, synthetic construct
  source 1..120: mol_type = other DNA
ccacaggatggggctcctcaagaatcgccgaaaatggatgcaggtcctgccagtggtcatccacagaaacccgatgtgtggacaaaattggaaaatgtcctgttttctttaaaatcaccg

SEQ ID NO: 3461 - DNA, 120 bp, synthetic construct
  source 1..120: mol_type = other DNA
ccacagaaacccgatgtgtggacaaaattggaaaatgtcctgttttctttaaaatcaccggagagtttctggaaacgcatcgagcaagagtttgccgcgcgttggatggtgtggatcggc

SEQ ID NO: 3462 - DNA, 120 bp, synthetic construct
  source 1..120: mol_type = other DNA
gagagtttctggaaacgcatcgagcaagagtttgccgcgcgttggatggtgtggatcggcggtatgatcatggcactgggtgtgattttcctgctgaaagcaggcagcgaacagggtctg

SEQ ID NO: 3463 - DNA, 120 bp, synthetic construct
  source 1..120: mol_type = other DNA
ggtatgatcatggcactgggtgtgattttcctgctgaaagcaggcagcgaacagggtctgttcgggccaaacttgcggattggtaccgccattgtgctgagtgtgctgatggttgttggg

SEQ ID NO: 3464 - DNA, 120 bp, synthetic construct
  source 1..120: mol_type = other DNA
ttcgggccaaacttgcggattggtaccgccattgtgctgagtgtgctgatggttgttgggggggagtggctcaggcgttcacgttttcagttgcccttggtcaatgccggttatatcccg

SEQ ID NO: 3465 - DNA, 120 bp, synthetic construct
  source 1..120: mol_type = other DNA
ggggagtggctcaggcgttcacgttttcagttgcccttggtcaatgccggttatatcccggcggcgctgagtggggccggtattctcggtctatttgcctcaatgctggcggctaaatat

SEQ ID NO: 3466 - DNA, 120 bp, synthetic construct
  source 1..120: mol_type = other DNA
gcggcgctgagtggggccggtattctcggtctatttgcctcaatgctggcggctaaatatctctacgacatgttcccgatgcccgttctcatgctgttgctcagcctgatttctctgttg

SEQ ID NO: 3467 - DNA, 120 bp, synthetic construct
  source 1..120: mol_type = other DNA
ctctacgacatgttcccgatgcccgttctcatgctgttgctcagcctgatttctctgttggcgatggtgctggcattgtggcaggggccatttatggcggccttggggctgcttggcgcc

SEQ ID NO: 3468 - DNA, 120 bp, synthetic construct
  source 1..120: mol_type = other DNA
gcgatggtgctggcattgtggcaggggccatttatggcggccttggggctgcttggcgcctataccgtcccgttatttgtttcgacgggcagcggtaatgtcaccgggctgttggcctac

SEQ ID NO: 3469 - DNA, 120 bp, synthetic construct
  source 1..120: mol_type = other DNA
tataccgtcccgttatttgtttcgacgggcagcggtaatgtcaccgggctgttggcctacctgttcctggttagtttggcgtctatcggcctgatgagccgtgtctatcggcactggcta

SEQ ID NO: 3470 - DNA, 120 bp, synthetic construct
  source 1..120: mol_type = other DNA
ctgttcctggttagtttggcgtctatcggcctgatgagccgtgtctatcggcactggctatggctgggggcgatggtcggaaactatctatggcttttggtttctttattcatagcaacg

SEQ ID NO: 3471 - DNA, 120 bp, synthetic construct
  source 1..120: mol_type = other DNA
tggctgggggcgatggtcggaaactatctatggcttttggtttctttattcatagcaacgtccgaacaccagttagcgcgttcactattcctgctagcaaccacatacggcttcctggcc

SEQ ID NO: 3472 - DNA, 120 bp, synthetic construct
  source 1..120: mol_type = other DNA
tccgaacaccagttagcgcgttcactattcctgctagcaaccacatacggcttcctggcctggccacatctggggtgggcgctaaaaagcaaaatacgttttcgccataatgactggaaa

SEQ ID NO: 3473 - DNA, 120 bp, synthetic construct
  source 1..120: mol_type = other DNA
tggccacatctggggtgggcgctaaaaagcaaaatacgttttcgccataatgactggaaaaactggcccccggctttgctggatccgttattaactgggttgattgccgggctttcgcta

SEQ ID NO: 3474 - DNA, 120 bp, synthetic construct
  source 1..120: mol_type = other DNA
aactggcccccggctttgctggatccgttattaactgggttgattgccgggctttcgctattagccttaacgttaagcgcaaatcattcgatcctggtctggagcacgttggtattctcc

SEQ ID NO: 3475 - DNA, 120 bp, synthetic construct
  source 1..120: mol_type = other DNA
ttagccttaacgttaagcgcaaatcattcgatcctggtctggagcacgttggtattctcctgtattagcctgttactgattgccagacgctcaccttcattggatttatttgttccactg

SEQ ID NO: 3476 - DNA, 120 bp, synthetic construct
  source 1..120: mol_type = other DNA
tgtattagcctgttactgattgccagacgctcaccttcattggatttatttgttccactggccgcgatattagccatttctccctttattaatgcaggaacgctgtttgagccagaaacc

SEQ ID NO: 3477 - DNA, 120 bp, synthetic construct
  source 1..120: mol_type = other DNA
gccgcgatattagccatttctccctttattaatgcaggaacgctgtttgagccagaaaccgtctggacgagtttgctcgcgctcagcacattagcgctattctgcgggatatatggtagc

SEQ ID NO: 3478 - DNA, 120 bp, synthetic construct
  source 1..120: mol_type = other DNA
gtctggacgagtttgctcgcgctcagcacattagcgctattctgcgggatatatggtagctaccaggtcacccggccggtttaccgcaagctgtggtgggcgttattgtcggtgctggtg

SEQ ID NO: 3479 - DNA, 120 bp, synthetic construct
  source 1..120: mol_type = other DNA
taccaggtcacccggccggtttaccgcaagctgtggtgggcgttattgtcggtgctggtgccaatgtatctcgttgcaagtacctattatgcctgtcgcgataattttgagctggctcca

SEQ ID NO: 3480 - DNA, 120 bp, synthetic construct
  source 1..120: mol_type = other DNA
ccaatgtatctcgttgcaagtacctattatgcctgtcgcgataattttgagctggctccagttaaatacacactgctggcggtttgtctggctatgtatatcgcgtggaatgcattcagt

SEQ ID NO: 3481 - DNA, 120 bp, synthetic construct
  source 1..120: mol_type = other DNA
gttaaatacacactgctggcggtttgtctggctatgtatatcgcgtggaatgcattcagtgatgggtatcgccgtggctcagcgctgttgcggacgatctatcaggtcgccgcccaactg

SEQ ID NO: 3482 - DNA, 120 bp, synthetic construct
  source 1..120: mol_type = other DNA
gatgggtatcgccgtggctcagcgctgttgcggacgatctatcaggtcgccgcccaactgacgttgacctttgcattatttatggctttcagccaggttacgctaaccctgctgctcgcg

SEQ ID NO: 3483 - DNA, 120 bp, synthetic construct
  source 1..120: mol_type = other DNA
acgttgacctttgcattatttatggctttcagccaggttacgctaaccctgctgctcgcgggtcagcttttagttttggtactctggcaacgttggcgacaggtttcgttactgtcttgg

SEQ ID NO: 3484 - DNA, 120 bp, synthetic construct
  source 1..120: mol_type = other DNA
ggtcagcttttagttttggtactctggcaacgttggcgacaggtttcgttactgtcttggattttgaaactgcatgcgatcatactgctggttcgtctgtcaatgaacccgtatatcctt

SEQ ID NO: 3485 - DNA, 120 bp, synthetic construct
  source 1..120: mol_type = other DNA
attttgaaactgcatgcgatcatactgctggttcgtctgtcaatgaacccgtatatccttggatattcctcgccgttgcacattggttcggtcgttattccttggacgctatacggtttt

SEQ ID NO: 3486 - DNA, 120 bp, synthetic construct
  source 1..120: mol_type = other DNA
ggatattcctcgccgttgcacattggttcggtcgttattccttggacgctatacggttttgggattccgattctctgcctgtggctaagttcacgctggttacctgcgcgtcgcggtgag

SEQ ID NO: 3487 - DNA, 120 bp, synthetic construct
  source 1..120: mol_type = other DNA
gggattccgattctctgcctgtggctaagttcacgctggttacctgcgcgtcgcggtgagcagaccgccaattggttagcggccaatgctatttatctgttggccttgtggatcaacgtt

SEQ ID NO: 3488 - DNA, 120 bp, synthetic construct
  source 1..120: mol_type = other DNA
cagaccgccaattggttagcggccaatgctatttatctgttggccttgtggatcaacgttgaattacgtcacctgctgcatggcagctatcatctgtcgctggatttcgcttctcttacc

SEQ ID NO: 3489 - DNA, 120 bp, synthetic construct
  source 1..120: mol_type = other DNA
gaattacgtcacctgctgcatggcagctatcatctgtcgctggatttcgcttctcttaccgattgtgcgttgcatggggtgaccttcgggctgatggcgctggcctacggctatcgtgaa

SEQ ID NO: 3490 - DNA, 120 bp, synthetic construct
  source 1..120: mol_type = other DNA
gattgtgcgttgcatggggtgaccttcgggctgatggcgctggcctacggctatcgtgaacagtttgcagattcgctacaacggatataccgcctggcggctaaaaccagtgccattctg

SEQ ID NO: 3491 - DNA, 120 bp, synthetic construct
  source 1..120: mol_type = other DNA
cagtttgcagattcgctacaacggatataccgcctggcggctaaaaccagtgccattctgatgctcaccctaacgttgctctgcctggttgtctttaaccccatctggtcagcacaacag

SEQ ID NO: 3492 - DNA, 120 bp, synthetic construct
  source 1..120: mol_type = other DNA
atgctcaccctaacgttgctctgcctggttgtctttaaccccatctggtcagcacaacaggttggcggcctaccgctgctgaatatggtgaccgttgcctatgcgatcccgatggtgttc

SEQ ID NO: 3493 - DNA, 120 bp, synthetic construct
  source 1..120: mol_type = other DNA
gttggcggcctaccgctgctgaatatggtgaccgttgcctatgcgatcccgatggtgttcatggtggtagcactaagatactggccagatcactggctagatatccgtctgaagccctac

SEQ ID NO: 3494 - DNA, 120 bp, synthetic construct
  source 1..120: mol_type = other DNA
atggtggtagcactaagatactggccagatcactggctagatatccgtctgaagccctacgttatcggtgcgattgcgctactgggaatggtgttcattaccttgacggtccgccagctc

SEQ ID NO: 3495 - DNA, 120 bp, synthetic construct
  source 1..120: mol_type = other DNA
gttatcggtgcgattgcgctactgggaatggtgttcattaccttgacggtccgccagctctggcatggtgaccggttggataatgatatcgtgtacagcggcgaacaatactcttactcc

SEQ ID NO: 3496 - DNA, 120 bp, synthetic construct
  source 1..120: mol_type = other DNA
tggcatggtgaccggttggataatgatatcgtgtacagcggcgaacaatactcttactccttagcgtggatgttaactgccattggcatgatgtacagcgcaatacactggcctaactat

SEQ ID NO: 3497 - DNA, 120 bp, synthetic construct
  source 1..120: mol_type = other DNA
ttagcgtggatgttaactgccattggcatgatgtacagcgcaatacactggcctaactataaagtgcgccgcgcctccctggggttgttggcgctcacgatcgtcaaactgttcctgtgg

SEQ ID NO: 3498 - DNA, 120 bp, synthetic construct
  source 1..120: mol_type = other DNA
aaagtgcgccgcgcctccctggggttgttggcgctcacgatcgtcaaactgttcctgtgggatatgtctggtcttgaagggctatatcgttcggtctcattcctcggtctggggctgtgt

SEQ ID NO: 3499 - DNA, 120 bp, synthetic construct
  source 1..120: mol_type = other DNA
gatatgtctggtcttgaagggctatatcgttcggtctcattcctcggtctggggctgtgtctggtagcgattggttggttctaccagaagtttgtcgttatgaaggaagtcattgagcaa

SEQ ID NO: 3500 - DNA, 120 bp, synthetic construct
  source 1..120: mol_type = other DNA
ctggtagcgattggttggttctaccagaagtttgtcgttatgaaggaagtcattgagcaaaacaaggatcagccgacagcggacgtggtacaaagcgggcaataatcgccatttgtctta

SEQ ID NO: 3501 - DNA, 120 bp, synthetic construct
  source 1..120: mol_type = other DNA
aacaaggatcagccgacagcggacgtggtacaaagcgggcaataatcgccatttgtcttaccggagcgtgcatcgactgatgtgggaaaatcaatatacagcaaggagtcagtgtgatta

SEQ ID NO: 3502 - DNA, 120 bp, synthetic construct
  source 1..120: mol_type = other DNA
ccggagcgtgcatcgactgatgtgggaaaatcaatatacagcaaggagtcagtgtgattaattttgtgaagttaatgtgtaatgtgaagttaatgtgtaaatggggggcgatattgatgt

SEQ ID NO: 3503 - DNA, 120 bp, synthetic construct
  source 1..120: mol_type = other DNA
attttgtgaagttaatgtgtaatgtgaagttaatgtgtaaatggggggcgatattgatgtcacccttctttctttctgcttgcgtaactaaccagctttcagatgatatccggggccatg

SEQ ID NO: 3504 - DNA, 120 bp, synthetic construct
  source 1..120: mol_type = other DNA
cacccttctttctttctgcttgcgtaactaaccagctttcagatgatatccggggccatgagaaaggctacacgcattataatgatgatattattgtcggcgtgtctttggctaagcagg

SEQ ID NO: 3505 - DNA, 120 bp, synthetic construct
  source 1..120: mol_type = other DNA
agaaaggctacacgcattataatgatgatattattgtcggcgtgtctttggctaagcagggtgataataaaaactgggcatttgtcggtacgcatttcgattatgtgttgtcatcgggag

SEQ ID NO: 3506 - DNA, 120 bp, synthetic construct
  source 1..120: mol_type = other DNA
gtgataataaaaactgggcatttgtcggtacgcatttcgattatgtgttgtcatcgggagccgacgagttcttaacgctattagttaccgggcagattgataaaaagaagattgaggtag

SEQ ID NO: 3507 - DNA, 120 bp, synthetic construct
  source 1..120: mol_type = other DNA
ccgacgagttcttaacgctattagttaccgggcagattgataaaaagaagattgaggtagtcagggacggtagctttaatcttaataagaaaaaggatggcttcacagggaaaatcgctc

SEQ ID NO: 3508 - DNA, 120 bp, synthetic construct
  source 1..120: mol_type = other DNA
tcagggacggtagctttaatcttaataagaaaaaggatggcttcacagggaaaatcgctctgaaatatcgttatcagacggcggaagagcgaggcaaaatagagccgctgataaaagggg

SEQ ID NO: 3509 - DNA, 120 bp, synthetic construct
  source 1..120: mol_type = other DNA
tgaaatatcgttatcagacggcggaagagcgaggcaaaatagagccgctgataaaaggggctgattggaattgtccaagcctcacggaaacaacgggtatttgcaatattaacctgaata

SEQ ID NO: 3510 - DNA, 120 bp, synthetic construct
  source 1..120: mol_type = other DNA
ctgattggaattgtccaagcctcacggaaacaacgggtatttgcaatattaacctgaataatctggtcggcactattcacagaaaaggtgctacaccggccgatatcttccgttttgaac

SEQ ID NO: 3511 - DNA, 120 bp, synthetic construct
  source 1..120: mol_type = other DNA
atctggtcggcactattcacagaaaaggtgctacaccggccgatatcttccgttttgaacatcctttgcaagtgaagttttatagtaaaaatacgacctcagctaagagggcgctttacc

SEQ ID NO: 3512 - DNA, 120 bp, synthetic construct
  source 1..120: mol_type = other DNA
atcctttgcaagtgaagttttatagtaaaaatacgacctcagctaagagggcgctttacccggtggccgtagcggcagatgtcgtgatgttgcccgtgtatctattgagtgctgctgccg

SEQ ID NO: 3513 - DNA, 120 bp, synthetic construct
  source 1..120: mol_type = other DNA
cggtggccgtagcggcagatgtcgtgatgttgcccgtgtatctattgagtgctgctgccgtggccgctttctatggtgtggtctcattgaattagtcgttctttttaaacccggctaaca

SEQ ID NO: 3514 - DNA, 120 bp, synthetic construct
  source 1..120: mol_type = other DNA
tggccgctttctatggtgtggtctcattgaattagtcgttctttttaaacccggctaacaaaatagagaggggtagcctaccgggcattaaacacaacagtgtccggtatcgcccaataa

SEQ ID NO: 3515 - DNA, 120 bp, synthetic construct
  source 1..120: mol_type = other DNA
aaatagagaggggtagcctaccgggcattaaacacaacagtgtccggtatcgcccaataataatgtttggccggtaaatgttaacacttggtttcaccccgttaaaataatcctccccac

SEQ ID NO: 3516 - DNA, 120 bp, synthetic construct
  source 1..120: mol_type = other DNA
taatgtttggccggtaaatgttaacacttggtttcaccccgttaaaataatcctccccacggtaaagttcccctttttagtgccgataacacacttaattaaacgtctttgtgttttgac

SEQ ID NO: 3517 - DNA, 120 bp, synthetic construct
  source 1..120: mol_type = other DNA
ggtaaagttcccctttttagtgccgataacacacttaattaaacgtctttgtgttttgacgtgtctgtgttttgtcgtactgatgaagggttaatatgttcaagcgtatgaaagtggtta

SEQ ID NO: 3518 - DNA, 120 bp, synthetic construct
  source 1..120: mol_type = other DNA
gtgtctgtgttttgtcgtactgatgaagggttaatatgttcaagcgtatgaaagtggttaccagcctgctgctggtattagtattatttggtgccttacaactggtatccggcgggcttt

SEQ ID NO: 3519 - DNA, 120 bp, synthetic construct
  source 1..120: mol_type = other DNA
ccagcctgctgctggtattagtattatttggtgccttacaactggtatccggcgggctttttttcaaatcattgcagaatgaccaggaaaacttcaacgttttacaagttattcgccagc

SEQ ID NO: 3520 - DNA, 120 bp, synthetic construct
  source 1..120: mol_type = other DNA
ttttcaaatcattgcagaatgaccaggaaaacttcaacgttttacaagttattcgccagcaacaatcggtattgaatgaaagctgggtctatctgttacaaacacgcaatacgttaaacc

SEQ ID NO: 3521 - DNA, 120 bp, synthetic construct
  source 1..120: mol_type = other DNA
aacaatcggtattgaatgaaagctgggtctatctgttacaaacacgcaatacgttaaaccgtgccggtgttcgttacatgatggatattaaccatactggcagtggccctacggtgaagg

SEQ ID NO: 3522 - DNA, 120 bp, synthetic construct
  source 1..120: mol_type = other DNA
gtgccggtgttcgttacatgatggatattaaccatactggcagtggccctacggtgaaggaccttatctcttcggctaaagggacgctaagcgtcgcggaagaccgcttcaaacgttacg

SEQ ID NO: 3523 - DNA, 120 bp, synthetic construct
  source 1..120: mol_type = other DNA
accttatctcttcggctaaagggacgctaagcgtcgcggaagaccgcttcaaacgttacgaaaaaatcccacaaaatagcagtcaggatccagaaggcgccaaaaaattaaaacagtcct

SEQ ID NO: 3524 - DNA, 120 bp, synthetic construct
  source 1..120: mol_type = other DNA
aaaaaatcccacaaaatagcagtcaggatccagaaggcgccaaaaaattaaaacagtcctacgaggaatattttagtgccttaaccgaactgattaatttgatggaaacgaacaaaatca

SEQ ID NO: 3525 - DNA, 120 bp, synthetic construct
  source 1..120: mol_type = other DNA
acgaggaatattttagtgccttaaccgaactgattaatttgatggaaacgaacaaaatcaatgagttcttcaatcaccccaccaccagtttccaaaatgaatttgagcaaaattacaaca

SEQ ID NO: 3526 - DNA, 120 bp, synthetic construct
  source 1..120: mol_type = other DNA
atgagttcttcaatcaccccaccaccagtttccaaaatgaatttgagcaaaattacaacaactatctgacgcaaaatgacggactgtatgattcggcggtcgaggacagtaatcaatcct

SEQ ID NO: 3527 - DNA, 120 bp, synthetic construct
  source 1..120: mol_type = other DNA
actatctgacgcaaaatgacggactgtatgattcggcggtcgaggacagtaatcaatcctttagctttgctatgggcgtggttattactgtactggtcgtcgtattagtgatgatgctcc

SEQ ID NO: 3528 - DNA, 120 bp, synthetic construct
  source 1..120: mol_type = other DNA
ttagctttgctatgggcgtggttattactgtactggtcgtcgtattagtgatgatgctccttgtctggctggggatgcaacagatcttaattcaccccctcaaccacctgattgcacaca

SEQ ID NO: 3529 - DNA, 120 bp, synthetic construct
  source 1..120: mol_type = other DNA
ttgtctggctggggatgcaacagatcttaattcaccccctcaaccacctgattgcacacattaaacatattgccaacggtgatttgacgcaaaatattgaagttcatggtcgcaacgaag

SEQ ID NO: 3530 - DNA, 120 bp, synthetic construct
  source 1..120: mol_type = other DNA
ttaaacatattgccaacggtgatttgacgcaaaatattgaagttcatggtcgcaacgaagtgggcacgttggctgctagcctgaaacacatgcaatctgaattggtcactatcgtcggcg

SEQ ID NO: 3531 - DNA, 120 bp, synthetic construct
  source 1..120: mol_type = other DNA
tgggcacgttggctgctagcctgaaacacatgcaatctgaattggtcactatcgtcggcgaggtgcgtgtaggcgctgatgctatctacagcggtgcgtcagaaattgcggtgggtaaca

SEQ ID NO: 3532 - DNA, 120 bp, synthetic construct
  source 1..120: mol_type = other DNA
aggtgcgtgtaggcgctgatgctatctacagcggtgcgtcagaaattgcggtgggtaacaatgatttatccgcccgtactgaacagcaagcggcatcattggaagaaacggctgccagca

SEQ ID NO: 3533 - DNA, 120 bp, synthetic construct
  source 1..120: mol_type = other DNA
atgatttatccgcccgtactgaacagcaagcggcatcattggaagaaacggctgccagcatggagcaattaaccgcaacggtgaaacagaacgctgaaaacgcccgtcaggcgagtcaat

SEQ ID NO: 3534 - DNA, 120 bp, synthetic construct
  source 1..120: mol_type = other DNA
tggagcaattaaccgcaacggtgaaacagaacgctgaaaacgcccgtcaggcgagtcaattagcattgagtgcctcagaaaccgctcagaaaggggggaaagtggtggcggatgttgtgc

SEQ ID NO: 3535 - DNA, 120 bp, synthetic construct
  source 1..120: mol_type = other DNA
tagcattgagtgcctcagaaaccgctcagaaaggggggaaagtggtggcggatgttgtgcaaaccatgcacgagatcgcggggagttcgcagaagattgccgacattaccagcgtcatcg

SEQ ID NO: 3536 - DNA, 120 bp, synthetic construct
  source 1..120: mol_type = other DNA
aaaccatgcacgagatcgcggggagttcgcagaagattgccgacattaccagcgtcatcgacggtatcgccttccagaccaatatcttggcattgaatgccgccgttgaagccgcccgtg

SEQ ID NO: 3537 - DNA, 120 bp, synthetic construct
  source 1..120: mol_type = other DNA
acggtatcgccttccagaccaatatcttggcattgaatgccgccgttgaagccgcccgtgcaggtgagcaaggccgtggttttgccgtggttgccggtgaagtgcgcaatttagcacaac

SEQ ID NO: 3538 - DNA, 120 bp, synthetic construct
  source 1..120: mol_type = other DNA
caggtgagcaaggccgtggttttgccgtggttgccggtgaagtgcgcaatttagcacaacgcagtgcacaggcggcgaaggaaattaaaggtctgattgacgattcggttaaccgggtag

SEQ ID NO: 3539 - DNA, 120 bp, synthetic construct
  source 1..120: mol_type = other DNA
gcagtgcacaggcggcgaaggaaattaaaggtctgattgacgattcggttaaccgggtagatctgggctcagtactggttgaaagtgccggtgaaaccatgggcgatatcgttaatgccg

SEQ ID NO: 3540 - DNA, 120 bp, synthetic construct
  source 1..120: mol_type = other DNA
atctgggctcagtactggttgaaagtgccggtgaaaccatgggcgatatcgttaatgccgtgacccgcgtgaccgacatcatgggcgaaatcgcttctgcctcagatgaacaaagtcgtg

SEQ ID NO: 3541 - DNA, 120 bp, synthetic construct
  source 1..120: mol_type = other DNA
tgacccgcgtgaccgacatcatgggcgaaatcgcttctgcctcagatgaacaaagtcgtggtattgaccagattggtcaggcagttgccgaaatggaccgcgtgacacagcaaaatgctt

SEQ ID NO: 3542 - DNA, 120 bp, synthetic construct
  source 1..120: mol_type = other DNA
gtattgaccagattggtcaggcagttgccgaaatggaccgcgtgacacagcaaaatgcttccttggtagaagaatcggcttccgccgccgcttcactggaagagcaagccagcatgttaa

SEQ ID NO: 3543 - DNA, 120 bp, synthetic construct
  source 1..120: mol_type = other DNA
ccttggtagaagaatcggcttccgccgccgcttcactggaagagcaagccagcatgttaactcaagcgatgtccgtatttgttctgagtgtggataacagtaattccactagcgacgtca

SEQ ID NO: 3544 - DNA, 120 bp, synthetic construct
  source 1..120: mol_type = other DNA
ctcaagcgatgtccgtatttgttctgagtgtggataacagtaattccactagcgacgtcagaaaagtcaaacaacccacgcaggaaatgaacagcacggctaaaaaagcgctgggaaata

SEQ ID NO: 3545 - DNA, 120 bp, synthetic construct
  source 1..120: mol_type = other DNA
gaaaagtcaaacaacccacgcaggaaatgaacagcacggctaaaaaagcgctgggaaataatctgcaagacaattgggaaactttctagacctataaccttcgagcttgacgctgttgac

SEQ ID NO: 3546 - DNA, 120 bp, synthetic construct
  source 1..120: mol_type = other DNA
atctgcaagacaattgggaaactttctagacctataaccttcgagcttgacgctgttgacgtgttagctgcgcgcactcatccgaatcacaaacttgagtcagcacatcgggatccgcct

SEQ ID NO: 3547 - DNA, 120 bp, synthetic construct
  source 1..120: mol_type = other DNA
gtgttagctgcgcgcactcatccgaatcacaaacttgagtcagcacatcgggatccgcctgctggccatttacctgccacgccaattgatttgggtgtatgcaaaataatattaataaag

SEQ ID NO: 3548 - DNA, 120 bp, synthetic construct
  source 1..120: mol_type = other DNA
gctggccatttacctgccacgccaattgatttgggtgtatgcaaaataatattaataaagtcggcctatgagccggctgagaagaggttacgatgtttggtcaaatccggatttctacca

SEQ ID NO: 3549 - DNA, 120 bp, synthetic construct
  source 1..120: mol_type = other DNA
tcggcctatgagccggctgagaagaggttacgatgtttggtcaaatccggatttctaccagttttttcctgctgctgatgtttctttgcgccatacagttaatttcaagtggtctatcat

SEQ ID NO: 3550 - DNA, 120 bp, synthetic construct
  source 1..120: mol_type = other DNA
gttttttcctgctgctgatgtttctttgcgccatacagttaatttcaagtggtctatcatttacggcttttcgctcagactaccaaaatttaaatcgagtggagttaagtagtcagcaac

SEQ ID NO: 3551 - DNA, 120 bp, synthetic construct
  source 1..120: mol_type = other DNA
ttacggcttttcgctcagactaccaaaatttaaatcgagtggagttaagtagtcagcaacgcgatgcattaagcctcagttgggtatctttgcttcaggcacgtaataccttaaaccgtg

SEQ ID NO: 3552 - DNA, 120 bp, synthetic construct
  source 1..120: mol_type = other DNA
gcgatgcattaagcctcagttgggtatctttgcttcaggcacgtaataccttaaaccgtgcggctactcgctcggcgctcaatgttcctcaggagcaagttaacgctttaatggggagtg

SEQ ID NO: 3553 - DNA, 120 bp, synthetic construct
  source 1..120: mol_type = other DNA
cggctactcgctcggcgctcaatgttcctcaggagcaagttaacgctttaatggggagtgcgcgcagtgcattgcagaaagctgaactttactttaatcagtttcaggcggtaccgcgcc

SEQ ID NO: 3554 - DNA, 120 bp, synthetic construct
  source 1..120: mol_type = other DNA
cgcgcagtgcattgcagaaagctgaactttactttaatcagtttcaggcggtaccgcgccttgatgagagtgagagcagtgggcaattactggatgcgaccaaaaacagttatcaaaacc

SEQ ID NO: 3555 - DNA, 120 bp, synthetic construct
  source 1..120: mol_type = other DNA
ttgatgagagtgagagcagtgggcaattactggatgcgaccaaaaacagttatcaaaaccttcgtagcgcattacgtgagttaattgattttctggaagcgggtgatttacaagcattta

SEQ ID NO: 3556 - DNA, 120 bp, synthetic construct
  source 1..120: mol_type = other DNA
ttcgtagcgcattacgtgagttaattgattttctggaagcgggtgatttacaagcatttatggatcaacccactcagaaaacgcaagatttgtttgaagcggatttcatccagtatttgc

SEQ ID NO: 3557 - DNA, 120 bp, synthetic construct
  source 1..120: mol_type = other DNA
tggatcaacccactcagaaaacgcaagatttgtttgaagcggatttcatccagtatttgcaatacgccaatgaggttattgccgatgccggtcagcagaatcagcaggcttatcagctct

SEQ ID NO: 3558 - DNA, 120 bp, synthetic construct
  source 1..120: mol_type = other DNA
aatacgccaatgaggttattgccgatgccggtcagcagaatcagcaggcttatcagctctcaatctggatatttagtggtgcgattctgatggttatcacgatggccatttcgtcgttga

SEQ ID NO: 3559 - DNA, 120 bp, synthetic construct
  source 1..120: mol_type = other DNA
caatctggatatttagtggtgcgattctgatggttatcacgatggccatttcgtcgttgatctggttgcgcaacatgtttgttcggccattagcgacgatgcgtgagcattttggccgca

SEQ ID NO: 3560 - DNA, 120 bp, synthetic construct
  source 1..120: mol_type = other DNA
tctggttgcgcaacatgtttgttcggccattagcgacgatgcgtgagcattttggccgcattgctcaaggggatttgtctgggcagatctcggtgactggccgtaatgaaatcagccaga

SEQ ID NO: 3561 - DNA, 120 bp, synthetic construct
  source 1..120: mol_type = other DNA
ttgctcaaggggatttgtctgggcagatctcggtgactggccgtaatgaaatcagccagatgttcgccagcttacgcaccatgcagcagtcgctgatctcaacggtcagcaatgtgcgtg

SEQ ID NO: 3562 - DNA, 120 bp, synthetic construct
  source 1..120: mol_type = other DNA
tgttcgccagcttacgcaccatgcagcagtcgctgatctcaacggtcagcaatgtgcgtgagggtaccgaatcgatgttgaccggtatccaggaaatttccgcaggtaacaacgatttat

SEQ ID NO: 3563 - DNA, 120 bp, synthetic construct
  source 1..120: mol_type = other DNA
agggtaccgaatcgatgttgaccggtatccaggaaatttccgcaggtaacaacgatttatcggcaagaactgaacagcaagcggcttccttggaacaaactgccgcgagtatggaacaac

SEQ ID NO: 3564 - DNA, 120 bp, synthetic construct
  source 1..120: mol_type = other DNA
cggcaagaactgaacagcaagcggcttccttggaacaaactgccgcgagtatggaacaactgaccgccacggtaaaacagaatgcggacaatgcgcatcaggccacggtactggcgcaag

SEQ ID NO: 3565 - DNA, 120 bp, synthetic construct
  source 1..120: mol_type = other DNA
tgaccgccacggtaaaacagaatgcggacaatgcgcatcaggccacggtactggcgcaagaggcttccggtacggcagctaaaggcggagaactgacggcgagtgtcgtcaccaccatgc

SEQ ID NO: 3566 - DNA, 120 bp, synthetic construct
  source 1..120: mol_type = other DNA
aggcttccggtacggcagctaaaggcggagaactgacggcgagtgtcgtcaccaccatgcatgcaatcgctaccagttcgcagaagattggtgcgatcaccagcgttatcgacggtattg

SEQ ID NO: 3567 - DNA, 120 bp, synthetic construct
  source 1..120: mol_type = other DNA
atgcaatcgctaccagttcgcagaagattggtgcgatcaccagcgttatcgacggtattgccttccaaaccaatattttggcactgaatgcggccgtggaggcggcccgtgcgggtgagc

SEQ ID NO: 3568 - DNA, 120 bp, synthetic construct
  source 1..120: mol_type = other DNA
ccttccaaaccaatattttggcactgaatgcggccgtggaggcggcccgtgcgggtgagcaagggcgtggttttgcggtggttgcgggtgaagtccgtaatttagcataacgcagtgcgc

SEQ ID NO: 3569 - DNA, 120 bp, synthetic construct
  source 1..120: mol_type = other DNA
aagggcgtggttttgcggtggttgcgggtgaagtccgtaatttagcataacgcagtgcgcaagcggccaaagagatcaaagggctgattgatgagtccgtcagccgtgtccgccaggggt

SEQ ID NO: 3570 - DNA, 120 bp, synthetic construct
  source 1..120: mol_type = other DNA
aagcggccaaagagatcaaagggctgattgatgagtccgtcagccgtgtccgccaggggtctacgctggtcgaaagtgcaggaactaccatggaagagatcgtccgctcggtggcgcgtg

SEQ ID NO: 3571 - DNA, 120 bp, synthetic construct
  source 1..120: mol_type = other DNA
ctacgctggtcgaaagtgcaggaactaccatggaagagatcgtccgctcggtggcgcgtgtgactgacattatgggggagatcgaatctgcttcggatgaacagagccggggtattgaac

SEQ ID NO: 3572 - DNA, 120 bp, synthetic construct
  source 1..120: mol_type = other DNA
tgactgacattatgggggagatcgaatctgcttcggatgaacagagccggggtattgaacaaatatcactcgccgtaacgcaaatggatcaggttactcagcaaaatgcgtcattagtgg

SEQ ID NO: 3573 - DNA, 120 bp, synthetic construct
  source 1..120: mol_type = other DNA
aaatatcactcgccgtaacgcaaatggatcaggttactcagcaaaatgcgtcattagtggaagaggccgcggcggcagccaatgcactggaagagcaggccagcatgctctccgatgccg

SEQ ID NO: 3574 - DNA, 120 bp, synthetic construct
  source 1..120: mol_type = other DNA
aagaggccgcggcggcagccaatgcactggaagagcaggccagcatgctctccgatgccgtctctgttttccgtttggggcaggggcacgacgaacagtcagttgcgggcaatagccagc

SEQ ID NO: 3575 - DNA, 120 bp, synthetic construct
  source 1..120: mol_type = other DNA
tctctgttttccgtttggggcaggggcacgacgaacagtcagttgcgggcaatagccagcaatcattggccacgcattattagtcgctcattatgggtcgatcagcatgagtggttccga

SEQ ID NO: 3576 - DNA, 120 bp, synthetic construct
  source 1..120: mol_type = other DNA
aatcattggccacgcattattagtcgctcattatgggtcgatcagcatgagtggttccgaccaggagtgacaatcgatcatcactcgtaacgggtcatcacgagtaacgacaagtggctg

SEQ ID NO: 3577 - DNA, 120 bp, synthetic construct
  source 1..120: mol_type = other DNA
ccaggagtgacaatcgatcatcactcgtaacgggtcatcacgagtaacgacaagtggctgtaaaggaaatcgtagagtgtcaaacagcgtaacgaagacggtattggggggtaaggttgg

SEQ ID NO: 3578 - DNA, 120 bp, synthetic construct
  source 1..120: mol_type = other DNA
taaaggaaatcgtagagtgtcaaacagcgtaacgaagacggtattggggggtaaggttggatgaaacgatcatcaatgaagtcagcgcctcaatcattacctcaagagtccgggtcgata

SEQ ID NO: 3579 - DNA, 120 bp, synthetic construct
  source 1..120: mol_type = other DNA
atgaaacgatcatcaatgaagtcagcgcctcaatcattacctcaagagtccgggtcgatactgacccaaatgattcaacggttgccgctgtcggatattcacttccggcgtatctgtcaa

SEQ ID NO: 3580 - DNA, 120 bp, synthetic construct
  source 1..120: mol_type = other DNA
ctgacccaaatgattcaacggttgccgctgtcggatattcacttccggcgtatctgtcaacttatctatcaacgggctggaattgttctggctgaacataagcgggaaatggtctataac

SEQ ID NO: 3581 - DNA, 120 bp, synthetic construct
  source 1..120: mol_type = other DNA
cttatctatcaacgggctggaattgttctggctgaacataagcgggaaatggtctataaccgcctggtcagacggttgagattactgaatatctctgattttggtcagtatctggccttg

SEQ ID NO: 3582 - DNA, 120 bp, synthetic construct
  source 1..120: mol_type = other DNA
cgcctggtcagacggttgagattactgaatatctctgattttggtcagtatctggccttgttggagagtgatccgaacagtgctgagtggcaggcatttgtgaatgcgttgaccactaac

SEQ ID NO: 3583 - DNA, 120 bp, synthetic construct
  source 1..120: mol_type = other DNA
ttggagagtgatccgaacagtgctgagtggcaggcatttgtgaatgcgttgaccactaacctgacggcattttttcgtgaggctcatcattttccgctcttggcagaacatgctcgtcag

SEQ ID NO: 3584 - DNA, 120 bp, synthetic construct
  source 1..120: mol_type = other DNA
ctgacggcattttttcgtgaggctcatcattttccgctcttggcagaacatgctcgtcagcgggcgggcggttattcagtctggagtacggcggcatcaaccggtgaagaaccttactcc

SEQ ID NO: 3585 - DNA, 120 bp, synthetic construct
  source 1..120: mol_type = other DNA
cgggcgggcggttattcagtctggagtacggcggcatcaaccggtgaagaaccttactccatcgctatgacgctgtgtgatgtgttaggaaatcgcgcgggagcctgccagatattggcc

SEQ ID NO: 3586 - DNA, 120 bp, synthetic construct
  source 1..120: mol_type = other DNA
atcgctatgacgctgtgtgatgtgttaggaaatcgcgcgggagcctgccagatattggccagcgatatcgatacacaggtactggagaaagctaccagcggtgtatatcggcaagatgaa

SEQ ID NO: 3587 - DNA, 120 bp, synthetic construct
  source 1..120: mol_type = other DNA
agcgatatcgatacacaggtactggagaaagctaccagcggtgtatatcggcaagatgaattgcgctcattgtcaacccagcagatgcaacgctactttttgcgaggtacgggcccgcat

SEQ ID NO: 3588 - DNA, 120 bp, synthetic construct
  source 1..120: mol_type = other DNA
ttgcgctcattgtcaacccagcagatgcaacgctactttttgcgaggtacgggcccgcatcagggcatggtgcgagttcgtcctgaactgaccaatttagtccagtttcagcagttgaat

SEQ ID NO: 3589 - DNA, 120 bp, synthetic construct
  source 1..120: mol_type = other DNA
cagggcatggtgcgagttcgtcctgaactgaccaatttagtccagtttcagcagttgaatttgctggcacctgagtgggcgctaccggggcaatttgatgccattttttgccgtaatgtc

SEQ ID NO: 3590 - DNA, 120 bp, synthetic construct
  source 1..120: mol_type = other DNA
ttgctggcacctgagtgggcgctaccggggcaatttgatgccattttttgccgtaatgtcatgatctattttgataaagagacgcaggaacgcattctgcgtcgttttgtacctttgcta

SEQ ID NO: 3591 - DNA, 120 bp, synthetic construct
  source 1..120: mol_type = other DNA
atgatctattttgataaagagacgcaggaacgcattctgcgtcgttttgtacctttgctaaaaccaggcggcctgatgttcgctggccactcggagaatttcagccagatcagtcgggaa

SEQ ID NO: 3592 - DNA, 120 bp, synthetic construct
  source 1..120: mol_type = other DNA
gtacctttgctaaaaccaggcggcctgatgttcgctggccactcggagaatttcagccagatcagtcgggaattctatttgcgcgggcagaccgtttatgggctgaccaaggagaggtga

SEQ ID NO: 3593 - DNA, 120 bp, synthetic construct
  source 1..120: mol_type = other DNA
taactctttggtaatcctaatgttactgacatttccggcttcacaatattattgtgatatacctgcatttcattgtaaaactccatgtcatcacaataaatcgggagaaaataatgacaa

SEQ ID NO: 3594 - DNA, 120 bp, synthetic construct
  source 1..120: mol_type = other DNA
acctgcatttcattgtaaaactccatgtcatcacaataaatcgggagaaaataatgacaatcaatagtattgtcatttcgtctttttatgacctccacatcgtaaccatcccgcttattt

SEQ ID NO: 3595 - DNA, 120 bp, synthetic construct
  source 1..120: mol_type = other DNA
tcaatagtattgtcatttcgtctttttatgacctccacatcgtaaccatcccgcttatttaaattataaataggcaaagagttataatatatgttgtacatgtgatgaacatactgatca

SEQ ID NO: 3596 - DNA, 120 bp, synthetic construct
  source 1..120: mol_type = other DNA
aaattataaataggcaaagagttataatatatgttgtacatgtgatgaacatactgatcatatgtatcattgaagaaaaaataagcatacaggcctttatctacctttatttcactatcg

SEQ ID NO: 3597 - DNA, 120 bp, synthetic construct
  source 1..120: mol_type = other DNA
tatgtatcattgaagaaaaaataagcatacaggcctttatctacctttatttcactatcgctgaaatgcttattcctatcccaaacaaccgttcttgcaataatgtcattcgttttatca

SEQ ID NO: 3598 - DNA, 120 bp, synthetic construct
  source 1..120: mol_type = other DNA
ctgaaatgcttattcctatcccaaacaaccgttcttgcaataatgtcattcgttttatcatgaaaggggattctgtttgatactgttatagctgtatttttcttcaacgaatcatataac

SEQ ID NO: 3599 - DNA, 120 bp, synthetic construct
  source 1..120: mol_type = other DNA
tgaaaggggattctgtttgatactgttatagctgtatttttcttcaacgaatcatataacttacccaatctacattttgaatctatcccagagtagaacactaaatccctaaaattaaag

SEQ ID NO: 3600 - DNA, 120 bp, synthetic construct
  source 1..120: mol_type = other DNA
ttacccaatctacattttgaatctatcccagagtagaacactaaatccctaaaattaaagcattgaccaattatatttctctctttaaggtaacagattcgtggttgaaggtattcacag

SEQ ID NO: 3601 - DNA, 120 bp, synthetic construct
  source 1..120: mol_type = other DNA
cattgaccaattatatttctctctttaaggtaacagattcgtggttgaaggtattcacagttaatttcccttctacccaacaaacctttaaaggaccaaaaagggatcatcctatactgc

SEQ ID NO: 3602 - DNA, 120 bp, synthetic construct
  source 1..120: mol_type = other DNA
ttaatttcccttctacccaacaaacctttaaaggaccaaaaagggatcatcctatactgccgtggggtataaccaaatattttcttaaattctctggtgaatgtctgttgcgaatcataa

SEQ ID NO: 3603 - DNA, 120 bp, synthetic construct
  source 1..120: mol_type = other DNA
cgtggggtataaccaaatattttcttaaattctctggtgaatgtctgttgcgaatcataaaaaagctttgctgatatctctattattgtcagcctggtaagccgtaatagtgcagcagct

SEQ ID NO: 3604 - DNA, 120 bp, synthetic construct
  source 1..120: mol_type = other DNA
aaaagctttgctgatatctctattattgtcagcctggtaagccgtaatagtgcagcagctctactagcccttctaactctaatatatgttccaataggcattccgacatattccttaaag

SEQ ID NO: 3605 - DNA, 120 bp, synthetic construct
  source 1..120: mol_type = other DNA
ctactagcccttctaactctaatatatgttccaataggcattccgacatattccttaaaggaaatttgcaaataccttctgctgaatcctgaatacaaaaccaaacagtcaatgttaatg

SEQ ID NO: 3606 - DNA, 120 bp, synthetic construct
  source 1..120: mol_type = other DNA
gaaatttgcaaataccttctgctgaatcctgaatacaaaaccaaacagtcaatgttaatgaatttcgactcgagattctcttctatatattgaataattgaatttacagtcatctgtttt

SEQ ID NO: 3607 - DNA, 120 bp, synthetic construct
  source 1..120: mol_type = other DNA
aatttcgactcgagattctcttctatatattgaataattgaatttacagtcatctgttttagcatgaatataacccaaatcaaaataatagcattctagatagtgggccggcgccgggac

SEQ ID NO: 3608 - DNA, 120 bp, synthetic construct
  source 1..120: mol_type = other DNA
agcatgaatataacccaaatcaaaataatagcattctagatagtgggccggcgccgggacttagctatttgcgcatacccagcaacaccaatcttagctatttgtgcacgcgcatcaata

SEQ ID NO: 3609 - DNA, 120 bp, synthetic construct
  source 1..120: mol_type = other DNA
ttagctatttgcgcatacccagcaacaccaatcttagctatttgtgcacgcgcatcaatatcaaaattagctatttgcgcaacaagcaagtggagtgcgcgaaaagctaaactttgtgtg

SEQ ID NO: 3610 - DNA, 120 bp, synthetic construct
  source 1..120: mol_type = other DNA
tcaaaattagctatttgcgcaacaagcaagtggagtgcgcgaaaagctaaactttgtgtgcatttttaaataaaattgttctcagtgaggctgtgctacggatataaaaatccccttcat

SEQ ID NO: 3611 - DNA, 120 bp, synthetic construct
  source 1..120: mol_type = other DNA
catttttaaataaaattgttctcagtgaggctgtgctacggatataaaaatccccttcatttgttacccacctttttacgcatatcgtcgatatgaaatgatggggagggggtgggaagg

SEQ ID NO: 3612 - DNA, 120 bp, synthetic construct
  source 1..120: mol_type = other DNA
ttgttacccacctttttacgcatatcgtcgatatgaaatgatggggagggggtgggaaggtgttgtcaccattccgtaaggaggttaagctcatgattttaaatagattaagtacgttag

SEQ ID NO: 3613 - DNA, 120 bp, synthetic construct
  source 1..120: mol_type = other DNA
tgttgtcaccattccgtaaggaggttaagctcatgattttaaatagattaagtacgttaggaattattactttcggcatgcttagttttgctgcgaactctgctcaaccagatatcaaat

SEQ ID NO: 3614 - DNA, 120 bp, synthetic construct
  source 1..120: mol_type = other DNA
gaattattactttcggcatgcttagttttgctgcgaactctgctcaaccagatatcaaattcgcaagcaaagagtatggcgtgactataggtgagagtaggatcatatacccgttagatg

SEQ ID NO: 3615 - DNA, 120 bp, synthetic construct
  source 1..120: mol_type = other DNA
tcgcaagcaaagagtatggcgtgactataggtgagagtaggatcatatacccgttagatgctgctggcgttatggtctcggtgaaaaacacccaagattatccggttctcattcagtcta

SEQ ID NO: 3616 - DNA, 120 bp, synthetic construct
  source 1..120: mol_type = other DNA
ctgctggcgttatggtctcggtgaaaaacacccaagattatccggttctcattcagtctaggatctacgacgagaataaagaaaaagaatcagaggatcctttcgtggtcactccgccat

SEQ ID NO: 3617 - DNA, 120 bp, synthetic construct
  source 1..120: mol_type = other DNA
ggatctacgacgagaataaagaaaaagaatcagaggatcctttcgtggtcactccgccattgtttcgattggatgctaagcaacaaaattctttgcgtatagctcaggctggaggtgttt

SEQ ID NO: 3618 - DNA, 120 bp, synthetic construct
  source 1..120: mol_type = other DNA
tgtttcgattggatgctaagcaacaaaattctttgcgtatagctcaggctggaggtgttttcccgcgagataaagagagcctaaagtggttatgcgtaaaagggattccaccaaaggatg

SEQ ID NO: 3619 - DNA, 120 bp, synthetic construct
  source 1..120: mol_type = other DNA
tcccgcgagataaagagagcctaaagtggttatgcgtaaaagggattccaccaaaggatgaagatatatgggttgatgatgcgacaaataagcaaaaattcaatccagacaaagatgtgg

SEQ ID NO: 3620 - DNA, 120 bp, synthetic construct
  source 1..120: mol_type = other DNA
aagatatatgggttgatgatgcgacaaataagcaaaaattcaatccagacaaagatgtgggagtgttcgtgcaattcgcaattaataattgcattaagcttttggttcgaccgaatgaat

SEQ ID NO: 3621 - DNA, 120 bp, synthetic construct
  source 1..120: mol_type = other DNA
gagtgttcgtgcaattcgcaattaataattgcattaagcttttggttcgaccgaatgaattaaaaggaacccctatacagtttgctgaaaacttaagctggaaagttgatggggggaagc

SEQ ID NO: 3622 - DNA, 120 bp, synthetic construct
  source 1..120: mol_type = other DNA
taaaaggaacccctatacagtttgctgaaaacttaagctggaaagttgatggggggaagctaattgctgaaaacccctcacctttctacatgaacataggtgaattaacatttggaggga

SEQ ID NO: 3623 - DNA, 120 bp, synthetic construct
  source 1..120: mol_type = other DNA
taattgctgaaaacccctcacctttctacatgaacataggtgaattaacatttggagggaaaagtattccttctcactatattccacctaaatcgacgtgggcttttgatttgccaaaag

SEQ ID NO: 3624 - DNA, 120 bp, synthetic construct
  source 1..120: mol_type = other DNA
aaagtattccttctcactatattccacctaaatcgacgtgggcttttgatttgccaaaaggactagcgggagcacgtaatgtttcgtggagaataattaatgatcagggagggttggatc

SEQ ID NO: 3625 - DNA, 120 bp, synthetic construct
  source 1..120: mol_type = other DNA
aaatcgacgtgggcttttgatttgccaaaaggactagcgggagcacgtaatgtttcgtggagaataattaatgatcagggagggttggatcgtttgtattccaaaaatgtgactttatga

SEQ ID NO: 3626 - DNA, 120 bp, synthetic construct
  source 1..120: mol_type = other DNA
tgaagaaaagttctattgtggcaaccattataactattctgtccgggagtgctaatgcagcatcatctcagttaataccaaatatatcccctgacagctttacagttgcagcctccaccg

SEQ ID NO: 3627 - DNA, 120 bp, synthetic construct
  source 1..120: mol_type = other DNA
catcatctcagttaataccaaatatatcccctgacagctttacagttgcagcctccaccgggatgctgagtggaaagtctcatgaaatgctttatgacgcagaaacaggaagaaagatca

SEQ ID NO: 3628 - DNA, 120 bp, synthetic construct
  source 1..120: mol_type = other DNA
ggatgctgagtggaaagtctcatgaaatgctttatgacgcagaaacaggaagaaagatcagccagttagactggaagatcaaaaatgtcgctatcctgaaaggtgatatatcctgggatc

SEQ ID NO: 3629 - DNA, 120 bp, synthetic construct
  source 1..120: mol_type = other DNA
gccagttagactggaagatcaaaaatgtcgctatcctgaaaggtgatatatcctgggatccatactcatttctgaccctgaatgccagggggtggacgtctctggcttccgggtcaggta

SEQ ID NO: 3630 - DNA, 120 bp, synthetic construct
  source 1..120: mol_type = other DNA
catactcatttctgaccctgaatgccagggggtggacgtctctggcttccgggtcaggtaatatggatgactacgactggatgaatgaaaatcaatctgagtggacagatcactcatctc

SEQ ID NO: 3631 - DNA, 120 bp, synthetic construct
  source 1..120: mol_type = other DNA
atatggatgactacgactggatgaatgaaaatcaatctgagtggacagatcactcatctcatcctgctacaaatgttaatcatgccaatgaatatgacctcaatgtgaaaggctggttac

SEQ ID NO: 3632 - DNA, 120 bp, synthetic construct
  source 1..120: mol_type = other DNA
atcctgctacaaatgttaatcatgccaatgaatatgacctcaatgtgaaaggctggttactccaggatgagaattataaagcaggtataacagcaggatatcaggaaacacgtttcagtt

SEQ ID NO: 3633 - DNA, 120 bp, synthetic construct
  source 1..120: mol_type = other DNA
tccaggatgagaattataaagcaggtataacagcaggatatcaggaaacacgtttcagttggacagctacaggtggttcatatagttataataatggagcttataccggaaacttcccga

SEQ ID NO: 3634 - DNA, 120 bp, synthetic construct
  source 1..120: mol_type = other DNA
ggacagctacaggtggttcatatagttataataatggagcttataccggaaacttcccgaaaggagtgcgggtaataggttataaccagcgcttttctatgccatatattggacttgcag

SEQ ID NO: 3635 - DNA, 120 bp, synthetic construct
  source 1..120: mol_type = other DNA
aaggagtgcgggtaataggttataaccagcgcttttctatgccatatattggacttgcaggccagtatcgcattaatgattttgagttaaatgcattatttaaattcagcgactgggttc

SEQ ID NO: 3636 - DNA, 120 bp, synthetic construct
  source 1..120: mol_type = other DNA
gccagtatcgcattaatgattttgagttaaatgcattatttaaattcagcgactgggttcgggcacatgataatgatgagcactatatgagagatcttactttccgtgagaagacatccg

SEQ ID NO: 3637 - DNA, 120 bp, synthetic construct
  source 1..120: mol_type = other DNA
gggcacatgataatgatgagcactatatgagagatcttactttccgtgagaagacatccggctcacgttattatggtaccgtaattaacgctggatattatgtcacacctaatgccaaag

SEQ ID NO: 3638 - DNA, 120 bp, synthetic construct
  source 1..120: mol_type = other DNA
gctcacgttattatggtaccgtaattaacgctggatattatgtcacacctaatgccaaagtctttgcggaatttacatacagtaaatatgatgagggcaaaggaggtactcagaccattg

SEQ ID NO: 3639 - DNA, 120 bp, synthetic construct
  source 1..120: mol_type = other DNA
tctttgcggaatttacatacagtaaatatgatgagggcaaaggaggtactcagaccattgataagaatagtggagattctgtctctattggcggagatgctgccggtatttccaataaaa

SEQ ID NO: 3640 - DNA, 120 bp, synthetic construct
  source 1..120: mol_type = other DNA
ataagaatagtggagattctgtctctattggcggagatgctgccggtatttccaataaaaattatactgtgacggcgggtctgcaatatcgcttctgaaaaatacagatcatatctctct

SEQ ID NO: 3641 - DNA, 120 bp, synthetic construct
  source 1..120: mol_type = other DNA
attatactgtgacggcgggtctgcaatatcgcttctgaaaaatacagatcatatctctcttttcatcctcccctagcggggaggatgtctgtggaaaggaggttggtgtttgaccaacct

SEQ ID NO: 3642 - DNA, 120 bp, synthetic construct
  source 1..120: mol_type = other DNA
tttcatcctcccctagcggggaggatgtctgtggaaaggaggttggtgtttgaccaaccttcagatgtgtgaaaaatcacctttttcaccataatgacggggcgctcattctgttgtttt

SEQ ID NO: 3643 - DNA, 120 bp, synthetic construct
  source 1..120: mol_type = other DNA
tcagatgtgtgaaaaatcacctttttcaccataatgacggggcgctcattctgttgttttgccttgacattctccacgtctttcagggcatggagaaggtcaaattagacatggaacgct

SEQ ID NO: 3644 - DNA, 120 bp, synthetic construct
  source 1..120: mol_type = other DNA
gccttgacattctccacgtctttcagggcatggagaaggtcaaattagacatggaacgctactctccttcctgtaggaagctcaacatccaagcttaatttgcctcccattgcttcaacg

SEQ ID NO: 3645 - DNA, 120 bp, synthetic construct
  source 1..120: mol_type = other DNA
actctccttcctgtaggaagctcaacatccaagcttaatttgcctcccattgcttcaacgtaacgctttaacgtcgccagctttaaatcatttccgcgctgctccagctttgttactgct

SEQ ID NO: 3646 - DNA, 120 bp, synthetic construct
  source 1..120: mol_type = other DNA
taacgctttaacgtcgccagctttaaatcatttccgcgctgctccagctttgttactgctggctggcttatacccatcgcctcagcaacttgtttttgtgataactggagttcttcacgc

SEQ ID NO: 3647 - DNA, 120 bp, synthetic construct
  source 1..120: mol_type = other DNA
ggctggcttatacccatcgcctcagcaacttgtttttgtgataactggagttcttcacgcatcatctgcaagccgacctcaagaatcatctcatctgccatttctttaattcgtgtctgg

SEQ ID NO: 3648 - DNA, 120 bp, synthetic construct
  source 1..120: mol_type = other DNA
ctggagttcttcacgcatcatctgcaagccgacctcaagaatcatctcatctgccatttctttaattcgtgtctggctttcaggtgaacgactggcaatcacctcatctaatgttctcat

SEQ ID NO: 3649 - DNA, 120 bp, synthetic construct
  source 1..120: mol_type = other DNA
agttgttgatctgtgtgaatcagactgcgacagttcgagtttgaagcgagagctaacaacagtatcaacaggtttaatttggatttggaaacgagagtttctggtcatgaaaaacccaaa

SEQ ID NO: 3650 - DNA, 120 bp, synthetic construct
  source 1..120: mol_type = other DNA
agtatcaacaggtttaatttggatttggaaacgagagtttctggtcatgaaaaacccaaagaagaaatccggaggattccggattgtcaatatgctaaaacgcggagtagcccgtgtaaa

SEQ ID NO: 3651 - DNA, 120 bp, synthetic construct
  source 1..120: mol_type = other DNA
gaagaaatccggaggattccggattgtcaatatgctaaaacgcggagtagcccgtgtaaaccccttggggggtttgaagaggctgccagccggacttctgctgggccatggacccatcag

SEQ ID NO: 3652 - DNA, 120 bp, synthetic construct
  source 1..120: mol_type = other DNA
ccccttggggggtttgaagaggctgccagccggacttctgctgggccatggacccatcagaatggttttggcgatactagccttcttgagattcacagcaatcaaaccatcactgggcct

SEQ ID NO: 3653 - DNA, 120 bp, synthetic construct
  source 1..120: mol_type = other DNA
aatggttttggcgatactagccttcttgagattcacagcaatcaaaccatcactgggcctcatcaatagatggggttccgtggggaagaaggaggctatggaaataataaaaaagttcaa

SEQ ID NO: 3654 - DNA, 120 bp, synthetic construct
  source 1..120: mol_type = other DNA
catcaatagatggggttccgtggggaagaaggaggctatggaaataataaaaaagttcaagaaagaccttgctgccatgttgagaattatcaatgctaggaaggagaggaagagacgtgg

SEQ ID NO: 3655 - DNA, 120 bp, synthetic construct
  source 1..120: mol_type = other DNA
gaaagaccttgctgccatgttgagaattatcaatgctaggaaggagaggaagagacgtggcgctgacaccagcatcggaatcgtcggcctcctgctgaccacagccatggcagccgagat

SEQ ID NO: 3656 - DNA, 120 bp, synthetic construct
  source 1..120: mol_type = other DNA
cgctgacaccagcatcggaatcgtcggcctcctgctgaccacagccatggcagccgagatcactagacgtgggagtgcatactacatgtacttggacaggagcgatgctggtaaggccat

SEQ ID NO: 3657 - DNA, 120 bp, synthetic construct
  source 1..120: mol_type = other DNA
cactagacgtgggagtgcatactacatgtacttggacaggagcgatgctggtaaggccatttcttttgccaccacattgggggtgaacaaatgccatgtacagatcatggacctcgggca

SEQ ID NO: 3658 - DNA, 120 bp, synthetic construct
  source 1..120: mol_type = other DNA
ttcttttgccaccacattgggggtgaacaaatgccatgtacagatcatggacctcgggcacatgtgtgacgccaccatgagttatgagtgccccatgctagacgagggagtggagccaga

SEQ ID NO: 3659 - DNA, 120 bp, synthetic construct
  source 1..120: mol_type = other DNA
catgtgtgacgccaccatgagttatgagtgccccatgctagacgagggagtggagccagatgacgtcgattgctggtgcaacacgacatcgacttgggttgtgtacggaacctgtcatca

SEQ ID NO: 3660 - DNA, 120 bp, synthetic construct
  source 1..120: mol_type = other DNA
tgacgtcgattgctggtgcaacacgacatcgacttgggttgtgtacggaacctgtcatcataaaaaaggtgaagcacgacgatccagaagagccgtgacgcttccttctcactccacgag

SEQ ID NO: 3661 - DNA, 120 bp, synthetic construct
  source 1..120: mol_type = other DNA
taaaaaaggtgaagcacgacgatccagaagagccgtgacgcttccttctcactccacgaggaagctgcaaacgcgatcgcagacttggctagagtcaagagaatacacaaagcacctgat

SEQ ID NO: 3662 - DNA, 120 bp, synthetic construct
  source 1..120: mol_type = other DNA
gaagctgcaaacgcgatcgcagacttggctagagtcaagagaatacacaaagcacctgatcaaggttgaaaattggatatttaggaaccccgggtttgcgctagtggctgtagctatagc

SEQ ID NO: 3663 - DNA, 120 bp, synthetic construct
  source 1..120: mol_type = other DNA
caaggttgaaaattggatatttaggaaccccgggtttgcgctagtggctgtagctatagcctggctcctgggaagctcgacgagccaaaaagttatatacttggtcatgatattgttgat

SEQ ID NO: 3664 - DNA, 120 bp, synthetic construct
  source 1..120: mol_type = other DNA
ctggctcctgggaagctcgacgagccaaaaagttatatacttggtcatgatattgttgattgccccggcatacagcattaggtgcataggagttagcaatagagatttcgtggagggcat

SEQ ID NO: 3665 - DNA, 120 bp, synthetic construct
  source 1..120: mol_type = other DNA
tgccccggcatacagcattaggtgcataggagttagcaatagagatttcgtggagggcatgtcaggtgggacctgggttgatgttgtcttggaacatgggggttgcgtcaccgtgatggc

SEQ ID NO: 3666 - DNA, 120 bp, synthetic construct
  source 1..120: mol_type = other DNA
gtcaggtgggacctgggttgatgttgtcttggaacatgggggttgcgtcaccgtgatggcacaggacaagccaacagttgatatcgagttggtcacgacaacggttagcaacatggccga

SEQ ID NO: 3667 - DNA, 120 bp, synthetic construct
  source 1..120: mol_type = other DNA
acaggacaagccaacagttgatatcgagttggtcacgacaacggttagcaacatggccgaggtaagatcctactgctatgaggcatcaatatcggacatggcttcggacagccgttgtcc

SEQ ID NO: 3668 - DNA, 120 bp, synthetic construct
  source 1..120: mol_type = other DNA
ggtaagatcctactgctatgaggcatcaatatcggacatggcttcggacagccgttgtccaacacaaggtgaagcctaccttgacaagcagtcagacactcaatatgtctgcaagagaac

SEQ ID NO: 3669 - DNA, 120 bp, synthetic construct
  source 1..120: mol_type = other DNA
aacacaaggtgaagcctaccttgacaagcagtcagacactcaatatgtctgcaagagaacattggtggatagaggttggggaaatgggtgtggactttttggcaaagggagcttggtgac

SEQ ID NO: 3670 - DNA, 120 bp, synthetic construct
  source 1..120: mol_type = other DNA
attggtggatagaggttggggaaatgggtgtggactttttggcaaagggagcttggtgacatgtgccaagtttacgtgctccaagaaaatgacaggcaagagcatccagccggagaactt

SEQ ID NO: 3671 - DNA, 120 bp, synthetic construct
  source 1..120: mol_type = other DNA
atgtgccaagtttacgtgctccaagaaaatgacaggcaagagcatccagccggagaacttggagtaccggataatgctatcagtgcatggatcccagcacagtgggatgattgtgaatga

SEQ ID NO: 3672 - DNA, 120 bp, synthetic construct
  source 1..120: mol_type = other DNA
ggagtaccggataatgctatcagtgcatggatcccagcacagtgggatgattgtgaatgacacaggacatgaaactgacgaaaacagagcaaaagtcgaggtcacacccaattcaccaag

SEQ ID NO: 3673 - DNA, 120 bp, synthetic construct
  source 1..120: mol_type = other DNA
cacaggacatgaaactgacgaaaacagagcaaaagtcgaggtcacacccaattcaccaagagcagaagcaaccttgggaggttttggaagcttgggacttgactgtgaaccaaggacagg

SEQ ID NO: 3674 - DNA, 120 bp, synthetic construct
  source 1..120: mol_type = other DNA
agcagaagcaaccttgggaggttttggaagcttgggacttgactgtgaaccaaggacaggccttgacttctcagatctgtattacctgaccatgaacaataagcattggttggtgcacaa

SEQ ID NO: 3675 - DNA, 120 bp, synthetic construct
  source 1..120: mol_type = other DNA
ccttgacttctcagatctgtattacctgaccatgaacaataagcattggttggtgcacaaggagtggtttcatgacatcccattaccttggcatgctggtgcagacactggaactccaca

SEQ ID NO: 3676 - DNA, 120 bp, synthetic construct
  source 1..120: mol_type = other DNA
ggagtggtttcatgacatcccattaccttggcatgctggtgcagacactggaactccacactggaacaacaaagaggcattggtggagttcaaggacgcccacgccaagaggcaaactgt

SEQ ID NO: 3677 - DNA, 120 bp, synthetic construct
  source 1..120: mol_type = other DNA
ctggaacaacaaagaggcattggtggagttcaaggacgcccacgccaagaggcaaactgttgtggttctggggagccaagagggagctgttcatacggccctcgctggagctttggaggc

SEQ ID NO: 3678 - DNA, 120 bp, synthetic construct
  source 1..120: mol_type = other DNA
tgtggttctggggagccaagagggagctgttcatacggccctcgctggagctttggaggctgagatggatggtgcaaagggaaggctattctctggccatttgaaatgccgcctaaaaat

SEQ ID NO: 3679 - DNA, 120 bp, synthetic construct
  source 1..120: mol_type = other DNA
tgagatggatggtgcaaagggaaggctattctctggccatttgaaatgccgcctaaaaatggacaagcttaggttgaagggtgtgtcatattccctgtgtaccgcagcgttcacatttac

SEQ ID NO: 3680 - DNA, 120 bp, synthetic construct
  source 1..120: mol_type = other DNA
ggacaagcttaggttgaagggtgtgtcatattccctgtgtaccgcagcgttcacatttaccaaggtcccagctgaaacattgcatggaacagtcacagtggaggtgcagtatgcagggac

SEQ ID NO: 3681 - DNA, 120 bp, synthetic construct
  source 1..120: mol_type = other DNA
caaggtcccagctgaaacattgcatggaacagtcacagtggaggtgcagtatgcagggacagacggaccctgcaaagtcccagcccagatggcggtggacatgcagaccctgaccccagt

SEQ ID NO: 3682 - DNA, 120 bp, synthetic construct
  source 1..120: mol_type = other DNA
agacggaccctgcaaagtcccagcccagatggcggtggacatgcagaccctgaccccagttggaaggctgataaccgccaatcctgtgatcactgaaagtactgagaattcaaagatgat

SEQ ID NO: 3683 - DNA, 120 bp, synthetic construct
  source 1..120: mol_type = other DNA
tggaaggctgataaccgccaatcctgtgatcactgaaagtactgagaattcaaagatgatgttggagctcgacccaccatttggggattcttacattgtcataggagtcggggacaagaa

SEQ ID NO: 3684 - DNA, 120 bp, synthetic construct
  source 1..120: mol_type = other DNA
gttggagctcgacccaccatttggggattcttacattgtcataggagtcggggacaagaaaatcacccatcactggcatcggagtggtagcaccatcggaaaggcatttgaagccactgt

SEQ ID NO: 3685 - DNA, 120 bp, synthetic construct
  source 1..120: mol_type = other DNA
aatcacccatcactggcatcggagtggtagcaccatcggaaaggcatttgaagccactgtgagaggtgccaagagaatggcagtcttgggggacacagcctgggactttggatcagttgg

SEQ ID NO: 3686 - DNA, 120 bp, synthetic construct
  source 1..120: mol_type = other DNA
gagaggtgccaagagaatggcagtcttgggggacacagcctgggactttggatcagttgggggtgtgtttaattcattgggtaagggtattcaccagatctttggagcagctttcaaatc

SEQ ID NO: 3687 - DNA, 120 bp, synthetic construct
  source 1..120: mol_type = other DNA
gggtgtgtttaattcattgggtaagggtattcaccagatctttggagcagctttcaaatcactgtttggaggaatgtcctggttctcacagatcctcataggcacactgttggtgtggtt

SEQ ID NO: 3688 - DNA, 120 bp, synthetic construct
  source 1..120: mol_type = other DNA
actgtttggaggaatgtcctggttctcacagatcctcataggcacactgttggtgtggttaggtttgaacacaaagaatggatctatctccctcacatgcttagccctggggggagtgat

SEQ ID NO: 3689 - DNA, 120 bp, synthetic construct
  source 1..120: mol_type = other DNA
aggtttgaacacaaagaatggatctatctccctcacatgcttagccctggggggagtgatgatcttcctttccacggctgtttctgctgatgttgggtgctcggtggacttctcaaaaaa

SEQ ID NO: 3690 - DNA, 120 bp, synthetic construct
  source 1..120: mol_type = other DNA
gatcttcctttccacggctgtttctgctgatgttgggtgctcggtggacttctcaaaaaaggaaacgagatgtggcacgggggtgttcgtctacaatgacgttgaagcctggagggaccg

SEQ ID NO: 3691 - DNA, 120 bp, synthetic construct
  source 1..120: mol_type = other DNA
ggaaacgagatgtggcacgggggtgttcgtctacaatgacgttgaagcctggagggaccggtacaagtaccatcctgactccccccgcagattggcagcagctgttaagcaggcttggga

SEQ ID NO: 3692 - DNA, 120 bp, synthetic construct
  source 1..120: mol_type = other DNA
gtacaagtaccatcctgactccccccgcagattggcagcagctgttaagcaggcttgggaagaggggatttgtgggatctcctccgtttcgagaatggaaaacatcatgtggaaatcagt

SEQ ID NO: 3693 - DNA, 120 bp, synthetic construct
  source 1..120: mol_type = other DNA
agaggggatttgtgggatctcctccgtttcgagaatggaaaacatcatgtggaaatcagtggaaggggagcttaatgcaatcctagaggagaatggagttcaactgacagttgtagtggg

SEQ ID NO: 3694 - DNA, 120 bp, synthetic construct
  source 1..120: mol_type = other DNA
ggaaggggagcttaatgcaatcctagaggagaatggagttcaactgacagttgtagtggggtctgtaaaaaaccctatgtggagaggtccacagagattgccagtgcctgtgaatgagct

SEQ ID NO: 3695 - DNA, 120 bp, synthetic construct
  source 1..120: mol_type = other DNA
gtctgtaaaaaaccctatgtggagaggtccacagagattgccagtgcctgtgaatgagctgccccatggctggaaagcctgggggaaatcgtactttgtcagagcagcaaagaccaacaa

SEQ ID NO: 3696 - DNA, 120 bp, synthetic construct
  source 1..120: mol_type = other DNA
gccccatggctggaaagcctgggggaaatcgtactttgtcagagcagcaaagaccaacaacagttttgttgtcgacggtgacacactgaaggagtgtccgctcaaacatagagcatggaa

SEQ ID NO: 3697 - DNA, 120 bp, synthetic construct
  source 1..120: mol_type = other DNA
cagttttgttgtcgacggtgacacactgaaggagtgtccgctcaaacatagagcatggaatagcttccttgtggaggatcacgggtttgggatcttccacaccagtgtttggctgaaggt

SEQ ID NO: 3698 - DNA, 120 bp, synthetic construct
  source 1..120: mol_type = other DNA
tagcttccttgtggaggatcacgggtttgggatcttccacaccagtgtttggctgaaggtcagagaggactactcactagagtgtgacccagccgtcataggaacagctgtcaagggaaa

SEQ ID NO: 3699 - DNA, 120 bp, synthetic construct
  source 1..120: mol_type = other DNA
cagagaggactactcactagagtgtgacccagccgtcataggaacagctgtcaagggaaaggaagctgcacacagtgatctaggctattggattgagagtgaaaagaatgacacatggag

SEQ ID NO: 3700 - DNA, 120 bp, synthetic construct
  source 1..120: mol_type = other DNA
ggaagctgcacacagtgatctaggctattggattgagagtgaaaagaatgacacatggaggctgaggagggctcatctgattgagatgaaaacatgtgagtggccaaagtctcacacact

SEQ ID NO: 3701 - DNA, 120 bp, synthetic construct
  source 1..120: mol_type = other DNA
gctgaggagggctcatctgattgagatgaaaacatgtgagtggccaaagtctcacacactgtggacagatggagtggaagaaagtgatctgatcatacccaagtccttagctggtccact

SEQ ID NO: 3702 - DNA, 120 bp, synthetic construct
  source 1..120: mol_type = other DNA
gtggacagatggagtggaagaaagtgatctgatcatacccaagtccttagctggtccactcagccaccacaacaccagagagggttacagaactcaagtgaaagggccatggcatagtga

SEQ ID NO: 3703 - DNA, 120 bp, synthetic construct
  source 1..120: mol_type = other DNA
cagccaccacaacaccagagagggttacagaactcaagtgaaagggccatggcatagtgaagagctcgaaatccggtttgaggagtgcccaggaaccaaggttcacgtggaggagacatg

SEQ ID NO: 3704 - DNA, 120 bp, synthetic construct
  source 1..120: mol_type = other DNA
agagctcgaaatccggtttgaggagtgcccaggaaccaaggttcacgtggaggagacatgcggaactagaggaccatctctgagatcaactactgctagtggaagggtcatagaggaatg

SEQ ID NO: 3705 - DNA, 120 bp, synthetic construct
  source 1..120: mol_type = other DNA
cggaactagaggaccatctctgagatcaactactgctagtggaagggtcatagaggaatggtgctgtagggaatgcacaatgcctccactatcgttccgggcgaaagacggctgctggta

SEQ ID NO: 3706 - DNA, 120 bp, synthetic construct
  source 1..120: mol_type = other DNA
gtgctgtagggaatgcacaatgcctccactatcgttccgggcgaaagacggctgctggtatggaatggagataaggcccagaaaggaaccagagagcaacttagtgaggtccatggtgac

SEQ ID NO: 3707 - DNA, 120 bp, synthetic construct
  source 1..120: mol_type = other DNA
tggaatggagataaggcccagaaaggaaccagagagcaacttagtgaggtccatggtgacagcaggatcaaccgatcatatggatcacttctctcttggagtgcttgtgattctactcat

SEQ ID NO: 3708 - DNA, 120 bp, synthetic construct
  source 1..120: mol_type = other DNA
agcaggatcaaccgatcatatggatcacttctctcttggagtgcttgtgattctactcatggtgcaggaaggtttgaagaagagaatgaccacaaagatcataatgagcacatcaatggc

SEQ ID NO: 3709 - DNA, 120 bp, synthetic construct
  source 1..120: mol_type = other DNA
ggtgcaggaaggtttgaagaagagaatgaccacaaagatcataatgagcacatcaatggcagtgctggtagccatggtcttgggaggattctcaatgagtgacctggctaagcttgtgat

SEQ ID NO: 3710 - DNA, 120 bp, synthetic construct
  source 1..120: mol_type = other DNA
agtgctggtagccatggtcttgggaggattctcaatgagtgacctggctaagcttgtgatcctgatgggtgctactttcgcagaaatgaacactggaggagatgtagctcacttggcatt

SEQ ID NO: 3711 - DNA, 120 bp, synthetic construct
  source 1..120: mol_type = other DNA
cctgatgggtgctactttcgcagaaatgaacactggaggagatgtagctcacttggcattggttgcggcatttaaagtcagaccagccttgttggtttccttcatcttcagagccaactg

SEQ ID NO: 3712 - DNA, 120 bp, synthetic construct
  source 1..120: mol_type = other DNA
ggttgcggcatttaaagtcagaccagccttgttggtttccttcatcttcagagccaactggacaccccgtgagagcatgctgctagccctggcttcgtgcctcctgcagactgcgatctc

SEQ ID NO: 3713 - DNA, 120 bp, synthetic construct
  source 1..120: mol_type = other DNA
gacaccccgtgagagcatgctgctagccctggcttcgtgcctcctgcagactgcgatctctgctcttgaaggcgagctgatggtcctcgttaatggatttgctttggcctggttggcaat

SEQ ID NO: 3714 - DNA, 120 bp, synthetic construct
  source 1..120: mol_type = other DNA
tgctcttgaaggcgagctgatggtcctcgttaatggatttgctttggcctggttggcaatacgagcaatggccgtgccacgcactgacaatatcgctctggcaattctggctgctctaac

SEQ ID NO: 3715 - DNA, 120 bp, synthetic construct
  source 1..120: mol_type = other DNA
acgagcaatggccgtgccacgcactgacaatatcgctctggcaattctggctgctctaacaccattagccagaggcacactgctcgtggcatggagagcgggcctcgccacttgtggagg

SEQ ID NO: 3716 - DNA, 120 bp, synthetic construct
  source 1..120: mol_type = other DNA
accattagccagaggcacactgctcgtggcatggagagcgggcctcgccacttgtggagggttcatgctcctttccctgaaagggaaaggtagtgtgaagaagaacctgccttttgtcat

SEQ ID NO: 3717 - DNA, 120 bp, synthetic construct
  source 1..120: mol_type = other DNA
gttcatgctcctttccctgaaagggaaaggtagtgtgaagaagaacctgccttttgtcatggccttggggttgaccgctgtgaggatagtggaccccatcaatgtggtaggactactgtt

SEQ ID NO: 3718 - DNA, 120 bp, synthetic construct
  source 1..120: mol_type = other DNA
ggccttggggttgaccgctgtgaggatagtggaccccatcaatgtggtaggactactgttactcacaaggagtggaaaacggagctggcctcctagtgaagtgcttacagctgttggcct

SEQ ID NO: 3719 - DNA, 120 bp, synthetic construct
  source 1..120: mol_type = other DNA
actcacaaggagtggaaaacggagctggcctcctagtgaagtgcttacagctgttggcctgatatgtgcactggccggagggtttgccaaggcagacatagagatggctgggcccatggc

SEQ ID NO: 3720 - DNA, 120 bp, synthetic construct
  source 1..120: mol_type = other DNA
gatatgtgcactggccggagggtttgccaaggcagacatagagatggctgggcccatggctgcagtgggcctgctaattgtcagttatgtggtctcgggaaagagtgtggacatgtacat

SEQ ID NO: 3721 - DNA, 120 bp, synthetic construct
  source 1..120: mol_type = other DNA
tgcagtgggcctgctaattgtcagttatgtggtctcgggaaagagtgtggacatgtacatcgaaagagcaggtgatatcacatgggaaaaagacgcggaagtcactggaaacagtcctcg

SEQ ID NO: 3722 - DNA, 120 bp, synthetic construct
  source 1..120: mol_type = other DNA
cgaaagagcaggtgatatcacatgggaaaaagacgcggaagtcactggaaacagtcctcggcttgacgtggcactagatgagagtggtgatttctccttggtagaggaggatggcccacc

SEQ ID NO: 3723 - DNA, 120 bp, synthetic construct
  source 1..120: mol_type = other DNA
gcttgacgtggcactagatgagagtggtgatttctccttggtagaggaggatggcccacccatgagagagatcatactcaaggtggttctgatggccatctgtggcatgaacccaatagc

SEQ ID NO: 3724 - DNA, 120 bp, synthetic construct
  source 1..120: mol_type = other DNA
catgagagagatcatactcaaggtggttctgatggccatctgtggcatgaacccaatagccatacccttcgctgcaggagcgtggtatgtgtatgtaaagactggaaaaaggagtggtgc

SEQ ID NO: 3725 - DNA, 120 bp, synthetic construct
  source 1..120: mol_type = other DNA
catacccttcgctgcaggagcgtggtatgtgtatgtaaagactggaaaaaggagtggtgccctctgggacgtgcctgctcccaaagaagtgaaaaaaggagagactacagatggagtgta

SEQ ID NO: 3726 - DNA, 120 bp, synthetic construct
  source 1..120: mol_type = other DNA
cctctgggacgtgcctgctcccaaagaagtgaaaaaaggagagactacagatggagtgtacagagtgatgactcgcagactgctgggttcaacacaggttggagtgggagtcatgcaaga

SEQ ID NO: 3727 - DNA, 120 bp, synthetic construct
  source 1..120: mol_type = other DNA
cagagtgatgactcgcagactgctgggttcaacacaggttggagtgggagtcatgcaagagggagtcttccacaccatgtggcacgtcacaaaaggagccgcattgaggagcggtgaagg

SEQ ID NO: 3728 - DNA, 120 bp, synthetic construct
  source 1..120: mol_type = other DNA
gggagtcttccacaccatgtggcacgtcacaaaaggagccgcattgaggagcggtgaaggaagacttgatccatattggggggacgtcaagcaggacttggtgtcatattgtgggccttg

SEQ ID NO: 3729 - DNA, 120 bp, synthetic construct
  source 1..120: mol_type = other DNA
aagacttgatccatattggggggacgtcaagcaggacttggtgtcatattgtgggccttggaagttggatgcagcctgggatggactaagtgaagtgcagcttttggccgtaccccccgg

SEQ ID NO: 3730 - DNA, 120 bp, synthetic construct
  source 1..120: mol_type = other DNA
gaagttggatgcagcctgggatggactaagtgaagtgcagcttttggccgtaccccccggagagagggctagaaacattcagactctgcctggaatattcaagacaaaggatggggacat

SEQ ID NO: 3731 - DNA, 120 bp, synthetic construct
  source 1..120: mol_type = other DNA
agagagggctagaaacattcagactctgcctggaatattcaagacaaaggatggggacatcggagcagtcgctctagactaccccgcaggaacctcaggatctccaatcctagacaaatg

SEQ ID NO: 3732 - DNA, 120 bp, synthetic construct
  source 1..120: mol_type = other DNA
cggagcagtcgctctagactaccccgcaggaacctcaggatctccaatcctagacaaatgcggaagagtgataggactttatggcaatggggttgtgatcaagaatggaagctatgttag

SEQ ID NO: 3733 - DNA, 120 bp, synthetic construct
  source 1..120: mol_type = other DNA
cggaagagtgataggactttatggcaatggggttgtgatcaagaatggaagctatgttagtgccataacccagggaaaaagggaggaggaggctccagttgagtgctttgaaccctcgat

SEQ ID NO: 3734 - DNA, 120 bp, synthetic construct
  source 1..120: mol_type = other DNA
tgccataacccagggaaaaagggaggaggaggctccagttgagtgctttgaaccctcgatgctgaggaagaagcagctaacagtcttggatctgcatccaggagccgggaaaaccaggag

SEQ ID NO: 3735 - DNA, 120 bp, synthetic construct
  source 1..120: mol_type = other DNA
gctgaggaagaagcagctaacagtcttggatctgcatccaggagccgggaaaaccaggagggttcttcctgaaatagtccgtgaagccataaagaagagacttcgcacagtgatcctagc

SEQ ID NO: 3736 - DNA, 120 bp, synthetic construct
  source 1..120: mol_type = other DNA
ggttcttcctgaaatagtccgtgaagccataaagaagagacttcgcacagtgatcctagcaccaaccagggtcgttgccgctgagatggaggaagccctaagaggactgccggtgcgtta

SEQ ID NO: 3737 - DNA, 120 bp, synthetic construct
  source 1..120: mol_type = other DNA
accaaccagggtcgttgccgctgagatggaggaagccctaagaggactgccggtgcgttacatgacaacagcagtcaacgtcacccactctgggacagaaatcgtcgatttgatgtgcca

SEQ ID NO: 3738 - DNA, 120 bp, synthetic construct
  source 1..120: mol_type = other DNA
catgacaacagcagtcaacgtcacccactctgggacagaaatcgtcgatttgatgtgccatgccaccttcacttcacgcctactacaacccatcagagtccccaactacaacctttacat

SEQ ID NO: 3739 - DNA, 120 bp, synthetic construct
  source 1..120: mol_type = other DNA
tgccaccttcacttcacgcctactacaacccatcagagtccccaactacaacctttacatcatggatgaagctcatttcacagatccctcaagcatagctgcacgaggatatatatcaac

SEQ ID NO: 3740 - DNA, 120 bp, synthetic construct
  source 1..120: mol_type = other DNA
catggatgaagctcatttcacagatccctcaagcatagctgcacgaggatatatatcaacaagggttgaaatgggcgaggcggctgctatcttcatgactgctacaccaccaggaacccg

SEQ ID NO: 3741 - DNA, 120 bp, synthetic construct
  source 1..120: mol_type = other DNA
aagggttgaaatgggcgaggcggctgctatcttcatgactgctacaccaccaggaacccgcgatgcgtttccggattccaactcaccaatcatggacacagaagtggaagttccagagag

SEQ ID NO: 3742 - DNA, 120 bp, synthetic construct
  source 1..120: mol_type = other DNA
cgatgcgtttccggattccaactcaccaatcatggacacagaagtggaagttccagagagagcctggagctcaggctttgactgggtgacggatcattctgggaaaacaatttggtttgt

SEQ ID NO: 3743 - DNA, 120 bp, synthetic construct
  source 1..120: mol_type = other DNA
agcctggagctcaggctttgactgggtgacggatcattctgggaaaacaatttggtttgttccaagtgtgagaaacggaaatgaaatcgcagcctgtctgacaaaggctggaaagcgggt

SEQ ID NO: 3744 - DNA, 120 bp, synthetic construct
  source 1..120: mol_type = other DNA
tccaagtgtgagaaacggaaatgaaatcgcagcctgtctgacaaaggctggaaagcgggtcatacagctcagcaggaagacttttgagacagagtttcagaagacaagaaatcaagagtg

SEQ ID NO: 3745 - DNA, 120 bp, synthetic construct
  source 1..120: mol_type = other DNA
catacagctcagcaggaagacttttgagacagagtttcagaagacaagaaatcaagagtgggactttgtcataacaactgacatttcagagatgggtgccaatttcaaggctgaccgggt

SEQ ID NO: 3746 - DNA, 120 bp, synthetic construct
  source 1..120: mol_type = other DNA
ggactttgtcataacaactgacatttcagagatgggtgccaatttcaaggctgaccgggtcatagattccaggagatgcctaaagccagtcatactcgatggcgagagagtcatcctggc

SEQ ID NO: 3747 - DNA, 120 bp, synthetic construct
  source 1..120: mol_type = other DNA
catagattccaggagatgcctaaagccagtcatactcgatggcgagagagtcatcctggctgggcccatgcctgtcacgcatgccagtgctgctcagaggagaggacgtgtaggcaggaa

SEQ ID NO: 3748 - DNA, 120 bp, synthetic construct
  source 1..120: mol_type = other DNA
tgggcccatgcctgtcacgcatgccagtgctgctcagaggagaggacgtgtaggcaggaaccccaacaaacctggagatgagtacatgtatggaggtgggtgtgcagagactgatgaaga

SEQ ID NO: 3749 - DNA, 120 bp, synthetic construct
  source 1..120: mol_type = other DNA
ccccaacaaacctggagatgagtacatgtatggaggtgggtgtgcagagactgatgaagaccatgcacactggcttgaagcaagaatgcttcttgacaacatttacctccaggatggcct

SEQ ID NO: 3750 - DNA, 120 bp, synthetic construct
  source 1..120: mol_type = other DNA
ccatgcacactggcttgaagcaagaatgcttcttgacaacatttacctccaggatggcctcatagcctcgctctatcggcctgaggccgacaaggtagccgccattgagggagagttcaa

SEQ ID NO: 3751 - DNA, 120 bp, synthetic construct
  source 1..120: mol_type = other DNA
catagcctcgctctatcggcctgaggccgacaaggtagccgccattgagggagagttcaagctgaggacagagcaaaggaagacctttgtggaactcatgaagagaggagaccttcccgt

SEQ ID NO: 3752 - DNA, 120 bp, synthetic construct
  source 1..120: mol_type = other DNA
gctgaggacagagcaaaggaagacctttgtggaactcatgaagagaggagaccttcccgtttggctggcctatcaagtagcatctgccggaataacttacacagatagaagatggtgctt

SEQ ID NO: 3753 - DNA, 120 bp, synthetic construct
  source 1..120: mol_type = other DNA
ttggctggcctatcaagtagcatctgccggaataacttacacagatagaagatggtgctttgatggcactaccaacaacaccataatggaagacagtgtaccagcagaggtgtggaccaa

SEQ ID NO: 3754 - DNA, 120 bp, synthetic construct
  source 1..120: mol_type = other DNA
tgatggcactaccaacaacaccataatggaagacagtgtaccagcagaggtgtggaccaagtatggagagaagagagtgcttaaaccgaggtggatggatgctagggtctgttcagatca

SEQ ID NO: 3755 - DNA, 120 bp, synthetic construct
  source 1..120: mol_type = other DNA
gtatggagagaagagagtgcttaaaccgaggtggatggatgctagggtctgttcagatcatgcggctctgaagtcgttcaaagaatttgccgctgggaagagaggagcggctttgggagt

SEQ ID NO: 3756 - DNA, 120 bp, synthetic construct
  source 1..120: mol_type = other DNA
tgcggctctgaagtcgttcaaagaatttgccgctgggaagagaggagcggctttgggagtaatggatgccctgggaacattgccaggacacatgacagagaggtttcaggaagccattga

SEQ ID NO: 3757 - DNA, 120 bp, synthetic construct
  source 1..120: mol_type = other DNA
aatggatgccctgggaacattgccaggacacatgacagagaggtttcaggaagccattgacaatctcgctgtgctcatgcgagcagagactggaagtaggccctacaaagcagcggcagc

SEQ ID NO: 3758 - DNA, 120 bp, synthetic construct
  source 1..120: mol_type = other DNA
caatctcgctgtgctcatgcgagcagagactggaagtaggccctacaaagcagcggcagctcaactgccggagaccttagagactatcatgcttctgggcttattgggaacagtttcgct

SEQ ID NO: 3759 - DNA, 120 bp, synthetic construct
  source 1..120: mol_type = other DNA
tcaactgccggagaccttagagactatcatgcttctgggcttattgggaacagtttcgctaggaatcttctttgtcttgatgcggaacaagggcatcgggaagatgggcttcggaatggt

SEQ ID NO: 3760 - DNA, 120 bp, synthetic construct
  source 1..120: mol_type = other DNA
aggaatcttctttgtcttgatgcggaacaagggcatcgggaagatgggcttcggaatggtaacccttggggccagcgcatggctcatgtggctttcggaaattgaaccagccagaatcgc

SEQ ID NO: 3761 - DNA, 120 bp, synthetic construct
  source 1..120: mol_type = other DNA
aacccttggggccagcgcatggctcatgtggctttcggaaattgaaccagccagaatcgcatgtgtcctcattgtcgtgtttttgttgctggtggtgctcatacccgagccagagaagca

SEQ ID NO: 3762 - DNA, 120 bp, synthetic construct
  source 1..120: mol_type = other DNA
atgtgtcctcattgtcgtgtttttgttgctggtggtgctcatacccgagccagagaagcaaagatctccccaggataatcaaatggcaatcatcatcatggtggcagttggccttctggg

SEQ ID NO: 3763 - DNA, 120 bp, synthetic construct
  source 1..120: mol_type = other DNA
aagatctccccaggataatcaaatggcaatcatcatcatggtggcagttggccttctgggtttgataactgcaaatgaactcggatggctggaaaggacaaaaagtgatatagctcatct

SEQ ID NO: 3764 - DNA, 120 bp, synthetic construct
  source 1..120: mol_type = other DNA
tttgataactgcaaatgaactcggatggctggaaaggacaaaaagtgatatagctcatctaatgagaaggaaagaagaggggacaaccatgggattctcaatggatattgatctgcggcc

SEQ ID NO: 3765 - DNA, 120 bp, synthetic construct
  source 1..120: mol_type = other DNA
aatgagaaggaaagaagaggggacaaccatgggattctcaatggatattgatctgcggccagcctccgcctgggctatttatgccgcattgacaactctcatcaccccagccgtccaaca

SEQ ID NO: 3766 - DNA, 120 bp, synthetic construct
  source 1..120: mol_type = other DNA
agcctccgcctgggctatttatgccgcattgacaactctcatcaccccagccgtccaacatgcggtaaccacctcatacaacaactactccctgatggcgatggccacacaagctggagt

SEQ ID NO: 3767 - DNA, 120 bp, synthetic construct
  source 1..120: mol_type = other DNA
tgcggtaaccacctcatacaacaactactccctgatggcgatggccacacaagctggagtgctgtttggcatgggcaaagggatgccattttatgcatgggactttggagtcccgctgct

SEQ ID NO: 3768 - DNA, 120 bp, synthetic construct
  source 1..120: mol_type = other DNA
gctgtttggcatgggcaaagggatgccattttatgcatgggactttggagtcccgctgctaatgatgggttgctactcacaattaacacccctgaccctgatagtggccatcattctgct

SEQ ID NO: 3769 - DNA, 120 bp, synthetic construct
  source 1..120: mol_type = other DNA
aatgatgggttgctactcacaattaacacccctgaccctgatagtggccatcattctgcttgtggcacactacatgtacttgatcccaggtttgcaggcagcagcagcacgtgctgccca

SEQ ID NO: 3770 - DNA, 120 bp, synthetic construct
  source 1..120: mol_type = other DNA
tgtggcacactacatgtacttgatcccaggtttgcaggcagcagcagcacgtgctgcccagaagaggacagcagctggcatcatgaagaatcccgttgtggatggaatagtggtgactga

SEQ ID NO: 3771 - DNA, 120 bp, synthetic construct
  source 1..120: mol_type = other DNA
gaagaggacagcagctggcatcatgaagaatcccgttgtggatggaatagtggtgactgacattgacacaatgacaattgacccccaagtggagaagaagatgggacaagtgttactcat

SEQ ID NO: 3772 - DNA, 120 bp, synthetic construct
  source 1..120: mol_type = other DNA
cattgacacaatgacaattgacccccaagtggagaagaagatgggacaagtgttactcatagcagtagctgtctccagtgctgtgctactgcggaccgcttggggatggggggaggctgg

SEQ ID NO: 3773 - DNA, 120 bp, synthetic construct
  source 1..120: mol_type = other DNA
agcagtagctgtctccagtgctgtgctactgcggaccgcttggggatggggggaggctggggctctgatcacagcagcaacctccaccttatgggaaggctctccaaacaaatactggaa

SEQ ID NO: 3774 - DNA, 120 bp, synthetic construct
  source 1..120: mol_type = other DNA
ggctctgatcacagcagcaacctccaccttatgggaaggctctccaaacaaatactggaactcctccacagccacctcactgtgcaacatctttagaggaagttatttggcaggggcttc

SEQ ID NO: 3775 - DNA, 120 bp, synthetic construct
  source 1..120: mol_type = other DNA
ctcctccacagccacctcactgtgcaacatctttagaggaagttatttggcaggggcttcccttatttacacagtgacaagaaatgccggtctggttaagagacgtggaggtggaacggg

SEQ ID NO: 3776 - DNA, 120 bp, synthetic construct
  source 1..120: mol_type = other DNA
ccttatttacacagtgacaagaaatgccggtctggttaagagacgtggaggtggaacgggagagaccctgggagagaagtggaaagcccgcctgaaccagatgtcggccttggagttcta

SEQ ID NO: 3777 - DNA, 120 bp, synthetic construct
  source 1..120: mol_type = other DNA
agagaccctgggagagaagtggaaagcccgcctgaaccagatgtcggccttggagttctactcttacaaaaagtcaggcatcaccgaagtgtgtagggaggaggcgcgccgcgccctcaa

SEQ ID NO: 3778 - DNA, 120 bp, synthetic construct
  source 1..120: mol_type = other DNA
ctcttacaaaaagtcaggcatcaccgaagtgtgtagggaggaggcgcgccgcgccctcaaggatggagtggccacaggaggacatgctgtatcccggggaagcgcaaagcttagatggtt

SEQ ID NO: 3779 - DNA, 120 bp, synthetic construct
  source 1..120: mol_type = other DNA
ggatggagtggccacaggaggacatgctgtatcccggggaagcgcaaagcttagatggttggtagagagaggatacctgcagccccatggaaaggttgttgaccttggatgtggcagagg

SEQ ID NO: 3780 - DNA, 120 bp, synthetic construct
  source 1..120: mol_type = other DNA
ggtagagagaggatacctgcagccccatggaaaggttgttgaccttggatgtggcagaggaggctggagttattacgctgccaccatccgtaaagtgcaggaggtcagaggatacacaaa

SEQ ID NO: 3781 - DNA, 120 bp, synthetic construct
  source 1..120: mol_type = other DNA
aggctggagttattacgctgccaccatccgtaaagtgcaggaggtcagaggatacacaaagggaggtcctggccatgaagagcccatgctggtgcaaagctatgggtggaacatagttcg

SEQ ID NO: 3782 - DNA, 120 bp, synthetic construct
  source 1..120: mol_type = other DNA
gggaggtcctggccatgaagagcccatgctggtgcaaagctatgggtggaacatagttcgcctcaagagtggagtggacgtcttccacatggcggctgaaccgtgtgacactctgctgtg

SEQ ID NO: 3783 - DNA, 120 bp, synthetic construct
  source 1..120: mol_type = other DNA
cctcaagagtggagtggacgtcttccacatggcggctgaaccgtgtgacactctgctgtgtgacataggcgagtcatcatccagtcctgaagtggaagagacgcgaacactcagagtgct

SEQ ID NO: 3784 - DNA, 120 bp, synthetic construct
  source 1..120: mol_type = other DNA
tgacataggcgagtcatcatccagtcctgaagtggaagagacgcgaacactcagagtgctctccatggtgggagactggcttgaaaaaagaccaggggccttctgcataaaggtgctgtg

SEQ ID NO: 3785 - DNA, 120 bp, synthetic construct
  source 1..120: mol_type = other DNA
ctccatggtgggagactggcttgaaaaaagaccaggggccttctgcataaaggtgctgtgcccatacaccagcacaatgatggagaccatggagcgactgcaacgtaggcatgggggagg

SEQ ID NO: 3786 - DNA, 120 bp, synthetic construct
  source 1..120: mol_type = other DNA
cccatacaccagcacaatgatggagaccatggagcgactgcaacgtaggcatgggggaggattagtcagagtgccattgtcccgcaactctacacatgagatgtattgggtctctggagc

SEQ ID NO: 3787 - DNA, 120 bp, synthetic construct
  source 1..120: mol_type = other DNA
attagtcagagtgccattgtcccgcaactctacacatgagatgtattgggtctctggagccaaaagtaacatcataaagagtgtgtccaccacaagtcagctcctcttgggacgcatgga

SEQ ID NO: 3788 - DNA, 120 bp, synthetic construct
  source 1..120: mol_type = other DNA
caaaagtaacatcataaagagtgtgtccaccacaagtcagctcctcttgggacgcatggaagggcctaggaggccagtgaaatatgaggaggatgtgaacctcggctcaggcacacgagc

SEQ ID NO: 3789 - DNA, 120 bp, synthetic construct
  source 1..120: mol_type = other DNA
agggcctaggaggccagtgaaatatgaggaggatgtgaacctcggctcaggcacacgagctgtggcaagctgcgctgaggctcccaacatgaagatcattggtaggcgcattgagagaat

SEQ ID NO: 3790 - DNA, 120 bp, synthetic construct
  source 1..120: mol_type = other DNA
tgtggcaagctgcgctgaggctcccaacatgaagatcattggtaggcgcattgagagaatccgcaatgaacatgcagagacatggttctttgatgaaaaccacccatacaggacatgggc

SEQ ID NO: 3791 - DNA, 120 bp, synthetic construct
  source 1..120: mol_type = other DNA
ccgcaatgaacatgcagagacatggttctttgatgaaaaccacccatacaggacatgggcctaccatgggagctacgaagcccccacgcaggggtcagcgtcatccctcgtgaacggggt

SEQ ID NO: 3792 - DNA, 120 bp, synthetic construct
  source 1..120: mol_type = other DNA
ctaccatgggagctacgaagcccccacgcaggggtcagcgtcatccctcgtgaacggggttgttagactcttgtcaaagccctgggatgtggtgactggagttacaggaatagctatgac

SEQ ID NO: 3793 - DNA, 120 bp, synthetic construct
  source 1..120: mol_type = other DNA
tgttagactcttgtcaaagccctgggatgtggtgactggagttacaggaatagctatgactgacaccacgccatacggccaacaaagagtcttcaaggaaaaagtggacaccagggtgcc

SEQ ID NO: 3794 - DNA, 120 bp, synthetic construct
  source 1..120: mol_type = other DNA
tgacaccacgccatacggccaacaaagagtcttcaaggaaaaagtggacaccagggtgccagatccccaagaaggcactcgccaagtgatgaacatggtatcgtcttggctatggaagga

SEQ ID NO: 3795 - DNA, 120 bp, synthetic construct
  source 1..120: mol_type = other DNA
agatccccaagaaggcactcgccaagtgatgaacatggtatcgtcttggctatggaaggagctgggaaaacgcaagcgaccacgtgtctgcaccaaagaagagttcattaataaggtgcg

SEQ ID NO: 3796 - DNA, 120 bp, synthetic construct
  source 1..120: mol_type = other DNA
gctgggaaaacgcaagcgaccacgtgtctgcaccaaagaagagttcattaataaggtgcgcagcaatgcagcactgggagcaatatttgaagaggaaaaagaatggaagacagctgtaga

SEQ ID NO: 3797 - DNA, 120 bp, synthetic construct
  source 1..120: mol_type = other DNA
cagcaatgcagcactgggagcaatatttgaagaggaaaaagaatggaagacagctgtagaagctgtgaatgatccaagattttgggctctagtggacaaggaaagagaacaccacctgag

SEQ ID NO: 3798 - DNA, 120 bp, synthetic construct
  source 1..120: mol_type = other DNA
agctgtgaatgatccaagattttgggctctagtggacaaggaaagagaacaccacctgagaggagagtgtcatagctgtgtgtacaacatgatgggcaaaagagaaaagaagcaaggaga

SEQ ID NO: 3799 - DNA, 120 bp, synthetic construct
  source 1..120: mol_type = other DNA
aggagagtgtcatagctgtgtgtacaacatgatgggcaaaagagaaaagaagcaaggagaattcgggaaagcaaaaggcagccgcgcaatctggtacatgtggttgggagccagattttt

SEQ ID NO: 3800 - DNA, 120 bp, synthetic construct
  source 1..120: mol_type = other DNA
attcgggaaagcaaaaggcagccgcgcaatctggtacatgtggttgggagccagatttttggagtttgaagctcttgggttcttgaacgaggaccactggatggggagagaaaactcagg

SEQ ID NO: 3801 - DNA, 120 bp, synthetic construct
  source 1..120: mol_type = other DNA
ggagtttgaagctcttgggttcttgaacgaggaccactggatggggagagaaaactcaggaggtggcgttgaagggctaggactgcaaaggcttggatatatcctagaagaaatgaaccg

SEQ ID NO: 3802 - DNA, 120 bp, synthetic construct
  source 1..120: mol_type = other DNA
aggtggcgttgaagggctaggactgcaaaggcttggatatatcctagaagaaatgaaccgggcaccaggaggaaagatgtatgcagatgacactgctggctgggacacccgcattagcaa

SEQ ID NO: 3803 - DNA, 120 bp, synthetic construct
  source 1..120: mol_type = other DNA
ggcaccaggaggaaagatgtatgcagatgacactgctggctgggacacccgcattagcaagtttgatctagagaatgaagccctgatcactaaccagatggaagaagggcacagagctct

SEQ ID NO: 3804 - DNA, 120 bp, synthetic construct
  source 1..120: mol_type = other DNA
gtttgatctagagaatgaagccctgatcactaaccagatggaagaagggcacagagctctggcgttggccgtgattaaatacacataccaaaacaaagtggtgaaggttctcagaccagc

SEQ ID NO: 3805 - DNA, 120 bp, synthetic construct
  source 1..120: mol_type = other DNA
ggcgttggccgtgattaaatacacataccaaaacaaagtggtgaaggttctcagaccagctgaaggagggaaaacagtcatggacatcatctcaagacaagaccagagagggagcggaca

SEQ ID NO: 3806 - DNA, 120 bp, synthetic construct
  source 1..120: mol_type = other DNA
tgaaggagggaaaacagtcatggacatcatctcaagacaagaccagagagggagcggacaagttgttacttatgctctcaacacattcaccaacctggtggtgcagcttatccggaacat

SEQ ID NO: 3807 - DNA, 120 bp, synthetic construct
  source 1..120: mol_type = other DNA
agttgttacttatgctctcaacacattcaccaacctggtggtgcagcttatccggaacatggaggctgaggaagtgctagagatgcatgatctgtggttgttgaggaagccagagaaagt

SEQ ID NO: 3808 - DNA, 120 bp, synthetic construct
  source 1..120: mol_type = other DNA
ggaggctgaggaagtgctagagatgcatgatctgtggttgttgaggaagccagagaaagtgaccagatggttgcagagcaatggatgggacagactcaaacggatggcagttagtggaga

SEQ ID NO: 3809 - DNA, 120 bp, synthetic construct
  source 1..120: mol_type = other DNA
gaccagatggttgcagagcaatggatgggacagactcaaacggatggcagttagtggagatgactgcgttgtaaagccaattgatgataggtttgcacatgccctcaggttcttgaatga

SEQ ID NO: 3810 - DNA, 120 bp, synthetic construct
  source 1..120: mol_type = other DNA
tgactgcgttgtaaagccaattgatgataggtttgcacatgccctcaggttcttgaatgacatgggaaaggttaggaaagacacacaggaatggaaaccctcgactggatggagcaattg

SEQ ID NO: 3811 - DNA, 120 bp, synthetic construct
  source 1..120: mol_type = other DNA
catgggaaaggttaggaaagacacacaggaatggaaaccctcgactggatggagcaattgggaagaggtcccgttctgttctcaccacttcaacaagctgcacctcaaggacgggagatc

SEQ ID NO: 3812 - DNA, 120 bp, synthetic construct
  source 1..120: mol_type = other DNA
ggaagaggtcccgttctgttctcaccacttcaacaagctgcacctcaaggacgggagatccattgtggtcccctgccgccaccaagatgaactgattggccgagcccgtgtctcaccagg

SEQ ID NO: 3813 - DNA, 120 bp, synthetic construct
  source 1..120: mol_type = other DNA
cattgtggtcccctgccgccaccaagatgaactgattggccgagcccgtgtctcaccaggggcaggatggagcatccgggagactgcttgtcttgcaaaatcatatgcacagatgtggca

SEQ ID NO: 3814 - DNA, 120 bp, synthetic construct
  source 1..120: mol_type = other DNA
ggcaggatggagcatccgggagactgcttgtcttgcaaaatcatatgcacagatgtggcagcttctttatttccacagaagagacctccgactgatggccaatgccatttgttcggctgt

SEQ ID NO: 3815 - DNA, 120 bp, synthetic construct
  source 1..120: mol_type = other DNA
gcttctttatttccacagaagagacctccgactgatggccaatgccatttgttcggctgtgccaattgactgggtaccaactgggagaaccacctggtcaatccatggaaagggagaatg

SEQ ID NO: 3816 - DNA, 120 bp, synthetic construct
  source 1..120: mol_type = other DNA
gccaattgactgggtaccaactgggagaaccacctggtcaatccatggaaagggagaatggatgactactgaggacatgctcatggtgtggaatagagtgtggattgaggagaacgacca

SEQ ID NO: 3817 - DNA, 120 bp, synthetic construct
  source 1..120: mol_type = other DNA
gatgactactgaggacatgctcatggtgtggaatagagtgtggattgaggagaacgaccacatggaggacaagacccctgtaacaaaatggacagacattccctatttgggaaaaaggga

SEQ ID NO: 3818 - DNA, 120 bp, synthetic construct
  source 1..120: mol_type = other DNA
catggaggacaagacccctgtaacaaaatggacagacattccctatttgggaaaaagggaggacttatggtgtggatcccttatagggcatagacctcgcaccacttgggctgagaacat

SEQ ID NO: 3819 - DNA, 120 bp, synthetic construct
  source 1..120: mol_type = other DNA
ggacttatggtgtggatcccttatagggcatagacctcgcaccacttgggctgagaacatcaaagacacagtcaacatggtgcgtaggatcataggtgatgaagaaaagttcatggacta

SEQ ID NO: 3820 - DNA, 120 bp, synthetic construct
  source 1..120: mol_type = other DNA
caaagacacagtcaacatggtgcgtaggatcataggtgatgaagaaaagttcatggactacctatccacccaagtacgctacttgggtgaggaagggtccacacctggagtgctgtaagc

SEQ ID NO: 3821 - DNA, 120 bp, synthetic construct
  source 1..120: mol_type = other DNA
cctatccacccaagtacgctacttgggtgaggaagggtccacacctggagtgctgtaagcatcaatttcaatgttgtcaggcctgctagtcagccacagtttggggaaagctgtgcagcc

SEQ ID NO: 3822 - DNA, 120 bp, synthetic construct
  source 1..120: mol_type = other DNA
atcaatttcaatgttgtcaggcctgctagtcagccacagtttggggaaagctgtgcagcctgtaacccccccaggagaagctgggaaaccaagctcatagtcaggccgataacgccatgg

SEQ ID NO: 3823 - DNA, 120 bp, synthetic construct
  source 1..120: mol_type = other DNA
tgtaacccccccaggagaagctgggaaaccaagctcatagtcaggccgataacgccatggcacggaaaaagccatgctgcctgtgagcccctcagaggacactgagtcaaaaaaccccac

SEQ ID NO: 3824 - DNA, 120 bp, synthetic construct
  source 1..120: mol_type = other DNA
cacggaaaaagccatgctgcctgtgagcccctcagaggacactgagtcaaaaaaccccacgcgcttggaagcgcaggatgggaaaagaaggtggcgaccttccccaccctttaatctggg

SEQ ID NO: 3825 - DNA, 120 bp, synthetic construct
  source 1..120: mol_type = other DNA
gcgcttggaagcgcaggatgggaaaagaaggtggcgaccttccccaccctttaatctggggcctgaactggagattagctgtgaatctccggcagaaggactagtggttagaggagaccc

SEQ ID NO: 3826 - DNA, 120 bp, synthetic construct
  source 1..120: mol_type = other DNA
gcctgaactggagattagctgtgaatctccggcagaaggactagtggttagaggagaccccccggaaaacgcaaaacagcatattgacgctgggaaagaccagagactccatgagtttcc

SEQ ID NO: 3827 - DNA, 120 bp, synthetic construct
  source 1..120: mol_type = other DNA
cccggaaaacgcaaaacagcatattgacgctgggaaagaccagagactccatgagtttccaccacgctggccgccaggcacagatcgccgaacagcggcggccggtgtggggaaatccat

SEQ ID NO: 3828 - DNA, 120 bp, synthetic construct
  source 1..120: mol_type = other DNA
aaacgcaaaacagcatattgacgctgggaaagaccagagactccatgagtttccaccacgctggccgccaggcacagatcgccgaacagcggcggccggtgtggggaaatccatgggtct